European Patent Application EP 4 649 951 A2, published November 19, 2025. Title: SIRNA COMPOSITIONS AND METHODS FOR SILENCING GPAM (GLYCEROL-3-PHOSPHATE ACYLTRANSFERASE 1, MITOCHONDRIAL) EXPRESSION. Applicant: ALNYLAM PHARMACEUTICALS, INC. Application US PCT/US2021/036643, filed June 9, 2021. The sequence listing filed with the application follows.

SEQUENCE LISTING (754 sequences)

SEQ ID NO: 1 - RNA, 6372 nt, Homo sapiens
  source 1..6372: mol_type = mRNA
gcgccactgcagctggcattggccgggactggaagtgcgggcttctgcagcagccgaagctggagctgctagggcagcagcggctcccctgttgtatggacattctgcacccgaaactgatagctgagtcctgaagttttatgttatgaaacagaagaactttcatcccagcacatgatttgggaattacactttgtgacatggatgaatctgcactgacccttggtacaatagatgtttcttatctgccacattcatcagaatacagtgttggtcgatgtaagcacacaagtgaggaatggggtgagtgtggctttagacccaccatcttcagatctgcaactttaaaatggaaagaaagcctaatgagtcggaaaaggccatttgttggaagatgttgttactcctgcactccccagagctgggacaaatttttcaaccccagtatcccgtctttgggtttgcggaatgttatttatatcaatgaaactcacacaagacaccgcggatggcttgcaagacgcctttcttacgttctttttattcaagagcgagatgtgcataagggcatgtttgccaccaatgtgactgaaaatgtgctgaacagcagtagagtacaagaggcaattgcagaagtggctgctgaattaaaccctgatggttctgcccagcagcaatcaaaagccgttaacaaagtgaaaaagaaagctaaaaggattcttcaagaaatggttgccactgtctcaccggcaatgatcagactgactgggtgggtgctgctaaaactgttcaacagcttcttttggaacattcaaattcacaaaggtcaacttgagatggttaaagctgcaactgagacgaatttgccgcttctgtttctaccagttcatagatcccatattgactatctgctgctcactttcattctcttctgccataacatcaaagcaccatacattgcttcaggcaataatctcaacatcccaatcttcagtaccttgatccataagcttgggggcttcttcatacgacgaaggctcgatgaaacaccagatggacggaaagatgttctctatagagctttgctccatgggcatatagttgaattacttcgacagcagcaattcttggagatcttcctggaaggcacacgttctaggagtggaaaaacctcttgtgctcgggcaggacttttgtcagttgtggtagatactctgtctaccaatgtcatcccagacatcttgataatacctgttggaatctcctatgatcgcattatcgaaggtcactacaatggtgaacaactgggcaaacctaagaagaatgagagcctgtggagtgtagcaagaggtgttattagaatgttacgaaaaaactatggttgtgtccgagtggattttgcacagccattttccttaaaggaatatttagaaagccaaagtcagaaaccggtgtctgctctactttccctggagcaagcgttgttaccagctatacttccttcaagacccagtgatgctgctgatgaaggtagagacacgtccattaatgagtccagaaatgcaacagatgaatccctacgaaggaggttgattgcaaatctggctgagcatattctattcactgctagcaagtcctgtgccattatgtccacacacattgtggcttgcctgctcctctacagacacaggcagggaattgatctctccacattggtcgaagacttctttgtgatgaaagaggaagtcctggctcgtgattttgacctggggttctcaggaaattcagaagatgtagtaatgcatgccatacagctgctgggaaattgtgtcacaatcacccacactagcaggaacgatgagttttttatcacccccagcacaactgtcccatcagtcttcgaactcaacttctacagcaatggggtacttcatgtctttatcatggaggccatcatagcttgcagcctttatgcagttctgaacaagaggggactggggggtcccactagcaccccacctaacctgatcagccaggagcagctggtgcggaaggcggccagcctgtgctaccttctctccaatgaaggcaccatctcactgccttgccagacattttaccaagtctgccatgaaacagtaggaaagtttatccagtatggcattcttacagtggcagagcacgatgaccaggaagatatcagtcctagtcttgctgagcagcagtgggacaagaagcttccagaacctttgtcttggagaagtgatgaagaagatgaagacagtgactttggggaggaacagcgagattgctacctgaaggtgagccaatccaaggagcaccagcagtttatcaccttcttacagagactccttgggcctttgctggaggcctacagctctgctgccatctttgttcacaacttcagtggtcctgttccagaacctgagtatctgcaaaagttgcacaaatacctaataaccagaacagaaagaaatgttgcagtatatgctgagagtgccacatattgtcttgtgaagaatgctgtgaaaatgtttaaggatattggggttttcaaggagaccaaacaaaagagagtgtctgttttagaactgagcagcacttttctacctcaatgcaaccgacaaaaacttctagaatatattctgagttttgtggtgctgtaggtaacgtgtggcactgctggcaaatgaaggtcatgagatgagttccttgtaggtaccagcttctggctcaagagttgaaggtgccatcgcagggtcaggcctgccctgtcccgaagtgatctcctggaagacaagtgccttctccctccatggatctgtgatcttcccagctctgcatcaacacagcagcctgcagataacacttggggggacctcagcctctattcgcaactcataatccgtagactacaagatgaaatctcaataaattatttttgagtttattaaagattgacattttaagtacaacttttaaggactaattactgtgatggacacagaaatgtagctgtgttctggaactgaatcttacatggtatacttagtgctgctgggtaatttgttggtatattatctggttagtggttaatgcttcctttaaaaataattgagtcatccattcactctttttcagttttatctgtcaatagtagctacatttttaatgggagcaccttttatcccaaagtgctttataaattgagtggactgatatatatcacacccaggtatcactgtgctgtcctttgctgtcagatttagaaatgtttttaagagctatgtgaaaacagacaatattagtttaggtcgggaactgagatattgtaatcaaatagttaacatcaggaagttaatttggctggcaaaattctagggaaacttggccagaaaactggtgttgaaggcttttgctcatataaacaagtgccattgagtttcaaatgaccagcaaatatatttagaacccttcctgttttatgtctgtacctcgtccacccctcaggtaatacctgcctctcacaggtacagctgtttcttggaaatcctccaaccaaatagcagttttcctaacttgattagcttgagctgacagactgttagaatacagttctctggccacagctgatgagggctttctgtactgcacacagattgtgtactgcaccccagtccaggtgactggtacccactcgagttgtgccgtgcacaacctgtccagtatatgcatgtggtggccctactgactggtaatggttagaggcatttatggatttttagctttgaggaaaaaccatgacttttaacaaatttttatgggttatatgcctaaacccttatgccacatagtggtaaataattatgaaaaatggtctgttcataattggtaggtgccttttgtgagcagggagcataattattggtttattatggtaattatggtgattttttaaatatcatgtaatgttaaaacgttttctaacagtttactgttgcttatctccaagatattatggaattaagaatttttccagatgagtgttacatagattctttgaatttagtataaaagtactgagaattaagtttgtacttccataagcttggattttaaacactgatagtatctcatgagtaatgtgtgttttgggagagggagggatgctgattgatatttcacattgtatgaaataccatgtttgaaactcatagcaataatgctatgctgttgtgatccctctcaagttctgcatttaaaatatattttttctttataggaattgatgtataccatgaagtcattgtcagttgtagtagctctgatgttgaatgagatatcatgttttagcattccattttactgactagggtagaagaacacttttcttggctacatttggaggatacccagggagtcttgggtgttccttatctggggaagcaaacatttcactagtctctttttttcatcctttaaattgtaaattaaggattactcaagctcaccattattcaagattgggactcgcttcccagtcgacactctgccctgcctgtcattgctgcaaagagctgctgctttgccaacctaagcaaagaaaatacggcttctcttgcattattttcccttttggttggtttgttttctagaagtacgttcagatgctttggggaatgcaatgtatgatttgctagctctctcaccacttaactcactgtgaggataaatatgcatgctttttgtaattaactggtgctttgaaaatcttttttaagggagaaaaatctcaaccaaagttatgctcatccagacaagctgacctttgagttaatttcagcacaactcattcttcagtgcctcatgactgaaaacaaaaaacaaaaaaacgaaagcatcttcacaatgaagcttccagatagcaccgttttgctaaaagatacattctcattgttttccaacagtgatggcttccacataaggttaaacaaactaggtgcttgtaaataatttattacagtttactctatcgcatttctgtaacatgaaatgcatgcccttcttcaggggaagactgtggtcaagttaaaaaaaaaaaacaatattaaacaacatgaaactgcagtctgtttttgaaaatgagaatgtcctaagtgattcagaagagaggagggaagttgtgcactctgaaaatgcatgaaaaacaaaggcaaaaactagtgggaaatgtgtagaactgttaactgagatggcttcgagtcttccttctggaatctgttaaatttcacaaagtcatgagggtaaatggagaaaatatttctgggattacaatgaatgtaagcccaaattgtggaattgccagtaacctggatggggaaaagcatttcccatagcactccatgtaatatgagtgctctgtgagatgttcatcagtgttttatagaaatggtgttgctgggaaaccaagtttgcacctggaaacttacaatgcactttagcgcagtaagggcttggcatccggtagtgaaaaactgtctaacccagcattgcccaaactattttgacaccaggacctttttctcctttgggatacttatgaacctctcactaatgtcctgtggagaacattttgggaaacactatgttagatagttctttaaggagacaaaacggtaatgaacagatagcactggggcagaatatgcatgcattttgtaacgtccagtgtggcgttgaatagatgtgtatttcctcccctgcagaaaataagcacagaaaattataatgtaggtgatcggagctctttcctttgatagagagaacagccccaatgatcctggctttttcactgaacgtatcagaatacatggatgaattggggtaaataaggttttaattcagatctagaagaaagtattgtacgtttgaatgcagatttttatccacagatagttgtagtgtttagacatgacaggacctatcgttgaggtttctaagacttactatgggctgtaaacctgttttttaaaactattttagaaacctgagacttgccgtctggcattttagtttaatacaaactaatgattgcatttgaaagagattcttgaccttatttctaaacgtctagagctctgaaatgtcttgatggaaggtattaaactatttgcctgttgtacaaagaaatgttaagactcgtgaaaagaattactataaggtactgtgaaataactgcgattttgtgagcaaaacatacttggaaatgctgattgatttttatgcttgttagtgtattgcaagaaacacagaaaatgtagttttgttttaataaaccaaaaattgaacata

SEQ ID NO: 2 - RNA, 6372 nt, Homo sapiens
  source 1..6372: mol_type = mRNA
tatgttcaatttttggtttattaaaacaaaactacattttctgtgtttcttgcaatacactaacaagcataaaaatcaatcagcatttccaagtatgttttgctcacaaaatcgcagttatttcacagtaccttatagtaattcttttcacgagtcttaacatttctttgtacaacaggcaaatagtttaataccttccatcaagacatttcagagctctagacgtttagaaataaggtcaagaatctctttcaaatgcaatcattagtttgtattaaactaaaatgccagacggcaagtctcaggtttctaaaatagttttaaaaaacaggtttacagcccatagtaagtcttagaaacctcaacgataggtcctgtcatgtctaaacactacaactatctgtggataaaaatctgcattcaaacgtacaatactttcttctagatctgaattaaaaccttatttaccccaattcatccatgtattctgatacgttcagtgaaaaagccaggatcattggggctgttctctctatcaaaggaaagagctccgatcacctacattataattttctgtgcttattttctgcaggggaggaaatacacatctattcaacgccacactggacgttacaaaatgcatgcatattctgccccagtgctatctgttcattaccgttttgtctccttaaagaactatctaacatagtgtttcccaaaatgttctccacaggacattagtgagaggttcataagtatcccaaaggagaaaaaggtcctggtgtcaaaatagtttgggcaatgctgggttagacagtttttcactaccggatgccaagcccttactgcgctaaagtgcattgtaagtttccaggtgcaaacttggtttcccagcaacaccatttctataaaacactgatgaacatctcacagagcactcatattacatggagtgctatgggaaatgcttttccccatccaggttactggcaattccacaatttgggcttacattcattgtaatcccagaaatattttctccatttaccctcatgactttgtgaaatttaacagattccagaaggaagactcgaagccatctcagttaacagttctacacatttcccactagtttttgcctttgtttttcatgcattttcagagtgcacaacttccctcctctcttctgaatcacttaggacattctcattttcaaaaacagactgcagtttcatgttgtttaatattgttttttttttttaacttgaccacagtcttcccctgaagaagggcatgcatttcatgttacagaaatgcgatagagtaaactgtaataaattatttacaagcacctagtttgtttaaccttatgtggaagccatcactgttggaaaacaatgagaatgtatcttttagcaaaacggtgctatctggaagcttcattgtgaagatgctttcgtttttttgttttttgttttcagtcatgaggcactgaagaatgagttgtgctgaaattaactcaaaggtcagcttgtctggatgagcataactttggttgagatttttctcccttaaaaaagattttcaaagcaccagttaattacaaaaagcatgcatatttatcctcacagtgagttaagtggtgagagagctagcaaatcatacattgcattccccaaagcatctgaacgtacttctagaaaacaaaccaaccaaaagggaaaataatgcaagagaagccgtattttctttgcttaggttggcaaagcagcagctctttgcagcaatgacaggcagggcagagtgtcgactgggaagcgagtcccaatcttgaataatggtgagcttgagtaatccttaatttacaatttaaaggatgaaaaaaagagactagtgaaatgtttgcttccccagataaggaacacccaagactccctgggtatcctccaaatgtagccaagaaaagtgttcttctaccctagtcagtaaaatggaatgctaaaacatgatatctcattcaacatcagagctactacaactgacaatgacttcatggtatacatcaattcctataaagaaaaaatatattttaaatgcagaacttgagagggatcacaacagcatagcattattgctatgagtttcaaacatggtatttcatacaatgtgaaatatcaatcagcatccctccctctcccaaaacacacattactcatgagatactatcagtgtttaaaatccaagcttatggaagtacaaacttaattctcagtacttttatactaaattcaaagaatctatgtaacactcatctggaaaaattcttaattccataatatcttggagataagcaacagtaaactgttagaaaacgttttaacattacatgatatttaaaaaatcaccataattaccataataaaccaataattatgctccctgctcacaaaaggcacctaccaattatgaacagaccatttttcataattatttaccactatgtggcataagggtttaggcatataacccataaaaatttgttaaaagtcatggtttttcctcaaagctaaaaatccataaatgcctctaaccattaccagtcagtagggccaccacatgcatatactggacaggttgtgcacggcacaactcgagtgggtaccagtcacctggactggggtgcagtacacaatctgtgtgcagtacagaaagccctcatcagctgtggccagagaactgtattctaacagtctgtcagctcaagctaatcaagttaggaaaactgctatttggttggaggatttccaagaaacagctgtacctgtgagaggcaggtattacctgaggggtggacgaggtacagacataaaacaggaagggttctaaatatatttgctggtcatttgaaactcaatggcacttgtttatatgagcaaaagccttcaacaccagttttctggccaagtttccctagaattttgccagccaaattaacttcctgatgttaactatttgattacaatatctcagttcccgacctaaactaatattgtctgttttcacatagctcttaaaaacatttctaaatctgacagcaaaggacagcacagtgatacctgggtgtgatatatatcagtccactcaatttataaagcactttgggataaaaggtgctcccattaaaaatgtagctactattgacagataaaactgaaaaagagtgaatggatgactcaattatttttaaaggaagcattaaccactaaccagataatataccaacaaattacccagcagcactaagtataccatgtaagattcagttccagaacacagctacatttctgtgtccatcacagtaattagtccttaaaagttgtacttaaaatgtcaatctttaataaactcaaaaataatttattgagatttcatcttgtagtctacggattatgagttgcgaatagaggctgaggtccccccaagtgttatctgcaggctgctgtgttgatgcagagctgggaagatcacagatccatggagggagaaggcacttgtcttccaggagatcacttcgggacagggcaggcctgaccctgcgatggcaccttcaactcttgagccagaagctggtacctacaaggaactcatctcatgaccttcatttgccagcagtgccacacgttacctacagcaccacaaaactcagaatatattctagaagtttttgtcggttgcattgaggtagaaaagtgctgctcagttctaaaacagacactctcttttgtttggtctccttgaaaaccccaatatccttaaacattttcacagcattcttcacaagacaatatgtggcactctcagcatatactgcaacatttctttctgttctggttattaggtatttgtgcaacttttgcagatactcaggttctggaacaggaccactgaagttgtgaacaaagatggcagcagagctgtaggcctccagcaaaggcccaaggagtctctgtaagaaggtgataaactgctggtgctccttggattggctcaccttcaggtagcaatctcgctgttcctccccaaagtcactgtcttcatcttcttcatcacttctccaagacaaaggttctggaagcttcttgtcccactgctgctcagcaagactaggactgatatcttcctggtcatcgtgctctgccactgtaagaatgccatactggataaactttcctactgtttcatggcagacttggtaaaatgtctggcaaggcagtgagatggtgccttcattggagagaaggtagcacaggctggccgccttccgcaccagctgctcctggctgatcaggttaggtggggtgctagtgggaccccccagtcccctcttgttcagaactgcataaaggctgcaagctatgatggcctccatgataaagacatgaagtaccccattgctgtagaagttgagttcgaagactgatgggacagttgtgctgggggtgataaaaaactcatcgttcctgctagtgtgggtgattgtgacacaatttcccagcagctgtatggcatgcattactacatcttctgaatttcctgagaaccccaggtcaaaatcacgagccaggacttcctctttcatcacaaagaagtcttcgaccaatgtggagagatcaattccctgcctgtgtctgtagaggagcaggcaagccacaatgtgtgtggacataatggcacaggacttgctagcagtgaatagaatatgctcagccagatttgcaatcaacctccttcgtagggattcatctgttgcatttctggactcattaatggacgtgtctctaccttcatcagcagcatcactgggtcttgaaggaagtatagctggtaacaacgcttgctccagggaaagtagagcagacaccggtttctgactttggctttctaaatattcctttaaggaaaatggctgtgcaaaatccactcggacacaaccatagttttttcgtaacattctaataacacctcttgctacactccacaggctctcattcttcttaggtttgcccagttgttcaccattgtagtgaccttcgataatgcgatcataggagattccaacaggtattatcaagatgtctgggatgacattggtagacagagtatctaccacaactgacaaaagtcctgcccgagcacaagaggtttttccactcctagaacgtgtgccttccaggaagatctccaagaattgctgctgtcgaagtaattcaactatatgcccatggagcaaagctctatagagaacatctttccgtccatctggtgtttcatcgagccttcgtcgtatgaagaagcccccaagcttatggatcaaggtactgaagattgggatgttgagattattgcctgaagcaatgtatggtgctttgatgttatggcagaagagaatgaaagtgagcagcagatagtcaatatgggatctatgaactggtagaaacagaagcggcaaattcgtctcagttgcagctttaaccatctcaagttgacctttgtgaatttgaatgttccaaaagaagctgttgaacagttttagcagcacccacccagtcagtctgatcattgccggtgagacagtggcaaccatttcttgaagaatccttttagctttctttttcactttgttaacggcttttgattgctgctgggcagaaccatcagggtttaattcagcagccacttctgcaattgcctcttgtactctactgctgttcagcacattttcagtcacattggtggcaaacatgcccttatgcacatctcgctcttgaataaaaagaacgtaagaaaggcgtcttgcaagccatccgcggtgtcttgtgtgagtttcattgatataaataacattccgcaaacccaaagacgggatactggggttgaaaaatttgtcccagctctggggagtgcaggagtaacaacatcttccaacaaatggccttttccgactcattaggctttctttccattttaaagttgcagatctgaagatggtgggtctaaagccacactcaccccattcctcacttgtgtgcttacatcgaccaacactgtattctgatgaatgtggcagataagaaacatctattgtaccaagggtcagtgcagattcatccatgtcacaaagtgtaattcccaaatcatgtgctgggatgaaagttcttctgtttcataacataaaacttcaggactcagctatcagtttcgggtgcagaatgtccatacaacaggggagccgctgctgccctagcagctccagcttcggctgctgcagaagcccgcacttccagtcccggccaatgccagctgcagtggcgc

SEQ ID NO: 3 - RNA, 6368 nt, Homo sapiens
  source 1..6368: mol_type = mRNA
gcgccactgcagctggcattggccgggactggaagtgcgggcttctgcagcagccgaagctggagctgctaggcagcggctcccctgttgtatggacattctgcacccgaaactgatagctgagtcctgaagttttatgttatgaaacagaagaactttcatcccagcacatgatttgggaattacactttgtgacatggatgaatctgcactgacccttggtacaatagatgtttcttatctgccacattcatcagaatacagtgttggtcgatgtaagcacacaagtgaggaatggggtgagtgtggctttagacccaccatcttcagatctgcaactttaaaatggaaagaaagcctaatgagtcggaaaaggccatttgttggaagatgttgttactcctgcactccccagagctgggacaaatttttcaaccccagtatcccgtctttgggtttgcggaatgttatttatatcaatgaaactcacacaagacaccgcggatggcttgcaagacgcctttcttacgttctttttattcaagagcgagatgtgcataagggcatgtttgccaccaatgtgactgaaaatgtgctgaacagcagtagagtacaagaggcaattgcagaagtggctgctgaattaaaccctgatggttctgcccagcagcaatcaaaagccgttaacaaagtgaaaaagaaagctaaaaggattcttcaagaaatggttgccactgtctcaccggcaatgatcagactgactgggtgggtgctgctaaaactgttcaacagcttcttttggaacattcaaattcacaaaggtcaacttgagatggttaaagctgcaactgagacgaatttgccgcttctgtttctaccagttcatagatcccatattgactatctgctgctcactttcattctcttctgccataacatcaaagcaccatacattgcttcaggcaataatctcaacatcccaatcttcagtaccttgatccataagcttgggggcttcttcatacgacgaaggctcgatgaaacaccagatggacggaaagatgttctctatagagctttgctccatgggcatatagttgaattacttcgacagcagcaattcttggagatcttcctggaaggcacacgttctaggagtggaaaaacctcttgtgctcgggcaggacttttgtcagttgtggtagatactctgtctaccaatgtcatcccagacatcttgataatacctgttggaatctcctatgatcgcattatcgaaggtcactacaatggtgaacaactgggcaaacctaagaagaatgagagcctgtggagtgtagcaagaggtgttattagaatgttacgaaaaaactatggttgtgtccgagtggattttgcacagccattttccttaaaggaatatttagaaagccaaagtcagaaaccggtgtctgctctactttccctggagcaagcgttgttaccagctatacttccttcaagacccagtgatgctgctgatgaaggtagagacacgtccattaatgagtccagaaatgcaacagatgaatccctacgaaggaggttgattgcaaatctggctgagcatattctattcactgctagcaagtcctgtgccattatgtccacacacattgtggcttgcctgctcctctacagacacaggcagggaattgatctctccacattggtcgaagacttctttgtgatgaaagaggaagtcctggctcgtgattttgacctggggttctcaggaaattcagaagatgtagtaatgcatgccatacagctgctgggaaattgtgtcacaatcacccacactagcaggaacgatgagttttttatcacccccagcacaactgtcccatcagtcttcgaactcaacttctacagcaatggggtacttcatgtctttatcatggaggccatcatagcttgcagcctttatgcagttctgaacaagaggggactggggggtcccactagcaccccacctaacctgatcagccaggagcagctggtgcggaaggcggccagcctgtgctaccttctctccaatgaaggcaccatctcactgccttgccagacattttaccaagtctgccatgaaacagtaggaaagtttatccagtatggcattcttacagtggcagagcacgatgaccaggaagatatcagtcctagtcttgctgagcagcagtgggacaagaagcttccagaacctttgtcttggagaagtgatgaagaagatgaagacagtgactttggggaggaacagcgagattgctacctgaaggtgagccaatccaaggagcaccagcagtttatcaccttcttacagagactccttgggcctttgctggaggcctacagctctgctgccatctttgttcacaacttcagtggtcctgttccagaacctgagtatctgcaaaagttgcacaaatacctaataaccagaacagaaagaaatgttgcagtatatgctgagagtgccacatattgtcttgtgaagaatgctgtgaaaatgtttaaggatattggggttttcaaggagaccaaacaaaagagagtgtctgttttagaactgagcagcacttttctacctcaatgcaaccgacaaaaacttctagaatatattctgagttttgtggtgctgtaggtaacgtgtggcactgctggcaaatgaaggtcatgagatgagttccttgtaggtaccagcttctggctcaagagttgaaggtgccatcgcagggtcaggcctgccctgtcccgaagtgatctcctggaagacaagtgccttctccctccatggatctgtgatcttcccagctctgcatcaacacagcagcctgcagataacacttggggggacctcagcctctattcgcaactcataatccgtagactacaagatgaaatctcaataaattatttttgagtttattaaagattgacattttaagtacaacttttaaggactaattactgtgatggacacagaaatgtagctgtgttctggaactgaatcttacatggtatacttagtgctgctgggtaatttgttggtatattatctggttagtggttaatgcttcctttaaaaataattgagtcatccattcactctttttcagttttatctgtcaatagtagctacatttttaatgggagcaccttttatcccaaagtgctttataaattgagtggactgatatatatcacacccaggtatcactgtgctgtcctttgctgtcagatttagaaatgtttttaagagctatgtgaaaacagacaatattagtttaggtcgggaactgagatattgtaatcaaatagttaacatcaggaagttaatttggctggcaaaattctagggaaacttggccagaaaactggtgttgaaggcttttgctcatataaacaagtgccattgagtttcaaatgaccagcaaatatatttagaacccttcctgttttatgtctgtacctcgtccacccctcaggtaatacctgcctctcacaggtacagctgtttcttggaaatcctccaaccaaatagcagttttcctaacttgattagcttgagctgacagactgttagaatacagttctctggccacagctgatgagggctttctgtactgcacacagattgtgtactgcaccccagtccaggtgactggtacccactcgagttgtgccgtgcacaacctgtccagtatatgcatgtggtggccctactgactggtaatggttagaggcatttatggatttttagctttgaggaaaaaccatgacttttaacaaatttttatgggttatatgcctaaacccttatgccacatagtggtaaataattatgaaaaatggtctgttcataattggtaggtgccttttgtgagcagggagcataattattggtttattatggtaattatggtgattttttaaatatcatgtaatgttaaaacgttttctaacagtttactgttgcttatctccaagatattatggaattaagaatttttccagatgagtgttacatagattctttgaatttagtataaaagtactgagaattaagtttgtacttccataagcttggattttaaacactgatagtatctcatgagtaatgtgtgttttgggagagggagggatgctgattgatatttcacattgtatgaaataccatgtttgaaactcatagcaataatgctatgctgttgtgatccctctcaagttctgcatttaaaatatattttttctttataggaattgatgtataccatgaagtcattgtcagttgtagtagctctgatgttgaatgagatatcatgttttagcattccattttactgactagggtagaagaacacttttcttggctacatttggaggatacccagggagtcttgggtgttccttatctggggaagcaaacatttcactagtctctttttttcatcctttaaattgtaaattaaggattactcaagctcaccattattcaagattgggactcgcttcccagtcgacactctgccctgcctgtcattgctgcaaagagctgctgctttgccaacctaagcaaagaaaatacggcttctcttgcattattttcccttttggttggtttgttttctagaagtacgttcagatgctttggggaatgcaatgtatgatttgctagctctctcaccacttaactcactgtgaggataaatatgcatgctttttgtaattaactggtgctttgaaaatcttttttaagggagaaaaatctcaaccaaagttatgctcatccagacaagctgacctttgagttaatttcagcacaactcattcttcagtgcctcatgactgaaaacaaaaaacaaaaaaacgaaagcatcttcacaatgaagcttccagatagcaccgttttgctaaaagatacattctcattgttttccaacagtgatggcttccacataaggttaaacaaactaggtgcttgtaaataatttattacagtttactctatcgcatttctgtaacatgaaatgcatgcccttcttcaggggaagactgtggtcaagttaaaaaaaaaaaacaatattaaacaacatgaaactgcagtctgtttttgaaaatgagaatgtcctaagtgattcagaagagaggagggaagttgtgcactctgaaaatgcatgaaaaacaaaggcaaaaactagtgggaaatgtgtagaactgttaactgagatggcttcgagtcttccttctggaatctgttaaatttcacaaagtcatgagggtaaatggagaaaatatttctgggattacaatgaatgtaagcccaaattgtggaattgccagtaacctggatggggaaaagcatttcccatagcactccatgtaatatgagtgctctgtgagatgttcatcagtgttttatagaaatggtgttgctgggaaaccaagtttgcacctggaaacttacaatgcactttagcgcagtaagggcttggcatccggtagtgaaaaactgtctaacccagcattgcccaaactattttgacaccaggacctttttctcctttgggatacttatgaacctctcactaatgtcctgtggagaacattttgggaaacactatgttagatagttctttaaggagacaaaacggtaatgaacagatagcactggggcagaatatgcatgcattttgtaacgtccagtgtggcgttgaatagatgtgtatttcctcccctgcagaaaataagcacagaaaattataatgtaggtgatcggagctctttcctttgatagagagaacagccccaatgatcctggctttttcactgaacgtatcagaatacatggatgaattggggtaaataaggttttaattcagatctagaagaaagtattgtacgtttgaatgcagatttttatccacagatagttgtagtgtttagacatgacaggacctatcgttgaggtttctaagacttactatgggctgtaaacctgttttttaaaactattttagaaacctgagacttgccgtctggcattttagtttaatacaaactaatgattgcatttgaaagagattcttgaccttatttctaaacgtctagagctctgaaatgtcttgatggaaggtattaaactatttgcctgttgtacaaagaaatgttaagactcgtgaaaagaattactataaggtactgtgaaataactgcgattttgtgagcaaaacatacttggaaatgctgattgatttttatgcttgttagtgtattgcaagaaacacagaaaatgtagttttgttttaataaaccaaaaattgaacata

SEQ ID NO: 4 - RNA, 6368 nt, Homo sapiens
  source 1..6368: mol_type = mRNA
tatgttcaatttttggtttattaaaacaaaactacattttctgtgtttcttgcaatacactaacaagcataaaaatcaatcagcatttccaagtatgttttgctcacaaaatcgcagttatttcacagtaccttatagtaattcttttcacgagtcttaacatttctttgtacaacaggcaaatagtttaataccttccatcaagacatttcagagctctagacgtttagaaataaggtcaagaatctctttcaaatgcaatcattagtttgtattaaactaaaatgccagacggcaagtctcaggtttctaaaatagttttaaaaaacaggtttacagcccatagtaagtcttagaaacctcaacgataggtcctgtcatgtctaaacactacaactatctgtggataaaaatctgcattcaaacgtacaatactttcttctagatctgaattaaaaccttatttaccccaattcatccatgtattctgatacgttcagtgaaaaagccaggatcattggggctgttctctctatcaaaggaaagagctccgatcacctacattataattttctgtgcttattttctgcaggggaggaaatacacatctattcaacgccacactggacgttacaaaatgcatgcatattctgccccagtgctatctgttcattaccgttttgtctccttaaagaactatctaacatagtgtttcccaaaatgttctccacaggacattagtgagaggttcataagtatcccaaaggagaaaaaggtcctggtgtcaaaatagtttgggcaatgctgggttagacagtttttcactaccggatgccaagcccttactgcgctaaagtgcattgtaagtttccaggtgcaaacttggtttcccagcaacaccatttctataaaacactgatgaacatctcacagagcactcatattacatggagtgctatgggaaatgcttttccccatccaggttactggcaattccacaatttgggcttacattcattgtaatcccagaaatattttctccatttaccctcatgactttgtgaaatttaacagattccagaaggaagactcgaagccatctcagttaacagttctacacatttcccactagtttttgcctttgtttttcatgcattttcagagtgcacaacttccctcctctcttctgaatcacttaggacattctcattttcaaaaacagactgcagtttcatgttgtttaatattgttttttttttttaacttgaccacagtcttcccctgaagaagggcatgcatttcatgttacagaaatgcgatagagtaaactgtaataaattatttacaagcacctagtttgtttaaccttatgtggaagccatcactgttggaaaacaatgagaatgtatcttttagcaaaacggtgctatctggaagcttcattgtgaagatgctttcgtttttttgttttttgttttcagtcatgaggcactgaagaatgagttgtgctgaaattaactcaaaggtcagcttgtctggatgagcataactttggttgagatttttctcccttaaaaaagattttcaaagcaccagttaattacaaaaagcatgcatatttatcctcacagtgagttaagtggtgagagagctagcaaatcatacattgcattccccaaagcatctgaacgtacttctagaaaacaaaccaaccaaaagggaaaataatgcaagagaagccgtattttctttgcttaggttggcaaagcagcagctctttgcagcaatgacaggcagggcagagtgtcgactgggaagcgagtcccaatcttgaataatggtgagcttgagtaatccttaatttacaatttaaaggatgaaaaaaagagactagtgaaatgtttgcttccccagataaggaacacccaagactccctgggtatcctccaaatgtagccaagaaaagtgttcttctaccctagtcagtaaaatggaatgctaaaacatgatatctcattcaacatcagagctactacaactgacaatgacttcatggtatacatcaattcctataaagaaaaaatatattttaaatgcagaacttgagagggatcacaacagcatagcattattgctatgagtttcaaacatggtatttcatacaatgtgaaatatcaatcagcatccctccctctcccaaaacacacattactcatgagatactatcagtgtttaaaatccaagcttatggaagtacaaacttaattctcagtacttttatactaaattcaaagaatctatgtaacactcatctggaaaaattcttaattccataatatcttggagataagcaacagtaaactgttagaaaacgttttaacattacatgatatttaaaaaatcaccataattaccataataaaccaataattatgctccctgctcacaaaaggcacctaccaattatgaacagaccatttttcataattatttaccactatgtggcataagggtttaggcatataacccataaaaatttgttaaaagtcatggtttttcctcaaagctaaaaatccataaatgcctctaaccattaccagtcagtagggccaccacatgcatatactggacaggttgtgcacggcacaactcgagtgggtaccagtcacctggactggggtgcagtacacaatctgtgtgcagtacagaaagccctcatcagctgtggccagagaactgtattctaacagtctgtcagctcaagctaatcaagttaggaaaactgctatttggttggaggatttccaagaaacagctgtacctgtgagaggcaggtattacctgaggggtggacgaggtacagacataaaacaggaagggttctaaatatatttgctggtcatttgaaactcaatggcacttgtttatatgagcaaaagccttcaacaccagttttctggccaagtttccctagaattttgccagccaaattaacttcctgatgttaactatttgattacaatatctcagttcccgacctaaactaatattgtctgttttcacatagctcttaaaaacatttctaaatctgacagcaaaggacagcacagtgatacctgggtgtgatatatatcagtccactcaatttataaagcactttgggataaaaggtgctcccattaaaaatgtagctactattgacagataaaactgaaaaagagtgaatggatgactcaattatttttaaaggaagcattaaccactaaccagataatataccaacaaattacccagcagcactaagtataccatgtaagattcagttccagaacacagctacatttctgtgtccatcacagtaattagtccttaaaagttgtacttaaaatgtcaatctttaataaactcaaaaataatttattgagatttcatcttgtagtctacggattatgagttgcgaatagaggctgaggtccccccaagtgttatctgcaggctgctgtgttgatgcagagctgggaagatcacagatccatggagggagaaggcacttgtcttccaggagatcacttcgggacagggcaggcctgaccctgcgatggcaccttcaactcttgagccagaagctggtacctacaaggaactcatctcatgaccttcatttgccagcagtgccacacgttacctacagcaccacaaaactcagaatatattctagaagtttttgtcggttgcattgaggtagaaaagtgctgctcagttctaaaacagacactctcttttgtttggtctccttgaaaaccccaatatccttaaacattttcacagcattcttcacaagacaatatgtggcactctcagcatatactgcaacatttctttctgttctggttattaggtatttgtgcaacttttgcagatactcaggttctggaacaggaccactgaagttgtgaacaaagatggcagcagagctgtaggcctccagcaaaggcccaaggagtctctgtaagaaggtgataaactgctggtgctccttggattggctcaccttcaggtagcaatctcgctgttcctccccaaagtcactgtcttcatcttcttcatcacttctccaagacaaaggttctggaagcttcttgtcccactgctgctcagcaagactaggactgatatcttcctggtcatcgtgctctgccactgtaagaatgccatactggataaactttcctactgtttcatggcagacttggtaaaatgtctggcaaggcagtgagatggtgccttcattggagagaaggtagcacaggctggccgccttccgcaccagctgctcctggctgatcaggttaggtggggtgctagtgggaccccccagtcccctcttgttcagaactgcataaaggctgcaagctatgatggcctccatgataaagacatgaagtaccccattgctgtagaagttgagttcgaagactgatgggacagttgtgctgggggtgataaaaaactcatcgttcctgctagtgtgggtgattgtgacacaatttcccagcagctgtatggcatgcattactacatcttctgaatttcctgagaaccccaggtcaaaatcacgagccaggacttcctctttcatcacaaagaagtcttcgaccaatgtggagagatcaattccctgcctgtgtctgtagaggagcaggcaagccacaatgtgtgtggacataatggcacaggacttgctagcagtgaatagaatatgctcagccagatttgcaatcaacctccttcgtagggattcatctgttgcatttctggactcattaatggacgtgtctctaccttcatcagcagcatcactgggtcttgaaggaagtatagctggtaacaacgcttgctccagggaaagtagagcagacaccggtttctgactttggctttctaaatattcctttaaggaaaatggctgtgcaaaatccactcggacacaaccatagttttttcgtaacattctaataacacctcttgctacactccacaggctctcattcttcttaggtttgcccagttgttcaccattgtagtgaccttcgataatgcgatcataggagattccaacaggtattatcaagatgtctgggatgacattggtagacagagtatctaccacaactgacaaaagtcctgcccgagcacaagaggtttttccactcctagaacgtgtgccttccaggaagatctccaagaattgctgctgtcgaagtaattcaactatatgcccatggagcaaagctctatagagaacatctttccgtccatctggtgtttcatcgagccttcgtcgtatgaagaagcccccaagcttatggatcaaggtactgaagattgggatgttgagattattgcctgaagcaatgtatggtgctttgatgttatggcagaagagaatgaaagtgagcagcagatagtcaatatgggatctatgaactggtagaaacagaagcggcaaattcgtctcagttgcagctttaaccatctcaagttgacctttgtgaatttgaatgttccaaaagaagctgttgaacagttttagcagcacccacccagtcagtctgatcattgccggtgagacagtggcaaccatttcttgaagaatccttttagctttctttttcactttgttaacggcttttgattgctgctgggcagaaccatcagggtttaattcagcagccacttctgcaattgcctcttgtactctactgctgttcagcacattttcagtcacattggtggcaaacatgcccttatgcacatctcgctcttgaataaaaagaacgtaagaaaggcgtcttgcaagccatccgcggtgtcttgtgtgagtttcattgatataaataacattccgcaaacccaaagacgggatactggggttgaaaaatttgtcccagctctggggagtgcaggagtaacaacatcttccaacaaatggccttttccgactcattaggctttctttccattttaaagttgcagatctgaagatggtgggtctaaagccacactcaccccattcctcacttgtgtgcttacatcgaccaacactgtattctgatgaatgtggcagataagaaacatctattgtaccaagggtcagtgcagattcatccatgtcacaaagtgtaattcccaaatcatgtgctgggatgaaagttcttctgtttcataacataaaacttcaggactcagctatcagtttcgggtgcagaatgtccatacaacaggggagccgctgcctagcagctccagcttcggctgctgcagaagcccgcacttccagtcccggccaatgccagctgcagtggcgc

SEQ ID NO: 5 - RNA, 5956 nt, Mus musculus
  source 1..5956: mol_type = mRNA
ggcgcgccgctgcagcaggcgcagagccgaagcgctggcagctgcgtgcgcccaggcgcgagctgccgggcgggtggagaggagcgcggtgcgctgtgcgcggtgcgggctgcggctgcagacgccgctgggccggagcgcggggtcagcacatggtttgggacttgcacgttctgccatggaggagtcttcagtgacagttggcacaatagacgtttcttatctgcccagttcatcggaatacagccttggccgatgtaaacacaccagtgaggactgggttgactgtgggttcaaacctaccttcttcagatctgcaacactgaaatggaaggagagccttatgagccggaagaggcccttcgtgggaaggtgctgctattcctgcacgccacagagctgggaaaggtttttcaaccccagtatcccatctctgggtttgcggaatgttatttatatcaatgaaacgcacacaaggcacagaggatggctggcgagacggctgtcttacatcctttttgttcaagagcgagacgtccataagggcatgtttgccaccagtgttactgagaatgtactgagcagcagcagagtccaagaggcaattgctgaagtggctgcggagttgaacccagatggatctgcccagcagcagtccaaagccatccagaaggtgaaaaggaaagccaggaagatcctccaggagatggtcgccaccgtctccccagggatgatcaggctgactggctgggtgttactaaagctcttcaacagcttcttctggaacattcagattcacaagggtcaactcgagatggtcaaggctgcaactgagacgaacctgccgctcttgtttctgccggtgcacagatcccacattgactacctgttgctcaccttcatcctcttttgccacaacatcaaggcgccgtacatcgcctcgggcaataatctcaacatccccgtcttcagtaccttgattcacaagcttgggggctttttcataagacggaggctcgatgaaaccccagatggacgcaaagacattctgtacagagcgttgctccatgggcatgtagttgaactcctccgacagcagcagttcctggagatcttcctggaaggcacccgctcccgcagtggcaagacctcctgtgcccgggcagggctcctctcagtggtagtggatactctgtcgtccaacaccatccccgacatcctcgtcatacccgtgggcatctcgtatgatcgcataatcgaaggtcactacaatggcgaacagttgggaaagcccaagaagaacgagagcctctggagtgtggcgagaggcgttatcagaatgctgcggaaaaactacggctacgtccgagtggattttgcacagccattttccttgaaggaatatttagaaggccagagtcagaaacctgtatctgcccccctttctctggagcaagcactgttaccagcgatccttccttcaagaccgaatgatgttgctgatgaacatcaagacctatccagtaacgagtccagaaacccagcagacgaagccttccgacgaaggctgattgcaaacctggctgagcacattctcttcaccgccagcaagtcctgcgctatcatgtccacccacattgtggcctgtctgctcctctacagacacaggcagggaatccatctctccacgcttgtggaagacttctttgtgatgaaggaggaagtcctagctcgcgatttcgacctaggcttctccgggaattcagaagatgtcgtcatgcatgctattcagcttctggggaactgtgtcacaatcacccacacgagcaggaaagatgagttttttattactcccagcacaactgtcccgtcagtctttgaactcaacttctacagcaatggcgtacttcatgtgttcatcatggaagccatcatagcttgcagcatctatgcagtcctgaataagaggtgctctggagggtccgctggaggcctcggcaacctgatcagccaggagcagctggtgaggaaggccgccagcctgtgctaccttctctctaacgaaggtaccatttctctgccctgccagactttttaccaagtttgtcatgagacagttggcaagttcatccagtatggcattctcacagtggcagagcaagatgaccaggaagatgtcagtcctggccttgcagaacagcagtgggacaagaagcttccggaactgaactggagaagtgacgaggaagatgaagacagtgactttggtgaggagcagcgagattgctatctcaaggtgagccagtccaaggagcaccagcaattcatcacctttcttcagaggcttctaggtcccctgctagaagcctacagctctgctgccatctttgtccacaacttcagcggtccagttcccgagtctgagtacctgcagaaactgcacaggtaccttatcaccaggacggaaaggaacgttgccgtgtacgctgagagtgccacatactgtctcgtgaagaacgctgtgaaaatgtttaaggacatcggggttttcaaagagaccaagcaaaagcgagtgtctgttctagaactgagcagtactttcctacctcagtgcaaccggcagaaactcctagagtatattctgagttttgtggtgctgtagcgatctctcagcacctatctcgagcgaggagctgatgagtcccttgcagcctccagtctgacccagagtggcaggtatcctggcatggcccagcctgccctaccccgaggagacttccaggaagacacgtgccttctgcccccgtggacctgcgctcctcccaacacagacgcagtggcctgcgcagagcactcagggccagtgccatctgtgattcatgatcactaggttataggtgaaatctcagtaagttattttggagtttattaaaggttcacattttaagtacaacttttcaggctagttactgtgatggacattgaggtgtttgtagaactgactcttatatagtaagtaataatgtttcctttaaaataattgggccatccattctctgtctccattatcgctgtcaacagaagttatggtttgtatgtgagccctttcctctcaactgctttactaaggagcaatgttgtcctgcgccggcacactcaagatgtatctgagtagctgcctgaaagcagatgacactgcagtcaggaggtgagaggctgaggaaagagccagcatcaggaggtgactctggttggcaagggtgagctgtgcttggccaggaaggtggcattaaaggctgtgctcacgtgacaagagtgcctttgagctgtaatgaccagtgtttagagtccctgttgctgatacctttgagtgattgacacctgctgcttttgaggagctcggctgcagtgatcactggcgtgtggcactctggctacaaactgctgacccaggggttccagacactgctcactcactgggtgctgtgctgtggctagtgtatggcttgtacccagatggcgcactgtgcagcctgtgtagcatgcacagtgacccagctgagtggcaggtggttggaggcaaggacatttatgtgggccacatacccaaacttcctgccatgtaaaggcgagtgattgtgaaagcacctctgttgtagtgggtaggtgcctttctcatgagcggggagcataactgttagttatttgtggtgattatggcagatttcaagatcacgtgacaatgcagtctctaattgttcactgtccatatatatgattttacggaattatgaatttttctgatgagtgttgtatagatgatttgaattgataaaagtattagggatgaggtttgtactttcctgaacttgaatttcaaacactaactgtatcctatgagtgacgtgtgtgttgggggagggtgggcctgcctggtgttacacagagcatggcgtggctggtctggagcgcatagcaataatactgtgctgtggtgacctccgcccttgccttgtgcatgtcacacctccttttcctttgcttcacttctgtcaactgtagcgactttggtgtgcagtgagatgctcacctttagcctctgctcccctaactaggctggcacttcccttggctgtacttgggggacacccagagaggctggtgtactcccttgggtttatctgtggggactcaagcattttattggtctctgtttttttttttttccctctaaatggaaactgtaggtggcttcctctgatctgtctgccagtgggtgttgctgccctgcttgtcagctctgcaaatgagcgctgctccccagcttgcgcagagacgtgtgcgtcccacgtcccttgccgtgctctcccttttggtaggtgttactttaagaactgcagtcagacttgctgttgcctgacaattaactcactgtgaggataggcacgcacgcttttcataattaactggtgctttgaaacctttcttatggaagaaaaatctcaaccaaagttatgctcttcctgacaagctgacccttgagttaattttagcacaactcattcttcagtgcctcattatgaaagacaaaaagcatcacaataaggcttccaggtagccctgttccctaatagaaacattccccttgttttccagcagtgggtggcttcctcgaacgattaaacaaactaggtgcttgtatataatttattacagtttactctactgcatttctgtcaagttgaaatgcatgcccttcaggggaagactgtgagtcaagtttaataaataaaaacctaatactaagcaatatgaagctgcactctgcttttaagtgaggccaagccaagtaagccagagggggaggggcatttgctttccaaatcctaaggaaaaatgaaggcaaaacaagtgttatgtccattcagccaggaacacactctagccttcctgactctcttaaactgtggacgtcaggaggccgaatgcagaaaagtatatctgggatggatggcagggaatagaagctaggactggagttcctgtcctgccgccttggttcctgcagtatcgtgatgccctgagatggggatccgtgggaacatgcagtgccctgcagtgccctgcggtgcggacaggactgcatctgatagtacacagactgatgcacgtagcatttcccaaactgtttggacctcaggaccttttcccctctgggacactgcatgccgtggaaaaccttttcagaaactacattcattgttctttaagcagaccaaaagtcacaacagtggcaggcaggctgcatgctttttgtatcgctcacgatgcactgtggtgtgctcgggtatctttcctcactggagagagcaagcacaggaagctggctgcagtgccttcctcatgaaggatctaccacaaccctggcctttttaaaactgagagtagcagaattaatagagaaattaaaaaattaaaattggggtaaataataaaggttttaattcagatctagaagaaaactgcacagttgaatgcagatttttatccatagataactgtagtgttttgaaatgataggccctacctttgaagtttctaagacttattatgggatgtaaatctgttttttaaaaacactttttaggggcttgagagctgccacctggcatttagtttagtgcggccagtgactgcttcaagagacttctgaccttgcttcccaacagctaaagggctaactgtctttatggaaggcacttgttacagtatttgcccattgtacagagcaatgctacattgttgtaaaaagaattgctattgtaaaaaagcactgtgtgactttgtgaaggacactgccttggaaatgttgactgacgtttatgcctggtgatagcatgtcccgagaagcatggacatggagttttgttttaataaaccagaaaaaaaaaacccg

SEQ ID NO: 6 - RNA, 5956 nt, Mus musculus
  source 1..5956: mol_type = mRNA
cgggttttttttttctggtttattaaaacaaaactccatgtccatgcttctcgggacatgctatcaccaggcataaacgtcagtcaacatttccaaggcagtgtccttcacaaagtcacacagtgcttttttacaatagcaattctttttacaacaatgtagcattgctctgtacaatgggcaaatactgtaacaagtgccttccataaagacagttagccctttagctgttgggaagcaaggtcagaagtctcttgaagcagtcactggccgcactaaactaaatgccaggtggcagctctcaagcccctaaaaagtgtttttaaaaaacagatttacatcccataataagtcttagaaacttcaaaggtagggcctatcatttcaaaacactacagttatctatggataaaaatctgcattcaactgtgcagttttcttctagatctgaattaaaacctttattatttaccccaattttaattttttaatttctctattaattctgctactctcagttttaaaaaggccagggttgtggtagatccttcatgaggaaggcactgcagccagcttcctgtgcttgctctctccagtgaggaaagatacccgagcacaccacagtgcatcgtgagcgatacaaaaagcatgcagcctgcctgccactgttgtgacttttggtctgcttaaagaacaatgaatgtagtttctgaaaaggttttccacggcatgcagtgtcccagaggggaaaaggtcctgaggtccaaacagtttgggaaatgctacgtgcatcagtctgtgtactatcagatgcagtcctgtccgcaccgcagggcactgcagggcactgcatgttcccacggatccccatctcagggcatcacgatactgcaggaaccaaggcggcaggacaggaactccagtcctagcttctattccctgccatccatcccagatatacttttctgcattcggcctcctgacgtccacagtttaagagagtcaggaaggctagagtgtgttcctggctgaatggacataacacttgttttgccttcatttttccttaggatttggaaagcaaatgcccctccccctctggcttacttggcttggcctcacttaaaagcagagtgcagcttcatattgcttagtattaggtttttatttattaaacttgactcacagtcttcccctgaagggcatgcatttcaacttgacagaaatgcagtagagtaaactgtaataaattatatacaagcacctagtttgtttaatcgttcgaggaagccacccactgctggaaaacaaggggaatgtttctattagggaacagggctacctggaagccttattgtgatgctttttgtctttcataatgaggcactgaagaatgagttgtgctaaaattaactcaagggtcagcttgtcaggaagagcataactttggttgagatttttcttccataagaaaggtttcaaagcaccagttaattatgaaaagcgtgcgtgcctatcctcacagtgagttaattgtcaggcaacagcaagtctgactgcagttcttaaagtaacacctaccaaaagggagagcacggcaagggacgtgggacgcacacgtctctgcgcaagctggggagcagcgctcatttgcagagctgacaagcagggcagcaacacccactggcagacagatcagaggaagccacctacagtttccatttagagggaaaaaaaaaaaaacagagaccaataaaatgcttgagtccccacagataaacccaagggagtacaccagcctctctgggtgtcccccaagtacagccaagggaagtgccagcctagttaggggagcagaggctaaaggtgagcatctcactgcacaccaaagtcgctacagttgacagaagtgaagcaaaggaaaaggaggtgtgacatgcacaaggcaagggcggaggtcaccacagcacagtattattgctatgcgctccagaccagccacgccatgctctgtgtaacaccaggcaggcccaccctcccccaacacacacgtcactcataggatacagttagtgtttgaaattcaagttcaggaaagtacaaacctcatccctaatacttttatcaattcaaatcatctatacaacactcatcagaaaaattcataattccgtaaaatcatatatatggacagtgaacaattagagactgcattgtcacgtgatcttgaaatctgccataatcaccacaaataactaacagttatgctccccgctcatgagaaaggcacctacccactacaacagaggtgctttcacaatcactcgcctttacatggcaggaagtttgggtatgtggcccacataaatgtccttgcctccaaccacctgccactcagctgggtcactgtgcatgctacacaggctgcacagtgcgccatctgggtacaagccatacactagccacagcacagcacccagtgagtgagcagtgtctggaacccctgggtcagcagtttgtagccagagtgccacacgccagtgatcactgcagccgagctcctcaaaagcagcaggtgtcaatcactcaaaggtatcagcaacagggactctaaacactggtcattacagctcaaaggcactcttgtcacgtgagcacagcctttaatgccaccttcctggccaagcacagctcacccttgccaaccagagtcacctcctgatgctggctctttcctcagcctctcacctcctgactgcagtgtcatctgctttcaggcagctactcagatacatcttgagtgtgccggcgcaggacaacattgctccttagtaaagcagttgagaggaaagggctcacatacaaaccataacttctgttgacagcgataatggagacagagaatggatggcccaattattttaaaggaaacattattacttactatataagagtcagttctacaaacacctcaatgtccatcacagtaactagcctgaaaagttgtacttaaaatgtgaacctttaataaactccaaaataacttactgagatttcacctataacctagtgatcatgaatcacagatggcactggccctgagtgctctgcgcaggccactgcgtctgtgttgggaggagcgcaggtccacgggggcagaaggcacgtgtcttcctggaagtctcctcggggtagggcaggctgggccatgccaggatacctgccactctgggtcagactggaggctgcaagggactcatcagctcctcgctcgagataggtgctgagagatcgctacagcaccacaaaactcagaatatactctaggagtttctgccggttgcactgaggtaggaaagtactgctcagttctagaacagacactcgcttttgcttggtctctttgaaaaccccgatgtccttaaacattttcacagcgttcttcacgagacagtatgtggcactctcagcgtacacggcaacgttcctttccgtcctggtgataaggtacctgtgcagtttctgcaggtactcagactcgggaactggaccgctgaagttgtggacaaagatggcagcagagctgtaggcttctagcaggggacctagaagcctctgaagaaaggtgatgaattgctggtgctccttggactggctcaccttgagatagcaatctcgctgctcctcaccaaagtcactgtcttcatcttcctcgtcacttctccagttcagttccggaagcttcttgtcccactgctgttctgcaaggccaggactgacatcttcctggtcatcttgctctgccactgtgagaatgccatactggatgaacttgccaactgtctcatgacaaacttggtaaaaagtctggcagggcagagaaatggtaccttcgttagagagaaggtagcacaggctggcggccttcctcaccagctgctcctggctgatcaggttgccgaggcctccagcggaccctccagagcacctcttattcaggactgcatagatgctgcaagctatgatggcttccatgatgaacacatgaagtacgccattgctgtagaagttgagttcaaagactgacgggacagttgtgctgggagtaataaaaaactcatctttcctgctcgtgtgggtgattgtgacacagttccccagaagctgaatagcatgcatgacgacatcttctgaattcccggagaagcctaggtcgaaatcgcgagctaggacttcctccttcatcacaaagaagtcttccacaagcgtggagagatggattccctgcctgtgtctgtagaggagcagacaggccacaatgtgggtggacatgatagcgcaggacttgctggcggtgaagagaatgtgctcagccaggtttgcaatcagccttcgtcggaaggcttcgtctgctgggtttctggactcgttactggataggtcttgatgttcatcagcaacatcattcggtcttgaaggaaggatcgctggtaacagtgcttgctccagagaaaggggggcagatacaggtttctgactctggccttctaaatattccttcaaggaaaatggctgtgcaaaatccactcggacgtagccgtagtttttccgcagcattctgataacgcctctcgccacactccagaggctctcgttcttcttgggctttcccaactgttcgccattgtagtgaccttcgattatgcgatcatacgagatgcccacgggtatgacgaggatgtcggggatggtgttggacgacagagtatccactaccactgagaggagccctgcccgggcacaggaggtcttgccactgcgggagcgggtgccttccaggaagatctccaggaactgctgctgtcggaggagttcaactacatgcccatggagcaacgctctgtacagaatgtctttgcgtccatctggggtttcatcgagcctccgtcttatgaaaaagcccccaagcttgtgaatcaaggtactgaagacggggatgttgagattattgcccgaggcgatgtacggcgccttgatgttgtggcaaaagaggatgaaggtgagcaacaggtagtcaatgtgggatctgtgcaccggcagaaacaagagcggcaggttcgtctcagttgcagccttgaccatctcgagttgacccttgtgaatctgaatgttccagaagaagctgttgaagagctttagtaacacccagccagtcagcctgatcatccctggggagacggtggcgaccatctcctggaggatcttcctggctttccttttcaccttctggatggctttggactgctgctgggcagatccatctgggttcaactccgcagccacttcagcaattgcctcttggactctgctgctgctcagtacattctcagtaacactggtggcaaacatgcccttatggacgtctcgctcttgaacaaaaaggatgtaagacagccgtctcgccagccatcctctgtgccttgtgtgcgtttcattgatataaataacattccgcaaacccagagatgggatactggggttgaaaaacctttcccagctctgtggcgtgcaggaatagcagcaccttcccacgaagggcctcttccggctcataaggctctccttccatttcagtgttgcagatctgaagaaggtaggtttgaacccacagtcaacccagtcctcactggtgtgtttacatcggccaaggctgtattccgatgaactgggcagataagaaacgtctattgtgccaactgtcactgaagactcctccatggcagaacgtgcaagtcccaaaccatgtgctgaccccgcgctccggcccagcggcgtctgcagccgcagcccgcaccgcgcacagcgcaccgcgctcctctccacccgcccggcagctcgcgcctgggcgcacgcagctgccagcgcttcggctctgcgcctgctgcagcggcgcgcc

SEQ ID NO: 7 - RNA, 6246 nt, Mus musculus
  source 1..6246: mol_type = mRNA
ctccactgttgcaaaaccatcctggactgttggctgctgcccgcggtgcttctctggggttactgctgtgtacccgaaggtctccagcttccagctacacaaataggcctctggaggagcttctaagtcacccacacctggggctgtcttcttctgaagctgtctgggacagctttgctagtcaactgattcaaaataactccagatatcacatcaaggatacaggaccagtaagcaaagccctgcagctccattcctgaacctgctatttatcaggagcctggcaaaagatcaccctgaacaaaatcagagggaaagaaaagatattaaagcagcggctctctcagggagagagactaggggaatcctagaagccacaagccaaagagctagaagccgatttgaatcttttggggaacaattattaaacaggagttgacacatggtttgggacttgcacgttctgccatggaggagtcttcagtgacagttggcacaatagacgtttcttatctgcccagttcatcggaatacagccttggccgatgtaaacacaccagtgaggactgggttgactgtgggttcaaacctaccttcttcagatctgcaacactgaaatggaaggagagccttatgagccggaagaggcccttcgtgggaaggtgctgctattcctgcacgccacagagctgggaaaggtttttcaaccccagtatcccatctctgggtttgcggaatgttatttatatcaatgaaacgcacacaaggcacagaggatggctggcgagacggctgtcttacatcctttttgttcaagagcgagacgtccataagggcatgtttgccaccagtgttactgagaatgtactgagcagcagcagagtccaagaggcaattgctgaagtggctgcggagttgaacccagatggatctgcccagcagcagtccaaagccatccagaaggtgaaaaggaaagccaggaagatcctccaggagatggtcgccaccgtctccccagggatgatcaggctgactggctgggtgttactaaagctcttcaacagcttcttctggaacattcagattcacaagggtcaactcgagatggtcaaggctgcaactgagacgaacctgccgctcttgtttctgccggtgcacagatcccacattgactacctgttgctcaccttcatcctcttttgccacaacatcaaggcgccgtacatcgcctcgggcaataatctcaacatccccgtcttcagtaccttgattcacaagcttgggggctttttcataagacggaggctcgatgaaaccccagatggacgcaaagacattctgtacagagcgttgctccatgggcatgtagttgaactcctccgacagcagcagttcctggagatcttcctggaaggcacccgctcccgcagtggcaagacctcctgtgcccgggcagggctcctctcagtggtagtggatactctgtcgtccaacaccatccccgacatcctcgtcatacccgtgggcatctcgtatgatcgcataatcgaaggtcactacaatggcgaacagttgggaaagcccaagaagaacgagagcctctggagtgtggcgagaggcgttatcagaatgctgcggaaaaactacggctacgtccgagtggattttgcacagccattttccttgaaggaatatttagaaggccagagtcagaaacctgtatctgcccccctttctctggagcaagcactgttaccagcgatccttccttcaagaccgaatgatgttgctgatgaacatcaagacctatccagtaacgagtccagaaacccagcagacgaagccttccgacgaaggctgattgcaaacctggctgagcacattctcttcaccgccagcaagtcctgcgctatcatgtccacccacattgtggcctgtctgctcctctacagacacaggcagggaatccatctctccacgcttgtggaagacttctttgtgatgaaggaggaagtcctagctcgcgatttcgacctaggcttctccgggaattcagaagatgtcgtcatgcatgctattcagcttctggggaactgtgtcacaatcacccacacgagcaggaaagatgagttttttattactcccagcacaactgtcccgtcagtctttgaactcaacttctacagcaatggcgtacttcatgtgttcatcatggaagccatcatagcttgcagcatctatgcagtcctgaataagaggtgctctggagggtccgctggaggcctcggcaacctgatcagccaggagcagctggtgaggaaggccgccagcctgtgctaccttctctctaacgaaggtaccatttctctgccctgccagactttttaccaagtttgtcatgagacagttggcaagttcatccagtatggcattctcacagtggcagagcaagatgaccaggaagatgtcagtcctggccttgcagaacagcagtgggacaagaagcttccggaactgaactggagaagtgacgaggaagatgaagacagtgactttggtgaggagcagcgagattgctatctcaaggtgagccagtccaaggagcaccagcaattcatcacctttcttcagaggcttctaggtcccctgctagaagcctacagctctgctgccatctttgtccacaacttcagcggtccagttcccgagtctgagtacctgcagaaactgcacaggtaccttatcaccaggacggaaaggaacgttgccgtgtacgctgagagtgccacatactgtctcgtgaagaacgctgtgaaaatgtttaaggacatcggggttttcaaagagaccaagcaaaagcgagtgtctgttctagaactgagcagtactttcctacctcagtgcaaccggcagaaactcctagagtatattctgagttttgtggtgctgtagcgatctctcagcacctatctcgagcgaggagctgatgagtcccttgcagcctccagtctgacccagagtggcaggtatcctggcatggcccagcctgccctaccccgaggagacttccaggaagacacgtgccttctgcccccgtggacctgcgctcctcccaacacagacgcagtggcctgcgcagagcactcagggccagtgccatctgtgattcatgatcactaggttataggtgaaatctcagtaagttattttggagtttattaaaggttcacattttaagtacaacttttcaggctagttactgtgatggacattgaggtgtttgtagaactgactcttatatagtaagtaataatgtttcctttaaaataattgggccatccattctctgtctccattatcgctgtcaacagaagttatggtttgtatgtgagccctttcctctcaactgctttactaaggagcaatgttgtcctgcgccggcacactcaagatgtatctgagtagctgcctgaaagcagatgacactgcagtcaggaggtgagaggctgaggaaagagccagcatcaggaggtgactctggttggcaagggtgagctgtgcttggccaggaaggtggcattaaaggctgtgctcacgtgacaagagtgcctttgagctgtaatgaccagtgtttagagtccctgttgctgatacctttgagtgattgacacctgctgcttttgaggagctcggctgcagtgatcactggcgtgtggcactctggctacaaactgctgacccaggggttccagacactgctcactcactgggtgctgtgctgtggctagtgtatggcttgtacccagatggcgcactgtgcagcctgtgtagcatgcacagtgacccagctgagtggcaggtggttggaggcaaggacatttatgtgggccacatacccaaacttcctgccatgtaaaggcgagtgattgtgaaagcacctctgttgtagtgggtaggtgcctttctcatgagcggggagcataactgttagttatttgtggtgattatggcagatttcaagatcacgtgacaatgcagtctctaattgttcactgtccatatatatgattttacggaattatgaatttttctgatgagtgttgtatagatgatttgaattgataaaagtattagggatgaggtttgtactttcctgaacttgaatttcaaacactaactgtatcctatgagtgacgtgtgtgttgggggagggtgggcctgcctggtgttacacagagcatggcgtggctggtctggagcgcatagcaataatactgtgctgtggtgacctccgcccttgccttgtgcatgtcacacctccttttcctttgcttcacttctgtcaactgtagcgactttggtgtgcagtgagatgctcacctttagcctctgctcccctaactaggctggcacttcccttggctgtacttgggggacacccagagaggctggtgtactcccttgggtttatctgtggggactcaagcattttattggtctctgtttttttttttttccctctaaatggaaactgtaggtggcttcctctgatctgtctgccagtgggtgttgctgccctgcttgtcagctctgcaaatgagcgctgctccccagcttgcgcagagacgtgtgcgtcccacgtcccttgccgtgctctcccttttggtaggtgttactttaagaactgcagtcagacttgctgttgcctgacaattaactcactgtgaggataggcacgcacgcttttcataattaactggtgctttgaaacctttcttatggaagaaaaatctcaaccaaagttatgctcttcctgacaagctgacccttgagttaattttagcacaactcattcttcagtgcctcattatgaaagacaaaaagcatcacaataaggcttccaggtagccctgttccctaatagaaacattccccttgttttccagcagtgggtggcttcctcgaacgattaaacaaactaggtgcttgtatataatttattacagtttactctactgcatttctgtcaagttgaaatgcatgcccttcaggggaagactgtgagtcaagtttaataaataaaaacctaatactaagcaatatgaagctgcactctgcttttaagtgaggccaagccaagtaagccagagggggaggggcatttgctttccaaatcctaaggaaaaatgaaggcaaaacaagtgttatgtccattcagccaggaacacactctagccttcctgactctcttaaactgtggacgtcaggaggccgaatgcagaaaagtatatctgggatggatggcagggaatagaagctaggactggagttcctgtcctgccgccttggttcctgcagtatcgtgatgccctgagatggggatccgtgggaacatgcagtgccctgcagtgccctgcggtgcggacaggactgcatctgatagtacacagactgatgcacgtagcatttcccaaactgtttggacctcaggaccttttcccctctgggacactgcatgccgtggaaaaccttttcagaaactacattcattgttctttaagcagaccaaaagtcacaacagtggcaggcaggctgcatgctttttgtatcgctcacgatgcactgtggtgtgctcgggtatctttcctcactggagagagcaagcacaggaagctggctgcagtgccttcctcatgaaggatctaccacaaccctggcctttttaaaactgagagtagcagaattaatagagaaattaaaaaattaaaattggggtaaataataaaggttttaattcagatctagaagaaaactgcacagttgaatgcagatttttatccatagataactgtagtgttttgaaatgataggccctacctttgaagtttctaagacttattatgggatgtaaatctgttttttaaaaacactttttaggggcttgagagctgccacctggcatttagtttagtgcggccagtgactgcttcaagagacttctgaccttgcttcccaacagctaaagggctaactgtctttatggaaggcacttgttacagtatttgcccattgtacagagcaatgctacattgttgtaaaaagaattgctattgtaaaaaagcactgtgtgactttgtgaaggacactgccttggaaatgttgactgacgtttatgcctggtgatagcatgtcccgagaagcatggacatggagttttgttttaataaaccagaaaaaaaaaacccg

SEQ ID NO: 8 - RNA, 6246 nt, Mus musculus
  source 1..6246: mol_type = mRNA
cgggttttttttttctggtttattaaaacaaaactccatgtccatgcttctcgggacatgctatcaccaggcataaacgtcagtcaacatttccaaggcagtgtccttcacaaagtcacacagtgcttttttacaatagcaattctttttacaacaatgtagcattgctctgtacaatgggcaaatactgtaacaagtgccttccataaagacagttagccctttagctgttgggaagcaaggtcagaagtctcttgaagcagtcactggccgcactaaactaaatgccaggtggcagctctcaagcccctaaaaagtgtttttaaaaaacagatttacatcccataataagtcttagaaacttcaaaggtagggcctatcatttcaaaacactacagttatctatggataaaaatctgcattcaactgtgcagttttcttctagatctgaattaaaacctttattatttaccccaattttaattttttaatttctctattaattctgctactctcagttttaaaaaggccagggttgtggtagatccttcatgaggaaggcactgcagccagcttcctgtgcttgctctctccagtgaggaaagatacccgagcacaccacagtgcatcgtgagcgatacaaaaagcatgcagcctgcctgccactgttgtgacttttggtctgcttaaagaacaatgaatgtagtttctgaaaaggttttccacggcatgcagtgtcccagaggggaaaaggtcctgaggtccaaacagtttgggaaatgctacgtgcatcagtctgtgtactatcagatgcagtcctgtccgcaccgcagggcactgcagggcactgcatgttcccacggatccccatctcagggcatcacgatactgcaggaaccaaggcggcaggacaggaactccagtcctagcttctattccctgccatccatcccagatatacttttctgcattcggcctcctgacgtccacagtttaagagagtcaggaaggctagagtgtgttcctggctgaatggacataacacttgttttgccttcatttttccttaggatttggaaagcaaatgcccctccccctctggcttacttggcttggcctcacttaaaagcagagtgcagcttcatattgcttagtattaggtttttatttattaaacttgactcacagtcttcccctgaagggcatgcatttcaacttgacagaaatgcagtagagtaaactgtaataaattatatacaagcacctagtttgtttaatcgttcgaggaagccacccactgctggaaaacaaggggaatgtttctattagggaacagggctacctggaagccttattgtgatgctttttgtctttcataatgaggcactgaagaatgagttgtgctaaaattaactcaagggtcagcttgtcaggaagagcataactttggttgagatttttcttccataagaaaggtttcaaagcaccagttaattatgaaaagcgtgcgtgcctatcctcacagtgagttaattgtcaggcaacagcaagtctgactgcagttcttaaagtaacacctaccaaaagggagagcacggcaagggacgtgggacgcacacgtctctgcgcaagctggggagcagcgctcatttgcagagctgacaagcagggcagcaacacccactggcagacagatcagaggaagccacctacagtttccatttagagggaaaaaaaaaaaaacagagaccaataaaatgcttgagtccccacagataaacccaagggagtacaccagcctctctgggtgtcccccaagtacagccaagggaagtgccagcctagttaggggagcagaggctaaaggtgagcatctcactgcacaccaaagtcgctacagttgacagaagtgaagcaaaggaaaaggaggtgtgacatgcacaaggcaagggcggaggtcaccacagcacagtattattgctatgcgctccagaccagccacgccatgctctgtgtaacaccaggcaggcccaccctcccccaacacacacgtcactcataggatacagttagtgtttgaaattcaagttcaggaaagtacaaacctcatccctaatacttttatcaattcaaatcatctatacaacactcatcagaaaaattcataattccgtaaaatcatatatatggacagtgaacaattagagactgcattgtcacgtgatcttgaaatctgccataatcaccacaaataactaacagttatgctccccgctcatgagaaaggcacctacccactacaacagaggtgctttcacaatcactcgcctttacatggcaggaagtttgggtatgtggcccacataaatgtccttgcctccaaccacctgccactcagctgggtcactgtgcatgctacacaggctgcacagtgcgccatctgggtacaagccatacactagccacagcacagcacccagtgagtgagcagtgtctggaacccctgggtcagcagtttgtagccagagtgccacacgccagtgatcactgcagccgagctcctcaaaagcagcaggtgtcaatcactcaaaggtatcagcaacagggactctaaacactggtcattacagctcaaaggcactcttgtcacgtgagcacagcctttaatgccaccttcctggccaagcacagctcacccttgccaaccagagtcacctcctgatgctggctctttcctcagcctctcacctcctgactgcagtgtcatctgctttcaggcagctactcagatacatcttgagtgtgccggcgcaggacaacattgctccttagtaaagcagttgagaggaaagggctcacatacaaaccataacttctgttgacagcgataatggagacagagaatggatggcccaattattttaaaggaaacattattacttactatataagagtcagttctacaaacacctcaatgtccatcacagtaactagcctgaaaagttgtacttaaaatgtgaacctttaataaactccaaaataacttactgagatttcacctataacctagtgatcatgaatcacagatggcactggccctgagtgctctgcgcaggccactgcgtctgtgttgggaggagcgcaggtccacgggggcagaaggcacgtgtcttcctggaagtctcctcggggtagggcaggctgggccatgccaggatacctgccactctgggtcagactggaggctgcaagggactcatcagctcctcgctcgagataggtgctgagagatcgctacagcaccacaaaactcagaatatactctaggagtttctgccggttgcactgaggtaggaaagtactgctcagttctagaacagacactcgcttttgcttggtctctttgaaaaccccgatgtccttaaacattttcacagcgttcttcacgagacagtatgtggcactctcagcgtacacggcaacgttcctttccgtcctggtgataaggtacctgtgcagtttctgcaggtactcagactcgggaactggaccgctgaagttgtggacaaagatggcagcagagctgtaggcttctagcaggggacctagaagcctctgaagaaaggtgatgaattgctggtgctccttggactggctcaccttgagatagcaatctcgctgctcctcaccaaagtcactgtcttcatcttcctcgtcacttctccagttcagttccggaagcttcttgtcccactgctgttctgcaaggccaggactgacatcttcctggtcatcttgctctgccactgtgagaatgccatactggatgaacttgccaactgtctcatgacaaacttggtaaaaagtctggcagggcagagaaatggtaccttcgttagagagaaggtagcacaggctggcggccttcctcaccagctgctcctggctgatcaggttgccgaggcctccagcggaccctccagagcacctcttattcaggactgcatagatgctgcaagctatgatggcttccatgatgaacacatgaagtacgccattgctgtagaagttgagttcaaagactgacgggacagttgtgctgggagtaataaaaaactcatctttcctgctcgtgtgggtgattgtgacacagttccccagaagctgaatagcatgcatgacgacatcttctgaattcccggagaagcctaggtcgaaatcgcgagctaggacttcctccttcatcacaaagaagtcttccacaagcgtggagagatggattccctgcctgtgtctgtagaggagcagacaggccacaatgtgggtggacatgatagcgcaggacttgctggcggtgaagagaatgtgctcagccaggtttgcaatcagccttcgtcggaaggcttcgtctgctgggtttctggactcgttactggataggtcttgatgttcatcagcaacatcattcggtcttgaaggaaggatcgctggtaacagtgcttgctccagagaaaggggggcagatacaggtttctgactctggccttctaaatattccttcaaggaaaatggctgtgcaaaatccactcggacgtagccgtagtttttccgcagcattctgataacgcctctcgccacactccagaggctctcgttcttcttgggctttcccaactgttcgccattgtagtgaccttcgattatgcgatcatacgagatgcccacgggtatgacgaggatgtcggggatggtgttggacgacagagtatccactaccactgagaggagccctgcccgggcacaggaggtcttgccactgcgggagcgggtgccttccaggaagatctccaggaactgctgctgtcggaggagttcaactacatgcccatggagcaacgctctgtacagaatgtctttgcgtccatctggggtttcatcgagcctccgtcttatgaaaaagcccccaagcttgtgaatcaaggtactgaagacggggatgttgagattattgcccgaggcgatgtacggcgccttgatgttgtggcaaaagaggatgaaggtgagcaacaggtagtcaatgtgggatctgtgcaccggcagaaacaagagcggcaggttcgtctcagttgcagccttgaccatctcgagttgacccttgtgaatctgaatgttccagaagaagctgttgaagagctttagtaacacccagccagtcagcctgatcatccctggggagacggtggcgaccatctcctggaggatcttcctggctttccttttcaccttctggatggctttggactgctgctgggcagatccatctgggttcaactccgcagccacttcagcaattgcctcttggactctgctgctgctcagtacattctcagtaacactggtggcaaacatgcccttatggacgtctcgctcttgaacaaaaaggatgtaagacagccgtctcgccagccatcctctgtgccttgtgtgcgtttcattgatataaataacattccgcaaacccagagatgggatactggggttgaaaaacctttcccagctctgtggcgtgcaggaatagcagcaccttcccacgaagggcctcttccggctcataaggctctccttccatttcagtgttgcagatctgaagaaggtaggtttgaacccacagtcaacccagtcctcactggtgtgtttacatcggccaaggctgtattccgatgaactgggcagataagaaacgtctattgtgccaactgtcactgaagactcctccatggcagaacgtgcaagtcccaaaccatgtgtcaactcctgtttaataattgttccccaaaagattcaaatcggcttctagctctttggcttgtggcttctaggattcccctagtctctctccctgagagagccgctgctttaatatcttttctttccctctgattttgttcagggtgatcttttgccaggctcctgataaatagcaggttcaggaatggagctgcagggctttgcttactggtcctgtatccttgatgtgatatctggagttattttgaatcagttgactagcaaagctgtcccagacagcttcagaagaagacagccccaggtgtgggtgacttagaagctcctccagaggcctatttgtgtagctggaagctggagaccttcgggtacacagcagtaaccccagagaagcaccgcgggcagcagccaacagtccaggatggttttgcaacagtggag

SEQ ID NO: 9 - RNA, 2646 nt, Rattus norvegicus
  source 1..2646: mol_type = mRNA
cacgaataagcctctggaggagctgctgaatcacccccgccccaggctgtcttctgaagctgtctggggatagctttgctaatcaactgactggaaataattccagacaccacatcaaggatacagctcatgttttgtttgggacttccacgttgagtcatggaggagtcttcagtgacaattggcacaatagacgtttcttatctgcccaattcatcagaatacagccttggccgatgtaaacacacgaatgaggactgggttgactgtggcttcaaacctaccttcttcagatccgcaacgctgaaatggaaggagagcctcatgagccggaagaggcccttcgtgggaaggtgttgctattcatgcacgcctcagagctgggaaaggtttttcaaccccagtatcccatctctgggtttgcggaatgttatttatatcaatgaaactcacacaaggcaccgaggatggctggcaagacggctttcttacatcctttttgttcaagagcgcgatgtccacaagggcatgtttgccaccagtatcactgacaatgtactgaatagcagcagagtccaagaggcaattgctgaagtggctgcagaattgaacccggatggatctgcccagcagcagtccaaagccatccagaaagtgaaaaggaaagccaggaagatcctccaggaaatggttgctacagtctcccccgggatgatcaggctgactggctgggtgttactaaagctcttcaacagcttcttctggaacattcagattcacaagggtcaacttgagatggtgaaagctgcaactgagacgaatctgccgctcttgtttctgccggtgcacagatcccacatcgactacctgctgctcaccttcatcctcttctgccacaacatcaaagctccatacatcgcctcgggcaacaacctcaacatccccatcttcagtaccttgattcacaagcttgggggctttttcataagacggaggcttgacgaaactccagatggacgcaaagacattctgtacagagcgttgctccatgggcatatagttgaactcctccgacagcagcagttcctggagatcttcctggaaggcacccgctcccgcagtggcaagacctcctgtgcccgggccgggctcctgtcagtggtagtggatactctgtcatccaacaccatccctgacatcctggtcatccctgtgggcatctcgtatgatcggataatcgaaggtcactacaatggtgaacagttgggcaagcccaagaagaatgaaagtctctggagtgtggcaagaggcgttatcagaatgctgcggaaaaactacggctatgtccgagtggactttgcacagccattttctttgaaggaatatttagaaggccaaagtcagaaacctgtatctgctcccctctctttggagcaagcactgttaccagcaatccttccttcaagacctgatgctgctgctgccgaacatgaagacatgtccagtaatgagtcgagaaacgcggcagacgaagccttccgaaggaggctgatcgcaaacctggcggagcacattctcttcaccgccagcaagtcctgcgctatcatgtccacccacattgtggcctgcctgctcctctacagacacaggcagggaatccacctctccacgctggtggaagacttctttgtgatgaaggaggaagtcctagctcgggattttgacctgggcttctccgggaattcagaagatgtagtcatgcatgctattcagcttctggggaactgtgtcacaatcacccacactagcaggaaggatgaattctttattactcccagcacaactgtcccgtccgtctttgaactcaacttctacagcaatggggtacttcatgtctttatcatggaagccatcatagcttgcagcatttatgcagtccagaataagaggggttccggagggtctgccggaggccttggcaacctgatcagccaggagcagctggtgcggaaggccgccagcctgtgctaccttctctctaatgaaggtaccatttctctgccctgccagacattttaccaggtttgtcaagagacagtaggaaagttcatccagtacggaattctcacagtggcagagcaagatgaccaggaagatgtcagtcctggccttgcagagcagcagtggaacaagaagcttccggagcctctgaactggagaagtgacgaagaagatgaggacagtgactttggtgaggagcagcgtgattgctacctgaaggtgagccaggccaaggagcaccagcaattcatcacctttctgcagaggcttctggggcccctgctagaagcctacagctctgctgccatctttgtccacaccttccgcggcccagtcccggagtctgagtacctgcagaagctgcacaggtaccttctcaccaggacggagaggaacgtcgcggtgtacgctgagagtgccacatactgtcttgtgaagaatgctgtgaaaatgtttaaggacatcggggttttcaaagagaccaagcagaagcgagcgtctgtcttagaactgagcaccactttcctacctcagggcagccggcagaagctcctggaatacattctgagcttcgtggtgctgtag

SEQ ID NO: 10 - RNA, 2646 nt, Rattus norvegicus
  source 1..2646: mol_type = mRNA
ctacagcaccacgaagctcagaatgtattccaggagcttctgccggctgccctgaggtaggaaagtggtgctcagttctaagacagacgctcgcttctgcttggtctctttgaaaaccccgatgtccttaaacattttcacagcattcttcacaagacagtatgtggcactctcagcgtacaccgcgacgttcctctccgtcctggtgagaaggtacctgtgcagcttctgcaggtactcagactccgggactgggccgcggaaggtgtggacaaagatggcagcagagctgtaggcttctagcaggggccccagaagcctctgcagaaaggtgatgaattgctggtgctccttggcctggctcaccttcaggtagcaatcacgctgctcctcaccaaagtcactgtcctcatcttcttcgtcacttctccagttcagaggctccggaagcttcttgttccactgctgctctgcaaggccaggactgacatcttcctggtcatcttgctctgccactgtgagaattccgtactggatgaactttcctactgtctcttgacaaacctggtaaaatgtctggcagggcagagaaatggtaccttcattagagagaaggtagcacaggctggcggccttccgcaccagctgctcctggctgatcaggttgccaaggcctccggcagaccctccggaacccctcttattctggactgcataaatgctgcaagctatgatggcttccatgataaagacatgaagtaccccattgctgtagaagttgagttcaaagacggacgggacagttgtgctgggagtaataaagaattcatccttcctgctagtgtgggtgattgtgacacagttccccagaagctgaatagcatgcatgactacatcttctgaattcccggagaagcccaggtcaaaatcccgagctaggacttcctccttcatcacaaagaagtcttccaccagcgtggagaggtggattccctgcctgtgtctgtagaggagcaggcaggccacaatgtgggtggacatgatagcgcaggacttgctggcggtgaagagaatgtgctccgccaggtttgcgatcagcctccttcggaaggcttcgtctgccgcgtttctcgactcattactggacatgtcttcatgttcggcagcagcagcatcaggtcttgaaggaaggattgctggtaacagtgcttgctccaaagagaggggagcagatacaggtttctgactttggccttctaaatattccttcaaagaaaatggctgtgcaaagtccactcggacatagccgtagtttttccgcagcattctgataacgcctcttgccacactccagagactttcattcttcttgggcttgcccaactgttcaccattgtagtgaccttcgattatccgatcatacgagatgcccacagggatgaccaggatgtcagggatggtgttggatgacagagtatccactaccactgacaggagcccggcccgggcacaggaggtcttgccactgcgggagcgggtgccttccaggaagatctccaggaactgctgctgtcggaggagttcaactatatgcccatggagcaacgctctgtacagaatgtctttgcgtccatctggagtttcgtcaagcctccgtcttatgaaaaagcccccaagcttgtgaatcaaggtactgaagatggggatgttgaggttgttgcccgaggcgatgtatggagctttgatgttgtggcagaagaggatgaaggtgagcagcaggtagtcgatgtgggatctgtgcaccggcagaaacaagagcggcagattcgtctcagttgcagctttcaccatctcaagttgacccttgtgaatctgaatgttccagaagaagctgttgaagagctttagtaacacccagccagtcagcctgatcatcccgggggagactgtagcaaccatttcctggaggatcttcctggctttccttttcactttctggatggctttggactgctgctgggcagatccatccgggttcaattctgcagccacttcagcaattgcctcttggactctgctgctattcagtacattgtcagtgatactggtggcaaacatgcccttgtggacatcgcgctcttgaacaaaaaggatgtaagaaagccgtcttgccagccatcctcggtgccttgtgtgagtttcattgatataaataacattccgcaaacccagagatgggatactggggttgaaaaacctttcccagctctgaggcgtgcatgaatagcaacaccttcccacgaagggcctcttccggctcatgaggctctccttccatttcagcgttgcggatctgaagaaggtaggtttgaagccacagtcaacccagtcctcattcgtgtgtttacatcggccaaggctgtattctgatgaattgggcagataagaaacgtctattgtgccaattgtcactgaagactcctccatgactcaacgtggaagtcccaaacaaaacatgagctgtatccttgatgtggtgtctggaattatttccagtcagttgattagcaaagctatccccagacagcttcagaagacagcctggggcgggggtgattcagcagctcctccagaggcttattcgtg

SEQ ID NO: 11 - RNA, 6262 nt, Macaca mulatta
  source 1..6262: mol_type = mRNA
ctgttgtatggacattctgcacccgaaactgatagctgagtcctgaagttttatgttatgaaacagaagaactttcatcccagcacatgatttgggaattacactttgtgacatggatgaatctgcactgacccttggtacaatagatgtttcttatctgccgaattcatcagaatacagtgttggtcgatgtaagcacacaagtgaggaatggggtgagtgtggttttagacctactgtcttcagatctgcaactttaaaatggaaagaaagcctaatgagtcggaaaaggccatttgttggaagatgttgttactcctgcactccccagagctgggacagatttttcaaccccagtatcccgtctttgggtttgcggaatgttatttatatcaatgaaactcacacaagacaccggggatggcttgcaagacgcctttcttatgttctttttattcaagagcgagatgtgcataagggcatgtttgccaccaatgtgactgaaaatgtgctgaacagcagtagagtacaagaggcaattgcagaagtggctgctgaattaaaccctgatggttctgcccagcagcaatcaaaagccgttaacaaagtgaaaaagaaagctaaaaggattcttcaagaaatggttgccactgtctcaccggcaatgatcagactgactgggtgggtgctgctaaaactgttcaacagcttcttttggaacattcaaattcacaaaggtcaacttgagatggttaaagctgcaactgagacgaatttgccgcttctgtttctaccagttcatagatcccatattgactatctgctgctcactttcattctcttctgccataacatcaaagcaccatacattgcttcaggcaataatctccatatcccaatcttcagtactttgatccataagcttgggggcttcttcatacgacgaaggctcgatgaaacaccagatggacggaaagatgttctctacagagctttgctccatgggcatatagttgaattacttcgacagcagcaattcttggagatcttcctggaaggcacacgttctaggagtggaaaaacctcctgtgctcgggcgggacttttgtcagttgtggtagatactctatctaccaatgtcatcccagacatcttgataatacctgttggaatctcctatgatcgtattatcgaaggtcactacaatggcgaacaactgggcaagccaaagaagaatgagagcctgtggagtatagcaagaggtgttattagaatgttacgaaaaaactatggttgtgtccgagtggattttgcacagccgttttccttaaaggaatatttagaaagccaaagtcagaaaccggtgtctgctccactttctctggagcaagcgttgttaccagctatacttccttcaagacccaatgatgctgctgatgaaggtagagacacatccattaatgagtccagaaatgcaacagatgaattcctacgaaggaggttgattgcaaatctggctgagcatattctattcactgctagcaagtcctgtgccattatgtccacacacattgtggcttgcctactcctctacagacacaggcagggaattgatctctccacattggtggaagacttctttgtgatgaaagaggaagtcctggctcgtgattttgacctggggttctcaggaaattcagaagatgtagtaatgcatgccatacagctgctgggaaattgcgtcacaatcactcacactagcaggaacgatgagttttttatcacccccagcacaactgtcccagcagtcttcgaactcaacttctacagcaatggggtacttcatgtctttatcatggaggccatcatagcttgcagcctttatgcagttctgaacaagaggggattaggggggcccactggcaccccacctaacctgatcagccaggagcagctggtgcggaaggcggccagcctgtgctaccttctctccaatgagggcaccatctcactgccttgccagacattttaccaagtgtgccatgaaacagtaggaaagtttatccagtatggcattcttacagtggcagagcacgatgaccaggaagatatcagtcctagtcttgctgagcagcagtgggacaagaagcttcctgaacctttgtcttggagaagtgatgaagaagatgaagacagtgactttggggaggaacagcgagattgctacctgaaggtgagccaatccaaggagcaccagcagtttatcaccttcttacagagactccttgggcctttgctggaggcctacagctctgctgccatctttgttcacaactttagcggccctgttccagaacctgaatatctgcaaaagttgcacaaatacctagtaaccagaacagaaagaaatgttgcagtatatgctgagagtgccacatactgtcttgtgaagaatgctgtgaaaatgtttaaggatattggggttttcaaggagaccaaacaaaagagagtgtctgttttagaactgagcagcacttttctacctcaatgcaaccggcaaaaacttctagaatatattctgagttttgtggtgctgtaggtaacgtgtggcaccgctggcaaatgaaggtcatgagatgagtcccttgtaggtaccagcttctggctcgagagttgaaggtgccgtcgcaaggtcacgcctgccctgtcccgcagtgatctcctggaagacaagtgccttctccctccatggatctgtgatcttcccagctctgcatccacacagcagcctgcagataacacttggggggacctcagcctctattcgcaactcacaatccgtagactacaagatgaaatctcaatacattattttggagtttattaaagattgacattttaagtacaacttttaaggactaattactgtgatggacacagaaatgtagctgtgttctagaactgaatcttatatggtatacttagtgctattgggtaatttgttggtatattatctggttaatggttaatgcttcctttaaaaataattgagtcatccattcactctttttcagttttatctttgtcaatagtagctacatttttaatgggagtaccttttatcccaagtgctttataaatgaatggactgatatatatcacacccaggtatcactgtgctgtcctttgcagtcagatatagaaaatgtttttaagaggtatgtgaaaacagacagtattagtttaggtcgggaactgagatattgtaatcaaatagttaacatcaggaagttaatttggctggcaaaattctagggaaacttggccagaaaactggtgttgaaggcttttgctcatataaaaaagtgccattgagttttaaatgaccagcaaatatttagaacccttcctgttttatgtctgtaccccgtctacccctcaggtaatacctgcttctcacgggtacagctgtttcttggaaatcctccaaccaaatagcaactttcctaacttgattagcttgagctgacagactctgttagaatacagtgctctggccacaactgatgagggctttctgtactgcacacagattgtgtactgcaccccagtccaggtgactggtgcccacttgagttgtgccgtgcacaacctgtccagtatatgcatgtggtggccctactgactggtaatggttagaggcatttgtgaatttttagctttgaggaaaaaccatgacttttaacaaatttttatgggttatatgcctaaaccattatgccacatagtggtaaataattatgaaaaatggtctgttcataattggtaggtgccttttgtgaacagggagcataattattagtttattatggtaattatggtgatttcttaaatatcatgtaatgttaaaacattttctaacagtttactgttgcttatctctaagatattatggaattaagaatttttccagatgagtgttacatagtttctttgaatttagtataaaaatactgagaattaagtttgtacttctataagcttgggttttaaacactaatagtgtctcatgagtaacgtgtgttttgggagagggagggatgctgattgatatttcacattgtatgaagtatcacgtttgaaactggtagcaataatgctatgctgttgtgatccctctcaagttctgcatttaaaagatattttttcttgataggaattgaggtactgttaagtcattgtcagttgtagtagctctgatgttaatgagataatcacgttttagcattccattttactgactagggtggaagaacacttttctcggctacatttggaggatacccagggagtcttgggtgttccttatgtggggaatcaagcatttcactagtctctttttttcatcctttaaattgtagattaaggattactcaagctcaccattattcaaggttgggactcacttcccagtggatactctgccctgcctgtcactgctgcaaagagctgctgcttcgccagcctaagcagagaaaatatggcttctcttgcattattttcccttttggttggtttgttttcgagaagtttgatcagatgctttgaggaatgcaatgtatgatttgctagctctcttaccacttaagtcactgtgaggataaatatgcatgcattttgtaattaactggtgctttgaaaatcttttttaagggagaaaaatctcaaccaaagttatgctcatccagacaagctgacctttgagttaatttcagcacaactcattcttcagtgcctcatgaccgaaaaacaaaaagcaaaaaagaaagcatcttcacaataaagcttccagatagcaccattttgctaaaagatacgttctcattgttttccaacagcgatggcttccatgtaaggttaaacaaactaggtgcttgtaaataattttattacagtttactctattgcatttctataacatgaaatgcatgcccttcaggggaagactgtgagtcaagttaaaaaaaaatattaagcaatatgcaactgctctctgtttttaaaaatgagaatgtcctaagtgattcagaagagaggaaggaatttatgtactcttaaaattgcatgaaaaacaaggcaaaaactagtgtgaaatgtgtagaactgttaactgagacggcattgagtcttccttctgaaatctgttaaatctcacaaagtcatgagggtatatggagaaaatatttctgggattacaatgaatgtaatcccagattgtggaatttccagtaacctggaccgggaaaagcatttcccatagtactccatgtaatatgagtgctctgtgagatgttcatcagtgttttatagaaatggtgttgctgggaactaagtttgcacatggagacttacaatgcactttagcgcagtaagggcttggcatctggcagtgaaaaactgttcaacccagcattgcccaaactattttgacatcaggacctttttctcctttgggatacctgtgaacctctcactactgtcctgtggagaacattttgggaaacgctgttagatagttctttaaggagacaaaacggtaatgaacacatggcactggggcagaattcacatgcattttgtaacatccagtgtggcatggaatagatgtgtatttcctcccctaaagaaaataagcacagaaaattatattgtaggtgatcggagctctttcctttgatagaaagaacagccccaatgatcctggctttttcactgaacatatcagaatacatggatgagttggggttaataaggttttcattcagatgtagaagaaagtattgtacaattgaatgcagatttttatccacagacagttgtagtgtttagacgtgacaggacctattgttgaggtttataagacttactatgggctgtaaacctattttttaaaactctttttagaaacctgagacttgtcatctggcattttagtttaatacaaactaatgattgcatttgaaagagattcttgaccttatttctgaacatctaaagctctgaaatgtcttgatggaaggtattaaactatttgcctgttgtataaagaaatgttaagactgttgtgaaaagaattactgtaaggtactgtgaaatgactgtgatttttgtgagcgaaacatacttggaaatactgaattgatttttatgcttgttaatgtattgcaagaaacacagaaaatgtagttttgttttaataaac

SEQ ID NO: 12 - RNA, 6262 nt, Macaca mulatta
  source 1..6262: mol_type = mRNA
gtttattaaaacaaaactacattttctgtgtttcttgcaatacattaacaagcataaaaatcaattcagtatttccaagtatgtttcgctcacaaaaatcacagtcatttcacagtaccttacagtaattcttttcacaacagtcttaacatttctttatacaacaggcaaatagtttaataccttccatcaagacatttcagagctttagatgttcagaaataaggtcaagaatctctttcaaatgcaatcattagtttgtattaaactaaaatgccagatgacaagtctcaggtttctaaaaagagttttaaaaaataggtttacagcccatagtaagtcttataaacctcaacaataggtcctgtcacgtctaaacactacaactgtctgtggataaaaatctgcattcaattgtacaatactttcttctacatctgaatgaaaaccttattaaccccaactcatccatgtattctgatatgttcagtgaaaaagccaggatcattggggctgttctttctatcaaaggaaagagctccgatcacctacaatataattttctgtgcttattttctttaggggaggaaatacacatctattccatgccacactggatgttacaaaatgcatgtgaattctgccccagtgccatgtgttcattaccgttttgtctccttaaagaactatctaacagcgtttcccaaaatgttctccacaggacagtagtgagaggttcacaggtatcccaaaggagaaaaaggtcctgatgtcaaaatagtttgggcaatgctgggttgaacagtttttcactgccagatgccaagcccttactgcgctaaagtgcattgtaagtctccatgtgcaaacttagttcccagcaacaccatttctataaaacactgatgaacatctcacagagcactcatattacatggagtactatgggaaatgcttttcccggtccaggttactggaaattccacaatctgggattacattcattgtaatcccagaaatattttctccatataccctcatgactttgtgagatttaacagatttcagaaggaagactcaatgccgtctcagttaacagttctacacatttcacactagtttttgccttgtttttcatgcaattttaagagtacataaattccttcctctcttctgaatcacttaggacattctcatttttaaaaacagagagcagttgcatattgcttaatatttttttttaacttgactcacagtcttcccctgaagggcatgcatttcatgttatagaaatgcaatagagtaaactgtaataaaattatttacaagcacctagtttgtttaaccttacatggaagccatcgctgttggaaaacaatgagaacgtatcttttagcaaaatggtgctatctggaagctttattgtgaagatgctttcttttttgctttttgtttttcggtcatgaggcactgaagaatgagttgtgctgaaattaactcaaaggtcagcttgtctggatgagcataactttggttgagatttttctcccttaaaaaagattttcaaagcaccagttaattacaaaatgcatgcatatttatcctcacagtgacttaagtggtaagagagctagcaaatcatacattgcattcctcaaagcatctgatcaaacttctcgaaaacaaaccaaccaaaagggaaaataatgcaagagaagccatattttctctgcttaggctggcgaagcagcagctctttgcagcagtgacaggcagggcagagtatccactgggaagtgagtcccaaccttgaataatggtgagcttgagtaatccttaatctacaatttaaaggatgaaaaaaagagactagtgaaatgcttgattccccacataaggaacacccaagactccctgggtatcctccaaatgtagccgagaaaagtgttcttccaccctagtcagtaaaatggaatgctaaaacgtgattatctcattaacatcagagctactacaactgacaatgacttaacagtacctcaattcctatcaagaaaaaatatcttttaaatgcagaacttgagagggatcacaacagcatagcattattgctaccagtttcaaacgtgatacttcatacaatgtgaaatatcaatcagcatccctccctctcccaaaacacacgttactcatgagacactattagtgtttaaaacccaagcttatagaagtacaaacttaattctcagtatttttatactaaattcaaagaaactatgtaacactcatctggaaaaattcttaattccataatatcttagagataagcaacagtaaactgttagaaaatgttttaacattacatgatatttaagaaatcaccataattaccataataaactaataattatgctccctgttcacaaaaggcacctaccaattatgaacagaccatttttcataattatttaccactatgtggcataatggtttaggcatataacccataaaaatttgttaaaagtcatggtttttcctcaaagctaaaaattcacaaatgcctctaaccattaccagtcagtagggccaccacatgcatatactggacaggttgtgcacggcacaactcaagtgggcaccagtcacctggactggggtgcagtacacaatctgtgtgcagtacagaaagccctcatcagttgtggccagagcactgtattctaacagagtctgtcagctcaagctaatcaagttaggaaagttgctatttggttggaggatttccaagaaacagctgtacccgtgagaagcaggtattacctgaggggtagacggggtacagacataaaacaggaagggttctaaatatttgctggtcatttaaaactcaatggcacttttttatatgagcaaaagccttcaacaccagttttctggccaagtttccctagaattttgccagccaaattaacttcctgatgttaactatttgattacaatatctcagttcccgacctaaactaatactgtctgttttcacatacctcttaaaaacattttctatatctgactgcaaaggacagcacagtgatacctgggtgtgatatatatcagtccattcatttataaagcacttgggataaaaggtactcccattaaaaatgtagctactattgacaaagataaaactgaaaaagagtgaatggatgactcaattatttttaaaggaagcattaaccattaaccagataatataccaacaaattacccaatagcactaagtataccatataagattcagttctagaacacagctacatttctgtgtccatcacagtaattagtccttaaaagttgtacttaaaatgtcaatctttaataaactccaaaataatgtattgagatttcatcttgtagtctacggattgtgagttgcgaatagaggctgaggtccccccaagtgttatctgcaggctgctgtgtggatgcagagctgggaagatcacagatccatggagggagaaggcacttgtcttccaggagatcactgcgggacagggcaggcgtgaccttgcgacggcaccttcaactctcgagccagaagctggtacctacaagggactcatctcatgaccttcatttgccagcggtgccacacgttacctacagcaccacaaaactcagaatatattctagaagtttttgccggttgcattgaggtagaaaagtgctgctcagttctaaaacagacactctcttttgtttggtctccttgaaaaccccaatatccttaaacattttcacagcattcttcacaagacagtatgtggcactctcagcatatactgcaacatttctttctgttctggttactaggtatttgtgcaacttttgcagatattcaggttctggaacagggccgctaaagttgtgaacaaagatggcagcagagctgtaggcctccagcaaaggcccaaggagtctctgtaagaaggtgataaactgctggtgctccttggattggctcaccttcaggtagcaatctcgctgttcctccccaaagtcactgtcttcatcttcttcatcacttctccaagacaaaggttcaggaagcttcttgtcccactgctgctcagcaagactaggactgatatcttcctggtcatcgtgctctgccactgtaagaatgccatactggataaactttcctactgtttcatggcacacttggtaaaatgtctggcaaggcagtgagatggtgccctcattggagagaaggtagcacaggctggccgccttccgcaccagctgctcctggctgatcaggttaggtggggtgccagtgggcccccctaatcccctcttgttcagaactgcataaaggctgcaagctatgatggcctccatgataaagacatgaagtaccccattgctgtagaagttgagttcgaagactgctgggacagttgtgctgggggtgataaaaaactcatcgttcctgctagtgtgagtgattgtgacgcaatttcccagcagctgtatggcatgcattactacatcttctgaatttcctgagaaccccaggtcaaaatcacgagccaggacttcctctttcatcacaaagaagtcttccaccaatgtggagagatcaattccctgcctgtgtctgtagaggagtaggcaagccacaatgtgtgtggacataatggcacaggacttgctagcagtgaatagaatatgctcagccagatttgcaatcaacctccttcgtaggaattcatctgttgcatttctggactcattaatggatgtgtctctaccttcatcagcagcatcattgggtcttgaaggaagtatagctggtaacaacgcttgctccagagaaagtggagcagacaccggtttctgactttggctttctaaatattcctttaaggaaaacggctgtgcaaaatccactcggacacaaccatagttttttcgtaacattctaataacacctcttgctatactccacaggctctcattcttctttggcttgcccagttgttcgccattgtagtgaccttcgataatacgatcataggagattccaacaggtattatcaagatgtctgggatgacattggtagatagagtatctaccacaactgacaaaagtcccgcccgagcacaggaggtttttccactcctagaacgtgtgccttccaggaagatctccaagaattgctgctgtcgaagtaattcaactatatgcccatggagcaaagctctgtagagaacatctttccgtccatctggtgtttcatcgagccttcgtcgtatgaagaagcccccaagcttatggatcaaagtactgaagattgggatatggagattattgcctgaagcaatgtatggtgctttgatgttatggcagaagagaatgaaagtgagcagcagatagtcaatatgggatctatgaactggtagaaacagaagcggcaaattcgtctcagttgcagctttaaccatctcaagttgacctttgtgaatttgaatgttccaaaagaagctgttgaacagttttagcagcacccacccagtcagtctgatcattgccggtgagacagtggcaaccatttcttgaagaatccttttagctttctttttcactttgttaacggcttttgattgctgctgggcagaaccatcagggtttaattcagcagccacttctgcaattgcctcttgtactctactgctgttcagcacattttcagtcacattggtggcaaacatgcccttatgcacatctcgctcttgaataaaaagaacataagaaaggcgtcttgcaagccatccccggtgtcttgtgtgagtttcattgatataaataacattccgcaaacccaaagacgggatactggggttgaaaaatctgtcccagctctggggagtgcaggagtaacaacatcttccaacaaatggccttttccgactcattaggctttctttccattttaaagttgcagatctgaagacagtaggtctaaaaccacactcaccccattcctcacttgtgtgcttacatcgaccaacactgtattctgatgaattcggcagataagaaacatctattgtaccaagggtcagtgcagattcatccatgtcacaaagtgtaattcccaaatcatgtgctgggatgaaagttcttctgtttcataacataaaacttcaggactcagctatcagtttcgggtgcagaatgtccatacaacag

SEQ ID NO: 13 - RNA, 6530 nt, Macaca fascicularis
  source 1..6530: mol_type = mRNA
tgtggtgtttcaaaactgctctgggagaatttgctgttgcgggggggactctttctgaggttactgtggagcacccaaagtccgtcagcctctggccgtgcagaggggcacccagaggaagtagaccttgcttcttattcacccacagcctgggactgtcttctccagagtctccatcacctttgctaatcgactgattggaaataattcctcaaacaccaccaagtcaaggatacaggcagcagcggctcccctgttgtatggacattctgcacccgaaactgatagctgagtcctgaagttttatgttatgaaacagaagaactttcatcccagcacatgatttgggaattacactttgtgacatggatgaatctgcactgacccttggtacaatagatgtttcttatctgccgaattcatcagaatacagtgttggtcgatgtaagcacacaagtgaggaatggggtgagtgtggttttagacctactgtcttcagatctgcaactttaaaatggaaagaaagcctaatgagtcggaaaaggccatttgttggaagatgttgttactcctgcactccccagagctgggacagatttttcaaccccagtatcccatctttgggtttgcggaatgttatttatatcaatgaaactcacacaagacaccggggatggcttgcaagacgcctttcttatgttctttttattcaagagcgagatgtgcataagggcatgtttgccaccaatgtgactgaaaatgtgctgaacagcagtagagtacaagaggcaattgcagaagtggctgctgaattaaaccctgatggttctgcccagcagcaatcaaaagccgttaacaaagtgaaaaagaaagctaaaaggattcttcaagaaatggttgccactgtctcaccggcaatgatcagactgactgggtgggtgctgctaaaactgttcaacagcttcttttggaacattcaaattcacaaaggtcaacttgagatggttaaagctgcaactgagacgaatttgccgcttctgtttctaccagttcatagatcccatattgactatctgctgctcactttcattctcttctgccataacatcaaagcaccatacattgcttcaggcaataatctccatatcccaatcttcagtactttgatccataagcttgggggcttcttcatacgacgaaggctcgatgaaacaccagatggacggaaagatgttctctacagagctttgctccatgggcatatagttgaattacttcgacagcagcaattcttggagatcttcctggaaggcacacgttctaggagtggaaaaacctcctgtgctcgggcgggacttttgtcagttgtggtagatactctatctaccaatgtcatcccagacatcttgataatacctgttggaatctcctatgatcgtattatcgaaggtcactacaatggcgaacaactgggcaagccaaagaagaatgagagcctgtggagtatagcaagaggtgttattagaatgttacgaaaaaactatggttgtgtccgagtggattttgcacagccgttttccttaaaggaatatttagaaagccaaagtcagaaaccggtgtctgctccactttctctggagcaagcgttgttaccagctatacttccttcaagacccaatgatgctgctgatgaaggtagagacacatccattaatgagtccagaaatgcaacagatgaattcctacgaaggaggttgattgcaaatctggctgagcatattctattcactgctagcaagtcctgtgccattatgtccacacacattgtggcttgcctactcctctacagacacaggcagggaattgatctctccacattggtggaagacttctttgtgatgaaagaggaagtcctggctcgtgattttgacctggggttctcaggaaattcagaagatgtagtaatgcatgccatacagctgctgggaaattgcgtcacaatcactcacactagcaggaacgatgagttttttatcacccccagcacaactgtcccagcagtcttcgaactcaacttctacagcaatggggtacttcatgtctttatcatggaggccatcatagcttgcagcctttatgcagttctgaacaagaggggattaggggggcccactggcaccccacctaacctgatcagccaggagcagctggtgcggaaggcggccagcctgtgctaccttctctccaatgagggcaccatctcactgccttgccagacattttaccaagtgtgccatgaaacagtaggaaagtttatccagtatggcattcttacagtggcagagcacgatgaccaggaagatatcagtcctagtcttgctgagcagcagtgggacaagaagcttcctgaacctttgtcttggagaagtgatgaagaagatgaagacagtgactttggggaggaacagcgagattgctacctgaaggtgagccaatccaaggagcaccagcagtttatcaccttcttacagagactccttgggcctttgctggaggcctacagctctgctgccatctttgttcacaactttagcggccctgttccagaacctgaatatctgcaaaagttgcacaaatacctagtaaccagaacagaaagaaatgttgcagtatatgctgagagtgccacatactgtcttgtgaagaatgctgtgaaaatgtttaaggatattggggttttcaaggagaccaaacaaaagagagtgtctgttttagaactgagcagcacttttctacctcaatgcaaccggcaaaaacttctagaatatattctgagttttgtggtgctgtaggtaacgtgtggcaccgctggcaaatgaaggtcatgagatgagtcccttgtaggtaccagcttctggctcgagagttgaaggtgccgtcgcaaggtcacgcctgccctgtcccgcagtgatctcctggaagacaagtgccttctccctccatggatctgtgatcttcccagctctgcatccacacagcagcctgcagataacacttggggggacctcagcctctattcgcaactcacaatccgtagactacaagatgaaatctcaatacattattttggagtttattaaagattgacattttaagtacaacttttaaggactaattactgtgatggacacagaaatgtagctgtgttctagaactgaatcttatatggtatacttagtgctattgggtaatttgttggtatattatctggttaatggttaatgcttcctttaaaaataattgagtcatccattcactctttttcagttttatctttgtcaatagtagctacatttttaatgggagtaccttttatcccaagtgctttataaatgaatggactgatatatatcacacccaggtatcactgtgctgtcctttgcagtcagatatagaaaatgtttttaagaggtatgtgaaaacagacagtattagtttaggtcgggaactgagatattgtaatcaaatagttaacatcaggaagttaatttggctggcaaaattctagggaaacttggccagaaaactggtgttgaaggcttttgctcatataaaaaagtgccattgagttttaaatgaccagcaaatatttagaacccttcctgttttatgtctgtaccccgtctacccctcaggtaatacctgcttctcacgggtacagctgtttcttggaaatcctccaaccaaatagcaactttcctaacttgattagcttgagctgacagactctgttagaatacagtgctctggccacaactgatgagggctttctgtactgcacacagattgtgtactgcaccccagtccaggtgactggtgcccacttgagttgtgccgtgcacaacctgtccagtatatgcatgtggtggccctactgactggtaatggttagaggcatttgtgaatttttagctttgaggaaaaaccatgacttttaacaaatttttatgggttatatgcctaaaccattatgccacgtagtggtaaataattatgaaaaatggtctgttcataattggtaggtgccttttgtgaacagggagcataattattagtttattatggtaattatggtgatttcttgaatatcatgtaatgttaaaacattttctaacagtttactgttgcttatctctaagatattatggaattaagaatttttccagatgagtgttacatagtttctttgaatttagtataaaaatactgagaattaagtttgtacttctataagcttgggttttaaacactaatagtgtctcatgagtaacgtgtgttttgggagagggagggatgctgattgatatttcacattgtatgaagtatcacgtttgaaactggtagcaataatgctatgctgttgtgatccctctcaagttctgcatttaaaagatattttttcttgataggaattgaggtactgttaagtcattgtcagttgtagtagctctgatgttaatgagataatcacgttttagcattccattttactgactagggtggaagaacacttttctcggctacatttggaggatacccagggagtcttgggtgttccttatgtggggaatcaaacatttcactagtctctttttttcatcctttaaattgtagattaaggattactcaagctcaccattattcaaggttgggactcacttcccagtggatactctgccctgcctgtcactgctgcaaagagctgctgcttcgccagcctaagcagagaaaatatggcttctcttgcattattttcccttttggttggtttgttttctagaagtttgatcagatgctttgaggaatgcaatgtatgatttgctagctctcttaccacttaagtcactgtgaggataaatatgcatgcattttgtaattaactggtgctttgaaaatcttttttaagggagaaaaatctcaaccaaagttatgctcatccagacaagctgacctttgagttaatttcagcacaactcattcttcagtgcctcatgaccgaaaaacaaaaaacaaaaaagaaagcatcttcacaataaagcttccagatagcaccgttttgctaaaagatacgttctcattgttttccaacagtgatggcttccatgtaaggttaaacaaactaggtgcttgtaaataattttattacagtttactctattgcatttctataacatgaaatgcatgcccttcaggggaagactgtgagtcaagttaaaaaaaaatattaagcaatatgcaactgctctctgtttttaaaaatgagaatgtcctaagtgattcagaagagaggaaggaatttatgtactcttaaaattgcatgaaaaacaaggcaaaaactagtgtgaaatgtgtagaactgttaactgagatggcattgagtcttccttctgaaatctgttaaatctcacaaagtcatgagggtatatggagaaaatatttctgggattacaatgaatgtaatcccagattgtggaatttccagtaacctggaccgggaaaagcatttcccatagtactccatgtaatatgagtgctctgtgagatgttcatcagtgttttatagaaatggtgttgctgggaactaagtttgcacatggagacttacaatgcactttagcgcagtaagggcttggcatctggcagtgaaaaactgttcaacccagcattgcccaaactattttgacatcaggacctttttctcctttgggatacctgtgaacctctcactactgtcctgtggagaacattttgggaaacactgttagatagttctttaaggagacaaaacggtaatgaacacatggcactggggcagaattcacatgcattttgtaacatccagtgtggcatggaatagatgtgtatttcctcccctaaagaaaataagcacagaaaattatattgtaggtgatcggagctctttcctttgatagaaagaacagccccaatgatcctggctttttcactgaacatatcagaatacatggatgagttggggttaataaggttttcattcagatgtagaagaaagtattgtacaattgaatgcagatttttatccacagacagttgtagtgtttagacgtgacaggacctatcgttgaggtttataagacttactatgggctgtaaacctattttttaaaactctttttagaaacctgagacttgtcatctggcattttagtttaatacaaactaatgattgcatttgaaagagattcttgaccttatttctgaacatctaaagctctgaaatgtcttgatggaaggtattaaactatttgcctgttgtataaagaaatgttaagactgttgtgaaaagaattactgtaaggtactgtgaaatgactgtgatttttgtgagcgaaacatacttggaaatactgaattgatttttatgcttgttaatgtattgcaagaaacacagaaaatgtaattttgttttaataaaccaaaaaatgaacata

SEQ ID NO: 14 - RNA, 6530 nt, Macaca fascicularis
  source 1..6530: mol_type = mRNA
tatgttcattttttggtttattaaaacaaaattacattttctgtgtttcttgcaatacattaacaagcataaaaatcaattcagtatttccaagtatgtttcgctcacaaaaatcacagtcatttcacagtaccttacagtaattcttttcacaacagtcttaacatttctttatacaacaggcaaatagtttaataccttccatcaagacatttcagagctttagatgttcagaaataaggtcaagaatctctttcaaatgcaatcattagtttgtattaaactaaaatgccagatgacaagtctcaggtttctaaaaagagttttaaaaaataggtttacagcccatagtaagtcttataaacctcaacgataggtcctgtcacgtctaaacactacaactgtctgtggataaaaatctgcattcaattgtacaatactttcttctacatctgaatgaaaaccttattaaccccaactcatccatgtattctgatatgttcagtgaaaaagccaggatcattggggctgttctttctatcaaaggaaagagctccgatcacctacaatataattttctgtgcttattttctttaggggaggaaatacacatctattccatgccacactggatgttacaaaatgcatgtgaattctgccccagtgccatgtgttcattaccgttttgtctccttaaagaactatctaacagtgtttcccaaaatgttctccacaggacagtagtgagaggttcacaggtatcccaaaggagaaaaaggtcctgatgtcaaaatagtttgggcaatgctgggttgaacagtttttcactgccagatgccaagcccttactgcgctaaagtgcattgtaagtctccatgtgcaaacttagttcccagcaacaccatttctataaaacactgatgaacatctcacagagcactcatattacatggagtactatgggaaatgcttttcccggtccaggttactggaaattccacaatctgggattacattcattgtaatcccagaaatattttctccatataccctcatgactttgtgagatttaacagatttcagaaggaagactcaatgccatctcagttaacagttctacacatttcacactagtttttgccttgtttttcatgcaattttaagagtacataaattccttcctctcttctgaatcacttaggacattctcatttttaaaaacagagagcagttgcatattgcttaatatttttttttaacttgactcacagtcttcccctgaagggcatgcatttcatgttatagaaatgcaatagagtaaactgtaataaaattatttacaagcacctagtttgtttaaccttacatggaagccatcactgttggaaaacaatgagaacgtatcttttagcaaaacggtgctatctggaagctttattgtgaagatgctttcttttttgttttttgtttttcggtcatgaggcactgaagaatgagttgtgctgaaattaactcaaaggtcagcttgtctggatgagcataactttggttgagatttttctcccttaaaaaagattttcaaagcaccagttaattacaaaatgcatgcatatttatcctcacagtgacttaagtggtaagagagctagcaaatcatacattgcattcctcaaagcatctgatcaaacttctagaaaacaaaccaaccaaaagggaaaataatgcaagagaagccatattttctctgcttaggctggcgaagcagcagctctttgcagcagtgacaggcagggcagagtatccactgggaagtgagtcccaaccttgaataatggtgagcttgagtaatccttaatctacaatttaaaggatgaaaaaaagagactagtgaaatgtttgattccccacataaggaacacccaagactccctgggtatcctccaaatgtagccgagaaaagtgttcttccaccctagtcagtaaaatggaatgctaaaacgtgattatctcattaacatcagagctactacaactgacaatgacttaacagtacctcaattcctatcaagaaaaaatatcttttaaatgcagaacttgagagggatcacaacagcatagcattattgctaccagtttcaaacgtgatacttcatacaatgtgaaatatcaatcagcatccctccctctcccaaaacacacgttactcatgagacactattagtgtttaaaacccaagcttatagaagtacaaacttaattctcagtatttttatactaaattcaaagaaactatgtaacactcatctggaaaaattcttaattccataatatcttagagataagcaacagtaaactgttagaaaatgttttaacattacatgatattcaagaaatcaccataattaccataataaactaataattatgctccctgttcacaaaaggcacctaccaattatgaacagaccatttttcataattatttaccactacgtggcataatggtttaggcatataacccataaaaatttgttaaaagtcatggtttttcctcaaagctaaaaattcacaaatgcctctaaccattaccagtcagtagggccaccacatgcatatactggacaggttgtgcacggcacaactcaagtgggcaccagtcacctggactggggtgcagtacacaatctgtgtgcagtacagaaagccctcatcagttgtggccagagcactgtattctaacagagtctgtcagctcaagctaatcaagttaggaaagttgctatttggttggaggatttccaagaaacagctgtacccgtgagaagcaggtattacctgaggggtagacggggtacagacataaaacaggaagggttctaaatatttgctggtcatttaaaactcaatggcacttttttatatgagcaaaagccttcaacaccagttttctggccaagtttccctagaattttgccagccaaattaacttcctgatgttaactatttgattacaatatctcagttcccgacctaaactaatactgtctgttttcacatacctcttaaaaacattttctatatctgactgcaaaggacagcacagtgatacctgggtgtgatatatatcagtccattcatttataaagcacttgggataaaaggtactcccattaaaaatgtagctactattgacaaagataaaactgaaaaagagtgaatggatgactcaattatttttaaaggaagcattaaccattaaccagataatataccaacaaattacccaatagcactaagtataccatataagattcagttctagaacacagctacatttctgtgtccatcacagtaattagtccttaaaagttgtacttaaaatgtcaatctttaataaactccaaaataatgtattgagatttcatcttgtagtctacggattgtgagttgcgaatagaggctgaggtccccccaagtgttatctgcaggctgctgtgtggatgcagagctgggaagatcacagatccatggagggagaaggcacttgtcttccaggagatcactgcgggacagggcaggcgtgaccttgcgacggcaccttcaactctcgagccagaagctggtacctacaagggactcatctcatgaccttcatttgccagcggtgccacacgttacctacagcaccacaaaactcagaatatattctagaagtttttgccggttgcattgaggtagaaaagtgctgctcagttctaaaacagacactctcttttgtttggtctccttgaaaaccccaatatccttaaacattttcacagcattcttcacaagacagtatgtggcactctcagcatatactgcaacatttctttctgttctggttactaggtatttgtgcaacttttgcagatattcaggttctggaacagggccgctaaagttgtgaacaaagatggcagcagagctgtaggcctccagcaaaggcccaaggagtctctgtaagaaggtgataaactgctggtgctccttggattggctcaccttcaggtagcaatctcgctgttcctccccaaagtcactgtcttcatcttcttcatcacttctccaagacaaaggttcaggaagcttcttgtcccactgctgctcagcaagactaggactgatatcttcctggtcatcgtgctctgccactgtaagaatgccatactggataaactttcctactgtttcatggcacacttggtaaaatgtctggcaaggcagtgagatggtgccctcattggagagaaggtagcacaggctggccgccttccgcaccagctgctcctggctgatcaggttaggtggggtgccagtgggcccccctaatcccctcttgttcagaactgcataaaggctgcaagctatgatggcctccatgataaagacatgaagtaccccattgctgtagaagttgagttcgaagactgctgggacagttgtgctgggggtgataaaaaactcatcgttcctgctagtgtgagtgattgtgacgcaatttcccagcagctgtatggcatgcattactacatcttctgaatttcctgagaaccccaggtcaaaatcacgagccaggacttcctctttcatcacaaagaagtcttccaccaatgtggagagatcaattccctgcctgtgtctgtagaggagtaggcaagccacaatgtgtgtggacataatggcacaggacttgctagcagtgaatagaatatgctcagccagatttgcaatcaacctccttcgtaggaattcatctgttgcatttctggactcattaatggatgtgtctctaccttcatcagcagcatcattgggtcttgaaggaagtatagctggtaacaacgcttgctccagagaaagtggagcagacaccggtttctgactttggctttctaaatattcctttaaggaaaacggctgtgcaaaatccactcggacacaaccatagttttttcgtaacattctaataacacctcttgctatactccacaggctctcattcttctttggcttgcccagttgttcgccattgtagtgaccttcgataatacgatcataggagattccaacaggtattatcaagatgtctgggatgacattggtagatagagtatctaccacaactgacaaaagtcccgcccgagcacaggaggtttttccactcctagaacgtgtgccttccaggaagatctccaagaattgctgctgtcgaagtaattcaactatatgcccatggagcaaagctctgtagagaacatctttccgtccatctggtgtttcatcgagccttcgtcgtatgaagaagcccccaagcttatggatcaaagtactgaagattgggatatggagattattgcctgaagcaatgtatggtgctttgatgttatggcagaagagaatgaaagtgagcagcagatagtcaatatgggatctatgaactggtagaaacagaagcggcaaattcgtctcagttgcagctttaaccatctcaagttgacctttgtgaatttgaatgttccaaaagaagctgttgaacagttttagcagcacccacccagtcagtctgatcattgccggtgagacagtggcaaccatttcttgaagaatccttttagctttctttttcactttgttaacggcttttgattgctgctgggcagaaccatcagggtttaattcagcagccacttctgcaattgcctcttgtactctactgctgttcagcacattttcagtcacattggtggcaaacatgcccttatgcacatctcgctcttgaataaaaagaacataagaaaggcgtcttgcaagccatccccggtgtcttgtgtgagtttcattgatataaataacattccgcaaacccaaagatgggatactggggttgaaaaatctgtcccagctctggggagtgcaggagtaacaacatcttccaacaaatggccttttccgactcattaggctttctttccattttaaagttgcagatctgaagacagtaggtctaaaaccacactcaccccattcctcacttgtgtgcttacatcgaccaacactgtattctgatgaattcggcagataagaaacatctattgtaccaagggtcagtgcagattcatccatgtcacaaagtgtaattcccaaatcatgtgctgggatgaaagttcttctgtttcataacataaaacttcaggactcagctatcagtttcgggtgcagaatgtccatacaacaggggagccgctgctgcctgtatccttgacttggtggtgtttgaggaattatttccaatcagtcgattagcaaaggtgatggagactctggagaagacagtcccaggctgtgggtgaataagaagcaaggtctacttcctctgggtgcccctctgcacggccagaggctgacggactttgggtgctccacagtaacctcagaaagagtcccccccgcaacagcaaattctcccagagcagttttgaaacaccaca

SEQ ID NO: 15 - RNA, 6413 nt, Macaca fascicularis
  source 1..6413: mol_type = mRNA
gcattggccgggacttgaagtgcggggtgctgcagcagccgaagccggagctgctagggtgcgaactgcgagagcaggtgtgggctgcgagaggctgctctggccgggagcgccgggacaagcagcagcggctcccctgttgtatggacattctgcacccgaaactgatagctgagtcctgaagttttatgttatgaaacagaagaactttcatcccagcacatgatttgggaattacactttgtgacatggatgaatctgcactgacccttggtacaatagatgtttcttatctgccgaattcatcagaatacagtgttggtcgatgtaagcacacaagtgaggaatggggtgagtgtggttttagacctactgtcttcagatctgcaactttaaaatggaaagaaagcctaatgagtcggaaaaggccatttgttggaagatgttgttactcctgcactccccagagctgggacagatttttcaaccccagtatcccatctttgggtttgcggaatgttatttatatcaatgaaactcacacaagacaccggggatggcttgcaagacgcctttcttatgttctttttattcaagagcgagatgtgcataagggcatgtttgccaccaatgtgactgaaaatgtgctgaacagcagtagagtacaagaggcaattgcagaagtggctgctgaattaaaccctgatggttctgcccagcagcaatcaaaagccgttaacaaagtgaaaaagaaagctaaaaggattcttcaagaaatggttgccactgtctcaccggcaatgatcagactgactgggtgggtgctgctaaaactgttcaacagcttcttttggaacattcaaattcacaaaggtcaacttgagatggttaaagctgcaactgagacgaatttgccgcttctgtttctaccagttcatagatcccatattgactatctgctgctcactttcattctcttctgccataacatcaaagcaccatacattgcttcaggcaataatctccatatcccaatcttcagtactttgatccataagcttgggggcttcttcatacgacgaaggctcgatgaaacaccagatggacggaaagatgttctctacagagctttgctccatgggcatatagttgaattacttcgacagcagcaattcttggagatcttcctggaaggcacacgttctaggagtggaaaaacctcctgtgctcgggcgggacttttgtcagttgtggtagatactctatctaccaatgtcatcccagacatcttgataatacctgttggaatctcctatgatcgtattatcgaaggtcactacaatggcgaacaactgggcaagccaaagaagaatgagagcctgtggagtatagcaagaggtgttattagaatgttacgaaaaaactatggttgtgtccgagtggattttgcacagccgttttccttaaaggaatatttagaaagccaaagtcagaaaccggtgtctgctccactttctctggagcaagcgttgttaccagctatacttccttcaagacccaatgatgctgctgatgaaggtagagacacatccattaatgagtccagaaatgcaacagatgaattcctacgaaggaggttgattgcaaatctggctgagcatattctattcactgctagcaagtcctgtgccattatgtccacacacattgtggcttgcctactcctctacagacacaggcagggaattgatctctccacattggtggaagacttctttgtgatgaaagaggaagtcctggctcgtgattttgacctggggttctcaggaaattcagaagatgtagtaatgcatgccatacagctgctgggaaattgcgtcacaatcactcacactagcaggaacgatgagttttttatcacccccagcacaactgtcccagcagtcttcgaactcaacttctacagcaatggggtacttcatgtctttatcatggaggccatcatagcttgcagcctttatgcagttctgaacaagaggggattaggggggcccactggcaccccacctaacctgatcagccaggagcagctggtgcggaaggcggccagcctgtgctaccttctctccaatgagggcaccatctcactgccttgccagacattttaccaagtgtgccatgaaacagtaggaaagtttatccagtatggcattcttacagtggcagagcacgatgaccaggaagatatcagtcctagtcttgctgagcagcagtgggacaagaagcttcctgaacctttgtcttggagaagtgatgaagaagatgaagacagtgactttggggaggaacagcgagattgctacctgaaggtgagccaatccaaggagcaccagcagtttatcaccttcttacagagactccttgggcctttgctggaggcctacagctctgctgccatctttgttcacaactttagcggccctgttccagaacctgaatatctgcaaaagttgcacaaatacctagtaaccagaacagaaagaaatgttgcagtatatgctgagagtgccacatactgtcttgtgaagaatgctgtgaaaatgtttaaggatattggggttttcaaggagaccaaacaaaagagagtgtctgttttagaactgagcagcacttttctacctcaatgcaaccggcaaaaacttctagaatatattctgagttttgtggtgctgtaggtaacgtgtggcaccgctggcaaatgaaggtcatgagatgagtcccttgtaggtaccagcttctggctcgagagttgaaggtgccgtcgcaaggtcacgcctgccctgtcccgcagtgatctcctggaagacaagtgccttctccctccatggatctgtgatcttcccagctctgcatccacacagcagcctgcagataacacttggggggacctcagcctctattcgcaactcacaatccgtagactacaagatgaaatctcaatacattattttggagtttattaaagattgacattttaagtacaacttttaaggactaattactgtgatggacacagaaatgtagctgtgttctagaactgaatcttatatggtatacttagtgctattgggtaatttgttggtatattatctggttaatggttaatgcttcctttaaaaataattgagtcatccattcactctttttcagttttatctttgtcaatagtagctacatttttaatgggagtaccttttatcccaagtgctttataaatgaatggactgatatatatcacacccaggtatcactgtgctgtcctttgcagtcagatatagaaaatgtttttaagaggtatgtgaaaacagacagtattagtttaggtcgggaactgagatattgtaatcaaatagttaacatcaggaagttaatttggctggcaaaattctagggaaacttggccagaaaactggtgttgaaggcttttgctcatataaaaaagtgccattgagttttaaatgaccagcaaatatttagaacccttcctgttttatgtctgtaccccgtctacccctcaggtaatacctgcttctcacgggtacagctgtttcttggaaatcctccaaccaaatagcaactttcctaacttgattagcttgagctgacagactctgttagaatacagtgctctggccacaactgatgagggctttctgtactgcacacagattgtgtactgcaccccagtccaggtgactggtgcccacttgagttgtgccgtgcacaacctgtccagtatatgcatgtggtggccctactgactggtaatggttagaggcatttgtgaatttttagctttgaggaaaaaccatgacttttaacaaatttttatgggttatatgcctaaaccattatgccacgtagtggtaaataattatgaaaaatggtctgttcataattggtaggtgccttttgtgaacagggagcataattattagtttattatggtaattatggtgatttcttgaatatcatgtaatgttaaaacattttctaacagtttactgttgcttatctctaagatattatggaattaagaatttttccagatgagtgttacatagtttctttgaatttagtataaaaatactgagaattaagtttgtacttctataagcttgggttttaaacactaatagtgtctcatgagtaacgtgtgttttgggagagggagggatgctgattgatatttcacattgtatgaagtatcacgtttgaaactggtagcaataatgctatgctgttgtgatccctctcaagttctgcatttaaaagatattttttcttgataggaattgaggtactgttaagtcattgtcagttgtagtagctctgatgttaatgagataatcacgttttagcattccattttactgactagggtggaagaacacttttctcggctacatttggaggatacccagggagtcttgggtgttccttatgtggggaatcaaacatttcactagtctctttttttcatcctttaaattgtagattaaggattactcaagctcaccattattcaaggttgggactcacttcccagtggatactctgccctgcctgtcactgctgcaaagagctgctgcttcgccagcctaagcagagaaaatatggcttctcttgcattattttcccttttggttggtttgttttctagaagtttgatcagatgctttgaggaatgcaatgtatgatttgctagctctcttaccacttaagtcactgtgaggataaatatgcatgcattttgtaattaactggtgctttgaaaatcttttttaagggagaaaaatctcaaccaaagttatgctcatccagacaagctgacctttgagttaatttcagcacaactcattcttcagtgcctcatgaccgaaaaacaaaaaacaaaaaagaaagcatcttcacaataaagcttccagatagcaccgttttgctaaaagatacgttctcattgttttccaacagtgatggcttccatgtaaggttaaacaaactaggtgcttgtaaataattttattacagtttactctattgcatttctataacatgaaatgcatgcccttcaggggaagactgtgagtcaagttaaaaaaaaatattaagcaatatgcaactgctctctgtttttaaaaatgagaatgtcctaagtgattcagaagagaggaaggaatttatgtactcttaaaattgcatgaaaaacaaggcaaaaactagtgtgaaatgtgtagaactgttaactgagatggcattgagtcttccttctgaaatctgttaaatctcacaaagtcatgagggtatatggagaaaatatttctgggattacaatgaatgtaatcccagattgtggaatttccagtaacctggaccgggaaaagcatttcccatagtactccatgtaatatgagtgctctgtgagatgttcatcagtgttttatagaaatggtgttgctgggaactaagtttgcacatggagacttacaatgcactttagcgcagtaagggcttggcatctggcagtgaaaaactgttcaacccagcattgcccaaactattttgacatcaggacctttttctcctttgggatacctgtgaacctctcactactgtcctgtggagaacattttgggaaacactgttagatagttctttaaggagacaaaacggtaatgaacacatggcactggggcagaattcacatgcattttgtaacatccagtgtggcatggaatagatgtgtatttcctcccctaaagaaaataagcacagaaaattatattgtaggtgatcggagctctttcctttgatagaaagaacagccccaatgatcctggctttttcactgaacatatcagaatacatggatgagttggggttaataaggttttcattcagatgtagaagaaagtattgtacaattgaatgcagatttttatccacagacagttgtagtgtttagacgtgacaggacctatcgttgaggtttataagacttactatgggctgtaaacctattttttaaaactctttttagaaacctgagacttgtcatctggcattttagtttaatacaaactaatgattgcatttgaaagagattcttgaccttatttctgaacatctaaagctctgaaatgtcttgatggaaggtattaaactatttgcctgttgtataaagaaatgttaagactgttgtgaaaagaattactgtaaggtactgtgaaatgactgtgatttttgtgagcgaaacatacttggaaatactgaattgatttttatgcttgttaatgtattgcaagaaacacagaaaatgtaattttgttttaataaaccaaaaaatgaacata

SEQ ID NO: 16 - RNA, 6413 nt, Macaca fascicularis
  source 1..6413: mol_type = mRNA
tatgttcattttttggtttattaaaacaaaattacattttctgtgtttcttgcaatacattaacaagcataaaaatcaattcagtatttccaagtatgtttcgctcacaaaaatcacagtcatttcacagtaccttacagtaattcttttcacaacagtcttaacatttctttatacaacaggcaaatagtttaataccttccatcaagacatttcagagctttagatgttcagaaataaggtcaagaatctctttcaaatgcaatcattagtttgtattaaactaaaatgccagatgacaagtctcaggtttctaaaaagagttttaaaaaataggtttacagcccatagtaagtcttataaacctcaacgataggtcctgtcacgtctaaacactacaactgtctgtggataaaaatctgcattcaattgtacaatactttcttctacatctgaatgaaaaccttattaaccccaactcatccatgtattctgatatgttcagtgaaaaagccaggatcattggggctgttctttctatcaaaggaaagagctccgatcacctacaatataattttctgtgcttattttctttaggggaggaaatacacatctattccatgccacactggatgttacaaaatgcatgtgaattctgccccagtgccatgtgttcattaccgttttgtctccttaaagaactatctaacagtgtttcccaaaatgttctccacaggacagtagtgagaggttcacaggtatcccaaaggagaaaaaggtcctgatgtcaaaatagtttgggcaatgctgggttgaacagtttttcactgccagatgccaagcccttactgcgctaaagtgcattgtaagtctccatgtgcaaacttagttcccagcaacaccatttctataaaacactgatgaacatctcacagagcactcatattacatggagtactatgggaaatgcttttcccggtccaggttactggaaattccacaatctgggattacattcattgtaatcccagaaatattttctccatataccctcatgactttgtgagatttaacagatttcagaaggaagactcaatgccatctcagttaacagttctacacatttcacactagtttttgccttgtttttcatgcaattttaagagtacataaattccttcctctcttctgaatcacttaggacattctcatttttaaaaacagagagcagttgcatattgcttaatatttttttttaacttgactcacagtcttcccctgaagggcatgcatttcatgttatagaaatgcaatagagtaaactgtaataaaattatttacaagcacctagtttgtttaaccttacatggaagccatcactgttggaaaacaatgagaacgtatcttttagcaaaacggtgctatctggaagctttattgtgaagatgctttcttttttgttttttgtttttcggtcatgaggcactgaagaatgagttgtgctgaaattaactcaaaggtcagcttgtctggatgagcataactttggttgagatttttctcccttaaaaaagattttcaaagcaccagttaattacaaaatgcatgcatatttatcctcacagtgacttaagtggtaagagagctagcaaatcatacattgcattcctcaaagcatctgatcaaacttctagaaaacaaaccaaccaaaagggaaaataatgcaagagaagccatattttctctgcttaggctggcgaagcagcagctctttgcagcagtgacaggcagggcagagtatccactgggaagtgagtcccaaccttgaataatggtgagcttgagtaatccttaatctacaatttaaaggatgaaaaaaagagactagtgaaatgtttgattccccacataaggaacacccaagactccctgggtatcctccaaatgtagccgagaaaagtgttcttccaccctagtcagtaaaatggaatgctaaaacgtgattatctcattaacatcagagctactacaactgacaatgacttaacagtacctcaattcctatcaagaaaaaatatcttttaaatgcagaacttgagagggatcacaacagcatagcattattgctaccagtttcaaacgtgatacttcatacaatgtgaaatatcaatcagcatccctccctctcccaaaacacacgttactcatgagacactattagtgtttaaaacccaagcttatagaagtacaaacttaattctcagtatttttatactaaattcaaagaaactatgtaacactcatctggaaaaattcttaattccataatatcttagagataagcaacagtaaactgttagaaaatgttttaacattacatgatattcaagaaatcaccataattaccataataaactaataattatgctccctgttcacaaaaggcacctaccaattatgaacagaccatttttcataattatttaccactacgtggcataatggtttaggcatataacccataaaaatttgttaaaagtcatggtttttcctcaaagctaaaaattcacaaatgcctctaaccattaccagtcagtagggccaccacatgcatatactggacaggttgtgcacggcacaactcaagtgggcaccagtcacctggactggggtgcagtacacaatctgtgtgcagtacagaaagccctcatcagttgtggccagagcactgtattctaacagagtctgtcagctcaagctaatcaagttaggaaagttgctatttggttggaggatttccaagaaacagctgtacccgtgagaagcaggtattacctgaggggtagacggggtacagacataaaacaggaagggttctaaatatttgctggtcatttaaaactcaatggcacttttttatatgagcaaaagccttcaacaccagttttctggccaagtttccctagaattttgccagccaaattaacttcctgatgttaactatttgattacaatatctcagttcccgacctaaactaatactgtctgttttcacatacctcttaaaaacattttctatatctgactgcaaaggacagcacagtgatacctgggtgtgatatatatcagtccattcatttataaagcacttgggataaaaggtactcccattaaaaatgtagctactattgacaaagataaaactgaaaaagagtgaatggatgactcaattatttttaaaggaagcattaaccattaaccagataatataccaacaaattacccaatagcactaagtataccatataagattcagttctagaacacagctacatttctgtgtccatcacagtaattagtccttaaaagttgtacttaaaatgtcaatctttaataaactccaaaataatgtattgagatttcatcttgtagtctacggattgtgagttgcgaatagaggctgaggtccccccaagtgttatctgcaggctgctgtgtggatgcagagctgggaagatcacagatccatggagggagaaggcacttgtcttccaggagatcactgcgggacagggcaggcgtgaccttgcgacggcaccttcaactctcgagccagaagctggtacctacaagggactcatctcatgaccttcatttgccagcggtgccacacgttacctacagcaccacaaaactcagaatatattctagaagtttttgccggttgcattgaggtagaaaagtgctgctcagttctaaaacagacactctcttttgtttggtctccttgaaaaccccaatatccttaaacattttcacagcattcttcacaagacagtatgtggcactctcagcatatactgcaacatttctttctgttctggttactaggtatttgtgcaacttttgcagatattcaggttctggaacagggccgctaaagttgtgaacaaagatggcagcagagctgtaggcctccagcaaaggcccaaggagtctctgtaagaaggtgataaactgctggtgctccttggattggctcaccttcaggtagcaatctcgctgttcctccccaaagtcactgtcttcatcttcttcatcacttctccaagacaaaggttcaggaagcttcttgtcccactgctgctcagcaagactaggactgatatcttcctggtcatcgtgctctgccactgtaagaatgccatactggataaactttcctactgtttcatggcacacttggtaaaatgtctggcaaggcagtgagatggtgccctcattggagagaaggtagcacaggctggccgccttccgcaccagctgctcctggctgatcaggttaggtggggtgccagtgggcccccctaatcccctcttgttcagaactgcataaaggctgcaagctatgatggcctccatgataaagacatgaagtaccccattgctgtagaagttgagttcgaagactgctgggacagttgtgctgggggtgataaaaaactcatcgttcctgctagtgtgagtgattgtgacgcaatttcccagcagctgtatggcatgcattactacatcttctgaatttcctgagaaccccaggtcaaaatcacgagccaggacttcctctttcatcacaaagaagtcttccaccaatgtggagagatcaattccctgcctgtgtctgtagaggagtaggcaagccacaatgtgtgtggacataatggcacaggacttgctagcagtgaatagaatatgctcagccagatttgcaatcaacctccttcgtaggaattcatctgttgcatttctggactcattaatggatgtgtctctaccttcatcagcagcatcattgggtcttgaaggaagtatagctggtaacaacgcttgctccagagaaagtggagcagacaccggtttctgactttggctttctaaatattcctttaaggaaaacggctgtgcaaaatccactcggacacaaccatagttttttcgtaacattctaataacacctcttgctatactccacaggctctcattcttctttggcttgcccagttgttcgccattgtagtgaccttcgataatacgatcataggagattccaacaggtattatcaagatgtctgggatgacattggtagatagagtatctaccacaactgacaaaagtcccgcccgagcacaggaggtttttccactcctagaacgtgtgccttccaggaagatctccaagaattgctgctgtcgaagtaattcaactatatgcccatggagcaaagctctgtagagaacatctttccgtccatctggtgtttcatcgagccttcgtcgtatgaagaagcccccaagcttatggatcaaagtactgaagattgggatatggagattattgcctgaagcaatgtatggtgctttgatgttatggcagaagagaatgaaagtgagcagcagatagtcaatatgggatctatgaactggtagaaacagaagcggcaaattcgtctcagttgcagctttaaccatctcaagttgacctttgtgaatttgaatgttccaaaagaagctgttgaacagttttagcagcacccacccagtcagtctgatcattgccggtgagacagtggcaaccatttcttgaagaatccttttagctttctttttcactttgttaacggcttttgattgctgctgggcagaaccatcagggtttaattcagcagccacttctgcaattgcctcttgtactctactgctgttcagcacattttcagtcacattggtggcaaacatgcccttatgcacatctcgctcttgaataaaaagaacataagaaaggcgtcttgcaagccatccccggtgtcttgtgtgagtttcattgatataaataacattccgcaaacccaaagatgggatactggggttgaaaaatctgtcccagctctggggagtgcaggagtaacaacatcttccaacaaatggccttttccgactcattaggctttctttccattttaaagttgcagatctgaagacagtaggtctaaaaccacactcaccccattcctcacttgtgtgcttacatcgaccaacactgtattctgatgaattcggcagataagaaacatctattgtaccaagggtcagtgcagattcatccatgtcacaaagtgtaattcccaaatcatgtgctgggatgaaagttcttctgtttcataacataaaacttcaggactcagctatcagtttcgggtgcagaatgtccatacaacaggggagccgctgctgcttgtcccggcgctcccggccagagcagcctctcgcagcccacacctgctctcgcagttcgcaccctagcagctccggcttcggctgctgcagcaccccgcacttcaagtcccggccaatgc

SEQ ID NO: 17 - RNA, 6411 nt, Macaca fascicularis
  source 1..6411: mol_type = mRNA
tccacgcgccggttgcgtcatcatggtgcgccattgcagcaggcattggccgggacttgaagtgcggggtgctgcagcagccgaagccggagctgctagggtgcgaactgcgagagcaggcagcagcggctcccctgttgtatggacattctgcacccgaaactgatagctgagtcctgaagttttatgttatgaaacagaagaactttcatcccagcacatgatttgggaattacactttgtgacatggatgaatctgcactgacccttggtacaatagatgtttcttatctgccgaattcatcagaatacagtgttggtcgatgtaagcacacaagtgaggaatggggtgagtgtggttttagacctactgtcttcagatctgcaactttaaaatggaaagaaagcctaatgagtcggaaaaggccatttgttggaagatgttgttactcctgcactccccagagctgggacagatttttcaaccccagtatcccatctttgggtttgcggaatgttatttatatcaatgaaactcacacaagacaccggggatggcttgcaagacgcctttcttatgttctttttattcaagagcgagatgtgcataagggcatgtttgccaccaatgtgactgaaaatgtgctgaacagcagtagagtacaagaggcaattgcagaagtggctgctgaattaaaccctgatggttctgcccagcagcaatcaaaagccgttaacaaagtgaaaaagaaagctaaaaggattcttcaagaaatggttgccactgtctcaccggcaatgatcagactgactgggtgggtgctgctaaaactgttcaacagcttcttttggaacattcaaattcacaaaggtcaacttgagatggttaaagctgcaactgagacgaatttgccgcttctgtttctaccagttcatagatcccatattgactatctgctgctcactttcattctcttctgccataacatcaaagcaccatacattgcttcaggcaataatctccatatcccaatcttcagtactttgatccataagcttgggggcttcttcatacgacgaaggctcgatgaaacaccagatggacggaaagatgttctctacagagctttgctccatgggcatatagttgaattacttcgacagcagcaattcttggagatcttcctggaaggcacacgttctaggagtggaaaaacctcctgtgctcgggcgggacttttgtcagttgtggtagatactctatctaccaatgtcatcccagacatcttgataatacctgttggaatctcctatgatcgtattatcgaaggtcactacaatggcgaacaactgggcaagccaaagaagaatgagagcctgtggagtatagcaagaggtgttattagaatgttacgaaaaaactatggttgtgtccgagtggattttgcacagccgttttccttaaaggaatatttagaaagccaaagtcagaaaccggtgtctgctccactttctctggagcaagcgttgttaccagctatacttccttcaagacccaatgatgctgctgatgaaggtagagacacatccattaatgagtccagaaatgcaacagatgaattcctacgaaggaggttgattgcaaatctggctgagcatattctattcactgctagcaagtcctgtgccattatgtccacacacattgtggcttgcctactcctctacagacacaggcagggaattgatctctccacattggtggaagacttctttgtgatgaaagaggaagtcctggctcgtgattttgacctggggttctcaggaaattcagaagatgtagtaatgcatgccatacagctgctgggaaattgcgtcacaatcactcacactagcaggaacgatgagttttttatcacccccagcacaactgtcccagcagtcttcgaactcaacttctacagcaatggggtacttcatgtctttatcatggaggccatcatagcttgcagcctttatgcagttctgaacaagaggggattaggggggcccactggcaccccacctaacctgatcagccaggagcagctggtgcggaaggcggccagcctgtgctaccttctctccaatgagggcaccatctcactgccttgccagacattttaccaagtgtgccatgaaacagtaggaaagtttatccagtatggcattcttacagtggcagagcacgatgaccaggaagatatcagtcctagtcttgctgagcagcagtgggacaagaagcttcctgaacctttgtcttggagaagtgatgaagaagatgaagacagtgactttggggaggaacagcgagattgctacctgaaggtgagccaatccaaggagcaccagcagtttatcaccttcttacagagactccttgggcctttgctggaggcctacagctctgctgccatctttgttcacaactttagcggccctgttccagaacctgaatatctgcaaaagttgcacaaatacctagtaaccagaacagaaagaaatgttgcagtatatgctgagagtgccacatactgtcttgtgaagaatgctgtgaaaatgtttaaggatattggggttttcaaggagaccaaacaaaagagagtgtctgttttagaactgagcagcacttttctacctcaatgcaaccggcaaaaacttctagaatatattctgagttttgtggtgctgtaggtaacgtgtggcaccgctggcaaatgaaggtcatgagatgagtcccttgtaggtaccagcttctggctcgagagttgaaggtgccgtcgcaaggtcacgcctgccctgtcccgcagtgatctcctggaagacaagtgccttctccctccatggatctgtgatcttcccagctctgcatccacacagcagcctgcagataacacttggggggacctcagcctctattcgcaactcacaatccgtagactacaagatgaaatctcaatacattattttggagtttattaaagattgacattttaagtacaacttttaaggactaattactgtgatggacacagaaatgtagctgtgttctagaactgaatcttatatggtatacttagtgctattgggtaatttgttggtatattatctggttaatggttaatgcttcctttaaaaataattgagtcatccattcactctttttcagttttatctttgtcaatagtagctacatttttaatgggagtaccttttatcccaagtgctttataaatgaatggactgatatatatcacacccaggtatcactgtgctgtcctttgcagtcagatatagaaaatgtttttaagaggtatgtgaaaacagacagtattagtttaggtcgggaactgagatattgtaatcaaatagttaacatcaggaagttaatttggctggcaaaattctagggaaacttggccagaaaactggtgttgaaggcttttgctcatataaaaaagtgccattgagttttaaatgaccagcaaatatttagaacccttcctgttttatgtctgtaccccgtctacccctcaggtaatacctgcttctcacgggtacagctgtttcttggaaatcctccaaccaaatagcaactttcctaacttgattagcttgagctgacagactctgttagaatacagtgctctggccacaactgatgagggctttctgtactgcacacagattgtgtactgcaccccagtccaggtgactggtgcccacttgagttgtgccgtgcacaacctgtccagtatatgcatgtggtggccctactgactggtaatggttagaggcatttgtgaatttttagctttgaggaaaaaccatgacttttaacaaatttttatgggttatatgcctaaaccattatgccacgtagtggtaaataattatgaaaaatggtctgttcataattggtaggtgccttttgtgaacagggagcataattattagtttattatggtaattatggtgatttcttgaatatcatgtaatgttaaaacattttctaacagtttactgttgcttatctctaagatattatggaattaagaatttttccagatgagtgttacatagtttctttgaatttagtataaaaatactgagaattaagtttgtacttctataagcttgggttttaaacactaatagtgtctcatgagtaacgtgtgttttgggagagggagggatgctgattgatatttcacattgtatgaagtatcacgtttgaaactggtagcaataatgctatgctgttgtgatccctctcaagttctgcatttaaaagatattttttcttgataggaattgaggtactgttaagtcattgtcagttgtagtagctctgatgttaatgagataatcacgttttagcattccattttactgactagggtggaagaacacttttctcggctacatttggaggatacccagggagtcttgggtgttccttatgtggggaatcaaacatttcactagtctctttttttcatcctttaaattgtagattaaggattactcaagctcaccattattcaaggttgggactcacttcccagtggatactctgccctgcctgtcactgctgcaaagagctgctgcttcgccagcctaagcagagaaaatatggcttctcttgcattattttcccttttggttggtttgttttctagaagtttgatcagatgctttgaggaatgcaatgtatgatttgctagctctcttaccacttaagtcactgtgaggataaatatgcatgcattttgtaattaactggtgctttgaaaatcttttttaagggagaaaaatctcaaccaaagttatgctcatccagacaagctgacctttgagttaatttcagcacaactcattcttcagtgcctcatgaccgaaaaacaaaaaacaaaaaagaaagcatcttcacaataaagcttccagatagcaccgttttgctaaaagatacgttctcattgttttccaacagtgatggcttccatgtaaggttaaacaaactaggtgcttgtaaataattttattacagtttactctattgcatttctataacatgaaatgcatgcccttcaggggaagactgtgagtcaagttaaaaaaaaatattaagcaatatgcaactgctctctgtttttaaaaatgagaatgtcctaagtgattcagaagagaggaaggaatttatgtactcttaaaattgcatgaaaaacaaggcaaaaactagtgtgaaatgtgtagaactgttaactgagatggcattgagtcttccttctgaaatctgttaaatctcacaaagtcatgagggtatatggagaaaatatttctgggattacaatgaatgtaatcccagattgtggaatttccagtaacctggaccgggaaaagcatttcccatagtactccatgtaatatgagtgctctgtgagatgttcatcagtgttttatagaaatggtgttgctgggaactaagtttgcacatggagacttacaatgcactttagcgcagtaagggcttggcatctggcagtgaaaaactgttcaacccagcattgcccaaactattttgacatcaggacctttttctcctttgggatacctgtgaacctctcactactgtcctgtggagaacattttgggaaacactgttagatagttctttaaggagacaaaacggtaatgaacacatggcactggggcagaattcacatgcattttgtaacatccagtgtggcatggaatagatgtgtatttcctcccctaaagaaaataagcacagaaaattatattgtaggtgatcggagctctttcctttgatagaaagaacagccccaatgatcctggctttttcactgaacatatcagaatacatggatgagttggggttaataaggttttcattcagatgtagaagaaagtattgtacaattgaatgcagatttttatccacagacagttgtagtgtttagacgtgacaggacctatcgttgaggtttataagacttactatgggctgtaaacctattttttaaaactctttttagaaacctgagacttgtcatctggcattttagtttaatacaaactaatgattgcatttgaaagagattcttgaccttatttctgaacatctaaagctctgaaatgtcttgatggaaggtattaaactatttgcctgttgtataaagaaatgttaagactgttgtgaaaagaattactgtaaggtactgtgaaatgactgtgatttttgtgagcgaaacatacttggaaatactgaattgatttttatgcttgttaatgtattgcaagaaacacagaaaatgtaattttgttttaataaaccaaaaaatgaacata

SEQ ID NO: 18 - RNA, 6411 nt, Macaca fascicularis
  source 1..6411: mol_type = mRNA
tatgttcattttttggtttattaaaacaaaattacattttctgtgtttcttgcaatacattaacaagcataaaaatcaattcagtatttccaagtatgtttcgctcacaaaaatcacagtcatttcacagtaccttacagtaattcttttcacaacagtcttaacatttctttatacaacaggcaaatagtttaataccttccatcaagacatttcagagctttagatgttcagaaataaggtcaagaatctctttcaaatgcaatcattagtttgtattaaactaaaatgccagatgacaagtctcaggtttctaaaaagagttttaaaaaataggtttacagcccatagtaagtcttataaacctcaacgataggtcctgtcacgtctaaacactacaactgtctgtggataaaaatctgcattcaattgtacaatactttcttctacatctgaatgaaaaccttattaaccccaactcatccatgtattctgatatgttcagtgaaaaagccaggatcattggggctgttctttctatcaaaggaaagagctccgatcacctacaatataattttctgtgcttattttctttaggggaggaaatacacatctattccatgccacactggatgttacaaaatgcatgtgaattctgccccagtgccatgtgttcattaccgttttgtctccttaaagaactatctaacagtgtttcccaaaatgttctccacaggacagtagtgagaggttcacaggtatcccaaaggagaaaaaggtcctgatgtcaaaatagtttgggcaatgctgggttgaacagtttttcactgccagatgccaagcccttactgcgctaaagtgcattgtaagtctccatgtgcaaacttagttcccagcaacaccatttctataaaacactgatgaacatctcacagagcactcatattacatggagtactatgggaaatgcttttcccggtccaggttactggaaattccacaatctgggattacattcattgtaatcccagaaatattttctccatataccctcatgactttgtgagatttaacagatttcagaaggaagactcaatgccatctcagttaacagttctacacatttcacactagtttttgccttgtttttcatgcaattttaagagtacataaattccttcctctcttctgaatcacttaggacattctcatttttaaaaacagagagcagttgcatattgcttaatatttttttttaacttgactcacagtcttcccctgaagggcatgcatttcatgttatagaaatgcaatagagtaaactgtaataaaattatttacaagcacctagtttgtttaaccttacatggaagccatcactgttggaaaacaatgagaacgtatcttttagcaaaacggtgctatctggaagctttattgtgaagatgctttcttttttgttttttgtttttcggtcatgaggcactgaagaatgagttgtgctgaaattaactcaaaggtcagcttgtctggatgagcataactttggttgagatttttctcccttaaaaaagattttcaaagcaccagttaattacaaaatgcatgcatatttatcctcacagtgacttaagtggtaagagagctagcaaatcatacattgcattcctcaaagcatctgatcaaacttctagaaaacaaaccaaccaaaagggaaaataatgcaagagaagccatattttctctgcttaggctggcgaagcagcagctctttgcagcagtgacaggcagggcagagtatccactgggaagtgagtcccaaccttgaataatggtgagcttgagtaatccttaatctacaatttaaaggatgaaaaaaagagactagtgaaatgtttgattccccacataaggaacacccaagactccctgggtatcctccaaatgtagccgagaaaagtgttcttccaccctagtcagtaaaatggaatgctaaaacgtgattatctcattaacatcagagctactacaactgacaatgacttaacagtacctcaattcctatcaagaaaaaatatcttttaaatgcagaacttgagagggatcacaacagcatagcattattgctaccagtttcaaacgtgatacttcatacaatgtgaaatatcaatcagcatccctccctctcccaaaacacacgttactcatgagacactattagtgtttaaaacccaagcttatagaagtacaaacttaattctcagtatttttatactaaattcaaagaaactatgtaacactcatctggaaaaattcttaattccataatatcttagagataagcaacagtaaactgttagaaaatgttttaacattacatgatattcaagaaatcaccataattaccataataaactaataattatgctccctgttcacaaaaggcacctaccaattatgaacagaccatttttcataattatttaccactacgtggcataatggtttaggcatataacccataaaaatttgttaaaagtcatggtttttcctcaaagctaaaaattcacaaatgcctctaaccattaccagtcagtagggccaccacatgcatatactggacaggttgtgcacggcacaactcaagtgggcaccagtcacctggactggggtgcagtacacaatctgtgtgcagtacagaaagccctcatcagttgtggccagagcactgtattctaacagagtctgtcagctcaagctaatcaagttaggaaagttgctatttggttggaggatttccaagaaacagctgtacccgtgagaagcaggtattacctgaggggtagacggggtacagacataaaacaggaagggttctaaatatttgctggtcatttaaaactcaatggcacttttttatatgagcaaaagccttcaacaccagttttctggccaagtttccctagaattttgccagccaaattaacttcctgatgttaactatttgattacaatatctcagttcccgacctaaactaatactgtctgttttcacatacctcttaaaaacattttctatatctgactgcaaaggacagcacagtgatacctgggtgtgatatatatcagtccattcatttataaagcacttgggataaaaggtactcccattaaaaatgtagctactattgacaaagataaaactgaaaaagagtgaatggatgactcaattatttttaaaggaagcattaaccattaaccagataatataccaacaaattacccaatagcactaagtataccatataagattcagttctagaacacagctacatttctgtgtccatcacagtaattagtccttaaaagttgtacttaaaatgtcaatctttaataaactccaaaataatgtattgagatttcatcttgtagtctacggattgtgagttgcgaatagaggctgaggtccccccaagtgttatctgcaggctgctgtgtggatgcagagctgggaagatcacagatccatggagggagaaggcacttgtcttccaggagatcactgcgggacagggcaggcgtgaccttgcgacggcaccttcaactctcgagccagaagctggtacctacaagggactcatctcatgaccttcatttgccagcggtgccacacgttacctacagcaccacaaaactcagaatatattctagaagtttttgccggttgcattgaggtagaaaagtgctgctcagttctaaaacagacactctcttttgtttggtctccttgaaaaccccaatatccttaaacattttcacagcattcttcacaagacagtatgtggcactctcagcatatactgcaacatttctttctgttctggttactaggtatttgtgcaacttttgcagatattcaggttctggaacagggccgctaaagttgtgaacaaagatggcagcagagctgtaggcctccagcaaaggcccaaggagtctctgtaagaaggtgataaactgctggtgctccttggattggctcaccttcaggtagcaatctcgctgttcctccccaaagtcactgtcttcatcttcttcatcacttctccaagacaaaggttcaggaagcttcttgtcccactgctgctcagcaagactaggactgatatcttcctggtcatcgtgctctgccactgtaagaatgccatactggataaactttcctactgtttcatggcacacttggtaaaatgtctggcaaggcagtgagatggtgccctcattggagagaaggtagcacaggctggccgccttccgcaccagctgctcctggctgatcaggttaggtggggtgccagtgggcccccctaatcccctcttgttcagaactgcataaaggctgcaagctatgatggcctccatgataaagacatgaagtaccccattgctgtagaagttgagttcgaagactgctgggacagttgtgctgggggtgataaaaaactcatcgttcctgctagtgtgagtgattgtgacgcaatttcccagcagctgtatggcatgcattactacatcttctgaatttcctgagaaccccaggtcaaaatcacgagccaggacttcctctttcatcacaaagaagtcttccaccaatgtggagagatcaattccctgcctgtgtctgtagaggagtaggcaagccacaatgtgtgtggacataatggcacaggacttgctagcagtgaatagaatatgctcagccagatttgcaatcaacctccttcgtaggaattcatctgttgcatttctggactcattaatggatgtgtctctaccttcatcagcagcatcattgggtcttgaaggaagtatagctggtaacaacgcttgctccagagaaagtggagcagacaccggtttctgactttggctttctaaatattcctttaaggaaaacggctgtgcaaaatccactcggacacaaccatagttttttcgtaacattctaataacacctcttgctatactccacaggctctcattcttctttggcttgcccagttgttcgccattgtagtgaccttcgataatacgatcataggagattccaacaggtattatcaagatgtctgggatgacattggtagatagagtatctaccacaactgacaaaagtcccgcccgagcacaggaggtttttccactcctagaacgtgtgccttccaggaagatctccaagaattgctgctgtcgaagtaattcaactatatgcccatggagcaaagctctgtagagaacatctttccgtccatctggtgtttcatcgagccttcgtcgtatgaagaagcccccaagcttatggatcaaagtactgaagattgggatatggagattattgcctgaagcaatgtatggtgctttgatgttatggcagaagagaatgaaagtgagcagcagatagtcaatatgggatctatgaactggtagaaacagaagcggcaaattcgtctcagttgcagctttaaccatctcaagttgacctttgtgaatttgaatgttccaaaagaagctgttgaacagttttagcagcacccacccagtcagtctgatcattgccggtgagacagtggcaaccatttcttgaagaatccttttagctttctttttcactttgttaacggcttttgattgctgctgggcagaaccatcagggtttaattcagcagccacttctgcaattgcctcttgtactctactgctgttcagcacattttcagtcacattggtggcaaacatgcccttatgcacatctcgctcttgaataaaaagaacataagaaaggcgtcttgcaagccatccccggtgtcttgtgtgagtttcattgatataaataacattccgcaaacccaaagatgggatactggggttgaaaaatctgtcccagctctggggagtgcaggagtaacaacatcttccaacaaatggccttttccgactcattaggctttctttccattttaaagttgcagatctgaagacagtaggtctaaaaccacactcaccccattcctcacttgtgtgcttacatcgaccaacactgtattctgatgaattcggcagataagaaacatctattgtaccaagggtcagtgcagattcatccatgtcacaaagtgtaattcccaaatcatgtgctgggatgaaagttcttctgtttcataacataaaacttcaggactcagctatcagtttcgggtgcagaatgtccatacaacaggggagccgctgctgcctgctctcgcagttcgcaccctagcagctccggcttcggctgctgcagcaccccgcacttcaagtcccggccaatgcctgctgcaatggcgcaccatgatgacgcaaccggcgcgtgga

SEQ ID NO: 19 - RNA, 6396 nt, Macaca fascicularis
  source 1..6396: mol_type = mRNA
tgcagcagccgaagccggagctgctagggtgcgaactgcgagagcaggtgtgggctgcgagaggctgctctggccgggagcgccgggacaagtgcgtggagctggcagcagcggctcccctgttgtatggacattctgcacccgaaactgatagctgagtcctgaagttttatgttatgaaacagaagaactttcatcccagcacatgatttgggaattacactttgtgacatggatgaatctgcactgacccttggtacaatagatgtttcttatctgccgaattcatcagaatacagtgttggtcgatgtaagcacacaagtgaggaatggggtgagtgtggttttagacctactgtcttcagatctgcaactttaaaatggaaagaaagcctaatgagtcggaaaaggccatttgttggaagatgttgttactcctgcactccccagagctgggacagatttttcaaccccagtatcccatctttgggtttgcggaatgttatttatatcaatgaaactcacacaagacaccggggatggcttgcaagacgcctttcttatgttctttttattcaagagcgagatgtgcataagggcatgtttgccaccaatgtgactgaaaatgtgctgaacagcagtagagtacaagaggcaattgcagaagtggctgctgaattaaaccctgatggttctgcccagcagcaatcaaaagccgttaacaaagtgaaaaagaaagctaaaaggattcttcaagaaatggttgccactgtctcaccggcaatgatcagactgactgggtgggtgctgctaaaactgttcaacagcttcttttggaacattcaaattcacaaaggtcaacttgagatggttaaagctgcaactgagacgaatttgccgcttctgtttctaccagttcatagatcccatattgactatctgctgctcactttcattctcttctgccataacatcaaagcaccatacattgcttcaggcaataatctccatatcccaatcttcagtactttgatccataagcttgggggcttcttcatacgacgaaggctcgatgaaacaccagatggacggaaagatgttctctacagagctttgctccatgggcatatagttgaattacttcgacagcagcaattcttggagatcttcctggaaggcacacgttctaggagtggaaaaacctcctgtgctcgggcgggacttttgtcagttgtggtagatactctatctaccaatgtcatcccagacatcttgataatacctgttggaatctcctatgatcgtattatcgaaggtcactacaatggcgaacaactgggcaagccaaagaagaatgagagcctgtggagtatagcaagaggtgttattagaatgttacgaaaaaactatggttgtgtccgagtggattttgcacagccgttttccttaaaggaatatttagaaagccaaagtcagaaaccggtgtctgctccactttctctggagcaagcgttgttaccagctatacttccttcaagacccaatgatgctgctgatgaaggtagagacacatccattaatgagtccagaaatgcaacagatgaattcctacgaaggaggttgattgcaaatctggctgagcatattctattcactgctagcaagtcctgtgccattatgtccacacacattgtggcttgcctactcctctacagacacaggcagggaattgatctctccacattggtggaagacttctttgtgatgaaagaggaagtcctggctcgtgattttgacctggggttctcaggaaattcagaagatgtagtaatgcatgccatacagctgctgggaaattgcgtcacaatcactcacactagcaggaacgatgagttttttatcacccccagcacaactgtcccagcagtcttcgaactcaacttctacagcaatggggtacttcatgtctttatcatggaggccatcatagcttgcagcctttatgcagttctgaacaagaggggattaggggggcccactggcaccccacctaacctgatcagccaggagcagctggtgcggaaggcggccagcctgtgctaccttctctccaatgagggcaccatctcactgccttgccagacattttaccaagtgtgccatgaaacagtaggaaagtttatccagtatggcattcttacagtggcagagcacgatgaccaggaagatatcagtcctagtcttgctgagcagcagtgggacaagaagcttcctgaacctttgtcttggagaagtgatgaagaagatgaagacagtgactttggggaggaacagcgagattgctacctgaaggtgagccaatccaaggagcaccagcagtttatcaccttcttacagagactccttgggcctttgctggaggcctacagctctgctgccatctttgttcacaactttagcggccctgttccagaacctgaatatctgcaaaagttgcacaaatacctagtaaccagaacagaaagaaatgttgcagtatatgctgagagtgccacatactgtcttgtgaagaatgctgtgaaaatgtttaaggatattggggttttcaaggagaccaaacaaaagagagtgtctgttttagaactgagcagcacttttctacctcaatgcaaccggcaaaaacttctagaatatattctgagttttgtggtgctgtaggtaacgtgtggcaccgctggcaaatgaaggtcatgagatgagtcccttgtaggtaccagcttctggctcgagagttgaaggtgccgtcgcaaggtcacgcctgccctgtcccgcagtgatctcctggaagacaagtgccttctccctccatggatctgtgatcttcccagctctgcatccacacagcagcctgcagataacacttggggggacctcagcctctattcgcaactcacaatccgtagactacaagatgaaatctcaatacattattttggagtttattaaagattgacattttaagtacaacttttaaggactaattactgtgatggacacagaaatgtagctgtgttctagaactgaatcttatatggtatacttagtgctattgggtaatttgttggtatattatctggttaatggttaatgcttcctttaaaaataattgagtcatccattcactctttttcagttttatctttgtcaatagtagctacatttttaatgggagtaccttttatcccaagtgctttataaatgaatggactgatatatatcacacccaggtatcactgtgctgtcctttgcagtcagatatagaaaatgtttttaagaggtatgtgaaaacagacagtattagtttaggtcgggaactgagatattgtaatcaaatagttaacatcaggaagttaatttggctggcaaaattctagggaaacttggccagaaaactggtgttgaaggcttttgctcatataaaaaagtgccattgagttttaaatgaccagcaaatatttagaacccttcctgttttatgtctgtaccccgtctacccctcaggtaatacctgcttctcacgggtacagctgtttcttggaaatcctccaaccaaatagcaactttcctaacttgattagcttgagctgacagactctgttagaatacagtgctctggccacaactgatgagggctttctgtactgcacacagattgtgtactgcaccccagtccaggtgactggtgcccacttgagttgtgccgtgcacaacctgtccagtatatgcatgtggtggccctactgactggtaatggttagaggcatttgtgaatttttagctttgaggaaaaaccatgacttttaacaaatttttatgggttatatgcctaaaccattatgccacgtagtggtaaataattatgaaaaatggtctgttcataattggtaggtgccttttgtgaacagggagcataattattagtttattatggtaattatggtgatttcttgaatatcatgtaatgttaaaacattttctaacagtttactgttgcttatctctaagatattatggaattaagaatttttccagatgagtgttacatagtttctttgaatttagtataaaaatactgagaattaagtttgtacttctataagcttgggttttaaacactaatagtgtctcatgagtaacgtgtgttttgggagagggagggatgctgattgatatttcacattgtatgaagtatcacgtttgaaactggtagcaataatgctatgctgttgtgatccctctcaagttctgcatttaaaagatattttttcttgataggaattgaggtactgttaagtcattgtcagttgtagtagctctgatgttaatgagataatcacgttttagcattccattttactgactagggtggaagaacacttttctcggctacatttggaggatacccagggagtcttgggtgttccttatgtggggaatcaaacatttcactagtctctttttttcatcctttaaattgtagattaaggattactcaagctcaccattattcaaggttgggactcacttcccagtggatactctgccctgcctgtcactgctgcaaagagctgctgcttcgccagcctaagcagagaaaatatggcttctcttgcattattttcccttttggttggtttgttttctagaagtttgatcagatgctttgaggaatgcaatgtatgatttgctagctctcttaccacttaagtcactgtgaggataaatatgcatgcattttgtaattaactggtgctttgaaaatcttttttaagggagaaaaatctcaaccaaagttatgctcatccagacaagctgacctttgagttaatttcagcacaactcattcttcagtgcctcatgaccgaaaaacaaaaaacaaaaaagaaagcatcttcacaataaagcttccagatagcaccgttttgctaaaagatacgttctcattgttttccaacagtgatggcttccatgtaaggttaaacaaactaggtgcttgtaaataattttattacagtttactctattgcatttctataacatgaaatgcatgcccttcaggggaagactgtgagtcaagttaaaaaaaaatattaagcaatatgcaactgctctctgtttttaaaaatgagaatgtcctaagtgattcagaagagaggaaggaatttatgtactcttaaaattgcatgaaaaacaaggcaaaaactagtgtgaaatgtgtagaactgttaactgagatggcattgagtcttccttctgaaatctgttaaatctcacaaagtcatgagggtatatggagaaaatatttctgggattacaatgaatgtaatcccagattgtggaatttccagtaacctggaccgggaaaagcatttcccatagtactccatgtaatatgagtgctctgtgagatgttcatcagtgttttatagaaatggtgttgctgggaactaagtttgcacatggagacttacaatgcactttagcgcagtaagggcttggcatctggcagtgaaaaactgttcaacccagcattgcccaaactattttgacatcaggacctttttctcctttgggatacctgtgaacctctcactactgtcctgtggagaacattttgggaaacactgttagatagttctttaaggagacaaaacggtaatgaacacatggcactggggcagaattcacatgcattttgtaacatccagtgtggcatggaatagatgtgtatttcctcccctaaagaaaataagcacagaaaattatattgtaggtgatcggagctctttcctttgatagaaagaacagccccaatgatcctggctttttcactgaacatatcagaatacatggatgagttggggttaataaggttttcattcagatgtagaagaaagtattgtacaattgaatgcagatttttatccacagacagttgtagtgtttagacgtgacaggacctatcgttgaggtttataagacttactatgggctgtaaacctattttttaaaactctttttagaaacctgagacttgtcatctggcattttagtttaatacaaactaatgattgcatttgaaagagattcttgaccttatttctgaacatctaaagctctgaaatgtcttgatggaaggtattaaactatttgcctgttgtataaagaaatgttaagactgttgtgaaaagaattactgtaaggtactgtgaaatgactgtgatttttgtgagcgaaacatacttggaaatactgaattgatttttatgcttgttaatgtattgcaagaaacacagaaaatgtaattttgttttaataaaccaaaaaatgaacata

SEQ ID NO: 20 - RNA, 6396 nt, Macaca fascicularis
  source 1..6396: mol_type = mRNA
tatgttcattttttggtttattaaaacaaaattacattttctgtgtttcttgcaatacattaacaagcataaaaatcaattcagtatttccaagtatgtttcgctcacaaaaatcacagtcatttcacagtaccttacagtaattcttttcacaacagtcttaacatttctttatacaacaggcaaatagtttaataccttccatcaagacatttcagagctttagatgttcagaaataaggtcaagaatctctttcaaatgcaatcattagtttgtattaaactaaaatgccagatgacaagtctcaggtttctaaaaagagttttaaaaaataggtttacagcccatagtaagtcttataaacctcaacgataggtcctgtcacgtctaaacactacaactgtctgtggataaaaatctgcattcaattgtacaatactttcttctacatctgaatgaaaaccttattaaccccaactcatccatgtattctgatatgttcagtgaaaaagccaggatcattggggctgttctttctatcaaaggaaagagctccgatcacctacaatataattttctgtgcttattttctttaggggaggaaatacacatctattccatgccacactggatgttacaaaatgcatgtgaattctgccccagtgccatgtgttcattaccgttttgtctccttaaagaactatctaacagtgtttcccaaaatgttctccacaggacagtagtgagaggttcacaggtatcccaaaggagaaaaaggtcctgatgtcaaaatagtttgggcaatgctgggttgaacagtttttcactgccagatgccaagcccttactgcgctaaagtgcattgtaagtctccatgtgcaaacttagttcccagcaacaccatttctataaaacactgatgaacatctcacagagcactcatattacatggagtactatgggaaatgcttttcccggtccaggttactggaaattccacaatctgggattacattcattgtaatcccagaaatattttctccatataccctcatgactttgtgagatttaacagatttcagaaggaagactcaatgccatctcagttaacagttctacacatttcacactagtttttgccttgtttttcatgcaattttaagagtacataaattccttcctctcttctgaatcacttaggacattctcatttttaaaaacagagagcagttgcatattgcttaatatttttttttaacttgactcacagtcttcccctgaagggcatgcatttcatgttatagaaatgcaatagagtaaactgtaataaaattatttacaagcacctagtttgtttaaccttacatggaagccatcactgttggaaaacaatgagaacgtatcttttagcaaaacggtgctatctggaagctttattgtgaagatgctttcttttttgttttttgtttttcggtcatgaggcactgaagaatgagttgtgctgaaattaactcaaaggtcagcttgtctggatgagcataactttggttgagatttttctcccttaaaaaagattttcaaagcaccagttaattacaaaatgcatgcatatttatcctcacagtgacttaagtggtaagagagctagcaaatcatacattgcattcctcaaagcatctgatcaaacttctagaaaacaaaccaaccaaaagggaaaataatgcaagagaagccatattttctctgcttaggctggcgaagcagcagctctttgcagcagtgacaggcagggcagagtatccactgggaagtgagtcccaaccttgaataatggtgagcttgagtaatccttaatctacaatttaaaggatgaaaaaaagagactagtgaaatgtttgattccccacataaggaacacccaagactccctgggtatcctccaaatgtagccgagaaaagtgttcttccaccctagtcagtaaaatggaatgctaaaacgtgattatctcattaacatcagagctactacaactgacaatgacttaacagtacctcaattcctatcaagaaaaaatatcttttaaatgcagaacttgagagggatcacaacagcatagcattattgctaccagtttcaaacgtgatacttcatacaatgtgaaatatcaatcagcatccctccctctcccaaaacacacgttactcatgagacactattagtgtttaaaacccaagcttatagaagtacaaacttaattctcagtatttttatactaaattcaaagaaactatgtaacactcatctggaaaaattcttaattccataatatcttagagataagcaacagtaaactgttagaaaatgttttaacattacatgatattcaagaaatcaccataattaccataataaactaataattatgctccctgttcacaaaaggcacctaccaattatgaacagaccatttttcataattatttaccactacgtggcataatggtttaggcatataacccataaaaatttgttaaaagtcatggtttttcctcaaagctaaaaattcacaaatgcctctaaccattaccagtcagtagggccaccacatgcatatactggacaggttgtgcacggcacaactcaagtgggcaccagtcacctggactggggtgcagtacacaatctgtgtgcagtacagaaagccctcatcagttgtggccagagcactgtattctaacagagtctgtcagctcaagctaatcaagttaggaaagttgctatttggttggaggatttccaagaaacagctgtacccgtgagaagcaggtattacctgaggggtagacggggtacagacataaaacaggaagggttctaaatatttgctggtcatttaaaactcaatggcacttttttatatgagcaaaagccttcaacaccagttttctggccaagtttccctagaattttgccagccaaattaacttcctgatgttaactatttgattacaatatctcagttcccgacctaaactaatactgtctgttttcacatacctcttaaaaacattttctatatctgactgcaaaggacagcacagtgatacctgggtgtgatatatatcagtccattcatttataaagcacttgggataaaaggtactcccattaaaaatgtagctactattgacaaagataaaactgaaaaagagtgaatggatgactcaattatttttaaaggaagcattaaccattaaccagataatataccaacaaattacccaatagcactaagtataccatataagattcagttctagaacacagctacatttctgtgtccatcacagtaattagtccttaaaagttgtacttaaaatgtcaatctttaataaactccaaaataatgtattgagatttcatcttgtagtctacggattgtgagttgcgaatagaggctgaggtccccccaagtgttatctgcaggctgctgtgtggatgcagagctgggaagatcacagatccatggagggagaaggcacttgtcttccaggagatcactgcgggacagggcaggcgtgaccttgcgacggcaccttcaactctcgagccagaagctggtacctacaagggactcatctcatgaccttcatttgccagcggtgccacacgttacctacagcaccacaaaactcagaatatattctagaagtttttgccggttgcattgaggtagaaaagtgctgctcagttctaaaacagacactctcttttgtttggtctccttgaaaaccccaatatccttaaacattttcacagcattcttcacaagacagtatgtggcactctcagcatatactgcaacatttctttctgttctggttactaggtatttgtgcaacttttgcagatattcaggttctggaacagggccgctaaagttgtgaacaaagatggcagcagagctgtaggcctccagcaaaggcccaaggagtctctgtaagaaggtgataaactgctggtgctccttggattggctcaccttcaggtagcaatctcgctgttcctccccaaagtcactgtcttcatcttcttcatcacttctccaagacaaaggttcaggaagcttcttgtcccactgctgctcagcaagactaggactgatatcttcctggtcatcgtgctctgccactgtaagaatgccatactggataaactttcctactgtttcatggcacacttggtaaaatgtctggcaaggcagtgagatggtgccctcattggagagaaggtagcacaggctggccgccttccgcaccagctgctcctggctgatcaggttaggtggggtgccagtgggcccccctaatcccctcttgttcagaactgcataaaggctgcaagctatgatggcctccatgataaagacatgaagtaccccattgctgtagaagttgagttcgaagactgctgggacagttgtgctgggggtgataaaaaactcatcgttcctgctagtgtgagtgattgtgacgcaatttcccagcagctgtatggcatgcattactacatcttctgaatttcctgagaaccccaggtcaaaatcacgagccaggacttcctctttcatcacaaagaagtcttccaccaatgtggagagatcaattccctgcctgtgtctgtagaggagtaggcaagccacaatgtgtgtggacataatggcacaggacttgctagcagtgaatagaatatgctcagccagatttgcaatcaacctccttcgtaggaattcatctgttgcatttctggactcattaatggatgtgtctctaccttcatcagcagcatcattgggtcttgaaggaagtatagctggtaacaacgcttgctccagagaaagtggagcagacaccggtttctgactttggctttctaaatattcctttaaggaaaacggctgtgcaaaatccactcggacacaaccatagttttttcgtaacattctaataacacctcttgctatactccacaggctctcattcttctttggcttgcccagttgttcgccattgtagtgaccttcgataatacgatcataggagattccaacaggtattatcaagatgtctgggatgacattggtagatagagtatctaccacaactgacaaaagtcccgcccgagcacaggaggtttttccactcctagaacgtgtgccttccaggaagatctccaagaattgctgctgtcgaagtaattcaactatatgcccatggagcaaagctctgtagagaacatctttccgtccatctggtgtttcatcgagccttcgtcgtatgaagaagcccccaagcttatggatcaaagtactgaagattgggatatggagattattgcctgaagcaatgtatggtgctttgatgttatggcagaagagaatgaaagtgagcagcagatagtcaatatgggatctatgaactggtagaaacagaagcggcaaattcgtctcagttgcagctttaaccatctcaagttgacctttgtgaatttgaatgttccaaaagaagctgttgaacagttttagcagcacccacccagtcagtctgatcattgccggtgagacagtggcaaccatttcttgaagaatccttttagctttctttttcactttgttaacggcttttgattgctgctgggcagaaccatcagggtttaattcagcagccacttctgcaattgcctcttgtactctactgctgttcagcacattttcagtcacattggtggcaaacatgcccttatgcacatctcgctcttgaataaaaagaacataagaaaggcgtcttgcaagccatccccggtgtcttgtgtgagtttcattgatataaataacattccgcaaacccaaagatgggatactggggttgaaaaatctgtcccagctctggggagtgcaggagtaacaacatcttccaacaaatggccttttccgactcattaggctttctttccattttaaagttgcagatctgaagacagtaggtctaaaaccacactcaccccattcctcacttgtgtgcttacatcgaccaacactgtattctgatgaattcggcagataagaaacatctattgtaccaagggtcagtgcagattcatccatgtcacaaagtgtaattcccaaatcatgtgctgggatgaaagttcttctgtttcataacataaaacttcaggactcagctatcagtttcgggtgcagaatgtccatacaacaggggagccgctgctgccagctccacgcacttgtcccggcgctcccggccagagcagcctctcgcagcccacacctgctctcgcagttcgcaccctagcagctccggcttcggctgctgca

SEQ ID NO: 21 - protein, 16 aa, unidentified
  source 1..16: note = RFGF peptide
AAVALLPAVLLALLAP

SEQ ID NO: 22 - protein, 11 aa, unidentified
  source 1..11: note = RFGF analogue peptide
AALLPVLLAAP

SEQ ID NO: 23 - protein, 13 aa, Human immunodeficiency virus 1
GRKKRRQRRRPPQ

SEQ ID NO: 24 - protein, 16 aa, Drosophila sp.
RQIKIWFQNRRMKWKK

SEQ ID NO: 25 - RNA, 21 nt, synthetic construct
  source 1..21: mol_type = other RNA
gtcctgaagttttatgttatt

SEQ ID NO: 26 - RNA, 21 nt, synthetic construct
  source 1..21: mol_type = other RNA
gttatgaaacagaagaacttt

SEQ ID NO: 27 - RNA, 21 nt, synthetic construct
  source 1..21: mol_type = other RNA
tgatttgggaattacactttt

SEQ ID NO: 28 - RNA, 21 nt, synthetic construct
  source 1..21: mol_type = other RNA
gtacaatagatgtttcttatt

SEQ ID NO: 29 - RNA, 21 nt, synthetic construct
  source 1..21: mol_type = other RNA
attcatcagaatacagtgttt

SEQ ID NO: 30 - RNA, 21 nt, synthetic construct
  source 1..21: mol_type = other RNA
cagatctgcaactttaaaatt

SEQ ID NO: 31 - RNA, 21 nt, synthetic construct
  source 1..21: mol_type = other RNA
aaatggaaagaaagcctaatt

SEQ ID NO: 32 - RNA, 21 nt, synthetic construct
  source 1..21: mol_type = other RNA
ttgttggaagatgttgttact

SEQ ID NO: 33 - RNA, 21 nt, synthetic construct
  source 1..21: mol_type = other RNA
gcggaatgttatttatatcat

SEQ ID NO: 34 - RNA, 21 nt, synthetic construct
  source 1..21: mol_type = other RNA
tatcaatgaaactcacacaat

SEQ ID NO: 35 - RNA, 21 nt, synthetic construct
  source 1..21: mol_type = other RNA
gacgcctttcttacgttcttt

SEQ ID NO: 36 - RNA, 21 nt, synthetic construct
  source 1..21: mol_type = other RNA
accaatgtgactgaaaatgtt

SEQ ID NO: 37 - RNA, 21 nt, synthetic construct
  source 1..21: mol_type = other RNA
aagccgttaacaaagtgaaat

SEQ ID NO: 38 - RNA, 21 nt, synthetic construct
  source 1..21: mol_type = other RNA
aaaaggattcttcaagaaatt

SEQ ID NO: 39 - RNA, 21 nt, synthetic construct
  source 1..21: mol_type = other RNA
tcttttggaacattcaaattt

SEQ ID NO: 40 - RNA, 21 nt, synthetic construct
  source 1..21: mol_type = other RNA
aaattcacaaaggtcaacttt

SEQ ID NO: 41 - RNA, 21 nt, synthetic construct
  source 1..21: mol_type = other RNA
tttctaccagttcatagatct

SEQ ID NO: 42 - RNA, 21 nt, synthetic construct
  source 1..21: mol_type = other RNA
agatcccatattgactatctt

SEQ ID NO: 43 - RNA, 21 nt, synthetic construct
  source 1..21: mol_type = other RNA
gctcactttcattctcttctt

SEQ ID NO: 44 - RNA, 21 nt, synthetic construct
  source 1..21: mol_type = other RNA
tcaggcaataatctcaacatt

SEQ ID NO: 45 - RNA, 21 nt, synthetic construct
  source 1..21: mol_type = other RNA
cttcagtaccttgatccatat

SEQ ID NO: 46 - RNA, 21 nt, synthetic construct
  source 1..21: mol_type = other RNA
gatgttctctatagagctttt

SEQ ID NO: 47 - RNA, 21 nt, synthetic construct
  source 1..21: mol_type = other RNA
ggcatatagttgaattacttt

SEQ ID NO: 48 - RNA, 21 nt, synthetic construct
  source 1..21: mol_type = other RNA
tagatactctgtctaccaatt

SEQ ID NO: 49 - RNA, 21 nt, synthetic construct
  source 1..21: mol_type = other RNA
cccagacatcttgataatact

SEQ ID NO: 50 - RNA, 21 nt, synthetic construct
  source 1..21: mol_type = other RNA
ctgttggaatctcctatgatt

SEQ ID NO: 51 - RNA, 21 nt, synthetic construct
  source 1..21: mol_type = other RNA
ctgggcaaacctaagaagaat

SEQ ID NO: 52 - RNA, 21 nt, synthetic construct
  source 1..21: mol_type = other RNA
gttattagaatgttacgaaat

SEQ ID NO: 53 - RNA, 21 nt, synthetic construct
  source 1..21: mol_type = other RNA
agccattttccttaaaggaat

SEQ ID NO: 54 - RNA, 21 nt, synthetic construct
  source 1..21: mol_type = other RNA
aatatttagaaagccaaagtt

SEQ ID NO: 55 - RNA, 21 nt, synthetic construct
  source 1..21: mol_type = other RNA
accagctatacttccttcaat

SEQ ID NO: 56 - RNA, 21 nt, synthetic construct
  source 1..21: mol_type = other RNA
taatgagtccagaaatgcaat

SEQ ID NO: 57 - RNA, 21 nt, synthetic construct
  source 1..21: mol_type = other RNA
aggaggttgattgcaaatctt

SEQ ID NO: 58 - RNA, 21 nt, synthetic construct
  source 1..21: mol_type = other RNA
gaagacttctttgtgatgaat

SEQ ID NO: 59 - RNA, 21 nt, synthetic construct
  source 1..21: mol_type = other RNA
aattcagaagatgtagtaatt

SEQ ID NO: 60 - RNA, 21 nt, synthetic construct
  source 1..21: mol_type = other RNA
agtcttcgaactcaacttctt

SEQ ID NO: 61 - RNA, 21 nt, synthetic construct
  source 1..21: mol_type = other RNA
tacttcatgtctttatcatgt

SEQ ID NO: 62 - RNA, 21 nt, synthetic construct
  source 1..21: mol_type = other RNA
ttatgcagttctgaacaagat

SEQ ID NO: 63 - RNA, 21 nt, synthetic construct
  source 1..21: mol_type = other RNA
gaaacagtaggaaagtttatt

SEQ ID NO: 64 - RNA, 21 nt, synthetic construct
  source 1..21: mol_type = other RNA
tggagaagtgatgaagaagat

SEQ ID NO: 65 - RNA, 21 nt, synthetic construct
  source 1..21: mol_type = other RNA
gtttatcaccttcttacagat

SEQ ID NO: 66 - RNA, 21 nt, synthetic construct
  source 1..21: mol_type = other RNA
gaacctgagtatctgcaaaat

SEQ ID NO: 67 - RNA, 21 nt, synthetic construct
  source 1..21: mol_type = other RNA
gttgcacaaatacctaataat

SEQ ID NO: 68 - RNA, 21 nt, synthetic construct
  source 1..21: mol_type = other RNA
taaccagaacagaaagaaatt

SEQ ID NO: 69 - RNA, 21 nt, synthetic construct
  source 1..21: mol_type = other RNA
catattgtcttgtgaagaatt

SEQ ID NO: 70 - RNA, 21 nt, synthetic construct
  source 1..21: mol_type = other RNA
aatgctgtgaaaatgtttaat

SEQ ID NO: 71 - RNA, 21 nt, synthetic construct
  source 1..21: mol_type = other RNA
agagtgtctgttttagaactt

SEQ ID NO: 72 - RNA, 21 nt, synthetic construct
  source 1..21: mol_type = other RNA
tatattctgagttttgtggtt

SEQ ID NO: 73 - RNA, 21 nt, synthetic construct
  source 1..21: mol_type = other RNA
atgagatgagttccttgtagt

SEQ ID NO: 74 - RNA, 21 nt, synthetic construct
  source 1..21: mol_type = other RNA
acaagatgaaatctcaataat

SEQ ID NO: 75 - RNA, 21 nt, synthetic construct
  source 1..21: mol_type = other RNA
acaacttttaaggactaattt

SEQ ID NO: 76 - RNA, 21 nt, synthetic construct
  source 1..21: mol_type = other RNA
aatcttacatggtatacttat

SEQ ID NO: 77 - RNA, 21 nt, synthetic construct
  source 1..21: mol_type = other RNA
tgttggtatattatctggttt

SEQ ID NO: 78 - RNA, 21 nt, synthetic construct
  source 1..21: mol_type = other RNA
ttagtggttaatgcttccttt

SEQ ID NO: 79 - RNA, 21 nt, synthetic construct
  source 1..21: mol_type = other RNA
tgagtcatccattcactcttt

SEQ ID NO: 80 - RNA, 21 nt, synthetic construct
  source 1..21: mol_type = other RNA
cagttttatctgtcaatagtt

SEQ ID NO: 81 - RNA, 21 nt, synthetic construct
  source 1..21: mol_type = other RNA
cccaaagtgctttataaattt

SEQ ID NO: 82 - RNA, 21 nt, synthetic construct
  source 1..21: mol_type = other RNA
tgtcagatttagaaatgtttt

SEQ ID NO: 83 - RNA, 21 nt, synthetic construct
  source 1..21: mol_type = other RNA
atgtgaaaacagacaatattt

SEQ ID NO: 84 - RNA, 21 nt, synthetic construct
  source 1..21: mol_type = other RNA
aactgagatattgtaatcaat

SEQ ID NO: 85 - RNA, 21 nt, synthetic construct
  source 1..21: mol_type = other RNA
taacatcaggaagttaatttt

SEQ ID NO: 86 - RNA, 21 nt, synthetic construct
  source 1..21: mol_type = other RNA
gcaaaattctagggaaacttt

SEQ ID NO: 87 - RNA, 21 nt, synthetic construct
  source 1..21: mol_type = other RNA
aaggcttttgctcatataaat

SEQ ID NO: 88 - RNA, 21 nt, synthetic construct
  source 1..21: mol_type = other RNA
tgccattgagtttcaaatgat

SEQ ID NO: 89 - RNA, 21 nt, synthetic construct
  source 1..21: mol_type = other RNA
gaccagcaaatatatttagat

SEQ ID NO: 90 - RNA, 21 nt, synthetic construct
  source 1..21: mol_type = other RNA
cttggaaatcctccaaccaat

SEQ ID NO: 91 - RNA, 21 nt, synthetic construct
  source 1..21: mol_type = other RNA
aaatagcagttttcctaactt

SEQ ID NO: 92 - RNA, 21 nt, synthetic construct
  source 1..21: mol_type = other RNA
agctgacagactgttagaatt

SEQ ID NO: 93 - RNA, 21 nt, synthetic construct
  source 1..21: mol_type = other RNA
ttagaggcatttatggatttt

SEQ ID NO: 94 - RNA, 21 nt, synthetic construct
  source 1..21: mol_type = other RNA
tatgggttatatgcctaaact

SEQ ID NO: 95 - RNA, 21 nt, synthetic construct
  source 1..21: mol_type = other RNA
ccacatagtggtaaataattt

SEQ ID NO: 96 - RNA, 21 nt, synthetic construct
  source 1..21: mol_type = other RNA
tggtctgttcataattggtat

SEQ ID NO: 97 - RNA, 21 nt, synthetic construct
  source 1..21: mol_type = other RNA
gagcataattattggtttatt

SEQ ID NO: 98 - RNA, 21 nt, synthetic construct
  source 1..21: mol_type = other RNA
tttattatggtaattatggtt

SEQ ID NO: 99 - RNA, 21 nt, synthetic construct
  source 1..21: mol_type = other RNA
taaaacgttttctaacagttt

SEQ ID NO: 100 - RNA, 21 nt, synthetic construct
  source 1..21: mol_type = other RNA
ctccaagatattatggaattt

SEQ ID NO: 101 - RNA, 21 nt, synthetic construct
  source 1..21: mol_type = other RNA
tgagtgttacatagattcttt

SEQ ID NO: 102 - RNA, 21 nt, synthetic construct
  source 1..21: mol_type = other RNA
agtactgagaattaagtttgt

SEQ ID NO: 103 - RNA, 21 nt, synthetic construct
  source 1..21: mol_type = other RNA
attttaaacactgatagtatt

SEQ ID NO: 104 - RNA, 21 nt, synthetic construct
  source 1..21: mol_type = other RNA
ctcatgagtaatgtgtgtttt

SEQ ID NO: 105 - RNA, 21 nt, synthetic construct
  source 1..21: mol_type = other RNA
atgctgattgatatttcacat

SEQ ID NO: 106 - RNA, 21 nt, synthetic construct
  source 1..21: mol_type = other RNA
tatgaaataccatgtttgaat

SEQ ID NO: 107 - RNA, 21 nt, synthetic construct
  source 1..21: mol_type = other RNA
ttgaaactcatagcaataatt

SEQ ID NO: 108 - RNA, 21 nt, synthetic construct
  source 1..21: mol_type = other RNA
taatgctatgctgttgtgatt

SEQ ID NO: 109 - RNA, 21 nt, synthetic construct
  source 1..21: mol_type = other RNA
caagttctgcatttaaaatat

SEQ ID NO: 110 - RNA, 21 nt, synthetic construct
  source 1..21: mol_type = other RNA
gatgtataccatgaagtcatt

SEQ ID NO: 111 - RNA, 21 nt, synthetic construct
  source 1..21: mol_type = other RNA
gttgtagtagctctgatgttt

SEQ ID NO: 112 - RNA, 21 nt, synthetic construct
  source 1..21: mol_type = other RNA
tgaatgagatatcatgttttt

SEQ ID NO: 113 - RNA, 21 nt, synthetic construct
  source 1..21: mol_type = other RNA
ttttagcattccattttactt

SEQ ID NO: 114 - RNA, 21 nt, synthetic construct
  source 1..21: mol_type = other RNA
taaattaaggattactcaagt

SEQ ID NO: 115 - RNA, 21 nt, synthetic construct
  source 1..21: mol_type = other RNA
gctcaccattattcaagattt

SEQ ID NO: 116 - RNA, 21 nt, synthetic construct
  source 1..21: mol_type = other RNA
ggcttctcttgcattattttt

SEQ ID NO: 117 - RNA, 21 nt, synthetic construct
  source 1..21: mol_type = other RNA
tggtttgttttctagaagtat

SEQ ID NO: 118 - RNA, 21 nt, synthetic construct
  source 1..21: mol_type = other RNA
ctggtgctttgaaaatctttt

SEQ ID NO: 119 - RNA, 21 nt, synthetic construct
  source 1..21: mol_type = other RNA
gctgacctttgagttaatttt

SEQ ID NO: 120 - RNA, 21 nt, synthetic construct
  source 1..21: mol_type = other RNA
agcacaactcattcttcagtt

SEQ ID NO: 121 - RNA, 21 nt, synthetic construct
  source 1..21: mol_type = other RNA
tgcctcatgactgaaaacaat

SEQ ID NO: 122 - RNA, 21 nt, synthetic construct
  source 1..21: mol_type = other RNA
cgaaagcatcttcacaatgat

SEQ ID NO: 123 - RNA, 21 nt, synthetic construct
  source 1..21: mol_type = other RNA
atagcaccgttttgctaaaat

SEQ ID NO: 124 - RNA, 21 nt, synthetic construct
  source 1..21: mol_type = other RNA
gatacattctcattgttttct

SEQ ID NO: 125 - RNA, 21 nt, synthetic construct
  source 1..21: mol_type = other RNA
tccacataaggttaaacaaat

SEQ ID NO: 126 - RNA, 21 nt, synthetic construct
  source 1..21: mol_type = other RNA
aggtgcttgtaaataatttat

SEQ ID NO: 127 - RNA, 21 nt, synthetic construct
  source 1..21: mol_type = other RNA
ctctatcgcatttctgtaact

SEQ ID NO: 128 - RNA, 21 nt, synthetic construct
  source 1..21: mol_type = other RNA
aaaatgagaatgtcctaagtt

SEQ ID NO: 129 - RNA, 21 nt, synthetic construct
  source 1..21: mol_type = other RNA
cactctgaaaatgcatgaaat

SEQ ID NO: 130 - RNA, 21 nt, synthetic construct
  source 1..21: mol_type = other RNA
aatgtgtagaactgttaactt

SEQ ID NO: 131 - RNA, 21 nt, synthetic construct
  source 1..21: mol_type = other RNA
cttctggaatctgttaaattt

SEQ ID NO: 132 - RNA, 21 nt, synthetic construct
  source 1..21: mol_type = other RNA
gagggtaaatggagaaaatat

SEQ ID NO: 133 - RNA, 21 nt, synthetic construct
  source 1..21: mol_type = other RNA
tgggattacaatgaatgtaat

SEQ ID NO: 134 - RNA, 21 nt, synthetic construct
  source 1..21: mol_type = other RNA
taagcccaaattgtggaattt

SEQ ID NO: 135 - RNA, 21 nt, synthetic construct
  source 1..21: mol_type = other RNA
tcatcagtgttttatagaaat

SEQ ID NO: 136 - RNA, 21 nt, synthetic construct
  source 1..21: mol_type = other RNA
attgcccaaactattttgact

SEQ ID NO: 137 - RNA, 21 nt, synthetic construct
  source 1..21: mol_type = other RNA
acttatgaacctctcactaat

SEQ ID NO: 138 - RNA, 21 nt, synthetic construct
  source 1..21: mol_type = other RNA
ttgggaaacactatgttagat

SEQ ID NO: 139 - RNA, 21 nt, synthetic construct
  source 1..21: mol_type = other RNA
agttctttaaggagacaaaat

SEQ ID NO: 140 - RNA, 21 nt, synthetic construct
  source 1..21: mol_type = other RNA
atatgcatgcattttgtaact

SEQ ID NO: 141 - RNA, 21 nt, synthetic construct
  source 1..21: mol_type = other RNA
cgttgaatagatgtgtatttt

SEQ ID NO: 142 - RNA, 21 nt, synthetic construct
  source 1..21: mol_type = other RNA
gaaaataagcacagaaaattt

SEQ ID NO: 143 - RNA, 21 nt, synthetic construct
  source 1..21: mol_type = other RNA
ttcactgaacgtatcagaatt

SEQ ID NO: 144 - RNA, 21 nt, synthetic construct
  source 1..21: mol_type = other RNA
taaataaggttttaattcagt

SEQ ID NO: 145 - RNA, 21 nt, synthetic construct
  source 1..21: mol_type = other RNA
cagatctagaagaaagtattt

SEQ ID NO: 146 - RNA, 21 nt, synthetic construct
  source 1..21: mol_type = other RNA
acagatagttgtagtgtttat

SEQ ID NO: 147 - RNA, 21 nt, synthetic construct
  source 1..21: mol_type = other RNA
gttgaggtttctaagacttat

SEQ ID NO: 148 - RNA, 21 nt, synthetic construct
  source 1..21: mol_type = other RNA
attttagaaacctgagacttt

SEQ ID NO: 149 - RNA, 21 nt, synthetic construct
  source 1..21: mol_type = other RNA
tctggcattttagtttaatat

SEQ ID NO: 150 - RNA, 21 nt, synthetic construct
  source 1..21: mol_type = other RNA
aactaatgattgcatttgaat

SEQ ID NO: 151 - RNA, 21 nt, synthetic construct
  source 1..21: mol_type = other RNA
aaagagattcttgaccttatt

SEQ ID NO: 152 - RNA, 21 nt, synthetic construct
  source 1..21: mol_type = other RNA
gagctctgaaatgtcttgatt

SEQ ID NO: 153 - RNA, 21 nt, synthetic construct
  source 1..21: mol_type = other RNA
tggaaggtattaaactatttt

SEQ ID NO: 154 - RNA, 21 nt, synthetic construct
  source 1..21: mol_type = other RNA
tgcctgttgtacaaagaaatt

SEQ ID NO: 155 - RNA, 21 nt, synthetic construct
  source 1..21: mol_type = other RNA
actcgtgaaaagaattactat

SEQ ID NO: 156 - RNA, 21 nt, synthetic construct
  source 1..21: mol_type = other RNA
tgaaataactgcgattttgtt

SEQ ID NO: 157 - RNA, 21 nt, synthetic construct
  source 1..21: mol_type = other RNA
ttggaaatgctgattgatttt

SEQ ID NO: 158 - RNA, 21 nt, synthetic construct
  source 1..21: mol_type = other RNA
ttagtgtattgcaagaaacat

SEQ ID NO: 159 - RNA, 21 nt, synthetic construct
  source 1..21: mol_type = other RNA
cagaaaatgtagttttgtttt

SEQ ID NO: 160 - RNA, 23 nt, synthetic construct
  source 1..23: mol_type = other RNA
aataacataaaacttcaggactc

SEQ ID NO: 161 - RNA, 23 nt, synthetic construct
  source 1..23: mol_type = other RNA
aaagttcttctgtttcataacat

SEQ ID NO: 162 - RNA, 23 nt, synthetic construct
  source 1..23: mol_type = other RNA
aaaagtgtaattcccaaatcatg

SEQ ID NO: 163 - RNA, 23 nt, synthetic construct
  source 1..23: mol_type = other RNA
aataagaaacatctattgtacca

SEQ ID NO: 164 - RNA, 23 nt, synthetic construct
  source 1..23: mol_type = other RNA
aaacactgtattctgatgaatgt

SEQ ID NO: 165 - RNA, 23 nt, synthetic construct
  source 1..23: mol_type = other RNA
aattttaaagttgcagatctgaa

SEQ ID NO: 166 - RNA, 23 nt, synthetic construct
  source 1..23: mol_type = other RNA
aattaggctttctttccatttta

SEQ ID NO: 167 - RNA, 23 nt, synthetic construct
  source 1..23: mol_type = other RNA
agtaacaacatcttccaacaaat

SEQ ID NO: 168 - RNA, 23 nt, synthetic construct
  source 1..23: mol_type = other RNA
atgatataaataacattccgcaa

SEQ ID NO: 169 - RNA, 23 nt, synthetic construct
  source 1..23: mol_type = other RNA
attgtgtgagtttcattgatata

SEQ ID NO: 170 - RNA, 23 nt, synthetic construct
  source 1..23: mol_type = other RNA
aaagaacgtaagaaaggcgtctt

SEQ ID NO: 171 - RNA, 23 nt, synthetic construct
  source 1..23: mol_type = other RNA
aacattttcagtcacattggtgg

SEQ ID NO: 172 - RNA, 23 nt, synthetic construct
  source 1..23: mol_type = other RNA
atttcactttgttaacggctttt

SEQ ID NO: 173 - RNA, 23 nt, synthetic construct
  source 1..23: mol_type = other RNA
aatttcttgaagaatccttttag

SEQ ID NO: 174 - RNA, 23 nt, synthetic construct
  source 1..23: mol_type = other RNA
aaatttgaatgttccaaaagaag

SEQ ID NO: 175 - RNA, 23 nt, synthetic construct
  source 1..23: mol_type = other RNA
aaagttgacctttgtgaatttga

SEQ ID NO: 176 - RNA, 23 nt, synthetic construct
  source 1..23: mol_type = other RNA
agatctatgaactggtagaaaca

SEQ ID NO: 177 - RNA, 23 nt, synthetic construct
  source 1..23: mol_type = other RNA
aagatagtcaatatgggatctat

SEQ ID NO: 178 - RNA, 23 nt, synthetic construct
  source 1..23: mol_type = other RNA
aagaagagaatgaaagtgagcag

SEQ ID NO: 179 - RNA, 23 nt, synthetic construct
  source 1..23: mol_type = other RNA
aatgttgagattattgcctgaag

SEQ ID NO: 180 - RNA, 23 nt, synthetic construct
  source 1..23: mol_type = other RNA
atatggatcaaggtactgaagat

SEQ ID NO: 181 - RNA, 23 nt, synthetic construct
  source 1..23: mol_type = other RNA
aaaagctctatagagaacatctt

SEQ ID NO: 182 - RNA, 23 nt, synthetic construct
  source 1..23: mol_type = other RNA
aaagtaattcaactatatgccca

SEQ ID NO: 183 - RNA, 23 nt, synthetic construct
  source 1..23: mol_type = other RNA
aattggtagacagagtatctacc

SEQ ID NO: 184 - RNA, 23 nt, synthetic construct
  source 1..23: mol_type = other RNA
agtattatcaagatgtctgggat

SEQ ID NO: 185 - RNA, 23 nt, synthetic construct
  source 1..23: mol_type = other RNA
aatcataggagattccaacaggt

SEQ ID NO: 186 - RNA, 23 nt, synthetic construct
  source 1..23: mol_type = other RNA
attcttcttaggtttgcccagtt

SEQ ID NO: 187 - RNA, 23 nt, synthetic construct
  source 1..23: mol_type = other RNA
atttcgtaacattctaataacac

SEQ ID NO: 188 - RNA, 23 nt, synthetic construct
  source 1..23: mol_type = other RNA
attcctttaaggaaaatggctgt

SEQ ID NO: 189 - RNA, 23 nt, synthetic construct
  source 1..23: mol_type = other RNA
aactttggctttctaaatattcc

SEQ ID NO: 190 - RNA, 23 nt, synthetic construct
  source 1..23: mol_type = other RNA
attgaaggaagtatagctggtaa

SEQ ID NO: 191 - RNA, 23 nt, synthetic construct
  source 1..23: mol_type = other RNA
attgcatttctggactcattaat

SEQ ID NO: 192 - RNA, 23 nt, synthetic construct
  source 1..23: mol_type = other RNA
aagatttgcaatcaacctccttc

SEQ ID NO: 193 - RNA, 23 nt, synthetic construct
  source 1..23: mol_type = other RNA
attcatcacaaagaagtcttcga

SEQ ID NO: 194 - RNA, 23 nt, synthetic construct
  source 1..23: mol_type = other RNA
aattactacatcttctgaatttc

SEQ ID NO: 195 - RNA, 23 nt, synthetic construct
  source 1..23: mol_type = other RNA
aagaagttgagttcgaagactga

SEQ ID NO: 196 - RNA, 23 nt, synthetic construct
  source 1..23: mol_type = other RNA
acatgataaagacatgaagtacc

SEQ ID NO: 197 - RNA, 23 nt, synthetic construct
  source 1..23: mol_type = other RNA
atcttgttcagaactgcataaag

SEQ ID NO: 198 - RNA, 23 nt, synthetic construct
  source 1..23: mol_type = other RNA
aataaactttcctactgtttcat

SEQ ID NO: 199 - RNA, 23 nt, synthetic construct
  source 1..23: mol_type = other RNA
atcttcttcatcacttctccaag

SEQ ID NO: 200 - RNA, 23 nt, synthetic construct
  source 1..23: mol_type = other RNA
atctgtaagaaggtgataaactg

SEQ ID NO: 201 - RNA, 23 nt, synthetic construct
  source 1..23: mol_type = other RNA
attttgcagatactcaggttctg

SEQ ID NO: 202 - RNA, 23 nt, synthetic construct
  source 1..23: mol_type = other RNA
attattaggtatttgtgcaactt

SEQ ID NO: 203 - RNA, 23 nt, synthetic construct
  source 1..23: mol_type = other RNA
aatttctttctgttctggttatt

SEQ ID NO: 204 - RNA, 23 nt, synthetic construct
  source 1..23: mol_type = other RNA
aattcttcacaagacaatatgtg

SEQ ID NO: 205 - RNA, 23 nt, synthetic construct
  source 1..23: mol_type = other RNA
attaaacattttcacagcattct

SEQ ID NO: 206 - RNA, 23 nt, synthetic construct
  source 1..23: mol_type = other RNA
aagttctaaaacagacactctct

SEQ ID NO: 207 - RNA, 23 nt, synthetic construct
  source 1..23: mol_type = other RNA
aaccacaaaactcagaatatatt

SEQ ID NO: 208 - RNA, 23 nt, synthetic construct
  source 1..23: mol_type = other RNA
actacaaggaactcatctcatga

SEQ ID NO: 209 - RNA, 23 nt, synthetic construct
  source 1..23: mol_type = other RNA
attattgagatttcatcttgtag

SEQ ID NO: 210 - RNA, 23 nt, synthetic construct
  source 1..23: mol_type = other RNA
aaattagtccttaaaagttgtac

SEQ ID NO: 211 - RNA, 23 nt, synthetic construct
  source 1..23: mol_type = other RNA
ataagtataccatgtaagattca

SEQ ID NO: 212 - RNA, 23 nt, synthetic construct
  source 1..23: mol_type = other RNA
aaaccagataatataccaacaaa

SEQ ID NO: 213 - RNA, 23 nt, synthetic construct
  source 1..23: mol_type = other RNA
aaaggaagcattaaccactaacc

SEQ ID NO: 214 - RNA, 23 nt, synthetic construct
  source 1..23: mol_type = other RNA
aaagagtgaatggatgactcaat

SEQ ID NO: 215 - RNA, 23 nt, synthetic construct
  source 1..23: mol_type = other RNA
aactattgacagataaaactgaa

SEQ ID NO: 216 - RNA, 23 nt, synthetic construct
  source 1..23: mol_type = other RNA
aaatttataaagcactttgggat

SEQ ID NO: 217 - RNA, 23 nt, synthetic construct
  source 1..23: mol_type = other RNA
aaaacatttctaaatctgacagc

SEQ ID NO: 218 - RNA, 23 nt, synthetic construct
  source 1..23: mol_type = other RNA
aaatattgtctgttttcacatag

SEQ ID NO: 219 - RNA, 23 nt, synthetic construct
  source 1..23: mol_type = other RNA
attgattacaatatctcagttcc

SEQ ID NO: 220 - RNA, 23 nt, synthetic construct
  source 1..23: mol_type = other RNA
aaaattaacttcctgatgttaac

SEQ ID NO: 221 - RNA, 23 nt, synthetic construct
  source 1..23: mol_type = other RNA
aaagtttccctagaattttgcca

SEQ ID NO: 222 - RNA, 23 nt, synthetic construct
  source 1..23: mol_type = other RNA
atttatatgagcaaaagccttca

SEQ ID NO: 223 - RNA, 23 nt, synthetic construct
  source 1..23: mol_type = other RNA
atcatttgaaactcaatggcact

SEQ ID NO: 224 - RNA, 23 nt, synthetic construct
  source 1..23: mol_type = other RNA
atctaaatatatttgctggtcat

SEQ ID NO: 225 - RNA, 23 nt, synthetic construct
  source 1..23: mol_type = other RNA
attggttggaggatttccaagaa

SEQ ID NO: 226 - RNA, 23 nt, synthetic construct
  source 1..23: mol_type = other RNA
aagttaggaaaactgctatttgg

SEQ ID NO: 227 - RNA, 23 nt, synthetic construct
  source 1..23: mol_type = other RNA
aattctaacagtctgtcagctca

SEQ ID NO: 228 - RNA, 23 nt, synthetic construct
  source 1..23: mol_type = other RNA
aaaatccataaatgcctctaacc

SEQ ID NO: 229 - RNA, 23 nt, synthetic construct
  source 1..23: mol_type = other RNA
agtttaggcatataacccataaa

SEQ ID NO: 230 - RNA, 23 nt, synthetic construct
  source 1..23: mol_type = other RNA
aaattatttaccactatgtggca

SEQ ID NO: 231 - RNA, 23 nt, synthetic construct
  source 1..23: mol_type = other RNA
ataccaattatgaacagaccatt

SEQ ID NO: 232 - RNA, 23 nt, synthetic construct
  source 1..23: mol_type = other RNA
aataaaccaataattatgctccc

SEQ ID NO: 233 - RNA, 23 nt, synthetic construct
  source 1..23: mol_type = other RNA
aaccataattaccataataaacc

SEQ ID NO: 234 - RNA, 23 nt, synthetic construct
  source 1..23: mol_type = other RNA
aaactgttagaaaacgttttaac

SEQ ID NO: 235 - RNA, 23 nt, synthetic construct
  source 1..23: mol_type = other RNA
aaattccataatatcttggagat

SEQ ID NO: 236 - RNA, 23 nt, synthetic construct
  source 1..23: mol_type = other RNA
aaagaatctatgtaacactcatc

SEQ ID NO: 237 - RNA, 23 nt, synthetic construct
  source 1..23: mol_type = other RNA
acaaacttaattctcagtacttt

SEQ ID NO: 238 - RNA, 23 nt, synthetic construct
  source 1..23: mol_type = other RNA
aatactatcagtgtttaaaatcc

SEQ ID NO: 239 - RNA, 23 nt, synthetic construct
  source 1..23: mol_type = other RNA
aaaacacacattactcatgagat

SEQ ID NO: 240 - RNA, 23 nt, synthetic construct
  source 1..23: mol_type = other RNA
atgtgaaatatcaatcagcatcc

SEQ ID NO: 241 - RNA, 23 nt, synthetic construct
  source 1..23: mol_type = other RNA
attcaaacatggtatttcataca

SEQ ID NO: 242 - RNA, 23 nt, synthetic construct
  source 1..23: mol_type = other RNA
aattattgctatgagtttcaaac

SEQ ID NO: 243 - RNA, 23 nt, synthetic construct
  source 1..23: mol_type = other RNA
aatcacaacagcatagcattatt

SEQ ID NO: 244 - RNA, 23 nt, synthetic construct
  source 1..23: mol_type = other RNA
atattttaaatgcagaacttgag

SEQ ID NO: 245 - RNA, 23 nt, synthetic construct
  source 1..23: mol_type = other RNA
aatgacttcatggtatacatcaa

SEQ ID NO: 246 - RNA, 23 nt, synthetic construct
  source 1..23: mol_type = other RNA
aaacatcagagctactacaactg

SEQ ID NO: 247 - RNA, 23 nt, synthetic construct
  source 1..23: mol_type = other RNA
aaaaacatgatatctcattcaac

SEQ ID NO: 248 - RNA, 23 nt, synthetic construct
  source 1..23: mol_type = other RNA
aagtaaaatggaatgctaaaaca

SEQ ID NO: 249 - RNA, 23 nt, synthetic construct
  source 1..23: mol_type = other RNA
acttgagtaatccttaatttaca

SEQ ID NO: 250 - RNA, 23 nt, synthetic construct
  source 1..23: mol_type = other RNA
aaatcttgaataatggtgagctt

SEQ ID NO: 251 - RNA, 23 nt, synthetic construct
  source 1..23: mol_type = other RNA
aaaaataatgcaagagaagccgt

SEQ ID NO: 252 - RNA, 23 nt, synthetic construct
  source 1..23: mol_type = other RNA
atacttctagaaaacaaaccaac

SEQ ID NO: 253 - RNA, 23 nt, synthetic construct
  source 1..23: mol_type = other RNA
aaaagattttcaaagcaccagtt

SEQ ID NO: 254 - RNA, 23 nt, synthetic construct
  source 1..23: mol_type = other RNA
aaaattaactcaaaggtcagctt

SEQ ID NO: 255 - RNA, 23 nt, synthetic construct
  source 1..23: mol_type = other RNA
aactgaagaatgagttgtgctga

SEQ ID NO: 256 - RNA, 23 nt, synthetic construct
  source 1..23: mol_type = other RNA
attgttttcagtcatgaggcact

SEQ ID NO: 257 - RNA, 23 nt, synthetic construct
  source 1..23: mol_type = other RNA
atcattgtgaagatgctttcgtt

SEQ ID NO: 258 - RNA, 23 nt, synthetic construct
  source 1..23: mol_type = other RNA
attttagcaaaacggtgctatct

SEQ ID NO: 259 - RNA, 23 nt, synthetic construct
  source 1..23: mol_type = other RNA
agaaaacaatgagaatgtatctt

SEQ ID NO: 260 - RNA, 23 nt, synthetic construct
  source 1..23: mol_type = other RNA
atttgtttaaccttatgtggaag

SEQ ID NO: 261 - RNA, 23 nt, synthetic construct
  source 1..23: mol_type = other RNA
ataaattatttacaagcacctag

SEQ ID NO: 262 - RNA, 23 nt, synthetic construct
  source 1..23: mol_type = other RNA
agttacagaaatgcgatagagta

SEQ ID NO: 263 - RNA, 23 nt, synthetic construct
  source 1..23: mol_type = other RNA
aacttaggacattctcattttca

SEQ ID NO: 264 - RNA, 23 nt, synthetic construct
  source 1..23: mol_type = other RNA
atttcatgcattttcagagtgca

SEQ ID NO: 265 - RNA, 23 nt, synthetic construct
  source 1..23: mol_type = other RNA
aagttaacagttctacacatttc

SEQ ID NO: 266 - RNA, 23 nt, synthetic construct
  source 1..23: mol_type = other RNA
aaatttaacagattccagaagga

SEQ ID NO: 267 - RNA, 23 nt, synthetic construct
  source 1..23: mol_type = other RNA
atattttctccatttaccctcat

SEQ ID NO: 268 - RNA, 23 nt, synthetic construct
  source 1..23: mol_type = other RNA
attacattcattgtaatcccaga

SEQ ID NO: 269 - RNA, 23 nt, synthetic construct
  source 1..23: mol_type = other RNA
aaattccacaatttgggcttaca

SEQ ID NO: 270 - RNA, 23 nt, synthetic construct
  source 1..23: mol_type = other RNA
atttctataaaacactgatgaac

SEQ ID NO: 271 - RNA, 23 nt, synthetic construct
  source 1..23: mol_type = other RNA
agtcaaaatagtttgggcaatgc

SEQ ID NO: 272 - RNA, 23 nt, synthetic construct
  source 1..23: mol_type = other RNA
attagtgagaggttcataagtat

SEQ ID NO: 273 - RNA, 23 nt, synthetic construct
  source 1..23: mol_type = other RNA
atctaacatagtgtttcccaaaa

SEQ ID NO: 274 - RNA, 23 nt, synthetic construct
  source 1..23: mol_type = other RNA
attttgtctccttaaagaactat

SEQ ID NO: 275 - RNA, 23 nt, synthetic construct
  source 1..23: mol_type = other RNA
agttacaaaatgcatgcatattc

SEQ ID NO: 276 - RNA, 23 nt, synthetic construct
  source 1..23: mol_type = other RNA
aaaatacacatctattcaacgcc

SEQ ID NO: 277 - RNA, 23 nt, synthetic construct
  source 1..23: mol_type = other RNA
aaattttctgtgcttattttctg

SEQ ID NO: 278 - RNA, 23 nt, synthetic construct
  source 1..23: mol_type = other RNA
aattctgatacgttcagtgaaaa

SEQ ID NO: 279 - RNA, 23 nt, synthetic construct
  source 1..23: mol_type = other RNA
actgaattaaaaccttatttacc

SEQ ID NO: 280 - RNA, 23 nt, synthetic construct
  source 1..23: mol_type = other RNA
aaatactttcttctagatctgaa

SEQ ID NO: 281 - RNA, 23 nt, synthetic construct
  source 1..23: mol_type = other RNA
ataaacactacaactatctgtgg

SEQ ID NO: 282 - RNA, 23 nt, synthetic construct
  source 1..23: mol_type = other RNA
ataagtcttagaaacctcaacga

SEQ ID NO: 283 - RNA, 23 nt, synthetic construct
  source 1..23: mol_type = other RNA
aaagtctcaggtttctaaaatag

SEQ ID NO: 284 - RNA, 23 nt, synthetic construct
  source 1..23: mol_type = other RNA
atattaaactaaaatgccagacg

SEQ ID NO: 285 - RNA, 23 nt, synthetic construct
  source 1..23: mol_type = other RNA
attcaaatgcaatcattagtttg

SEQ ID NO: 286 - RNA, 23 nt, synthetic construct
  source 1..23: mol_type = other RNA
aataaggtcaagaatctctttca

SEQ ID NO: 287 - RNA, 23 nt, synthetic construct
  source 1..23: mol_type = other RNA
aatcaagacatttcagagctcta

SEQ ID NO: 288 - RNA, 23 nt, synthetic construct
  source 1..23: mol_type = other RNA
aaaatagtttaataccttccatc

SEQ ID NO: 289 - RNA, 23 nt, synthetic construct
  source 1..23: mol_type = other RNA
aatttctttgtacaacaggcaaa

SEQ ID NO: 290 - RNA, 23 nt, synthetic construct
  source 1..23: mol_type = other RNA
atagtaattcttttcacgagtct

SEQ ID NO: 291 - RNA, 23 nt, synthetic construct
  source 1..23: mol_type = other RNA
aacaaaatcgcagttatttcaca

SEQ ID NO: 292 - RNA, 23 nt, synthetic construct
  source 1..23: mol_type = other RNA
aaaatcaatcagcatttccaagt

SEQ ID NO: 293 - RNA, 23 nt, synthetic construct
  source 1..23: mol_type = other RNA
atgtttcttgcaatacactaaca

SEQ ID NO: 294 - RNA, 23 nt, synthetic construct
  source 1..23: mol_type = other RNA
aaaacaaaactacattttctgtg

SEQ ID NO: 295 - RNA, 21 nt, synthetic construct
  source 1..21: mol_type = other RNA
  modified_base 1: mod_base = OTHER; note = 2'-O-methylguanosine-3'-phosphorothioate
  modified_base 2: mod_base = OTHER; note = 2'-O-methyluridine-3'-phosphorothioate
  modified_base 3: mod_base = OTHER; note = 2'-O-methylcytidine-3'-phosphate
  modified_base 4: mod_base = OTHER; note = 2'-O-methylcytidine-3'-phosphate
  modified_base 5: mod_base = OTHER; note = 2'-O-methyluridine-3'-phosphate
  modified_base 6: mod_base = OTHER; note = 2'-O-methylguanosine-3'-phosphate
  modified_base 7: mod_base = OTHER; note = 2'-deoxy-2'-fluoroadenosine-3'-phosphate
  modified_base 8: mod_base = OTHER; note = 2'-O-methyladenosine-3'-phosphate
  modified_base 9: mod_base = OTHER; note = 2'-deoxy-2'-fluoroguanosine-3'-phosphate
  modified_base 10: mod_base = OTHER; note = 2'-deoxy-2'-fluorouridine-3'-phosphate
  modified_base 11: mod_base = OTHER; note = 2'-deoxy-2'-fluorouridine-3'-phosphate
  modified_base 12: mod_base = OTHER; note = 2'-O-methyluridine-3'-phosphate
  modified_base 13: mod_base = OTHER; note = 2'-O-methyluridine-3'-phosphate
  modified_base 14: mod_base = OTHER; note = 2'-O-methyladenosine-3'-phosphate
  modified_base 15: mod_base = OTHER; note = 2'-O-methyluridine-3'-phosphate
  modified_base 16: mod_base = OTHER; note = 2'-O-methylguanosine-3'-phosphate
  modified_base 17: mod_base = OTHER; note = 2'-O-methyluridine-3'-phosphate
  modified_base 18: mod_base = OTHER; note = 2'-O-methyluridine-3'-phosphate
  modified_base 19: mod_base = OTHER; note = 2'-O-methyladenosine-3'-phosphate
  modified_base 20: mod_base = OTHER; note = 2'-O-methyluridine-3'-phosphate
  modified_base 21: mod_base = OTHER; note = 2'-O-methyluridine-3'-phosphate ((2S,4R)-1-[29-[[2-(acetylamino)-2-deoxy-beta-D-galactopyranosyl]oxy]-14,14-bis[[3-[[3-[[5-[[2-(acetylamino)-2-deoxy-beta-D-galactopyranosyl]oxy]-1-oxopentyl]amino]propyl]amino]-3-oxopropoxy]methyl]-1,12,19,25-tetraoxo-16-oxa-13,20,24-triazanonacos-1-yl]-4-hydroxy-2-pyrrolidinyl)methyl ester
gtcctgaagttttatgttatt

SEQ ID NO: 296 - RNA, 21 nt, synthetic construct
  source 1..21: mol_type = other RNA
  modified_base 1: mod_base = OTHER; note = 2'-O-methylguanosine-3'-phosphorothioate
  modified_base 2: mod_base = OTHER; note = 2'-O-methyluridine-3'-phosphorothioate
  modified_base 3: mod_base = OTHER; note = 2'-O-methyluridine-3'-phosphate
  modified_base 4: mod_base = OTHER; note = 2'-O-methyladenosine-3'-phosphate
  modified_base 5: mod_base = OTHER; note = 2'-O-methyluridine-3'-phosphate
  modified_base 6: mod_base = OTHER; note = 2'-O-methylguanosine-3'-phosphate
  modified_base 7: mod_base = OTHER; note = 2'-deoxy-2'-fluoroadenosine-3'-phosphate
  modified_base 8: mod_base = OTHER; note = 2'-O-methyladenosine-3'-phosphate
  modified_base 9: mod_base = OTHER; note = 2'-deoxy-2'-fluoroadenosine-3'-phosphate
  modified_base 10: mod_base = OTHER; note = 2'-deoxy-2'-fluorocytidine-3'-phosphate
  modified_base 11: mod_base = OTHER; note = 2'-deoxy-2'-fluoroadenosine-3'-phosphate
  modified_base 12: mod_base = OTHER; note = 2'-O-methylguanosine-3'-phosphate
  modified_base 13: mod_base = OTHER; note = 2'-O-methyladenosine-3'-phosphate
  modified_base 14: mod_base = OTHER; note = 2'-O-methyladenosine-3'-phosphate
  modified_base 15: mod_base = OTHER; note = 2'-O-methylguanosine-3'-phosphate
  modified_base 16: mod_base = OTHER; note = 2'-O-methyladenosine-3'-phosphate
  modified_base 17: mod_base = OTHER; note = 2'-O-methyladenosine-3'-phosphate
  modified_base 18: mod_base = OTHER; note = 2'-O-methylcytidine-3'-phosphate
  modified_base 19: mod_base = OTHER; note = 2'-O-methyluridine-3'-phosphate
  modified_base 20: mod_base = OTHER; note = 2'-O-methyluridine-3'-phosphate
  modified_base 21: mod_base = OTHER; note = 2'-O-methyluridine-3'-phosphate ((2S,4R)-1-[29-[[2-(acetylamino)-2-deoxy-beta-D-galactopyranosyl]oxy]-14,14-bis[[3-[[3-[[5-[[2-(acetylamino)-2-deoxy-beta-D-galactopyranosyl]oxy]-1-oxopentyl]amino]propyl]amino]-3-oxopropoxy]methyl]-1,12,19,25-tetraoxo-16-oxa-13,20,24-triazanonacos-1-yl]-4-hydroxy-2-pyrrolidinyl)methyl ester
gttatgaaacagaagaacttt

SEQ ID NO: 297 - RNA, 21 nt, synthetic construct
  source 1..21: mol_type = other RNA
  modified_base 1: mod_base = OTHER; note = 2'-O-methyluridine-3'-phosphorothioate
  modified_base 2: mod_base = OTHER; note = 2'-O-methylguanosine-3'-phosphorothioate
  modified_base 3: mod_base = OTHER; note = 2'-O-methyladenosine-3'-phosphate
  modified_base 4: mod_base = OTHER; note = 2'-O-methyluridine-3'-phosphate
  modified_base 5: mod_base = OTHER; note = 2'-O-methyluridine-3'-phosphate
  modified_base 6: mod_base = OTHER; note = 2'-O-methyluridine-3'-phosphate
  modified_base 7: mod_base = OTHER; note = 2'-deoxy-2'-fluoroguanosine-3'-phosphate
  modified_base 8: mod_base = OTHER; note = 2'-O-methylguanosine-3'-phosphate
  modified_base 9: mod_base = OTHER; note = 2'-deoxy-2'-fluoroguanosine-3'-phosphate
  modified_base 10: mod_base = OTHER; note = 2'-deoxy-2'-fluoroadenosine-3'-phosphate
  modified_base 11: mod_base = OTHER; note = 2'-deoxy-2'-fluoroadenosine-3'-phosphate
  modified_base 12: mod_base = OTHER; note = 2'-O-methyluridine-3'-phosphate
  modified_base 13: mod_base = OTHER; note = 2'-O-methyluridine-3'-phosphate
  modified_base 14: mod_base = OTHER; note = 2'-O-methyladenosine-3'-phosphate
  modified_base 15: mod_base = OTHER; note = 2'-O-methylcytidine-3'-phosphate
  modified_base 16: mod_base = OTHER; note = 2'-O-methyladenosine-3'-phosphate
  modified_base 17: mod_base = OTHER; note = 2'-O-methylcytidine-3'-phosphate
  modified_base 18: mod_base = OTHER; note = 2'-O-methyluridine-3'-phosphate
  modified_base 19: mod_base = OTHER; note = 2'-O-methyluridine-3'-phosphate
  modified_base 20: mod_base = OTHER; note = 2'-O-methyluridine-3'-phosphate
  modified_base 21: mod_base = OTHER; note = 2'-O-methyluridine-3'-phosphate ((2S,4R)-1-[29-[[2-(acetylamino)-2-deoxy-beta-D-galactopyranosyl]oxy]-14,14-bis[[3-[[3-[[5-[[2-(acetylamino)-2-deoxy-beta-D-galactopyranosyl]oxy]-1-oxopentyl]amino]propyl]amino]-3-oxopropoxy]methyl]-1,12,19,25-tetraoxo-16-oxa-13,20,24-triazanonacos-1-yl]-4-hydroxy-2-pyrrolidinyl)methyl ester
tgatttgggaattacactttt

SEQ ID NO: 298 - RNA, 21 nt, synthetic construct
  source 1..21: mol_type = other RNA
  modified_base 1: mod_base = OTHER; note = 2'-O-methylguanosine-3'-phosphorothioate
  modified_base 2: mod_base = OTHER; note = 2'-O-methyluridine-3'-phosphorothioate
  modified_base 3: mod_base = OTHER; note = 2'-O-methyladenosine-3'-phosphate
  modified_base 4: mod_base = OTHER; note = 2'-O-methylcytidine-3'-phosphate
  modified_base 5: mod_base = OTHER; note = 2'-O-methyladenosine-3'-phosphate
  modified_base 6: mod_base = OTHER; note = 2'-O-methyladenosine-3'-phosphate
  modified_base 7: mod_base = OTHER; note = 2'-deoxy-2'-fluorouridine-3'-phosphate
  modified_base 8: mod_base = OTHER; note = 2'-O-methyladenosine-3'-phosphate
  modified_base 9: mod_base = OTHER; note = 2'-deoxy-2'-fluoroguanosine-3'-phosphate
  modified_base 10: mod_base = OTHER; note = 2'-deoxy-2'-fluoroadenosine-3'-phosphate
  modified_base 11: mod_base = OTHER; note = 2'-deoxy-2'-fluorouridine-3'-phosphate
  modified_base 12: mod_base = OTHER; note = 2'-O-methylguanosine-3'-phosphate
  modified_base 13: mod_base = OTHER; note = 2'-O-methyluridine-3'-phosphate
  modified_base 14: mod_base = OTHER; note = 2'-O-methyluridine-3'-phosphate
  modified_base 15: mod_base = OTHER; note = 2'-O-methyluridine-3'-phosphate
  modified_base 16: mod_base = OTHER; note = 2'-O-methylcytidine-3'-phosphate
  modified_base 17: mod_base = OTHER; note = 2'-O-methyluridine-3'-phosphate
  modified_base 18: mod_base = OTHER; note = 2'-O-methyluridine-3'-phosphate
  modified_base 19: mod_base = OTHER; note = 2'-O-methyladenosine-3'-phosphate
  modified_base 20: mod_base = OTHER; note = 2'-O-methyluridine-3'-phosphate
  modified_base 21: mod_base = OTHER; note = 2'-O-methyluridine-3'-phosphate ((2S,4R)-1-[29-[[2-(acetylamino)-2-deoxy-beta-D-galactopyranosyl]oxy]-14,14-bis[[3-[[3-[[5-[[2-(acetylamino)-2-deoxy-beta-D-galactopyranosyl]oxy]-1-oxopentyl]amino]propyl]amino]-3-oxopropoxy]methyl]-1,12,19,25-tetraoxo-16-oxa-13,20,24-triazanonacos-1-yl]-4-hydroxy-2-pyrrolidinyl)methyl ester
gtacaatagatgtttcttatt

SEQ ID NO: 299 - RNA, 21 nt, synthetic construct
  source 1..21: mol_type = other RNA
  modified_base 1: mod_base = OTHER; note = 2'-O-methyladenosine-3'-phosphorothioate
  modified_base 2: mod_base = OTHER; note = 2'-O-methyluridine-3'-phosphorothioate
  modified_base 3: mod_base = OTHER; note = 2'-O-methyluridine-3'-phosphate
  modified_base 4: mod_base = OTHER; note = 2'-O-methylcytidine-3'-phosphate
  modified_base 5: mod_base = OTHER; note = 2'-O-methyladenosine-3'-phosphate
  modified_base 6: mod_base = OTHER; note = 2'-O-methyluridine-3'-phosphate
  modified_base 7: mod_base = OTHER; note = 2'-deoxy-2'-fluorocytidine-3'-phosphate
  modified_base 8: mod_base = OTHER; note = 2'-O-methyladenosine-3'-phosphate
  modified_base 9: mod_base = OTHER; note = 2'-deoxy-2'-fluoroguanosine-3'-phosphate
  modified_base 10: mod_base = OTHER; note = 2'-deoxy-2'-fluoroadenosine-3'-phosphate
  modified_base 11: mod_base = OTHER; note = 2'-deoxy-2'-fluoroadenosine-3'-phosphate
  modified_base 12: mod_base = OTHER; note = 2'-O-methyluridine-3'-phosphate
  modified_base 13: mod_base = OTHER; note = 2'-O-methyladenosine-3'-phosphate
  modified_base 14: mod_base = OTHER; note = 2'-O-methylcytidine-3'-phosphate
  modified_base 15: mod_base = OTHER; note = 2'-O-methyladenosine-3'-phosphate
  modified_base 16: mod_base = OTHER; note = 2'-O-methylguanosine-3'-phosphate
  modified_base 17: mod_base = OTHER; note = 2'-O-methyluridine-3'-phosphate
  modified_base 18: mod_base = OTHER; note = 2'-O-methylguanosine-3'-phosphate
  modified_base 19: mod_base = OTHER; note = 2'-O-methyluridine-3'-phosphate
  modified_base 20: mod_base = OTHER; note = 2'-O-methyluridine-3'-phosphate
  modified_base 21: mod_base = OTHER; note = 2'-O-methyluridine-3'-phosphate ((2S,4R)-1-[29-[[2-(acetylamino)-2-deoxy-beta-D-galactopyranosyl]oxy]-14,14-bis[[3-[[3-[[5-[[2-(acetylamino)-2-deoxy-beta-D-galactopyranosyl]oxy]-1-oxopentyl]amino]propyl]amino]-3-oxopropoxy]methyl]-1,12,19,25-tetraoxo-16-oxa-13,20,24-triazanonacos-1-yl]-4-hydroxy-2-pyrrolidinyl)methyl ester
attcatcagaatacagtgttt

SEQ ID NO: 300 - RNA, 21 nt, synthetic construct
  source 1..21: mol_type = other RNA
  modified_base 1: mod_base = OTHER; note = 2'-O-methylcytidine-3'-phosphorothioate
  modified_base 2: mod_base = OTHER; note = 2'-O-methyladenosine-3'-phosphorothioate
  modified_base 3: mod_base = OTHER; note = 2'-O-methylguanosine-3'-phosphate
  modified_base 4: mod_base = OTHER; note = 2'-O-methyladenosine-3'-phosphate
  modified_base 5: mod_base = OTHER; note = 2'-O-methyluridine-3'-phosphate
  modified_base 6: mod_base = OTHER; note = 2'-O-methylcytidine-3'-phosphate
  modified_base 7: mod_base = OTHER; note = 2'-deoxy-2'-fluorouridine-3'-phosphate
  modified_base 8: mod_base = OTHER; note = 2'-O-methylguanosine-3'-phosphate
  modified_base 9: mod_base = OTHER; note = 2'-deoxy-2'-fluorocytidine-3'-phosphate
  modified_base 10: mod_base = OTHER; note = 2'-deoxy-2'-fluoroadenosine-3'-phosphate
  modified_base 11: mod_base = OTHER; note = 2'-deoxy-2'-fluoroadenosine-3'-phosphate
  modified_base 12: mod_base = OTHER; note = 2'-O-methylcytidine-3'-phosphate
  modified_base 13: mod_base = OTHER; note = 2'-O-methyluridine-3'-phosphate
  modified_base 14: mod_base = OTHER; note = 2'-O-methyluridine-3'-phosphate
  modified_base 15: mod_base = OTHER; note = 2'-O-methyluridine-3'-phosphate
  modified_base 16: mod_base = OTHER; note = 2'-O-methyladenosine-3'-phosphate
  modified_base 17: mod_base = OTHER; note = 2'-O-methyladenosine-3'-phosphate
  modified_base 18: mod_base = OTHER; note = 2'-O-methyladenosine-3'-phosphate
  modified_base 19: mod_base = OTHER; note = 2'-O-methyladenosine-3'-phosphate
  modified_base 20: mod_base = OTHER; note = 2'-O-methyluridine-3'-phosphate
  modified_base 21: mod_base = OTHER; note = 2'-O-methyluridine-3'-phosphate ((2S,4R)-1-[29-[[2-(acetylamino)-2-deoxy-beta-D-galactopyranosyl]oxy]-14,14-bis[[3-[[3-[[5-[[2-(acetylamino)-2-deoxy-beta-D-galactopyranosyl]oxy]-1-oxopentyl]amino]propyl]amino]-3-oxopropoxy]methyl]-1,12,19,25-tetraoxo-16-oxa-13,20,24-triazanonacos-1-yl]-4-hydroxy-2-pyrrolidinyl)methyl ester
cagatctgcaactttaaaatt

SEQ ID NO: 301 - RNA, 21 nt, synthetic construct
  source 1..21: mol_type = other RNA
  modified_base 1: mod_base = OTHER; note = 2'-O-methyladenosine-3'-phosphorothioate
  modified_base 2: mod_base = OTHER; note = 2'-O-methyladenosine-3'-phosphorothioate
  modified_base 3: mod_base = OTHER; note = 2'-O-methyladenosine-3'-phosphate
  modified_base 4: mod_base = OTHER; note = 2'-O-methyluridine-3'-phosphate
  modified_base 5: mod_base = OTHER; note = 2'-O-methylguanosine-3'-phosphate
  modified_base 6: mod_base = OTHER; note = 2'-O-methylguanosine-3'-phosphate
  modified_base 7: mod_base = OTHER; note = 2'-deoxy-2'-fluoroadenosine-3'-phosphate
  modified_base 8: mod_base = OTHER; note = 2'-O-methyladenosine-3'-phosphate
  modified_base 9: mod_base = OTHER; note = 2'-deoxy-2'-fluoroadenosine-3'-phosphate
  modified_base 10: mod_base = OTHER; note = 2'-deoxy-2'-fluoroguanosine-3'-phosphate
  modified_base 11: mod_base = OTHER; note = 2'-deoxy-2'-fluoroadenosine-3'-phosphate
  modified_base 12: mod_base = OTHER; note = 2'-O-methyladenosine-3'-phosphate
  modified_base 13: mod_base = OTHER; note = 2'-O-methyladenosine-3'-phosphate
  modified_base 14: mod_base = OTHER; note = 2'-O-methylguanosine-3'-phosphate
  modified_base 15: mod_base = OTHER; note = 2'-O-methylcytidine-3'-phosphate
  modified_base 16: mod_base = OTHER; note = 2'-O-methylcytidine-3'-phosphate
  modified_base 17: mod_base = OTHER; note = 2'-O-methyluridine-3'-phosphate
  modified_base 18: mod_base = OTHER; note = 2'-O-methyladenosine-3'-phosphate
  modified_base 19: mod_base = OTHER; note = 2'-O-methyladenosine-3'-phosphate
  modified_base 20: mod_base = OTHER; note = 2'-O-methyluridine-3'-phosphate
  modified_base 21: mod_base = OTHER; note = 2'-O-methyluridine-3'-phosphate ((2S,4R)-1-[29-[[2-(acetylamino)-2-deoxy-beta-D-galactopyranosyl]oxy]-14,14-bis[[3-[[3-[[5-[[2-(acetylamino)-2-deoxy-beta-D-galactopyranosyl]oxy]-1-oxopentyl]amino]propyl]amino]-3-oxopropoxy]methyl]-1,12,19,25-tetraoxo-16-oxa-13,20,24-triazanonacos-1-yl]-4-hydroxy-2-pyrrolidinyl)methyl ester
aaatggaaagaaagcctaatt

SEQ ID NO: 302 - RNA, 21 nt, synthetic construct
  source 1..21: mol_type = other RNA
  modified_base 1: mod_base = OTHER; note = 2'-O-methyluridine-3'-phosphorothioate
  modified_base 2: mod_base = OTHER; note = 2'-O-methyluridine-3'-phosphorothioate
  modified_base 3: mod_base = OTHER; note = 2'-O-methylguanosine-3'-phosphate
  modified_base 4: mod_base = OTHER; note = 2'-O-methyluridine-3'-phosphate
  modified_base 5: mod_base = OTHER; note = 2'-O-methyluridine-3'-phosphate
  modified_base 6: mod_base = OTHER; note = 2'-O-methylguanosine-3'-phosphate
  modified_base 7: mod_base = OTHER; note = 2'-deoxy-2'-fluoroguanosine-3'-phosphate
  modified_base 8: mod_base = OTHER; note = 2'-O-methyladenosine-3'-phosphate
  modified_base 9: mod_base = OTHER; note = 2'-deoxy-2'-fluoroadenosine-3'-phosphate
  modified_base 10: mod_base = OTHER; note = 2'-deoxy-2'-fluoroguanosine-3'-phosphate
  modified_base 11: mod_base = OTHER; note = 2'-deoxy-2'-fluoroadenosine-3'-phosphate
  modified_base 12: mod_base = OTHER; note = 2'-O-methyluridine-3'-phosphate
  modified_base 13: mod_base = OTHER; note = 2'-O-methylguanosine-3'-phosphate
  modified_base 14: mod_base = OTHER; note = 2'-O-methyluridine-3'-phosphate
  modified_base 15: mod_base = OTHER; note = 2'-O-methyluridine-3'-phosphate
  modified_base 16: mod_base = OTHER; note = 2'-O-methylguanosine-3'-phosphate
  modified_base 17: mod_base = OTHER; note = 2'-O-methyluridine-3'-phosphate
  modified_base 18: mod_base = OTHER; note = 2'-O-methyluridine-3'-phosphate
  modified_base 19: mod_base = OTHER; note = 2'-O-methyladenosine-3'-phosphate
  modified_base 20: mod_base = OTHER; note = 2'-O-methylcytidine-3'-phosphate
  modified_base 21: mod_base = OTHER; note = 2'-O-methyluridine-3'-phosphate ((2S,4R)-1-[29-[[2-(acetylamino)-2-deoxy-beta-D-galactopyranosyl]oxy]-14,14-bis[[3-[[3-[[5-[[2-(acetylamino)-2-deoxy-beta-D-galactopyranosyl]oxy]-1-oxopentyl]amino]propyl]amino]-3-oxopropoxy]methyl]-1,12,19,25-tetraoxo-16-oxa-13,20,24-triazanonacos-1-yl]-4-hydroxy-2-pyrrolidinyl)methyl ester
ttgttggaagatgttgttact

SEQ ID NO: 303 - RNA, 21 nt, synthetic construct
  source 1..21: mol_type = other RNA
  modified_base 1: mod_base = OTHER; note = 2'-O-methylguanosine-3'-phosphorothioate
  modified_base 2: mod_base = OTHER; note = 2'-O-methylcytidine-3'-phosphorothioate
  modified_base 3: mod_base = OTHER; note = 2'-O-methylguanosine-3'-phosphate
  modified_base 4: mod_base = OTHER; note = 2'-O-methylguanosine-3'-phosphate
  modified_base 5: mod_base = OTHER; note = 2'-O-methyladenosine-3'-phosphate
  modified_base 6: mod_base = OTHER; note = 2'-O-methyladenosine-3'-phosphate
  modified_base 7: mod_base = OTHER; note = 2'-deoxy-2'-fluorouridine-3'-phosphate
  modified_base 8: mod_base = OTHER; note = 2'-O-methylguanosine-3'-phosphate
  modified_base 9: mod_base = OTHER; note = 2'-deoxy-2'-fluorouridine-3'-phosphate
  modified_base 10: mod_base = OTHER; note = 2'-deoxy-2'-fluorouridine-3'-phosphate
  modified_base 11: mod_base = OTHER; note = 2'-deoxy-2'-fluoroadenosine-3'-phosphate
  modified_base 12: mod_base = OTHER; note = 2'-O-methyluridine-3'-phosphate
  modified_base 13: mod_base = OTHER; note = 2'-O-methyluridine-3'-phosphate
  modified_base 14: mod_base = OTHER; note = 2'-O-methyluridine-3'-phosphate
  modified_base 15: mod_base = OTHER; note = 2'-O-methyladenosine-3'-phosphate
  modified_base 16: mod_base = OTHER; note = 2'-O-methyluridine-3'-phosphate
  modified_base 17: mod_base = OTHER; note = 2'-O-methyladenosine-3'-phosphate
  modified_base 18: mod_base = OTHER; note = 2'-O-methyluridine-3'-phosphate
  modified_base 19: mod_base = OTHER; note = 2'-O-methylcytidine-3'-phosphate
  modified_base 20: mod_base = OTHER; note = 2'-O-methyladenosine-3'-phosphate
  modified_base 21: mod_base = OTHER; note = 2'-O-methyluridine-3'-phosphate ((2S,4R)-1-[29-[[2-(acetylamino)-2-deoxy-beta-D-galactopyranosyl]oxy]-14,14-bis[[3-[[3-[[5-[[2-(acetylamino)-2-deoxy-beta-D-galactopyranosyl]oxy]-1-oxopentyl]amino]propyl]amino]-3-oxopropoxy]methyl]-1,12,19,25-tetraoxo-16-oxa-13,20,24-triazanonacos-1-yl]-4-hydroxy-2-pyrrolidinyl)methyl ester
gcggaatgttatttatatcat

SEQ ID NO: 304 - RNA, 21 nt, synthetic construct
  source 1..21: mol_type = other RNA
  modified_base 1: mod_base = OTHER; note = 2'-O-methyluridine-3'-phosphorothioate
  modified_base 2: mod_base = OTHER; note = 2'-O-methyladenosine-3'-phosphorothioate
  modified_base 3: mod_base = OTHER; note = 2'-O-methyluridine-3'-phosphate
  modified_base 4: mod_base = OTHER; note = 2'-O-methylcytidine-3'-phosphate
  modified_base 5: mod_base = OTHER; note = 2'-O-methyladenosine-3'-phosphate
  modified_base 6: mod_base = OTHER; note = 2'-O-methyladenosine-3'-phosphate
  modified_base 7: mod_base = OTHER; note = 2'-deoxy-2'-fluorouridine-3'-phosphate
  modified_base 8: mod_base = OTHER; note = 2'-O-methylguanosine-3'-phosphate
  modified_base 9: mod_base = OTHER; note = 2'-deoxy-2'-fluoroadenosine-3'-phosphate
  modified_base 10: mod_base = OTHER; note = 2'-deoxy-2'-fluoroadenosine-3'-phosphate
  modified_base 11: mod_base = OTHER; note = 2'-deoxy-2'-fluoroadenosine-3'-phosphate
  modified_base 12: mod_base = OTHER; note = 2'-O-methylcytidine-3'-phosphate
  modified_base 13: mod_base = OTHER; note = 2'-O-methyluridine-3'-phosphate
  modified_base 14: mod_base = OTHER; note = 2'-O-methylcytidine-3'-phosphate
  modified_base 15: mod_base = OTHER; note = 2'-O-methyladenosine-3'-phosphate
  modified_base 16: mod_base = OTHER; note = 2'-O-methylcytidine-3'-phosphate
  modified_base 17: mod_base = OTHER; note = 2'-O-methyladenosine-3'-phosphate
  modified_base 18: mod_base = OTHER; note = 2'-O-methylcytidine-3'-phosphate
  modified_base 19: mod_base = OTHER; note = 2'-O-methyladenosine-3'-phosphate
  modified_base 20: mod_base = OTHER; note = 2'-O-methyladenosine-3'-phosphate
  modified_base 21: mod_base = OTHER; note = 2'-O-methyluridine-3'-phosphate ((2S,4R)-1-[29-[[2-(acetylamino)-2-deoxy-beta-D-galactopyranosyl]oxy]-14,14-bis[[3-[[3-[[5-[[2-(acetylamino)-2-deoxy-beta-D-galactopyranosyl]oxy]-1-oxopentyl]amino]propyl]amino]-3-oxopropoxy]methyl]-1,12,19,25-tetraoxo-16-oxa-13,20,24-triazanonacos-1-yl]-4-hydroxy-2-pyrrolidinyl)methyl ester
tatcaatgaaactcacacaat

SEQ ID NO: 305 - RNA, 21 nt, synthetic construct
  source 1..21: mol_type = other RNA
  modified_base 1: mod_base = OTHER; note = 2'-O-methylguanosine-3'-phosphorothioate
  modified_base 2: mod_base = OTHER; note = 2'-O-methyladenosine-3'-phosphorothioate
  modified_base 3: mod_base = OTHER; note = 2'-O-methylcytidine-3'-phosphate
  modified_base 4: mod_base = OTHER; note = 2'-O-methylguanosine-3'-phosphate
  modified_base 5: mod_base = OTHER; note = 2'-O-methylcytidine-3'-phosphate
  modified_base 6: mod_base = OTHER; note = 2'-O-methylcytidine-3'-phosphate
  modified_base 7: mod_base = OTHER; note = 2'-deoxy-2'-fluorouridine-3'-phosphate
  modified_base 8: mod_base = OTHER; note = 2'-O-methyluridine-3'-phosphate
  modified_base 9: mod_base = OTHER; note = 2'-deoxy-2'-fluorouridine-3'-phosphate
  modified_base 10: mod_base = OTHER; note = 2'-deoxy-2'-fluorocytidine-3'-phosphate
  modified_base 11: mod_base = OTHER; note = 2'-deoxy-2'-fluorouridine-3'-phosphate
  modified_base 12: mod_base = OTHER; note = 2'-O-methyluridine-3'-phosphate
  modified_base 13: mod_base = OTHER; note = 2'-O-methyladenosine-3'-phosphate
  modified_base 14: mod_base = OTHER; note = 2'-O-methylcytidine-3'-phosphate
  modified_base 15: mod_base = OTHER; note = 2'-O-methylguanosine-3'-phosphate
  modified_base 16: mod_base = OTHER; note = 2'-O-methyluridine-3'-phosphate
  modified_base 17: mod_base = OTHER; note = 2'-O-methyluridine-3'-phosphate
  modified_base 18: mod_base = OTHER; note = 2'-O-methylcytidine-3'-phosphate
  modified_base 19: mod_base = OTHER; note = 2'-O-methyluridine-3'-phosphate
  modified_base 20: mod_base = OTHER; note = 2'-O-methyluridine-3'-phosphate
  modified_base 21: mod_base = OTHER; note = 2'-O-methyluridine-3'-phosphate ((2S,4R)-1-[29-[[2-(acetylamino)-2-deoxy-beta-D-galactopyranosyl]oxy]-14,14-bis[[3-[[3-[[5-[[2-(acetylamino)-2-deoxy-beta-D-galactopyranosyl]oxy]-1-oxopentyl]amino]propyl]amino]-3-oxopropoxy]methyl]-1,12,19,25-tetraoxo-16-oxa-13,20,24-triazanonacos-1-yl]-4-hydroxy-2-pyrrolidinyl)methyl ester
gacgcctttcttacgttcttt

SEQ ID NO: 306 - RNA, 21 nt, synthetic construct
  source 1..21: mol_type = other RNA
  modified_base 1: mod_base = OTHER; note = 2'-O-methyladenosine-3'-phosphorothioate
  modified_base 2: mod_base = OTHER; note = 2'-O-methylcytidine-3'-phosphorothioate
  modified_base 3: mod_base = OTHER; note = 2'-O-methylcytidine-3'-phosphate
  modified_base 4: mod_base = OTHER; note = 2'-O-methyladenosine-3'-phosphate
  modified_base 5: mod_base = OTHER; note = 2'-O-methyladenosine-3'-phosphate
  modified_base 6: mod_base = OTHER; note = 2'-O-methyluridine-3'-phosphate
  modified_base 7: mod_base = OTHER; note = 2'-deoxy-2'-fluoroguanosine-3'-phosphate
  modified_base 8: mod_base = OTHER; note = 2'-O-methyluridine-3'-phosphate
  modified_base 9: mod_base = OTHER; note = 2'-deoxy-2'-fluoroguanosine-3'-phosphate
  modified_base 10: mod_base = OTHER; note = 2'-deoxy-2'-fluoroadenosine-3'-phosphate
  modified_base 11: mod_base = OTHER; note = 2'-deoxy-2'-fluorocytidine-3'-phosphate
  modified_base 12: mod_base = OTHER; note = 2'-O-methyluridine-3'-phosphate
  modified_base 13: mod_base = OTHER; note = 2'-O-methylguanosine-3'-phosphate
  modified_base 14: mod_base = OTHER; note = 2'-O-methyladenosine-3'-phosphate
  modified_base 15: mod_base = OTHER; note = 2'-O-methyladenosine-3'-phosphate
  modified_base 16: mod_base = OTHER; note = 2'-O-methyladenosine-3'-phosphate
  modified_base 17: mod_base = OTHER; note = 2'-O-methyladenosine-3'-phosphate
  modified_base 18: mod_base = OTHER; note = 2'-O-methyluridine-3'-phosphate
  modified_base 19: mod_base = OTHER; note = 2'-O-methylguanosine-3'-phosphate
  modified_base 20: mod_base = OTHER; note = 2'-O-methyluridine-3'-phosphate
  modified_base 21: mod_base = OTHER; note = 2'-O-methyluridine-3'-phosphate ((2S,4R)-1-[29-[[2-(acetylamino)-2-deoxy-beta-D-galactopyranosyl]oxy]-14,14-bis[[3-[[3-[[5-[[2-(acetylamino)-2-deoxy-beta-D-galactopyranosyl]oxy]-1-oxopentyl]amino]propyl]amino]-3-oxopropoxy]methyl]-1,12,19,25-tetraoxo-16-oxa-13,20,24-triazanonacos-1-yl]-4-hydroxy-2-pyrrolidinyl)methyl ester
accaatgtgactgaaaatgtt

SEQ ID NO: 307 - RNA, 21 nt, synthetic construct
  source 1..21: mol_type = other RNA
  modified_base 1: mod_base = OTHER; note = 2'-O-methyladenosine-3'-phosphorothioate
  modified_base 2: mod_base = OTHER; note = 2'-O-methyladenosine-3'-phosphorothioate
  modified_base 3: mod_base = OTHER; note = 2'-O-methylguanosine-3'-phosphate
  modified_base 4: mod_base = OTHER; note = 2'-O-methylcytidine-3'-phosphate
  modified_base 5: mod_base = OTHER; note = 2'-O-methylcytidine-3'-phosphate
  modified_base 6: mod_base = OTHER; note = 2'-O-methylguanosine-3'-phosphate
  modified_base 7: mod_base = OTHER; note = 2'-deoxy-2'-fluorouridine-3'-phosphate
  modified_base 8: mod_base = OTHER; note = 2'-O-methyluridine-3'-phosphate
  modified_base 9: mod_base = OTHER; note = 2'-deoxy-2'-fluoroadenosine-3'-phosphate
  modified_base 10: mod_base = OTHER; note = 2'-deoxy-2'-fluoroadenosine-3'-phosphate
  modified_base 11: mod_base = OTHER; note = 2'-deoxy-2'-fluorocytidine-3'-phosphate
  modified_base 12: mod_base = OTHER; note = 2'-O-methyladenosine-3'-phosphate
  modified_base 13: mod_base = OTHER; note = 2'-O-methyladenosine-3'-phosphate
  modified_base 14: mod_base = OTHER; note = 2'-O-methyladenosine-3'-phosphate
  modified_base 15: mod_base = OTHER; note = 2'-O-methylguanosine-3'-phosphate
  modified_base 16: mod_base = OTHER; note = 2'-O-methyluridine-3'-phosphate
  modified_base 17: mod_base = OTHER; note = 2'-O-methylguanosine-3'-phosphate
  modified_base 18: mod_base = OTHER; note = 2'-O-methyladenosine-3'-phosphate
  modified_base 19: mod_base = OTHER; note = 2'-O-methyladenosine-3'-phosphate
  modified_base 20: mod_base = OTHER; note = 2'-O-methyladenosine-3'-phosphate
  modified_base 21: mod_base = OTHER; note = 2'-O-methyluridine-3'-phosphate ((2S,4R)-1-[29-[[2-(acetylamino)-2-deoxy-beta-D-galactopyranosyl]oxy]-14,14-bis[[3-[[3-[[5-[[2-(acetylamino)-2-deoxy-beta-D-galactopyranosyl]oxy]-1-oxopentyl]amino]propyl]amino]-3-oxopropoxy]methyl]-1,12,19,25-tetraoxo-16-oxa-13,20,24-triazanonacos-1-yl]-4-hydroxy-2-pyrrolidinyl)methyl ester
aagccgttaacaaagtgaaat

SEQ ID NO: 308 - RNA, 21 nt, synthetic construct
  source 1..21: mol_type = other RNA
  modified_base 1: mod_base = OTHER; note = 2'-O-methyladenosine-3'-phosphorothioate
  modified_base 2: mod_base = OTHER; note = 2'-O-methyladenosine-3'-phosphorothioate
  modified_base 3: mod_base = OTHER; note = 2'-O-methyladenosine-3'-phosphate
  modified_base 4: mod_base = OTHER; note = 2'-O-methyladenosine-3'-phosphate
  modified_base 5: mod_base = OTHER; note = 2'-O-methylguanosine-3'-phosphate
  modified_base 6: mod_base = OTHER; note = 2'-O-methylguanosine-3'-phosphate
  modified_base 7: mod_base = OTHER; note = 2'-deoxy-2'-fluoroadenosine-3'-phosphate
  modified_base 8: mod_base = OTHER; note = 2'-O-methyluridine-3'-phosphate
  modified_base 9: mod_base = OTHER; note = 2'-deoxy-2'-fluorouridine-3'-phosphate
  modified_base 10: mod_base = OTHER; note = 2'-deoxy-2'-fluorocytidine-3'-phosphate
  modified_base 11: mod_base = OTHER; note = 2'-deoxy-2'-fluorouridine-3'-phosphate
  modified_base 12: mod_base = OTHER; note = 2'-O-methyluridine-3'-phosphate
  modified_base 13: mod_base = OTHER; note = 2'-O-methylcytidine-3'-phosphate
  modified_base 14: mod_base = OTHER; note = 2'-O-methyladenosine-3'-phosphate
  modified_base 15: mod_base = OTHER; note = 2'-O-methyladenosine-3'-phosphate
  modified_base 16: mod_base = OTHER; note = 2'-O-methylguanosine-3'-phosphate
  modified_base 17: mod_base = OTHER; note = 2'-O-methyladenosine-3'-phosphate
  modified_base 18: mod_base = OTHER; note = 2'-O-methyladenosine-3'-phosphate
  modified_base 19: mod_base = OTHER; note = 2'-O-methyladenosine-3'-phosphate
  modified_base 20: mod_base = OTHER; note = 2'-O-methyluridine-3'-phosphate
  modified_base 21: mod_base = OTHER; note = 2'-O-methyluridine-3'-phosphate ((2S,4R)-1-[29-[[2-(acetylamino)-2-deoxy-beta-D-galactopyranosyl]oxy]-14,14-bis[[3-[[3-[[5-[[2-(acetylamino)-2-deoxy-beta-D-galactopyranosyl]oxy]-1-oxopentyl]amino]propyl]amino]-3-oxopropoxy]methyl]-1,12,19,25-tetraoxo-16-oxa-13,20,24-triazanonacos-1-yl]-4-hydroxy-2-pyrrolidinyl)methyl ester
aaaaggattcttcaagaaatt

SEQ ID NO: 309 - RNA, 21 nt, synthetic construct
  source 1..21: mol_type = other RNA
  modified_base 1: mod_base = OTHER; note = 2'-O-methyluridine-3'-phosphorothioate
  modified_base 2: mod_base = OTHER; note = 2'-O-methylcytidine-3'-phosphorothioate
  modified_base 3: mod_base = OTHER; note = 2'-O-methyluridine-3'-phosphate
  modified_base 4: mod_base = OTHER; note = 2'-O-methyluridine-3'-phosphate
  modified_base 5: mod_base = OTHER; note = 2'-O-methyluridine-3'-phosphate
  modified_base 6: mod_base = OTHER; note = 2'-O-methyluridine-3'-phosphate
  modified_base 7: mod_base = OTHER; note = 2'-deoxy-2'-fluoroguanosine-3'-phosphate
  modified_base 8: mod_base = OTHER; note = 2'-O-methylguanosine-3'-phosphate
  modified_base 9: mod_base = OTHER; note = 2'-deoxy-2'-fluoroadenosine-3'-phosphate
  modified_base 10: mod_base = OTHER; note = 2'-deoxy-2'-fluoroadenosine-3'-phosphate
  modified_base 11: mod_base = OTHER; note = 2'-deoxy-2'-fluorocytidine-3'-phosphate
  modified_base 12: mod_base = OTHER; note = 2'-O-methyladenosine-3'-phosphate
  modified_base 13: mod_base = OTHER; note = 2'-O-methyluridine-3'-phosphate
  modified_base 14: mod_base = OTHER; note = 2'-O-methyluridine-3'-phosphate
  modified_base 15: mod_base = OTHER; note = 2'-O-methylcytidine-3'-phosphate
  modified_base 16: mod_base = OTHER; note = 2'-O-methyladenosine-3'-phosphate
  modified_base 17: mod_base = OTHER; note = 2'-O-methyladenosine-3'-phosphate
  modified_base 18: mod_base = OTHER; note = 2'-O-methyladenosine-3'-phosphate
  modified_base 19: mod_base = OTHER; note = 2'-O-methyluridine-3'-phosphate
  modified_base 20: mod_base = OTHER; note = 2'-O-methyluridine-3'-phosphate
  modified_base 21: mod_base = OTHER; note = 2'-O-methyluridine-3'-phosphate ((2S,4R)-1-[29-[[2-(acetylamino)-2-deoxy-beta-D-galactopyranosyl]oxy]-14,14-bis[[3-[[3-[[5-[[2-(acetylamino)-2-deoxy-beta-D-galactopyranosyl]oxy]-1-oxopentyl]amino]propyl]amino]-3-oxopropoxy]methyl]-1,12,19,25-tetraoxo-16-oxa-13,20,24-triazanonacos-1-yl]-4-hydroxy-2-pyrrolidinyl)methyl ester
tcttttggaacattcaaattt

SEQ ID NO: 310 - RNA, 21 nt, synthetic construct
  source 1..21: mol_type = other RNA
  modified_base 1: mod_base = OTHER; note = 2'-O-methyladenosine-3'-phosphorothioate
  modified_base 2: mod_base = OTHER; note = 2'-O-methyladenosine-3'-phosphorothioate
  modified_base 3: mod_base = OTHER; note = 2'-O-methyladenosine-3'-phosphate
  modified_base 4: mod_base = OTHER; note = 2'-O-methyluridine-3'-phosphate
  modified_base 5: mod_base = OTHER; note = 2'-O-methyluridine-3'-phosphate
  modified_base 6: mod_base = OTHER; note = 2'-O-methylcytidine-3'-phosphate
  modified_base 7: mod_base = OTHER; note = 2'-deoxy-2'-fluoroadenosine-3'-phosphate
  modified_base 8: mod_base = OTHER; note = 2'-O-methylcytidine-3'-phosphate
  modified_base 9: mod_base = OTHER; note = 2'-deoxy-2'-fluoroadenosine-3'-phosphate
  modified_base 10: mod_base = OTHER; note = 2'-deoxy-2'-fluoroadenosine-3'-phosphate
  modified_base 11: mod_base = OTHER; note = 2'-deoxy-2'-fluoroadenosine-3'-phosphate
  modified_base 12: mod_base = OTHER; note = 2'-O-methylguanosine-3'-phosphate
  modified_base 13: mod_base = OTHER; note = 2'-O-methylguanosine-3'-phosphate
  modified_base 14: mod_base = OTHER; note = 2'-O-methyluridine-3'-phosphate
  modified_base 15: mod_base = OTHER; note = 2'-O-methylcytidine-3'-phosphate
  modified_base 16: mod_base = OTHER; note = 2'-O-methyladenosine-3'-phosphate
  modified_base 17: mod_base = OTHER; note = 2'-O-methyladenosine-3'-phosphate
  modified_base 18: mod_base = OTHER; note = 2'-O-methylcytidine-3'-phosphate
  modified_base 19: mod_base = OTHER; note = 2'-O-methyluridine-3'-phosphate
  modified_base 20: mod_base = OTHER; note = 2'-O-methyluridine-3'-phosphate
  modified_base 21: mod_base = OTHER; note = 2'-O-methyluridine-3'-phosphate ((2S,4R)-1-[29-[[2-(acetylamino)-2-deoxy-beta-D-galactopyranosyl]oxy]-14,14-bis[[3-[[3-[[5-[[2-(acetylamino)-2-deoxy-beta-D-galactopyranosyl]oxy]-1-oxopentyl]amino]propyl]amino]-3-oxopropoxy]methyl]-1,12,19,25-tetraoxo-16-oxa-13,20,24-triazanonacos-1-yl]-4-hydroxy-2-pyrrolidinyl)methyl ester
aaattcacaaaggtcaacttt

SEQ ID NO: 311 - RNA, 21 nt, synthetic construct
  source 1..21: mol_type = other RNA
  modified_base 1: mod_base = OTHER; note = 2'-O-methyluridine-3'-phosphorothioate
  modified_base 2: mod_base = OTHER; note = 2'-O-methyluridine-3'-phosphorothioate
  modified_base 3: mod_base = OTHER; note = 2'-O-methyluridine-3'-phosphate
  modified_base 4: mod_base = OTHER; note = 2'-O-methylcytidine-3'-phosphate
  modified_base 5: mod_base = OTHER; note = 2'-O-methyluridine-3'-phosphate
  modified_base 6: mod_base = OTHER; note = 2'-O-methyladenosine-3'-phosphate
  modified_base 7: mod_base = OTHER; note = 2'-deoxy-2'-fluorocytidine-3'-phosphate
  modified_base 8: mod_base = OTHER; note = 2'-O-methylcytidine-3'-phosphate
  modified_base 9: mod_base = OTHER; note = 2'-deoxy-2'-fluoroadenosine-3'-phosphate
  modified_base 10: mod_base = OTHER; note = 2'-deoxy-2'-fluoroguanosine-3'-phosphate
  modified_base 11: mod_base = OTHER; note = 2'-deoxy-2'-fluorouridine-3'-phosphate
  modified_base 12: mod_base = OTHER; note = 2'-O-methyluridine-3'-phosphate
  modified_base 13: mod_base = OTHER; note = 2'-O-methylcytidine-3'-phosphate
  modified_base 14: mod_base = OTHER; note = 2'-O-methyladenosine-3'-phosphate
  modified_base 15: mod_base = OTHER; note = 2'-O-methyluridine-3'-phosphate
  modified_base 16: mod_base = OTHER; note = 2'-O-methyladenosine-3'-phosphate
  modified_base 17: mod_base = OTHER; note = 2'-O-methylguanosine-3'-phosphate
  modified_base 18: mod_base = OTHER; note = 2'-O-methyladenosine-3'-phosphate
  modified_base 19: mod_base = OTHER; note = 2'-O-methyluridine-3'-phosphate
  modified_base 20: mod_base = OTHER; note = 2'-O-methylcytidine-3'-phosphate
  modified_base 21: mod_base = OTHER; note = 2'-O-methyluridine-3'-phosphate ((2S,4R)-1-[29-[[2-(acetylamino)-2-deoxy-beta-D-galactopyranosyl]oxy]-14,14-bis[[3-[[3-[[5-[[2-(acetylamino)-2-deoxy-beta-D-galactopyranosyl]oxy]-1-oxopentyl]amino]propyl]amino]-3-oxopropoxy]methyl]-1,12,19,25-tetraoxo-16-oxa-13,20,24-triazanonacos-1-yl]-4-hydroxy-2-pyrrolidinyl)methyl ester
tttctaccagttcatagatct

SEQ ID NO: 312 - RNA, 21 nt, synthetic construct
  source 1..21: mol_type = other RNA
  modified_base 1: mod_base = OTHER; note = 2'-O-methyladenosine-3'-phosphorothioate
  modified_base 2: mod_base = OTHER; note = 2'-O-methylguanosine-3'-phosphorothioate
  modified_base 3: mod_base = OTHER; note = 2'-O-methyladenosine-3'-phosphate
  modified_base 4: mod_base = OTHER; note = 2'-O-methyluridine-3'-phosphate
  modified_base 5: mod_base = OTHER; note = 2'-O-methylcytidine-3'-phosphate
  modified_base 6: mod_base = OTHER; note = 2'-O-methylcytidine-3'-phosphate
  modified_base 7: mod_base = OTHER; note = 2'-deoxy-2'-fluorocytidine-3'-phosphate
  modified_base 8: mod_base = OTHER; note = 2'-O-methyladenosine-3'-phosphate
  modified_base 9: mod_base = OTHER; note = 2'-deoxy-2'-fluorouridine-3'-phosphate
  modified_base 10: mod_base = OTHER; note = 2'-deoxy-2'-fluoroadenosine-3'-phosphate
  modified_base 11: mod_base = OTHER; note = 2'-deoxy-2'-fluorouridine-3'-phosphate
  modified_base 12: mod_base = OTHER; note = 2'-O-methyluridine-3'-phosphate
  modified_base 13: mod_base = OTHER; note = 2'-O-methylguanosine-3'-phosphate
  modified_base 14: mod_base = OTHER; note = 2'-O-methyladenosine-3'-phosphate
  modified_base 15: mod_base = OTHER; note = 2'-O-methylcytidine-3'-phosphate
  modified_base 16: mod_base = OTHER; note = 2'-O-methyluridine-3'-phosphate
  modified_base 17: mod_base = OTHER; note = 2'-O-methyladenosine-3'-phosphate
  modified_base 18: mod_base = OTHER; note = 2'-O-methyluridine-3'-phosphate
  modified_base 19: mod_base = OTHER; note = 2'-O-methylcytidine-3'-phosphate
  modified_base 20: mod_base = OTHER; note = 2'-O-methyluridine-3'-phosphate
  modified_base 21: mod_base = OTHER; note = 2'-O-methyluridine-3'-phosphate ((2S,4R)-1-[29-[[2-(acetylamino)-2-deoxy-beta-D-galactopyranosyl]oxy]-14,14-bis[[3-[[3-[[5-[[2-(acetylamino)-2-deoxy-beta-D-galactopyranosyl]oxy]-1-oxopentyl]amino]propyl]amino]-3-oxopropoxy]methyl]-1,12,19,25-tetraoxo-16-oxa-13,20,24-triazanonacos-1-yl]-4-hydroxy-2-pyrrolidinyl)methyl ester
agatcccatattgactatctt

SEQ ID NO: 313 - RNA, 21 nt, synthetic construct
  source 1..21: mol_type = other RNA
  modified_base 1: mod_base = OTHER; note = 2'-O-methylguanosine-3'-phosphorothioate
  modified_base 2: mod_base = OTHER; note = 2'-O-methylcytidine-3'-phosphorothioate
  modified_base 3: mod_base = OTHER; note = 2'-O-methyluridine-3'-phosphate
  modified_base 4: mod_base = OTHER; note = 2'-O-methylcytidine-3'-phosphate
  modified_base 5: mod_base = OTHER; note = 2'-O-methyladenosine-3'-phosphate
  modified_base 6: mod_base = OTHER; note = 2'-O-methylcytidine-3'-phosphate
  modified_base 7: mod_base = OTHER; note = 2'-deoxy-2'-fluorouridine-3'-phosphate
  modified_base 8: mod_base = OTHER; note = 2'-O-methyluridine-3'-phosphate
  modified_base 9: mod_base = OTHER; note = 2'-deoxy-2'-fluorouridine-3'-phosphate
  modified_base 10: mod_base = OTHER; note = 2'-deoxy-2'-fluorocytidine-3'-phosphate
  modified_base 11: mod_base = OTHER; note = 2'-deoxy-2'-fluoroadenosine-3'-phosphate
  modified_base 12: mod_base = OTHER; note = 2'-O-methyluridine-3'-phosphate
  modified_base 13: mod_base = OTHER; note = 2'-O-methyluridine-3'-phosphate
  modified_base 14: mod_base = OTHER; note = 2'-O-methylcytidine-3'-phosphate
  modified_base 15: mod_base = OTHER; note = 2'-O-methyluridine-3'-phosphate
  modified_base 16: mod_base = OTHER; note = 2'-O-methylcytidine-3'-phosphate
  modified_base 17: mod_base = OTHER; note = 2'-O-methyluridine-3'-phosphate
  modified_base 18: mod_base = OTHER; note = 2'-O-methyluridine-3'-phosphate
  modified_base 19: mod_base = OTHER; note = 2'-O-methylcytidine-3'-phosphate
  modified_base 20: mod_base = OTHER; note = 2'-O-methyluridine-3'-phosphate
  modified_base 21: mod_base = OTHER; note = 2'-O-methyluridine-3'-phosphate ((2S,4R)-1-[29-[[2-(acetylamino)-2-deoxy-beta-D-galactopyranosyl]oxy]-14,14-bis[[3-[[3-[[5-[[2-(acetylamino)-2-deoxy-beta-D-galactopyranosyl]oxy]-1-oxopentyl]amino]propyl]amino]-3-oxopropoxy]methyl]-1,12,19,25-tetraoxo-16-oxa-13,20,24-triazanonacos-1-yl]-4-hydroxy-2-pyrrolidinyl)methyl ester
gctcactttcattctcttctt

SEQ ID NO: 314 - RNA, 21 nt, synthetic construct
  source 1..21: mol_type = other RNA
  modified_base 1: mod_base = OTHER; note = 2'-O-methyluridine-3'-phosphorothioate
  modified_base 2: mod_base = OTHER; note = 2'-O-methylcytidine-3'-phosphorothioate
  modified_base 3: mod_base = OTHER; note = 2'-O-methyladenosine-3'-phosphate
  modified_base 4: mod_base = OTHER; note = 2'-O-methylguanosine-3'-phosphate
  modified_base 5: mod_base = OTHER; note = 2'-O-methylguanosine-3'-phosphate
  modified_base 6: mod_base = OTHER; note = 2'-O-methylcytidine-3'-phosphate
  modified_base 7: mod_base = OTHER; note = 2'-deoxy-2'-fluoroadenosine-3'-phosphate
  modified_base 8: mod_base = OTHER; note = 2'-O-methyladenosine-3'-phosphate
  modified_base 9: mod_base = OTHER; note = 2'-deoxy-2'-fluorouridine-3'-phosphate
  modified_base 10: mod_base = OTHER; note = 2'-deoxy-2'-fluoroadenosine-3'-phosphate
  modified_base 11: mod_base = OTHER; note = 2'-deoxy-2'-fluoroadenosine-3'-phosphate
  modified_base 12: mod_base = OTHER; note = 2'-O-methyluridine-3'-phosphate
  modified_base 13: mod_base = OTHER; note = 2'-O-methylcytidine-3'-phosphate
  modified_base 14: mod_base = OTHER; note = 2'-O-methyluridine-3'-phosphate
  modified_base 15: mod_base = OTHER; note = 2'-O-methylcytidine-3'-phosphate
  modified_base 16: mod_base = OTHER; note = 2'-O-methyladenosine-3'-phosphate
  modified_base 17: mod_base = OTHER; note = 2'-O-methyladenosine-3'-phosphate
  modified_base 18: mod_base = OTHER; note = 2'-O-methylcytidine-3'-phosphate
  modified_base 19: mod_base = OTHER; note = 2'-O-methyladenosine-3'-phosphate
  modified_base 20: mod_base = OTHER; note = 2'-O-methyluridine-3'-phosphate
  modified_base 21: mod_base = OTHER; note = 2'-O-methyluridine-3'-phosphate ((2S,4R)-1-[29-[[2-(acetylamino)-2-deoxy-beta-D-galactopyranosyl]oxy]-14,14-bis[[3-[[3-[[5-[[2-(acetylamino)-2-deoxy-beta-D-galactopyranosyl]oxy]-1-oxopentyl]amino]propyl]amino]-3-oxopropoxy]methyl]-1,12,19,25-tetraoxo-16-oxa-13,20,24-triazanonacos-1-yl]-4-hydroxy-2-pyrrolidinyl)methyl ester
tcaggcaataatctcaacatt

SEQ ID NO: 315 - RNA, 21 nt, synthetic construct
  source 1..21: mol_type = other RNA
  modified_base 1: mod_base = OTHER; note = 2'-O-methylcytidine-3'-phosphorothioate
  modified_base 2: mod_base = OTHER; note = 2'-O-methyluridine-3'-phosphorothioate
  modified_base 3: mod_base = OTHER; note = 2'-O-methyluridine-3'-phosphate
  modified_base 4: mod_base = OTHER; note = 2'-O-methylcytidine-3'-phosphate
  modified_base 5: mod_base = OTHER; note = 2'-O-methyladenosine-3'-phosphate
  modified_base 6: mod_base = OTHER; note = 2'-O-methylguanosine-3'-phosphate
  modified_base 7: mod_base = OTHER; note = 2'-deoxy-2'-fluorouridine-3'-phosphate
  modified_base 8: mod_base = OTHER; note = 2'-O-methyladenosine-3'-phosphate
  modified_base 9: mod_base = OTHER; note = 2'-deoxy-2'-fluorocytidine-3'-phosphate
  modified_base 10: mod_base = OTHER; note = 2'-deoxy-2'-fluorocytidine-3'-phosphate
  modified_base 11: mod_base = OTHER; note = 2'-deoxy-2'-fluorouridine-3'-phosphate
  modified_base 12: mod_base = OTHER; note = 2'-O-methyluridine-3'-phosphate
  modified_base 13: mod_base = OTHER; note = 2'-O-methylguanosine-3'-phosphate
  modified_base 14: mod_base = OTHER; note = 2'-O-methyladenosine-3'-phosphate
  modified_base 15: mod_base = OTHER; note = 2'-O-methyluridine-3'-phosphate
  modified_base 16: mod_base = OTHER; note = 2'-O-methylcytidine-3'-phosphate
  modified_base 17: mod_base = OTHER; note = 2'-O-methylcytidine-3'-phosphate
  modified_base 18: mod_base = OTHER; note = 2'-O-methyladenosine-3'-phosphate
  modified_base 19: mod_base = OTHER; note = 2'-O-methyluridine-3'-phosphate
  modified_base 20: mod_base = OTHER; note = 2'-O-methyladenosine-3'-phosphate
  modified_base 21: mod_base = OTHER; note = 2'-O-methyluridine-3'-phosphate ((2S,4R)-1-[29-[[2-(acetylamino)-2-deoxy-beta-D-galactopyranosyl]oxy]-14,14-bis[[3-[[3-[[5-[[2-(acetylamino)-2-deoxy-beta-D-galactopyranosyl]oxy]-1-oxopentyl]amino]propyl]amino]-3-oxopropoxy]methyl]-1,12,19,25-tetraoxo-16-oxa-13,20,24-triazanonacos-1-yl]-4-hydroxy-2-pyrrolidinyl)methyl ester
cttcagtaccttgatccatat

SEQ ID NO: 316 - RNA, 21 nt, synthetic construct
  source 1..21: mol_type = other RNA
  modified_base 1: mod_base = OTHER; note = 2'-O-methylguanosine-3'-phosphorothioate
  modified_base 2: mod_base = OTHER; note = 2'-O-methyladenosine-3'-phosphorothioate
  modified_base 3: mod_base = OTHER; note = 2'-O-methyluridine-3'-phosphate
  modified_base 4: mod_base = OTHER; note = 2'-O-methylguanosine-3'-phosphate
  modified_base 5: mod_base = OTHER; note = 2'-O-methyluridine-3'-phosphate
  modified_base 6: mod_base = OTHER; note = 2'-O-methyluridine-3'-phosphate
  modified_base 7: mod_base = OTHER; note = 2'-deoxy-2'-fluorocytidine-3'-phosphate
  modified_base 8: mod_base = OTHER; note = 2'-O-methyluridine-3'-phosphate
  modified_base 9: mod_base = OTHER; note = 2'-deoxy-2'-fluorocytidine-3'-phosphate
  modified_base 10: mod_base = OTHER; note = 2'-deoxy-2'-fluorouridine-3'-phosphate
  modified_base 11: mod_base = OTHER; note = 2'-deoxy-2'-fluoroadenosine-3'-phosphate
  modified_base 12: mod_base = OTHER; note = 2'-O-methyluridine-3'-phosphate
  modified_base 13: mod_base = OTHER; note = 2'-O-methyladenosine-3'-phosphate
  modified_base 14: mod_base = OTHER; note = 2'-O-methylguanosine-3'-phosphate
  modified_base 15: mod_base = OTHER; note = 2'-O-methyladenosine-3'-phosphate
  modified_base 16: mod_base = OTHER; note = 2'-O-methylguanosine-3'-phosphate
  modified_base 17: mod_base = OTHER; note = 2'-O-methylcytidine-3'-phosphate
  modified_base 18: mod_base = OTHER; note = 2'-O-methyluridine-3'-phosphate
  modified_base 19: mod_base = OTHER; note = 2'-O-methyluridine-3'-phosphate
  modified_base 20: mod_base = OTHER; note = 2'-O-methyluridine-3'-phosphate
  modified_base 21: mod_base = OTHER; note = 2'-O-methyluridine-3'-phosphate ((2S,4R)-1-[29-[[2-(acetylamino)-2-deoxy-beta-D-galactopyranosyl]oxy]-14,14-bis[[3-[[3-[[5-[[2-(acetylamino)-2-deoxy-beta-D-galactopyranosyl]oxy]-1-oxopentyl]amino]propyl]amino]-3-oxopropoxy]methyl]-1,12,19,25-tetraoxo-16-oxa-13,20,24-triazanonacos-1-yl]-4-hydroxy-2-pyrrolidinyl)methyl ester
gatgttctctatagagctttt

SEQ ID NO: 317 - RNA, 21 nt, synthetic construct
  source 1..21: mol_type = other RNA
  modified_base 1: mod_base = OTHER; note = 2'-O-methylguanosine-3'-phosphorothioate
  modified_base 2: mod_base = OTHER; note = 2'-O-methylguanosine-3'-phosphorothioate
  modified_base 3: mod_base = OTHER; note = 2'-O-methylcytidine-3'-phosphate
  modified_base 4: mod_base = OTHER; note = 2'-O-methyladenosine-3'-phosphate
  modified_base 5: mod_base = OTHER; note = 2'-O-methyluridine-3'-phosphate
  modified_base 6: mod_base = OTHER; note = 2'-O-methyladenosine-3'-phosphate
  modified_base 7: mod_base = OTHER; note = 2'-deoxy-2'-fluorouridine-3'-phosphate
  modified_base 8: mod_base = OTHER; note = 2'-O-methyladenosine-3'-phosphate
  modified_base 9: mod_base = OTHER; note = 2'-deoxy-2'-fluoroguanosine-3'-phosphate
  modified_base 10: mod_base = OTHER; note = 2'-deoxy-2'-fluorouridine-3'-phosphate
  modified_base 11: mod_base = OTHER; note = 2'-deoxy-2'-fluorouridine-3'-phosphate
  modified_base 12: mod_base = OTHER; note = 2'-O-methylguanosine-3'-phosphate
  modified_base 13: mod_base = OTHER; note = 2'-O-methyladenosine-3'-phosphate
  modified_base 14: mod_base = OTHER; note = 2'-O-methyladenosine-3'-phosphate
  modified_base 15: mod_base = OTHER; note = 2'-O-methyluridine-3'-phosphate
  modified_base 16: mod_base = OTHER; note = 2'-O-methyluridine-3'-phosphate
  modified_base 17: mod_base = OTHER; note = 2'-O-methyladenosine-3'-phosphate
  modified_base 18: mod_base = OTHER; note = 2'-O-methylcytidine-3'-phosphate
  modified_base 19: mod_base = OTHER; note = 2'-O-methyluridine-3'-phosphate
  modified_base 20: mod_base = OTHER; note = 2'-O-methyluridine-3'-phosphate
  modified_base 21: mod_base = OTHER; note = 2'-O-methyluridine-3'-phosphate ((2S,4R)-1-[29-[[2-(acetylamino)-2-deoxy-beta-D-galactopyranosyl]oxy]-14,14-bis[[3-[[3-[[5-[[2-(acetylamino)-2-deoxy-beta-D-galactopyranosyl]oxy]-1-oxopentyl]amino]propyl]amino]-3-oxopropoxy]methyl]-1,12,19,25-tetraoxo-16-oxa-13,20,24-triazanonacos-1-yl]-4-hydroxy-2-pyrrolidinyl)methyl ester
ggcatatagttgaattacttt

SEQ ID NO: 318 - RNA, 21 nt, synthetic construct
  source 1..21: mol_type = other RNA
  modified_base 1: mod_base = OTHER; note = 2'-O-methyluridine-3'-phosphorothioate
  modified_base 2: mod_base = OTHER; note = 2'-O-methyladenosine-3'-phosphorothioate
  modified_base 3: mod_base = OTHER; note = 2'-O-methylguanosine-3'-phosphate
  modified_base 4: mod_base = OTHER; note = 2'-O-methyladenosine-3'-phosphate
  modified_base 5: mod_base = OTHER; note = 2'-O-methyluridine-3'-phosphate
  modified_base 6: mod_base = OTHER; note = 2'-O-methyladenosine-3'-phosphate
  modified_base 7: mod_base = OTHER; note = 2'-deoxy-2'-fluorocytidine-3'-phosphate
  modified_base 8: mod_base = OTHER; note = 2'-O-methyluridine-3'-phosphate
  modified_base 9: mod_base = OTHER; note = 2'-deoxy-2'-fluorocytidine-3'-phosphate
  modified_base 10: mod_base = OTHER; note = 2'-deoxy-2'-fluorouridine-3'-phosphate
  modified_base 11: mod_base = OTHER; note = 2'-deoxy-2'-fluoroguanosine-3'-phosphate
  modified_base 12: mod_base = OTHER; note = 2'-O-methyluridine-3'-phosphate
  modified_base 13: mod_base = OTHER; note = 2'-O-methylcytidine-3'-phosphate
  modified_base 14: mod_base = OTHER; note = 2'-O-methyluridine-3'-phosphate
  modified_base 15: mod_base = OTHER; note = 2'-O-methyladenosine-3'-phosphate
  modified_base 16: mod_base = OTHER; note = 2'-O-methylcytidine-3'-phosphate
  modified_base 17: mod_base = OTHER; note = 2'-O-methylcytidine-3'-phosphate
  modified_base 18: mod_base = OTHER; note = 2'-O-methyladenosine-3'-phosphate
  modified_base 19: mod_base = OTHER; note = 2'-O-methyladenosine-3'-phosphate
  modified_base 20: mod_base = OTHER; note = 2'-O-methyluridine-3'-phosphate
  modified_base 21: mod_base = OTHER; note = 2'-O-methyluridine-3'-phosphate ((2S,4R)-1-[29-[[2-(acetylamino)-2-deoxy-beta-D-galactopyranosyl]oxy]-14,14-bis[[3-[[3-[[5-[[2-(acetylamino)-2-deoxy-beta-D-galactopyranosyl]oxy]-1-oxopentyl]amino]propyl]amino]-3-oxopropoxy]methyl]-1,12,19,25-tetraoxo-16-oxa-13,20,24-triazanonacos-1-yl]-4-hydroxy-2-pyrrolidinyl)methyl ester
tagatactctgtctaccaatt

SEQ ID NO: 319 - RNA, 21 nt, synthetic construct
  source 1..21: mol_type = other RNA
  modified_base 1: mod_base = OTHER; note = 2'-O-methylcytidine-3'-phosphorothioate
  modified_base 2: mod_base = OTHER; note = 2'-O-methylcytidine-3'-phosphorothioate
  modified_base 3: mod_base = OTHER; note = 2'-O-methylcytidine-3'-phosphate
  modified_base 4: mod_base = OTHER; note = 2'-O-methyladenosine-3'-phosphate
  modified_base 5: mod_base = OTHER; note = 2'-O-methylguanosine-3'-phosphate
  modified_base 6: mod_base = OTHER; note = 2'-O-methyladenosine-3'-phosphate
  modified_base 7: mod_base = OTHER; note = 2'-deoxy-2'-fluorocytidine-3'-phosphate
  modified_base 8: mod_base = OTHER; note = 2'-O-methyladenosine-3'-phosphate
  modified_base 9: mod_base = OTHER; note = 2'-deoxy-2'-fluorouridine-3'-phosphate
  modified_base 10: mod_base = OTHER; note = 2'-deoxy-2'-fluorocytidine-3'-phosphate
  modified_base 11: mod_base = OTHER; note = 2'-deoxy-2'-fluorouridine-3'-phosphate
  modified_base 12: mod_base = OTHER; note = 2'-O-methyluridine-3'-phosphate
  modified_base 13: mod_base = OTHER; note = 2'-O-methylguanosine-3'-phosphate
  modified_base 14: mod_base = OTHER; note = 2'-O-methyladenosine-3'-phosphate
  modified_base 15: mod_base = OTHER; note = 2'-O-methyluridine-3'-phosphate
  modified_base 16: mod_base = OTHER; note = 2'-O-methyladenosine-3'-phosphate
  modified_base 17: mod_base = OTHER; note = 2'-O-methyladenosine-3'-phosphate
  modified_base 18: mod_base = OTHER; note = 2'-O-methyluridine-3'-phosphate
  modified_base 19: mod_base = OTHER; note = 2'-O-methyladenosine-3'-phosphate
  modified_base 20: mod_base = OTHER; note = 2'-O-methylcytidine-3'-phosphate
  modified_base 21: mod_base = OTHER; note = 2'-O-methyluridine-3'-phosphate ((2S,4R)-1-[29-[[2-(acetylamino)-2-deoxy-beta-D-galactopyranosyl]oxy]-14,14-bis[[3-[[3-[[5-[[2-(acetylamino)-2-deoxy-beta-D-galactopyranosyl]oxy]-1-oxopentyl]amino]propyl]amino]-3-oxopropoxy]methyl]-1,12,19,25-tetraoxo-16-oxa-13,20,24-triazanonacos-1-yl]-4-hydroxy-2-pyrrolidinyl)methyl ester
cccagacatcttgataatact

SEQ ID NO: 320 - RNA, 21 nt, synthetic construct
  source 1..21: mol_type = other RNA
  modified_base 1: mod_base = OTHER; note = 2'-O-methylcytidine-3'-phosphorothioate
  modified_base 2: mod_base = OTHER; note = 2'-O-methyluridine-3'-phosphorothioate
  modified_base 3: mod_base = OTHER; note = 2'-O-methylguanosine-3'-phosphate
  modified_base 4: mod_base = OTHER; note = 2'-O-methyluridine-3'-phosphate
  modified_base 5: mod_base = OTHER; note = 2'-O-methyluridine-3'-phosphate
  modified_base 6: mod_base = OTHER; note = 2'-O-methylguanosine-3'-phosphate
  modified_base 7: mod_base = OTHER; note = 2'-deoxy-2'-fluoroguanosine-3'-phosphate
  modified_base 8: mod_base = OTHER; note = 2'-O-methyladenosine-3'-phosphate
  modified_base 9: mod_base = OTHER; note = 2'-deoxy-2'-fluoroadenosine-3'-phosphate
  modified_base 10: mod_base = OTHER; note = 2'-deoxy-2'-fluorouridine-3'-phosphate
  modified_base 11: mod_base = OTHER; note = 2'-deoxy-2'-fluorocytidine-3'-phosphate
  modified_base 12: mod_base = OTHER; note = 2'-O-methyluridine-3'-phosphate
  modified_base 13: mod_base = OTHER; note = 2'-O-methylcytidine-3'-phosphate
  modified_base 14: mod_base = OTHER; note = 2'-O-methylcytidine-3'-phosphate
  modified_base 15: mod_base = OTHER; note = 2'-O-methyluridine-3'-phosphate
  modified_base 16: mod_base = OTHER; note = 2'-O-methyladenosine-3'-phosphate
  modified_base 17: mod_base = OTHER; note = 2'-O-methyluridine-3'-phosphate
  modified_base 18: mod_base = OTHER; note = 2'-O-methylguanosine-3'-phosphate
  modified_base 19: mod_base = OTHER; note = 2'-O-methyladenosine-3'-phosphate
  modified_base 20: mod_base = OTHER; note = 2'-O-methyluridine-3'-phosphate
  modified_base 21: mod_base = OTHER; note = 2'-O-methyluridine-3'-phosphate ((2S,4R)-1-[29-[[2-(acetylamino)-2-deoxy-beta-D-galactopyranosyl]oxy]-14,14-bis[[3-[[3-[[5-[[2-(acetylamino)-2-deoxy-beta-D-galactopyranosyl]oxy]-1-oxopentyl]amino]propyl]amino]-3-oxopropoxy]methyl]-1,12,19,25-tetraoxo-16-oxa-13,20,24-triazanonacos-1-yl]-4-hydroxy-2-pyrrolidinyl)methyl ester
ctgttggaatctcctatgatt

SEQ ID NO: 321 - RNA, 21 nt, synthetic construct
  source 1..21: mol_type = other RNA
  modified_base 1: mod_base = OTHER; note = 2'-O-methylcytidine-3'-phosphorothioate
  modified_base 2: mod_base = OTHER; note = 2'-O-methyluridine-3'-phosphorothioate
  modified_base 3: mod_base = OTHER; note = 2'-O-methylguanosine-3'-phosphate
  modified_base 4: mod_base = OTHER; note = 2'-O-methylguanosine-3'-phosphate
  modified_base 5: mod_base = OTHER; note = 2'-O-methylguanosine-3'-phosphate
  modified_base 6: mod_base = OTHER; note = 2'-O-methylcytidine-3'-phosphate
  modified_base 7: mod_base = OTHER; note = 2'-deoxy-2'-fluoroadenosine-3'-phosphate
  modified_base 8: mod_base = OTHER; note = 2'-O-methyladenosine-3'-phosphate
  modified_base 9: mod_base = OTHER; note = 2'-deoxy-2'-fluoroadenosine-3'-phosphate
  modified_base 10: mod_base = OTHER; note = 2'-deoxy-2'-fluorocytidine-3'-phosphate
  modified_base 11: mod_base = OTHER; note = 2'-deoxy-2'-fluorocytidine-3'-phosphate
  modified_base 12: mod_base = OTHER; note = 2'-O-methyluridine-3'-phosphate
  modified_base 13: mod_base = OTHER; note = 2'-O-methyladenosine-3'-phosphate
  modified_base 14: mod_base = OTHER; note = 2'-O-methyladenosine-3'-phosphate
  modified_base 15: mod_base = OTHER; note = 2'-O-methylguanosine-3'-phosphate
  modified_base 16: mod_base = OTHER; note = 2'-O-methyladenosine-3'-phosphate
  modified_base 17: mod_base = OTHER; note = 2'-O-methyladenosine-3'-phosphate
  modified_base 18: mod_base = OTHER; note = 2'-O-methylguanosine-3'-phosphate
  modified_base 19: mod_base = OTHER; note = 2'-O-methyladenosine-3'-phosphate
  modified_base 20: mod_base = OTHER; note = 2'-O-methyladenosine-3'-phosphate
  modified_base 21: mod_base = OTHER; note = 2'-O-methyluridine-3'-phosphate ((2S,4R)-1-[29-[[2-(acetylamino)-2-deoxy-beta-D-galactopyranosyl]oxy]-14,14-bis[[3-[[3-[[5-[[2-(acetylamino)-2-deoxy-beta-D-galactopyranosyl]oxy]-1-oxopentyl]amino]propyl]amino]-3-oxopropoxy]methyl]-1,12,19,25-tetraoxo-16-oxa-13,20,24-triazanonacos-1-yl]-4-hydroxy-2-pyrrolidinyl)methyl ester
ctgggcaaacctaagaagaat

SEQ ID NO: 322 - RNA, 21 nt, synthetic construct
  source 1..21: mol_type = other RNA
  modified_base 1: mod_base = OTHER; note = 2'-O-methylguanosine-3'-phosphorothioate
  modified_base 2: mod_base = OTHER; note = 2'-O-methyluridine-3'-phosphorothioate
  modified_base 3: mod_base = OTHER; note = 2'-O-methyluridine-3'-phosphate
  modified_base 4: mod_base = OTHER; note = 2'-O-methyladenosine-3'-phosphate
  modified_base 5: mod_base = OTHER; note = 2'-O-methyluridine-3'-phosphate
  modified_base 6: mod_base = OTHER; note = 2'-O-methyluridine-3'-phosphate
  modified_base 7: mod_base = OTHER; note = 2'-deoxy-2'-fluoroadenosine-3'-phosphate
  modified_base 8: mod_base = OTHER; note = 2'-O-methylguanosine-3'-phosphate
  modified_base 9: mod_base = OTHER; note = 2'-deoxy-2'-fluoroadenosine-3'-phosphate
  modified_base 10: mod_base = OTHER; note = 2'-deoxy-2'-fluoroadenosine-3'-phosphate
  modified_base 11: mod_base = OTHER; note = 2'-deoxy-2'-fluorouridine-3'-phosphate
  modified_base 12: mod_base = OTHER; note = 2'-O-methylguanosine-3'-phosphate
  modified_base 13: mod_base = OTHER; note = 2'-O-methyluridine-3'-phosphate
  modified_base 14: mod_base = OTHER; note = 2'-O-methyluridine-3'-phosphate
  modified_base 15: mod_base = OTHER; note = 2'-O-methyladenosine-3'-phosphate
  modified_base 16: mod_base = OTHER; note = 2'-O-methylcytidine-3'-phosphate
  modified_base 17: mod_base = OTHER; note = 2'-O-methylguanosine-3'-phosphate
  modified_base 18: mod_base = OTHER; note = 2'-O-methyladenosine-3'-phosphate
  modified_base 19: mod_base = OTHER; note = 2'-O-methyladenosine-3'-phosphate
  modified_base 20: mod_base = OTHER; note = 2'-O-methyladenosine-3'-phosphate
  modified_base 21: mod_base = OTHER; note = 2'-O-methyluridine-3'-phosphate ((2S,4R)-1-[29-[[2-(acetylamino)-2-deoxy-beta-D-galactopyranosyl]oxy]-14,14-bis[[3-[[3-[[5-[[2-(acetylamino)-2-deoxy-beta-D-galactopyranosyl]oxy]-1-oxopentyl]amino]propyl]amino]-3-oxopropoxy]methyl]-1,12,19,25-tetraoxo-16-oxa-13,20,24-triazanonacos-1-yl]-4-hydroxy-2-pyrrolidinyl)methyl ester
gttattagaatgttacgaaat

SEQ ID NO: 323 - RNA, 21 nt, synthetic construct
  source 1..21: mol_type = other RNA
  modified_base 1: mod_base = OTHER; note = 2'-O-methyladenosine-3'-phosphorothioate
  modified_base 2: mod_base = OTHER; note = 2'-O-methylguanosine-3'-phosphorothioate
  modified_base 3: mod_base = OTHER; note = 2'-O-methylcytidine-3'-phosphate
  modified_base 4: mod_base = OTHER; note = 2'-O-methylcytidine-3'-phosphate
  modified_base 5: mod_base = OTHER; note = 2'-O-methyladenosine-3'-phosphate
  modified_base 6: mod_base = OTHER; note = 2'-O-methyluridine-3'-phosphate
  modified_base 7: mod_base = OTHER; note = 2'-deoxy-2'-fluorouridine-3'-phosphate
  modified_base 8: mod_base = OTHER; note = 2'-O-methyluridine-3'-phosphate
  modified_base 9: mod_base = OTHER; note = 2'-deoxy-2'-fluorouridine-3'-phosphate
  modified_base 10: mod_base = OTHER; note = 2'-deoxy-2'-fluorocytidine-3'-phosphate
  modified_base 11: mod_base = OTHER; note = 2'-deoxy-2'-fluorocytidine-3'-phosphate
  modified_base 12: mod_base = OTHER; note = 2'-O-methyluridine-3'-phosphate
  modified_base 13: mod_base = OTHER; note = 2'-O-methyluridine-3'-phosphate
  modified_base 14: mod_base = OTHER; note = 2'-O-methyladenosine-3'-phosphate
  modified_base 15: mod_base = OTHER; note = 2'-O-methyladenosine-3'-phosphate
  modified_base 16: mod_base = OTHER; note = 2'-O-methyladenosine-3'-phosphate
  modified_base 17: mod_base = OTHER; note = 2'-O-methylguanosine-3'-phosphate
  modified_base 18: mod_base = OTHER; note = 2'-O-methylguanosine-3'-phosphate
  modified_base 19: mod_base = OTHER; note = 2'-O-methyladenosine-3'-phosphate
  modified_base 20: mod_base = OTHER; note = 2'-O-methyladenosine-3'-phosphate
  modified_base 21: mod_base = OTHER; note = 2'-O-methyluridine-3'-phosphate ((2S,4R)-1-[29-[[2-(acetylamino)-2-deoxy-beta-D-galactopyranosyl]oxy]-14,14-bis[[3-[[3-[[5-[[2-(acetylamino)-2-deoxy-beta-D-galactopyranosyl]oxy]-1-oxopentyl]amino]propyl]amino]-3-oxopropoxy]methyl]-1,12,19,25-tetraoxo-16-oxa-13,20,24-triazanonacos-1-yl]-4-hydroxy-2-pyrrolidinyl)methyl ester
agccattttccttaaaggaat

SEQ ID NO: 324 - RNA, 21 nt, synthetic construct
  source 1..21: mol_type = other RNA
  modified_base 1: mod_base = OTHER; note = 2'-O-methyladenosine-3'-phosphorothioate
  modified_base 2: mod_base = OTHER; note = 2'-O-methyladenosine-3'-phosphorothioate
  modified_base 3: mod_base = OTHER; note = 2'-O-methyluridine-3'-phosphate
  modified_base 4: mod_base = OTHER; note = 2'-O-methyladenosine-3'-phosphate
  modified_base 5: mod_base = OTHER; note = 2'-O-methyluridine-3'-phosphate
  modified_base 6: mod_base = OTHER; note = 2'-O-methyluridine-3'-phosphate
  modified_base 7: mod_base = OTHER; note = 2'-deoxy-2'-fluorouridine-3'-phosphate
  modified_base 8: mod_base = OTHER; note = 2'-O-methyladenosine-3'-phosphate
  modified_base 9: mod_base = OTHER; note = 2'-deoxy-2'-fluoroguanosine-3'-phosphate
  modified_base 10: mod_base = OTHER; note = 2'-deoxy-2'-fluoroadenosine-3'-phosphate
  modified_base 11: mod_base = OTHER; note = 2'-deoxy-2'-fluoroadenosine-3'-phosphate
  modified_base 12: mod_base = OTHER; note = 2'-O-methyladenosine-3'-phosphate
  modified_base 13: mod_base = OTHER; note = 2'-O-methylguanosine-3'-phosphate
  modified_base 14: mod_base = OTHER; note = 2'-O-methylcytidine-3'-phosphate
  modified_base 15: mod_base = OTHER; note = 2'-O-methylcytidine-3'-phosphate
  modified_base 16: mod_base = OTHER; note = 2'-O-methyladenosine-3'-phosphate
  modified_base 17: mod_base = OTHER; note = 2'-O-methyladenosine-3'-phosphate
  modified_base 18: mod_base = OTHER; note = 2'-O-methyladenosine-3'-phosphate
  modified_base 19: mod_base = OTHER; note = 2'-O-methylguanosine-3'-phosphate
  modified_base 20: mod_base = OTHER; note = 2'-O-methyluridine-3'-phosphate
  modified_base 21: mod_base = OTHER; note = 2'-O-methyluridine-3'-phosphate ((2S,4R)-1-[29-[[2-(acetylamino)-2-deoxy-beta-D-galactopyranosyl]oxy]-14,14-bis[[3-[[3-[[5-[[2-(acetylamino)-2-deoxy-beta-D-galactopyranosyl]oxy]-1-oxopentyl]amino]propyl]amino]-3-oxopropoxy]methyl]-1,12,19,25-tetraoxo-16-oxa-13,20,24-triazanonacos-1-yl]-4-hydroxy-2-pyrrolidinyl)methyl ester
aatatttagaaagccaaagtt

SEQ ID NO: 325 - RNA, 21 nt, synthetic construct
  source 1..21: mol_type = other RNA
  modified_base 1: mod_base = OTHER; note = 2'-O-methyladenosine-3'-phosphorothioate
  modified_base 2: mod_base = OTHER; note = 2'-O-methylcytidine-3'-phosphorothioate
  modified_base 3: mod_base = OTHER; note = 2'-O-methylcytidine-3'-phosphate
  modified_base 4: mod_base = OTHER; note = 2'-O-methyladenosine-3'-phosphate
  modified_base 5: mod_base = OTHER; note = 2'-O-methylguanosine-3'-phosphate
  modified_base 6: mod_base = OTHER; note = 2'-O-methylcytidine-3'-phosphate
  modified_base 7: mod_base = OTHER; note = 2'-deoxy-2'-fluorouridine-3'-phosphate
  modified_base 8: mod_base = OTHER; note = 2'-O-methyladenosine-3'-phosphate
  modified_base 9: mod_base = OTHER; note = 2'-deoxy-2'-fluorouridine-3'-phosphate
  modified_base 10: mod_base = OTHER; note = 2'-deoxy-2'-fluoroadenosine-3'-phosphate
  modified_base 11: mod_base = OTHER; note = 2'-deoxy-2'-fluorocytidine-3'-phosphate
  modified_base 12: mod_base = OTHER; note = 2'-O-methyluridine-3'-phosphate
  modified_base 13: mod_base = OTHER; note = 2'-O-methyluridine-3'-phosphate
  modified_base 14: mod_base = OTHER; note = 2'-O-methylcytidine-3'-phosphate
  modified_base 15: mod_base = OTHER; note = 2'-O-methylcytidine-3'-phosphate
  modified_base 16: mod_base = OTHER; note = 2'-O-methyluridine-3'-phosphate
  modified_base 17: mod_base = OTHER; note = 2'-O-methyluridine-3'-phosphate
  modified_base 18: mod_base = OTHER; note = 2'-O-methylcytidine-3'-phosphate
  modified_base 19: mod_base = OTHER; note = 2'-O-methyladenosine-3'-phosphate
  modified_base 20: mod_base = OTHER; note = 2'-O-methyladenosine-3'-phosphate
  modified_base 21: mod_base = OTHER; note = 2'-O-methyluridine-3'-phosphate ((2S,4R)-1-[29-[[2-(acetylamino)-2-deoxy-beta-D-galactopyranosyl]oxy]-14,14-bis[[3-[[3-[[5-[[2-(acetylamino)-2-deoxy-beta-D-galactopyranosyl]oxy]-1-oxopentyl]amino]propyl]amino]-3-oxopropoxy]methyl]-1,12,19,25-tetraoxo-16-oxa-13,20,24-triazanonacos-1-yl]-4-hydroxy-2-pyrrolidinyl)methyl ester
accagctatacttccttcaat

SEQ ID NO: 326 - RNA, 21 nt, synthetic construct
  source 1..21: mol_type = other RNA
  modified_base 1: mod_base = OTHER; note = 2'-O-methyluridine-3'-phosphorothioate
  modified_base 2: mod_base = OTHER; note = 2'-O-methyladenosine-3'-phosphorothioate
  modified_base 3: mod_base = OTHER; note = 2'-O-methyladenosine-3'-phosphate
  modified_base 4: mod_base = OTHER; note = 2'-O-methyluridine-3'-phosphate
  modified_base 5: mod_base = OTHER; note = 2'-O-methylguanosine-3'-phosphate
  modified_base 6: mod_base = OTHER; note = 2'-O-methyladenosine-3'-phosphate
  modified_base 7: mod_base = OTHER; note = 2'-deoxy-2'-fluoroguanosine-3'-phosphate
  modified_base 8: mod_base = OTHER; note = 2'-O-methyluridine-3'-phosphate
  modified_base 9: mod_base = OTHER; note = 2'-deoxy-2'-fluorocytidine-3'-phosphate
  modified_base 10: mod_base = OTHER; note = 2'-deoxy-2'-fluorocytidine-3'-phosphate
  modified_base 11: mod_base = OTHER; note = 2'-deoxy-2'-fluoroadenosine-3'-phosphate
  modified_base 12: mod_base = OTHER; note = 2'-O-methylguanosine-3'-phosphate
  modified_base 13: mod_base = OTHER; note = 2'-O-methyladenosine-3'-phosphate
  modified_base 14: mod_base = OTHER; note = 2'-O-methyladenosine-3'-phosphate
  modified_base 15: mod_base = OTHER; note = 2'-O-methyladenosine-3'-phosphate
  modified_base 16: mod_base = OTHER; note = 2'-O-methyluridine-3'-phosphate
  modified_base 17: mod_base = OTHER; note = 2'-O-methylguanosine-3'-phosphate
  modified_base 18: mod_base = OTHER; note = 2'-O-methylcytidine-3'-phosphate
  modified_base 19: mod_base = OTHER; note = 2'-O-methyladenosine-3'-phosphate
  modified_base 20: mod_base = OTHER; note = 2'-O-methyladenosine-3'-phosphate
  modified_base 21: mod_base = OTHER; note = 2'-O-methyluridine-3'-phosphate ((2S,4R)-1-[29-[[2-(acetylamino)-2-deoxy-beta-D-galactopyranosyl]oxy]-14,14-bis[[3-[[3-[[5-[[2-(acetylamino)-2-deoxy-beta-D-galactopyranosyl]oxy]-1-oxopentyl]amino]propyl]amino]-3-oxopropoxy]methyl]-1,12,19,25-tetraoxo-16-oxa-13,20,24-triazanonacos-1-yl]-4-hydroxy-2-pyrrolidinyl)methyl ester
taatgagtccagaaatgcaat

SEQ ID NO: 327 - RNA, 21 nt, synthetic construct
  source 1..21: mol_type = other RNA
  modified_base 1: mod_base = OTHER; note = 2'-O-methyladenosine-3'-phosphorothioate
  modified_base 2: mod_base = OTHER; note = 2'-O-methylguanosine-3'-phosphorothioate
  modified_base 3: mod_base = OTHER; note = 2'-O-methylguanosine-3'-phosphate
  modified_base 4: mod_base = OTHER; note = 2'-O-methyladenosine-3'-phosphate
  modified_base 5: mod_base = OTHER; note = 2'-O-methylguanosine-3'-phosphate
  modified_base 6: mod_base = OTHER; note = 2'-O-methylguanosine-3'-phosphate
  modified_base 7: mod_base = OTHER; note = 2'-deoxy-2'-fluorouridine-3'-phosphate
  modified_base 8: mod_base = OTHER; note = 2'-O-methyluridine-3'-phosphate
  modified_base 9: mod_base = OTHER; note = 2'-deoxy-2'-fluoroguanosine-3'-phosphate
  modified_base 10: mod_base = OTHER; note = 2'-deoxy-2'-fluoroadenosine-3'-phosphate
  modified_base 11: mod_base = OTHER; note = 2'-deoxy-2'-fluorouridine-3'-phosphate
  modified_base 12: mod_base = OTHER; note = 2'-O-methyluridine-3'-phosphate
  modified_base 13: mod_base = OTHER; note = 2'-O-methylguanosine-3'-phosphate
  modified_base 14: mod_base = OTHER; note = 2'-O-methylcytidine-3'-phosphate
  modified_base 15: mod_base = OTHER; note = 2'-O-methyladenosine-3'-phosphate
  modified_base 16: mod_base = OTHER; note = 2'-O-methyladenosine-3'-phosphate
  modified_base 17: mod_base = OTHER; note = 2'-O-methyladenosine-3'-phosphate
  modified_base 18: mod_base = OTHER; note = 2'-O-methyluridine-3'-phosphate
  modified_base 19: mod_base = OTHER; note = 2'-O-methylcytidine-3'-phosphate
  modified_base 20: mod_base = OTHER; note = 2'-O-methyluridine-3'-phosphate
  modified_base 21: mod_base = OTHER; note = 2'-O-methyluridine-3'-phosphate ((2S,4R)-1-[29-[[2-(acetylamino)-2-deoxy-beta-D-galactopyranosyl]oxy]-14,14-bis[[3-[[3-[[5-[[2-(acetylamino)-2-deoxy-beta-D-galactopyranosyl]oxy]-1-oxopentyl]amino]propyl]amino]-3-oxopropoxy]methyl]-1,12,19,25-tetraoxo-16-oxa-13,20,24-triazanonacos-1-yl]-4-hydroxy-2-pyrrolidinyl)methyl ester
aggaggttgattgcaaatctt

SEQ ID NO: 328 - RNA, 21 nt, synthetic construct
  source 1..21: mol_type = other RNA
  modified_base 1: mod_base = OTHER; note = 2'-O-methylguanosine-3'-phosphorothioate
  modified_base 2: mod_base = OTHER; note = 2'-O-methyladenosine-3'-phosphorothioate
  modified_base 3: mod_base = OTHER; note = 2'-O-methyladenosine-3'-phosphate
  modified_base 4: mod_base = OTHER; note = 2'-O-methylguanosine-3'-phosphate
  modified_base 5: mod_base = OTHER; note = 2'-O-methyladenosine-3'-phosphate
  modified_base 6: mod_base = OTHER; note = 2'-O-methylcytidine-3'-phosphate
  modified_base 7: mod_base = OTHER; note = 2'-deoxy-2'-fluorouridine-3'-phosphate
  modified_base 8: mod_base = OTHER; note = 2'-O-methyluridine-3'-phosphate
  modified_base 9: mod_base = OTHER; note = 2'-deoxy-2'-fluorocytidine-3'-phosphate
  modified_base 10: mod_base = OTHER; note = 2'-deoxy-2'-fluorouridine-3'-phosphate
  modified_base 11: mod_base = OTHER; note = 2'-deoxy-2'-fluorouridine-3'-phosphate
  modified_base 12: mod_base = OTHER; note = 2'-O-methyluridine-3'-phosphate
  modified_base 13: mod_base = OTHER; note = 2'-O-methylguanosine-3'-phosphate
  modified_base 14: mod_base = OTHER; note = 2'-O-methyluridine-3'-phosphate
  modified_base 15: mod_base = OTHER; note = 2'-O-methylguanosine-3'-phosphate
  modified_base 16: mod_base = OTHER; note = 2'-O-methyladenosine-3'-phosphate
  modified_base 17: mod_base = OTHER; note = 2'-O-methyluridine-3'-phosphate
  modified_base 18: mod_base = OTHER; note = 2'-O-methylguanosine-3'-phosphate
  modified_base 19: mod_base = OTHER; note = 2'-O-methyladenosine-3'-phosphate
  modified_base 20: mod_base = OTHER; note = 2'-O-methyladenosine-3'-phosphate
  modified_base 21: mod_base = OTHER; note = 2'-O-methyluridine-3'-phosphate ((2S,4R)-1-[29-[[2-(acetylamino)-2-deoxy-beta-D-galactopyranosyl]oxy]-14,14-bis[[3-[[3-[[5-[[2-(acetylamino)-2-deoxy-beta-D-galactopyranosyl]oxy]-1-oxopentyl]amino]propyl]amino]-3-oxopropoxy]methyl]-1,12,19,25-tetraoxo-16-oxa-13,20,24-triazanonacos-1-yl]-4-hydroxy-2-pyrrolidinyl)methyl ester
gaagacttctttgtgatgaat

SEQ ID NO: 329 - RNA, 21 nt, synthetic construct
  source 1..21: mol_type = other RNA
  modified_base 1: mod_base = OTHER; note = 2'-O-methyladenosine-3'-phosphorothioate
  modified_base 2: mod_base = OTHER; note = 2'-O-methyladenosine-3'-phosphorothioate
  modified_base 3: mod_base = OTHER; note = 2'-O-methyluridine-3'-phosphate
  modified_base 4: mod_base = OTHER; note = 2'-O-methyluridine-3'-phosphate
  modified_base 5: mod_base = OTHER; note = 2'-O-methylcytidine-3'-phosphate
  modified_base 6: mod_base = OTHER; note = 2'-O-methyladenosine-3'-phosphate
  modified_base 7: mod_base = OTHER; note = 2'-deoxy-2'-fluoroguanosine-3'-phosphate
  modified_base 8: mod_base = OTHER; note = 2'-O-methyladenosine-3'-phosphate
  modified_base 9: mod_base = OTHER; note = 2'-deoxy-2'-fluoroadenosine-3'-phosphate
  modified_base 10: mod_base = OTHER; note = 2'-deoxy-2'-fluoroguanosine-3'-phosphate
  modified_base 11: mod_base = OTHER; note = 2'-deoxy-2'-fluoroadenosine-3'-phosphate
  modified_base 12: mod_base = OTHER; note = 2'-O-methyluridine-3'-phosphate
  modified_base 13: mod_base = OTHER; note = 2'-O-methylguanosine-3'-phosphate
  modified_base 14: mod_base = OTHER; note = 2'-O-methyluridine-3'-phosphate
  modified_base 15: mod_base = OTHER; note = 2'-O-methyladenosine-3'-phosphate
  modified_base 16: mod_base = OTHER; note = 2'-O-methylguanosine-3'-phosphate
  modified_base 17: mod_base = OTHER; note = 2'-O-methyluridine-3'-phosphate
  modified_base 18: mod_base = OTHER; note = 2'-O-methyladenosine-3'-phosphate
  modified_base 19: mod_base = OTHER; note = 2'-O-methyladenosine-3'-phosphate
  modified_base 20: mod_base = OTHER; note = 2'-O-methyluridine-3'-phosphate
  modified_base 21: mod_base = OTHER; note = 2'-O-methyluridine-3'-phosphate ((2S,4R)-1-[29-[[2-(acetylamino)-2-deoxy-beta-D-galactopyranosyl]oxy]-14,14-bis[[3-[[3-[[5-[[2-(acetylamino)-2-deoxy-beta-D-galactopyranosyl]oxy]-1-oxopentyl]amino]propyl]amino]-3-oxopropoxy]methyl]-1,12,19,25-tetraoxo-16-oxa-13,20,24-triazanonacos-1-yl]-4-hydroxy-2-pyrrolidinyl)methyl ester
aattcagaagatgtagtaatt

SEQ ID NO: 330 - RNA, 21 nt, synthetic construct
  source 1..21: mol_type = other RNA
  modified_base 1: mod_base = OTHER; note = 2'-O-methyladenosine-3'-phosphorothioate
  modified_base 2: mod_base = OTHER; note = 2'-O-methylguanosine-3'-phosphorothioate
  modified_base 3: mod_base = OTHER; note = 2'-O-methyluridine-3'-phosphate
  modified_base 4: mod_base = OTHER; note = 2'-O-methylcytidine-3'-phosphate
  modified_base 5: mod_base = OTHER; note = 2'-O-methyluridine-3'-phosphate
  modified_base 6: mod_base = OTHER; note = 2'-O-methyluridine-3'-phosphate
  modified_base 7: mod_base = OTHER; note = 2'-deoxy-2'-fluorocytidine-3'-phosphate
  modified_base 8: mod_base = OTHER; note = 2'-O-methylguanosine-3'-phosphate
  modified_base 9: mod_base = OTHER; note = 2'-deoxy-2'-fluoroadenosine-3'-phosphate
  modified_base 10: mod_base = OTHER; note = 2'-deoxy-2'-fluoroadenosine-3'-phosphate
  modified_base 11: mod_base = OTHER; note = 2'-deoxy-2'-fluorocytidine-3'-phosphate
  modified_base 12: mod_base = OTHER; note = 2'-O-methyluridine-3'-phosphate
  modified_base 13: mod_base = OTHER; note = 2'-O-methylcytidine-3'-phosphate
  modified_base 14: mod_base = OTHER; note = 2'-O-methyladenosine-3'-phosphate
  modified_base 15: mod_base = OTHER; note = 2'-O-methyladenosine-3'-phosphate
  modified_base 16: mod_base = OTHER; note = 2'-O-methylcytidine-3'-phosphate
  modified_base 17: mod_base = OTHER; note = 2'-O-methyluridine-3'-phosphate
  modified_base 18: mod_base = OTHER; note = 2'-O-methyluridine-3'-phosphate
  modified_base 19: mod_base = OTHER; note = 2'-O-methylcytidine-3'-phosphate
  modified_base 20: mod_base = OTHER; note = 2'-O-methyluridine-3'-phosphate
  modified_base 21: mod_base = OTHER; note = 2'-O-methyluridine-3'-phosphate ((2S,4R)-1-[29-[[2-(acetylamino)-2-deoxy-beta-D-galactopyranosyl]oxy]-14,14-bis[[3-[[3-[[5-[[2-(acetylamino)-2-deoxy-beta-D-galactopyranosyl]oxy]-1-oxopentyl]amino]propyl]amino]-3-oxopropoxy]methyl]-1,12,19,25-tetraoxo-16-oxa-13,20,24-triazanonacos-1-yl]-4-hydroxy-2-pyrrolidinyl)methyl ester
agtcttcgaactcaacttctt

SEQ ID NO: 331 - RNA, 21 nt, synthetic construct
  source 1..21: mol_type = other RNA
  modified_base 1: mod_base = OTHER; note = 2'-O-methyluridine-3'-phosphorothioate
  modified_base 2: mod_base = OTHER; note = 2'-O-methyladenosine-3'-phosphorothioate
  modified_base 3: mod_base = OTHER; note = 2'-O-methylcytidine-3'-phosphate
  modified_base 4: mod_base = OTHER; note = 2'-O-methyluridine-3'-phosphate
  modified_base 5: mod_base = OTHER; note = 2'-O-methyluridine-3'-phosphate
  modified_base 6: mod_base = OTHER; note = 2'-O-methylcytidine-3'-phosphate
  modified_base 7: mod_base = OTHER; note = 2'-deoxy-2'-fluoroadenosine-3'-phosphate
  modified_base 8: mod_base = OTHER; note = 2'-O-methyluridine-3'-phosphate
  modified_base 9: mod_base = OTHER; note = 2'-deoxy-2'-fluoroguanosine-3'-phosphate
  modified_base 10: mod_base = OTHER; note = 2'-deoxy-2'-fluorouridine-3'-phosphate
  modified_base 11: mod_base = OTHER; note = 2'-deoxy-2'-fluorocytidine-3'-phosphate
  modified_base 12: mod_base = OTHER; note = 2'-O-methyluridine-3'-phosphate
  modified_base 13: mod_base = OTHER; note = 2'-O-methyluridine-3'-phosphate
  modified_base 14: mod_base = OTHER; note = 2'-O-methyluridine-3'-phosphate
  modified_base 15: mod_base = OTHER; note = 2'-O-methyladenosine-3'-phosphate
  modified_base 16: mod_base = OTHER; note = 2'-O-methyluridine-3'-phosphate
  modified_base 17: mod_base = OTHER; note = 2'-O-methylcytidine-3'-phosphate
  modified_base 18: mod_base = OTHER; note = 2'-O-methyladenosine-3'-phosphate
  modified_base 19: mod_base = OTHER; note = 2'-O-methyluridine-3'-phosphate
  modified_base 20: mod_base = OTHER; note = 2'-O-methylguanosine-3'-phosphate
  modified_base 21: mod_base = OTHER; note = 2'-O-methyluridine-3'-phosphate ((2S,4R)-1-[29-[[2-(acetylamino)-2-deoxy-beta-D-galactopyranosyl]oxy]-14,14-bis[[3-[[3-[[5-[[2-(acetylamino)-2-deoxy-beta-D-galactopyranosyl]oxy]-1-oxopentyl]amino]propyl]amino]-3-oxopropoxy]methyl]-1,12,19,25-tetraoxo-16-oxa-13,20,24-triazanonacos-1-yl]-4-hydroxy-2-pyrrolidinyl)methyl ester
tacttcatgtctttatcatgt

SEQ ID NO: 332 - RNA, 21 nt, synthetic construct
  source 1..21: mol_type = other RNA
  modified_base 1: mod_base = OTHER; note = 2'-O-methyluridine-3'-phosphorothioate
  modified_base 2: mod_base = OTHER; note = 2'-O-methyluridine-3'-phosphorothioate
  modified_base 3: mod_base = OTHER; note = 2'-O-methyladenosine-3'-phosphate
  modified_base 4: mod_base = OTHER; note = 2'-O-methyluridine-3'-phosphate
  modified_base 5: mod_base = OTHER; note = 2'-O-methylguanosine-3'-phosphate
  modified_base 6: mod_base = OTHER; note = 2'-O-methylcytidine-3'-phosphate
  modified_base 7: mod_base = OTHER; note = 2'-deoxy-2'-fluoroadenosine-3'-phosphate
  modified_base 8: mod_base = OTHER; note = 2'-O-methylguanosine-3'-phosphate
  modified_base 9: mod_base = OTHER; note = 2'-deoxy-2'-fluorouridine-3'-phosphate
  modified_base 10: mod_base = OTHER; note = 2'-deoxy-2'-fluorouridine-3'-phosphate
  modified_base 11: mod_base = OTHER; note = 2'-deoxy-2'-fluorocytidine-3'-phosphate
  modified_base 12: mod_base = OTHER; note = 2'-O-methyluridine-3'-phosphate
  modified_base 13: mod_base = OTHER; note = 2'-O-methylguanosine-3'-phosphate
  modified_base 14: mod_base = OTHER; note = 2'-O-methyladenosine-3'-phosphate
  modified_base 15: mod_base = OTHER; note = 2'-O-methyladenosine-3'-phosphate
  modified_base 16: mod_base = OTHER; note = 2'-O-methylcytidine-3'-phosphate
  modified_base 17: mod_base = OTHER; note = 2'-O-methyladenosine-3'-phosphate
  modified_base 18: mod_base = OTHER; note = 2'-O-methyladenosine-3'-phosphate
  modified_base 19: mod_base = OTHER; note = 2'-O-methylguanosine-3'-phosphate
  modified_base 20: mod_base = OTHER; note = 2'-O-methyladenosine-3'-phosphate
  modified_base 21: mod_base = OTHER; note = 2'-O-methyluridine-3'-phosphate ((2S,4R)-1-[29-[[2-(acetylamino)-2-deoxy-beta-D-galactopyranosyl]oxy]-14,14-bis[[3-[[3-[[5-[[2-(acetylamino)-2-deoxy-beta-D-galactopyranosyl]oxy]-1-oxopentyl]amino]propyl]amino]-3-oxopropoxy]methyl]-1,12,19,25-tetraoxo-16-oxa-13,20,24-triazanonacos-1-yl]-4-hydroxy-2-pyrrolidinyl)methyl ester
ttatgcagttctgaacaagat

SEQ ID NO: 333 - RNA, 21 nt, synthetic construct
  source 1..21: mol_type = other RNA
  modified_base 1: mod_base = OTHER; note = 2'-O-methylguanosine-3'-phosphorothioate
  modified_base 2: mod_base = OTHER; note = 2'-O-methyladenosine-3'-phosphorothioate
  modified_base 3: mod_base = OTHER; note = 2'-O-methyladenosine-3'-phosphate
  modified_base 4: mod_base = OTHER; note = 2'-O-methyladenosine-3'-phosphate
  modified_base 5: mod_base = OTHER; note = 2'-O-methylcytidine-3'-phosphate
  modified_base 6: mod_base = OTHER; note = 2'-O-methyladenosine-3'-phosphate
  modified_base 7: mod_base = OTHER; note = 2'-deoxy-2'-fluoroguanosine-3'-phosphate
  modified_base 8: mod_base = OTHER; note = 2'-O-methyluridine-3'-phosphate
  modified_base 9: mod_base = OTHER; note = 2'-deoxy-2'-fluoroadenosine-3'-phosphate
  modified_base 10: mod_base = OTHER; note = 2'-deoxy-2'-fluoroguanosine-3'-phosphate
  modified_base 11: mod_base = OTHER; note = 2'-deoxy-2'-fluoroguanosine-3'-phosphate
  modified_base 12: mod_base = OTHER; note = 2'-O-methyladenosine-3'-phosphate
  modified_base 13: mod_base = OTHER; note = 2'-O-methyladenosine-3'-phosphate
  modified_base 14: mod_base = OTHER; note = 2'-O-methyladenosine-3'-phosphate
  modified_base 15: mod_base = OTHER; note = 2'-O-methylguanosine-3'-phosphate
  modified_base 16: mod_base = OTHER; note = 2'-O-methyluridine-3'-phosphate
  modified_base 17: mod_base = OTHER; note = 2'-O-methyluridine-3'-phosphate
  modified_base 18: mod_base = OTHER; note = 2'-O-methyluridine-3'-phosphate
  modified_base 19: mod_base = OTHER; note = 2'-O-methyladenosine-3'-phosphate
  modified_base 20: mod_base = OTHER; note = 2'-O-methyluridine-3'-phosphate
  modified_base 21: mod_base = OTHER; note = 2'-O-methyluridine-3'-phosphate ((2S,4R)-1-[29-[[2-(acetylamino)-2-deoxy-beta-D-galactopyranosyl]oxy]-14,14-bis[[3-[[3-[[5-[[2-(acetylamino)-2-deoxy-beta-D-galactopyranosyl]oxy]-1-oxopentyl]amino]propyl]amino]-3-oxopropoxy]methyl]-1,12,19,25-tetraoxo-16-oxa-13,20,24-triazanonacos-1-yl]-4-hydroxy-2-pyrrolidinyl)methyl ester
gaaacagtaggaaagtttatt

SEQ ID NO: 334 - RNA, 21 nt, synthetic construct
  source 1..21: mol_type = other RNA
  modified_base 1: mod_base = OTHER; note = 2'-O-methyluridine-3'-phosphorothioate
  modified_base 2: mod_base = OTHER; note = 2'-O-methylguanosine-3'-phosphorothioate
  modified_base 3: mod_base = OTHER; note = 2'-O-methylguanosine-3'-phosphate
  modified_base 4: mod_base = OTHER; note = 2'-O-methyladenosine-3'-phosphate
  modified_base 5: mod_base = OTHER; note = 2'-O-methylguanosine-3'-phosphate
  modified_base 6: mod_base = OTHER; note = 2'-O-methyladenosine-3'-phosphate
  modified_base 7: mod_base = OTHER; note = 2'-deoxy-2'-fluoroadenosine-3'-phosphate
  modified_base 8: mod_base = OTHER; note = 2'-O-methylguanosine-3'-phosphate
  modified_base 9: mod_base = OTHER; note = 2'-deoxy-2'-fluorouridine-3'-phosphate
  modified_base 10: mod_base = OTHER; note = 2'-deoxy-2'-fluoroguanosine-3'-phosphate
  modified_base 11: mod_base = OTHER; note = 2'-deoxy-2'-fluoroadenosine-3'-phosphate
  modified_base 12: mod_base = OTHER; note = 2'-O-methyluridine-3'-phosphate
  modified_base 13: mod_base = OTHER; note = 2'-O-methylguanosine-3'-phosphate
  modified_base 14: mod_base = OTHER; note = 2'-O-methyladenosine-3'-phosphate
  modified_base 15: mod_base = OTHER; note = 2'-O-methyladenosine-3'-phosphate
  modified_base 16: mod_base = OTHER; note = 2'-O-methylguanosine-3'-phosphate
  modified_base 17: mod_base = OTHER; note = 2'-O-methyladenosine-3'-phosphate
  modified_base 18: mod_base = OTHER; note = 2'-O-methyladenosine-3'-phosphate
  modified_base 19: mod_base = OTHER; note = 2'-O-methylguanosine-3'-phosphate
  modified_base 20: mod_base = OTHER; note = 2'-O-methyladenosine-3'-phosphate
  modified_base 21: mod_base = OTHER; note = 2'-O-methyluridine-3'-phosphate ((2S,4R)-1-[29-[[2-(acetylamino)-2-deoxy-beta-D-galactopyranosyl]oxy]-14,14-bis[[3-[[3-[[5-[[2-(acetylamino)-2-deoxy-beta-D-galactopyranosyl]oxy]-1-oxopentyl]amino]propyl]amino]-3-oxopropoxy]methyl]-1,12,19,25-tetraoxo-16-oxa-13,20,24-triazanonacos-1-yl]-4-hydroxy-2-pyrrolidinyl)methyl ester
tggagaagtgatgaagaagat

SEQ ID NO: 335 - RNA, 21 nt, synthetic construct
  source 1..21: mol_type = other RNA
  modified_base 1: mod_base = OTHER; note = 2'-O-methylguanosine-3'-phosphorothioate
  modified_base 2: mod_base = OTHER; note = 2'-O-methyluridine-3'-phosphorothioate
  modified_base 3: mod_base = OTHER; note = 2'-O-methyluridine-3'-phosphate
  modified_base 4: mod_base = OTHER; note = 2'-O-methyluridine-3'-phosphate
  modified_base 5: mod_base = OTHER; note = 2'-O-methyladenosine-3'-phosphate
  modified_base 6: mod_base = OTHER; note = 2'-O-methyluridine-3'-phosphate
  modified_base 7: mod_base = OTHER; note = 2'-deoxy-2'-fluorocytidine-3'-phosphate
  modified_base 8: mod_base = OTHER; note = 2'-O-methyladenosine-3'-phosphate
  modified_base 9: mod_base = OTHER; note = 2'-deoxy-2'-fluorocytidine-3'-phosphate
  modified_base 10: mod_base = OTHER; note = 2'-deoxy-2'-fluorocytidine-3'-phosphate
  modified_base 11: mod_base = OTHER; note = 2'-deoxy-2'-fluorouridine-3'-phosphate
  modified_base 12: mod_base = OTHER; note = 2'-O-methyluridine-3'-phosphate
  modified_base 13: mod_base = OTHER; note = 2'-O-methylcytidine-3'-phosphate
  modified_base 14: mod_base = OTHER; note = 2'-O-methyluridine-3'-phosphate
  modified_base 15: mod_base = OTHER; note = 2'-O-methyluridine-3'-phosphate
  modified_base 16: mod_base = OTHER; note = 2'-O-methyladenosine-3'-phosphate
  modified_base 17: mod_base = OTHER; note = 2'-O-methylcytidine-3'-phosphate
  modified_base 18: mod_base = OTHER; note = 2'-O-methyladenosine-3'-phosphate
  modified_base 19: mod_base = OTHER; note = 2'-O-methylguanosine-3'-phosphate
  modified_base 20: mod_base = OTHER; note = 2'-O-methyladenosine-3'-phosphate
  modified_base 21: mod_base = OTHER; note = 2'-O-methyluridine-3'-phosphate ((2S,4R)-1-[29-[[2-(acetylamino)-2-deoxy-beta-D-galactopyranosyl]oxy]-14,14-bis[[3-[[3-[[5-[[2-(acetylamino)-2-deoxy-beta-D-galactopyranosyl]oxy]-1-oxopentyl]amino]propyl]amino]-3-oxopropoxy]methyl]-1,12,19,25-tetraoxo-16-oxa-13,20,24-triazanonacos-1-yl]-4-hydroxy-2-pyrrolidinyl)methyl ester
gtttatcaccttcttacagat

SEQ ID NO: 336 - RNA, 21 nt, synthetic construct
  source 1..21: mol_type = other RNA
  modified_base 1: mod_base = OTHER; note = 2'-O-methylguanosine-3'-phosphorothioate
  modified_base 2: mod_base = OTHER; note = 2'-O-methyladenosine-3'-phosphorothioate
  modified_base 3: mod_base = OTHER; note = 2'-O-methyladenosine-3'-phosphate
  modified_base 4: mod_base = OTHER; note = 2'-O-methylcytidine-3'-phosphate
  modified_base 5: mod_base = OTHER; note = 2'-O-methylcytidine-3'-phosphate
  modified_base 6: mod_base = OTHER; note = 2'-O-methyluridine-3'-phosphate
  modified_base 7: mod_base = OTHER; note = 2'-deoxy-2'-fluoroguanosine-3'-phosphate
  modified_base 8: mod_base = OTHER; note = 2'-O-methyladenosine-3'-phosphate
  modified_base 9: mod_base = OTHER; note = 2'-deoxy-2'-fluoroguanosine-3'-phosphate
  modified_base 10: mod_base = OTHER; note = 2'-deoxy-2'-fluorouridine-3'-phosphate
  modified_base 11: mod_base = OTHER; note = 2'-deoxy-2'-fluoroadenosine-3'-phosphate
  modified_base 12: mod_base = OTHER; note = 2'-O-methyluridine-3'-phosphate
  modified_base 13: mod_base = OTHER; note = 2'-O-methylcytidine-3'-phosphate
  modified_base 14: mod_base = OTHER; note = 2'-O-methyluridine-3'-phosphate
  modified_base 15: mod_base = OTHER; note = 2'-O-methylguanosine-3'-phosphate
  modified_base 16: mod_base = OTHER; note = 2'-O-methylcytidine-3'-phosphate
  modified_base 17: mod_base = OTHER; note = 2'-O-methyladenosine-3'-phosphate
  modified_base 18: mod_base = OTHER; note = 2'-O-methyladenosine-3'-phosphate
  modified_base 19: mod_base = OTHER; note = 2'-O-methyladenosine-3'-phosphate
  modified_base 20: mod_base = OTHER; note = 2'-O-methyladenosine-3'-phosphate
  modified_base 21: mod_base = OTHER; note = 2'-O-methyluridine-3'-phosphate ((2S,4R)-1-[29-[[2-(acetylamino)-2-deoxy-beta-D-galactopyranosyl]oxy]-14,14-bis[[3-[[3-[[5-[[2-(acetylamino)-2-deoxy-beta-D-galactopyranosyl]oxy]-1-oxopentyl]amino]propyl]amino]-3-oxopropoxy]methyl]-1,12,19,25-tetraoxo-16-oxa-13,20,24-triazanonacos-1-yl]-4-hydroxy-2-pyrrolidinyl)methyl ester
gaacctgagtatctgcaaaat

SEQ ID NO: 337 - RNA, 21 nt, synthetic construct
  source 1..21: mol_type = other RNA
  modified_base 1: mod_base = OTHER; note = 2'-O-methylguanosine-3'-phosphorothioate
  modified_base 2: mod_base = OTHER; note = 2'-O-methyluridine-3'-phosphorothioate
  modified_base 3: mod_base = OTHER; note = 2'-O-methyluridine-3'-phosphate
  modified_base 4: mod_base = OTHER; note = 2'-O-methylguanosine-3'-phosphate
  modified_base 5: mod_base = OTHER; note = 2'-O-methylcytidine-3'-phosphate
  modified_base 6: mod_base = OTHER; note = 2'-O-methyladenosine-3'-phosphate
  modified_base 7: mod_base = OTHER; note = 2'-deoxy-2'-fluorocytidine-3'-phosphate
  modified_base 8: mod_base = OTHER; note = 2'-O-methyladenosine-3'-phosphate
  modified_base 9: mod_base = OTHER; note = 2'-deoxy-2'-fluoroadenosine-3'-phosphate
  modified_base 10: mod_base = OTHER; note = 2'-deoxy-2'-fluoroadenosine-3'-phosphate
  modified_base 11: mod_base = OTHER; note = 2'-deoxy-2'-fluorouridine-3'-phosphate
  modified_base 12: mod_base = OTHER; note = 2'-O-methyladenosine-3'-phosphate
  modified_base 13: mod_base = OTHER; note = 2'-O-methylcytidine-3'-phosphate
  modified_base 14: mod_base = OTHER; note = 2'-O-methylcytidine-3'-phosphate
  modified_base 15: mod_base = OTHER; note = 2'-O-methyluridine-3'-phosphate
  modified_base 16: mod_base = OTHER; note = 2'-O-methyladenosine-3'-phosphate
  modified_base 17: mod_base = OTHER; note = 2'-O-methyladenosine-3'-phosphate
  modified_base 18: mod_base = OTHER; note = 2'-O-methyluridine-3'-phosphate
  modified_base 19: mod_base = OTHER; note = 2'-O-methyladenosine-3'-phosphate
  modified_base 20: mod_base = OTHER; note = 2'-O-methyladenosine-3'-phosphate
  modified_base 21: mod_base = OTHER; note = 2'-O-methyluridine-3'-phosphate ((2S,4R)-1-[29-[[2-(acetylamino)-2-deoxy-beta-D-galactopyranosyl]oxy]-14,14-bis[[3-[[3-[[5-[[2-(acetylamino)-2-deoxy-beta-D-galactopyranosyl]oxy]-1-oxopentyl]amino]propyl]amino]-3-oxopropoxy]methyl]-1,12,19,25-tetraoxo-16-oxa-13,20,24-triazanonacos-1-yl]-4-hydroxy-2-pyrrolidinyl)methyl ester
gttgcacaaatacctaataat

SEQ ID NO: 338 - RNA, 21 nt, synthetic construct
  source 1..21: mol_type = other RNA
  modified_base 1: mod_base = OTHER; note = 2'-O-methyluridine-3'-phosphorothioate
  modified_base 2: mod_base = OTHER; note = 2'-O-methyladenosine-3'-phosphorothioate
  modified_base 3: mod_base = OTHER; note = 2'-O-methyladenosine-3'-phosphate
  modified_base 4: mod_base = OTHER; note = 2'-O-methylcytidine-3'-phosphate
  modified_base 5: mod_base = OTHER; note = 2'-O-methylcytidine-3'-phosphate
  modified_base 6: mod_base = OTHER; note = 2'-O-methyladenosine-3'-phosphate
  modified_base 7: mod_base = OTHER; note = 2'-deoxy-2'-fluoroguanosine-3'-phosphate
  modified_base 8: mod_base = OTHER; note = 2'-O-methyladenosine-3'-phosphate
  modified_base 9: mod_base = OTHER; note = 2'-deoxy-2'-fluoroadenosine-3'-phosphate
  modified_base 10: mod_base = OTHER; note = 2'-deoxy-2'-fluorocytidine-3'-phosphate
  modified_base 11: mod_base = OTHER; note = 2'-deoxy-2'-fluoroadenosine-3'-phosphate
  modified_base 12: mod_base = OTHER; note = 2'-O-methylguanosine-3'-phosphate
  modified_base 13: mod_base = OTHER; note = 2'-O-methyladenosine-3'-phosphate
  modified_base 14: mod_base = OTHER; note = 2'-O-methyladenosine-3'-phosphate
  modified_base 15: mod_base = OTHER; note = 2'-O-methyladenosine-3'-phosphate
  modified_base 16: mod_base = OTHER; note = 2'-O-methylguanosine-3'-phosphate
  modified_base 17: mod_base = OTHER; note = 2'-O-methyladenosine-3'-phosphate
  modified_base 18: mod_base = OTHER; note = 2'-O-methyladenosine-3'-phosphate
  modified_base 19: mod_base = OTHER; note = 2'-O-methyladenosine-3'-phosphate
  modified_base 20: mod_base = OTHER; note = 2'-O-methyluridine-3'-phosphate
  modified_base 21: mod_base = OTHER; note = 2'-O-methyluridine-3'-phosphate ((2S,4R)-1-[29-[[2-(acetylamino)-2-deoxy-beta-D-galactopyranosyl]oxy]-14,14-bis[[3-[[3-[[5-[[2-(acetylamino)-2-deoxy-beta-D-galactopyranosyl]oxy]-1-oxopentyl]amino]propyl]amino]-3-oxopropoxy]methyl]-1,12,19,25-tetraoxo-16-oxa-13,20,24-triazanonacos-1-yl]-4-hydroxy-2-pyrrolidinyl)methyl ester
taaccagaacagaaagaaatt

SEQ ID NO: 339 - RNA, 21 nt, synthetic construct
  source 1..21: mol_type = other RNA
  modified_base 1: mod_base = OTHER; note = 2'-O-methylcytidine-3'-phosphorothioate
  modified_base 2: mod_base = OTHER; note = 2'-O-methyladenosine-3'-phosphorothioate
  modified_base 3: mod_base = OTHER; note = 2'-O-methyluridine-3'-phosphate
  modified_base 4: mod_base = OTHER; note = 2'-O-methyladenosine-3'-phosphate
  modified_base 5: mod_base = OTHER; note = 2'-O-methyluridine-3'-phosphate
  modified_base 6: mod_base = OTHER; note = 2'-O-methyluridine-3'-phosphate
  modified_base 7: mod_base = OTHER; note = 2'-deoxy-2'-fluoroguanosine-3'-phosphate
  modified_base 8: mod_base = OTHER; note = 2'-O-methyluridine-3'-phosphate
  modified_base 9: mod_base = OTHER; note = 2'-deoxy-2'-fluorocytidine-3'-phosphate
  modified_base 10: mod_base = OTHER; note = 2'-deoxy-2'-fluorouridine-3'-phosphate
  modified_base 11: mod_base = OTHER; note = 2'-deoxy-2'-fluorouridine-3'-phosphate
  modified_base 12: mod_base = OTHER; note = 2'-O-methylguanosine-3'-phosphate
  modified_base 13: mod_base = OTHER; note = 2'-O-methyluridine-3'-phosphate
  modified_base 14: mod_base = OTHER; note = 2'-O-methylguanosine-3'-phosphate
  modified_base 15: mod_base = OTHER; note = 2'-O-methyladenosine-3'-phosphate
  modified_base 16: mod_base = OTHER; note = 2'-O-methyladenosine-3'-phosphate
  modified_base 17: mod_base = OTHER; note = 2'-O-methylguanosine-3'-phosphate
  modified_base 18: mod_base = OTHER; note = 2'-O-methyladenosine-3'-phosphate
  modified_base 19: mod_base = OTHER; note = 2'-O-methyladenosine-3'-phosphate
  modified_base 20: mod_base = OTHER; note = 2'-O-methyluridine-3'-phosphate
  modified_base 21: mod_base = OTHER; note = 2'-O-methyluridine-3'-phosphate ((2S,4R)-1-[29-[[2-(acetylamino)-2-deoxy-beta-D-galactopyranosyl]oxy]-14,14-bis[[3-[[3-[[5-[[2-(acetylamino)-2-deoxy-beta-D-galactopyranosyl]oxy]-1-oxopentyl]amino]propyl]amino]-3-oxopropoxy]methyl]-1,12,19,25-tetraoxo-16-oxa-13,20,24-triazanonacos-1-yl]-4-hydroxy-2-pyrrolidinyl)methyl ester
catattgtcttgtgaagaatt

SEQ ID NO: 340 - RNA, 21 nt, synthetic construct
  source 1..21: mol_type = other RNA
  modified_base 1: mod_base = OTHER; note = 2'-O-methyladenosine-3'-phosphorothioate
  modified_base 2: mod_base = OTHER; note = 2'-O-methyladenosine-3'-phosphorothioate
  modified_base 3: mod_base = OTHER; note = 2'-O-methyluridine-3'-phosphate
  modified_base 4: mod_base = OTHER; note = 2'-O-methylguanosine-3'-phosphate
  modified_base 5: mod_base = OTHER; note = 2'-O-methylcytidine-3'-phosphate
  modified_base 6: mod_base = OTHER; note = 2'-O-methyluridine-3'-phosphate
  modified_base 7: mod_base = OTHER; note = 2'-deoxy-2'-fluoroguanosine-3'-phosphate
  modified_base 8: mod_base = OTHER; note = 2'-O-methyluridine-3'-phosphate
  modified_base 9: mod_base = OTHER; note = 2'-deoxy-2'-fluoroguanosine-3'-phosphate
  modified_base 10: mod_base = OTHER; note = 2'-deoxy-2'-fluoroadenosine-3'-phosphate
  modified_base 11: mod_base = OTHER; note = 2'-deoxy-2'-fluoroadenosine-3'-phosphate
  modified_base 12: mod_base = OTHER; note = 2'-O-methyladenosine-3'-phosphate
  modified_base 13: mod_base = OTHER; note = 2'-O-methyladenosine-3'-phosphate
  modified_base 14: mod_base = OTHER; note = 2'-O-methyluridine-3'-phosphate
  modified_base 15: mod_base = OTHER; note = 2'-O-methylguanosine-3'-phosphate
  modified_base 16: mod_base = OTHER; note = 2'-O-methyluridine-3'-phosphate
  modified_base 17: mod_base = OTHER; note = 2'-O-methyluridine-3'-phosphate
  modified_base 18: mod_base = OTHER; note = 2'-O-methyluridine-3'-phosphate
  modified_base 19: mod_base = OTHER; note = 2'-O-methyladenosine-3'-phosphate
  modified_base 20: mod_base = OTHER; note = 2'-O-methyladenosine-3'-phosphate
  modified_base 21: mod_base = OTHER; note = 2'-O-methyluridine-3'-phosphate ((2S,4R)-1-[29-[[2-(acetylamino)-2-deoxy-beta-D-galactopyranosyl]oxy]-14,14-bis[[3-[[3-[[5-[[2-(acetylamino)-2-deoxy-beta-D-galactopyranosyl]oxy]-1-oxopentyl]amino]propyl]amino]-3-oxopropoxy]methyl]-1,12,19,25-tetraoxo-16-oxa-13,20,24-triazanonacos-1-yl]-4-hydroxy-2-pyrrolidinyl)methyl ester
aatgctgtgaaaatgtttaat

SEQ ID NO: 341 - RNA, 21 nt, synthetic construct
  source 1..21: mol_type = other RNA
  modified_base 1: mod_base = OTHER; note = 2'-O-methyladenosine-3'-phosphorothioate
  modified_base 2: mod_base = OTHER; note = 2'-O-methylguanosine-3'-phosphorothioate
  modified_base 3: mod_base = OTHER; note = 2'-O-methyladenosine-3'-phosphate
  modified_base 4: mod_base = OTHER; note = 2'-O-methylguanosine-3'-phosphate
  modified_base 5: mod_base = OTHER; note = 2'-O-methyluridine-3'-phosphate
  modified_base 6: mod_base = OTHER; note = 2'-O-methylguanosine-3'-phosphate
  modified_base 7: mod_base = OTHER; note = 2'-deoxy-2'-fluorouridine-3'-phosphate
  modified_base 8: mod_base = OTHER; note = 2'-O-methylcytidine-3'-phosphate
  modified_base 9: mod_base = OTHER; note = 2'-deoxy-2'-fluorouridine-3'-phosphate
  modified_base 10: mod_base = OTHER; note = 2'-deoxy-2'-fluoroguanosine-3'-phosphate
  modified_base 11: mod_base = OTHER; note = 2'-deoxy-2'-fluorouridine-3'-phosphate
  modified_base 12: mod_base = OTHER; note = 2'-O-methyluridine-3'-phosphate
  modified_base 13: mod_base = OTHER; note = 2'-O-methyluridine-3'-phosphate
  modified_base 14: mod_base = OTHER; note = 2'-O-methyluridine-3'-phosphate
  modified_base 15: mod_base = OTHER; note = 2'-O-methyladenosine-3'-phosphate
  modified_base 16: mod_base = OTHER; note = 2'-O-methylguanosine-3'-phosphate
  modified_base 17: mod_base = OTHER; note = 2'-O-methyladenosine-3'-phosphate
  modified_base 18: mod_base = OTHER; note = 2'-O-methyladenosine-3'-phosphate
  modified_base 19: mod_base = OTHER; note = 2'-O-methylcytidine-3'-phosphate
  modified_base 20: mod_base = OTHER; note = 2'-O-methyluridine-3'-phosphate
  modified_base 21: mod_base = OTHER; note = 2'-O-methyluridine-3'-phosphate ((2S,4R)-1-[29-[[2-(acetylamino)-2-deoxy-beta-D-galactopyranosyl]oxy]-14,14-bis[[3-[[3-[[5-[[2-(acetylamino)-2-deoxy-beta-D-galactopyranosyl]oxy]-1-oxopentyl]amino]propyl]amino]-3-oxopropoxy]methyl]-1,12,19,25-tetraoxo-16-oxa-13,20,24-triazanonacos-1-yl]-4-hydroxy-2-pyrrolidinyl)methyl ester
agagtgtctgttttagaactt

SEQ ID NO: 342 - RNA, 21 nt, synthetic construct
  source 1..21: mol_type = other RNA
  modified_base 1: mod_base = OTHER; note = 2'-O-methyluridine-3'-phosphorothioate
  modified_base 2: mod_base = OTHER; note = 2'-O-methyladenosine-3'-phosphorothioate
  modified_base 3: mod_base = OTHER; note = 2'-O-methyluridine-3'-phosphate
  modified_base 4: mod_base = OTHER; note = 2'-O-methyladenosine-3'-phosphate
  modified_base 5: mod_base = OTHER; note = 2'-O-methyluridine-3'-phosphate
  modified_base 6: mod_base = OTHER; note = 2'-O-methyluridine-3'-phosphate
  modified_base 7: mod_base = OTHER; note = 2'-deoxy-2'-fluorocytidine-3'-phosphate
  modified_base 8: mod_base = OTHER; note = 2'-O-methyluridine-3'-phosphate
  modified_base 9: mod_base = OTHER; note = 2'-deoxy-2'-fluoroguanosine-3'-phosphate
  modified_base 10: mod_base = OTHER; note = 2'-deoxy-2'-fluoroadenosine-3'-phosphate
  modified_base 11: mod_base = OTHER; note = 2'-deoxy-2'-fluoroguanosine-3'-phosphate
  modified_base 12: mod_base = OTHER; note = 2'-O-methyluridine-3'-phosphate
  modified_base 13: mod_base = OTHER; note = 2'-O-methyluridine-3'-phosphate
  modified_base 14: mod_base = OTHER; note = 2'-O-methyluridine-3'-phosphate
  modified_base 15: mod_base = OTHER; note = 2'-O-methyluridine-3'-phosphate
  modified_base 16: mod_base = OTHER; note = 2'-O-methylguanosine-3'-phosphate
  modified_base 17: mod_base = OTHER; note = 2'-O-methyluridine-3'-phosphate
  modified_base 18: mod_base = OTHER; note = 2'-O-methylguanosine-3'-phosphate
  modified_base 19: mod_base = OTHER; note = 2'-O-methylguanosine-3'-phosphate
  modified_base 20: mod_base = OTHER; note = 2'-O-methyluridine-3'-phosphate
  modified_base 21: mod_base = OTHER; note = 2'-O-methyluridine-3'-phosphate ((2S,4R)-1-[29-[[2-(acetylamino)-2-deoxy-beta-D-galactopyranosyl]oxy]-14,14-bis[[3-[[3-[[5-[[2-(acetylamino)-2-deoxy-beta-D-galactopyranosyl]oxy]-1-oxopentyl]amino]propyl]amino]-3-oxopropoxy]methyl]-1,12,19,25-tetraoxo-16-oxa-13,20,24-triazanonacos-1-yl]-4-hydroxy-2-pyrrolidinyl)methyl ester
tatattctgagttttgtggtt

SEQ ID NO: 343 - RNA, 21 nt, synthetic construct
  source 1..21: mol_type = other RNA
  modified_base 1: mod_base = OTHER; note = 2'-O-methyladenosine-3'-phosphorothioate
  modified_base 2: mod_base = OTHER; note = 2'-O-methyluridine-3'-phosphorothioate
  modified_base 3: mod_base = OTHER; note = 2'-O-methylguanosine-3'-phosphate
  modified_base 4: mod_base = OTHER; note = 2'-O-methyladenosine-3'-phosphate
  modified_base 5: mod_base = OTHER; note = 2'-O-methylguanosine-3'-phosphate
  modified_base 6: mod_base = OTHER; note = 2'-O-methyladenosine-3'-phosphate
  modified_base 7: mod_base = OTHER; note = 2'-deoxy-2'-fluorouridine-3'-phosphate
  modified_base 8: mod_base = OTHER; note = 2'-O-methylguanosine-3'-phosphate
  modified_base 9: mod_base = OTHER; note = 2'-deoxy-2'-fluoroadenosine-3'-phosphate
  modified_base 10: mod_base = OTHER; note = 2'-deoxy-2'-fluoroguanosine-3'-phosphate
  modified_base 11: mod_base = OTHER; note = 2'-deoxy-2'-fluorouridine-3'-phosphate
  modified_base 12: mod_base = OTHER; note = 2'-O-methyluridine-3'-phosphate
  modified_base 13: mod_base = OTHER; note = 2'-O-methylcytidine-3'-phosphate
  modified_base 14: mod_base = OTHER; note = 2'-O-methylcytidine-3'-phosphate
  modified_base 15: mod_base = OTHER; note = 2'-O-methyluridine-3'-phosphate
  modified_base 16: mod_base = OTHER; note = 2'-O-methyluridine-3'-phosphate
  modified_base 17: mod_base = OTHER; note = 2'-O-methylguanosine-3'-phosphate
  modified_base 18: mod_base = OTHER; note = 2'-O-methyluridine-3'-phosphate
  modified_base 19: mod_base = OTHER; note = 2'-O-methyladenosine-3'-phosphate
  modified_base 20: mod_base = OTHER; note = 2'-O-methylguanosine-3'-phosphate
  modified_base 21: mod_base = OTHER; note = 2'-O-methyluridine-3'-phosphate ((2S,4R)-1-[29-[[2-(acetylamino)-2-deoxy-beta-D-galactopyranosyl]oxy]-14,14-bis[[3-[[3-[[5-[[2-(acetylamino)-2-deoxy-beta-D-galactopyranosyl]oxy]-1-oxopentyl]amino]propyl]amino]-3-oxopropoxy]methyl]-1,12,19,25-tetraoxo-16-oxa-13,20,24-triazanonacos-1-yl]-4-hydroxy-2-pyrrolidinyl)methyl ester
atgagatgagttccttgtagt

SEQ ID NO: 344 - RNA, 21 nt, synthetic construct
  source 1..21: mol_type = other RNA
  modified_base 1: mod_base = OTHER; note = 2'-O-methyladenosine-3'-phosphorothioate
  modified_base 2: mod_base = OTHER; note = 2'-O-methylcytidine-3'-phosphorothioate
  modified_base 3: mod_base = OTHER; note = 2'-O-methyladenosine-3'-phosphate
  modified_base 4: mod_base = OTHER; note = 2'-O-methyladenosine-3'-phosphate
  modified_base 5: mod_base = OTHER; note = 2'-O-methylguanosine-3'-phosphate
  modified_base 6: mod_base = OTHER; note = 2'-O-methyladenosine-3'-phosphate
  modified_base 7: mod_base = OTHER; note = 2'-deoxy-2'-fluorouridine-3'-phosphate
  modified_base 8: mod_base = OTHER; note = 2'-O-methylguanosine-3'-phosphate
  modified_base 9: mod_base = OTHER; note = 2'-deoxy-2'-fluoroadenosine-3'-phosphate
  modified_base 10: mod_base = OTHER; note = 2'-deoxy-2'-fluoroadenosine-3'-phosphate
  modified_base 11: mod_base = OTHER; note = 2'-deoxy-2'-fluoroadenosine-3'-phosphate
  modified_base 12: mod_base = OTHER; note = 2'-O-methyluridine-3'-phosphate
  modified_base 13: mod_base = OTHER; note = 2'-O-methylcytidine-3'-phosphate
  modified_base 14: mod_base = OTHER; note = 2'-O-methyluridine-3'-phosphate
  modified_base 15: mod_base = OTHER; note = 2'-O-methylcytidine-3'-phosphate
  modified_base 16: mod_base = OTHER; note = 2'-O-methyladenosine-3'-phosphate
  modified_base 17: mod_base = OTHER; note = 2'-O-methyladenosine-3'-phosphate
  modified_base 18: mod_base = OTHER; note = 2'-O-methyluridine-3'-phosphate
  modified_base 19: mod_base = OTHER; note = 2'-O-methyladenosine-3'-phosphate
  modified_base 20: mod_base = OTHER; note = 2'-O-methyladenosine-3'-phosphate
  modified_base 21: mod_base = OTHER; note = 2'-O-methyluridine-3'-phosphate ((2S,4R)-1-[29-[[2-(acetylamino)-2-deoxy-beta-D-galactopyranosyl]oxy]-14,14-bis[[3-[[3-[[5-[[2-(acetylamino)-2-deoxy-beta-D-galactopyranosyl]oxy]-1-oxopentyl]amino]propyl]amino]-3-oxopropoxy]methyl]-1,12,19,25-tetraoxo-16-oxa-13,20,24-triazanonacos-1-yl]-4-hydroxy-2-pyrrolidinyl)methyl ester
acaagatgaaatctcaataat

SEQ ID NO: 345 - RNA, 21 nt, synthetic construct
  source 1..21: mol_type = other RNA
  modified_base 1: mod_base = OTHER; note = 2'-O-methyladenosine-3'-phosphorothioate
  modified_base 2: mod_base = OTHER; note = 2'-O-methylcytidine-3'-phosphorothioate
  modified_base 3: mod_base = OTHER; note = 2'-O-methyladenosine-3'-phosphate
  modified_base 4: mod_base = OTHER; note = 2'-O-methyladenosine-3'-phosphate
  modified_base 5: mod_base = OTHER; note = 2'-O-methylcytidine-3'-phosphate
  modified_base 6: mod_base = OTHER; note = 2'-O-methyluridine-3'-phosphate
  modified_base 7: mod_base = OTHER; note = 2'-deoxy-2'-fluorouridine-3'-phosphate
  modified_base 8: mod_base = OTHER; note = 2'-O-methyluridine-3'-phosphate
  modified_base 9: mod_base = OTHER; note = 2'-deoxy-2'-fluorouridine-3'-phosphate
  modified_base 10: mod_base = OTHER; note = 2'-deoxy-2'-fluoroadenosine-3'-phosphate
  modified_base 11: mod_base = OTHER; note = 2'-deoxy-2'-fluoroadenosine-3'-phosphate
  modified_base 12: mod_base = OTHER; note = 2'-O-methylguanosine-3'-phosphate
  modified_base 13: mod_base = OTHER; note = 2'-O-methylguanosine-3'-phosphate
  modified_base 14: mod_base = OTHER; note = 2'-O-methyladenosine-3'-phosphate
  modified_base 15: mod_base = OTHER; note = 2'-O-methylcytidine-3'-phosphate
  modified_base 16: mod_base = OTHER; note = 2'-O-methyluridine-3'-phosphate
  modified_base 17: mod_base = OTHER; note = 2'-O-methyladenosine-3'-phosphate
  modified_base 18: mod_base = OTHER; note = 2'-O-methyladenosine-3'-phosphate
  modified_base 19: mod_base = OTHER; note = 2'-O-methyluridine-3'-phosphate
  modified_base 20: mod_base = OTHER; note = 2'-O-methyluridine-3'-phosphate
  modified_base 21: mod_base = OTHER; note = 2'-O-methyluridine-3'-phosphate ((2S,4R)-1-[29-[[2-(acetylamino)-2-deoxy-beta-D-galactopyranosyl]oxy]-14,14-bis[[3-[[3-[[5-[[2-(acetylamino)-2-deoxy-beta-D-galactopyranosyl]oxy]-1-oxopentyl]amino]propyl]amino]-3-oxopropoxy]methyl]-1,12,19,25-tetraoxo-16-oxa-13,20,24-triazanonacos-1-yl]-4-hydroxy-2-pyrrolidinyl)methyl ester
acaacttttaaggactaattt

SEQ ID NO: 346 - RNA, 21 nt, synthetic construct
  source 1..21: mol_type = other RNA
  modified_base 1: mod_base = OTHER; note = 2'-O-methyladenosine-3'-phosphorothioate
  modified_base 2: mod_base = OTHER; note = 2'-O-methyladenosine-3'-phosphorothioate
  modified_base 3: mod_base = OTHER; note = 2'-O-methyluridine-3'-phosphate
  modified_base 4: mod_base = OTHER; note = 2'-O-methylcytidine-3'-phosphate
  modified_base 5: mod_base = OTHER; note = 2'-O-methyluridine-3'-phosphate
  modified_base 6: mod_base = OTHER; note = 2'-O-methyluridine-3'-phosphate
  modified_base 7: mod_base = OTHER; note = 2'-deoxy-2'-fluoroadenosine-3'-phosphate
  modified_base 8: mod_base = OTHER; note = 2'-O-methylcytidine-3'-phosphate
  modified_base 9: mod_base = OTHER; note = 2'-deoxy-2'-fluoroadenosine-3'-phosphate
  modified_base 10: mod_base = OTHER; note = 2'-deoxy-2'-fluorouridine-3'-phosphate
  modified_base 11: mod_base = OTHER; note = 2'-deoxy-2'-fluoroguanosine-3'-phosphate
  modified_base 12: mod_base = OTHER; note = 2'-O-methylguanosine-3'-phosphate
  modified_base 13: mod_base = OTHER; note = 2'-O-methyluridine-3'-phosphate
  modified_base 14: mod_base = OTHER; note = 2'-O-methyladenosine-3'-phosphate
  modified_base 15: mod_base = OTHER; note = 2'-O-methyluridine-3'-phosphate
  modified_base 16: mod_base = OTHER; note = 2'-O-methyladenosine-3'-phosphate
  modified_base 17: mod_base = OTHER; note = 2'-O-methylcytidine-3'-phosphate
  modified_base 18: mod_base = OTHER; note = 2'-O-methyluridine-3'-phosphate
  modified_base 19: mod_base = OTHER; note = 2'-O-methyluridine-3'-phosphate
  modified_base 20: mod_base = OTHER; note = 2'-O-methyladenosine-3'-phosphate
  modified_base 21: mod_base = OTHER; note = 2'-O-methyluridine-3'-phosphate ((2S,4R)-1-[29-[[2-(acetylamino)-2-deoxy-beta-D-galactopyranosyl]oxy]-14,14-bis[[3-[[3-[[5-[[2-(acetylamino)-2-deoxy-beta-D-galactopyranosyl]oxy]-1-oxopentyl]amino]propyl]amino]-3-oxopropoxy]methyl]-1,12,19,25-tetraoxo-16-oxa-13,20,24-triazanonacos-1-yl]-4-hydroxy-2-pyrrolidinyl)methyl ester
aatcttacatggtatacttat

SEQ ID NO: 347 - RNA, 21 nt, synthetic construct
  source 1..21: mol_type = other RNA
  modified_base 1: mod_base = OTHER; note = 2'-O-methyluridine-3'-phosphorothioate
  modified_base 2: mod_base = OTHER; note = 2'-O-methylguanosine-3'-phosphorothioate
  modified_base 3: mod_base = OTHER; note = 2'-O-methyluridine-3'-phosphate
  modified_base 4: mod_base = OTHER; note = 2'-O-methyluridine-3'-phosphate
  modified_base 5: mod_base = OTHER; note = 2'-O-methylguanosine-3'-phosphate
  modified_base 6: mod_base = OTHER; note = 2'-O-methylguanosine-3'-phosphate
  modified_base 7: mod_base = OTHER; note = 2'-deoxy-2'-fluorouridine-3'-phosphate
  modified_base 8: mod_base = OTHER; note = 2'-O-methyladenosine-3'-phosphate
  modified_base 9: mod_base = OTHER; note = 2'-deoxy-2'-fluorouridine-3'-phosphate
  modified_base 10: mod_base = OTHER; note = 2'-deoxy-2'-fluoroadenosine-3'-phosphate
  modified_base 11: mod_base = OTHER; note = 2'-deoxy-2'-fluorouridine-3'-phosphate
  modified_base 12: mod_base = OTHER; note = 2'-O-methyluridine-3'-phosphate
  modified_base 13: mod_base = OTHER; note = 2'-O-methyladenosine-3'-phosphate
  modified_base 14: mod_base = OTHER; note = 2'-O-methyluridine-3'-phosphate
  modified_base 15: mod_base = OTHER; note = 2'-O-methylcytidine-3'-phosphate
  modified_base 16: mod_base = OTHER; note = 2'-O-methyluridine-3'-phosphate
  modified_base 17: mod_base = OTHER; note = 2'-O-methylguanosine-3'-phosphate
  modified_base 18: mod_base = OTHER; note = 2'-O-methylguanosine-3'-phosphate
  modified_base 19: mod_base = OTHER; note = 2'-O-methyluridine-3'-phosphate
  modified_base 20: mod_base = OTHER; note = 2'-O-methyluridine-3'-phosphate
  modified_base 21: mod_base = OTHER; note = 2'-O-methyluridine-3'-phosphate ((2S,4R)-1-[29-[[2-(acetylamino)-2-deoxy-beta-D-galactopyranosyl]oxy]-14,14-bis[[3-[[3-[[5-[[2-(acetylamino)-2-deoxy-beta-D-galactopyranosyl]oxy]-1-oxopentyl]amino]propyl]amino]-3-oxopropoxy]methyl]-1,12,19,25-tetraoxo-16-oxa-13,20,24-triazanonacos-1-yl]-4-hydroxy-2-pyrrolidinyl)methyl ester
tgttggtatattatctggttt

SEQ ID NO: 348 - RNA, 21 nt, synthetic construct
  source 1..21: mol_type = other RNA
  modified_base 1: mod_base = OTHER; note = 2'-O-methyluridine-3'-phosphorothioate
  modified_base 2: mod_base = OTHER; note = 2'-O-methyluridine-3'-phosphorothioate
  modified_base 3: mod_base = OTHER; note = 2'-O-methyladenosine-3'-phosphate
  modified_base 4: mod_base = OTHER; note = 2'-O-methylguanosine-3'-phosphate
  modified_base 5: mod_base = OTHER; note = 2'-O-methyluridine-3'-phosphate
  modified_base 6: mod_base = OTHER; note = 2'-O-methylguanosine-3'-phosphate
  modified_base 7: mod_base = OTHER; note = 2'-deoxy-2'-fluoroguanosine-3'-phosphate
  modified_base 8: mod_base = OTHER; note = 2'-O-methyluridine-3'-phosphate
  modified_base 9: mod_base = OTHER; note = 2'-deoxy-2'-fluorouridine-3'-phosphate
  modified_base 10: mod_base = OTHER; note = 2'-deoxy-2'-fluoroadenosine-3'-phosphate
  modified_base 11: mod_base = OTHER; note = 2'-deoxy-2'-fluoroadenosine-3'-phosphate
  modified_base 12: mod_base = OTHER; note = 2'-O-methyluridine-3'-phosphate
  modified_base 13: mod_base = OTHER; note = 2'-O-methylguanosine-3'-phosphate
  modified_base 14: mod_base = OTHER; note = 2'-O-methylcytidine-3'-phosphate
  modified_base 15: mod_base = OTHER; note = 2'-O-methyluridine-3'-phosphate
  modified_base 16: mod_base = OTHER; note = 2'-O-methyluridine-3'-phosphate
  modified_base 17: mod_base = OTHER; note = 2'-O-methylcytidine-3'-phosphate
  modified_base 18: mod_base = OTHER; note = 2'-O-methylcytidine-3'-phosphate
  modified_base 19: mod_base = OTHER; note = 2'-O-methyluridine-3'-phosphate
  modified_base 20: mod_base = OTHER; note = 2'-O-methyluridine-3'-phosphate
  modified_base 21: mod_base = OTHER; note = 2'-O-methyluridine-3'-phosphate ((2S,4R)-1-[29-[[2-(acetylamino)-2-deoxy-beta-D-galactopyranosyl]oxy]-14,14-bis[[3-[[3-[[5-[[2-(acetylamino)-2-deoxy-beta-D-galactopyranosyl]oxy]-1-oxopentyl]amino]propyl]amino]-3-oxopropoxy]methyl]-1,12,19,25-tetraoxo-16-oxa-13,20,24-triazanonacos-1-yl]-4-hydroxy-2-pyrrolidinyl)methyl ester
ttagtggttaatgcttccttt

SEQ ID NO: 349 - RNA, 21 nt, synthetic construct
  source 1..21: mol_type = other RNA
  modified_base 1: mod_base = OTHER; note = 2'-O-methyluridine-3'-phosphorothioate
  modified_base 2: mod_base = OTHER; note = 2'-O-methylguanosine-3'-phosphorothioate
  modified_base 3: mod_base = OTHER; note = 2'-O-methyladenosine-3'-phosphate
  modified_base 4: mod_base = OTHER; note = 2'-O-methylguanosine-3'-phosphate
  modified_base 5: mod_base = OTHER; note = 2'-O-methyluridine-3'-phosphate
  modified_base 6: mod_base = OTHER; note = 2'-O-methylcytidine-3'-phosphate
  modified_base 7: mod_base = OTHER; note = 2'-deoxy-2'-fluoroadenosine-3'-phosphate
  modified_base 8: mod_base = OTHER; note = 2'-O-methyluridine-3'-phosphate
  modified_base 9: mod_base = OTHER; note = 2'-deoxy-2'-fluorocytidine-3'-phosphate
  modified_base 10: mod_base = OTHER; note = 2'-deoxy-2'-fluorocytidine-3'-phosphate
  modified_base 11: mod_base = OTHER; note = 2'-deoxy-2'-fluoroadenosine-3'-phosphate
  modified_base 12: mod_base = OTHER; note = 2'-O-methyluridine-3'-phosphate
  modified_base 13: mod_base = OTHER; note = 2'-O-methyluridine-3'-phosphate
  modified_base 14: mod_base = OTHER; note = 2'-O-methylcytidine-3'-phosphate
  modified_base 15: mod_base = OTHER; note = 2'-O-methyladenosine-3'-phosphate
  modified_base 16: mod_base = OTHER; note = 2'-O-methylcytidine-3'-phosphate
  modified_base 17: mod_base = OTHER; note = 2'-O-methyluridine-3'-phosphate
  modified_base 18: mod_base = OTHER; note = 2'-O-methylcytidine-3'-phosphate
  modified_base 19: mod_base = OTHER; note = 2'-O-methyluridine-3'-phosphate
  modified_base 20: mod_base = OTHER; note = 2'-O-methyluridine-3'-phosphate
  modified_base 21: mod_base = OTHER; note = 2'-O-methyluridine-3'-phosphate ((2S,4R)-1-[29-[[2-(acetylamino)-2-deoxy-beta-D-galactopyranosyl]oxy]-14,14-bis[[3-[[3-[[5-[[2-(acetylamino)-2-deoxy-beta-D-galactopyranosyl]oxy]-1-oxopentyl]amino]propyl]amino]-3-oxopropoxy]methyl]-1,12,19,25-tetraoxo-16-oxa-13,20,24-triazanonacos-1-yl]-4-hydroxy-2-pyrrolidinyl)methyl ester
tgagtcatccattcactcttt

SEQ ID NO: 350 - RNA, 21 nt, synthetic construct
  source 1..21: mol_type = other RNA
  modified_base 1: mod_base = OTHER; note = 2'-O-methylcytidine-3'-phosphorothioate
  modified_base 2: mod_base = OTHER; note = 2'-O-methyladenosine-3'-phosphorothioate
  modified_base 3: mod_base = OTHER; note = 2'-O-methylguanosine-3'-phosphate
  modified_base 4: mod_base = OTHER; note = 2'-O-methyluridine-3'-phosphate
  modified_base 5: mod_base = OTHER; note = 2'-O-methyluridine-3'-phosphate
  modified_base 6: mod_base = OTHER; note = 2'-O-methyluridine-3'-phosphate
  modified_base 7: mod_base = OTHER; note = 2'-deoxy-2'-fluorouridine-3'-phosphate
  modified_base 8: mod_base = OTHER; note = 2'-O-methyladenosine-3'-phosphate
  modified_base 9: mod_base = OTHER; note = 2'-deoxy-2'-fluorouridine-3'-phosphate
  modified_base 10: mod_base = OTHER; note = 2'-deoxy-2'-fluorocytidine-3'-phosphate
  modified_base 11: mod_base = OTHER; note = 2'-deoxy-2'-fluorouridine-3'-phosphate
  modified_base 12: mod_base = OTHER; note = 2'-O-methylguanosine-3'-phosphate
  modified_base 13: mod_base = OTHER; note = 2'-O-methyluridine-3'-phosphate
  modified_base 14: mod_base = OTHER; note = 2'-O-methylcytidine-3'-phosphate
  modified_base 15: mod_base = OTHER; note = 2'-O-methyladenosine-3'-phosphate
  modified_base 16: mod_base = OTHER; note = 2'-O-methyladenosine-3'-phosphate
  modified_base 17: mod_base = OTHER; note = 2'-O-methyluridine-3'-phosphate
  modified_base 18: mod_base = OTHER; note = 2'-O-methyladenosine-3'-phosphate
  modified_base 19: mod_base = OTHER; note = 2'-O-methylguanosine-3'-phosphate
  modified_base 20: mod_base = OTHER; note = 2'-O-methyluridine-3'-phosphate
  modified_base 21: mod_base = OTHER; note = 2'-O-methyluridine-3'-phosphate ((2S,4R)-1-[29-[[2-(acetylamino)-2-deoxy-beta-D-galactopyranosyl]oxy]-14,14-bis[[3-[[3-[[5-[[2-(acetylamino)-2-deoxy-beta-D-galactopyranosyl]oxy]-1-oxopentyl]amino]propyl]amino]-3-oxopropoxy]methyl]-1,12,19,25-tetraoxo-16-oxa-13,20,24-triazanonacos-1-yl]-4-hydroxy-2-pyrrolidinyl)methyl ester
cagttttatctgtcaatagtt

SEQ ID NO: 351 - RNA, 21 nt, synthetic construct
  source 1..21: mol_type = other RNA
  modified_base 1: mod_base = OTHER; note = 2'-O-methylcytidine-3'-phosphorothioate
  modified_base 2: mod_base = OTHER; note = 2'-O-methylcytidine-3'-phosphorothioate
  modified_base 3: mod_base = OTHER; note = 2'-O-methylcytidine-3'-phosphate
  modified_base 4: mod_base = OTHER; note = 2'-O-methyladenosine-3'-phosphate
  modified_base 5: mod_base = OTHER; note = 2'-O-methyladenosine-3'-phosphate
  modified_base 6: mod_base = OTHER; note = 2'-O-methyladenosine-3'-phosphate
  modified_base 7: mod_base = OTHER; note = 2'-deoxy-2'-fluoroguanosine-3'-phosphate
  modified_base 8: mod_base = OTHER; note = 2'-O-methyluridine-3'-phosphate
  modified_base 9: mod_base = OTHER; note = 2'-deoxy-2'-fluoroguanosine-3'-phosphate
  modified_base 10: mod_base = OTHER; note = 2'-deoxy-2'-fluorocytidine-3'-phosphate
  modified_base 11: mod_base = OTHER; note = 2'-deoxy-2'-fluorouridine-3'-phosphate
  modified_base 12: mod_base = OTHER; note = 2'-O-methyluridine-3'-phosphate
  modified_base 13: mod_base = OTHER; note = 2'-O-methyluridine-3'-phosphate
  modified_base 14: mod_base = OTHER; note = 2'-O-methyladenosine-3'-phosphate
  modified_base 15: mod_base = OTHER; note = 2'-O-methyluridine-3'-phosphate
  modified_base 16: mod_base = OTHER; note = 2'-O-methyladenosine-3'-phosphate
  modified_base 17: mod_base = OTHER; note = 2'-O-methyladenosine-3'-phosphate
  modified_base 18: mod_base = OTHER; note = 2'-O-methyladenosine-3'-phosphate
  modified_base 19: mod_base = OTHER; note = 2'-O-methyluridine-3'-phosphate
  modified_base 20: mod_base = OTHER; note = 2'-O-methyluridine-3'-phosphate
  modified_base 21: mod_base = OTHER; note = 2'-O-methyluridine-3'-phosphate ((2S,4R)-1-[29-[[2-(acetylamino)-2-deoxy-beta-D-galactopyranosyl]oxy]-14,14-bis[[3-[[3-[[5-[[2-(acetylamino)-2-deoxy-beta-D-galactopyranosyl]oxy]-1-oxopentyl]amino]propyl]amino]-3-oxopropoxy]methyl]-1,12,19,25-tetraoxo-16-oxa-13,20,24-triazanonacos-1-yl]-4-hydroxy-2-pyrrolidinyl)methyl ester
cccaaagtgctttataaattt

SEQ ID NO: 352 - RNA, 21 nt, synthetic construct
  source 1..21: mol_type = other RNA
  modified_base 1: mod_base = OTHER; note = 2'-O-methyluridine-3'-phosphorothioate
  modified_base 2: mod_base = OTHER; note = 2'-O-methylguanosine-3'-phosphorothioate
  modified_base 3: mod_base = OTHER; note = 2'-O-methyluridine-3'-phosphate
  modified_base 4: mod_base = OTHER; note = 2'-O-methylcytidine-3'-phosphate
  modified_base 5: mod_base = OTHER; note = 2'-O-methyladenosine-3'-phosphate
  modified_base 6: mod_base = OTHER; note = 2'-O-methylguanosine-3'-phosphate
  modified_base 7: mod_base = OTHER; note = 2'-deoxy-2'-fluoroadenosine-3'-phosphate
  modified_base 8: mod_base = OTHER; note = 2'-O-methyluridine-3'-phosphate
  modified_base 9: mod_base = OTHER; note = 2'-deoxy-2'-fluorouridine-3'-phosphate
  modified_base 10: mod_base = OTHER; note = 2'-deoxy-2'-fluorouridine-3'-phosphate
  modified_base 11: mod_base = OTHER; note = 2'-deoxy-2'-fluoroadenosine-3'-phosphate
  modified_base 12: mod_base = OTHER; note = 2'-O-methylguanosine-3'-phosphate
  modified_base 13: mod_base = OTHER; note = 2'-O-methyladenosine-3'-phosphate
  modified_base 14: mod_base = OTHER; note = 2'-O-methyladenosine-3'-phosphate
  modified_base 15: mod_base = OTHER; note = 2'-O-methyladenosine-3'-phosphate
  modified_base 16: mod_base = OTHER; note = 2'-O-methyluridine-3'-phosphate
  modified_base 17: mod_base = OTHER; note = 2'-O-methylguanosine-3'-phosphate
  modified_base 18: mod_base = OTHER; note = 2'-O-methyluridine-3'-phosphate
  modified_base 19: mod_base = OTHER; note = 2'-O-methyluridine-3'-phosphate
  modified_base 20: mod_base = OTHER; note = 2'-O-methyluridine-3'-phosphate
  modified_base 21: mod_base = OTHER; note = 2'-O-methyluridine-3'-phosphate ((2S,4R)-1-[29-[[2-(acetylamino)-2-deoxy-beta-D-galactopyranosyl]oxy]-14,14-bis[[3-[[3-[[5-[[2-(acetylamino)-2-deoxy-beta-D-galactopyranosyl]oxy]-1-oxopentyl]amino]propyl]amino]-3-oxopropoxy]methyl]-1,12,19,25-tetraoxo-16-oxa-13,20,24-triazanonacos-1-yl]-4-hydroxy-2-pyrrolidinyl)methyl ester
tgtcagatttagaaatgtttt

SEQ ID NO: 353 - RNA, 21 nt, synthetic construct
  source 1..21: mol_type = other RNA
  modified_base 1: mod_base = OTHER; note = 2'-O-methyladenosine-3'-phosphorothioate
  modified_base 2: mod_base = OTHER; note = 2'-O-methyluridine-3'-phosphorothioate
  modified_base 3: mod_base = OTHER; note = 2'-O-methylguanosine-3'-phosphate
  modified_base 4: mod_base = OTHER; note = 2'-O-methyluridine-3'-phosphate
  modified_base 5: mod_base = OTHER; note = 2'-O-methylguanosine-3'-phosphate
  modified_base 6: mod_base = OTHER; note = 2'-O-methyladenosine-3'-phosphate
  modified_base 7: mod_base = OTHER; note = 2'-deoxy-2'-fluoroadenosine-3'-phosphate
  modified_base 8: mod_base = OTHER; note = 2'-O-methyladenosine-3'-phosphate
  modified_base 9: mod_base = OTHER; note = 2'-deoxy-2'-fluoroadenosine-3'-phosphate
  modified_base 10: mod_base = OTHER; note = 2'-deoxy-2'-fluorocytidine-3'-phosphate
  modified_base 11: mod_base = OTHER; note = 2'-deoxy-2'-fluoroadenosine-3'-phosphate
  modified_base 12: mod_base = OTHER; note = 2'-O-methylguanosine-3'-phosphate
  modified_base 13: mod_base = OTHER; note = 2'-O-methyladenosine-3'-phosphate
  modified_base 14: mod_base = OTHER; note = 2'-O-methylcytidine-3'-phosphate
  modified_base 15: mod_base = OTHER; note = 2'-O-methyladenosine-3'-phosphate
  modified_base 16: mod_base = OTHER; note = 2'-O-methyladenosine-3'-phosphate
  modified_base 17: mod_base = OTHER; note = 2'-O-methyluridine-3'-phosphate
  modified_base 18: mod_base = OTHER; note = 2'-O-methyladenosine-3'-phosphate
  modified_base 19: mod_base = OTHER; note = 2'-O-methyluridine-3'-phosphate
  modified_base 20: mod_base = OTHER; note = 2'-O-methyluridine-3'-phosphate
  modified_base 21: mod_base = OTHER; note = 2'-O-methyluridine-3'-phosphate ((2S,4R)-1-[29-[[2-(acetylamino)-2-deoxy-beta-D-galactopyranosyl]oxy]-14,14-bis[[3-[[3-[[5-[[2-(acetylamino)-2-deoxy-beta-D-galactopyranosyl]oxy]-1-oxopentyl]amino]propyl]amino]-3-oxopropoxy]methyl]-1,12,19,25-tetraoxo-16-oxa-13,20,24-triazanonacos-1-yl]-4-hydroxy-2-pyrrolidinyl)methyl ester
atgtgaaaacagacaatattt

SEQ ID NO: 354 - RNA, 21 nt, synthetic construct
  source 1..21: mol_type = other RNA
  modified_base 1: mod_base = OTHER; note = 2'-O-methyladenosine-3'-phosphorothioate
  modified_base 2: mod_base = OTHER; note = 2'-O-methyladenosine-3'-phosphorothioate
  modified_base 3: mod_base = OTHER; note = 2'-O-methylcytidine-3'-phosphate
  modified_base 4: mod_base = OTHER; note = 2'-O-methyluridine-3'-phosphate
  modified_base 5: mod_base = OTHER; note = 2'-O-methylguanosine-3'-phosphate
  modified_base 6: mod_base = OTHER; note = 2'-O-methyladenosine-3'-phosphate
  modified_base 7: mod_base = OTHER; note = 2'-deoxy-2'-fluoroguanosine-3'-phosphate
  modified_base 8: mod_base = OTHER; note = 2'-O-methyladenosine-3'-phosphate
  modified_base 9: mod_base = OTHER; note = 2'-deoxy-2'-fluorouridine-3'-phosphate
  modified_base 10: mod_base = OTHER; note = 2'-deoxy-2'-fluoroadenosine-3'-phosphate
  modified_base 11: mod_base = OTHER; note = 2'-deoxy-2'-fluorouridine-3'-phosphate
  modified_base 12: mod_base = OTHER; note = 2'-O-methyluridine-3'-phosphate
  modified_base 13: mod_base = OTHER; note = 2'-O-methylguanosine-3'-phosphate
  modified_base 14: mod_base = OTHER; note = 2'-O-methyluridine-3'-phosphate
  modified_base 15: mod_base = OTHER; note = 2'-O-methyladenosine-3'-phosphate
  modified_base 16: mod_base = OTHER; note = 2'-O-methyladenosine-3'-phosphate
  modified_base 17: mod_base = OTHER; note = 2'-O-methyluridine-3'-phosphate
  modified_base 18: mod_base = OTHER; note = 2'-O-methylcytidine-3'-phosphate
  modified_base 19: mod_base = OTHER; note = 2'-O-methyladenosine-3'-phosphate
  modified_base 20: mod_base = OTHER; note = 2'-O-methyladenosine-3'-phosphate
  modified_base 21: mod_base = OTHER; note = 2'-O-methyluridine-3'-phosphate ((2S,4R)-1-[29-[[2-(acetylamino)-2-deoxy-beta-D-galactopyranosyl]oxy]-14,14-bis[[3-[[3-[[5-[[2-(acetylamino)-2-deoxy-beta-D-galactopyranosyl]oxy]-1-oxopentyl]amino]propyl]amino]-3-oxopropoxy]methyl]-1,12,19,25-tetraoxo-16-oxa-13,20,24-triazanonacos-1-yl]-4-hydroxy-2-pyrrolidinyl)methyl ester
aactgagatattgtaatcaat

SEQ ID NO: 355 - RNA, 21 nt, synthetic construct
  source 1..21: mol_type = other RNA
  modified_base 1: mod_base = OTHER; note = 2'-O-methyluridine-3'-phosphorothioate
  modified_base 2: mod_base = OTHER; note = 2'-O-methyladenosine-3'-phosphorothioate
  modified_base 3: mod_base = OTHER; note = 2'-O-methyladenosine-3'-phosphate
  modified_base 4: mod_base = OTHER; note = 2'-O-methylcytidine-3'-phosphate
  modified_base 5: mod_base = OTHER; note = 2'-O-methyladenosine-3'-phosphate
  modified_base 6: mod_base = OTHER; note = 2'-O-methyluridine-3'-phosphate
  modified_base 7: mod_base = OTHER; note = 2'-deoxy-2'-fluorocytidine-3'-phosphate
  modified_base 8: mod_base = OTHER; note = 2'-O-methyladenosine-3'-phosphate
  modified_base 9: mod_base = OTHER; note = 2'-deoxy-2'-fluoroguanosine-3'-phosphate
  modified_base 10: mod_base = OTHER; note = 2'-deoxy-2'-fluoroguanosine-3'-phosphate
  modified_base 11: mod_base = OTHER; note = 2'-deoxy-2'-fluoroadenosine-3'-phosphate
  modified_base 12: mod_base = OTHER; note = 2'-O-methyladenosine-3'-phosphate
  modified_base 13: mod_base = OTHER; note = 2'-O-methylguanosine-3'-phosphate
  modified_base 14: mod_base = OTHER; note = 2'-O-methyluridine-3'-phosphate
  modified_base 15: mod_base = OTHER; note = 2'-O-methyluridine-3'-phosphate
  modified_base 16: mod_base = OTHER; note = 2'-O-methyladenosine-3'-phosphate
  modified_base 17: mod_base = OTHER; note = 2'-O-methyladenosine-3'-phosphate
  modified_base 18: mod_base = OTHER; note = 2'-O-methyluridine-3'-phosphate
  modified_base 19: mod_base = OTHER; note = 2'-O-methyluridine-3'-phosphate
  modified_base 20: mod_base = OTHER; note = 2'-O-methyluridine-3'-phosphate
  modified_base 21: mod_base = OTHER; note = 2'-O-methyluridine-3'-phosphate ((2S,4R)-1-[29-[[2-(acetylamino)-2-deoxy-beta-D-galactopyranosyl]oxy]-14,14-bis[[3-[[3-[[5-[[2-(acetylamino)-2-deoxy-beta-D-galactopyranosyl]oxy]-1-oxopentyl]amino]propyl]amino]-3-oxopropoxy]methyl]-1,12,19,25-tetraoxo-16-oxa-13,20,24-triazanonacos-1-yl]-4-hydroxy-2-pyrrolidinyl)methyl ester
taacatcaggaagttaatttt

SEQ ID NO: 356 - RNA, 21 nt, synthetic construct
  source 1..21: mol_type = other RNA
  modified_base 1: mod_base = OTHER; note = 2'-O-methylguanosine-3'-phosphorothioate
  modified_base 2: mod_base = OTHER; note = 2'-O-methylcytidine-3'-phosphorothioate
  modified_base 3: mod_base = OTHER; note = 2'-O-methyladenosine-3'-phosphate
  modified_base 4: mod_base = OTHER; note = 2'-O-methyladenosine-3'-phosphate
  modified_base 5: mod_base = OTHER; note = 2'-O-methyladenosine-3'-phosphate
  modified_base 6: mod_base = OTHER; note = 2'-O-methyladenosine-3'-phosphate
  modified_base 7: mod_base = OTHER; note = 2'-deoxy-2'-fluorouridine-3'-phosphate
  modified_base 8: mod_base = OTHER; note = 2'-O-methyluridine-3'-phosphate
  modified_base 9: mod_base = OTHER; note = 2'-deoxy-2'-fluorocytidine-3'-phosphate
  modified_base 10: mod_base = OTHER; note = 2'-deoxy-2'-fluorouridine-3'-phosphate
  modified_base 11: mod_base = OTHER; note = 2'-deoxy-2'-fluoroadenosine-3'-phosphate
  modified_base 12: mod_base = OTHER; note = 2'-O-methylguanosine-3'-phosphate
  modified_base 13: mod_base = OTHER; note = 2'-O-methylguanosine-3'-phosphate
  modified_base 14: mod_base = OTHER; note = 2'-O-methylguanosine-3'-phosphate
  modified_base 15: mod_base = OTHER; note = 2'-O-methyladenosine-3'-phosphate
  modified_base 16: mod_base = OTHER; note = 2'-O-methyladenosine-3'-phosphate
  modified_base 17: mod_base = OTHER; note = 2'-O-methyladenosine-3'-phosphate
  modified_base 18: mod_base = OTHER; note = 2'-O-methylcytidine-3'-phosphate
  modified_base 19: mod_base = OTHER; note = 2'-O-methyluridine-3'-phosphate
  modified_base 20: mod_base = OTHER; note = 2'-O-methyluridine-3'-phosphate
  modified_base 21: mod_base = OTHER; note = 2'-O-methyluridine-3'-phosphate ((2S,4R)-1-[29-[[2-(acetylamino)-2-deoxy-beta-D-galactopyranosyl]oxy]-14,14-bis[[3-[[3-[[5-[[2-(acetylamino)-2-deoxy-beta-D-galactopyranosyl]oxy]-1-oxopentyl]amino]propyl]amino]-3-oxopropoxy]methyl]-1,12,19,25-tetraoxo-16-oxa-13,20,24-triazanonacos-1-yl]-4-hydroxy-2-pyrrolidinyl)methyl ester
gcaaaattctagggaaacttt

SEQ ID NO: 357 - RNA, 21 nt, synthetic construct
  source 1..21: mol_type = other RNA
  modified_base 1: mod_base = OTHER; note = 2'-O-methyladenosine-3'-phosphorothioate
  modified_base 2: mod_base = OTHER; note = 2'-O-methyladenosine-3'-phosphorothioate
  modified_base 3: mod_base = OTHER; note = 2'-O-methylguanosine-3'-phosphate
  modified_base 4: mod_base = OTHER; note = 2'-O-methylguanosine-3'-phosphate
  modified_base 5: mod_base = OTHER; note = 2'-O-methylcytidine-3'-phosphate
  modified_base 6: mod_base = OTHER; note = 2'-O-methyluridine-3'-phosphate
  modified_base 7: mod_base = OTHER; note = 2'-deoxy-2'-fluorouridine-3'-phosphate
  modified_base 8: mod_base = OTHER; note = 2'-O-methyluridine-3'-phosphate
  modified_base 9: mod_base = OTHER; note = 2'-deoxy-2'-fluorouridine-3'-phosphate
  modified_base 10: mod_base = OTHER; note = 2'-deoxy-2'-fluoroguanosine-3'-phosphate
  modified_base 11: mod_base = OTHER; note = 2'-deoxy-2'-fluorocytidine-3'-phosphate
  modified_base 12: mod_base = OTHER; note = 2'-O-methyluridine-3'-phosphate
  modified_base 13: mod_base = OTHER; note = 2'-O-methylcytidine-3'-phosphate
  modified_base 14: mod_base = OTHER; note = 2'-O-methyladenosine-3'-phosphate
  modified_base 15: mod_base = OTHER; note = 2'-O-methyluridine-3'-phosphate
  modified_base 16: mod_base = OTHER; note = 2'-O-methyladenosine-3'-phosphate
  modified_base 17: mod_base = OTHER; note = 2'-O-methyluridine-3'-phosphate
  modified_base 18: mod_base = OTHER; note = 2'-O-methyladenosine-3'-phosphate
  modified_base 19: mod_base = OTHER; note = 2'-O-methyladenosine-3'-phosphate
  modified_base 20: mod_base = OTHER; note = 2'-O-methyladenosine-3'-phosphate
  modified_base 21: mod_base = OTHER; note = 2'-O-methyluridine-3'-phosphate ((2S,4R)-1-[29-[[2-(acetylamino)-2-deoxy-beta-D-galactopyranosyl]oxy]-14,14-bis[[3-[[3-[[5-[[2-(acetylamino)-2-deoxy-beta-D-galactopyranosyl]oxy]-1-oxopentyl]amino]propyl]amino]-3-oxopropoxy]methyl]-1,12,19,25-tetraoxo-16-oxa-13,20,24-triazanonacos-1-yl]-4-hydroxy-2-pyrrolidinyl)methyl ester
aaggcttttgctcatataaat

SEQ ID NO: 358 - RNA, 21 nt, synthetic construct
  source 1..21: mol_type = other RNA
  modified_base 1: mod_base = OTHER; note = 2'-O-methyluridine-3'-phosphorothioate
  modified_base 2: mod_base = OTHER; note = 2'-O-methylguanosine-3'-phosphorothioate
  modified_base 3: mod_base = OTHER; note = 2'-O-methylcytidine-3'-phosphate
  modified_base 4: mod_base = OTHER; note = 2'-O-methylcytidine-3'-phosphate
  modified_base 5: mod_base = OTHER; note = 2'-O-methyladenosine-3'-phosphate
  modified_base 6: mod_base = OTHER; note = 2'-O-methyluridine-3'-phosphate
  modified_base 7: mod_base = OTHER; note = 2'-deoxy-2'-fluorouridine-3'-phosphate
  modified_base 8: mod_base = OTHER; note = 2'-O-methylguanosine-3'-phosphate
  modified_base 9: mod_base = OTHER; note = 2'-deoxy-2'-fluoroadenosine-3'-phosphate
  modified_base 10: mod_base = OTHER; note = 2'-deoxy-2'-fluoroguanosine-3'-phosphate
  modified_base 11: mod_base = OTHER; note = 2'-deoxy-2'-fluorouridine-3'-phosphate
  modified_base 12: mod_base = OTHER; note = 2'-O-methyluridine-3'-phosphate
  modified_base 13: mod_base = OTHER; note = 2'-O-methyluridine-3'-phosphate
  modified_base 14: mod_base = OTHER; note = 2'-O-methylcytidine-3'-phosphate
  modified_base 15: mod_base = OTHER; note = 2'-O-methyladenosine-3'-phosphate
  modified_base 16: mod_base = OTHER; note = 2'-O-methyladenosine-3'-phosphate
  modified_base 17: mod_base = OTHER; note = 2'-O-methyladenosine-3'-phosphate
  modified_base 18: mod_base = OTHER; note = 2'-O-methyluridine-3'-phosphate
  modified_base 19: mod_base = OTHER; note = 2'-O-methylguanosine-3'-phosphate
  modified_base 20: mod_base = OTHER; note = 2'-O-methyladenosine-3'-phosphate
  modified_base 21: mod_base = OTHER; note = 2'-O-methyluridine-3'-phosphate ((2S,4R)-1-[29-[[2-(acetylamino)-2-deoxy-beta-D-galactopyranosyl]oxy]-14,14-bis[[3-[[3-[[5-[[2-(acetylamino)-2-deoxy-beta-D-galactopyranosyl]oxy]-1-oxopentyl]amino]propyl]amino]-3-oxopropoxy]methyl]-1,12,19,25-tetraoxo-16-oxa-13,20,24-triazanonacos-1-yl]-4-hydroxy-2-pyrrolidinyl)methyl ester
tgccattgagtttcaaatgat

SEQ ID NO: 359 - RNA, 21 nt, synthetic construct
  source 1..21: mol_type = other RNA
  modified_base 1: mod_base = OTHER; note = 2'-O-methylguanosine-3'-phosphorothioate
  modified_base 2: mod_base = OTHER; note = 2'-O-methyladenosine-3'-phosphorothioate
  modified_base 3: mod_base = OTHER; note = 2'-O-methylcytidine-3'-phosphate
  modified_base 4: mod_base = OTHER; note = 2'-O-methylcytidine-3'-phosphate
  modified_base 5: mod_base = OTHER; note = 2'-O-methyladenosine-3'-phosphate
  modified_base 6: mod_base = OTHER; note = 2'-O-methylguanosine-3'-phosphate
  modified_base 7: mod_base = OTHER; note = 2'-deoxy-2'-fluorocytidine-3'-phosphate
  modified_base 8: mod_base = OTHER; note = 2'-O-methyladenosine-3'-phosphate
  modified_base 9: mod_base = OTHER; note = 2'-deoxy-2'-fluoroadenosine-3'-phosphate
  modified_base 10: mod_base = OTHER; note = 2'-deoxy-2'-fluoroadenosine-3'-phosphate
  modified_base 11: mod_base = OTHER; note = 2'-deoxy-2'-fluorouridine-3'-phosphate
  modified_base 12: mod_base = OTHER; note = 2'-O-methyladenosine-3'-phosphate
  modified_base 13: mod_base = OTHER; note = 2'-O-methyluridine-3'-phosphate
  modified_base 14: mod_base = OTHER; note = 2'-O-methyladenosine-3'-phosphate
  modified_base 15: mod_base = OTHER; note = 2'-O-methyluridine-3'-phosphate
  modified_base 16: mod_base = OTHER; note = 2'-O-methyluridine-3'-phosphate
  modified_base 17: mod_base = OTHER; note = 2'-O-methyluridine-3'-phosphate
  modified_base 18: mod_base = OTHER; note = 2'-O-methyladenosine-3'-phosphate
  modified_base 19: mod_base = OTHER; note = 2'-O-methylguanosine-3'-phosphate
  modified_base 20: mod_base = OTHER; note = 2'-O-methyladenosine-3'-phosphate
  modified_base 21: mod_base = OTHER; note = 2'-O-methyluridine-3'-phosphate ((2S,4R)-1-[29-[[2-(acetylamino)-2-deoxy-beta-D-galactopyranosyl]oxy]-14,14-bis[[3-[[3-[[5-[[2-(acetylamino)-2-deoxy-beta-D-galactopyranosyl]oxy]-1-oxopentyl]amino]propyl]amino]-3-oxopropoxy]methyl]-1,12,19,25-tetraoxo-16-oxa-13,20,24-triazanonacos-1-yl]-4-hydroxy-2-pyrrolidinyl)methyl ester
gaccagcaaatatatttagat

SEQ ID NO: 360 - RNA, 21 nt, synthetic construct
  source 1..21: mol_type = other RNA
  modified_base 1: mod_base = OTHER; note = 2'-O-methylcytidine-3'-phosphorothioate
  modified_base 2: mod_base = OTHER; note = 2'-O-methyluridine-3'-phosphorothioate
  modified_base 3: mod_base = OTHER; note = 2'-O-methyluridine-3'-phosphate
  modified_base 4: mod_base = OTHER; note = 2'-O-methylguanosine-3'-phosphate
  modified_base 5: mod_base = OTHER; note = 2'-O-methylguanosine-3'-phosphate
  modified_base 6: mod_base = OTHER; note = 2'-O-methyladenosine-3'-phosphate
  modified_base 7: mod_base = OTHER; note = 2'-deoxy-2'-fluoroadenosine-3'-phosphate
  modified_base 8: mod_base = OTHER; note = 2'-O-methyladenosine-3'-phosphate
  modified_base 9: mod_base = OTHER; note = 2'-deoxy-2'-fluorouridine-3'-phosphate
  modified_base 10: mod_base = OTHER; note = 2'-deoxy-2'-fluorocytidine-3'-phosphate
  modified_base 11: mod_base = OTHER; note = 2'-deoxy-2'-fluorocytidine-3'-phosphate
  modified_base 12: mod_base = OTHER; note = 2'-O-methyluridine-3'-phosphate
  modified_base 13: mod_base = OTHER; note = 2'-O-methylcytidine-3'-phosphate
  modified_base 14: mod_base = OTHER; note = 2'-O-methylcytidine-3'-phosphate
  modified_base 15: mod_base = OTHER; note = 2'-O-methyladenosine-3'-phosphate
  modified_base 16: mod_base = OTHER; note = 2'-O-methyladenosine-3'-phosphate
  modified_base 17: mod_base = OTHER; note = 2'-O-methylcytidine-3'-phosphate
  modified_base 18: mod_base = OTHER; note = 2'-O-methylcytidine-3'-phosphate
  modified_base 19: mod_base = OTHER; note = 2'-O-methyladenosine-3'-phosphate
  modified_base 20: mod_base = OTHER; note = 2'-O-methyladenosine-3'-phosphate
  modified_base 21: mod_base = OTHER; note = 2'-O-methyluridine-3'-phosphate ((2S,4R)-1-[29-[[2-(acetylamino)-2-deoxy-beta-D-galactopyranosyl]oxy]-14,14-bis[[3-[[3-[[5-[[2-(acetylamino)-2-deoxy-beta-D-galactopyranosyl]oxy]-1-oxopentyl]amino]propyl]amino]-3-oxopropoxy]methyl]-1,12,19,25-tetraoxo-16-oxa-13,20,24-triazanonacos-1-yl]-4-hydroxy-2-pyrrolidinyl)methyl ester
cttggaaatcctccaaccaat

SEQ ID NO: 361 - RNA, 21 nt, synthetic construct
  source 1..21: mol_type = other RNA
  modified_base 1: mod_base = OTHER; note = 2'-O-methyladenosine-3'-phosphorothioate
  modified_base 2: mod_base = OTHER; note = 2'-O-methyladenosine-3'-phosphorothioate
  modified_base 3: mod_base = OTHER; note = 2'-O-methyladenosine-3'-phosphate
  modified_base 4: mod_base = OTHER; note = 2'-O-methyluridine-3'-phosphate
  modified_base 5: mod_base = OTHER; note = 2'-O-methyladenosine-3'-phosphate
  modified_base 6: mod_base = OTHER; note = 2'-O-methylguanosine-3'-phosphate
  modified_base 7: mod_base = OTHER; note = 2'-deoxy-2'-fluorocytidine-3'-phosphate
  modified_base 8: mod_base = OTHER; note = 2'-O-methyladenosine-3'-phosphate
  modified_base 9: mod_base = OTHER; note = 2'-deoxy-2'-fluoroguanosine-3'-phosphate
  modified_base 10: mod_base = OTHER; note = 2'-deoxy-2'-fluorouridine-3'-phosphate
  modified_base 11: mod_base = OTHER; note = 2'-deoxy-2'-fluorouridine-3'-phosphate
  modified_base 12: mod_base = OTHER; note = 2'-O-methyluridine-3'-phosphate
  modified_base 13: mod_base = OTHER; note = 2'-O-methyluridine-3'-phosphate
  modified_base 14: mod_base = OTHER; note = 2'-O-methylcytidine-3'-phosphate
  modified_base 15: mod_base = OTHER; note = 2'-O-methylcytidine-3'-phosphate
  modified_base 16: mod_base = OTHER; note = 2'-O-methyluridine-3'-phosphate
  modified_base 17: mod_base = OTHER; note = 2'-O-methyladenosine-3'-phosphate
  modified_base 18: mod_base = OTHER; note = 2'-O-methyladenosine-3'-phosphate
  modified_base 19: mod_base = OTHER; note = 2'-O-methylcytidine-3'-phosphate
  modified_base 20: mod_base = OTHER; note = 2'-O-methyluridine-3'-phosphate
  modified_base 21: mod_base = OTHER; note = 2'-O-methyluridine-3'-phosphate ((2S,4R)-1-[29-[[2-(acetylamino)-2-deoxy-beta-D-galactopyranosyl]oxy]-14,14-bis[[3-[[3-[[5-[[2-(acetylamino)-2-deoxy-beta-D-galactopyranosyl]oxy]-1-oxopentyl]amino]propyl]amino]-3-oxopropoxy]methyl]-1,12,19,25-tetraoxo-16-oxa-13,20,24-triazanonacos-1-yl]-4-hydroxy-2-pyrrolidinyl)methyl ester
aaatagcagttttcctaactt

SEQ ID NO: 362 - RNA, 21 nt, synthetic construct
  source 1..21: mol_type = other RNA
  modified_base 1: mod_base = OTHER; note = 2'-O-methyladenosine-3'-phosphorothioate
  modified_base 2: mod_base = OTHER; note = 2'-O-methylguanosine-3'-phosphorothioate
  modified_base 3: mod_base = OTHER; note = 2'-O-methylcytidine-3'-phosphate
  modified_base 4: mod_base = OTHER; note = 2'-O-methyluridine-3'-phosphate
  modified_base 5: mod_base = OTHER; note = 2'-O-methylguanosine-3'-phosphate
  modified_base 6: mod_base = OTHER; note = 2'-O-methyladenosine-3'-phosphate
  modified_base 7: mod_base = OTHER; note = 2'-deoxy-2'-fluorocytidine-3'-phosphate
  modified_base 8: mod_base = OTHER; note = 2'-O-methyladenosine-3'-phosphate
  modified_base 9: mod_base = OTHER; note = 2'-deoxy-2'-fluoroguanosine-3'-phosphate
  modified_base 10: mod_base = OTHER; note = 2'-deoxy-2'-fluoroadenosine-3'-phosphate
  modified_base 11: mod_base = OTHER; note = 2'-deoxy-2'-fluorocytidine-3'-phosphate
  modified_base 12: mod_base = OTHER; note = 2'-O-methyluridine-3'-phosphate
  modified_base 13: mod_base = OTHER; note = 2'-O-methylguanosine-3'-phosphate
  modified_base 14: mod_base = OTHER; note = 2'-O-methyluridine-3'-phosphate
  modified_base 15: mod_base = OTHER; note = 2'-O-methyluridine-3'-phosphate
  modified_base 16: mod_base = OTHER; note = 2'-O-methyladenosine-3'-phosphate
  modified_base 17: mod_base = OTHER; note = 2'-O-methylguanosine-3'-phosphate
  modified_base 18: mod_base = OTHER; note = 2'-O-methyladenosine-3'-phosphate
  modified_base 19: mod_base = OTHER; note = 2'-O-methyladenosine-3'-phosphate
  modified_base 20: mod_base = OTHER; note = 2'-O-methyluridine-3'-phosphate
  modified_base 21: mod_base = OTHER; note = 2'-O-methyluridine-3'-phosphate ((2S,4R)-1-[29-[[2-(acetylamino)-2-deoxy-beta-D-galactopyranosyl]oxy]-14,14-bis[[3-[[3-[[5-[[2-(acetylamino)-2-deoxy-beta-D-galactopyranosyl]oxy]-1-oxopentyl]amino]propyl]amino]-3-oxopropoxy]methyl]-1,12,19,25-tetraoxo-16-oxa-13,20,24-triazanonacos-1-yl]-4-hydroxy-2-pyrrolidinyl)methyl ester
agctgacagactgttagaatt

SEQ ID NO: 363 - RNA, 21 nt, synthetic construct
  source 1..21: mol_type = other RNA
  modified_base 1: mod_base = OTHER; note = 2'-O-methyluridine-3'-phosphorothioate
  modified_base 2: mod_base = OTHER; note = 2'-O-methyluridine-3'-phosphorothioate
  modified_base 3: mod_base = OTHER; note = 2'-O-methyladenosine-3'-phosphate
  modified_base 4: mod_base = OTHER; note = 2'-O-methylguanosine-3'-phosphate
  modified_base 5: mod_base = OTHER; note = 2'-O-methyladenosine-3'-phosphate
  modified_base 6: mod_base = OTHER; note = 2'-O-methylguanosine-3'-phosphate
  modified_base 7: mod_base = OTHER; note = 2'-deoxy-2'-fluoroguanosine-3'-phosphate
  modified_base 8: mod_base = OTHER; note = 2'-O-methylcytidine-3'-phosphate
  modified_base 9: mod_base = OTHER; note = 2'-deoxy-2'-fluoroadenosine-3'-phosphate
  modified_base 10: mod_base = OTHER; note = 2'-deoxy-2'-fluorouridine-3'-phosphate
  modified_base 11: mod_base = OTHER; note = 2'-deoxy-2'-fluorouridine-3'-phosphate
  modified_base 12: mod_base = OTHER; note = 2'-O-methyluridine-3'-phosphate
  modified_base 13: mod_base = OTHER; note = 2'-O-methyladenosine-3'-phosphate
  modified_base 14: mod_base = OTHER; note = 2'-O-methyluridine-3'-phosphate
  modified_base 15: mod_base = OTHER; note = 2'-O-methylguanosine-3'-phosphate
  modified_base 16: mod_base = OTHER; note = 2'-O-methylguanosine-3'-phosphate
  modified_base 17: mod_base = OTHER; note = 2'-O-methyladenosine-3'-phosphate
  modified_base 18: mod_base = OTHER; note = 2'-O-methyluridine-3'-phosphate
  modified_base 19: mod_base = OTHER; note = 2'-O-methyluridine-3'-phosphate
  modified_base 20: mod_base = OTHER; note = 2'-O-methyluridine-3'-phosphate
  modified_base 21: mod_base = OTHER; note = 2'-O-methyluridine-3'-phosphate ((2S,4R)-1-[29-[[2-(acetylamino)-2-deoxy-beta-D-galactopyranosyl]oxy]-14,14-bis[[3-[[3-[[5-[[2-(acetylamino)-2-deoxy-beta-D-galactopyranosyl]oxy]-1-oxopentyl]amino]propyl]amino]-3-oxopropoxy]methyl]-1,12,19,25-tetraoxo-16-oxa-13,20,24-triazanonacos-1-yl]-4-hydroxy-2-pyrrolidinyl)methyl ester
ttagaggcatttatggatttt

SEQ ID NO: 364 - RNA, 21 nt, synthetic construct
  source 1..21: mol_type = other RNA
  modified_base 1: mod_base = OTHER; note = 2'-O-methyluridine-3'-phosphorothioate
  modified_base 2: mod_base = OTHER; note = 2'-O-methyladenosine-3'-phosphorothioate
  modified_base 3: mod_base = OTHER; note = 2'-O-methyluridine-3'-phosphate
  modified_base 4: mod_base = OTHER; note = 2'-O-methylguanosine-3'-phosphate
  modified_base 5: mod_base = OTHER; note = 2'-O-methylguanosine-3'-phosphate
  modified_base 6: mod_base = OTHER; note = 2'-O-methylguanosine-3'-phosphate
  modified_base 7: mod_base = OTHER; note = 2'-deoxy-2'-fluorouridine-3'-phosphate
  modified_base 8: mod_base = OTHER; note = 2'-O-methyluridine-3'-phosphate
  modified_base 9: mod_base = OTHER; note = 2'-deoxy-2'-fluoroadenosine-3'-phosphate
  modified_base 10: mod_base = OTHER; note = 2'-deoxy-2'-fluorouridine-3'-phosphate
  modified_base 11: mod_base = OTHER; note = 2'-deoxy-2'-fluoroadenosine-3'-phosphate
  modified_base 12: mod_base = OTHER; note = 2'-O-methyluridine-3'-phosphate
  modified_base 13: mod_base = OTHER; note = 2'-O-methylguanosine-3'-phosphate
  modified_base 14: mod_base = OTHER; note = 2'-O-methylcytidine-3'-phosphate
  modified_base 15: mod_base = OTHER; note = 2'-O-methylcytidine-3'-phosphate
  modified_base 16: mod_base = OTHER; note = 2'-O-methyluridine-3'-phosphate
  modified_base 17: mod_base = OTHER; note = 2'-O-methyladenosine-3'-phosphate
  modified_base 18: mod_base = OTHER; note = 2'-O-methyladenosine-3'-phosphate
  modified_base 19: mod_base = OTHER; note = 2'-O-methyladenosine-3'-phosphate
  modified_base 20: mod_base = OTHER; note = 2'-O-methylcytidine-3'-phosphate
  modified_base 21: mod_base = OTHER; note = 2'-O-methyluridine-3'-phosphate ((2S,4R)-1-[29-[[2-(acetylamino)-2-deoxy-beta-D-galactopyranosyl]oxy]-14,14-bis[[3-[[3-[[5-[[2-(acetylamino)-2-deoxy-beta-D-galactopyranosyl]oxy]-1-oxopentyl]amino]propyl]amino]-3-oxopropoxy]methyl]-1,12,19,25-tetraoxo-16-oxa-13,20,24-triazanonacos-1-yl]-4-hydroxy-2-pyrrolidinyl)methyl ester
tatgggttatatgcctaaact

SEQ ID NO: 365 - RNA, 21 nt, synthetic construct
  source 1..21: mol_type = other RNA
  modified_base 1: mod_base = OTHER; note = 2'-O-methylcytidine-3'-phosphorothioate
  modified_base 2: mod_base = OTHER; note = 2'-O-methylcytidine-3'-phosphorothioate
  modified_base 3: mod_base = OTHER; note = 2'-O-methyladenosine-3'-phosphate
  modified_base 4: mod_base = OTHER; note = 2'-O-methylcytidine-3'-phosphate
  modified_base 5: mod_base = OTHER; note = 2'-O-methyladenosine-3'-phosphate
  modified_base 6: mod_base = OTHER; note = 2'-O-methyluridine-3'-phosphate
  modified_base 7: mod_base = OTHER; note = 2'-deoxy-2'-fluoroadenosine-3'-phosphate
  modified_base 8: mod_base = OTHER; note = 2'-O-methylguanosine-3'-phosphate
  modified_base 9: mod_base = OTHER; note = 2'-deoxy-2'-fluorouridine-3'-phosphate
  modified_base 10: mod_base = OTHER; note = 2'-deoxy-2'-fluoroguanosine-3'-phosphate
  modified_base 11: mod_base = OTHER; note = 2'-deoxy-2'-fluoroguanosine-3'-phosphate
  modified_base 12: mod_base = OTHER; note = 2'-O-methyluridine-3'-phosphate
  modified_base 13: mod_base = OTHER; note = 2'-O-methyladenosine-3'-phosphate
  modified_base 14: mod_base = OTHER; note = 2'-O-methyladenosine-3'-phosphate
  modified_base 15: mod_base = OTHER; note = 2'-O-methyladenosine-3'-phosphate
  modified_base 16: mod_base = OTHER; note = 2'-O-methyluridine-3'-phosphate
  modified_base 17: mod_base = OTHER; note = 2'-O-methyladenosine-3'-phosphate
  modified_base 18: mod_base = OTHER; note = 2'-O-methyladenosine-3'-phosphate
  modified_base 19: mod_base = OTHER; note = 2'-O-methyluridine-3'-phosphate
  modified_base 20: mod_base = OTHER; note = 2'-O-methyluridine-3'-phosphate
  modified_base 21: mod_base = OTHER; note = 2'-O-methyluridine-3'-phosphate ((2S,4R)-1-[29-[[2-(acetylamino)-2-deoxy-beta-D-galactopyranosyl]oxy]-14,14-bis[[3-[[3-[[5-[[2-(acetylamino)-2-deoxy-beta-D-galactopyranosyl]oxy]-1-oxopentyl]amino]propyl]amino]-3-oxopropoxy]methyl]-1,12,19,25-tetraoxo-16-oxa-13,20,24-triazanonacos-1-yl]-4-hydroxy-2-pyrrolidinyl)methyl ester
ccacatagtggtaaataattt

SEQ ID NO: 366 - RNA, 21 nt, synthetic construct
  source 1..21: mol_type = other RNA
  modified_base 1: mod_base = OTHER; note = 2'-O-methyluridine-3'-phosphorothioate
  modified_base 2: mod_base = OTHER; note = 2'-O-methylguanosine-3'-phosphorothioate
  modified_base 3: mod_base = OTHER; note = 2'-O-methylguanosine-3'-phosphate
  modified_base 4: mod_base = OTHER; note = 2'-O-methyluridine-3'-phosphate
  modified_base 5: mod_base = OTHER; note = 2'-O-methylcytidine-3'-phosphate
  modified_base 6: mod_base = OTHER; note = 2'-O-methyluridine-3'-phosphate
  modified_base 7: mod_base = OTHER; note = 2'-deoxy-2'-fluoroguanosine-3'-phosphate
  modified_base 8: mod_base = OTHER; note = 2'-O-methyluridine-3'-phosphate
  modified_base 9: mod_base = OTHER; note = 2'-deoxy-2'-fluorouridine-3'-phosphate
  modified_base 10: mod_base = OTHER; note = 2'-deoxy-2'-fluorocytidine-3'-phosphate
  modified_base 11: mod_base = OTHER; note = 2'-deoxy-2'-fluoroadenosine-3'-phosphate
  modified_base 12: mod_base = OTHER; note = 2'-O-methyluridine-3'-phosphate
  modified_base 13: mod_base = OTHER; note = 2'-O-methyladenosine-3'-phosphate
  modified_base 14: mod_base = OTHER; note = 2'-O-methyladenosine-3'-phosphate
  modified_base 15: mod_base = OTHER; note = 2'-O-methyluridine-3'-phosphate
  modified_base 16: mod_base = OTHER; note = 2'-O-methyluridine-3'-phosphate
  modified_base 17: mod_base = OTHER; note = 2'-O-methylguanosine-3'-phosphate
  modified_base 18: mod_base = OTHER; note = 2'-O-methylguanosine-3'-phosphate
  modified_base 19: mod_base = OTHER; note = 2'-O-methyluridine-3'-phosphate
  modified_base 20: mod_base = OTHER; note = 2'-O-methyladenosine-3'-phosphate
  modified_base 21: mod_base = OTHER; note = 2'-O-methyluridine-3'-phosphate ((2S,4R)-1-[29-[[2-(acetylamino)-2-deoxy-beta-D-galactopyranosyl]oxy]-14,14-bis[[3-[[3-[[5-[[2-(acetylamino)-2-deoxy-beta-D-galactopyranosyl]oxy]-1-oxopentyl]amino]propyl]amino]-3-oxopropoxy]methyl]-1,12,19,25-tetraoxo-16-oxa-13,20,24-triazanonacos-1-yl]-4-hydroxy-2-pyrrolidinyl)methyl ester
tggtctgttcataattggtat

SEQ ID NO: 367 - RNA, 21 nt, synthetic construct
  source 1..21: mol_type = other RNA
  modified_base 1: mod_base = OTHER; note = 2'-O-methylguanosine-3'-phosphorothioate
  modified_base 2: mod_base = OTHER; note = 2'-O-methyladenosine-3'-phosphorothioate
  modified_base 3: mod_base = OTHER; note = 2'-O-methylguanosine-3'-phosphate
  modified_base 4: mod_base = OTHER; note = 2'-O-methylcytidine-3'-phosphate
  modified_base 5: mod_base = OTHER; note = 2'-O-methyladenosine-3'-phosphate
  modified_base 6: mod_base = OTHER; note = 2'-O-methyluridine-3'-phosphate
  modified_base 7: mod_base = OTHER; note = 2'-deoxy-2'-fluoroadenosine-3'-phosphate
  modified_base 8: mod_base = OTHER; note = 2'-O-methyladenosine-3'-phosphate
  modified_base 9: mod_base = OTHER; note = 2'-deoxy-2'-fluorouridine-3'-phosphate
  modified_base 10: mod_base = OTHER; note = 2'-deoxy-2'-fluorouridine-3'-phosphate
  modified_base 11: mod_base = OTHER; note = 2'-deoxy-2'-fluoroadenosine-3'-phosphate
  modified_base 12: mod_base = OTHER; note = 2'-O-methyluridine-3'-phosphate
  modified_base 13: mod_base = OTHER; note = 2'-O-methyluridine-3'-phosphate
  modified_base 14: mod_base = OTHER; note = 2'-O-methylguanosine-3'-phosphate
  modified_base 15: mod_base = OTHER; note = 2'-O-methylguanosine-3'-phosphate
  modified_base 16: mod_base = OTHER; note = 2'-O-methyluridine-3'-phosphate
  modified_base 17: mod_base = OTHER; note = 2'-O-methyluridine-3'-phosphate
  modified_base 18: mod_base = OTHER; note = 2'-O-methyluridine-3'-phosphate
  modified_base 19: mod_base = OTHER; note = 2'-O-methyladenosine-3'-phosphate
  modified_base 20: mod_base = OTHER; note = 2'-O-methyluridine-3'-phosphate
  modified_base 21: mod_base = OTHER; note = 2'-O-methyluridine-3'-phosphate ((2S,4R)-1-[29-[[2-(acetylamino)-2-deoxy-beta-D-galactopyranosyl]oxy]-14,14-bis[[3-[[3-[[5-[[2-(acetylamino)-2-deoxy-beta-D-galactopyranosyl]oxy]-1-oxopentyl]amino]propyl]amino]-3-oxopropoxy]methyl]-1,12,19,25-tetraoxo-16-oxa-13,20,24-triazanonacos-1-yl]-4-hydroxy-2-pyrrolidinyl)methyl ester
gagcataattattggtttatt

SEQ ID NO: 368 - RNA, 21 nt, synthetic construct
  source 1..21: mol_type = other RNA
  modified_base 1: mod_base = OTHER; note = 2'-O-methyluridine-3'-phosphorothioate
  modified_base 2: mod_base = OTHER; note = 2'-O-methyluridine-3'-phosphorothioate
  modified_base 3: mod_base = OTHER; note = 2'-O-methyluridine-3'-phosphate
  modified_base 4: mod_base = OTHER; note = 2'-O-methyladenosine-3'-phosphate
  modified_base 5: mod_base = OTHER; note = 2'-O-methyluridine-3'-phosphate
  modified_base 6: mod_base = OTHER; note = 2'-O-methyluridine-3'-phosphate
  modified_base 7: mod_base = OTHER; note = 2'-deoxy-2'-fluoroadenosine-3'-phosphate
  modified_base 8: mod_base = OTHER; note = 2'-O-methyluridine-3'-phosphate
  modified_base 9: mod_base = OTHER; note = 2'-deoxy-2'-fluoroguanosine-3'-phosphate
  modified_base 10: mod_base = OTHER; note = 2'-deoxy-2'-fluoroguanosine-3'-phosphate
  modified_base 11: mod_base = OTHER; note = 2'-deoxy-2'-fluorouridine-3'-phosphate
  modified_base 12: mod_base = OTHER; note = 2'-O-methyladenosine-3'-phosphate
  modified_base 13: mod_base = OTHER; note = 2'-O-methyladenosine-3'-phosphate
  modified_base 14: mod_base = OTHER; note = 2'-O-methyluridine-3'-phosphate
  modified_base 15: mod_base = OTHER; note = 2'-O-methyluridine-3'-phosphate
  modified_base 16: mod_base = OTHER; note = 2'-O-methyladenosine-3'-phosphate
  modified_base 17: mod_base = OTHER; note = 2'-O-methyluridine-3'-phosphate
  modified_base 18: mod_base = OTHER; note = 2'-O-methylguanosine-3'-phosphate
  modified_base 19: mod_base = OTHER; note = 2'-O-methylguanosine-3'-phosphate
  modified_base 20: mod_base = OTHER; note = 2'-O-methyluridine-3'-phosphate
  modified_base 21: mod_base = OTHER; note = 2'-O-methyluridine-3'-phosphate ((2S,4R)-1-[29-[[2-(acetylamino)-2-deoxy-beta-D-galactopyranosyl]oxy]-14,14-bis[[3-[[3-[[5-[[2-(acetylamino)-2-deoxy-beta-D-galactopyranosyl]oxy]-1-oxopentyl]amino]propyl]amino]-3-oxopropoxy]methyl]-1,12,19,25-tetraoxo-16-oxa-13,20,24-triazanonacos-1-yl]-4-hydroxy-2-pyrrolidinyl)methyl ester
tttattatggtaattatggtt

SEQ ID NO: 369 - RNA, 21 nt, synthetic construct
  source 1..21: mol_type = other RNA
  modified_base 1: mod_base = OTHER; note = 2'-O-methyluridine-3'-phosphorothioate
  modified_base 2: mod_base = OTHER; note = 2'-O-methyladenosine-3'-phosphorothioate
  modified_base 3: mod_base = OTHER; note = 2'-O-methyladenosine-3'-phosphate
  modified_base 4: mod_base = OTHER; note = 2'-O-methyladenosine-3'-phosphate
  modified_base 5: mod_base = OTHER; note = 2'-O-methyladenosine-3'-phosphate
  modified_base 6: mod_base = OTHER; note = 2'-O-methylcytidine-3'-phosphate
  modified_base 7: mod_base = OTHER; note = 2'-deoxy-2'-fluoroguanosine-3'-phosphate
  modified_base 8: mod_base = OTHER; note = 2'-O-methyluridine-3'-phosphate
  modified_base 9: mod_base = OTHER; note = 2'-deoxy-2'-fluorouridine-3'-phosphate
  modified_base 10: mod_base = OTHER; note = 2'-deoxy-2'-fluorouridine-3'-phosphate
  modified_base 11: mod_base = OTHER; note = 2'-deoxy-2'-fluorouridine-3'-phosphate
  modified_base 12: mod_base = OTHER; note = 2'-O-methylcytidine-3'-phosphate
  modified_base 13: mod_base = OTHER; note = 2'-O-methyluridine-3'-phosphate
  modified_base 14: mod_base = OTHER; note = 2'-O-methyladenosine-3'-phosphate
  modified_base 15: mod_base = OTHER; note = 2'-O-methyladenosine-3'-phosphate
  modified_base 16: mod_base = OTHER; note = 2'-O-methylcytidine-3'-phosphate
  modified_base 17: mod_base = OTHER; note = 2'-O-methyladenosine-3'-phosphate
  modified_base 18: mod_base = OTHER; note = 2'-O-methylguanosine-3'-phosphate
  modified_base 19: mod_base = OTHER; note = 2'-O-methyluridine-3'-phosphate
  modified_base 20: mod_base = OTHER; note = 2'-O-methyluridine-3'-phosphate
  modified_base 21: mod_base = OTHER; note = 2'-O-methyluridine-3'-phosphate ((2S,4R)-1-[29-[[2-(acetylamino)-2-deoxy-beta-D-galactopyranosyl]oxy]-14,14-bis[[3-[[3-[[5-[[2-(acetylamino)-2-deoxy-beta-D-galactopyranosyl]oxy]-1-oxopentyl]amino]propyl]amino]-3-oxopropoxy]methyl]-1,12,19,25-tetraoxo-16-oxa-13,20,24-triazanonacos-1-yl]-4-hydroxy-2-pyrrolidinyl)methyl ester
taaaacgttttctaacagttt

SEQ ID NO: 370 - RNA, 21 nt, synthetic construct
  source 1..21: mol_type = other RNA
  modified_base 1: mod_base = OTHER; note = 2'-O-methylcytidine-3'-phosphorothioate
  modified_base 2: mod_base = OTHER; note = 2'-O-methyluridine-3'-phosphorothioate
  modified_base 3: mod_base = OTHER; note = 2'-O-methylcytidine-3'-phosphate
  modified_base 4: mod_base = OTHER; note = 2'-O-methylcytidine-3'-phosphate
  modified_base 5: mod_base = OTHER; note = 2'-O-methyladenosine-3'-phosphate
  modified_base 6: mod_base = OTHER; note = 2'-O-methyladenosine-3'-phosphate
  modified_base 7: mod_base = OTHER; note = 2'-deoxy-2'-fluoroguanosine-3'-phosphate
  modified_base 8: mod_base = OTHER; note = 2'-O-methyladenosine-3'-phosphate
  modified_base 9: mod_base = OTHER; note = 2'-deoxy-2'-fluorouridine-3'-phosphate
  modified_base 10: mod_base = OTHER; note = 2'-deoxy-2'-fluoroadenosine-3'-phosphate
  modified_base 11: mod_base = OTHER; note = 2'-deoxy-2'-fluorouridine-3'-phosphate
  modified_base 12: mod_base = OTHER; note = 2'-O-methyluridine-3'-phosphate
  modified_base 13: mod_base = OTHER; note = 2'-O-methyladenosine-3'-phosphate
  modified_base 14: mod_base = OTHER; note = 2'-O-methyluridine-3'-phosphate
  modified_base 15: mod_base = OTHER; note = 2'-O-methylguanosine-3'-phosphate
  modified_base 16: mod_base = OTHER; note = 2'-O-methylguanosine-3'-phosphate
  modified_base 17: mod_base = OTHER; note = 2'-O-methyladenosine-3'-phosphate
  modified_base 18: mod_base = OTHER; note = 2'-O-methyladenosine-3'-phosphate
  modified_base 19: mod_base = OTHER; note = 2'-O-methyluridine-3'-phosphate
  modified_base 20: mod_base = OTHER; note = 2'-O-methyluridine-3'-phosphate
  modified_base 21: mod_base = OTHER; note = 2'-O-methyluridine-3'-phosphate ((2S,4R)-1-[29-[[2-(acetylamino)-2-deoxy-beta-D-galactopyranosyl]oxy]-14,14-bis[[3-[[3-[[5-[[2-(acetylamino)-2-deoxy-beta-D-galactopyranosyl]oxy]-1-oxopentyl]amino]propyl]amino]-3-oxopropoxy]methyl]-1,12,19,25-tetraoxo-16-oxa-13,20,24-triazanonacos-1-yl]-4-hydroxy-2-pyrrolidinyl)methyl ester
ctccaagatattatggaattt

SEQ ID NO: 371 - RNA, 21 nt, synthetic construct
  source 1..21: mol_type = other RNA
  modified_base 1: mod_base = OTHER; note = 2'-O-methyluridine-3'-phosphorothioate
  modified_base 2: mod_base = OTHER; note = 2'-O-methylguanosine-3'-phosphorothioate
  modified_base 3: mod_base = OTHER; note = 2'-O-methyladenosine-3'-phosphate
  modified_base 4: mod_base = OTHER; note = 2'-O-methylguanosine-3'-phosphate
  modified_base 5: mod_base = OTHER; note = 2'-O-methyluridine-3'-phosphate
  modified_base 6: mod_base = OTHER; note = 2'-O-methylguanosine-3'-phosphate
  modified_base 7: mod_base = OTHER; note = 2'-deoxy-2'-fluorouridine-3'-phosphate
  modified_base 8: mod_base = OTHER; note = 2'-O-methyluridine-3'-phosphate
  modified_base 9: mod_base = OTHER; note = 2'-deoxy-2'-fluoroadenosine-3'-phosphate
  modified_base 10: mod_base = OTHER; note = 2'-deoxy-2'-fluorocytidine-3'-phosphate
  modified_base 11: mod_base = OTHER; note = 2'-deoxy-2'-fluoroadenosine-3'-phosphate
  modified_base 12: mod_base = OTHER; note = 2'-O-methyluridine-3'-phosphate
  modified_base 13: mod_base = OTHER; note = 2'-O-methyladenosine-3'-phosphate
  modified_base 14: mod_base = OTHER; note = 2'-O-methylguanosine-3'-phosphate
  modified_base 15: mod_base = OTHER; note = 2'-O-methyladenosine-3'-phosphate
  modified_base 16: mod_base = OTHER; note = 2'-O-methyluridine-3'-phosphate
  modified_base 17: mod_base = OTHER; note = 2'-O-methyluridine-3'-phosphate
  modified_base 18: mod_base = OTHER; note = 2'-O-methylcytidine-3'-phosphate
  modified_base 19: mod_base = OTHER; note = 2'-O-methyluridine-3'-phosphate
  modified_base 20: mod_base = OTHER; note = 2'-O-methyluridine-3'-phosphate
  modified_base 21: mod_base = OTHER; note = 2'-O-methyluridine-3'-phosphate ((2S,4R)-1-[29-[[2-(acetylamino)-2-deoxy-beta-D-galactopyranosyl]oxy]-14,14-bis[[3-[[3-[[5-[[2-(acetylamino)-2-deoxy-beta-D-galactopyranosyl]oxy]-1-oxopentyl]amino]propyl]amino]-3-oxopropoxy]methyl]-1,12,19,25-tetraoxo-16-oxa-13,20,24-triazanonacos-1-yl]-4-hydroxy-2-pyrrolidinyl)methyl ester
tgagtgttacatagattcttt

SEQ ID NO: 372 - RNA, 21 nt, synthetic construct
  source 1..21: mol_type = other RNA
  modified_base 1: mod_base = OTHER; note = 2'-O-methyladenosine-3'-phosphorothioate
  modified_base 2: mod_base = OTHER; note = 2'-O-methylguanosine-3'-phosphorothioate
  modified_base 3: mod_base = OTHER; note = 2'-O-methyluridine-3'-phosphate
  modified_base 4: mod_base = OTHER; note = 2'-O-methyladenosine-3'-phosphate
  modified_base 5: mod_base = OTHER; note = 2'-O-methylcytidine-3'-phosphate
  modified_base 6: mod_base = OTHER; note = 2'-O-methyluridine-3'-phosphate
  modified_base 7: mod_base = OTHER; note = 2'-deoxy-2'-fluoroguanosine-3'-phosphate
  modified_base 8: mod_base = OTHER; note = 2'-O-methyladenosine-3'-phosphate
  modified_base 9: mod_base = OTHER; note = 2'-deoxy-2'-fluoroguanosine-3'-phosphate
  modified_base 10: mod_base = OTHER; note = 2'-deoxy-2'-fluoroadenosine-3'-phosphate
  modified_base 11: mod_base = OTHER; note = 2'-deoxy-2'-fluoroadenosine-3'-phosphate
  modified_base 12: mod_base = OTHER; note = 2'-O-methyluridine-3'-phosphate
  modified_base 13: mod_base = OTHER; note = 2'-O-methyluridine-3'-phosphate
  modified_base 14: mod_base = OTHER; note = 2'-O-methyladenosine-3'-phosphate
  modified_base 15: mod_base = OTHER; note = 2'-O-methyladenosine-3'-phosphate
  modified_base 16: mod_base = OTHER; note = 2'-O-methylguanosine-3'-phosphate
  modified_base 17: mod_base = OTHER; note = 2'-O-methyluridine-3'-phosphate
  modified_base 18: mod_base = OTHER; note = 2'-O-methyluridine-3'-phosphate
  modified_base 19: mod_base = OTHER; note = 2'-O-methyluridine-3'-phosphate
  modified_base 20: mod_base = OTHER; note = 2'-O-methylguanosine-3'-phosphate
  modified_base 21: mod_base = OTHER; note = 2'-O-methyluridine-3'-phosphate ((2S,4R)-1-[29-[[2-(acetylamino)-2-deoxy-beta-D-galactopyranosyl]oxy]-14,14-bis[[3-[[3-[[5-[[2-(acetylamino)-2-deoxy-beta-D-galactopyranosyl]oxy]-1-oxopentyl]amino]propyl]amino]-3-oxopropoxy]methyl]-1,12,19,25-tetraoxo-16-oxa-13,20,24-triazanonacos-1-yl]-4-hydroxy-2-pyrrolidinyl)methyl ester
agtactgagaattaagtttgt

SEQ ID NO: 373 - RNA, 21 nt, synthetic construct
  source 1..21: mol_type = other RNA
  modified_base 1: mod_base = OTHER; note = 2'-O-methyladenosine-3'-phosphorothioate
  modified_base 2: mod_base = OTHER; note = 2'-O-methyluridine-3'-phosphorothioate
  modified_base 3: mod_base = OTHER; note = 2'-O-methyluridine-3'-phosphate
  modified_base 4: mod_base = OTHER; note = 2'-O-methyluridine-3'-phosphate
  modified_base 5: mod_base = OTHER; note = 2'-O-methyluridine-3'-phosphate
  modified_base 6: mod_base = OTHER; note = 2'-O-methyladenosine-3'-phosphate
  modified_base 7: mod_base = OTHER; note = 2'-deoxy-2'-fluoroadenosine-3'-phosphate
  modified_base 8: mod_base = OTHER; note = 2'-O-methyladenosine-3'-phosphate
  modified_base 9: mod_base = OTHER; note = 2'-deoxy-2'-fluorocytidine-3'-phosphate
  modified_base 10: mod_base = OTHER; note = 2'-deoxy-2'-fluoroadenosine-3'-phosphate
  modified_base 11: mod_base = OTHER; note = 2'-deoxy-2'-fluorocytidine-3'-phosphate
  modified_base 12: mod_base = OTHER; note = 2'-O-methyluridine-3'-phosphate
  modified_base 13: mod_base = OTHER; note = 2'-O-methylguanosine-3'-phosphate
  modified_base 14: mod_base = OTHER; note = 2'-O-methyladenosine-3'-phosphate
  modified_base 15: mod_base = OTHER; note = 2'-O-methyluridine-3'-phosphate
  modified_base 16: mod_base = OTHER; note = 2'-O-methyladenosine-3'-phosphate
  modified_base 17: mod_base = OTHER; note = 2'-O-methylguanosine-3'-phosphate
  modified_base 18: mod_base = OTHER; note = 2'-O-methyluridine-3'-phosphate
  modified_base 19: mod_base = OTHER; note = 2'-O-methyladenosine-3'-phosphate
  modified_base 20: mod_base = OTHER; note = 2'-O-methyluridine-3'-phosphate
  modified_base 21: mod_base = OTHER; note = 2'-O-methyluridine-3'-phosphate ((2S,4R)-1-[29-[[2-(acetylamino)-2-deoxy-beta-D-galactopyranosyl]oxy]-14,14-bis[[3-[[3-[[5-[[2-(acetylamino)-2-deoxy-beta-D-galactopyranosyl]oxy]-1-oxopentyl]amino]propyl]amino]-3-oxopropoxy]methyl]-1,12,19,25-tetraoxo-16-oxa-13,20,24-triazanonacos-1-yl]-4-hydroxy-2-pyrrolidinyl)methyl ester
attttaaacactgatagtatt

SEQ ID NO: 374 - RNA, 21 nt, synthetic construct
  source 1..21: mol_type = other RNA
  modified_base 1: mod_base = OTHER; note = 2'-O-methylcytidine-3'-phosphorothioate
  modified_base 2: mod_base = OTHER; note = 2'-O-methyluridine-3'-phosphorothioate
  modified_base 3: mod_base = OTHER; note = 2'-O-methylcytidine-3'-phosphate
  modified_base 4: mod_base = OTHER; note = 2'-O-methyladenosine-3'-phosphate
  modified_base 5: mod_base = OTHER; note = 2'-O-methyluridine-3'-phosphate
  modified_base 6: mod_base = OTHER; note = 2'-O-methylguanosine-3'-phosphate
  modified_base 7: mod_base = OTHER; note = 2'-deoxy-2'-fluoroadenosine-3'-phosphate
  modified_base 8: mod_base = OTHER; note = 2'-O-methylguanosine-3'-phosphate
  modified_base 9: mod_base = OTHER; note = 2'-deoxy-2'-fluorouridine-3'-phosphate
  modified_base 10: mod_base = OTHER; note = 2'-deoxy-2'-fluoroadenosine-3'-phosphate
  modified_base 11: mod_base = OTHER; note = 2'-deoxy-2'-fluoroadenosine-3'-phosphate
  modified_base 12: mod_base = OTHER; note = 2'-O-methyluridine-3'-phosphate
  modified_base 13: mod_base = OTHER; note = 2'-O-methylguanosine-3'-phosphate
  modified_base 14: mod_base = OTHER; note = 2'-O-methyluridine-3'-phosphate
  modified_base 15: mod_base = OTHER; note = 2'-O-methylguanosine-3'-phosphate
  modified_base 16: mod_base = OTHER; note = 2'-O-methyluridine-3'-phosphate
  modified_base 17: mod_base = OTHER; note = 2'-O-methylguanosine-3'-phosphate
  modified_base 18: mod_base = OTHER; note = 2'-O-methyluridine-3'-phosphate
  modified_base 19: mod_base = OTHER; note = 2'-O-methyluridine-3'-phosphate
  modified_base 20: mod_base = OTHER; note = 2'-O-methyluridine-3'-phosphate
  modified_base 21: mod_base = OTHER; note = 2'-O-methyluridine-3'-phosphate ((2S,4R)-1-[29-[[2-(acetylamino)-2-deoxy-beta-D-galactopyranosyl]oxy]-14,14-bis[[3-[[3-[[5-[[2-(acetylamino)-2-deoxy-beta-D-galactopyranosyl]oxy]-1-oxopentyl]amino]propyl]amino]-3-oxopropoxy]methyl]-1,12,19,25-tetraoxo-16-oxa-13,20,24-triazanonacos-1-yl]-4-hydroxy-2-pyrrolidinyl)methyl ester
ctcatgagtaatgtgtgtttt

SEQ ID NO: 375 - RNA, 21 nt, synthetic construct
  source 1..21: mol_type = other RNA
  modified_base 1: mod_base = OTHER; note = 2'-O-methyladenosine-3'-phosphorothioate
  modified_base 2: mod_base = OTHER; note = 2'-O-methyluridine-3'-phosphorothioate
  modified_base 3: mod_base = OTHER; note = 2'-O-methylguanosine-3'-phosphate
  modified_base 4: mod_base = OTHER; note = 2'-O-methylcytidine-3'-phosphate
  modified_base 5: mod_base = OTHER; note = 2'-O-methyluridine-3'-phosphate
  modified_base 6: mod_base = OTHER; note = 2'-O-methylguanosine-3'-phosphate
  modified_base 7: mod_base = OTHER; note = 2'-deoxy-2'-fluoroadenosine-3'-phosphate
  modified_base 8: mod_base = OTHER; note = 2'-O-methyluridine-3'-phosphate
  modified_base 9: mod_base = OTHER; note = 2'-deoxy-2'-fluorouridine-3'-phosphate
  modified_base 10: mod_base = OTHER; note = 2'-deoxy-2'-fluoroguanosine-3'-phosphate
  modified_base 11: mod_base = OTHER; note = 2'-deoxy-2'-fluoroadenosine-3'-phosphate
  modified_base 12: mod_base = OTHER; note = 2'-O-methyluridine-3'-phosphate
  modified_base 13: mod_base = OTHER; note = 2'-O-methyladenosine-3'-phosphate
  modified_base 14: mod_base = OTHER; note = 2'-O-methyluridine-3'-phosphate
  modified_base 15: mod_base = OTHER; note = 2'-O-methyluridine-3'-phosphate
  modified_base 16: mod_base = OTHER; note = 2'-O-methyluridine-3'-phosphate
  modified_base 17: mod_base = OTHER; note = 2'-O-methylcytidine-3'-phosphate
  modified_base 18: mod_base = OTHER; note = 2'-O-methyladenosine-3'-phosphate
  modified_base 19: mod_base = OTHER; note = 2'-O-methylcytidine-3'-phosphate
  modified_base 20: mod_base = OTHER; note = 2'-O-methyladenosine-3'-phosphate
  modified_base 21: mod_base = OTHER; note = 2'-O-methyluridine-3'-phosphate ((2S,4R)-1-[29-[[2-(acetylamino)-2-deoxy-beta-D-galactopyranosyl]oxy]-14,14-bis[[3-[[3-[[5-[[2-(acetylamino)-2-deoxy-beta-D-galactopyranosyl]oxy]-1-oxopentyl]amino]propyl]amino]-3-oxopropoxy]methyl]-1,12,19,25-tetraoxo-16-oxa-13,20,24-triazanonacos-1-yl]-4-hydroxy-2-pyrrolidinyl)methyl ester
atgctgattgatatttcacat

SEQ ID NO: 376 - RNA, 21 nt, synthetic construct
  source 1..21: mol_type = other RNA
  modified_base 1: mod_base = OTHER; note = 2'-O-methyluridine-3'-phosphorothioate
  modified_base 2: mod_base = OTHER; note = 2'-O-methyladenosine-3'-phosphorothioate
  modified_base 3: mod_base = OTHER; note = 2'-O-methyluridine-3'-phosphate
  modified_base 4: mod_base = OTHER; note = 2'-O-methylguanosine-3'-phosphate
  modified_base 5: mod_base = OTHER; note = 2'-O-methyladenosine-3'-phosphate
  modified_base 6: mod_base = OTHER; note = 2'-O-methyladenosine-3'-phosphate
  modified_base 7: mod_base = OTHER; note = 2'-deoxy-2'-fluoroadenosine-3'-phosphate
  modified_base 8: mod_base = OTHER; note = 2'-O-methyluridine-3'-phosphate
  modified_base 9: mod_base = OTHER; note = 2'-deoxy-2'-fluoroadenosine-3'-phosphate
  modified_base 10: mod_base = OTHER; note = 2'-deoxy-2'-fluorocytidine-3'-phosphate
  modified_base 11: mod_base = OTHER; note = 2'-deoxy-2'-fluorocytidine-3'-phosphate
  modified_base 12: mod_base = OTHER; note = 2'-O-methyladenosine-3'-phosphate
  modified_base 13: mod_base = OTHER; note = 2'-O-methyluridine-3'-phosphate
  modified_base 14: mod_base = OTHER; note = 2'-O-methylguanosine-3'-phosphate
  modified_base 15: mod_base = OTHER; note = 2'-O-methyluridine-3'-phosphate
  modified_base 16: mod_base = OTHER; note = 2'-O-methyluridine-3'-phosphate
  modified_base 17: mod_base = OTHER; note = 2'-O-methyluridine-3'-phosphate
  modified_base 18: mod_base = OTHER; note = 2'-O-methylguanosine-3'-phosphate
  modified_base 19: mod_base = OTHER; note = 2'-O-methyladenosine-3'-phosphate
  modified_base 20: mod_base = OTHER; note = 2'-O-methyladenosine-3'-phosphate
  modified_base 21: mod_base = OTHER; note = 2'-O-methyluridine-3'-phosphate ((2S,4R)-1-[29-[[2-(acetylamino)-2-deoxy-beta-D-galactopyranosyl]oxy]-14,14-bis[[3-[[3-[[5-[[2-(acetylamino)-2-deoxy-beta-D-galactopyranosyl]oxy]-1-oxopentyl]amino]propyl]amino]-3-oxopropoxy]methyl]-1,12,19,25-tetraoxo-16-oxa-13,20,24-triazanonacos-1-yl]-4-hydroxy-2-pyrrolidinyl)methyl ester
tatgaaataccatgtttgaat

SEQ ID NO: 377 - RNA, 21 nt, synthetic construct
  source 1..21: mol_type = other RNA
  modified_base 1: mod_base = OTHER; note = 2'-O-methyluridine-3'-phosphorothioate
  modified_base 2: mod_base = OTHER; note = 2'-O-methyluridine-3'-phosphorothioate
  modified_base 3: mod_base = OTHER; note = 2'-O-methylguanosine-3'-phosphate
  modified_base 4: mod_base = OTHER; note = 2'-O-methyladenosine-3'-phosphate
  modified_base 5: mod_base = OTHER; note = 2'-O-methyladenosine-3'-phosphate
  modified_base 6: mod_base = OTHER; note = 2'-O-methyladenosine-3'-phosphate
  modified_base 7: mod_base = OTHER; note = 2'-deoxy-2'-fluorocytidine-3'-phosphate
  modified_base 8: mod_base = OTHER; note = 2'-O-methyluridine-3'-phosphate
  modified_base 9: mod_base = OTHER; note = 2'-deoxy-2'-fluorocytidine-3'-phosphate
  modified_base 10: mod_base = OTHER; note = 2'-deoxy-2'-fluoroadenosine-3'-phosphate
  modified_base 11: mod_base = OTHER; note = 2'-deoxy-2'-fluorouridine-3'-phosphate
  modified_base 12: mod_base = OTHER; note = 2'-O-methyladenosine-3'-phosphate
  modified_base 13: mod_base = OTHER; note = 2'-O-methylguanosine-3'-phosphate
  modified_base 14: mod_base = OTHER; note = 2'-O-methylcytidine-3'-phosphate
  modified_base 15: mod_base = OTHER; note = 2'-O-methyladenosine-3'-phosphate
  modified_base 16: mod_base = OTHER; note = 2'-O-methyladenosine-3'-phosphate
  modified_base 17: mod_base = OTHER; note = 2'-O-methyluridine-3'-phosphate
  modified_base 18: mod_base = OTHER; note = 2'-O-methyladenosine-3'-phosphate
  modified_base 19: mod_base = OTHER; note = 2'-O-methyladenosine-3'-phosphate
  modified_base 20: mod_base = OTHER; note = 2'-O-methyluridine-3'-phosphate
  modified_base 21: mod_base = OTHER; note = 2'-O-methyluridine-3'-phosphate ((2S,4R)-1-[29-[[2-(acetylamino)-2-deoxy-beta-D-galactopyranosyl]oxy]-14,14-bis[[3-[[3-[[5-[[2-(acetylamino)-2-deoxy-beta-D-galactopyranosyl]oxy]-1-oxopentyl]amino]propyl]amino]-3-oxopropoxy]methyl]-1,12,19,25-tetraoxo-16-oxa-13,20,24-triazanonacos-1-yl]-4-hydroxy-2-pyrrolidinyl)methyl ester
ttgaaactcatagcaataatt

SEQ ID NO: 378 - RNA, 21 nt, synthetic construct
  source 1..21: mol_type = other RNA
  modified_base 1: mod_base = OTHER; note = 2'-O-methyluridine-3'-phosphorothioate
  modified_base 2: mod_base = OTHER; note = 2'-O-methyladenosine-3'-phosphorothioate
  modified_base 3: mod_base = OTHER; note = 2'-O-methyladenosine-3'-phosphate
  modified_base 4: mod_base = OTHER; note = 2'-O-methyluridine-3'-phosphate
  modified_base 5: mod_base = OTHER; note = 2'-O-methylguanosine-3'-phosphate
  modified_base 6: mod_base = OTHER; note = 2'-O-methylcytidine-3'-phosphate
  modified_base 7: mod_base = OTHER; note = 2'-deoxy-2'-fluorouridine-3'-phosphate
  modified_base 8: mod_base = OTHER; note = 2'-O-methyladenosine-3'-phosphate
  modified_base 9: mod_base = OTHER; note = 2'-deoxy-2'-fluorouridine-3'-phosphate
  modified_base 10: mod_base = OTHER; note = 2'-deoxy-2'-fluoroguanosine-3'-phosphate
  modified_base 11: mod_base = OTHER; note = 2'-deoxy-2'-fluorocytidine-3'-phosphate
  modified_base 12: mod_base = OTHER; note = 2'-O-methyluridine-3'-phosphate
  modified_base 13: mod_base = OTHER; note = 2'-O-methylguanosine-3'-phosphate
  modified_base 14: mod_base = OTHER; note = 2'-O-methyluridine-3'-phosphate
  modified_base 15: mod_base = OTHER; note = 2'-O-methyluridine-3'-phosphate
  modified_base 16: mod_base = OTHER; note = 2'-O-methylguanosine-3'-phosphate
  modified_base 17: mod_base = OTHER; note = 2'-O-methyluridine-3'-phosphate
  modified_base 18: mod_base = OTHER; note = 2'-O-methylguanosine-3'-phosphate
  modified_base 19: mod_base = OTHER; note = 2'-O-methyladenosine-3'-phosphate
  modified_base 20: mod_base = OTHER; note = 2'-O-methyluridine-3'-phosphate
  modified_base 21: mod_base = OTHER; note = 2'-O-methyluridine-3'-phosphate ((2S,4R)-1-[29-[[2-(acetylamino)-2-deoxy-beta-D-galactopyranosyl]oxy]-14,14-bis[[3-[[3-[[5-[[2-(acetylamino)-2-deoxy-beta-D-galactopyranosyl]oxy]-1-oxopentyl]amino]propyl]amino]-3-oxopropoxy]methyl]-1,12,19,25-tetraoxo-16-oxa-13,20,24-triazanonacos-1-yl]-4-hydroxy-2-pyrrolidinyl)methyl ester
taatgctatgctgttgtgatt

SEQ ID NO: 379 - RNA, 21 nt, synthetic construct
  source 1..21: mol_type = other RNA
  modified_base 1: mod_base = OTHER; note = 2'-O-methylcytidine-3'-phosphorothioate
  modified_base 2: mod_base = OTHER; note = 2'-O-methyladenosine-3'-phosphorothioate
  modified_base 3: mod_base = OTHER; note = 2'-O-methyladenosine-3'-phosphate
  modified_base 4: mod_base = OTHER; note = 2'-O-methylguanosine-3'-phosphate
  modified_base 5: mod_base = OTHER; note = 2'-O-methyluridine-3'-phosphate
  modified_base 6: mod_base = OTHER; note = 2'-O-methyluridine-3'-phosphate
  modified_base 7: mod_base = OTHER; note = 2'-deoxy-2'-fluorocytidine-3'-phosphate
  modified_base 8: mod_base = OTHER; note = 2'-O-methyluridine-3'-phosphate
  modified_base 9: mod_base = OTHER; note = 2'-deoxy-2'-fluoroguanosine-3'-phosphate
  modified_base 10: mod_base = OTHER; note = 2'-deoxy-2'-fluorocytidine-3'-phosphate
  modified_base 11: mod_base = OTHER; note = 2'-deoxy-2'-fluoroadenosine-3'-phosphate
  modified_base 12: mod_base = OTHER; note = 2'-O-methyluridine-3'-phosphate
  modified_base 13: mod_base = OTHER; note = 2'-O-methyluridine-3'-phosphate
  modified_base 14: mod_base = OTHER; note = 2'-O-methyluridine-3'-phosphate
  modified_base 15: mod_base = OTHER; note = 2'-O-methyladenosine-3'-phosphate
  modified_base 16: mod_base = OTHER; note = 2'-O-methyladenosine-3'-phosphate
  modified_base 17: mod_base = OTHER; note = 2'-O-methyladenosine-3'-phosphate
  modified_base 18: mod_base = OTHER; note = 2'-O-methyladenosine-3'-phosphate
  modified_base 19: mod_base = OTHER; note = 2'-O-methyluridine-3'-phosphate
  modified_base 20: mod_base = OTHER; note = 2'-O-methyladenosine-3'-phosphate
  modified_base 21: mod_base = OTHER; note = 2'-O-methyluridine-3'-phosphate ((2S,4R)-1-[29-[[2-(acetylamino)-2-deoxy-beta-D-galactopyranosyl]oxy]-14,14-bis[[3-[[3-[[5-[[2-(acetylamino)-2-deoxy-beta-D-galactopyranosyl]oxy]-1-oxopentyl]amino]propyl]amino]-3-oxopropoxy]methyl]-1,12,19,25-tetraoxo-16-oxa-13,20,24-triazanonacos-1-yl]-4-hydroxy-2-pyrrolidinyl)methyl ester
caagttctgcatttaaaatat

SEQ ID NO: 380 - RNA, 21 nt, synthetic construct
  source 1..21: mol_type = other RNA
  modified_base 1: mod_base = OTHER; note = 2'-O-methylguanosine-3'-phosphorothioate
  modified_base 2: mod_base = OTHER; note = 2'-O-methyladenosine-3'-phosphorothioate
  modified_base 3: mod_base = OTHER; note = 2'-O-methyluridine-3'-phosphate
  modified_base 4: mod_base = OTHER; note = 2'-O-methylguanosine-3'-phosphate
  modified_base 5: mod_base = OTHER; note = 2'-O-methyluridine-3'-phosphate
  modified_base 6: mod_base = OTHER; note = 2'-O-methyladenosine-3'-phosphate
  modified_base 7: mod_base = OTHER; note = 2'-deoxy-2'-fluorouridine-3'-phosphate
  modified_base 8: mod_base = OTHER; note = 2'-O-methyladenosine-3'-phosphate
  modified_base 9: mod_base = OTHER; note = 2'-deoxy-2'-fluorocytidine-3'-phosphate
  modified_base 10: mod_base = OTHER; note = 2'-deoxy-2'-fluorocytidine-3'-phosphate
  modified_base 11: mod_base = OTHER; note = 2'-deoxy-2'-fluoroadenosine-3'-phosphate
  modified_base 12: mod_base = OTHER; note = 2'-O-methyluridine-3'-phosphate
  modified_base 13: mod_base = OTHER; note = 2'-O-methylguanosine-3'-phosphate
  modified_base 14: mod_base = OTHER; note = 2'-O-methyladenosine-3'-phosphate
  modified_base 15: mod_base = OTHER; note = 2'-O-methyladenosine-3'-phosphate
  modified_base 16: mod_base = OTHER; note = 2'-O-methylguanosine-3'-phosphate
  modified_base 17: mod_base = OTHER; note = 2'-O-methyluridine-3'-phosphate
  modified_base 18: mod_base = OTHER; note = 2'-O-methylcytidine-3'-phosphate
  modified_base 19: mod_base = OTHER; note = 2'-O-methyladenosine-3'-phosphate
  modified_base 20: mod_base = OTHER; note = 2'-O-methyluridine-3'-phosphate
  modified_base 21: mod_base = OTHER; note = 2'-O-methyluridine-3'-phosphate ((2S,4R)-1-[29-[[2-(acetylamino)-2-deoxy-beta-D-galactopyranosyl]oxy]-14,14-bis[[3-[[3-[[5-[[2-(acetylamino)-2-deoxy-beta-D-galactopyranosyl]oxy]-1-oxopentyl]amino]propyl]amino]-3-oxopropoxy]methyl]-1,12,19,25-tetraoxo-16-oxa-13,20,24-triazanonacos-1-yl]-4-hydroxy-2-pyrrolidinyl)methyl ester
gatgtataccatgaagtcatt

SEQ ID NO: 381 - RNA, 21 nt, synthetic construct
  source 1..21: mol_type = other RNA
  modified_base 1: mod_base = OTHER; note = 2'-O-methylguanosine-3'-phosphorothioate
  modified_base 2: mod_base = OTHER; note = 2'-O-methyluridine-3'-phosphorothioate
  modified_base 3: mod_base = OTHER; note = 2'-O-methyluridine-3'-phosphate
  modified_base 4: mod_base = OTHER; note = 2'-O-methylguanosine-3'-phosphate
  modified_base 5: mod_base = OTHER; note = 2'-O-methyluridine-3'-phosphate
  modified_base 6: mod_base = OTHER; note = 2'-O-methyladenosine-3'-phosphate
  modified_base 7: mod_base = OTHER; note = 2'-deoxy-2'-fluoroguanosine-3'-phosphate
  modified_base 8: mod_base = OTHER; note = 2'-O-methyluridine-3'-phosphate
  modified_base 9: mod_base = OTHER; note = 2'-deoxy-2'-fluoroadenosine-3'-phosphate
  modified_base 10: mod_base = OTHER; note = 2'-deoxy-2'-fluoroguanosine-3'-phosphate
  modified_base 11: mod_base = OTHER; note = 2'-deoxy-2'-fluorocytidine-3'-phosphate
  modified_base 12: mod_base = OTHER; note = 2'-O-methyluridine-3'-phosphate
  modified_base 13: mod_base = OTHER; note = 2'-O-methylcytidine-3'-phosphate
  modified_base 14: mod_base = OTHER; note = 2'-O-methyluridine-3'-phosphate
  modified_base 15: mod_base = OTHER; note = 2'-O-methylguanosine-3'-phosphate
  modified_base 16: mod_base = OTHER; note = 2'-O-methyladenosine-3'-phosphate
  modified_base 17: mod_base = OTHER; note = 2'-O-methyluridine-3'-phosphate
  modified_base 18: mod_base = OTHER; note = 2'-O-methylguanosine-3'-phosphate
  modified_base 19: mod_base = OTHER; note = 2'-O-methyluridine-3'-phosphate
  modified_base 20: mod_base = OTHER; note = 2'-O-methyluridine-3'-phosphate
  modified_base 21: mod_base = OTHER; note = 2'-O-methyluridine-3'-phosphate ((2S,4R)-1-[29-[[2-(acetylamino)-2-deoxy-beta-D-galactopyranosyl]oxy]-14,14-bis[[3-[[3-[[5-[[2-(acetylamino)-2-deoxy-beta-D-galactopyranosyl]oxy]-1-oxopentyl]amino]propyl]amino]-3-oxopropoxy]methyl]-1,12,19,25-tetraoxo-16-oxa-13,20,24-triazanonacos-1-yl]-4-hydroxy-2-pyrrolidinyl)methyl ester
gttgtagtagctctgatgttt

SEQ ID NO: 382 - RNA, 21 nt, synthetic construct
  source 1..21: mol_type = other RNA
  modified_base 1: mod_base = OTHER; note = 2'-O-methyluridine-3'-phosphorothioate
  modified_base 2: mod_base = OTHER; note = 2'-O-methylguanosine-3'-phosphorothioate
  modified_base 3: mod_base = OTHER; note = 2'-O-methyladenosine-3'-phosphate
  modified_base 4: mod_base = OTHER; note = 2'-O-methyladenosine-3'-phosphate
  modified_base 5: mod_base = OTHER; note = 2'-O-methyluridine-3'-phosphate
  modified_base 6: mod_base = OTHER; note = 2'-O-methylguanosine-3'-phosphate
  modified_base 7: mod_base = OTHER; note = 2'-deoxy-2'-fluoroadenosine-3'-phosphate
  modified_base 8: mod_base = OTHER; note = 2'-O-methylguanosine-3'-phosphate
  modified_base 9: mod_base = OTHER; note = 2'-deoxy-2'-fluoroadenosine-3'-phosphate
  modified_base 10: mod_base = OTHER; note = 2'-deoxy-2'-fluorouridine-3'-phosphate
  modified_base 11: mod_base = OTHER; note = 2'-deoxy-2'-fluoroadenosine-3'-phosphate
  modified_base 12: mod_base = OTHER; note = 2'-O-methyluridine-3'-phosphate
  modified_base 13: mod_base = OTHER; note = 2'-O-methylcytidine-3'-phosphate
  modified_base 14: mod_base = OTHER; note = 2'-O-methyladenosine-3'-phosphate
  modified_base 15: mod_base = OTHER; note = 2'-O-methyluridine-3'-phosphate
  modified_base 16: mod_base = OTHER; note = 2'-O-methylguanosine-3'-phosphate
  modified_base 17: mod_base = OTHER; note = 2'-O-methyluridine-3'-phosphate
  modified_base 18: mod_base = OTHER; note = 2'-O-methyluridine-3'-phosphate
  modified_base 19: mod_base = OTHER; note = 2'-O-methyluridine-3'-phosphate
  modified_base 20: mod_base = OTHER; note = 2'-O-methyluridine-3'-phosphate
  modified_base 21: mod_base = OTHER; note = 2'-O-methyluridine-3'-phosphate ((2S,4R)-1-[29-[[2-(acetylamino)-2-deoxy-beta-D-galactopyranosyl]oxy]-14,14-bis[[3-[[3-[[5-[[2-(acetylamino)-2-deoxy-beta-D-galactopyranosyl]oxy]-1-oxopentyl]amino]propyl]amino]-3-oxopropoxy]methyl]-1,12,19,25-tetraoxo-16-oxa-13,20,24-triazanonacos-1-yl]-4-hydroxy-2-pyrrolidinyl)methyl ester
tgaatgagatatcatgttttt

SEQ ID NO: 383 - RNA, 21 nt, synthetic construct
  source 1..21: mol_type = other RNA
  modified_base 1: mod_base = OTHER; note = 2'-O-methyluridine-3'-phosphorothioate
  modified_base 2: mod_base = OTHER; note = 2'-O-methyluridine-3'-phosphorothioate
  modified_base 3: mod_base = OTHER; note = 2'-O-methyluridine-3'-phosphate
  modified_base 4: mod_base = OTHER; note = 2'-O-methyluridine-3'-phosphate
  modified_base 5: mod_base = OTHER; note = 2'-O-methyladenosine-3'-phosphate
  modified_base 6: mod_base = OTHER; note = 2'-O-methylguanosine-3'-phosphate
  modified_base 7: mod_base = OTHER; note = 2'-deoxy-2'-fluorocytidine-3'-phosphate
  modified_base 8: mod_base = OTHER; note = 2'-O-methyladenosine-3'-phosphate
  modified_base 9: mod_base = OTHER; note = 2'-deoxy-2'-fluorouridine-3'-phosphate
  modified_base 10: mod_base = OTHER; note = 2'-deoxy-2'-fluorouridine-3'-phosphate
  modified_base 11: mod_base = OTHER; note = 2'-deoxy-2'-fluorocytidine-3'-phosphate
  modified_base 12: mod_base = OTHER; note = 2'-O-methylcytidine-3'-phosphate
  modified_base 13: mod_base = OTHER; note = 2'-O-methyladenosine-3'-phosphate
  modified_base 14: mod_base = OTHER; note = 2'-O-methyluridine-3'-phosphate
  modified_base 15: mod_base = OTHER; note = 2'-O-methyluridine-3'-phosphate
  modified_base 16: mod_base = OTHER; note = 2'-O-methyluridine-3'-phosphate
  modified_base 17: mod_base = OTHER; note = 2'-O-methyluridine-3'-phosphate
  modified_base 18: mod_base = OTHER; note = 2'-O-methyladenosine-3'-phosphate
  modified_base 19: mod_base = OTHER; note = 2'-O-methylcytidine-3'-phosphate
  modified_base 20: mod_base = OTHER; note = 2'-O-methyluridine-3'-phosphate
  modified_base 21: mod_base = OTHER; note = 2'-O-methyluridine-3'-phosphate ((2S,4R)-1-[29-[[2-(acetylamino)-2-deoxy-beta-D-galactopyranosyl]oxy]-14,14-bis[[3-[[3-[[5-[[2-(acetylamino)-2-deoxy-beta-D-galactopyranosyl]oxy]-1-oxopentyl]amino]propyl]amino]-3-oxopropoxy]methyl]-1,12,19,25-tetraoxo-16-oxa-13,20,24-triazanonacos-1-yl]-4-hydroxy-2-pyrrolidinyl)methyl ester
ttttagcattccattttactt

SEQ ID NO: 384 - RNA, 21 nt, synthetic construct
  source 1..21: mol_type = other RNA
  modified_base 1: mod_base = OTHER; note = 2'-O-methyluridine-3'-phosphorothioate
  modified_base 2: mod_base = OTHER; note = 2'-O-methyladenosine-3'-phosphorothioate
  modified_base 3: mod_base = OTHER; note = 2'-O-methyladenosine-3'-phosphate
  modified_base 4: mod_base = OTHER; note = 2'-O-methyladenosine-3'-phosphate
  modified_base 5: mod_base = OTHER; note = 2'-O-methyluridine-3'-phosphate
  modified_base 6: mod_base = OTHER; note = 2'-O-methyluridine-3'-phosphate
  modified_base 7: mod_base = OTHER; note = 2'-deoxy-2'-fluoroadenosine-3'-phosphate
  modified_base 8: mod_base = OTHER; note = 2'-O-methyladenosine-3'-phosphate
  modified_base 9: mod_base = OTHER; note = 2'-deoxy-2'-fluoroguanosine-3'-phosphate
  modified_base 10: mod_base = OTHER; note = 2'-deoxy-2'-fluoroguanosine-3'-phosphate
  modified_base 11: mod_base = OTHER; note = 2'-deoxy-2'-fluoroadenosine-3'-phosphate
  modified_base 12: mod_base = OTHER; note = 2'-O-methyluridine-3'-phosphate
  modified_base 13: mod_base = OTHER; note = 2'-O-methyluridine-3'-phosphate
  modified_base 14: mod_base = OTHER; note = 2'-O-methyladenosine-3'-phosphate
  modified_base 15: mod_base = OTHER; note = 2'-O-methylcytidine-3'-phosphate
  modified_base 16: mod_base = OTHER; note = 2'-O-methyluridine-3'-phosphate
  modified_base 17: mod_base = OTHER; note = 2'-O-methylcytidine-3'-phosphate
  modified_base 18: mod_base = OTHER; note = 2'-O-methyladenosine-3'-phosphate
  modified_base 19: mod_base = OTHER; note = 2'-O-methyladenosine-3'-phosphate
  modified_base 20: mod_base = OTHER; note = 2'-O-methylguanosine-3'-phosphate
  modified_base 21: mod_base = OTHER; note = 2'-O-methyluridine-3'-phosphate ((2S,4R)-1-[29-[[2-(acetylamino)-2-deoxy-beta-D-galactopyranosyl]oxy]-14,14-bis[[3-[[3-[[5-[[2-(acetylamino)-2-deoxy-beta-D-galactopyranosyl]oxy]-1-oxopentyl]amino]propyl]amino]-3-oxopropoxy]methyl]-1,12,19,25-tetraoxo-16-oxa-13,20,24-triazanonacos-1-yl]-4-hydroxy-2-pyrrolidinyl)methyl ester
taaattaaggattactcaagt

SEQ ID NO: 385 - RNA, 21 nt, synthetic construct
  source 1..21: mol_type = other RNA
  modified_base 1: mod_base = OTHER; note = 2'-O-methylguanosine-3'-phosphorothioate
  modified_base 2: mod_base = OTHER; note = 2'-O-methylcytidine-3'-phosphorothioate
  modified_base 3: mod_base = OTHER; note = 2'-O-methyluridine-3'-phosphate
  modified_base 4: mod_base = OTHER; note = 2'-O-methylcytidine-3'-phosphate
  modified_base 5: mod_base = OTHER; note = 2'-O-methyladenosine-3'-phosphate
  modified_base 6: mod_base = OTHER; note = 2'-O-methylcytidine-3'-phosphate
  modified_base 7: mod_base = OTHER; note = 2'-deoxy-2'-fluorocytidine-3'-phosphate
  modified_base 8: mod_base = OTHER; note = 2'-O-methyladenosine-3'-phosphate
  modified_base 9: mod_base = OTHER; note = 2'-deoxy-2'-fluorouridine-3'-phosphate
  modified_base 10: mod_base = OTHER; note = 2'-deoxy-2'-fluorouridine-3'-phosphate
  modified_base 11: mod_base = OTHER; note = 2'-deoxy-2'-fluoroadenosine-3'-phosphate
  modified_base 12: mod_base = OTHER; note = 2'-O-methyluridine-3'-phosphate
  modified_base 13: mod_base = OTHER; note = 2'-O-methyluridine-3'-phosphate
  modified_base 14: mod_base = OTHER; note = 2'-O-methylcytidine-3'-phosphate
  modified_base 15: mod_base = OTHER; note = 2'-O-methyladenosine-3'-phosphate
  modified_base 16: mod_base = OTHER; note = 2'-O-methyladenosine-3'-phosphate
  modified_base 17: mod_base = OTHER; note = 2'-O-methylguanosine-3'-phosphate
  modified_base 18: mod_base = OTHER; note = 2'-O-methyladenosine-3'-phosphate
  modified_base 19: mod_base = OTHER; note = 2'-O-methyluridine-3'-phosphate
  modified_base 20: mod_base = OTHER; note = 2'-O-methyluridine-3'-phosphate
  modified_base 21: mod_base = OTHER; note = 2'-O-methyluridine-3'-phosphate ((2S,4R)-1-[29-[[2-(acetylamino)-2-deoxy-beta-D-galactopyranosyl]oxy]-14,14-bis[[3-[[3-[[5-[[2-(acetylamino)-2-deoxy-beta-D-galactopyranosyl]oxy]-1-oxopentyl]amino]propyl]amino]-3-oxopropoxy]methyl]-1,12,19,25-tetraoxo-16-oxa-13,20,24-triazanonacos-1-yl]-4-hydroxy-2-pyrrolidinyl)methyl ester
gctcaccattattcaagattt

SEQ ID NO: 386 - RNA, 21 nt, synthetic construct
  source 1..21: mol_type = other RNA
  modified_base 1: mod_base = OTHER; note = 2'-O-methylguanosine-3'-phosphorothioate
  modified_base 2: mod_base = OTHER; note = 2'-O-methylguanosine-3'-phosphorothioate
  modified_base 3: mod_base = OTHER; note = 2'-O-methylcytidine-3'-phosphate
  modified_base 4: mod_base = OTHER; note = 2'-O-methyluridine-3'-phosphate
  modified_base 5: mod_base = OTHER; note = 2'-O-methyluridine-3'-phosphate
  modified_base 6: mod_base = OTHER; note = 2'-O-methylcytidine-3'-phosphate
  modified_base 7: mod_base = OTHER; note = 2'-deoxy-2'-fluorouridine-3'-phosphate
  modified_base 8: mod_base = OTHER; note = 2'-O-methylcytidine-3'-phosphate
  modified_base 9: mod_base = OTHER; note = 2'-deoxy-2'-fluorouridine-3'-phosphate
  modified_base 10: mod_base = OTHER; note = 2'-deoxy-2'-fluorouridine-3'-phosphate
  modified_base 11: mod_base = OTHER; note = 2'-deoxy-2'-fluoroguanosine-3'-phosphate
  modified_base 12: mod_base = OTHER; note = 2'-O-methylcytidine-3'-phosphate
  modified_base 13: mod_base = OTHER; note = 2'-O-methyladenosine-3'-phosphate
  modified_base 14: mod_base = OTHER; note = 2'-O-methyluridine-3'-phosphate
  modified_base 15: mod_base = OTHER; note = 2'-O-methyluridine-3'-phosphate
  modified_base 16: mod_base = OTHER; note = 2'-O-methyladenosine-3'-phosphate
  modified_base 17: mod_base = OTHER; note = 2'-O-methyluridine-3'-phosphate
  modified_base 18: mod_base = OTHER; note = 2'-O-methyluridine-3'-phosphate
  modified_base 19: mod_base = OTHER; note = 2'-O-methyluridine-3'-phosphate
  modified_base 20: mod_base = OTHER; note = 2'-O-methyluridine-3'-phosphate
  modified_base 21: mod_base = OTHER; note = 2'-O-methyluridine-3'-phosphate ((2S,4R)-1-[29-[[2-(acetylamino)-2-deoxy-beta-D-galactopyranosyl]oxy]-14,14-bis[[3-[[3-[[5-[[2-(acetylamino)-2-deoxy-beta-D-galactopyranosyl]oxy]-1-oxopentyl]amino]propyl]amino]-3-oxopropoxy]methyl]-1,12,19,25-tetraoxo-16-oxa-13,20,24-triazanonacos-1-yl]-4-hydroxy-2-pyrrolidinyl)methyl ester
ggcttctcttgcattattttt

SEQ ID NO: 387 - RNA, 21 nt, synthetic construct
  source 1..21: mol_type = other RNA
  modified_base 1: mod_base = OTHER; note = 2'-O-methyluridine-3'-phosphorothioate
  modified_base 2: mod_base = OTHER; note = 2'-O-methylguanosine-3'-phosphorothioate
  modified_base 3: mod_base = OTHER; note = 2'-O-methylguanosine-3'-phosphate
  modified_base 4: mod_base = OTHER; note = 2'-O-methyluridine-3'-phosphate
  modified_base 5: mod_base = OTHER; note = 2'-O-methyluridine-3'-phosphate
  modified_base 6: mod_base = OTHER; note = 2'-O-methyluridine-3'-phosphate
  modified_base 7: mod_base = OTHER; note = 2'-deoxy-2'-fluoroguanosine-3'-phosphate
  modified_base 8: mod_base = OTHER; note = 2'-O-methyluridine-3'-phosphate
  modified_base 9: mod_base = OTHER; note = 2'-deoxy-2'-fluorouridine-3'-phosphate
  modified_base 10: mod_base = OTHER; note = 2'-deoxy-2'-fluorouridine-3'-phosphate
  modified_base 11: mod_base = OTHER; note = 2'-deoxy-2'-fluorouridine-3'-phosphate
  modified_base 12: mod_base = OTHER; note = 2'-O-methylcytidine-3'-phosphate
  modified_base 13: mod_base = OTHER; note = 2'-O-methyluridine-3'-phosphate
  modified_base 14: mod_base = OTHER; note = 2'-O-methyladenosine-3'-phosphate
  modified_base 15: mod_base = OTHER; note = 2'-O-methylguanosine-3'-phosphate
  modified_base 16: mod_base = OTHER; note = 2'-O-methyladenosine-3'-phosphate
  modified_base 17: mod_base = OTHER; note = 2'-O-methyladenosine-3'-phosphate
  modified_base 18: mod_base = OTHER; note = 2'-O-methylguanosine-3'-phosphate
  modified_base 19: mod_base = OTHER; note = 2'-O-methyluridine-3'-phosphate
  modified_base 20: mod_base = OTHER; note = 2'-O-methyladenosine-3'-phosphate
  modified_base 21: mod_base = OTHER; note = 2'-O-methyluridine-3'-phosphate ((2S,4R)-1-[29-[[2-(acetylamino)-2-deoxy-beta-D-galactopyranosyl]oxy]-14,14-bis[[3-[[3-[[5-[[2-(acetylamino)-2-deoxy-beta-D-galactopyranosyl]oxy]-1-oxopentyl]amino]propyl]amino]-3-oxopropoxy]methyl]-1,12,19,25-tetraoxo-16-oxa-13,20,24-triazanonacos-1-yl]-4-hydroxy-2-pyrrolidinyl)methyl ester
tggtttgttttctagaagtat

SEQ ID NO: 388 - RNA, 21 nt, synthetic construct
  source 1..21: mol_type = other RNA
  modified_base 1: mod_base = OTHER; note = 2'-O-methylcytidine-3'-phosphorothioate
  modified_base 2: mod_base = OTHER; note = 2'-O-methyluridine-3'-phosphorothioate
  modified_base 3: mod_base = OTHER; note = 2'-O-methylguanosine-3'-phosphate
  modified_base 4: mod_base = OTHER; note = 2'-O-methylguanosine-3'-phosphate
  modified_base 5: mod_base = OTHER; note = 2'-O-methyluridine-3'-phosphate
  modified_base 6: mod_base = OTHER; note = 2'-O-methylguanosine-3'-phosphate
  modified_base 7: mod_base = OTHER; note = 2'-deoxy-2'-fluorocytidine-3'-phosphate
  modified_base 8: mod_base = OTHER; note = 2'-O-methyluridine-3'-phosphate
  modified_base 9: mod_base = OTHER; note = 2'-deoxy-2'-fluorouridine-3'-phosphate
  modified_base 10: mod_base = OTHER; note = 2'-deoxy-2'-fluorouridine-3'-phosphate
  modified_base 11: mod_base = OTHER; note = 2'-deoxy-2'-fluoroguanosine-3'-phosphate
  modified_base 12: mod_base = OTHER; note = 2'-O-methyladenosine-3'-phosphate
  modified_base 13: mod_base = OTHER; note = 2'-O-methyladenosine-3'-phosphate
  modified_base 14: mod_base = OTHER; note = 2'-O-methyladenosine-3'-phosphate
  modified_base 15: mod_base = OTHER; note = 2'-O-methyladenosine-3'-phosphate
  modified_base 16: mod_base = OTHER; note = 2'-O-methyluridine-3'-phosphate
  modified_base 17: mod_base = OTHER; note = 2'-O-methylcytidine-3'-phosphate
  modified_base 18: mod_base = OTHER; note = 2'-O-methyluridine-3'-phosphate
  modified_base 19: mod_base = OTHER; note = 2'-O-methyluridine-3'-phosphate
  modified_base 20: mod_base = OTHER; note = 2'-O-methyluridine-3'-phosphate
  modified_base 21: mod_base = OTHER; note = 2'-O-methyluridine-3'-phosphate ((2S,4R)-1-[29-[[2-(acetylamino)-2-deoxy-beta-D-galactopyranosyl]oxy]-14,14-bis[[3-[[3-[[5-[[2-(acetylamino)-2-deoxy-beta-D-galactopyranosyl]oxy]-1-oxopentyl]amino]propyl]amino]-3-oxopropoxy]methyl]-1,12,19,25-tetraoxo-16-oxa-13,20,24-triazanonacos-1-yl]-4-hydroxy-2-pyrrolidinyl)methyl ester
ctggtgctttgaaaatctttt

SEQ ID NO: 389 - RNA, 21 nt, synthetic construct
  source 1..21: mol_type = other RNA
  modified_base 1: mod_base = OTHER; note = 2'-O-methylguanosine-3'-phosphorothioate
  modified_base 2: mod_base = OTHER; note = 2'-O-methylcytidine-3'-phosphorothioate
  modified_base 3: mod_base = OTHER; note = 2'-O-methyluridine-3'-phosphate
  modified_base 4: mod_base = OTHER; note = 2'-O-methylguanosine-3'-phosphate
  modified_base 5: mod_base = OTHER; note = 2'-O-methyladenosine-3'-phosphate
  modified_base 6: mod_base = OTHER; note = 2'-O-methylcytidine-3'-phosphate
  modified_base 7: mod_base = OTHER; note = 2'-deoxy-2'-fluorocytidine-3'-phosphate
  modified_base 8: mod_base = OTHER; note = 2'-O-methyluridine-3'-phosphate
  modified_base 9: mod_base = OTHER; note = 2'-deoxy-2'-fluorouridine-3'-phosphate
  modified_base 10: mod_base = OTHER; note = 2'-deoxy-2'-fluorouridine-3'-phosphate
  modified_base 11: mod_base = OTHER; note = 2'-deoxy-2'-fluoroguanosine-3'-phosphate
  modified_base 12: mod_base = OTHER; note = 2'-O-methyladenosine-3'-phosphate
  modified_base 13: mod_base = OTHER; note = 2'-O-methylguanosine-3'-phosphate
  modified_base 14: mod_base = OTHER; note = 2'-O-methyluridine-3'-phosphate
  modified_base 15: mod_base = OTHER; note = 2'-O-methyluridine-3'-phosphate
  modified_base 16: mod_base = OTHER; note = 2'-O-methyladenosine-3'-phosphate
  modified_base 17: mod_base = OTHER; note = 2'-O-methyladenosine-3'-phosphate
  modified_base 18: mod_base = OTHER; note = 2'-O-methyluridine-3'-phosphate
  modified_base 19: mod_base = OTHER; note = 2'-O-methyluridine-3'-phosphate
  modified_base 20: mod_base = OTHER; note = 2'-O-methyluridine-3'-phosphate
  modified_base 21: mod_base = OTHER; note = 2'-O-methyluridine-3'-phosphate ((2S,4R)-1-[29-[[2-(acetylamino)-2-deoxy-beta-D-galactopyranosyl]oxy]-14,14-bis[[3-[[3-[[5-[[2-(acetylamino)-2-deoxy-beta-D-galactopyranosyl]oxy]-1-oxopentyl]amino]propyl]amino]-3-oxopropoxy]methyl]-1,12,19,25-tetraoxo-16-oxa-13,20,24-triazanonacos-1-yl]-4-hydroxy-2-pyrrolidinyl)methyl ester
gctgacctttgagttaatttt

SEQ ID NO: 390 - RNA, 21 nt, synthetic construct
  source 1..21: mol_type = other RNA
  modified_base 1: mod_base = OTHER; note = 2'-O-methyladenosine-3'-phosphorothioate
  modified_base 2: mod_base = OTHER; note = 2'-O-methylguanosine-3'-phosphorothioate
  modified_base 3: mod_base = OTHER; note = 2'-O-methylcytidine-3'-phosphate
  modified_base 4: mod_base = OTHER; note = 2'-O-methyladenosine-3'-phosphate
  modified_base 5: mod_base = OTHER; note = 2'-O-methylcytidine-3'-phosphate
  modified_base 6: mod_base = OTHER; note = 2'-O-methyladenosine-3'-phosphate
  modified_base 7: mod_base = OTHER; note = 2'-deoxy-2'-fluoroadenosine-3'-phosphate
  modified_base 8: mod_base = OTHER; note = 2'-O-methylcytidine-3'-phosphate
  modified_base 9: mod_base = OTHER; note = 2'-deoxy-2'-fluorouridine-3'-phosphate
  modified_base 10: mod_base = OTHER; note = 2'-deoxy-2'-fluorocytidine-3'-phosphate
  modified_base 11: mod_base = OTHER; note = 2'-deoxy-2'-fluoroadenosine-3'-phosphate
  modified_base 12: mod_base = OTHER; note = 2'-O-methyluridine-3'-phosphate
  modified_base 13: mod_base = OTHER; note = 2'-O-methyluridine-3'-phosphate
  modified_base 14: mod_base = OTHER; note = 2'-O-methylcytidine-3'-phosphate
  modified_base 15: mod_base = OTHER; note = 2'-O-methyluridine-3'-phosphate
  modified_base 16: mod_base = OTHER; note = 2'-O-methyluridine-3'-phosphate
  modified_base 17: mod_base = OTHER; note = 2'-O-methylcytidine-3'-phosphate
  modified_base 18: mod_base = OTHER; note = 2'-O-methyladenosine-3'-phosphate
  modified_base 19: mod_base = OTHER; note = 2'-O-methylguanosine-3'-phosphate
  modified_base 20: mod_base = OTHER; note = 2'-O-methyluridine-3'-phosphate
  modified_base 21: mod_base = OTHER; note = 2'-O-methyluridine-3'-phosphate ((2S,4R)-1-[29-[[2-(acetylamino)-2-deoxy-beta-D-galactopyranosyl]oxy]-14,14-bis[[3-[[3-[[5-[[2-(acetylamino)-2-deoxy-beta-D-galactopyranosyl]oxy]-1-oxopentyl]amino]propyl]amino]-3-oxopropoxy]methyl]-1,12,19,25-tetraoxo-16-oxa-13,20,24-triazanonacos-1-yl]-4-hydroxy-2-pyrrolidinyl)methyl ester
agcacaactcattcttcagtt

SEQ ID NO: 391 - RNA, 21 nt, synthetic construct
  source 1..21: mol_type = other RNA
  modified_base 1: mod_base = OTHER; note = 2'-O-methyluridine-3'-phosphorothioate
  modified_base 2: mod_base = OTHER; note = 2'-O-methylguanosine-3'-phosphorothioate
  modified_base 3: mod_base = OTHER; note = 2'-O-methylcytidine-3'-phosphate
  modified_base 4: mod_base = OTHER; note = 2'-O-methylcytidine-3'-phosphate
  modified_base 5: mod_base = OTHER; note = 2'-O-methyluridine-3'-phosphate
  modified_base 6: mod_base = OTHER; note = 2'-O-methylcytidine-3'-phosphate
  modified_base 7: mod_base = OTHER; note = 2'-deoxy-2'-fluoroadenosine-3'-phosphate
  modified_base 8: mod_base = OTHER; note = 2'-O-methyluridine-3'-phosphate
  modified_base 9: mod_base = OTHER; note = 2'-deoxy-2'-fluoroguanosine-3'-phosphate
  modified_base 10: mod_base = OTHER; note = 2'-deoxy-2'-fluoroadenosine-3'-phosphate
  modified_base 11: mod_base = OTHER; note = 2'-deoxy-2'-fluorocytidine-3'-phosphate
  modified_base 12: mod_base = OTHER; note = 2'-O-methyluridine-3'-phosphate
  modified_base 13: mod_base = OTHER; note = 2'-O-methylguanosine-3'-phosphate
  modified_base 14: mod_base = OTHER; note = 2'-O-methyladenosine-3'-phosphate
  modified_base 15: mod_base = OTHER; note = 2'-O-methyladenosine-3'-phosphate
  modified_base 16: mod_base = OTHER; note = 2'-O-methyladenosine-3'-phosphate
  modified_base 17: mod_base = OTHER; note = 2'-O-methyladenosine-3'-phosphate
  modified_base 18: mod_base = OTHER; note = 2'-O-methylcytidine-3'-phosphate
  modified_base 19: mod_base = OTHER; note = 2'-O-methyladenosine-3'-phosphate
  modified_base 20: mod_base = OTHER; note = 2'-O-methyladenosine-3'-phosphate
  modified_base 21: mod_base = OTHER; note = 2'-O-methyluridine-3'-phosphate ((2S,4R)-1-[29-[[2-(acetylamino)-2-deoxy-beta-D-galactopyranosyl]oxy]-14,14-bis[[3-[[3-[[5-[[2-(acetylamino)-2-deoxy-beta-D-galactopyranosyl]oxy]-1-oxopentyl]amino]propyl]amino]-3-oxopropoxy]methyl]-1,12,19,25-tetraoxo-16-oxa-13,20,24-triazanonacos-1-yl]-4-hydroxy-2-pyrrolidinyl)methyl ester
tgcctcatgactgaaaacaat

SEQ ID NO: 392 - RNA, 21 nt, synthetic construct
  source 1..21: mol_type = other RNA
  modified_base 1: mod_base = OTHER; note = 2'-O-methylcytidine-3'-phosphorothioate
  modified_base 2: mod_base = OTHER; note = 2'-O-methylguanosine-3'-phosphorothioate
  modified_base 3: mod_base = OTHER; note = 2'-O-methyladenosine-3'-phosphate
  modified_base 4: mod_base = OTHER; note = 2'-O-methyladenosine-3'-phosphate
  modified_base 5: mod_base = OTHER; note = 2'-O-methyladenosine-3'-phosphate
  modified_base 6: mod_base = OTHER; note = 2'-O-methylguanosine-3'-phosphate
  modified_base 7: mod_base = OTHER; note = 2'-deoxy-2'-fluorocytidine-3'-phosphate
  modified_base 8: mod_base = OTHER; note = 2'-O-methyladenosine-3'-phosphate
  modified_base 9: mod_base = OTHER; note = 2'-deoxy-2'-fluorouridine-3'-phosphate
  modified_base 10: mod_base = OTHER; note = 2'-deoxy-2'-fluorocytidine-3'-phosphate
  modified_base 11: mod_base = OTHER; note = 2'-deoxy-2'-fluorouridine-3'-phosphate
  modified_base 12: mod_base = OTHER; note = 2'-O-methyluridine-3'-phosphate
  modified_base 13: mod_base = OTHER; note = 2'-O-methylcytidine-3'-phosphate
  modified_base 14: mod_base = OTHER; note = 2'-O-methyladenosine-3'-phosphate
  modified_base 15: mod_base = OTHER; note = 2'-O-methylcytidine-3'-phosphate
  modified_base 16: mod_base = OTHER; note = 2'-O-methyladenosine-3'-phosphate
  modified_base 17: mod_base = OTHER; note = 2'-O-methyladenosine-3'-phosphate
  modified_base 18: mod_base = OTHER; note = 2'-O-methyluridine-3'-phosphate
  modified_base 19: mod_base = OTHER; note = 2'-O-methylguanosine-3'-phosphate
  modified_base 20: mod_base = OTHER; note = 2'-O-methyladenosine-3'-phosphate
  modified_base 21: mod_base = OTHER; note = 2'-O-methyluridine-3'-phosphate ((2S,4R)-1-[29-[[2-(acetylamino)-2-deoxy-beta-D-galactopyranosyl]oxy]-14,14-bis[[3-[[3-[[5-[[2-(acetylamino)-2-deoxy-beta-D-galactopyranosyl]oxy]-1-oxopentyl]amino]propyl]amino]-3-oxopropoxy]methyl]-1,12,19,25-tetraoxo-16-oxa-13,20,24-triazanonacos-1-yl]-4-hydroxy-2-pyrrolidinyl)methyl ester
cgaaagcatcttcacaatgat

SEQ ID NO: 393 - RNA, 21 nt, synthetic construct
  source 1..21: mol_type = other RNA
  modified_base 1: mod_base = OTHER; note = 2'-O-methyladenosine-3'-phosphorothioate
  modified_base 2: mod_base = OTHER; note = 2'-O-methyluridine-3'-phosphorothioate
  modified_base 3: mod_base = OTHER; note = 2'-O-methyladenosine-3'-phosphate
  modified_base 4: mod_base = OTHER; note = 2'-O-methylguanosine-3'-phosphate
  modified_base 5: mod_base = OTHER; note = 2'-O-methylcytidine-3'-phosphate
  modified_base 6: mod_base = OTHER; note = 2'-O-methyladenosine-3'-phosphate
  modified_base 7: mod_base = OTHER; note = 2'-deoxy-2'-fluorocytidine-3'-phosphate
  modified_base 8: mod_base = OTHER; note = 2'-O-methylcytidine-3'-phosphate
  modified_base 9: mod_base = OTHER; note = 2'-deoxy-2'-fluoroguanosine-3'-phosphate
  modified_base 10: mod_base = OTHER; note = 2'-deoxy-2'-fluorouridine-3'-phosphate
  modified_base 11: mod_base = OTHER; note = 2'-deoxy-2'-fluorouridine-3'-phosphate
  modified_base 12: mod_base = OTHER; note = 2'-O-methyluridine-3'-phosphate
  modified_base 13: mod_base = OTHER; note = 2'-O-methyluridine-3'-phosphate
  modified_base 14: mod_base = OTHER; note = 2'-O-methylguanosine-3'-phosphate
  modified_base 15: mod_base = OTHER; note = 2'-O-methylcytidine-3'-phosphate
  modified_base 16: mod_base = OTHER; note = 2'-O-methyluridine-3'-phosphate
  modified_base 17: mod_base = OTHER; note = 2'-O-methyladenosine-3'-phosphate
  modified_base 18: mod_base = OTHER; note = 2'-O-methyladenosine-3'-phosphate
  modified_base 19: mod_base = OTHER; note = 2'-O-methyladenosine-3'-phosphate
  modified_base 20: mod_base = OTHER; note = 2'-O-methyladenosine-3'-phosphate
  modified_base 21: mod_base = OTHER; note = 2'-O-methyluridine-3'-phosphate ((2S,4R)-1-[29-[[2-(acetylamino)-2-deoxy-beta-D-galactopyranosyl]oxy]-14,14-bis[[3-[[3-[[5-[[2-(acetylamino)-2-deoxy-beta-D-galactopyranosyl]oxy]-1-oxopentyl]amino]propyl]amino]-3-oxopropoxy]methyl]-1,12,19,25-tetraoxo-16-oxa-13,20,24-triazanonacos-1-yl]-4-hydroxy-2-pyrrolidinyl)methyl ester
atagcaccgttttgctaaaat

SEQ ID NO: 394 - RNA, 21 nt, synthetic construct
  source 1..21: mol_type = other RNA
  modified_base 1: mod_base = OTHER; note = 2'-O-methylguanosine-3'-phosphorothioate
  modified_base 2: mod_base = OTHER; note = 2'-O-methyladenosine-3'-phosphorothioate
  modified_base 3: mod_base = OTHER; note = 2'-O-methyluridine-3'-phosphate
  modified_base 4: mod_base = OTHER; note = 2'-O-methyladenosine-3'-phosphate
  modified_base 5: mod_base = OTHER; note = 2'-O-methylcytidine-3'-phosphate
  modified_base 6: mod_base = OTHER; note = 2'-O-methyladenosine-3'-phosphate
  modified_base 7: mod_base = OTHER; note = 2'-deoxy-2'-fluorouridine-3'-phosphate
  modified_base 8: mod_base = OTHER; note = 2'-O-methyluridine-3'-phosphate
  modified_base 9: mod_base = OTHER; note = 2'-deoxy-2'-fluorocytidine-3'-phosphate
  modified_base 10: mod_base = OTHER; note = 2'-deoxy-2'-fluorouridine-3'-phosphate
  modified_base 11: mod_base = OTHER; note = 2'-deoxy-2'-fluorocytidine-3'-phosphate
  modified_base 12: mod_base = OTHER; note = 2'-O-methyladenosine-3'-phosphate
  modified_base 13: mod_base = OTHER; note = 2'-O-methyluridine-3'-phosphate
  modified_base 14: mod_base = OTHER; note = 2'-O-methyluridine-3'-phosphate
  modified_base 15: mod_base = OTHER; note = 2'-O-methylguanosine-3'-phosphate
  modified_base 16: mod_base = OTHER; note = 2'-O-methyluridine-3'-phosphate
  modified_base 17: mod_base = OTHER; note = 2'-O-methyluridine-3'-phosphate
  modified_base 18: mod_base = OTHER; note = 2'-O-methyluridine-3'-phosphate
  modified_base 19: mod_base = OTHER; note = 2'-O-methyluridine-3'-phosphate
  modified_base 20: mod_base = OTHER; note = 2'-O-methylcytidine-3'-phosphate
  modified_base 21: mod_base = OTHER; note = 2'-O-methyluridine-3'-phosphate ((2S,4R)-1-[29-[[2-(acetylamino)-2-deoxy-beta-D-galactopyranosyl]oxy]-14,14-bis[[3-[[3-[[5-[[2-(acetylamino)-2-deoxy-beta-D-galactopyranosyl]oxy]-1-oxopentyl]amino]propyl]amino]-3-oxopropoxy]methyl]-1,12,19,25-tetraoxo-16-oxa-13,20,24-triazanonacos-1-yl]-4-hydroxy-2-pyrrolidinyl)methyl ester
gatacattctcattgttttct

SEQ ID NO: 395 - RNA, 21 nt, synthetic construct
  source 1..21: mol_type = other RNA
  modified_base 1: mod_base = OTHER; note = 2'-O-methyluridine-3'-phosphorothioate
  modified_base 2: mod_base = OTHER; note = 2'-O-methylcytidine-3'-phosphorothioate
  modified_base 3: mod_base = OTHER; note = 2'-O-methylcytidine-3'-phosphate
  modified_base 4: mod_base = OTHER; note = 2'-O-methyladenosine-3'-phosphate
  modified_base 5: mod_base = OTHER; note = 2'-O-methylcytidine-3'-phosphate
  modified_base 6: mod_base = OTHER; note = 2'-O-methyladenosine-3'-phosphate
  modified_base 7: mod_base = OTHER; note = 2'-deoxy-2'-fluorouridine-3'-phosphate
  modified_base 8: mod_base = OTHER; note = 2'-O-methyladenosine-3'-phosphate
  modified_base 9: mod_base = OTHER; note = 2'-deoxy-2'-fluoroadenosine-3'-phosphate
  modified_base 10: mod_base = OTHER; note = 2'-deoxy-2'-fluoroguanosine-3'-phosphate
  modified_base 11: mod_base = OTHER; note = 2'-deoxy-2'-fluoroguanosine-3'-phosphate
  modified_base 12: mod_base = OTHER; note = 2'-O-methyluridine-3'-phosphate
  modified_base 13: mod_base = OTHER; note = 2'-O-methyluridine-3'-phosphate
  modified_base 14: mod_base = OTHER; note = 2'-O-methyladenosine-3'-phosphate
  modified_base 15: mod_base = OTHER; note = 2'-O-methyladenosine-3'-phosphate
  modified_base 16: mod_base = OTHER; note = 2'-O-methyladenosine-3'-phosphate
  modified_base 17: mod_base = OTHER; note = 2'-O-methylcytidine-3'-phosphate
  modified_base 18: mod_base = OTHER; note = 2'-O-methyladenosine-3'-phosphate
  modified_base 19: mod_base = OTHER; note = 2'-O-methyladenosine-3'-phosphate
  modified_base 20: mod_base = OTHER; note = 2'-O-methyladenosine-3'-phosphate
  modified_base 21: mod_base = OTHER; note = 2'-O-methyluridine-3'-phosphate ((2S,4R)-1-[29-[[2-(acetylamino)-2-deoxy-beta-D-galactopyranosyl]oxy]-14,14-bis[[3-[[3-[[5-[[2-(acetylamino)-2-deoxy-beta-D-galactopyranosyl]oxy]-1-oxopentyl]amino]propyl]amino]-3-oxopropoxy]methyl]-1,12,19,25-tetraoxo-16-oxa-13,20,24-triazanonacos-1-yl]-4-hydroxy-2-pyrrolidinyl)methyl ester
tccacataaggttaaacaaat

SEQ ID NO: 396 - RNA, 21 nt, synthetic construct
  source 1..21: mol_type = other RNA
  modified_base 1: mod_base = OTHER; note = 2'-O-methyladenosine-3'-phosphorothioate
  modified_base 2: mod_base = OTHER; note = 2'-O-methylguanosine-3'-phosphorothioate
  modified_base 3: mod_base = OTHER; note = 2'-O-methylguanosine-3'-phosphate
  modified_base 4: mod_base = OTHER; note = 2'-O-methyluridine-3'-phosphate
  modified_base 5: mod_base = OTHER; note = 2'-O-methylguanosine-3'-phosphate
  modified_base 6: mod_base = OTHER; note = 2'-O-methylcytidine-3'-phosphate
  modified_base 7: mod_base = OTHER; note = 2'-deoxy-2'-fluorouridine-3'-phosphate
  modified_base 8: mod_base = OTHER; note = 2'-O-methyluridine-3'-phosphate
  modified_base 9: mod_base = OTHER; note = 2'-deoxy-2'-fluoroguanosine-3'-phosphate
  modified_base 10: mod_base = OTHER; note = 2'-deoxy-2'-fluorouridine-3'-phosphate
  modified_base 11: mod_base = OTHER; note = 2'-deoxy-2'-fluoroadenosine-3'-phosphate
  modified_base 12: mod_base = OTHER; note = 2'-O-methyladenosine-3'-phosphate
  modified_base 13: mod_base = OTHER; note = 2'-O-methyladenosine-3'-phosphate
  modified_base 14: mod_base = OTHER; note = 2'-O-methyluridine-3'-phosphate
  modified_base 15: mod_base = OTHER; note = 2'-O-methyladenosine-3'-phosphate
  modified_base 16: mod_base = OTHER; note = 2'-O-methyladenosine-3'-phosphate
  modified_base 17: mod_base = OTHER; note = 2'-O-methyluridine-3'-phosphate
  modified_base 18: mod_base = OTHER; note = 2'-O-methyluridine-3'-phosphate
  modified_base 19: mod_base = OTHER; note = 2'-O-methyluridine-3'-phosphate
  modified_base 20: mod_base = OTHER; note = 2'-O-methyladenosine-3'-phosphate
  modified_base 21: mod_base = OTHER; note = 2'-O-methyluridine-3'-phosphate ((2S,4R)-1-[29-[[2-(acetylamino)-2-deoxy-beta-D-galactopyranosyl]oxy]-14,14-bis[[3-[[3-[[5-[[2-(acetylamino)-2-deoxy-beta-D-galactopyranosyl]oxy]-1-oxopentyl]amino]propyl]amino]-3-oxopropoxy]methyl]-1,12,19,25-tetraoxo-16-oxa-13,20,24-triazanonacos-1-yl]-4-hydroxy-2-pyrrolidinyl)methyl ester
aggtgcttgtaaataatttat

SEQ ID NO: 397 - RNA, 21 nt, synthetic construct
  source 1..21: mol_type = other RNA
  modified_base 1: mod_base = OTHER; note = 2'-O-methylcytidine-3'-phosphorothioate
  modified_base 2: mod_base = OTHER; note = 2'-O-methyluridine-3'-phosphorothioate
  modified_base 3: mod_base = OTHER; note = 2'-O-methylcytidine-3'-phosphate
  modified_base 4: mod_base = OTHER; note = 2'-O-methyluridine-3'-phosphate
  modified_base 5: mod_base = OTHER; note = 2'-O-methyladenosine-3'-phosphate
  modified_base 6: mod_base = OTHER; note = 2'-O-methyluridine-3'-phosphate
  modified_base 7: mod_base = OTHER; note = 2'-deoxy-2'-fluorocytidine-3'-phosphate
  modified_base 8: mod_base = OTHER; note = 2'-O-methylguanosine-3'-phosphate
  modified_base 9: mod_base = OTHER; note = 2'-deoxy-2'-fluorocytidine-3'-phosphate
  modified_base 10: mod_base = OTHER; note = 2'-deoxy-2'-fluoroadenosine-3'-phosphate
  modified_base 11: mod_base = OTHER; note = 2'-deoxy-2'-fluorouridine-3'-phosphate
  modified_base 12: mod_base = OTHER; note = 2'-O-methyluridine-3'-phosphate
  modified_base 13: mod_base = OTHER; note = 2'-O-methyluridine-3'-phosphate
  modified_base 14: mod_base = OTHER; note = 2'-O-methylcytidine-3'-phosphate
  modified_base 15: mod_base = OTHER; note = 2'-O-methyluridine-3'-phosphate
  modified_base 16: mod_base = OTHER; note = 2'-O-methylguanosine-3'-phosphate
  modified_base 17: mod_base = OTHER; note = 2'-O-methyluridine-3'-phosphate
  modified_base 18: mod_base = OTHER; note = 2'-O-methyladenosine-3'-phosphate
  modified_base 19: mod_base = OTHER; note = 2'-O-methyladenosine-3'-phosphate
  modified_base 20: mod_base = OTHER; note = 2'-O-methylcytidine-3'-phosphate
  modified_base 21: mod_base = OTHER; note = 2'-O-methyluridine-3'-phosphate ((2S,4R)-1-[29-[[2-(acetylamino)-2-deoxy-beta-D-galactopyranosyl]oxy]-14,14-bis[[3-[[3-[[5-[[2-(acetylamino)-2-deoxy-beta-D-galactopyranosyl]oxy]-1-oxopentyl]amino]propyl]amino]-3-oxopropoxy]methyl]-1,12,19,25-tetraoxo-16-oxa-13,20,24-triazanonacos-1-yl]-4-hydroxy-2-pyrrolidinyl)methyl ester
ctctatcgcatttctgtaact

SEQ ID NO: 398 - RNA, 21 nt, synthetic construct
  source 1..21: mol_type = other RNA
  modified_base 1: mod_base = OTHER; note = 2'-O-methyladenosine-3'-phosphorothioate
  modified_base 2: mod_base = OTHER; note = 2'-O-methyladenosine-3'-phosphorothioate
  modified_base 3: mod_base = OTHER; note = 2'-O-methyladenosine-3'-phosphate
  modified_base 4: mod_base = OTHER; note = 2'-O-methyladenosine-3'-phosphate
  modified_base 5: mod_base = OTHER; note = 2'-O-methyluridine-3'-phosphate
  modified_base 6: mod_base = OTHER; note = 2'-O-methylguanosine-3'-phosphate
  modified_base 7: mod_base = OTHER; note = 2'-deoxy-2'-fluoroadenosine-3'-phosphate
  modified_base 8: mod_base = OTHER; note = 2'-O-methylguanosine-3'-phosphate
  modified_base 9: mod_base = OTHER; note = 2'-deoxy-2'-fluoroadenosine-3'-phosphate
  modified_base 10: mod_base = OTHER; note = 2'-deoxy-2'-fluoroadenosine-3'-phosphate
  modified_base 11: mod_base = OTHER; note = 2'-deoxy-2'-fluorouridine-3'-phosphate
  modified_base 12: mod_base = OTHER; note = 2'-O-methylguanosine-3'-phosphate
  modified_base 13: mod_base = OTHER; note = 2'-O-methyluridine-3'-phosphate
  modified_base 14: mod_base = OTHER; note = 2'-O-methylcytidine-3'-phosphate
  modified_base 15: mod_base = OTHER; note = 2'-O-methylcytidine-3'-phosphate
  modified_base 16: mod_base = OTHER; note = 2'-O-methyluridine-3'-phosphate
  modified_base 17: mod_base = OTHER; note = 2'-O-methyladenosine-3'-phosphate
  modified_base 18: mod_base = OTHER; note = 2'-O-methyladenosine-3'-phosphate
  modified_base 19: mod_base = OTHER; note = 2'-O-methylguanosine-3'-phosphate
  modified_base 20: mod_base = OTHER; note = 2'-O-methyluridine-3'-phosphate
  modified_base 21: mod_base = OTHER; note = 2'-O-methyluridine-3'-phosphate ((2S,4R)-1-[29-[[2-(acetylamino)-2-deoxy-beta-D-galactopyranosyl]oxy]-14,14-bis[[3-[[3-[[5-[[2-(acetylamino)-2-deoxy-beta-D-galactopyranosyl]oxy]-1-oxopentyl]amino]propyl]amino]-3-oxopropoxy]methyl]-1,12,19,25-tetraoxo-16-oxa-13,20,24-triazanonacos-1-yl]-4-hydroxy-2-pyrrolidinyl)methyl ester
aaaatgagaatgtcctaagtt

SEQ ID NO: 399 - RNA, 21 nt, synthetic construct
  source 1..21: mol_type = other RNA
  modified_base 1: mod_base = OTHER; note = 2'-O-methylcytidine-3'-phosphorothioate
  modified_base 2: mod_base = OTHER; note = 2'-O-methyladenosine-3'-phosphorothioate
  modified_base 3: mod_base = OTHER; note = 2'-O-methylcytidine-3'-phosphate
  modified_base 4: mod_base = OTHER; note = 2'-O-methyluridine-3'-phosphate
  modified_base 5: mod_base = OTHER; note = 2'-O-methylcytidine-3'-phosphate
  modified_base 6: mod_base = OTHER; note = 2'-O-methyluridine-3'-phosphate
  modified_base 7: mod_base = OTHER; note = 2'-deoxy-2'-fluoroguanosine-3'-phosphate
  modified_base 8: mod_base = OTHER; note = 2'-O-methyladenosine-3'-phosphate
  modified_base 9: mod_base = OTHER; note = 2'-deoxy-2'-fluoroadenosine-3'-phosphate
  modified_base 10: mod_base = OTHER; note = 2'-deoxy-2'-fluoroadenosine-3'-phosphate
  modified_base 11: mod_base = OTHER; note = 2'-deoxy-2'-fluoroadenosine-3'-phosphate
  modified_base 12: mod_base = OTHER; note = 2'-O-methyluridine-3'-phosphate
  modified_base 13: mod_base = OTHER; note = 2'-O-methylguanosine-3'-phosphate
  modified_base 14: mod_base = OTHER; note = 2'-O-methylcytidine-3'-phosphate
  modified_base 15: mod_base = OTHER; note = 2'-O-methyladenosine-3'-phosphate
  modified_base 16: mod_base = OTHER; note = 2'-O-methyluridine-3'-phosphate
  modified_base 17: mod_base = OTHER; note = 2'-O-methylguanosine-3'-phosphate
  modified_base 18: mod_base = OTHER; note = 2'-O-methyladenosine-3'-phosphate
  modified_base 19: mod_base = OTHER; note = 2'-O-methyladenosine-3'-phosphate
  modified_base 20: mod_base = OTHER; note = 2'-O-methyladenosine-3'-phosphate
  modified_base 21: mod_base = OTHER; note = 2'-O-methyluridine-3'-phosphate ((2S,4R)-1-[29-[[2-(acetylamino)-2-deoxy-beta-D-galactopyranosyl]oxy]-14,14-bis[[3-[[3-[[5-[[2-(acetylamino)-2-deoxy-beta-D-galactopyranosyl]oxy]-1-oxopentyl]amino]propyl]amino]-3-oxopropoxy]methyl]-1,12,19,25-tetraoxo-16-oxa-13,20,24-triazanonacos-1-yl]-4-hydroxy-2-pyrrolidinyl)methyl ester
cactctgaaaatgcatgaaat

SEQ ID NO: 400 - RNA, 21 nt, synthetic construct
  source 1..21: mol_type = other RNA
  modified_base 1: mod_base = OTHER; note = 2'-O-methyladenosine-3'-phosphorothioate
  modified_base 2: mod_base = OTHER; note = 2'-O-methyladenosine-3'-phosphorothioate
  modified_base 3: mod_base = OTHER; note = 2'-O-methyluridine-3'-phosphate
  modified_base 4: mod_base = OTHER; note = 2'-O-methylguanosine-3'-phosphate
  modified_base 5: mod_base = OTHER; note = 2'-O-methyluridine-3'-phosphate
  modified_base 6: mod_base = OTHER; note = 2'-O-methylguanosine-3'-phosphate
  modified_base 7: mod_base = OTHER; note = 2'-deoxy-2'-fluorouridine-3'-phosphate
  modified_base 8: mod_base = OTHER; note = 2'-O-methyladenosine-3'-phosphate
  modified_base 9: mod_base = OTHER; note = 2'-deoxy-2'-fluoroguanosine-3'-phosphate
  modified_base 10: mod_base = OTHER; note = 2'-deoxy-2'-fluoroadenosine-3'-phosphate
  modified_base 11: mod_base = OTHER; note = 2'-deoxy-2'-fluoroadenosine-3'-phosphate
  modified_base 12: mod_base = OTHER; note = 2'-O-methylcytidine-3'-phosphate
  modified_base 13: mod_base = OTHER; note = 2'-O-methyluridine-3'-phosphate
  modified_base 14: mod_base = OTHER; note = 2'-O-methylguanosine-3'-phosphate
  modified_base 15: mod_base = OTHER; note = 2'-O-methyluridine-3'-phosphate
  modified_base 16: mod_base = OTHER; note = 2'-O-methyluridine-3'-phosphate
  modified_base 17: mod_base = OTHER; note = 2'-O-methyladenosine-3'-phosphate
  modified_base 18: mod_base = OTHER; note = 2'-O-methyladenosine-3'-phosphate
  modified_base 19: mod_base = OTHER; note = 2'-O-methylcytidine-3'-phosphate
  modified_base 20: mod_base = OTHER; note = 2'-O-methyluridine-3'-phosphate
  modified_base 21: mod_base = OTHER; note = 2'-O-methyluridine-3'-phosphate ((2S,4R)-1-[29-[[2-(acetylamino)-2-deoxy-beta-D-galactopyranosyl]oxy]-14,14-bis[[3-[[3-[[5-[[2-(acetylamino)-2-deoxy-beta-D-galactopyranosyl]oxy]-1-oxopentyl]amino]propyl]amino]-3-oxopropoxy]methyl]-1,12,19,25-tetraoxo-16-oxa-13,20,24-triazanonacos-1-yl]-4-hydroxy-2-pyrrolidinyl)methyl ester
aatgtgtagaactgttaactt

SEQ ID NO: 401 - RNA, 21 nt, synthetic construct
  source 1..21: mol_type = other RNA
  modified_base 1: mod_base = OTHER; note = 2'-O-methylcytidine-3'-phosphorothioate
  modified_base 2: mod_base = OTHER; note = 2'-O-methyluridine-3'-phosphorothioate
  modified_base 3: mod_base = OTHER; note = 2'-O-methyluridine-3'-phosphate
  modified_base 4: mod_base = OTHER; note = 2'-O-methylcytidine-3'-phosphate
  modified_base 5: mod_base = OTHER; note = 2'-O-methyluridine-3'-phosphate
  modified_base 6: mod_base = OTHER; note = 2'-O-methylguanosine-3'-phosphate
  modified_base 7: mod_base = OTHER; note = 2'-deoxy-2'-fluoroguanosine-3'-phosphate
  modified_base 8: mod_base = OTHER; note = 2'-O-methyladenosine-3'-phosphate
  modified_base 9: mod_base = OTHER; note = 2'-deoxy-2'-fluoroadenosine-3'-phosphate
  modified_base 10: mod_base = OTHER; note = 2'-deoxy-2'-fluorouridine-3'-phosphate
  modified_base 11: mod_base = OTHER; note = 2'-deoxy-2'-fluorocytidine-3'-phosphate
  modified_base 12: mod_base = OTHER; note = 2'-O-methyluridine-3'-phosphate
  modified_base 13: mod_base = OTHER; note = 2'-O-methylguanosine-3'-phosphate
  modified_base 14: mod_base = OTHER; note = 2'-O-methyluridine-3'-phosphate
  modified_base 15: mod_base = OTHER; note = 2'-O-methyluridine-3'-phosphate
  modified_base 16: mod_base = OTHER; note = 2'-O-methyladenosine-3'-phosphate
  modified_base 17: mod_base = OTHER; note = 2'-O-methyladenosine-3'-phosphate
  modified_base 18: mod_base = OTHER; note = 2'-O-methyladenosine-3'-phosphate
  modified_base 19: mod_base = OTHER; note = 2'-O-methyluridine-3'-phosphate
  modified_base 20: mod_base = OTHER; note = 2'-O-methyluridine-3'-phosphate
  modified_base 21: mod_base = OTHER; note = 2'-O-methyluridine-3'-phosphate ((2S,4R)-1-[29-[[2-(acetylamino)-2-deoxy-beta-D-galactopyranosyl]oxy]-14,14-bis[[3-[[3-[[5-[[2-(acetylamino)-2-deoxy-beta-D-galactopyranosyl]oxy]-1-oxopentyl]amino]propyl]amino]-3-oxopropoxy]methyl]-1,12,19,25-tetraoxo-16-oxa-13,20,24-triazanonacos-1-yl]-4-hydroxy-2-pyrrolidinyl)methyl ester
cttctggaatctgttaaattt

SEQ ID NO: 402 - RNA, 21 nt, synthetic construct
  source 1..21: mol_type = other RNA
  modified_base 1: mod_base = OTHER; note = 2'-O-methylguanosine-3'-phosphorothioate
  modified_base 2: mod_base = OTHER; note = 2'-O-methyladenosine-3'-phosphorothioate
  modified_base 3: mod_base = OTHER; note = 2'-O-methylguanosine-3'-phosphate
  modified_base 4: mod_base = OTHER; note = 2'-O-methylguanosine-3'-phosphate
  modified_base 5: mod_base = OTHER; note = 2'-O-methylguanosine-3'-phosphate
  modified_base 6: mod_base = OTHER; note = 2'-O-methyluridine-3'-phosphate
  modified_base 7: mod_base = OTHER; note = 2'-deoxy-2'-fluoroadenosine-3'-phosphate
  modified_base 8: mod_base = OTHER; note = 2'-O-methyladenosine-3'-phosphate
  modified_base 9: mod_base = OTHER; note = 2'-deoxy-2'-fluoroadenosine-3'-phosphate
  modified_base 10: mod_base = OTHER; note = 2'-deoxy-2'-fluorouridine-3'-phosphate
  modified_base 11: mod_base = OTHER; note = 2'-deoxy-2'-fluoroguanosine-3'-phosphate
  modified_base 12: mod_base = OTHER; note = 2'-O-methylguanosine-3'-phosphate
  modified_base 13: mod_base = OTHER; note = 2'-O-methyladenosine-3'-phosphate
  modified_base 14: mod_base = OTHER; note = 2'-O-methylguanosine-3'-phosphate
  modified_base 15: mod_base = OTHER; note = 2'-O-methyladenosine-3'-phosphate
  modified_base 16: mod_base = OTHER; note = 2'-O-methyladenosine-3'-phosphate
  modified_base 17: mod_base = OTHER; note = 2'-O-methyladenosine-3'-phosphate
  modified_base 18: mod_base = OTHER; note = 2'-O-methyladenosine-3'-phosphate
  modified_base 19: mod_base = OTHER; note = 2'-O-methyluridine-3'-phosphate
  modified_base 20: mod_base = OTHER; note = 2'-O-methyladenosine-3'-phosphate
  modified_base 21: mod_base = OTHER; note = 2'-O-methyluridine-3'-phosphate ((2S,4R)-1-[29-[[2-(acetylamino)-2-deoxy-beta-D-galactopyranosyl]oxy]-14,14-bis[[3-[[3-[[5-[[2-(acetylamino)-2-deoxy-beta-D-galactopyranosyl]oxy]-1-oxopentyl]amino]propyl]amino]-3-oxopropoxy]methyl]-1,12,19,25-tetraoxo-16-oxa-13,20,24-triazanonacos-1-yl]-4-hydroxy-2-pyrrolidinyl)methyl ester
gagggtaaatggagaaaatat

SEQ ID NO: 403 - RNA, 21 nt, synthetic construct
  source 1..21: mol_type = other RNA
  modified_base 1: mod_base = OTHER; note = 2'-O-methyluridine-3'-phosphorothioate
  modified_base 2: mod_base = OTHER; note = 2'-O-methylguanosine-3'-phosphorothioate
  modified_base 3: mod_base = OTHER; note = 2'-O-methylguanosine-3'-phosphate
  modified_base 4: mod_base = OTHER; note = 2'-O-methylguanosine-3'-phosphate
  modified_base 5: mod_base = OTHER; note = 2'-O-methyladenosine-3'-phosphate
  modified_base 6: mod_base = OTHER; note = 2'-O-methyluridine-3'-phosphate
  modified_base 7: mod_base = OTHER; note = 2'-deoxy-2'-fluorouridine-3'-phosphate
  modified_base 8: mod_base = OTHER; note = 2'-O-methyladenosine-3'-phosphate
  modified_base 9: mod_base = OTHER; note = 2'-deoxy-2'-fluorocytidine-3'-phosphate
  modified_base 10: mod_base = OTHER; note = 2'-deoxy-2'-fluoroadenosine-3'-phosphate
  modified_base 11: mod_base = OTHER; note = 2'-deoxy-2'-fluoroadenosine-3'-phosphate
  modified_base 12: mod_base = OTHER; note = 2'-O-methyluridine-3'-phosphate
  modified_base 13: mod_base = OTHER; note = 2'-O-methylguanosine-3'-phosphate
  modified_base 14: mod_base = OTHER; note = 2'-O-methyladenosine-3'-phosphate
  modified_base 15: mod_base = OTHER; note = 2'-O-methyladenosine-3'-phosphate
  modified_base 16: mod_base = OTHER; note = 2'-O-methyluridine-3'-phosphate
  modified_base 17: mod_base = OTHER; note = 2'-O-methylguanosine-3'-phosphate
  modified_base 18: mod_base = OTHER; note = 2'-O-methyluridine-3'-phosphate
  modified_base 19: mod_base = OTHER; note = 2'-O-methyladenosine-3'-phosphate
  modified_base 20: mod_base = OTHER; note = 2'-O-methyladenosine-3'-phosphate
  modified_base 21: mod_base = OTHER; note = 2'-O-methyluridine-3'-phosphate ((2S,4R)-1-[29-[[2-(acetylamino)-2-deoxy-beta-D-galactopyranosyl]oxy]-14,14-bis[[3-[[3-[[5-[[2-(acetylamino)-2-deoxy-beta-D-galactopyranosyl]oxy]-1-oxopentyl]amino]propyl]amino]-3-oxopropoxy]methyl]-1,12,19,25-tetraoxo-16-oxa-13,20,24-triazanonacos-1-yl]-4-hydroxy-2-pyrrolidinyl)methyl ester
tgggattacaatgaatgtaat

SEQ ID NO: 404 - RNA, 21 nt, synthetic construct
  source 1..21: mol_type = other RNA
  modified_base 1: mod_base = OTHER; note = 2'-O-methyluridine-3'-phosphorothioate
  modified_base 2: mod_base = OTHER; note = 2'-O-methyladenosine-3'-phosphorothioate
  modified_base 3: mod_base = OTHER; note = 2'-O-methyladenosine-3'-phosphate
  modified_base 4: mod_base = OTHER; note = 2'-O-methylguanosine-3'-phosphate
  modified_base 5: mod_base = OTHER; note = 2'-O-methylcytidine-3'-phosphate
  modified_base 6: mod_base = OTHER; note = 2'-O-methylcytidine-3'-phosphate
  modified_base 7: mod_base = OTHER; note = 2'-deoxy-2'-fluorocytidine-3'-phosphate
  modified_base 8: mod_base = OTHER; note = 2'-O-methyladenosine-3'-phosphate
  modified_base 9: mod_base = OTHER; note = 2'-deoxy-2'-fluoroadenosine-3'-phosphate
  modified_base 10: mod_base = OTHER; note = 2'-deoxy-2'-fluoroadenosine-3'-phosphate
  modified_base 11: mod_base = OTHER; note = 2'-deoxy-2'-fluorouridine-3'-phosphate
  modified_base 12: mod_base = OTHER; note = 2'-O-methyluridine-3'-phosphate
  modified_base 13: mod_base = OTHER; note = 2'-O-methylguanosine-3'-phosphate
  modified_base 14: mod_base = OTHER; note = 2'-O-methyluridine-3'-phosphate
  modified_base 15: mod_base = OTHER; note = 2'-O-methylguanosine-3'-phosphate
  modified_base 16: mod_base = OTHER; note = 2'-O-methylguanosine-3'-phosphate
  modified_base 17: mod_base = OTHER; note = 2'-O-methyladenosine-3'-phosphate
  modified_base 18: mod_base = OTHER; note = 2'-O-methyladenosine-3'-phosphate
  modified_base 19: mod_base = OTHER; note = 2'-O-methyluridine-3'-phosphate
  modified_base 20: mod_base = OTHER; note = 2'-O-methyluridine-3'-phosphate
  modified_base 21: mod_base = OTHER; note = 2'-O-methyluridine-3'-phosphate ((2S,4R)-1-[29-[[2-(acetylamino)-2-deoxy-beta-D-galactopyranosyl]oxy]-14,14-bis[[3-[[3-[[5-[[2-(acetylamino)-2-deoxy-beta-D-galactopyranosyl]oxy]-1-oxopentyl]amino]propyl]amino]-3-oxopropoxy]methyl]-1,12,19,25-tetraoxo-16-oxa-13,20,24-triazanonacos-1-yl]-4-hydroxy-2-pyrrolidinyl)methyl ester
taagcccaaattgtggaattt

SEQ ID NO: 405 - RNA, 21 nt, synthetic construct
  source 1..21: mol_type = other RNA
  modified_base 1: mod_base = OTHER; note = 2'-O-methyluridine-3'-phosphorothioate
  modified_base 2: mod_base = OTHER; note = 2'-O-methylcytidine-3'-phosphorothioate
  modified_base 3: mod_base = OTHER; note = 2'-O-methyladenosine-3'-phosphate
  modified_base 4: mod_base = OTHER; note = 2'-O-methyluridine-3'-phosphate
  modified_base 5: mod_base = OTHER; note = 2'-O-methylcytidine-3'-phosphate
  modified_base 6: mod_base = OTHER; note = 2'-O-methyladenosine-3'-phosphate
  modified_base 7: mod_base = OTHER; note = 2'-deoxy-2'-fluoroguanosine-3'-phosphate
  modified_base 8: mod_base = OTHER; note = 2'-O-methyluridine-3'-phosphate
  modified_base 9: mod_base = OTHER; note = 2'-deoxy-2'-fluoroguanosine-3'-phosphate
  modified_base 10: mod_base = OTHER; note = 2'-deoxy-2'-fluorouridine-3'-phosphate
  modified_base 11: mod_base = OTHER; note = 2'-deoxy-2'-fluorouridine-3'-phosphate
  modified_base 12: mod_base = OTHER; note = 2'-O-methyluridine-3'-phosphate
  modified_base 13: mod_base = OTHER; note = 2'-O-methyluridine-3'-phosphate
  modified_base 14: mod_base = OTHER; note = 2'-O-methyladenosine-3'-phosphate
  modified_base 15: mod_base = OTHER; note = 2'-O-methyluridine-3'-phosphate
  modified_base 16: mod_base = OTHER; note = 2'-O-methyladenosine-3'-phosphate
  modified_base 17: mod_base = OTHER; note = 2'-O-methylguanosine-3'-phosphate
  modified_base 18: mod_base = OTHER; note = 2'-O-methyladenosine-3'-phosphate
  modified_base 19: mod_base = OTHER; note = 2'-O-methyladenosine-3'-phosphate
  modified_base 20: mod_base = OTHER; note = 2'-O-methyladenosine-3'-phosphate
  modified_base 21: mod_base = OTHER; note = 2'-O-methyluridine-3'-phosphate ((2S,4R)-1-[29-[[2-(acetylamino)-2-deoxy-beta-D-galactopyranosyl]oxy]-14,14-bis[[3-[[3-[[5-[[2-(acetylamino)-2-deoxy-beta-D-galactopyranosyl]oxy]-1-oxopentyl]amino]propyl]amino]-3-oxopropoxy]methyl]-1,12,19,25-tetraoxo-16-oxa-13,20,24-triazanonacos-1-yl]-4-hydroxy-2-pyrrolidinyl)methyl ester
tcatcagtgttttatagaaat

SEQ ID NO: 406 - RNA, 21 nt, synthetic construct
  source 1..21: mol_type = other RNA
  modified_base 1: mod_base = OTHER; note = 2'-O-methyladenosine-3'-phosphorothioate
  modified_base 2: mod_base = OTHER; note = 2'-O-methyluridine-3'-phosphorothioate
  modified_base 3: mod_base = OTHER; note = 2'-O-methyluridine-3'-phosphate
  modified_base 4: mod_base = OTHER; note = 2'-O-methylguanosine-3'-phosphate
  modified_base 5: mod_base = OTHER; note = 2'-O-methylcytidine-3'-phosphate
  modified_base 6: mod_base = OTHER; note = 2'-O-methylcytidine-3'-phosphate
  modified_base 7: mod_base = OTHER; note = 2'-deoxy-2'-fluorocytidine-3'-phosphate
  modified_base 8: mod_base = OTHER; note = 2'-O-methyladenosine-3'-phosphate
  modified_base 9: mod_base = OTHER; note = 2'-deoxy-2'-fluoroadenosine-3'-phosphate
  modified_base 10: mod_base = OTHER; note = 2'-deoxy-2'-fluoroadenosine-3'-phosphate
  modified_base 11: mod_base = OTHER; note = 2'-deoxy-2'-fluorocytidine-3'-phosphate
  modified_base 12: mod_base = OTHER; note = 2'-O-methyluridine-3'-phosphate
  modified_base 13: mod_base = OTHER; note = 2'-O-methyladenosine-3'-phosphate
  modified_base 14: mod_base = OTHER; note = 2'-O-methyluridine-3'-phosphate
  modified_base 15: mod_base = OTHER; note = 2'-O-methyluridine-3'-phosphate
  modified_base 16: mod_base = OTHER; note = 2'-O-methyluridine-3'-phosphate
  modified_base 17: mod_base = OTHER; note = 2'-O-methyluridine-3'-phosphate
  modified_base 18: mod_base = OTHER; note = 2'-O-methylguanosine-3'-phosphate
  modified_base 19: mod_base = OTHER; note = 2'-O-methyladenosine-3'-phosphate
  modified_base 20: mod_base = OTHER; note = 2'-O-methylcytidine-3'-phosphate
  modified_base 21: mod_base = OTHER; note = 2'-O-methyluridine-3'-phosphate ((2S,4R)-1-[29-[[2-(acetylamino)-2-deoxy-beta-D-galactopyranosyl]oxy]-14,14-bis[[3-[[3-[[5-[[2-(acetylamino)-2-deoxy-beta-D-galactopyranosyl]oxy]-1-oxopentyl]amino]propyl]amino]-3-oxopropoxy]methyl]-1,12,19,25-tetraoxo-16-oxa-13,20,24-triazanonacos-1-yl]-4-hydroxy-2-pyrrolidinyl)methyl ester
attgcccaaactattttgact

SEQ ID NO: 407 - RNA, 21 nt, synthetic construct
  source 1..21: mol_type = other RNA
  modified_base 1: mod_base = OTHER; note = 2'-O-methyladenosine-3'-phosphorothioate
  modified_base 2: mod_base = OTHER; note = 2'-O-methylcytidine-3'-phosphorothioate
  modified_base 3: mod_base = OTHER; note = 2'-O-methyluridine-3'-phosphate
  modified_base 4: mod_base = OTHER; note = 2'-O-methyluridine-3'-phosphate
  modified_base 5: mod_base = OTHER; note = 2'-O-methyladenosine-3'-phosphate
  modified_base 6: mod_base = OTHER; note = 2'-O-methyluridine-3'-phosphate
  modified_base 7: mod_base = OTHER; note = 2'-deoxy-2'-fluoroguanosine-3'-phosphate
  modified_base 8: mod_base = OTHER; note = 2'-O-methyladenosine-3'-phosphate
  modified_base 9: mod_base = OTHER; note = 2'-deoxy-2'-fluoroadenosine-3'-phosphate
  modified_base 10: mod_base = OTHER; note = 2'-deoxy-2'-fluorocytidine-3'-phosphate
  modified_base 11: mod_base = OTHER; note = 2'-deoxy-2'-fluorocytidine-3'-phosphate
  modified_base 12: mod_base = OTHER; note = 2'-O-methyluridine-3'-phosphate
  modified_base 13: mod_base = OTHER; note = 2'-O-methylcytidine-3'-phosphate
  modified_base 14: mod_base = OTHER; note = 2'-O-methyluridine-3'-phosphate
  modified_base 15: mod_base = OTHER; note = 2'-O-methylcytidine-3'-phosphate
  modified_base 16: mod_base = OTHER; note = 2'-O-methyladenosine-3'-phosphate
  modified_base 17: mod_base = OTHER; note = 2'-O-methylcytidine-3'-phosphate
  modified_base 18: mod_base = OTHER; note = 2'-O-methyluridine-3'-phosphate
  modified_base 19: mod_base = OTHER; note = 2'-O-methyladenosine-3'-phosphate
  modified_base 20: mod_base = OTHER; note = 2'-O-methyladenosine-3'-phosphate
  modified_base 21: mod_base = OTHER; note = 2'-O-methyluridine-3'-phosphate ((2S,4R)-1-[29-[[2-(acetylamino)-2-deoxy-beta-D-galactopyranosyl]oxy]-14,14-bis[[3-[[3-[[5-[[2-(acetylamino)-2-deoxy-beta-D-galactopyranosyl]oxy]-1-oxopentyl]amino]propyl]amino]-3-oxopropoxy]methyl]-1,12,19,25-tetraoxo-16-oxa-13,20,24-triazanonacos-1-yl]-4-hydroxy-2-pyrrolidinyl)methyl ester
acttatgaacctctcactaat

SEQ ID NO: 408 - RNA, 21 nt, synthetic construct
  source 1..21: mol_type = other RNA
  modified_base 1: mod_base = OTHER; note = 2'-O-methyluridine-3'-phosphorothioate
  modified_base 2: mod_base = OTHER; note = 2'-O-methyluridine-3'-phosphorothioate
  modified_base 3: mod_base = OTHER; note = 2'-O-methylguanosine-3'-phosphate
  modified_base 4: mod_base = OTHER; note = 2'-O-methylguanosine-3'-phosphate
  modified_base 5: mod_base = OTHER; note = 2'-O-methylguanosine-3'-phosphate
  modified_base 6: mod_base = OTHER; note = 2'-O-methyladenosine-3'-phosphate
  modified_base 7: mod_base = OTHER; note = 2'-deoxy-2'-fluoroadenosine-3'-phosphate
  modified_base 8: mod_base = OTHER; note = 2'-O-methyladenosine-3'-phosphate
  modified_base 9: mod_base = OTHER; note = 2'-deoxy-2'-fluorocytidine-3'-phosphate
  modified_base 10: mod_base = OTHER; note = 2'-deoxy-2'-fluoroadenosine-3'-phosphate
  modified_base 11: mod_base = OTHER; note = 2'-deoxy-2'-fluorocytidine-3'-phosphate
  modified_base 12: mod_base = OTHER; note = 2'-O-methyluridine-3'-phosphate
  modified_base 13: mod_base = OTHER; note = 2'-O-methyladenosine-3'-phosphate
  modified_base 14: mod_base = OTHER; note = 2'-O-methyluridine-3'-phosphate
  modified_base 15: mod_base = OTHER; note = 2'-O-methylguanosine-3'-phosphate
  modified_base 16: mod_base = OTHER; note = 2'-O-methyluridine-3'-phosphate
  modified_base 17: mod_base = OTHER; note = 2'-O-methyluridine-3'-phosphate
  modified_base 18: mod_base = OTHER; note = 2'-O-methyladenosine-3'-phosphate
  modified_base 19: mod_base = OTHER; note = 2'-O-methylguanosine-3'-phosphate
  modified_base 20: mod_base = OTHER; note = 2'-O-methyladenosine-3'-phosphate
  modified_base 21: mod_base = OTHER; note = 2'-O-methyluridine-3'-phosphate ((2S,4R)-1-[29-[[2-(acetylamino)-2-deoxy-beta-D-galactopyranosyl]oxy]-14,14-bis[[3-[[3-[[5-[[2-(acetylamino)-2-deoxy-beta-D-galactopyranosyl]oxy]-1-oxopentyl]amino]propyl]amino]-3-oxopropoxy]methyl]-1,12,19,25-tetraoxo-16-oxa-13,20,24-triazanonacos-1-yl]-4-hydroxy-2-pyrrolidinyl)methyl ester
ttgggaaacactatgttagat

SEQ ID NO: 409 - RNA, 21 nt, synthetic construct
  source 1..21: mol_type = other RNA
  modified_base 1: mod_base = OTHER; note = 2'-O-methyladenosine-3'-phosphorothioate
  modified_base 2: mod_base = OTHER; note = 2'-O-methylguanosine-3'-phosphorothioate
  modified_base 3: mod_base = OTHER; note = 2'-O-methyluridine-3'-phosphate
  modified_base 4: mod_base = OTHER; note = 2'-O-methyluridine-3'-phosphate
  modified_base 5: mod_base = OTHER; note = 2'-O-methylcytidine-3'-phosphate
  modified_base 6: mod_base = OTHER; note = 2'-O-methyluridine-3'-phosphate
  modified_base 7: mod_base = OTHER; note = 2'-deoxy-2'-fluorouridine-3'-phosphate
  modified_base 8: mod_base = OTHER; note = 2'-O-methyluridine-3'-phosphate
  modified_base 9: mod_base = OTHER; note = 2'-deoxy-2'-fluoroadenosine-3'-phosphate
  modified_base 10: mod_base = OTHER; note = 2'-deoxy-2'-fluoroadenosine-3'-phosphate
  modified_base 11: mod_base = OTHER; note = 2'-deoxy-2'-fluoroguanosine-3'-phosphate
  modified_base 12: mod_base = OTHER; note = 2'-O-methylguanosine-3'-phosphate
  modified_base 13: mod_base = OTHER; note = 2'-O-methyladenosine-3'-phosphate
  modified_base 14: mod_base = OTHER; note = 2'-O-methylguanosine-3'-phosphate
  modified_base 15: mod_base = OTHER; note = 2'-O-methyladenosine-3'-phosphate
  modified_base 16: mod_base = OTHER; note = 2'-O-methylcytidine-3'-phosphate
  modified_base 17: mod_base = OTHER; note = 2'-O-methyladenosine-3'-phosphate
  modified_base 18: mod_base = OTHER; note = 2'-O-methyladenosine-3'-phosphate
  modified_base 19: mod_base = OTHER; note = 2'-O-methyladenosine-3'-phosphate
  modified_base 20: mod_base = OTHER; note = 2'-O-methyladenosine-3'-phosphate
  modified_base 21: mod_base = OTHER; note = 2'-O-methyluridine-3'-phosphate ((2S,4R)-1-[29-[[2-(acetylamino)-2-deoxy-beta-D-galactopyranosyl]oxy]-14,14-bis[[3-[[3-[[5-[[2-(acetylamino)-2-deoxy-beta-D-galactopyranosyl]oxy]-1-oxopentyl]amino]propyl]amino]-3-oxopropoxy]methyl]-1,12,19,25-tetraoxo-16-oxa-13,20,24-triazanonacos-1-yl]-4-hydroxy-2-pyrrolidinyl)methyl ester
agttctttaaggagacaaaat

SEQ ID NO: 410 - RNA, 21 nt, synthetic construct
  source 1..21: mol_type = other RNA
  modified_base 1: mod_base = OTHER; note = 2'-O-methyladenosine-3'-phosphorothioate
  modified_base 2: mod_base = OTHER; note = 2'-O-methyluridine-3'-phosphorothioate
  modified_base 3: mod_base = OTHER; note = 2'-O-methyladenosine-3'-phosphate
  modified_base 4: mod_base = OTHER; note = 2'-O-methyluridine-3'-phosphate
  modified_base 5: mod_base = OTHER; note = 2'-O-methylguanosine-3'-phosphate
  modified_base 6: mod_base = OTHER; note = 2'-O-methylcytidine-3'-phosphate
  modified_base 7: mod_base = OTHER; note = 2'-deoxy-2'-fluoroadenosine-3'-phosphate
  modified_base 8: mod_base = OTHER; note = 2'-O-methyluridine-3'-phosphate
  modified_base 9: mod_base = OTHER; note = 2'-deoxy-2'-fluoroguanosine-3'-phosphate
  modified_base 10: mod_base = OTHER; note = 2'-deoxy-2'-fluorocytidine-3'-phosphate
  modified_base 11: mod_base = OTHER; note = 2'-deoxy-2'-fluoroadenosine-3'-phosphate
  modified_base 12: mod_base = OTHER; note = 2'-O-methyluridine-3'-phosphate
  modified_base 13: mod_base = OTHER; note = 2'-O-methyluridine-3'-phosphate
  modified_base 14: mod_base = OTHER; note = 2'-O-methyluridine-3'-phosphate
  modified_base 15: mod_base = OTHER; note = 2'-O-methyluridine-3'-phosphate
  modified_base 16: mod_base = OTHER; note = 2'-O-methylguanosine-3'-phosphate
  modified_base 17: mod_base = OTHER; note = 2'-O-methyluridine-3'-phosphate
  modified_base 18: mod_base = OTHER; note = 2'-O-methyladenosine-3'-phosphate
  modified_base 19: mod_base = OTHER; note = 2'-O-methyladenosine-3'-phosphate
  modified_base 20: mod_base = OTHER; note = 2'-O-methylcytidine-3'-phosphate
  modified_base 21: mod_base = OTHER; note = 2'-O-methyluridine-3'-phosphate ((2S,4R)-1-[29-[[2-(acetylamino)-2-deoxy-beta-D-galactopyranosyl]oxy]-14,14-bis[[3-[[3-[[5-[[2-(acetylamino)-2-deoxy-beta-D-galactopyranosyl]oxy]-1-oxopentyl]amino]propyl]amino]-3-oxopropoxy]methyl]-1,12,19,25-tetraoxo-16-oxa-13,20,24-triazanonacos-1-yl]-4-hydroxy-2-pyrrolidinyl)methyl ester
atatgcatgcattttgtaact

SEQ ID NO: 411 - RNA, 21 nt, synthetic construct
  source 1..21: mol_type = other RNA
  modified_base 1: mod_base = OTHER; note = 2'-O-methylcytidine-3'-phosphorothioate
  modified_base 2: mod_base = OTHER; note = 2'-O-methylguanosine-3'-phosphorothioate
  modified_base 3: mod_base = OTHER; note = 2'-O-methyluridine-3'-phosphate
  modified_base 4: mod_base = OTHER; note = 2'-O-methyluridine-3'-phosphate
  modified_base 5: mod_base = OTHER; note = 2'-O-methylguanosine-3'-phosphate
  modified_base 6: mod_base = OTHER; note = 2'-O-methyladenosine-3'-phosphate
  modified_base 7: mod_base = OTHER; note = 2'-deoxy-2'-fluoroadenosine-3'-phosphate
  modified_base 8: mod_base = OTHER; note = 2'-O-methyluridine-3'-phosphate
  modified_base 9: mod_base = OTHER; note = 2'-deoxy-2'-fluoroadenosine-3'-phosphate
  modified_base 10: mod_base = OTHER; note = 2'-deoxy-2'-fluoroguanosine-3'-phosphate
  modified_base 11: mod_base = OTHER; note = 2'-deoxy-2'-fluoroadenosine-3'-phosphate
  modified_base 12: mod_base = OTHER; note = 2'-O-methyluridine-3'-phosphate
  modified_base 13: mod_base = OTHER; note = 2'-O-methylguanosine-3'-phosphate
  modified_base 14: mod_base = OTHER; note = 2'-O-methyluridine-3'-phosphate
  modified_base 15: mod_base = OTHER; note = 2'-O-methylguanosine-3'-phosphate
  modified_base 16: mod_base = OTHER; note = 2'-O-methyluridine-3'-phosphate
  modified_base 17: mod_base = OTHER; note = 2'-O-methyladenosine-3'-phosphate
  modified_base 18: mod_base = OTHER; note = 2'-O-methyluridine-3'-phosphate
  modified_base 19: mod_base = OTHER; note = 2'-O-methyluridine-3'-phosphate
  modified_base 20: mod_base = OTHER; note = 2'-O-methyluridine-3'-phosphate
  modified_base 21: mod_base = OTHER; note = 2'-O-methyluridine-3'-phosphate ((2S,4R)-1-[29-[[2-(acetylamino)-2-deoxy-beta-D-galactopyranosyl]oxy]-14,14-bis[[3-[[3-[[5-[[2-(acetylamino)-2-deoxy-beta-D-galactopyranosyl]oxy]-1-oxopentyl]amino]propyl]amino]-3-oxopropoxy]methyl]-1,12,19,25-tetraoxo-16-oxa-13,20,24-triazanonacos-1-yl]-4-hydroxy-2-pyrrolidinyl)methyl ester
cgttgaatagatgtgtatttt

SEQ ID NO: 412 - RNA, 21 nt, synthetic construct
  source 1..21: mol_type = other RNA
  modified_base 1: mod_base = OTHER; note = 2'-O-methylguanosine-3'-phosphorothioate
  modified_base 2: mod_base = OTHER; note = 2'-O-methyladenosine-3'-phosphorothioate
  modified_base 3: mod_base = OTHER; note = 2'-O-methyladenosine-3'-phosphate
  modified_base 4: mod_base = OTHER; note = 2'-O-methyladenosine-3'-phosphate
  modified_base 5: mod_base = OTHER; note = 2'-O-methyladenosine-3'-phosphate
  modified_base 6: mod_base = OTHER; note = 2'-O-methyluridine-3'-phosphate
  modified_base 7: mod_base = OTHER; note = 2'-deoxy-2'-fluoroadenosine-3'-phosphate
  modified_base 8: mod_base = OTHER; note = 2'-O-methyladenosine-3'-phosphate
  modified_base 9: mod_base = OTHER; note = 2'-deoxy-2'-fluoroguanosine-3'-phosphate
  modified_base 10: mod_base = OTHER; note = 2'-deoxy-2'-fluorocytidine-3'-phosphate
  modified_base 11: mod_base = OTHER; note = 2'-deoxy-2'-fluoroadenosine-3'-phosphate
  modified_base 12: mod_base = OTHER; note = 2'-O-methylcytidine-3'-phosphate
  modified_base 13: mod_base = OTHER; note = 2'-O-methyladenosine-3'-phosphate
  modified_base 14: mod_base = OTHER; note = 2'-O-methylguanosine-3'-phosphate
  modified_base 15: mod_base = OTHER; note = 2'-O-methyladenosine-3'-phosphate
  modified_base 16: mod_base = OTHER; note = 2'-O-methyladenosine-3'-phosphate
  modified_base 17: mod_base = OTHER; note = 2'-O-methyladenosine-3'-phosphate
  modified_base 18: mod_base = OTHER; note = 2'-O-methyladenosine-3'-phosphate
  modified_base 19: mod_base = OTHER; note = 2'-O-methyluridine-3'-phosphate
  modified_base 20: mod_base = OTHER; note = 2'-O-methyluridine-3'-phosphate
  modified_base 21: mod_base = OTHER; note = 2'-O-methyluridine-3'-phosphate ((2S,4R)-1-[29-[[2-(acetylamino)-2-deoxy-beta-D-galactopyranosyl]oxy]-14,14-bis[[3-[[3-[[5-[[2-(acetylamino)-2-deoxy-beta-D-galactopyranosyl]oxy]-1-oxopentyl]amino]propyl]amino]-3-oxopropoxy]methyl]-1,12,19,25-tetraoxo-16-oxa-13,20,24-triazanonacos-1-yl]-4-hydroxy-2-pyrrolidinyl)methyl ester
gaaaataagcacagaaaattt

SEQ ID NO: 413 - RNA, 21 nt, synthetic construct
  source 1..21: mol_type = other RNA
  modified_base 1: mod_base = OTHER; note = 2'-O-methyluridine-3'-phosphorothioate
  modified_base 2: mod_base = OTHER; note = 2'-O-methyluridine-3'-phosphorothioate
  modified_base 3: mod_base = OTHER; note = 2'-O-methylcytidine-3'-phosphate
  modified_base 4: mod_base = OTHER; note = 2'-O-methyladenosine-3'-phosphate
  modified_base 5: mod_base = OTHER; note = 2'-O-methylcytidine-3'-phosphate
  modified_base 6: mod_base = OTHER; note = 2'-O-methyluridine-3'-phosphate
  modified_base 7: mod_base = OTHER; note = 2'-deoxy-2'-fluoroguanosine-3'-phosphate
  modified_base 8: mod_base = OTHER; note = 2'-O-methyladenosine-3'-phosphate
  modified_base 9: mod_base = OTHER; note = 2'-deoxy-2'-fluoroadenosine-3'-phosphate
  modified_base 10: mod_base = OTHER; note = 2'-deoxy-2'-fluorocytidine-3'-phosphate
  modified_base 11: mod_base = OTHER; note = 2'-deoxy-2'-fluoroguanosine-3'-phosphate
  modified_base 12: mod_base = OTHER; note = 2'-O-methyluridine-3'-phosphate
  modified_base 13: mod_base = OTHER; note = 2'-O-methyladenosine-3'-phosphate
  modified_base 14: mod_base = OTHER; note = 2'-O-methyluridine-3'-phosphate
  modified_base 15: mod_base = OTHER; note = 2'-O-methylcytidine-3'-phosphate
  modified_base 16: mod_base = OTHER; note = 2'-O-methyladenosine-3'-phosphate
  modified_base 17: mod_base = OTHER; note = 2'-O-methylguanosine-3'-phosphate
  modified_base 18: mod_base = OTHER; note = 2'-O-methyladenosine-3'-phosphate
  modified_base 19: mod_base = OTHER; note = 2'-O-methyladenosine-3'-phosphate
  modified_base 20: mod_base = OTHER; note = 2'-O-methyluridine-3'-phosphate
  modified_base 21: mod_base = OTHER; note = 2'-O-methyluridine-3'-phosphate ((2S,4R)-1-[29-[[2-(acetylamino)-2-deoxy-beta-D-galactopyranosyl]oxy]-14,14-bis[[3-[[3-[[5-[[2-(acetylamino)-2-deoxy-beta-D-galactopyranosyl]oxy]-1-oxopentyl]amino]propyl]amino]-3-oxopropoxy]methyl]-1,12,19,25-tetraoxo-16-oxa-13,20,24-triazanonacos-1-yl]-4-hydroxy-2-pyrrolidinyl)methyl ester
ttcactgaacgtatcagaatt

SEQ ID NO: 414 - RNA, 21 nt, synthetic construct
  source 1..21: mol_type = other RNA
  modified_base 1: mod_base = OTHER; note = 2'-O-methyluridine-3'-phosphorothioate
  modified_base 2: mod_base = OTHER; note = 2'-O-methyladenosine-3'-phosphorothioate
  modified_base 3: mod_base = OTHER; note = 2'-O-methyladenosine-3'-phosphate
  modified_base 4: mod_base = OTHER; note = 2'-O-methyladenosine-3'-phosphate
  modified_base 5: mod_base = OTHER; note = 2'-O-methyluridine-3'-phosphate
  modified_base 6: mod_base = OTHER; note = 2'-O-methyladenosine-3'-phosphate
  modified_base 7: mod_base = OTHER; note = 2'-deoxy-2'-fluoroadenosine-3'-phosphate
  modified_base 8: mod_base = OTHER; note = 2'-O-methylguanosine-3'-phosphate
  modified_base 9: mod_base = OTHER; note = 2'-deoxy-2'-fluoroguanosine-3'-phosphate
  modified_base 10: mod_base = OTHER; note = 2'-deoxy-2'-fluorouridine-3'-phosphate
  modified_base 11: mod_base = OTHER; note = 2'-deoxy-2'-fluorouridine-3'-phosphate
  modified_base 12: mod_base = OTHER; note = 2'-O-methyluridine-3'-phosphate
  modified_base 13: mod_base = OTHER; note = 2'-O-methyluridine-3'-phosphate
  modified_base 14: mod_base = OTHER; note = 2'-O-methyladenosine-3'-phosphate
  modified_base 15: mod_base = OTHER; note = 2'-O-methyladenosine-3'-phosphate
  modified_base 16: mod_base = OTHER; note = 2'-O-methyluridine-3'-phosphate
  modified_base 17: mod_base = OTHER; note = 2'-O-methyluridine-3'-phosphate
  modified_base 18: mod_base = OTHER; note = 2'-O-methylcytidine-3'-phosphate
  modified_base 19: mod_base = OTHER; note = 2'-O-methyladenosine-3'-phosphate
  modified_base 20: mod_base = OTHER; note = 2'-O-methylguanosine-3'-phosphate
  modified_base 21: mod_base = OTHER; note = 2'-O-methyluridine-3'-phosphate ((2S,4R)-1-[29-[[2-(acetylamino)-2-deoxy-beta-D-galactopyranosyl]oxy]-14,14-bis[[3-[[3-[[5-[[2-(acetylamino)-2-deoxy-beta-D-galactopyranosyl]oxy]-1-oxopentyl]amino]propyl]amino]-3-oxopropoxy]methyl]-1,12,19,25-tetraoxo-16-oxa-13,20,24-triazanonacos-1-yl]-4-hydroxy-2-pyrrolidinyl)methyl ester
taaataaggttttaattcagt

SEQ ID NO: 415 - RNA, 21 nt, synthetic construct
  source 1..21: mol_type = other RNA
  modified_base 1: mod_base = OTHER; note = 2'-O-methylcytidine-3'-phosphorothioate
  modified_base 2: mod_base = OTHER; note = 2'-O-methyladenosine-3'-phosphorothioate
  modified_base 3: mod_base = OTHER; note = 2'-O-methylguanosine-3'-phosphate
  modified_base 4: mod_base = OTHER; note = 2'-O-methyladenosine-3'-phosphate
  modified_base 5: mod_base = OTHER; note = 2'-O-methyluridine-3'-phosphate
  modified_base 6: mod_base = OTHER; note = 2'-O-methylcytidine-3'-phosphate
  modified_base 7: mod_base = OTHER; note = 2'-deoxy-2'-fluorouridine-3'-phosphate
  modified_base 8: mod_base = OTHER; note = 2'-O-methyladenosine-3'-phosphate
  modified_base 9: mod_base = OTHER; note = 2'-deoxy-2'-fluoroguanosine-3'-phosphate
  modified_base 10: mod_base = OTHER; note = 2'-deoxy-2'-fluoroadenosine-3'-phosphate
  modified_base 11: mod_base = OTHER; note = 2'-deoxy-2'-fluoroadenosine-3'-phosphate
  modified_base 12: mod_base = OTHER; note = 2'-O-methylguanosine-3'-phosphate
  modified_base 13: mod_base = OTHER; note = 2'-O-methyladenosine-3'-phosphate
  modified_base 14: mod_base = OTHER; note = 2'-O-methyladenosine-3'-phosphate
  modified_base 15: mod_base = OTHER; note = 2'-O-methyladenosine-3'-phosphate
  modified_base 16: mod_base = OTHER; note = 2'-O-methylguanosine-3'-phosphate
  modified_base 17: mod_base = OTHER; note = 2'-O-methyluridine-3'-phosphate
  modified_base 18: mod_base = OTHER; note = 2'-O-methyladenosine-3'-phosphate
  modified_base 19: mod_base = OTHER; note = 2'-O-methyluridine-3'-phosphate
  modified_base 20: mod_base = OTHER; note = 2'-O-methyluridine-3'-phosphate
  modified_base 21: mod_base = OTHER; note = 2'-O-methyluridine-3'-phosphate ((2S,4R)-1-[29-[[2-(acetylamino)-2-deoxy-beta-D-galactopyranosyl]oxy]-14,14-bis[[3-[[3-[[5-[[2-(acetylamino)-2-deoxy-beta-D-galactopyranosyl]oxy]-1-oxopentyl]amino]propyl]amino]-3-oxopropoxy]methyl]-1,12,19,25-tetraoxo-16-oxa-13,20,24-triazanonacos-1-yl]-4-hydroxy-2-pyrrolidinyl)methyl ester
cagatctagaagaaagtattt

SEQ ID NO: 416 - RNA, 21 nt, synthetic construct
  source 1..21: mol_type = other RNA
  modified_base 1: mod_base = OTHER; note = 2'-O-methyladenosine-3'-phosphorothioate
  modified_base 2: mod_base = OTHER; note = 2'-O-methylcytidine-3'-phosphorothioate
  modified_base 3: mod_base = OTHER; note = 2'-O-methyladenosine-3'-phosphate
  modified_base 4: mod_base = OTHER; note = 2'-O-methylguanosine-3'-phosphate
  modified_base 5: mod_base = OTHER; note = 2'-O-methyladenosine-3'-phosphate
  modified_base 6: mod_base = OTHER; note = 2'-O-methyluridine-3'-phosphate
  modified_base 7: mod_base = OTHER; note = 2'-deoxy-2'-fluoroadenosine-3'-phosphate
  modified_base 8: mod_base = OTHER; note = 2'-O-methylguanosine-3'-phosphate
  modified_base 9: mod_base = OTHER; note = 2'-deoxy-2'-fluorouridine-3'-phosphate
  modified_base 10: mod_base = OTHER; note = 2'-deoxy-2'-fluorouridine-3'-phosphate
  modified_base 11: mod_base = OTHER; note = 2'-deoxy-2'-fluoroguanosine-3'-phosphate
  modified_base 12: mod_base = OTHER; note = 2'-O-methyluridine-3'-phosphate
  modified_base 13: mod_base = OTHER; note = 2'-O-methyladenosine-3'-phosphate
  modified_base 14: mod_base = OTHER; note = 2'-O-methylguanosine-3'-phosphate
  modified_base 15: mod_base = OTHER; note = 2'-O-methyluridine-3'-phosphate
  modified_base 16: mod_base = OTHER; note = 2'-O-methylguanosine-3'-phosphate
  modified_base 17: mod_base = OTHER; note = 2'-O-methyluridine-3'-phosphate
  modified_base 18: mod_base = OTHER; note = 2'-O-methyluridine-3'-phosphate
  modified_base 19: mod_base = OTHER; note = 2'-O-methyluridine-3'-phosphate
  modified_base 20: mod_base = OTHER; note = 2'-O-methyladenosine-3'-phosphate
  modified_base 21: mod_base = OTHER; note = 2'-O-methyluridine-3'-phosphate ((2S,4R)-1-[29-[[2-(acetylamino)-2-deoxy-beta-D-galactopyranosyl]oxy]-14,14-bis[[3-[[3-[[5-[[2-(acetylamino)-2-deoxy-beta-D-galactopyranosyl]oxy]-1-oxopentyl]amino]propyl]amino]-3-oxopropoxy]methyl]-1,12,19,25-tetraoxo-16-oxa-13,20,24-triazanonacos-1-yl]-4-hydroxy-2-pyrrolidinyl)methyl ester
acagatagttgtagtgtttat

SEQ ID NO: 417 - RNA, 21 nt, synthetic construct
  source 1..21: mol_type = other RNA
  modified_base 1: mod_base = OTHER; note = 2'-O-methylguanosine-3'-phosphorothioate
  modified_base 2: mod_base = OTHER; note = 2'-O-methyluridine-3'-phosphorothioate
  modified_base 3: mod_base = OTHER; note = 2'-O-methyluridine-3'-phosphate
  modified_base 4: mod_base = OTHER; note = 2'-O-methylguanosine-3'-phosphate
  modified_base 5: mod_base = OTHER; note = 2'-O-methyladenosine-3'-phosphate
  modified_base 6: mod_base = OTHER; note = 2'-O-methylguanosine-3'-phosphate
  modified_base 7: mod_base = OTHER; note = 2'-deoxy-2'-fluoroguanosine-3'-phosphate
  modified_base 8: mod_base = OTHER; note = 2'-O-methyluridine-3'-phosphate
  modified_base 9: mod_base = OTHER; note = 2'-deoxy-2'-fluorouridine-3'-phosphate
  modified_base 10: mod_base = OTHER; note = 2'-deoxy-2'-fluorouridine-3'-phosphate
  modified_base 11: mod_base = OTHER; note = 2'-deoxy-2'-fluorocytidine-3'-phosphate
  modified_base 12: mod_base = OTHER; note = 2'-O-methyluridine-3'-phosphate
  modified_base 13: mod_base = OTHER; note = 2'-O-methyladenosine-3'-phosphate
  modified_base 14: mod_base = OTHER; note = 2'-O-methyladenosine-3'-phosphate
  modified_base 15: mod_base = OTHER; note = 2'-O-methylguanosine-3'-phosphate
  modified_base 16: mod_base = OTHER; note = 2'-O-methyladenosine-3'-phosphate
  modified_base 17: mod_base = OTHER; note = 2'-O-methylcytidine-3'-phosphate
  modified_base 18: mod_base = OTHER; note = 2'-O-methyluridine-3'-phosphate
  modified_base 19: mod_base = OTHER; note = 2'-O-methyluridine-3'-phosphate
  modified_base 20: mod_base = OTHER; note = 2'-O-methyladenosine-3'-phosphate
  modified_base 21: mod_base = OTHER; note = 2'-O-methyluridine-3'-phosphate ((2S,4R)-1-[29-[[2-(acetylamino)-2-deoxy-beta-D-galactopyranosyl]oxy]-14,14-bis[[3-[[3-[[5-[[2-(acetylamino)-2-deoxy-beta-D-galactopyranosyl]oxy]-1-oxopentyl]amino]propyl]amino]-3-oxopropoxy]methyl]-1,12,19,25-tetraoxo-16-oxa-13,20,24-triazanonacos-1-yl]-4-hydroxy-2-pyrrolidinyl)methyl ester
gttgaggtttctaagacttat

SEQ ID NO: 418 - RNA, 21 nt, synthetic construct
  source 1..21: mol_type = other RNA
  modified_base 1: mod_base = OTHER; note = 2'-O-methyladenosine-3'-phosphorothioate
  modified_base 2: mod_base = OTHER; note = 2'-O-methyluridine-3'-phosphorothioate
  modified_base 3: mod_base = OTHER; note = 2'-O-methyluridine-3'-phosphate
  modified_base 4: mod_base = OTHER; note = 2'-O-methyluridine-3'-phosphate
  modified_base 5: mod_base = OTHER; note = 2'-O-methyluridine-3'-phosphate
  modified_base 6: mod_base = OTHER; note = 2'-O-methyladenosine-3'-phosphate
  modified_base 7: mod_base = OTHER; note = 2'-deoxy-2'-fluoroguanosine-3'-phosphate
  modified_base 8: mod_base = OTHER; note = 2'-O-methyladenosine-3'-phosphate
  modified_base 9: mod_base = OTHER; note = 2'-deoxy-2'-fluoroadenosine-3'-phosphate
  modified_base 10: mod_base = OTHER; note = 2'-deoxy-2'-fluoroadenosine-3'-phosphate
  modified_base 11: mod_base = OTHER; note = 2'-deoxy-2'-fluorocytidine-3'-phosphate
  modified_base 12: mod_base = OTHER; note = 2'-O-methylcytidine-3'-phosphate
  modified_base 13: mod_base = OTHER; note = 2'-O-methyluridine-3'-phosphate
  modified_base 14: mod_base = OTHER; note = 2'-O-methylguanosine-3'-phosphate
  modified_base 15: mod_base = OTHER; note = 2'-O-methyladenosine-3'-phosphate
  modified_base 16: mod_base = OTHER; note = 2'-O-methylguanosine-3'-phosphate
  modified_base 17: mod_base = OTHER; note = 2'-O-methyladenosine-3'-phosphate
  modified_base 18: mod_base = OTHER; note = 2'-O-methylcytidine-3'-phosphate
  modified_base 19: mod_base = OTHER; note = 2'-O-methyluridine-3'-phosphate
  modified_base 20: mod_base = OTHER; note = 2'-O-methyluridine-3'-phosphate
  modified_base 21: mod_base = OTHER; note = 2'-O-methyluridine-3'-phosphate ((2S,4R)-1-[29-[[2-(acetylamino)-2-deoxy-beta-D-galactopyranosyl]oxy]-14,14-bis[[3-[[3-[[5-[[2-(acetylamino)-2-deoxy-beta-D-galactopyranosyl]oxy]-1-oxopentyl]amino]propyl]amino]-3-oxopropoxy]methyl]-1,12,19,25-tetraoxo-16-oxa-13,20,24-triazanonacos-1-yl]-4-hydroxy-2-pyrrolidinyl)methyl ester
attttagaaacctgagacttt

SEQ ID NO: 419 - RNA, 21 nt, synthetic construct
  source 1..21: mol_type = other RNA
  modified_base 1: mod_base = OTHER; note = 2'-O-methyluridine-3'-phosphorothioate
  modified_base 2: mod_base = OTHER; note = 2'-O-methylcytidine-3'-phosphorothioate
  modified_base 3: mod_base = OTHER; note = 2'-O-methyluridine-3'-phosphate
  modified_base 4: mod_base = OTHER; note = 2'-O-methylguanosine-3'-phosphate
  modified_base 5: mod_base = OTHER; note = 2'-O-methylguanosine-3'-phosphate
  modified_base 6: mod_base = OTHER; note = 2'-O-methylcytidine-3'-phosphate
  modified_base 7: mod_base = OTHER; note = 2'-deoxy-2'-fluoroadenosine-3'-phosphate
  modified_base 8: mod_base = OTHER; note = 2'-O-methyluridine-3'-phosphate
  modified_base 9: mod_base = OTHER; note = 2'-deoxy-2'-fluorouridine-3'-phosphate
  modified_base 10: mod_base = OTHER; note = 2'-deoxy-2'-fluorouridine-3'-phosphate
  modified_base 11: mod_base = OTHER; note = 2'-deoxy-2'-fluorouridine-3'-phosphate
  modified_base 12: mod_base = OTHER; note = 2'-O-methyladenosine-3'-phosphate
  modified_base 13: mod_base = OTHER; note = 2'-O-methylguanosine-3'-phosphate
  modified_base 14: mod_base = OTHER; note = 2'-O-methyluridine-3'-phosphate
  modified_base 15: mod_base = OTHER; note = 2'-O-methyluridine-3'-phosphate
  modified_base 16: mod_base = OTHER; note = 2'-O-methyluridine-3'-phosphate
  modified_base 17: mod_base = OTHER; note = 2'-O-methyladenosine-3'-phosphate
  modified_base 18: mod_base = OTHER; note = 2'-O-methyladenosine-3'-phosphate
  modified_base 19: mod_base = OTHER; note = 2'-O-methyluridine-3'-phosphate
  modified_base 20: mod_base = OTHER; note = 2'-O-methyladenosine-3'-phosphate
  modified_base 21: mod_base = OTHER; note = 2'-O-methyluridine-3'-phosphate ((2S,4R)-1-[29-[[2-(acetylamino)-2-deoxy-beta-D-galactopyranosyl]oxy]-14,14-bis[[3-[[3-[[5-[[2-(acetylamino)-2-deoxy-beta-D-galactopyranosyl]oxy]-1-oxopentyl]amino]propyl]amino]-3-oxopropoxy]methyl]-1,12,19,25-tetraoxo-16-oxa-13,20,24-triazanonacos-1-yl]-4-hydroxy-2-pyrrolidinyl)methyl ester
tctggcattttagtttaatat

SEQ ID NO: 420 - RNA, 21 nt, synthetic construct
  source 1..21: mol_type = other RNA
  modified_base 1: mod_base = OTHER; note = 2'-O-methyladenosine-3'-phosphorothioate
  modified_base 2: mod_base = OTHER; note = 2'-O-methyladenosine-3'-phosphorothioate
  modified_base 3: mod_base = OTHER; note = 2'-O-methylcytidine-3'-phosphate
  modified_base 4: mod_base = OTHER; note = 2'-O-methyluridine-3'-phosphate
  modified_base 5: mod_base = OTHER; note = 2'-O-methyladenosine-3'-phosphate
  modified_base 6: mod_base = OTHER; note = 2'-O-methyladenosine-3'-phosphate
  modified_base 7: mod_base = OTHER; note = 2'-deoxy-2'-fluorouridine-3'-phosphate
  modified_base 8: mod_base = OTHER; note = 2'-O-methylguanosine-3'-phosphate
  modified_base 9: mod_base = OTHER; note = 2'-deoxy-2'-fluoroadenosine-3'-phosphate
  modified_base 10: mod_base = OTHER; note = 2'-deoxy-2'-fluorouridine-3'-phosphate
  modified_base 11: mod_base = OTHER; note = 2'-deoxy-2'-fluorouridine-3'-phosphate
  modified_base 12: mod_base = OTHER; note = 2'-O-methylguanosine-3'-phosphate
  modified_base 13: mod_base = OTHER; note = 2'-O-methylcytidine-3'-phosphate
  modified_base 14: mod_base = OTHER; note = 2'-O-methyladenosine-3'-phosphate
  modified_base 15: mod_base = OTHER; note = 2'-O-methyluridine-3'-phosphate
  modified_base 16: mod_base = OTHER; note = 2'-O-methyluridine-3'-phosphate
  modified_base 17: mod_base = OTHER; note = 2'-O-methyluridine-3'-phosphate
  modified_base 18: mod_base = OTHER; note = 2'-O-methylguanosine-3'-phosphate
  modified_base 19: mod_base = OTHER; note = 2'-O-methyladenosine-3'-phosphate
  modified_base 20: mod_base = OTHER; note = 2'-O-methyladenosine-3'-phosphate
  modified_base 21: mod_base = OTHER; note = 2'-O-methyluridine-3'-phosphate ((2S,4R)-1-[29-[[2-(acetylamino)-2-deoxy-beta-D-galactopyranosyl]oxy]-14,14-bis[[3-[[3-[[5-[[2-(acetylamino)-2-deoxy-beta-D-galactopyranosyl]oxy]-1-oxopentyl]amino]propyl]amino]-3-oxopropoxy]methyl]-1,12,19,25-tetraoxo-16-oxa-13,20,24-triazanonacos-1-yl]-4-hydroxy-2-pyrrolidinyl)methyl ester
aactaatgattgcatttgaat

SEQ ID NO: 421 - RNA, 21 nt, synthetic construct
  source 1..21: mol_type = other RNA
  modified_base 1: mod_base = OTHER; note = 2'-O-methyladenosine-3'-phosphorothioate
  modified_base 2: mod_base = OTHER; note = 2'-O-methyladenosine-3'-phosphorothioate
  modified_base 3: mod_base = OTHER; note = 2'-O-methyladenosine-3'-phosphate
  modified_base 4: mod_base = OTHER; note = 2'-O-methylguanosine-3'-phosphate
  modified_base 5: mod_base = OTHER; note = 2'-O-methyladenosine-3'-phosphate
  modified_base 6: mod_base = OTHER; note = 2'-O-methylguanosine-3'-phosphate
  modified_base 7: mod_base = OTHER; note = 2'-deoxy-2'-fluoroadenosine-3'-phosphate
  modified_base 8: mod_base = OTHER; note = 2'-O-methyluridine-3'-phosphate
  modified_base 9: mod_base = OTHER; note = 2'-deoxy-2'-fluorouridine-3'-phosphate
  modified_base 10: mod_base = OTHER; note = 2'-deoxy-2'-fluorocytidine-3'-phosphate
  modified_base 11: mod_base = OTHER; note = 2'-deoxy-2'-fluorouridine-3'-phosphate
  modified_base 12: mod_base = OTHER; note = 2'-O-methyluridine-3'-phosphate
  modified_base 13: mod_base = OTHER; note = 2'-O-methylguanosine-3'-phosphate
  modified_base 14: mod_base = OTHER; note = 2'-O-methyladenosine-3'-phosphate
  modified_base 15: mod_base = OTHER; note = 2'-O-methylcytidine-3'-phosphate
  modified_base 16: mod_base = OTHER; note = 2'-O-methylcytidine-3'-phosphate
  modified_base 17: mod_base = OTHER; note = 2'-O-methyluridine-3'-phosphate
  modified_base 18: mod_base = OTHER; note = 2'-O-methyluridine-3'-phosphate
  modified_base 19: mod_base = OTHER; note = 2'-O-methyladenosine-3'-phosphate
  modified_base 20: mod_base = OTHER; note = 2'-O-methyluridine-3'-phosphate
  modified_base 21: mod_base = OTHER; note = 2'-O-methyluridine-3'-phosphate ((2S,4R)-1-[29-[[2-(acetylamino)-2-deoxy-beta-D-galactopyranosyl]oxy]-14,14-bis[[3-[[3-[[5-[[2-(acetylamino)-2-deoxy-beta-D-galactopyranosyl]oxy]-1-oxopentyl]amino]propyl]amino]-3-oxopropoxy]methyl]-1,12,19,25-tetraoxo-16-oxa-13,20,24-triazanonacos-1-yl]-4-hydroxy-2-pyrrolidinyl)methyl ester
aaagagattcttgaccttatt

SEQ ID NO: 422 - RNA, 21 nt, synthetic construct
  source 1..21: mol_type = other RNA
  modified_base 1: mod_base = OTHER; note = 2'-O-methylguanosine-3'-phosphorothioate
  modified_base 2: mod_base = OTHER; note = 2'-O-methyladenosine-3'-phosphorothioate
  modified_base 3: mod_base = OTHER; note = 2'-O-methylguanosine-3'-phosphate
  modified_base 4: mod_base = OTHER; note = 2'-O-methylcytidine-3'-phosphate
  modified_base 5: mod_base = OTHER; note = 2'-O-methyluridine-3'-phosphate
  modified_base 6: mod_base = OTHER; note = 2'-O-methylcytidine-3'-phosphate
  modified_base 7: mod_base = OTHER; note = 2'-deoxy-2'-fluorouridine-3'-phosphate
  modified_base 8: mod_base = OTHER; note = 2'-O-methylguanosine-3'-phosphate
  modified_base 9: mod_base = OTHER; note = 2'-deoxy-2'-fluoroadenosine-3'-phosphate
  modified_base 10: mod_base = OTHER; note = 2'-deoxy-2'-fluoroadenosine-3'-phosphate
  modified_base 11: mod_base = OTHER; note = 2'-deoxy-2'-fluoroadenosine-3'-phosphate
  modified_base 12: mod_base = OTHER; note = 2'-O-methyluridine-3'-phosphate
  modified_base 13: mod_base = OTHER; note = 2'-O-methylguanosine-3'-phosphate
  modified_base 14: mod_base = OTHER; note = 2'-O-methyluridine-3'-phosphate
  modified_base 15: mod_base = OTHER; note = 2'-O-methylcytidine-3'-phosphate
  modified_base 16: mod_base = OTHER; note = 2'-O-methyluridine-3'-phosphate
  modified_base 17: mod_base = OTHER; note = 2'-O-methyluridine-3'-phosphate
  modified_base 18: mod_base = OTHER; note = 2'-O-methylguanosine-3'-phosphate
  modified_base 19: mod_base = OTHER; note = 2'-O-methyladenosine-3'-phosphate
  modified_base 20: mod_base = OTHER; note = 2'-O-methyluridine-3'-phosphate
  modified_base 21: mod_base = OTHER; note = 2'-O-methyluridine-3'-phosphate ((2S,4R)-1-[29-[[2-(acetylamino)-2-deoxy-beta-D-galactopyranosyl]oxy]-14,14-bis[[3-[[3-[[5-[[2-(acetylamino)-2-deoxy-beta-D-galactopyranosyl]oxy]-1-oxopentyl]amino]propyl]amino]-3-oxopropoxy]methyl]-1,12,19,25-tetraoxo-16-oxa-13,20,24-triazanonacos-1-yl]-4-hydroxy-2-pyrrolidinyl)methyl ester
gagctctgaaatgtcttgatt

SEQ ID NO: 423 - RNA, 21 nt, synthetic construct
  source 1..21: mol_type = other RNA
  modified_base 1: mod_base = OTHER; note = 2'-O-methyluridine-3'-phosphorothioate
  modified_base 2: mod_base = OTHER; note = 2'-O-methylguanosine-3'-phosphorothioate
  modified_base 3: mod_base = OTHER; note = 2'-O-methylguanosine-3'-phosphate
  modified_base 4: mod_base = OTHER; note = 2'-O-methyladenosine-3'-phosphate
  modified_base 5: mod_base = OTHER; note = 2'-O-methyladenosine-3'-phosphate
  modified_base 6: mod_base = OTHER; note = 2'-O-methylguanosine-3'-phosphate
  modified_base 7: mod_base = OTHER; note = 2'-deoxy-2'-fluoroguanosine-3'-phosphate
  modified_base 8: mod_base = OTHER; note = 2'-O-methyluridine-3'-phosphate
  modified_base 9: mod_base = OTHER; note = 2'-deoxy-2'-fluoroadenosine-3'-phosphate
  modified_base 10: mod_base = OTHER; note = 2'-deoxy-2'-fluorouridine-3'-phosphate
  modified_base 11: mod_base = OTHER; note = 2'-deoxy-2'-fluorouridine-3'-phosphate
  modified_base 12: mod_base = OTHER; note = 2'-O-methyladenosine-3'-phosphate
  modified_base 13: mod_base = OTHER; note = 2'-O-methyladenosine-3'-phosphate
  modified_base 14: mod_base = OTHER; note = 2'-O-methyladenosine-3'-phosphate
  modified_base 15: mod_base = OTHER; note = 2'-O-methylcytidine-3'-phosphate
  modified_base 16: mod_base = OTHER; note = 2'-O-methyluridine-3'-phosphate
  modified_base 17: mod_base = OTHER; note = 2'-O-methyladenosine-3'-phosphate
  modified_base 18: mod_base = OTHER; note = 2'-O-methyluridine-3'-phosphate
  modified_base 19: mod_base = OTHER; note = 2'-O-methyluridine-3'-phosphate
  modified_base 20: mod_base = OTHER; note = 2'-O-methyluridine-3'-phosphate
  modified_base 21: mod_base = OTHER; note = 2'-O-methyluridine-3'-phosphate ((2S,4R)-1-[29-[[2-(acetylamino)-2-deoxy-beta-D-galactopyranosyl]oxy]-14,14-bis[[3-[[3-[[5-[[2-(acetylamino)-2-deoxy-beta-D-galactopyranosyl]oxy]-1-oxopentyl]amino]propyl]amino]-3-oxopropoxy]methyl]-1,12,19,25-tetraoxo-16-oxa-13,20,24-triazanonacos-1-yl]-4-hydroxy-2-pyrrolidinyl)methyl ester
tggaaggtattaaactatttt

SEQ ID NO: 424 - RNA, 21 nt, synthetic construct
  source 1..21: mol_type = other RNA
  modified_base 1: mod_base = OTHER; note = 2'-O-methyluridine-3'-phosphorothioate
  modified_base 2: mod_base = OTHER; note = 2'-O-methylguanosine-3'-phosphorothioate
  modified_base 3: mod_base = OTHER; note = 2'-O-methylcytidine-3'-phosphate
  modified_base 4: mod_base = OTHER; note = 2'-O-methylcytidine-3'-phosphate
  modified_base 5: mod_base = OTHER; note = 2'-O-methyluridine-3'-phosphate
  modified_base 6: mod_base = OTHER; note = 2'-O-methylguanosine-3'-phosphate
  modified_base 7: mod_base = OTHER; note = 2'-deoxy-2'-fluorouridine-3'-phosphate
  modified_base 8: mod_base = OTHER; note = 2'-O-methyluridine-3'-phosphate
  modified_base 9: mod_base = OTHER; note = 2'-deoxy-2'-fluoroguanosine-3'-phosphate
  modified_base 10: mod_base = OTHER; note = 2'-deoxy-2'-fluorouridine-3'-phosphate
  modified_base 11: mod_base = OTHER; note = 2'-deoxy-2'-fluoroadenosine-3'-phosphate
  modified_base 12: mod_base = OTHER; note = 2'-O-methylcytidine-3'-phosphate
  modified_base 13: mod_base = OTHER; note = 2'-O-methyladenosine-3'-phosphate
  modified_base 14: mod_base = OTHER; note = 2'-O-methyladenosine-3'-phosphate
  modified_base 15: mod_base = OTHER; note = 2'-O-methyladenosine-3'-phosphate
  modified_base 16: mod_base = OTHER; note = 2'-O-methylguanosine-3'-phosphate
  modified_base 17: mod_base = OTHER; note = 2'-O-methyladenosine-3'-phosphate
  modified_base 18: mod_base = OTHER; note = 2'-O-methyladenosine-3'-phosphate
  modified_base 19: mod_base = OTHER; note = 2'-O-methyladenosine-3'-phosphate
  modified_base 20: mod_base = OTHER; note = 2'-O-methyluridine-3'-phosphate
  modified_base 21: mod_base = OTHER; note = 2'-O-methyluridine-3'-phosphate ((2S,4R)-1-[29-[[2-(acetylamino)-2-deoxy-beta-D-galactopyranosyl]oxy]-14,14-bis[[3-[[3-[[5-[[2-(acetylamino)-2-deoxy-beta-D-galactopyranosyl]oxy]-1-oxopentyl]amino]propyl]amino]-3-oxopropoxy]methyl]-1,12,19,25-tetraoxo-16-oxa-13,20,24-triazanonacos-1-yl]-4-hydroxy-2-pyrrolidinyl)methyl ester
tgcctgttgtacaaagaaatt

SEQ ID NO: 425 - RNA, 21 nt, synthetic construct
  source 1..21: mol_type = other RNA
  modified_base 1: mod_base = OTHER; note = 2'-O-methyladenosine-3'-phosphorothioate
  modified_base 2: mod_base = OTHER; note = 2'-O-methylcytidine-3'-phosphorothioate
  modified_base 3: mod_base = OTHER; note = 2'-O-methyluridine-3'-phosphate
  modified_base 4: mod_base = OTHER; note = 2'-O-methylcytidine-3'-phosphate
  modified_base 5: mod_base = OTHER; note = 2'-O-methylguanosine-3'-phosphate
  modified_base 6: mod_base = OTHER; note = 2'-O-methyluridine-3'-phosphate
  modified_base 7: mod_base = OTHER; note = 2'-deoxy-2'-fluoroguanosine-3'-phosphate
  modified_base 8: mod_base = OTHER; note = 2'-O-methyladenosine-3'-phosphate
  modified_base 9: mod_base = OTHER; note = 2'-deoxy-2'-fluoroadenosine-3'-phosphate
  modified_base 10: mod_base = OTHER; note = 2'-deoxy-2'-fluoroadenosine-3'-phosphate
  modified_base 11: mod_base = OTHER; note = 2'-deoxy-2'-fluoroadenosine-3'-phosphate
  modified_base 12: mod_base = OTHER; note = 2'-O-methylguanosine-3'-phosphate
  modified_base 13: mod_base = OTHER; note = 2'-O-methyladenosine-3'-phosphate
  modified_base 14: mod_base = OTHER; note = 2'-O-methyladenosine-3'-phosphate
  modified_base 15: mod_base = OTHER; note = 2'-O-methyluridine-3'-phosphate
  modified_base 16: mod_base = OTHER; note = 2'-O-methyluridine-3'-phosphate
  modified_base 17: mod_base = OTHER; note = 2'-O-methyladenosine-3'-phosphate
  modified_base 18: mod_base = OTHER; note = 2'-O-methylcytidine-3'-phosphate
  modified_base 19: mod_base = OTHER; note = 2'-O-methyluridine-3'-phosphate
  modified_base 20: mod_base = OTHER; note = 2'-O-methyladenosine-3'-phosphate
  modified_base 21: mod_base = OTHER; note = 2'-O-methyluridine-3'-phosphate ((2S,4R)-1-[29-[[2-(acetylamino)-2-deoxy-beta-D-galactopyranosyl]oxy]-14,14-bis[[3-[[3-[[5-[[2-(acetylamino)-2-deoxy-beta-D-galactopyranosyl]oxy]-1-oxopentyl]amino]propyl]amino]-3-oxopropoxy]methyl]-1,12,19,25-tetraoxo-16-oxa-13,20,24-triazanonacos-1-yl]-4-hydroxy-2-pyrrolidinyl)methyl ester
actcgtgaaaagaattactat

SEQ ID NO: 426 - RNA, 21 nt, synthetic construct
  source 1..21: mol_type = other RNA
  modified_base 1: mod_base = OTHER; note = 2'-O-methyluridine-3'-phosphorothioate
  modified_base 2: mod_base = OTHER; note = 2'-O-methylguanosine-3'-phosphorothioate
  modified_base 3: mod_base = OTHER; note = 2'-O-methyladenosine-3'-phosphate
  modified_base 4: mod_base = OTHER; note = 2'-O-methyladenosine-3'-phosphate
  modified_base 5: mod_base = OTHER; note = 2'-O-methyladenosine-3'-phosphate
  modified_base 6: mod_base = OTHER; note = 2'-O-methyluridine-3'-phosphate
  modified_base 7: mod_base = OTHER; note = 2'-deoxy-2'-fluoroadenosine-3'-phosphate
  modified_base 8: mod_base = OTHER; note = 2'-O-methyladenosine-3'-phosphate
  modified_base 9: mod_base = OTHER; note = 2'-deoxy-2'-fluorocytidine-3'-phosphate
  modified_base 10: mod_base = OTHER; note = 2'-deoxy-2'-fluorouridine-3'-phosphate
  modified_base 11: mod_base = OTHER; note = 2'-deoxy-2'-fluoroguanosine-3'-phosphate
  modified_base 12: mod_base = OTHER; note = 2'-O-methylcytidine-3'-phosphate
  modified_base 13: mod_base = OTHER; note = 2'-O-methylguanosine-3'-phosphate
  modified_base 14: mod_base = OTHER; note = 2'-O-methyladenosine-3'-phosphate
  modified_base 15: mod_base = OTHER; note = 2'-O-methyluridine-3'-phosphate
  modified_base 16: mod_base = OTHER; note = 2'-O-methyluridine-3'-phosphate
  modified_base 17: mod_base = OTHER; note = 2'-O-methyluridine-3'-phosphate
  modified_base 18: mod_base = OTHER; note = 2'-O-methyluridine-3'-phosphate
  modified_base 19: mod_base = OTHER; note = 2'-O-methylguanosine-3'-phosphate
  modified_base 20: mod_base = OTHER; note = 2'-O-methyluridine-3'-phosphate
  modified_base 21: mod_base = OTHER; note = 2'-O-methyluridine-3'-phosphate ((2S,4R)-1-[29-[[2-(acetylamino)-2-deoxy-beta-D-galactopyranosyl]oxy]-14,14-bis[[3-[[3-[[5-[[2-(acetylamino)-2-deoxy-beta-D-galactopyranosyl]oxy]-1-oxopentyl]amino]propyl]amino]-3-oxopropoxy]methyl]-1,12,19,25-tetraoxo-16-oxa-13,20,24-triazanonacos-1-yl]-4-hydroxy-2-pyrrolidinyl)methyl ester
tgaaataactgcgattttgtt

SEQ ID NO: 427 - RNA, 21 nt, synthetic construct
  source 1..21: mol_type = other RNA
  modified_base 1: mod_base = OTHER; note = 2'-O-methyluridine-3'-phosphorothioate
  modified_base 2: mod_base = OTHER; note = 2'-O-methyluridine-3'-phosphorothioate
  modified_base 3: mod_base = OTHER; note = 2'-O-methylguanosine-3'-phosphate
  modified_base 4: mod_base = OTHER; note = 2'-O-methylguanosine-3'-phosphate
  modified_base 5: mod_base = OTHER; note = 2'-O-methyladenosine-3'-phosphate
  modified_base 6: mod_base = OTHER; note = 2'-O-methyladenosine-3'-phosphate
  modified_base 7: mod_base = OTHER; note = 2'-deoxy-2'-fluoroadenosine-3'-phosphate
  modified_base 8: mod_base = OTHER; note = 2'-O-methyluridine-3'-phosphate
  modified_base 9: mod_base = OTHER; note = 2'-deoxy-2'-fluoroguanosine-3'-phosphate
  modified_base 10: mod_base = OTHER; note = 2'-deoxy-2'-fluorocytidine-3'-phosphate
  modified_base 11: mod_base = OTHER; note = 2'-deoxy-2'-fluorouridine-3'-phosphate
  modified_base 12: mod_base = OTHER; note = 2'-O-methylguanosine-3'-phosphate
  modified_base 13: mod_base = OTHER; note = 2'-O-methyladenosine-3'-phosphate
  modified_base 14: mod_base = OTHER; note = 2'-O-methyluridine-3'-phosphate
  modified_base 15: mod_base = OTHER; note = 2'-O-methyluridine-3'-phosphate
  modified_base 16: mod_base = OTHER; note = 2'-O-methylguanosine-3'-phosphate
  modified_base 17: mod_base = OTHER; note = 2'-O-methyladenosine-3'-phosphate
  modified_base 18: mod_base = OTHER; note = 2'-O-methyluridine-3'-phosphate
  modified_base 19: mod_base = OTHER; note = 2'-O-methyluridine-3'-phosphate
  modified_base 20: mod_base = OTHER; note = 2'-O-methyluridine-3'-phosphate
  modified_base 21: mod_base = OTHER; note = 2'-O-methyluridine-3'-phosphate ((2S,4R)-1-[29-[[2-(acetylamino)-2-deoxy-beta-D-galactopyranosyl]oxy]-14,14-bis[[3-[[3-[[5-[[2-(acetylamino)-2-deoxy-beta-D-galactopyranosyl]oxy]-1-oxopentyl]amino]propyl]amino]-3-oxopropoxy]methyl]-1,12,19,25-tetraoxo-16-oxa-13,20,24-triazanonacos-1-yl]-4-hydroxy-2-pyrrolidinyl)methyl ester
ttggaaatgctgattgatttt

SEQ ID NO: 428 - RNA, 21 nt, synthetic construct
  source 1..21: mol_type = other RNA
  modified_base 1: mod_base = OTHER; note = 2'-O-methyluridine-3'-phosphorothioate
  modified_base 2: mod_base = OTHER; note = 2'-O-methyluridine-3'-phosphorothioate
  modified_base 3: mod_base = OTHER; note = 2'-O-methyladenosine-3'-phosphate
  modified_base 4: mod_base = OTHER; note = 2'-O-methylguanosine-3'-phosphate
  modified_base 5: mod_base = OTHER; note = 2'-O-methyluridine-3'-phosphate
  modified_base 6: mod_base = OTHER; note = 2'-O-methylguanosine-3'-phosphate
  modified_base 7: mod_base = OTHER; note = 2'-deoxy-2'-fluorouridine-3'-phosphate
  modified_base 8: mod_base = OTHER; note = 2'-O-methyladenosine-3'-phosphate
  modified_base 9: mod_base = OTHER; note = 2'-deoxy-2'-fluorouridine-3'-phosphate
  modified_base 10: mod_base = OTHER; note = 2'-deoxy-2'-fluorouridine-3'-phosphate
  modified_base 11: mod_base = OTHER; note = 2'-deoxy-2'-fluoroguanosine-3'-phosphate
  modified_base 12: mod_base = OTHER; note = 2'-O-methylcytidine-3'-phosphate
  modified_base 13: mod_base = OTHER; note = 2'-O-methyladenosine-3'-phosphate
  modified_base 14: mod_base = OTHER; note = 2'-O-methyladenosine-3'-phosphate
  modified_base 15: mod_base = OTHER; note = 2'-O-methylguanosine-3'-phosphate
  modified_base 16: mod_base = OTHER; note = 2'-O-methyladenosine-3'-phosphate
  modified_base 17: mod_base = OTHER; note = 2'-O-methyladenosine-3'-phosphate
  modified_base 18: mod_base = OTHER; note = 2'-O-methyladenosine-3'-phosphate
  modified_base 19: mod_base = OTHER; note = 2'-O-methylcytidine-3'-phosphate
  modified_base 20: mod_base = OTHER; note = 2'-O-methyladenosine-3'-phosphate
  modified_base 21: mod_base = OTHER; note = 2'-O-methyluridine-3'-phosphate ((2S,4R)-1-[29-[[2-(acetylamino)-2-deoxy-beta-D-galactopyranosyl]oxy]-14,14-bis[[3-[[3-[[5-[[2-(acetylamino)-2-deoxy-beta-D-galactopyranosyl]oxy]-1-oxopentyl]amino]propyl]amino]-3-oxopropoxy]methyl]-1,12,19,25-tetraoxo-16-oxa-13,20,24-triazanonacos-1-yl]-4-hydroxy-2-pyrrolidinyl)methyl ester
ttagtgtattgcaagaaacat

SEQ ID NO: 429 - RNA, 21 nt, synthetic construct
  source 1..21: mol_type = other RNA
  modified_base 1: mod_base = OTHER; note = 2'-O-methylcytidine-3'-phosphorothioate
  modified_base 2: mod_base = OTHER; note = 2'-O-methyladenosine-3'-phosphorothioate
  modified_base 3: mod_base = OTHER; note = 2'-O-methylguanosine-3'-phosphate
  modified_base 4: mod_base = OTHER; note = 2'-O-methyladenosine-3'-phosphate
  modified_base 5: mod_base = OTHER; note = 2'-O-methyladenosine-3'-phosphate
  modified_base 6: mod_base = OTHER; note = 2'-O-methyladenosine-3'-phosphate
  modified_base 7: mod_base = OTHER; note = 2'-deoxy-2'-fluoroadenosine-3'-phosphate
  modified_base 8: mod_base = OTHER; note = 2'-O-methyluridine-3'-phosphate
  modified_base 9: mod_base = OTHER; note = 2'-deoxy-2'-fluoroguanosine-3'-phosphate
  modified_base 10: mod_base = OTHER; note = 2'-deoxy-2'-fluorouridine-3'-phosphate
  modified_base 11: mod_base = OTHER; note = 2'-deoxy-2'-fluoroadenosine-3'-phosphate
  modified_base 12: mod_base = OTHER; note = 2'-O-methylguanosine-3'-phosphate
  modified_base 13: mod_base = OTHER; note = 2'-O-methyluridine-3'-phosphate
  modified_base 14: mod_base = OTHER; note = 2'-O-methyluridine-3'-phosphate
  modified_base 15: mod_base = OTHER; note = 2'-O-methyluridine-3'-phosphate
  modified_base 16: mod_base = OTHER; note = 2'-O-methyluridine-3'-phosphate
  modified_base 17: mod_base = OTHER; note = 2'-O-methylguanosine-3'-phosphate
  modified_base 18: mod_base = OTHER; note = 2'-O-methyluridine-3'-phosphate
  modified_base 19: mod_base = OTHER; note = 2'-O-methyluridine-3'-phosphate
  modified_base 20: mod_base = OTHER; note = 2'-O-methyluridine-3'-phosphate
  modified_base 21: mod_base = OTHER; note = 2'-O-methyluridine-3'-phosphate ((2S,4R)-1-[29-[[2-(acetylamino)-2-deoxy-beta-D-galactopyranosyl]oxy]-14,14-bis[[3-[[3-[[5-[[2-(acetylamino)-2-deoxy-beta-D-galactopyranosyl]oxy]-1-oxopentyl]amino]propyl]amino]-3-oxopropoxy]methyl]-1,12,19,25-tetraoxo-16-oxa-13,20,24-triazanonacos-1-yl]-4-hydroxy-2-pyrrolidinyl)methyl ester
cagaaaatgtagttttgtttt

SEQ ID NO: 430 - RNA, 23 nt, synthetic construct
  source 1..23: mol_type = other RNA
  modified_base 1: mod_base = OTHER; note = 2'-O-methyladenosine-3'-phosphorothioate
  modified_base 2: mod_base = OTHER; note = 2'-deoxy-2'-fluoroadenosine-3'-phosphorothioate
  modified_base 3: mod_base = OTHER; note = 2'-O-methyluridine-3'-phosphate
  modified_base 4: mod_base = OTHER; note = 2'-O-methyladenosine-3'-phosphate
  modified_base 5: mod_base = OTHER; note = 2'-O-methyladenosine-3'-phosphate
  modified_base 6: mod_base = OTHER; note = 2'-deoxy-2'-fluorocytidine-3'-phosphate
  modified_base 7: mod_base = OTHER; note = 2'-O-methyladenosine-3'-phosphate
  modified_base 8: mod_base = OTHER; note = 2'-deoxy-2'-fluorouridine-3'-phosphate
  modified_base 9: mod_base = OTHER; note = 2'-deoxy-2'-fluoroadenosine-3'-phosphate
  modified_base 10: mod_base = OTHER; note = 2'-O-methyladenosine-3'-phosphate
  modified_base 11: mod_base = OTHER; note = 2'-O-methyladenosine-3'-phosphate
  modified_base 12: mod_base = OTHER; note = 2'-O-methyladenosine-3'-phosphate
  modified_base 13: mod_base = OTHER; note = 2'-O-methylcytidine-3'-phosphate
  modified_base 14: mod_base = OTHER; note = 2'-deoxy-2'-fluorouridine-3'-phosphate
  modified_base 15: mod_base = OTHER; note = 2'-O-methyluridine-3'-phosphate
  modified_base 16: mod_base = OTHER; note = 2'-deoxy-2'-fluorocytidine-3'-phosphate
  modified_base 17: mod_base = OTHER; note = 2'-O-methyladenosine-3'-phosphate
  modified_base 18: mod_base = OTHER; note = 2'-O-methylguanosine-3'-phosphate
  modified_base 19: mod_base = OTHER; note = 2'-O-methylguanosine-3'-phosphate
  modified_base 20: mod_base = OTHER; note = 2'-O-methyladenosine-3'-phosphate
  modified_base 21: mod_base = OTHER; note = 2'-O-methylcytidine-3'-phosphorothioate
  modified_base 22: mod_base = OTHER; note = 2'-O-methyluridine-3'-phosphorothioate
  modified_base 23: mod_base = OTHER; note = 2'-O-methylcytidine
aataacataaaacttcaggactc

SEQ ID NO: 431 - RNA, 23 nt, synthetic construct
  source 1..23: mol_type = other RNA
  modified_base 1: mod_base = OTHER; note = 2'-O-methyladenosine-3'-phosphorothioate
  modified_base 2: mod_base = OTHER; note = 2'-deoxy-2'-fluoroadenosine-3'-phosphorothioate
  modified_base 3: mod_base = OTHER; note = 2'-O-methyladenosine-3'-phosphate
  modified_base 4: mod_base = OTHER; note = 2'-O-methylguanosine-3'-phosphate
  modified_base 5: mod_base = OTHER; note = 2'-O-methyluridine-3'-phosphate
  modified_base 6: mod_base = OTHER; note = 2'-deoxy-2'-fluorouridine-3'-phosphate
  modified_base 7: mod_base = OTHER; note = 2'-O-methylcytidine-3'-phosphate
  modified_base 8: mod_base = OTHER; note = 2'-deoxy-2'-fluorouridine-3'-phosphate
  modified_base 9: mod_base = OTHER; note = 2'-deoxy-2'-fluorouridine-3'-phosphate
  modified_base 10: mod_base = OTHER; note = 2'-O-methylcytidine-3'-phosphate
  modified_base 11: mod_base = OTHER; note = 2'-O-methyluridine-3'-phosphate
  modified_base 12: mod_base = OTHER; note = 2'-O-methylguanosine-3'-phosphate
  modified_base 13: mod_base = OTHER; note = 2'-O-methyluridine-3'-phosphate
  modified_base 14: mod_base = OTHER; note = 2'-deoxy-2'-fluorouridine-3'-phosphate
  modified_base 15: mod_base = OTHER; note = 2'-O-methyluridine-3'-phosphate
  modified_base 16: mod_base = OTHER; note = 2'-deoxy-2'-fluorocytidine-3'-phosphate
  modified_base 17: mod_base = OTHER; note = 2'-O-methyladenosine-3'-phosphate
  modified_base 18: mod_base = OTHER; note = 2'-O-methyluridine-3'-phosphate
  modified_base 19: mod_base = OTHER; note = 2'-O-methyladenosine-3'-phosphate
  modified_base 20: mod_base = OTHER; note = 2'-O-methyladenosine-3'-phosphate
  modified_base 21: mod_base = OTHER; note = 2'-O-methylcytidine-3'-phosphorothioate
  modified_base 22: mod_base = OTHER; note = 2'-O-methyladenosine-3'-phosphorothioate
  modified_base 23: mod_base = OTHER; note = 2'-O-methyluridine
aaagttcttctgtttcataacat

SEQ ID NO: 432 - RNA, 23 nt, synthetic construct
  source 1..23: mol_type = other RNA
  modified_base 1: mod_base = OTHER; note = 2'-O-methyladenosine-3'-phosphorothioate
  modified_base 2: mod_base = OTHER; note = 2'-deoxy-2'-fluoroadenosine-3'-phosphorothioate
  modified_base 3: mod_base = OTHER; note = 2'-O-methyladenosine-3'-phosphate
  modified_base 4: mod_base = OTHER; note = 2'-O-methyladenosine-3'-phosphate
  modified_base 5: mod_base = OTHER; note = 2'-O-methylguanosine-3'-phosphate
  modified_base 6: mod_base = OTHER; note = 2'-deoxy-2'-fluorouridine-3'-phosphate
  modified_base 7: mod_base = OTHER; note = 2'-O-methylguanosine-3'-phosphate
  modified_base 8: mod_base = OTHER; note = 2'-deoxy-2'-fluorouridine-3'-phosphate
  modified_base 9: mod_base = OTHER; note = 2'-deoxy-2'-fluoroadenosine-3'-phosphate
  modified_base 10: mod_base = OTHER; note = 2'-O-methyladenosine-3'-phosphate
  modified_base 11: mod_base = OTHER; note = 2'-O-methyluridine-3'-phosphate
  modified_base 12: mod_base = OTHER; note = 2'-O-methyluridine-3'-phosphate
  modified_base 13: mod_base = OTHER; note = 2'-O-methylcytidine-3'-phosphate
  modified_base 14: mod_base = OTHER; note = 2'-deoxy-2'-fluorocytidine-3'-phosphate
  modified_base 15: mod_base = OTHER; note = 2'-O-methylcytidine-3'-phosphate
  modified_base 16: mod_base = OTHER; note = 2'-deoxy-2'-fluoroadenosine-3'-phosphate
  modified_base 17: mod_base = OTHER; note = 2'-O-methyladenosine-3'-phosphate
  modified_base 18: mod_base = OTHER; note = 2'-O-methyladenosine-3'-phosphate
  modified_base 19: mod_base = OTHER; note = 2'-O-methyluridine-3'-phosphate
  modified_base 20: mod_base = OTHER; note = 2'-O-methylcytidine-3'-phosphate
  modified_base 21: mod_base = OTHER; note = 2'-O-methyladenosine-3'-phosphorothioate
  modified_base 22: mod_base = OTHER; note = 2'-O-methyluridine-3'-phosphorothioate
  modified_base 23: mod_base = OTHER; note = 2'-O-methylguanosine
aaaagtgtaattcccaaatcatg

SEQ ID NO: 433 - RNA, 23 nt, synthetic construct
  source 1..23: mol_type = other RNA
  modified_base 1: mod_base = OTHER; note = 2'-O-methyladenosine-3'-phosphorothioate
  modified_base 2: mod_base = OTHER; note = 2'-deoxy-2'-fluoroadenosine-3'-phosphorothioate
  modified_base 3: mod_base = OTHER; note = 2'-O-methyluridine-3'-phosphate
  modified_base 4: mod_base = OTHER; note = 2'-O-methyladenosine-3'-phosphate
  modified_base 5: mod_base = OTHER; note = 2'-O-methyladenosine-3'-phosphate
  modified_base 6: mod_base = OTHER; note = 2'-deoxy-2'-fluoroguanosine-3'-phosphate
  modified_base 7: mod_base = OTHER; note = 2'-O-methyladenosine-3'-phosphate
  modified_base 8: mod_base = OTHER; note = 2'-deoxy-2'-fluoroadenosine-3'-phosphate
  modified_base 9: mod_base = OTHER; note = 2'-deoxy-2'-fluoroadenosine-3'-phosphate
  modified_base 10: mod_base = OTHER; note = 2'-O-methylcytidine-3'-phosphate
  modified_base 11: mod_base = OTHER; note = 2'-O-methyladenosine-3'-phosphate
  modified_base 12: mod_base = OTHER; note = 2'-O-methyluridine-3'-phosphate
  modified_base 13: mod_base = OTHER; note = 2'-O-methylcytidine-3'-phosphate
  modified_base 14: mod_base = OTHER; note = 2'-deoxy-2'-fluorouridine-3'-phosphate
  modified_base 15: mod_base = OTHER; note = 2'-O-methyladenosine-3'-phosphate
  modified_base 16: mod_base = OTHER; note = 2'-deoxy-2'-fluorouridine-3'-phosphate
  modified_base 17: mod_base = OTHER; note = 2'-O-methyluridine-3'-phosphate
  modified_base 18: mod_base = OTHER; note = 2'-O-methylguanosine-3'-phosphate
  modified_base 19: mod_base = OTHER; note = 2'-O-methyluridine-3'-phosphate
  modified_base 20: mod_base = OTHER; note = 2'-O-methyladenosine-3'-phosphate
  modified_base 21: mod_base = OTHER; note = 2'-O-methylcytidine-3'-phosphorothioate
  modified_base 22: mod_base = OTHER; note = 2'-O-methylcytidine-3'-phosphorothioate
  modified_base 23: mod_base = OTHER; note = 2'-O-methyladenosine
aataagaaacatctattgtacca

SEQ ID NO: 434 - RNA, 23 nt, synthetic construct
  source 1..23: mol_type = other RNA
  modified_base 1: mod_base = OTHER; note = 2'-O-methyladenosine-3'-phosphorothioate
  modified_base 2: mod_base = OTHER; note = 2'-deoxy-2'-fluoroadenosine-3'-phosphorothioate
  modified_base 3: mod_base = OTHER; note = 2'-O-methyladenosine-3'-phosphate
  modified_base 4: mod_base = OTHER; note = 2'-O-methylcytidine-3'-phosphate
  modified_base 5: mod_base = OTHER; note = 2'-O-methyladenosine-3'-phosphate
  modified_base 6: mod_base = OTHER; note = 2'-deoxy-2'-fluorocytidine-3'-phosphate
  modified_base 7: mod_base = OTHER; note = 2'-O-methyluridine-3'-phosphate
  modified_base 8: mod_base = OTHER; note = 2'-deoxy-2'-fluoroguanosine-3'-phosphate
  modified_base 9: mod_base = OTHER; note = 2'-deoxy-2'-fluorouridine-3'-phosphate
  modified_base 10: mod_base = OTHER; note = 2'-O-methyladenosine-3'-phosphate
  modified_base 11: mod_base = OTHER; note = 2'-O-methyluridine-3'-phosphate
  modified_base 12: mod_base = OTHER; note = 2'-O-methyluridine-3'-phosphate
  modified_base 13: mod_base = OTHER; note = 2'-O-methylcytidine-3'-phosphate
  modified_base 14: mod_base = OTHER; note = 2'-deoxy-2'-fluorouridine-3'-phosphate
  modified_base 15: mod_base = OTHER; note = 2'-O-methylguanosine-3'-phosphate
  modified_base 16: mod_base = OTHER; note = 2'-deoxy-2'-fluoroadenosine-3'-phosphate
  modified_base 17: mod_base = OTHER; note = 2'-O-methyluridine-3'-phosphate
  modified_base 18: mod_base = OTHER; note = 2'-O-methylguanosine-3'-phosphate
  modified_base 19: mod_base = OTHER; note = 2'-O-methyladenosine-3'-phosphate
  modified_base 20: mod_base = OTHER; note = 2'-O-methyladenosine-3'-phosphate
  modified_base 21: mod_base = OTHER; note = 2'-O-methyluridine-3'-phosphorothioate
  modified_base 22: mod_base = OTHER; note = 2'-O-methylguanosine-3'-phosphorothioate
  modified_base 23: mod_base = OTHER; note = 2'-O-methyluridine
aaacactgtattctgatgaatgt

SEQ ID NO: 435 - RNA, 23 nt, synthetic construct
  source 1..23: mol_type = other RNA
  modified_base 1: mod_base = OTHER; note = 2'-O-methyladenosine-3'-phosphorothioate
  modified_base 2: mod_base = OTHER; note = 2'-deoxy-2'-fluoroadenosine-3'-phosphorothioate
  modified_base 3: mod_base = OTHER; note = 2'-O-methyluridine-3'-phosphate
  modified_base 4: mod_base = OTHER; note = 2'-O-methyluridine-3'-phosphate
  modified_base 5: mod_base = OTHER; note = 2'-O-methyluridine-3'-phosphate
  modified_base 6: mod_base = OTHER; note = 2'-deoxy-2'-fluorouridine-3'-phosphate
  modified_base 7: mod_base = OTHER; note = 2'-O-methyladenosine-3'-phosphate
  modified_base 8: mod_base = OTHER; note = 2'-deoxy-2'-fluoroadenosine-3'-phosphate
  modified_base 9: mod_base = OTHER; note = 2'-deoxy-2'-fluoroadenosine-3'-phosphate
  modified_base 10: mod_base = OTHER; note = 2'-O-methylguanosine-3'-phosphate
  modified_base 11: mod_base = OTHER; note = 2'-O-methyluridine-3'-phosphate
  modified_base 12: mod_base = OTHER; note = 2'-O-methyluridine-3'-phosphate
  modified_base 13: mod_base = OTHER; note = 2'-O-methylguanosine-3'-phosphate
  modified_base 14: mod_base = OTHER; note = 2'-deoxy-2'-fluorocytidine-3'-phosphate
  modified_base 15: mod_base = OTHER; note = 2'-O-methyladenosine-3'-phosphate
  modified_base 16: mod_base = OTHER; note = 2'-deoxy-2'-fluoroguanosine-3'-phosphate
  modified_base 17: mod_base = OTHER; note = 2'-O-methyladenosine-3'-phosphate
  modified_base 18: mod_base = OTHER; note = 2'-O-methyluridine-3'-phosphate
  modified_base 19: mod_base = OTHER; note = 2'-O-methylcytidine-3'-phosphate
  modified_base 20: mod_base = OTHER; note = 2'-O-methyluridine-3'-phosphate
  modified_base 21: mod_base = OTHER; note = 2'-O-methylguanosine-3'-phosphorothioate
  modified_base 22: mod_base = OTHER; note = 2'-O-methyladenosine-3'-phosphorothioate
  modified_base 23: mod_base = OTHER; note = 2'-O-methyladenosine
aattttaaagttgcagatctgaa

SEQ ID NO: 436 - RNA, 23 nt, synthetic construct
  source 1..23: mol_type = other RNA
  modified_base 1: mod_base = OTHER; note = 2'-O-methyladenosine-3'-phosphorothioate
  modified_base 2: mod_base = OTHER; note = 2'-deoxy-2'-fluoroadenosine-3'-phosphorothioate
  modified_base 3: mod_base = OTHER; note = 2'-O-methyluridine-3'-phosphate
  modified_base 4: mod_base = OTHER; note = 2'-O-methyluridine-3'-phosphate
  modified_base 5: mod_base = OTHER; note = 2'-O-methyladenosine-3'-phosphate
  modified_base 6: mod_base = OTHER; note = 2'-deoxy-2'-fluoroguanosine-3'-phosphate
  modified_base 7: mod_base = OTHER; note = 2'-O-methylguanosine-3'-phosphate
  modified_base 8: mod_base = OTHER; note = 2'-deoxy-2'-fluorocytidine-3'-phosphate
  modified_base 9: mod_base = OTHER; note = 2'-deoxy-2'-fluorouridine-3'-phosphate
  modified_base 10: mod_base = OTHER; note = 2'-O-methyluridine-3'-phosphate
  modified_base 11: mod_base = OTHER; note = 2'-O-methyluridine-3'-phosphate
  modified_base 12: mod_base = OTHER; note = 2'-O-methylcytidine-3'-phosphate
  modified_base 13: mod_base = OTHER; note = 2'-O-methyluridine-3'-phosphate
  modified_base 14: mod_base = OTHER; note = 2'-deoxy-2'-fluorouridine-3'-phosphate
  modified_base 15: mod_base = OTHER; note = 2'-O-methyluridine-3'-phosphate
  modified_base 16: mod_base = OTHER; note = 2'-deoxy-2'-fluorocytidine-3'-phosphate
  modified_base 17: mod_base = OTHER; note = 2'-O-methylcytidine-3'-phosphate
  modified_base 18: mod_base = OTHER; note = 2'-O-methyladenosine-3'-phosphate
  modified_base 19: mod_base = OTHER; note = 2'-O-methyluridine-3'-phosphate
  modified_base 20: mod_base = OTHER; note = 2'-O-methyluridine-3'-phosphate
  modified_base 21: mod_base = OTHER; note = 2'-O-methyluridine-3'-phosphorothioate
  modified_base 22: mod_base = OTHER; note = 2'-O-methyluridine-3'-phosphorothioate
  modified_base 23: mod_base = OTHER; note = 2'-O-methyladenosine
aattaggctttctttccatttta

SEQ ID NO: 437 - RNA, 23 nt, synthetic construct
  source 1..23: mol_type = other RNA
  modified_base 1: mod_base = OTHER; note = 2'-O-methyladenosine-3'-phosphorothioate
  modified_base 2: mod_base = OTHER; note = 2'-deoxy-2'-fluoroguanosine-3'-phosphorothioate
  modified_base 3: mod_base = OTHER; note = 2'-O-methyluridine-3'-phosphate
  modified_base 4: mod_base = OTHER; note = 2'-O-methyladenosine-3'-phosphate
  modified_base 5: mod_base = OTHER; note = 2'-O-methyladenosine-3'-phosphate
  modified_base 6: mod_base = OTHER; note = 2'-deoxy-2'-fluorocytidine-3'-phosphate
  modified_base 7: mod_base = OTHER; note = 2'-O-methyladenosine-3'-phosphate
  modified_base 8: mod_base = OTHER; note = 2'-deoxy-2'-fluoroadenosine-3'-phosphate
  modified_base 9: mod_base = OTHER; note = 2'-deoxy-2'-fluorocytidine-3'-phosphate
  modified_base 10: mod_base = OTHER; note = 2'-O-methyladenosine-3'-phosphate
  modified_base 11: mod_base = OTHER; note = 2'-O-methyluridine-3'-phosphate
  modified_base 12: mod_base = OTHER; note = 2'-O-methylcytidine-3'-phosphate
  modified_base 13: mod_base = OTHER; note = 2'-O-methyluridine-3'-phosphate
  modified_base 14: mod_base = OTHER; note = 2'-deoxy-2'-fluorouridine-3'-phosphate
  modified_base 15: mod_base = OTHER; note = 2'-O-methylcytidine-3'-phosphate
  modified_base 16: mod_base = OTHER; note = 2'-deoxy-2'-fluorocytidine-3'-phosphate
  modified_base 17: mod_base = OTHER; note = 2'-O-methyladenosine-3'-phosphate
  modified_base 18: mod_base = OTHER; note = 2'-O-methyladenosine-3'-phosphate
  modified_base 19: mod_base = OTHER; note = 2'-O-methylcytidine-3'-phosphate
  modified_base 20: mod_base = OTHER; note = 2'-O-methyladenosine-3'-phosphate
  modified_base 21: mod_base = OTHER; note = 2'-O-methyladenosine-3'-phosphorothioate
  modified_base 22: mod_base = OTHER; note = 2'-O-methyladenosine-3'-phosphorothioate
  modified_base 23: mod_base = OTHER; note = 2'-O-methyluridine
agtaacaacatcttccaacaaat

SEQ ID NO: 438 - RNA, 23 nt, synthetic construct
  source 1..23: mol_type = other RNA
  modified_base 1: mod_base = OTHER; note = 2'-O-methyladenosine-3'-phosphorothioate
  modified_base 2: mod_base = OTHER; note = 2'-deoxy-2'-fluorouridine-3'-phosphorothioate
  modified_base 3: mod_base = OTHER; note = 2'-O-methylguanosine-3'-phosphate
  modified_base 4: mod_base = OTHER; note = 2'-O-methyladenosine-3'-phosphate
  modified_base 5: mod_base = OTHER; note = 2'-O-methyluridine-3'-phosphate
  modified_base 6: mod_base = OTHER; note = 2'-deoxy-2'-fluoroadenosine-3'-phosphate
  modified_base 7: mod_base = OTHER; note = 2'-O-methyluridine-3'-phosphate
  modified_base 8: mod_base = OTHER; note = 2'-deoxy-2'-fluoroadenosine-3'-phosphate
  modified_base 9: mod_base = OTHER; note = 2'-deoxy-2'-fluoroadenosine-3'-phosphate
  modified_base 10: mod_base = OTHER; note = 2'-O-methyladenosine-3'-phosphate
  modified_base 11: mod_base = OTHER; note = 2'-O-methyluridine-3'-phosphate
  modified_base 12: mod_base = OTHER; note = 2'-O-methyladenosine-3'-phosphate
  modified_base 13: mod_base = OTHER; note = 2'-O-methyladenosine-3'-phosphate
  modified_base 14: mod_base = OTHER; note = 2'-deoxy-2'-fluorocytidine-3'-phosphate
  modified_base 15: mod_base = OTHER; note = 2'-O-methyladenosine-3'-phosphate
  modified_base 16: mod_base = OTHER; note = 2'-deoxy-2'-fluorouridine-3'-phosphate
  modified_base 17: mod_base = OTHER; note = 2'-O-methyluridine-3'-phosphate
  modified_base 18: mod_base = OTHER; note = 2'-O-methylcytidine-3'-phosphate
  modified_base 19: mod_base = OTHER; note = 2'-O-methylcytidine-3'-phosphate
  modified_base 20: mod_base = OTHER; note = 2'-O-methylguanosine-3'-phosphate
  modified_base 21: mod_base = OTHER; note = 2'-O-methylcytidine-3'-phosphorothioate
  modified_base 22: mod_base = OTHER; note = 2'-O-methyladenosine-3'-phosphorothioate
  modified_base 23: mod_base = OTHER; note = 2'-O-methyladenosine
atgatataaataacattccgcaa

SEQ ID NO: 439 - RNA, 23 nt, synthetic construct
  source 1..23: mol_type = other RNA
  modified_base 1: mod_base = OTHER; note = 2'-O-methyladenosine-3'-phosphorothioate
  modified_base 2: mod_base = OTHER; note = 2'-deoxy-2'-fluorouridine-3'-phosphorothioate
  modified_base 3: mod_base = OTHER; note = 2'-O-methyluridine-3'-phosphate
  modified_base 4: mod_base = OTHER; note = 2'-O-methylguanosine-3'-phosphate
  modified_base 5: mod_base = OTHER; note = 2'-O-methyluridine-3'-phosphate
  modified_base 6: mod_base = OTHER; note = 2'-deoxy-2'-fluoroguanosine-3'-phosphate
  modified_base 7: mod_base = OTHER; note = 2'-O-methyluridine-3'-phosphate
  modified_base 8: mod_base = OTHER; note = 2'-deoxy-2'-fluoroguanosine-3'-phosphate
  modified_base 9: mod_base = OTHER; note = 2'-deoxy-2'-fluoroadenosine-3'-phosphate
  modified_base 10: mod_base = OTHER; note = 2'-O-methylguanosine-3'-phosphate
  modified_base 11: mod_base = OTHER; note = 2'-O-methyluridine-3'-phosphate
  modified_base 12: mod_base = OTHER; note = 2'-O-methyluridine-3'-phosphate
  modified_base 13: mod_base = OTHER; note = 2'-O-methyluridine-3'-phosphate
  modified_base 14: mod_base = OTHER; note = 2'-deoxy-2'-fluorocytidine-3'-phosphate
  modified_base 15: mod_base = OTHER; note = 2'-O-methyladenosine-3'-phosphate
  modified_base 16: mod_base = OTHER; note = 2'-deoxy-2'-fluorouridine-3'-phosphate
  modified_base 17: mod_base = OTHER; note = 2'-O-methyluridine-3'-phosphate
  modified_base 18: mod_base = OTHER; note = 2'-O-methylguanosine-3'-phosphate
  modified_base 19: mod_base = OTHER; note = 2'-O-methyladenosine-3'-phosphate
  modified_base 20: mod_base = OTHER; note = 2'-O-methyluridine-3'-phosphate
  modified_base 21: mod_base = OTHER; note = 2'-O-methyladenosine-3'-phosphorothioate
  modified_base 22: mod_base = OTHER; note = 2'-O-methyluridine-3'-phosphorothioate
  modified_base 23: mod_base = OTHER; note = 2'-O-methyladenosine
attgtgtgagtttcattgatata

SEQ ID NO: 440 - RNA, 23 nt, synthetic construct
  source 1..23: mol_type = other RNA
  modified_base 1: mod_base = OTHER; note = 2'-O-methyladenosine-3'-phosphorothioate
  modified_base 2: mod_base = OTHER; note = 2'-deoxy-2'-fluoroadenosine-3'-phosphorothioate
  modified_base 3: mod_base = OTHER; note = 2'-O-methyladenosine-3'-phosphate
  modified_base 4: mod_base = OTHER; note = 2'-O-methylguanosine-3'-phosphate
  modified_base 5: mod_base = OTHER; note = 2'-O-methyladenosine-3'-phosphate
  modified_base 6: mod_base = OTHER; note = 2'-deoxy-2'-fluoroadenosine-3'-phosphate
  modified_base 7: mod_base = OTHER; note = 2'-O-methylcytidine-3'-phosphate
  modified_base 8: mod_base = OTHER; note = 2'-deoxy-2'-fluoroguanosine-3'-phosphate
  modified_base 9: mod_base = OTHER; note = 2'-deoxy-2'-fluorouridine-3'-phosphate
  modified_base 10: mod_base = OTHER; note = 2'-O-methyladenosine-3'-phosphate
  modified_base 11: mod_base = OTHER; note = 2'-O-methyladenosine-3'-phosphate
  modified_base 12: mod_base = OTHER; note = 2'-O-methylguanosine-3'-phosphate
  modified_base 13: mod_base = OTHER; note = 2'-O-methyladenosine-3'-phosphate
  modified_base 14: mod_base = OTHER; note = 2'-deoxy-2'-fluoroadenosine-3'-phosphate
  modified_base 15: mod_base = OTHER; note = 2'-O-methyladenosine-3'-phosphate
  modified_base 16: mod_base = OTHER; note = 2'-deoxy-2'-fluoroguanosine-3'-phosphate
  modified_base 17: mod_base = OTHER; note = 2'-O-methylguanosine-3'-phosphate
  modified_base 18: mod_base = OTHER; note = 2'-O-methylcytidine-3'-phosphate
  modified_base 19: mod_base = OTHER; note = 2'-O-methylguanosine-3'-phosphate
  modified_base 20: mod_base = OTHER; note = 2'-O-methyluridine-3'-phosphate
  modified_base 21: mod_base = OTHER; note = 2'-O-methylcytidine-3'-phosphorothioate
  modified_base 22: mod_base = OTHER; note = 2'-O-methyluridine-3'-phosphorothioate
  modified_base 23: mod_base = OTHER; note = 2'-O-methyluridine
aaagaacgtaagaaaggcgtctt

SEQ ID NO: 441 - RNA, 23 nt, synthetic construct
  source 1..23: mol_type = other RNA
  modified_base 1: mod_base = OTHER; note = 2'-O-methyladenosine-3'-phosphorothioate
  modified_base 2: mod_base = OTHER; note = 2'-deoxy-2'-fluoroadenosine-3'-phosphorothioate
  modified_base 3: mod_base = OTHER; note = 2'-O-methylcytidine-3'-phosphate
  modified_base 4: mod_base = OTHER; note = 2'-O-methyladenosine-3'-phosphate
  modified_base 5: mod_base = OTHER; note = 2'-O-methyluridine-3'-phosphate
  modified_base 6: mod_base = OTHER; note = 2'-deoxy-2'-fluorouridine-3'-phosphate
  modified_base 7: mod_base = OTHER; note = 2'-O-methyluridine-3'-phosphate
  modified_base 8: mod_base = OTHER; note = 2'-deoxy-2'-fluorouridine-3'-phosphate
  modified_base 9: mod_base = OTHER; note = 2'-deoxy-2'-fluorocytidine-3'-phosphate
  modified_base 10: mod_base = OTHER; note = 2'-O-methyladenosine-3'-phosphate
  modified_base 11: mod_base = OTHER; note = 2'-O-methylguanosine-3'-phosphate
  modified_base 12: mod_base = OTHER; note = 2'-O-methyluridine-3'-phosphate
  modified_base 13: mod_base = OTHER; note = 2'-O-methylcytidine-3'-phosphate
  modified_base 14: mod_base = OTHER; note = 2'-deoxy-2'-fluoroadenosine-3'-phosphate
  modified_base 15: mod_base = OTHER; note = 2'-O-methylcytidine-3'-phosphate
  modified_base 16: mod_base = OTHER; note = 2'-deoxy-2'-fluoroadenosine-3'-phosphate
  modified_base 17: mod_base = OTHER; note = 2'-O-methyluridine-3'-phosphate
  modified_base 18: mod_base = OTHER; note = 2'-O-methyluridine-3'-phosphate
  modified_base 19: mod_base = OTHER; note = 2'-O-methylguanosine-3'-phosphate
  modified_base 20: mod_base = OTHER; note = 2'-O-methylguanosine-3'-phosphate
  modified_base 21: mod_base = OTHER; note = 2'-O-methyluridine-3'-phosphorothioate
  modified_base 22: mod_base = OTHER; note = 2'-O-methylguanosine-3'-phosphorothioate
  modified_base 23: mod_base = OTHER; note = 2'-O-methylguanosine
aacattttcagtcacattggtgg

SEQ ID NO: 442 - RNA, 23 nt, synthetic construct
  source 1..23: mol_type = other RNA
  modified_base 1: mod_base = OTHER; note = 2'-O-methyladenosine-3'-phosphorothioate
  modified_base 2: mod_base = OTHER; note = 2'-deoxy-2'-fluorouridine-3'-phosphorothioate
  modified_base 3: mod_base = OTHER; note = 2'-O-methyluridine-3'-phosphate
  modified_base 4: mod_base = OTHER; note = 2'-O-methyluridine-3'-phosphate
  modified_base 5: mod_base = OTHER; note = 2'-O-methylcytidine-3'-phosphate
  modified_base 6: mod_base = OTHER; note = 2'-deoxy-2'-fluoroadenosine-3'-phosphate
  modified_base 7: mod_base = OTHER; note = 2'-O-methylcytidine-3'-phosphate
  modified_base 8: mod_base = OTHER; note = 2'-deoxy-2'-fluorouridine-3'-phosphate
  modified_base 9: mod_base = OTHER; note = 2'-deoxy-2'-fluorouridine-3'-phosphate
  modified_base 10: mod_base = OTHER; note = 2'-O-methyluridine-3'-phosphate
  modified_base 11: mod_base = OTHER; note = 2'-O-methylguanosine-3'-phosphate
  modified_base 12: mod_base = OTHER; note = 2'-O-methyluridine-3'-phosphate
  modified_base 13: mod_base = OTHER; note = 2'-O-methyluridine-3'-phosphate
  modified_base 14: mod_base = OTHER; note = 2'-deoxy-2'-fluoroadenosine-3'-phosphate
  modified_base 15: mod_base = OTHER; note = 2'-O-methyladenosine-3'-phosphate
  modified_base 16: mod_base = OTHER; note = 2'-deoxy-2'-fluorocytidine-3'-phosphate
  modified_base 17: mod_base = OTHER; note = 2'-O-methylguanosine-3'-phosphate
  modified_base 18: mod_base = OTHER; note = 2'-O-methylguanosine-3'-phosphate
  modified_base 19: mod_base = OTHER; note = 2'-O-methylcytidine-3'-phosphate
  modified_base 20: mod_base = OTHER; note = 2'-O-methyluridine-3'-phosphate
  modified_base 21: mod_base = OTHER; note = 2'-O-methyluridine-3'-phosphorothioate
  modified_base 22: mod_base = OTHER; note = 2'-O-methyluridine-3'-phosphorothioate
  modified_base 23: mod_base = OTHER; note = 2'-O-methyluridine
atttcactttgttaacggctttt

SEQ ID NO: 443 - RNA, 23 nt, synthetic construct
  source 1..23: mol_type = other RNA
  modified_base 1: mod_base = OTHER; note = 2'-O-methyladenosine-3'-phosphorothioate
  modified_base 2: mod_base = OTHER; note = 2'-deoxy-2'-fluoroadenosine-3'-phosphorothioate
  modified_base 3: mod_base = OTHER; note = 2'-O-methyluridine-3'-phosphate
  modified_base 4: mod_base = OTHER; note = 2'-O-methyluridine-3'-phosphate
  modified_base 5: mod_base = OTHER; note = 2'-O-methyluridine-3'-phosphate
  modified_base 6: mod_base = OTHER; note = 2'-deoxy-2'-fluorocytidine-3'-phosphate
  modified_base 7: mod_base = OTHER; note = 2'-O-methyluridine-3'-phosphate
  modified_base 8: mod_base = OTHER; note = 2'-deoxy-2'-fluorouridine-3'-phosphate
  modified_base 9: mod_base = OTHER; note = 2'-deoxy-2'-fluoroguanosine-3'-phosphate
  modified_base 10: mod_base = OTHER; note = 2'-O-methyladenosine-3'-phosphate
  modified_base 11: mod_base = OTHER; note = 2'-O-methyladenosine-3'-phosphate
  modified_base 12: mod_base = OTHER; note = 2'-O-methylguanosine-3'-phosphate
  modified_base 13: mod_base = OTHER; note = 2'-O-methyladenosine-3'-phosphate
  modified_base 14: mod_base = OTHER; note = 2'-deoxy-2'-fluoroadenosine-3'-phosphate
  modified_base 15: mod_base = OTHER; note = 2'-O-methyluridine-3'-phosphate
  modified_base 16: mod_base = OTHER; note = 2'-deoxy-2'-fluorocytidine-3'-phosphate
  modified_base 17: mod_base = OTHER; note = 2'-O-methylcytidine-3'-phosphate
  modified_base 18: mod_base = OTHER; note = 2'-O-methyluridine-3'-phosphate
  modified_base 19: mod_base = OTHER; note = 2'-O-methyluridine-3'-phosphate
  modified_base 20: mod_base = OTHER; note = 2'-O-methyluridine-3'-phosphate
  modified_base 21: mod_base = OTHER; note = 2'-O-methyluridine-3'-phosphorothioate
  modified_base 22: mod_base = OTHER; note = 2'-O-methyladenosine-3'-phosphorothioate
  modified_base 23: mod_base = OTHER; note = 2'-O-methylguanosine
aatttcttgaagaatccttttag

SEQ ID NO: 444 - RNA, 23 nt, synthetic construct
  source 1..23: mol_type = other RNA
  modified_base 1: mod_base = OTHER; note = 2'-O-methyladenosine-3'-phosphorothioate
  modified_base 2: mod_base = OTHER; note = 2'-deoxy-2'-fluoroadenosine-3'-phosphorothioate
  modified_base 3: mod_base = OTHER; note = 2'-O-methyladenosine-3'-phosphate
  modified_base 4: mod_base = OTHER; note = 2'-O-methyluridine-3'-phosphate
  modified_base 5: mod_base = OTHER; note = 2'-O-methyluridine-3'-phosphate
  modified_base 6: mod_base = OTHER; note = 2'-deoxy-2'-fluorouridine-3'-phosphate
  modified_base 7: mod_base = OTHER; note = 2'-O-methylguanosine-3'-phosphate
  modified_base 8: mod_base = OTHER; note = 2'-deoxy-2'-fluoroadenosine-3'-phosphate
  modified_base 9: mod_base = OTHER; note = 2'-deoxy-2'-fluoroadenosine-3'-phosphate
  modified_base 10: mod_base = OTHER; note = 2'-O-methyluridine-3'-phosphate
  modified_base 11: mod_base = OTHER; note = 2'-O-methylguanosine-3'-phosphate
  modified_base 12: mod_base = OTHER; note = 2'-O-methyluridine-3'-phosphate
  modified_base 13: mod_base = OTHER; note = 2'-O-methyluridine-3'-phosphate
  modified_base 14: mod_base = OTHER; note = 2'-deoxy-2'-fluorocytidine-3'-phosphate
  modified_base 15: mod_base = OTHER; note = 2'-O-methylcytidine-3'-phosphate
  modified_base 16: mod_base = OTHER; note = 2'-deoxy-2'-fluoroadenosine-3'-phosphate
  modified_base 17: mod_base = OTHER; note = 2'-O-methyladenosine-3'-phosphate
  modified_base 18: mod_base = OTHER; note = 2'-O-methyladenosine-3'-phosphate
  modified_base 19: mod_base = OTHER; note = 2'-O-methyladenosine-3'-phosphate
  modified_base 20: mod_base = OTHER; note = 2'-O-methylguanosine-3'-phosphate
  modified_base 21: mod_base = OTHER; note = 2'-O-methyladenosine-3'-phosphorothioate
  modified_base 22: mod_base = OTHER; note = 2'-O-methyladenosine-3'-phosphorothioate
  modified_base 23: mod_base = OTHER; note = 2'-O-methylguanosine
aaatttgaatgttccaaaagaag

SEQ ID NO: 445 - RNA, 23 nt, synthetic construct
  source 1..23: mol_type = other RNA
  modified_base 1: mod_base = OTHER; note = 2'-O-methyladenosine-3'-phosphorothioate
  modified_base 2: mod_base = OTHER; note = 2'-deoxy-2'-fluoroadenosine-3'-phosphorothioate
  modified_base 3: mod_base = OTHER; note = 2'-O-methyladenosine-3'-phosphate
  modified_base 4: mod_base = OTHER; note = 2'-O-methylguanosine-3'-phosphate
  modified_base 5: mod_base = OTHER; note = 2'-O-methyluridine-3'-phosphate
  modified_base 6: mod_base = OTHER; note = 2'-deoxy-2'-fluorouridine-3'-phosphate
  modified_base 7: mod_base = OTHER; note = 2'-O-methylguanosine-3'-phosphate
  modified_base 8: mod_base = OTHER; note = 2'-deoxy-2'-fluoroadenosine-3'-phosphate
  modified_base 9: mod_base = OTHER; note = 2'-deoxy-2'-fluorocytidine-3'-phosphate
  modified_base 10: mod_base = OTHER; note = 2'-O-methylcytidine-3'-phosphate
  modified_base 11: mod_base = OTHER; note = 2'-O-methyluridine-3'-phosphate
  modified_base 12: mod_base = OTHER; note = 2'-O-methyluridine-3'-phosphate
  modified_base 13: mod_base = OTHER; note = 2'-O-methyluridine-3'-phosphate
  modified_base 14: mod_base = OTHER; note = 2'-deoxy-2'-fluoroguanosine-3'-phosphate
  modified_base 15: mod_base = OTHER; note = 2'-O-methyluridine-3'-phosphate
  modified_base 16: mod_base = OTHER; note = 2'-deoxy-2'-fluoroguanosine-3'-phosphate
  modified_base 17: mod_base = OTHER; note = 2'-O-methyladenosine-3'-phosphate
  modified_base 18: mod_base = OTHER; note = 2'-O-methyladenosine-3'-phosphate
  modified_base 19: mod_base = OTHER; note = 2'-O-methyluridine-3'-phosphate
  modified_base 20: mod_base = OTHER; note = 2'-O-methyluridine-3'-phosphate
  modified_base 21: mod_base = OTHER; note = 2'-O-methyluridine-3'-phosphorothioate
  modified_base 22: mod_base = OTHER; note = 2'-O-methylguanosine-3'-phosphorothioate
  modified_base 23: mod_base = OTHER; note = 2'-O-methyladenosine
aaagttgacctttgtgaatttga

SEQ ID NO: 446 - RNA, 23 nt, synthetic construct
  source 1..23: mol_type = other RNA
  modified_base 1: mod_base = OTHER; note = 2'-O-methyladenosine-3'-phosphorothioate
  modified_base 2: mod_base = OTHER; note = 2'-deoxy-2'-fluoroguanosine-3'-phosphorothioate
  modified_base 3: mod_base = OTHER; note = 2'-O-methyladenosine-3'-phosphate
  modified_base 4: mod_base = OTHER; note = 2'-O-methyluridine-3'-phosphate
  modified_base 5: mod_base = OTHER; note = 2'-O-methylcytidine-3'-phosphate
  modified_base 6: mod_base = OTHER; note = 2'-deoxy-2'-fluorouridine-3'-phosphate
  modified_base 7: mod_base = OTHER; note = 2'-O-methyladenosine-3'-phosphate
  modified_base 8: mod_base = OTHER; note = 2'-deoxy-2'-fluorouridine-3'-phosphate
  modified_base 9: mod_base = OTHER; note = 2'-deoxy-2'-fluoroguanosine-3'-phosphate
  modified_base 10: mod_base = OTHER; note = 2'-O-methyladenosine-3'-phosphate
  modified_base 11: mod_base = OTHER; note = 2'-O-methyladenosine-3'-phosphate
  modified_base 12: mod_base = OTHER; note = 2'-O-methylcytidine-3'-phosphate
  modified_base 13: mod_base = OTHER; note = 2'-O-methyluridine-3'-phosphate
  modified_base 14: mod_base = OTHER; note = 2'-deoxy-2'-fluoroguanosine-3'-phosphate
  modified_base 15: mod_base = OTHER; note = 2'-O-methylguanosine-3'-phosphate
  modified_base 16: mod_base = OTHER; note = 2'-deoxy-2'-fluorouridine-3'-phosphate
  modified_base 17: mod_base = OTHER; note = 2'-O-methyladenosine-3'-phosphate
  modified_base 18: mod_base = OTHER; note = 2'-O-methylguanosine-3'-phosphate
  modified_base 19: mod_base = OTHER; note = 2'-O-methyladenosine-3'-phosphate
  modified_base 20: mod_base = OTHER; note = 2'-O-methyladenosine-3'-phosphate
  modified_base 21: mod_base = OTHER; note = 2'-O-methyladenosine-3'-phosphorothioate
  modified_base 22: mod_base = OTHER; note = 2'-O-methylcytidine-3'-phosphorothioate
  modified_base 23: mod_base = OTHER; note = 2'-O-methyladenosine
agatctatgaactggtagaaaca

SEQ ID NO: 447 - RNA, 23 nt, synthetic construct
  source 1..23: mol_type = other RNA
  modified_base 1: mod_base = OTHER; note = 2'-O-methyladenosine-3'-phosphorothioate
  modified_base 2: mod_base = OTHER; note = 2'-deoxy-2'-fluoroadenosine-3'-phosphorothioate
  modified_base 3: mod_base = OTHER; note = 2'-O-methylguanosine-3'-phosphate
  modified_base 4: mod_base = OTHER; note = 2'-O-methyladenosine-3'-phosphate
  modified_base 5: mod_base = OTHER; note = 2'-O-methyluridine-3'-phosphate
  modified_base 6: mod_base = OTHER; note = 2'-deoxy-2'-fluoroadenosine-3'-phosphate
  modified_base 7: mod_base = OTHER; note = 2'-O-methylguanosine-3'-phosphate
  modified_base 8: mod_base = OTHER; note = 2'-deoxy-2'-fluorouridine-3'-phosphate
  modified_base 9: mod_base = OTHER; note = 2'-deoxy-2'-fluorocytidine-3'-phosphate
  modified_base 10: mod_base = OTHER; note = 2'-O-methyladenosine-3'-phosphate
  modified_base 11: mod_base = OTHER; note = 2'-O-methyladenosine-3'-phosphate
  modified_base 12: mod_base = OTHER; note = 2'-O-methyluridine-3'-phosphate
  modified_base 13: mod_base = OTHER; note = 2'-O-methyladenosine-3'-phosphate
  modified_base 14: mod_base = OTHER; note = 2'-deoxy-2'-fluorouridine-3'-phosphate
  modified_base 15: mod_base = OTHER; note = 2'-O-methylguanosine-3'-phosphate
  modified_base 16: mod_base = OTHER; note = 2'-deoxy-2'-fluoroguanosine-3'-phosphate
  modified_base 17: mod_base = OTHER; note = 2'-O-methylguanosine-3'-phosphate
  modified_base 18: mod_base = OTHER; note = 2'-O-methyladenosine-3'-phosphate
  modified_base 19: mod_base = OTHER; note = 2'-O-methyluridine-3'-phosphate
  modified_base 20: mod_base = OTHER; note = 2'-O-methylcytidine-3'-phosphate
  modified_base 21: mod_base = OTHER; note = 2'-O-methyluridine-3'-phosphorothioate
  modified_base 22: mod_base = OTHER; note = 2'-O-methyladenosine-3'-phosphorothioate
  modified_base 23: mod_base = OTHER; note = 2'-O-methyluridine
aagatagtcaatatgggatctat

SEQ ID NO: 448 - RNA, 23 nt, synthetic construct
  source 1..23: mol_type = other RNA
  modified_base 1: mod_base = OTHER; note = 2'-O-methyladenosine-3'-phosphorothioate
  modified_base 2: mod_base = OTHER; note = 2'-deoxy-2'-fluoroadenosine-3'-phosphorothioate
  modified_base 3: mod_base = OTHER; note = 2'-O-methylguanosine-3'-phosphate
  modified_base 4: mod_base = OTHER; note = 2'-O-methyladenosine-3'-phosphate
  modified_base 5: mod_base = OTHER; note = 2'-O-methyladenosine-3'-phosphate
  modified_base 6: mod_base = OTHER; note = 2'-deoxy-2'-fluoroguanosine-3'-phosphate
  modified_base 7: mod_base = OTHER; note = 2'-O-methyladenosine-3'-phosphate
  modified_base 8: mod_base = OTHER; note = 2'-deoxy-2'-fluoroguanosine-3'-phosphate
  modified_base 9: mod_base = OTHER; note = 2'-deoxy-2'-fluoroadenosine-3'-phosphate
  modified_base 10: mod_base = OTHER; note = 2'-O-methyladenosine-3'-phosphate
  modified_base 11: mod_base = OTHER; note = 2'-O-methyluridine-3'-phosphate
  modified_base 12: mod_base = OTHER; note = 2'-O-methylguanosine-3'-phosphate
  modified_base 13: mod_base = OTHER; note = 2'-O-methyladenosine-3'-phosphate
  modified_base 14: mod_base = OTHER; note = 2'-deoxy-2'-fluoroadenosine-3'-phosphate
  modified_base 15: mod_base = OTHER; note = 2'-O-methyladenosine-3'-phosphate
  modified_base 16: mod_base = OTHER; note = 2'-deoxy-2'-fluoroguanosine-3'-phosphate
  modified_base 17: mod_base = OTHER; note = 2'-O-methyluridine-3'-phosphate
  modified_base 18: mod_base = OTHER; note = 2'-O-methylguanosine-3'-phosphate
  modified_base 19: mod_base = OTHER; note = 2'-O-methyladenosine-3'-phosphate
  modified_base 20: mod_base = OTHER; note = 2'-O-methylguanosine-3'-phosphate
  modified_base 21: mod_base = OTHER; note = 2'-O-methylcytidine-3'-phosphorothioate
  modified_base 22: mod_base = OTHER; note = 2'-O-methyladenosine-3'-phosphorothioate
  modified_base 23: mod_base = OTHER; note = 2'-O-methylguanosine
aagaagagaatgaaagtgagcag

SEQ ID NO: 449 - RNA, 23 nt, synthetic construct
  source 1..23: mol_type = other RNA
  modified_base 1: mod_base = OTHER; note = 2'-O-methyladenosine-3'-phosphorothioate
  modified_base 2: mod_base = OTHER; note = 2'-deoxy-2'-fluoroadenosine-3'-phosphorothioate
  modified_base 3: mod_base = OTHER; note = 2'-O-methyluridine-3'-phosphate
  modified_base 4: mod_base = OTHER; note = 2'-O-methylguanosine-3'-phosphate
  modified_base 5: mod_base = OTHER; note = 2'-O-methyluridine-3'-phosphate
  modified_base 6: mod_base = OTHER; note = 2'-deoxy-2'-fluorouridine-3'-phosphate
  modified_base 7: mod_base = OTHER; note = 2'-O-methylguanosine-3'-phosphate
  modified_base 8: mod_base = OTHER; note = 2'-deoxy-2'-fluoroadenosine-3'-phosphate
  modified_base 9: mod_base = OTHER; note = 2'-deoxy-2'-fluoroguanosine-3'-phosphate
  modified_base 10: mod_base = OTHER; note = 2'-O-methyladenosine-3'-phosphate
  modified_base 11: mod_base = OTHER; note = 2'-O-methyluridine-3'-phosphate
  modified_base 12: mod_base = OTHER; note = 2'-O-methyluridine-3'-phosphate
  modified_base 13: mod_base = OTHER; note = 2'-O-methyladenosine-3'-phosphate
  modified_base 14: mod_base = OTHER; note = 2'-deoxy-2'-fluorouridine-3'-phosphate
  modified_base 15: mod_base = OTHER; note = 2'-O-methyluridine-3'-phosphate
  modified_base 16: mod_base = OTHER; note = 2'-deoxy-2'-fluoroguanosine-3'-phosphate
  modified_base 17: mod_base = OTHER; note = 2'-O-methylcytidine-3'-phosphate
  modified_base 18: mod_base = OTHER; note = 2'-O-methylcytidine-3'-phosphate
  modified_base 19: mod_base = OTHER; note = 2'-O-methyluridine-3'-phosphate
  modified_base 20: mod_base = OTHER; note = 2'-O-methylguanosine-3'-phosphate
  modified_base 21: mod_base = OTHER; note = 2'-O-methyladenosine-3'-phosphorothioate
  modified_base 22: mod_base = OTHER; note = 2'-O-methyladenosine-3'-phosphorothioate
  modified_base 23: mod_base = OTHER; note = 2'-O-methylguanosine
aatgttgagattattgcctgaag

SEQ ID NO: 450 - RNA, 23 nt, synthetic construct
  source 1..23: mol_type = other RNA
  modified_base 1: mod_base = OTHER; note = 2'-O-methyladenosine-3'-phosphorothioate
  modified_base 2: mod_base = OTHER; note = 2'-deoxy-2'-fluorouridine-3'-phosphorothioate
  modified_base 3: mod_base = OTHER; note = 2'-O-methyladenosine-3'-phosphate
  modified_base 4: mod_base = OTHER; note = 2'-O-methyluridine-3'-phosphate
  modified_base 5: mod_base = OTHER; note = 2'-O-methylguanosine-3'-phosphate
  modified_base 6: mod_base = OTHER; note = 2'-deoxy-2'-fluoroguanosine-3'-phosphate
  modified_base 7: mod_base = OTHER; note = 2'-O-methyladenosine-3'-phosphate
  modified_base 8: mod_base = OTHER; note = 2'-deoxy-2'-fluorouridine-3'-phosphate
  modified_base 9: mod_base = OTHER; note = 2'-deoxy-2'-fluorocytidine-3'-phosphate
  modified_base 10: mod_base = OTHER; note = 2'-O-methyladenosine-3'-phosphate
  modified_base 11: mod_base = OTHER; note = 2'-O-methyladenosine-3'-phosphate
  modified_base 12: mod_base = OTHER; note = 2'-O-methylguanosine-3'-phosphate
  modified_base 13: mod_base = OTHER; note = 2'-O-methylguanosine-3'-phosphate
  modified_base 14: mod_base = OTHER; note = 2'-deoxy-2'-fluorouridine-3'-phosphate
  modified_base 15: mod_base = OTHER; note = 2'-O-methyladenosine-3'-phosphate
  modified_base 16: mod_base = OTHER; note = 2'-deoxy-2'-fluorocytidine-3'-phosphate
  modified_base 17: mod_base = OTHER; note = 2'-O-methyluridine-3'-phosphate
  modified_base 18: mod_base = OTHER; note = 2'-O-methylguanosine-3'-phosphate
  modified_base 19: mod_base = OTHER; note = 2'-O-methyladenosine-3'-phosphate
  modified_base 20: mod_base = OTHER; note = 2'-O-methyladenosine-3'-phosphate
  modified_base 21: mod_base = OTHER; note = 2'-O-methylguanosine-3'-phosphorothioate
  modified_base 22: mod_base = OTHER; note = 2'-O-methyladenosine-3'-phosphorothioate
  modified_base 23: mod_base = OTHER; note = 2'-O-methyluridine
atatggatcaaggtactgaagat

SEQ ID NO: 451 - RNA, 23 nt, synthetic construct
  source 1..23: mol_type = other RNA
  modified_base 1: mod_base = OTHER; note = 2'-O-methyladenosine-3'-phosphorothioate
  modified_base 2: mod_base = OTHER; note = 2'-deoxy-2'-fluoroadenosine-3'-phosphorothioate
  modified_base 3: mod_base = OTHER; note = 2'-O-methyladenosine-3'-phosphate
  modified_base 4: mod_base = OTHER; note = 2'-O-methyladenosine-3'-phosphate
  modified_base 5: mod_base = OTHER; note = 2'-O-methylguanosine-3'-phosphate
  modified_base 6: mod_base = OTHER; note = 2'-deoxy-2'-fluorocytidine-3'-phosphate
  modified_base 7: mod_base = OTHER; note = 2'-O-methyluridine-3'-phosphate
  modified_base 8: mod_base = OTHER; note = 2'-deoxy-2'-fluorocytidine-3'-phosphate
  modified_base 9: mod_base = OTHER; note = 2'-deoxy-2'-fluorouridine-3'-phosphate
  modified_base 10: mod_base = OTHER; note = 2'-O-methyladenosine-3'-phosphate
  modified_base 11: mod_base = OTHER; note = 2'-O-methyluridine-3'-phosphate
  modified_base 12: mod_base = OTHER; note = 2'-O-methyladenosine-3'-phosphate
  modified_base 13: mod_base = OTHER; note = 2'-O-methylguanosine-3'-phosphate
  modified_base 14: mod_base = OTHER; note = 2'-deoxy-2'-fluoroadenosine-3'-phosphate
  modified_base 15: mod_base = OTHER; note = 2'-O-methylguanosine-3'-phosphate
  modified_base 16: mod_base = OTHER; note = 2'-deoxy-2'-fluoroadenosine-3'-phosphate
  modified_base 17: mod_base = OTHER; note = 2'-O-methyladenosine-3'-phosphate
  modified_base 18: mod_base = OTHER; note = 2'-O-methylcytidine-3'-phosphate
  modified_base 19: mod_base = OTHER; note = 2'-O-methyladenosine-3'-phosphate
  modified_base 20: mod_base = OTHER; note = 2'-O-methyluridine-3'-phosphate
  modified_base 21: mod_base = OTHER; note = 2'-O-methylcytidine-3'-phosphorothioate
  modified_base 22: mod_base = OTHER; note = 2'-O-methyluridine-3'-phosphorothioate
  modified_base 23: mod_base = OTHER; note = 2'-O-methyluridine
aaaagctctatagagaacatctt

SEQ ID NO: 452 - RNA, 23 nt, synthetic construct
  source 1..23: mol_type = other RNA
  modified_base 1: mod_base = OTHER; note = 2'-O-methyladenosine-3'-phosphorothioate
  modified_base 2: mod_base = OTHER; note = 2'-deoxy-2'-fluoroadenosine-3'-phosphorothioate
  modified_base 3: mod_base = OTHER; note = 2'-O-methyladenosine-3'-phosphate
  modified_base 4: mod_base = OTHER; note = 2'-O-methylguanosine-3'-phosphate
  modified_base 5: mod_base = OTHER; note = 2'-O-methyluridine-3'-phosphate
  modified_base 6: mod_base = OTHER; note = 2'-deoxy-2'-fluoroadenosine-3'-phosphate
  modified_base 7: mod_base = OTHER; note = 2'-O-methyladenosine-3'-phosphate
  modified_base 8: mod_base = OTHER; note = 2'-deoxy-2'-fluorouridine-3'-phosphate
  modified_base 9: mod_base = OTHER; note = 2'-deoxy-2'-fluorouridine-3'-phosphate
  modified_base 10: mod_base = OTHER; note = 2'-O-methylcytidine-3'-phosphate
  modified_base 11: mod_base = OTHER; note = 2'-O-methyladenosine-3'-phosphate
  modified_base 12: mod_base = OTHER; note = 2'-O-methyladenosine-3'-phosphate
  modified_base 13: mod_base = OTHER; note = 2'-O-methylcytidine-3'-phosphate
  modified_base 14: mod_base = OTHER; note = 2'-deoxy-2'-fluorouridine-3'-phosphate
  modified_base 15: mod_base = OTHER; note = 2'-O-methyladenosine-3'-phosphate
  modified_base 16: mod_base = OTHER; note = 2'-deoxy-2'-fluorouridine-3'-phosphate
  modified_base 17: mod_base = OTHER; note = 2'-O-methyladenosine-3'-phosphate
  modified_base 18: mod_base = OTHER; note = 2'-O-methyluridine-3'-phosphate
  modified_base 19: mod_base = OTHER; note = 2'-O-methylguanosine-3'-phosphate
  modified_base 20: mod_base = OTHER; note = 2'-O-methylcytidine-3'-phosphate
  modified_base 21: mod_base = OTHER; note = 2'-O-methylcytidine-3'-phosphorothioate
  modified_base 22: mod_base = OTHER; note = 2'-O-methylcytidine-3'-phosphorothioate
  modified_base 23: mod_base = OTHER; note = 2'-O-methyladenosine
aaagtaattcaactatatgccca

SEQ ID NO: 453 - RNA, 23 nt, synthetic construct
  source 1..23: mol_type = other RNA
  modified_base 1: mod_base = OTHER; note = 2'-O-methyladenosine-3'-phosphorothioate
  modified_base 2: mod_base = OTHER; note = 2'-deoxy-2'-fluoroadenosine-3'-phosphorothioate
  modified_base 3: mod_base = OTHER; note = 2'-O-methyluridine-3'-phosphate
  modified_base 4: mod_base = OTHER; note = 2'-O-methyluridine-3'-phosphate
  modified_base 5: mod_base = OTHER; note = 2'-O-methylguanosine-3'-phosphate
  modified_base 6: mod_base = OTHER; note = 2'-deoxy-2'-fluoroguanosine-3'-phosphate
  modified_base 7: mod_base = OTHER; note = 2'-O-methyluridine-3'-phosphate
  modified_base 8: mod_base = OTHER; note = 2'-deoxy-2'-fluoroadenosine-3'-phosphate
  modified_base 9: mod_base = OTHER; note = 2'-deoxy-2'-fluoroguanosine-3'-phosphate
  modified_base 10: mod_base = OTHER; note = 2'-O-methyladenosine-3'-phosphate
  modified_base 11: mod_base = OTHER; note = 2'-O-methylcytidine-3'-phosphate
  modified_base 12: mod_base = OTHER; note = 2'-O-methyladenosine-3'-phosphate
  modified_base 13: mod_base = OTHER; note = 2'-O-methylguanosine-3'-phosphate
  modified_base 14: mod_base = OTHER; note = 2'-deoxy-2'-fluoroadenosine-3'-phosphate
  modified_base 15: mod_base = OTHER; note = 2'-O-methylguanosine-3'-phosphate
  modified_base 16: mod_base = OTHER; note = 2'-deoxy-2'-fluorouridine-3'-phosphate
  modified_base 17: mod_base = OTHER; note = 2'-O-methyladenosine-3'-phosphate
  modified_base 18: mod_base = OTHER; note = 2'-O-methyluridine-3'-phosphate
  modified_base 19: mod_base = OTHER; note = 2'-O-methylcytidine-3'-phosphate
  modified_base 20: mod_base = OTHER; note = 2'-O-methyluridine-3'-phosphate
  modified_base 21: mod_base = OTHER; note = 2'-O-methyladenosine-3'-phosphorothioate
  modified_base 22: mod_base = OTHER; note = 2'-O-methylcytidine-3'-phosphorothioate
  modified_base 23: mod_base = OTHER; note = 2'-O-methylcytidine
aattggtagacagagtatctacc

SEQ ID NO: 454 - RNA, 23 nt, synthetic construct
  source 1..23: mol_type = other RNA
  modified_base 1: mod_base = OTHER; note = 2'-O-methyladenosine-3'-phosphorothioate
  modified_base 2: mod_base = OTHER; note = 2'-deoxy-2'-fluoroguanosine-3'-phosphorothioate
  modified_base 3: mod_base = OTHER; note = 2'-O-methyluridine-3'-phosphate
  modified_base 4: mod_base = OTHER; note = 2'-O-methyladenosine-3'-phosphate
  modified_base 5: mod_base = OTHER; note = 2'-O-methyluridine-3'-phosphate
  modified_base 6: mod_base = OTHER; note = 2'-deoxy-2'-fluorouridine-3'-phosphate
  modified_base 7: mod_base = OTHER; note = 2'-O-methyladenosine-3'-phosphate
  modified_base 8: mod_base = OTHER; note = 2'-deoxy-2'-fluorouridine-3'-phosphate
  modified_base 9: mod_base = OTHER; note = 2'-deoxy-2'-fluorocytidine-3'-phosphate
  modified_base 10: mod_base = OTHER; note = 2'-O-methyladenosine-3'-phosphate
  modified_base 11: mod_base = OTHER; note = 2'-O-methyladenosine-3'-phosphate
  modified_base 12: mod_base = OTHER; note = 2'-O-methylguanosine-3'-phosphate
  modified_base 13: mod_base = OTHER; note = 2'-O-methyladenosine-3'-phosphate
  modified_base 14: mod_base = OTHER; note = 2'-deoxy-2'-fluorouridine-3'-phosphate
  modified_base 15: mod_base = OTHER; note = 2'-O-methylguanosine-3'-phosphate
  modified_base 16: mod_base = OTHER; note = 2'-deoxy-2'-fluorouridine-3'-phosphate
  modified_base 17: mod_base = OTHER; note = 2'-O-methylcytidine-3'-phosphate
  modified_base 18: mod_base = OTHER; note = 2'-O-methyluridine-3'-phosphate
  modified_base 19: mod_base = OTHER; note = 2'-O-methylguanosine-3'-phosphate
  modified_base 20: mod_base = OTHER; note = 2'-O-methylguanosine-3'-phosphate
  modified_base 21: mod_base = OTHER; note = 2'-O-methylguanosine-3'-phosphorothioate
  modified_base 22: mod_base = OTHER; note = 2'-O-methyladenosine-3'-phosphorothioate
  modified_base 23: mod_base = OTHER; note = 2'-O-methyluridine
agtattatcaagatgtctgggat

SEQ ID NO: 455 - RNA, 23 nt, synthetic construct
  source 1..23: mol_type = other RNA
  modified_base 1: mod_base = OTHER; note = 2'-O-methyladenosine-3'-phosphorothioate
  modified_base 2: mod_base = OTHER; note = 2'-deoxy-2'-fluoroadenosine-3'-phosphorothioate
  modified_base 3: mod_base = OTHER; note = 2'-O-methyluridine-3'-phosphate
  modified_base 4: mod_base = OTHER; note = 2'-O-methylcytidine-3'-phosphate
  modified_base 5: mod_base = OTHER; note = 2'-O-methyladenosine-3'-phosphate
  modified_base 6: mod_base = OTHER; note = 2'-deoxy-2'-fluorouridine-3'-phosphate
  modified_base 7: mod_base = OTHER; note = 2'-O-methyladenosine-3'-phosphate
  modified_base 8: mod_base = OTHER; note = 2'-deoxy-2'-fluoroguanosine-3'-phosphate
  modified_base 9: mod_base = OTHER; note = 2'-deoxy-2'-fluoroguanosine-3'-phosphate
  modified_base 10: mod_base = OTHER; note = 2'-O-methyladenosine-3'-phosphate
  modified_base 11: mod_base = OTHER; note = 2'-O-methylguanosine-3'-phosphate
  modified_base 12: mod_base = OTHER; note = 2'-O-methyladenosine-3'-phosphate
  modified_base 13: mod_base = OTHER; note = 2'-O-methyluridine-3'-phosphate
  modified_base 14: mod_base = OTHER; note = 2'-deoxy-2'-fluorouridine-3'-phosphate
  modified_base 15: mod_base = OTHER; note = 2'-O-methylcytidine-3'-phosphate
  modified_base 16: mod_base = OTHER; note = 2'-deoxy-2'-fluorocytidine-3'-phosphate
  modified_base 17: mod_base = OTHER; note = 2'-O-methyladenosine-3'-phosphate
  modified_base 18: mod_base = OTHER; note = 2'-O-methyladenosine-3'-phosphate
  modified_base 19: mod_base = OTHER; note = 2'-O-methylcytidine-3'-phosphate
  modified_base 20: mod_base = OTHER; note = 2'-O-methyladenosine-3'-phosphate
  modified_base 21: mod_base = OTHER; note = 2'-O-methylguanosine-3'-phosphorothioate
  modified_base 22: mod_base = OTHER; note = 2'-O-methylguanosine-3'-phosphorothioate
  modified_base 23: mod_base = OTHER; note = 2'-O-methyluridine
aatcataggagattccaacaggt

SEQ ID NO: 456 - RNA, 23 nt, synthetic construct
  source 1..23: mol_type = other RNA
  modified_base 1: mod_base = OTHER; note = 2'-O-methyladenosine-3'-phosphorothioate
  modified_base 2: mod_base = OTHER; note = 2'-deoxy-2'-fluorouridine-3'-phosphorothioate
  modified_base 3: mod_base = OTHER; note = 2'-O-methyluridine-3'-phosphate
  modified_base 4: mod_base = OTHER; note = 2'-O-methylcytidine-3'-phosphate
  modified_base 5: mod_base = OTHER; note = 2'-O-methyluridine-3'-phosphate
  modified_base 6: mod_base = OTHER; note = 2'-deoxy-2'-fluorouridine-3'-phosphate
  modified_base 7: mod_base = OTHER; note = 2'-O-methylcytidine-3'-phosphate
  modified_base 8: mod_base = OTHER; note = 2'-deoxy-2'-fluorouridine-3'-phosphate
  modified_base 9: mod_base = OTHER; note = 2'-deoxy-2'-fluorouridine-3'-phosphate
  modified_base 10: mod_base = OTHER; note = 2'-O-methyladenosine-3'-phosphate
  modified_base 11: mod_base = OTHER; note = 2'-O-methylguanosine-3'-phosphate
  modified_base 12: mod_base = OTHER; note = 2'-O-methylguanosine-3'-phosphate
  modified_base 13: mod_base = OTHER; note = 2'-O-methyluridine-3'-phosphate
  modified_base 14: mod_base = OTHER; note = 2'-deoxy-2'-fluorouridine-3'-phosphate
  modified_base 15: mod_base = OTHER; note = 2'-O-methyluridine-3'-phosphate
  modified_base 16: mod_base = OTHER; note = 2'-deoxy-2'-fluoroguanosine-3'-phosphate
  modified_base 17: mod_base = OTHER; note = 2'-O-methylcytidine-3'-phosphate
  modified_base 18: mod_base = OTHER; note = 2'-O-methylcytidine-3'-phosphate
  modified_base 19: mod_base = OTHER; note = 2'-O-methylcytidine-3'-phosphate
  modified_base 20: mod_base = OTHER; note = 2'-O-methyladenosine-3'-phosphate
  modified_base 21: mod_base = OTHER; note = 2'-O-methylguanosine-3'-phosphorothioate
  modified_base 22: mod_base = OTHER; note = 2'-O-methyluridine-3'-phosphorothioate
  modified_base 23: mod_base = OTHER; note = 2'-O-methyluridine
attcttcttaggtttgcccagtt

SEQ ID NO: 457 - RNA, 23 nt, synthetic construct
  source 1..23: mol_type = other RNA
  modified_base 1: mod_base = OTHER; note = 2'-O-methyladenosine-3'-phosphorothioate
  modified_base 2: mod_base = OTHER; note = 2'-deoxy-2'-fluorouridine-3'-phosphorothioate
  modified_base 3: mod_base = OTHER; note = 2'-O-methyluridine-3'-phosphate
  modified_base 4: mod_base = OTHER; note = 2'-O-methyluridine-3'-phosphate
  modified_base 5: mod_base = OTHER; note = 2'-O-methylcytidine-3'-phosphate
  modified_base 6: mod_base = OTHER; note = 2'-deoxy-2'-fluoroguanosine-3'-phosphate
  modified_base 7: mod_base = OTHER; note = 2'-O-methyluridine-3'-phosphate
  modified_base 8: mod_base = OTHER; note = 2'-deoxy-2'-fluoroadenosine-3'-phosphate
  modified_base 9: mod_base = OTHER; note = 2'-deoxy-2'-fluoroadenosine-3'-phosphate
  modified_base 10: mod_base = OTHER; note = 2'-O-methylcytidine-3'-phosphate
  modified_base 11: mod_base = OTHER; note = 2'-O-methyladenosine-3'-phosphate
  modified_base 12: mod_base = OTHER; note = 2'-O-methyluridine-3'-phosphate
  modified_base 13: mod_base = OTHER; note = 2'-O-methyluridine-3'-phosphate
  modified_base 14: mod_base = OTHER; note = 2'-deoxy-2'-fluorocytidine-3'-phosphate
  modified_base 15: mod_base = OTHER; note = 2'-O-methyluridine-3'-phosphate
  modified_base 16: mod_base = OTHER; note = 2'-deoxy-2'-fluoroadenosine-3'-phosphate
  modified_base 17: mod_base = OTHER; note = 2'-O-methyladenosine-3'-phosphate
  modified_base 18: mod_base = OTHER; note = 2'-O-methyluridine-3'-phosphate
  modified_base 19: mod_base = OTHER; note = 2'-O-methyladenosine-3'-phosphate
  modified_base 20: mod_base = OTHER; note = 2'-O-methyladenosine-3'-phosphate
  modified_base 21: mod_base = OTHER; note = 2'-O-methylcytidine-3'-phosphorothioate
  modified_base 22: mod_base = OTHER; note = 2'-O-methyladenosine-3'-phosphorothioate
  modified_base 23: mod_base = OTHER; note = 2'-O-methylcytidine
atttcgtaacattctaataacac

SEQ ID NO: 458 - RNA, 23 nt, synthetic construct
  source 1..23: mol_type = other RNA
  modified_base 1: mod_base = OTHER; note = 2'-O-methyladenosine-3'-phosphorothioate
  modified_base 2: mod_base = OTHER; note = 2'-deoxy-2'-fluorouridine-3'-phosphorothioate
  modified_base 3: mod_base = OTHER; note = 2'-O-methyluridine-3'-phosphate
  modified_base 4: mod_base = OTHER; note = 2'-O-methylcytidine-3'-phosphate
  modified_base 5: mod_base = OTHER; note = 2'-O-methylcytidine-3'-phosphate
  modified_base 6: mod_base = OTHER; note = 2'-deoxy-2'-fluorouridine-3'-phosphate
  modified_base 7: mod_base = OTHER; note = 2'-O-methyluridine-3'-phosphate
  modified_base 8: mod_base = OTHER; note = 2'-deoxy-2'-fluorouridine-3'-phosphate
  modified_base 9: mod_base = OTHER; note = 2'-deoxy-2'-fluoroadenosine-3'-phosphate
  modified_base 10: mod_base = OTHER; note = 2'-O-methyladenosine-3'-phosphate
  modified_base 11: mod_base = OTHER; note = 2'-O-methylguanosine-3'-phosphate
  modified_base 12: mod_base = OTHER; note = 2'-O-methylguanosine-3'-phosphate
  modified_base 13: mod_base = OTHER; note = 2'-O-methyladenosine-3'-phosphate
  modified_base 14: mod_base = OTHER; note = 2'-deoxy-2'-fluoroadenosine-3'-phosphate
  modified_base 15: mod_base = OTHER; note = 2'-O-methyladenosine-3'-phosphate
  modified_base 16: mod_base = OTHER; note = 2'-deoxy-2'-fluoroadenosine-3'-phosphate
  modified_base 17: mod_base = OTHER; note = 2'-O-methyluridine-3'-phosphate
  modified_base 18: mod_base = OTHER; note = 2'-O-methylguanosine-3'-phosphate
  modified_base 19: mod_base = OTHER; note = 2'-O-methylguanosine-3'-phosphate
  modified_base 20: mod_base = OTHER; note = 2'-O-methylcytidine-3'-phosphate
  modified_base 21: mod_base = OTHER; note = 2'-O-methyluridine-3'-phosphorothioate
  modified_base 22: mod_base = OTHER; note = 2'-O-methylguanosine-3'-phosphorothioate
  modified_base 23: mod_base = OTHER; note = 2'-O-methyluridine
attcctttaaggaaaatggctgt

SEQ ID NO: 459 - RNA, 23 nt, synthetic construct
  source 1..23: mol_type = other RNA
  modified_base 1: mod_base = OTHER; note = 2'-O-methyladenosine-3'-phosphorothioate
  modified_base 2: mod_base = OTHER; note = 2'-deoxy-2'-fluoroadenosine-3'-phosphorothioate
  modified_base 3: mod_base = OTHER; note = 2'-O-methylcytidine-3'-phosphate
  modified_base 4: mod_base = OTHER; note = 2'-O-methyluridine-3'-phosphate
  modified_base 5: mod_base = OTHER; note = 2'-O-methyluridine-3'-phosphate
  modified_base 6: mod_base = OTHER; note = 2'-deoxy-2'-fluorouridine-3'-phosphate
  modified_base 7: mod_base = OTHER; note = 2'-O-methylguanosine-3'-phosphate
  modified_base 8: mod_base = OTHER; note = 2'-deoxy-2'-fluoroguanosine-3'-phosphate
  modified_base 9: mod_base = OTHER; note = 2'-deoxy-2'-fluorocytidine-3'-phosphate
  modified_base 10: mod_base = OTHER; note = 2'-O-methyluridine-3'-phosphate
  modified_base 11: mod_base = OTHER; note = 2'-O-methyluridine-3'-phosphate
  modified_base 12: mod_base = OTHER; note = 2'-O-methyluridine-3'-phosphate
  modified_base 13: mod_base = OTHER; note = 2'-O-methylcytidine-3'-phosphate
  modified_base 14: mod_base = OTHER; note = 2'-deoxy-2'-fluorouridine-3'-phosphate
  modified_base 15: mod_base = OTHER; note = 2'-O-methyladenosine-3'-phosphate
  modified_base 16: mod_base = OTHER; note = 2'-deoxy-2'-fluoroadenosine-3'-phosphate
  modified_base 17: mod_base = OTHER; note = 2'-O-methyladenosine-3'-phosphate
  modified_base 18: mod_base = OTHER; note = 2'-O-methyluridine-3'-phosphate
  modified_base 19: mod_base = OTHER; note = 2'-O-methyladenosine-3'-phosphate
  modified_base 20: mod_base = OTHER; note = 2'-O-methyluridine-3'-phosphate
  modified_base 21: mod_base = OTHER; note = 2'-O-methyluridine-3'-phosphorothioate
  modified_base 22: mod_base = OTHER; note = 2'-O-methylcytidine-3'-phosphorothioate
  modified_base 23: mod_base = OTHER; note = 2'-O-methylcytidine
aactttggctttctaaatattcc

SEQ ID NO: 460 - RNA, 23 nt, synthetic construct
  source 1..23: mol_type = other RNA
  modified_base 1: mod_base = OTHER; note = 2'-O-methyladenosine-3'-phosphorothioate
  modified_base 2: mod_base = OTHER; note = 2'-deoxy-2'-fluorouridine-3'-phosphorothioate
  modified_base 3: mod_base = OTHER; note = 2'-O-methyluridine-3'-phosphate
  modified_base 4: mod_base = OTHER; note = 2'-O-methylguanosine-3'-phosphate
  modified_base 5: mod_base = OTHER; note = 2'-O-methyladenosine-3'-phosphate
  modified_base 6: mod_base = OTHER; note = 2'-deoxy-2'-fluoroadenosine-3'-phosphate
  modified_base 7: mod_base = OTHER; note = 2'-O-methylguanosine-3'-phosphate
  modified_base 8: mod_base = OTHER; note = 2'-deoxy-2'-fluoroguanosine-3'-phosphate
  modified_base 9: mod_base = OTHER; note = 2'-deoxy-2'-fluoroadenosine-3'-phosphate
  modified_base 10: mod_base = OTHER; note = 2'-O-methyladenosine-3'-phosphate
  modified_base 11: mod_base = OTHER; note = 2'-O-methylguanosine-3'-phosphate
  modified_base 12: mod_base = OTHER; note = 2'-O-methyluridine-3'-phosphate
  modified_base 13: mod_base = OTHER; note = 2'-O-methyladenosine-3'-phosphate
  modified_base 14: mod_base = OTHER; note = 2'-deoxy-2'-fluorouridine-3'-phosphate
  modified_base 15: mod_base = OTHER; note = 2'-O-methyladenosine-3'-phosphate
  modified_base 16: mod_base = OTHER; note = 2'-deoxy-2'-fluoroguanosine-3'-phosphate
  modified_base 17: mod_base = OTHER; note = 2'-O-methylcytidine-3'-phosphate
  modified_base 18: mod_base = OTHER; note = 2'-O-methyluridine-3'-phosphate
  modified_base 19: mod_base = OTHER; note = 2'-O-methylguanosine-3'-phosphate
  modified_base 20: mod_base = OTHER; note = 2'-O-methylguanosine-3'-phosphate
  modified_base 21: mod_base = OTHER; note = 2'-O-methyluridine-3'-phosphorothioate
  modified_base 22: mod_base = OTHER; note = 2'-O-methyladenosine-3'-phosphorothioate
  modified_base 23: mod_base = OTHER; note = 2'-O-methyladenosine
attgaaggaagtatagctggtaa

SEQ ID NO: 461 - RNA, 23 nt, synthetic construct
  source 1..23: mol_type = other RNA
  modified_base 1: mod_base = OTHER; note = 2'-O-methyladenosine-3'-phosphorothioate
  modified_base 2: mod_base = OTHER; note = 2'-deoxy-2'-fluorouridine-3'-phosphorothioate
  modified_base 3: mod_base = OTHER; note = 2'-O-methyluridine-3'-phosphate
  modified_base 4: mod_base = OTHER; note = 2'-O-methylguanosine-3'-phosphate
  modified_base 5: mod_base = OTHER; note = 2'-O-methylcytidine-3'-phosphate
  modified_base 6: mod_base = OTHER; note = 2'-deoxy-2'-fluoroadenosine-3'-phosphate
  modified_base 7: mod_base = OTHER; note = 2'-O-methyluridine-3'-phosphate
  modified_base 8: mod_base = OTHER; note = 2'-deoxy-2'-fluorouridine-3'-phosphate
  modified_base 9: mod_base = OTHER; note = 2'-deoxy-2'-fluorouridine-3'-phosphate
  modified_base 10: mod_base = OTHER; note = 2'-O-methylcytidine-3'-phosphate
  modified_base 11: mod_base = OTHER; note = 2'-O-methyluridine-3'-phosphate
  modified_base 12: mod_base = OTHER; note = 2'-O-methylguanosine-3'-phosphate
  modified_base 13: mod_base = OTHER; note = 2'-O-methylguanosine-3'-phosphate
  modified_base 14: mod_base = OTHER; note = 2'-deoxy-2'-fluoroadenosine-3'-phosphate
  modified_base 15: mod_base = OTHER; note = 2'-O-methylcytidine-3'-phosphate
  modified_base 16: mod_base = OTHER; note = 2'-deoxy-2'-fluorouridine-3'-phosphate
  modified_base 17: mod_base = OTHER; note = 2'-O-methylcytidine-3'-phosphate
  modified_base 18: mod_base = OTHER; note = 2'-O-methyladenosine-3'-phosphate
  modified_base 19: mod_base = OTHER; note = 2'-O-methyluridine-3'-phosphate
  modified_base 20: mod_base = OTHER; note = 2'-O-methyluridine-3'-phosphate
  modified_base 21: mod_base = OTHER; note = 2'-O-methyladenosine-3'-phosphorothioate
  modified_base 22: mod_base = OTHER; note = 2'-O-methyladenosine-3'-phosphorothioate
  modified_base 23: mod_base = OTHER; note = 2'-O-methyluridine
attgcatttctggactcattaat

SEQ ID NO: 462 - RNA, 23 nt, synthetic construct
  source 1..23: mol_type = other RNA
  modified_base 1: mod_base = OTHER; note = 2'-O-methyladenosine-3'-phosphorothioate
  modified_base 2: mod_base = OTHER; note = 2'-deoxy-2'-fluoroadenosine-3'-phosphorothioate
  modified_base 3: mod_base = OTHER; note = 2'-O-methylguanosine-3'-phosphate
  modified_base 4: mod_base = OTHER; note = 2'-O-methyladenosine-3'-phosphate
  modified_base 5: mod_base = OTHER; note = 2'-O-methyluridine-3'-phosphate
  modified_base 6: mod_base = OTHER; note = 2'-deoxy-2'-fluorouridine-3'-phosphate
  modified_base 7: mod_base = OTHER; note = 2'-O-methyluridine-3'-phosphate
  modified_base 8: mod_base = OTHER; note = 2'-deoxy-2'-fluoroguanosine-3'-phosphate
  modified_base 9: mod_base = OTHER; note = 2'-deoxy-2'-fluorocytidine-3'-phosphate
  modified_base 10: mod_base = OTHER; note = 2'-O-methyladenosine-3'-phosphate
  modified_base 11: mod_base = OTHER; note = 2'-O-methyladenosine-3'-phosphate
  modified_base 12: mod_base = OTHER; note = 2'-O-methyluridine-3'-phosphate
  modified_base 13: mod_base = OTHER; note = 2'-O-methylcytidine-3'-phosphate
  modified_base 14: mod_base = OTHER; note = 2'-deoxy-2'-fluoroadenosine-3'-phosphate
  modified_base 15: mod_base = OTHER; note = 2'-O-methyladenosine-3'-phosphate
  modified_base 16: mod_base = OTHER; note = 2'-deoxy-2'-fluorocytidine-3'-phosphate
  modified_base 17: mod_base = OTHER; note = 2'-O-methylcytidine-3'-phosphate
  modified_base 18: mod_base = OTHER; note = 2'-O-methyluridine-3'-phosphate
  modified_base 19: mod_base = OTHER; note = 2'-O-methylcytidine-3'-phosphate
  modified_base 20: mod_base = OTHER; note = 2'-O-methylcytidine-3'-phosphate
  modified_base 21: mod_base = OTHER; note = 2'-O-methyluridine-3'-phosphorothioate
  modified_base 22: mod_base = OTHER; note = 2'-O-methyluridine-3'-phosphorothioate
  modified_base 23: mod_base = OTHER; note = 2'-O-methylcytidine
aagatttgcaatcaacctccttc

SEQ ID NO: 463 - RNA, 23 nt, synthetic construct
  source 1..23: mol_type = other RNA
  modified_base 1: mod_base = OTHER; note = 2'-O-methyladenosine-3'-phosphorothioate
  modified_base 2: mod_base = OTHER; note = 2'-deoxy-2'-fluorouridine-3'-phosphorothioate
  modified_base 3: mod_base = OTHER; note = 2'-O-methyluridine-3'-phosphate
  modified_base 4: mod_base = OTHER; note = 2'-O-methylcytidine-3'-phosphate
  modified_base 5: mod_base = OTHER; note = 2'-O-methyladenosine-3'-phosphate
  modified_base 6: mod_base = OTHER; note = 2'-deoxy-2'-fluorouridine-3'-phosphate
  modified_base 7: mod_base = OTHER; note = 2'-O-methylcytidine-3'-phosphate
  modified_base 8: mod_base = OTHER; note = 2'-deoxy-2'-fluoroadenosine-3'-phosphate
  modified_base 9: mod_base = OTHER; note = 2'-deoxy-2'-fluorocytidine-3'-phosphate
  modified_base 10: mod_base = OTHER; note = 2'-O-methyladenosine-3'-phosphate
  modified_base 11: mod_base = OTHER; note = 2'-O-methyladenosine-3'-phosphate
  modified_base 12: mod_base = OTHER; note = 2'-O-methyladenosine-3'-phosphate
  modified_base 13: mod_base = OTHER; note = 2'-O-methylguanosine-3'-phosphate
  modified_base 14: mod_base = OTHER; note = 2'-deoxy-2'-fluoroadenosine-3'-phosphate
  modified_base 15: mod_base = OTHER; note = 2'-O-methyladenosine-3'-phosphate
  modified_base 16: mod_base = OTHER; note = 2'-deoxy-2'-fluoroguanosine-3'-phosphate
  modified_base 17: mod_base = OTHER; note = 2'-O-methyluridine-3'-phosphate
  modified_base 18: mod_base = OTHER; note = 2'-O-methylcytidine-3'-phosphate
  modified_base 19: mod_base = OTHER; note = 2'-O-methyluridine-3'-phosphate
  modified_base 20: mod_base = OTHER; note = 2'-O-methyluridine-3'-phosphate
  modified_base 21: mod_base = OTHER; note = 2'-O-methylcytidine-3'-phosphorothioate
  modified_base 22: mod_base = OTHER; note = 2'-O-methylguanosine-3'-phosphorothioate
  modified_base 23: mod_base = OTHER; note = 2'-O-methyladenosine
attcatcacaaagaagtcttcga

SEQ ID NO: 464 - RNA, 23 nt, synthetic construct
  source 1..23: mol_type = other RNA
  modified_base 1: mod_base = OTHER; note = 2'-O-methyladenosine-3'-phosphorothioate
  modified_base 2: mod_base = OTHER; note = 2'-deoxy-2'-fluoroadenosine-3'-phosphorothioate
  modified_base 3: mod_base = OTHER; note = 2'-O-methyluridine-3'-phosphate
  modified_base 4: mod_base = OTHER; note = 2'-O-methyluridine-3'-phosphate
  modified_base 5: mod_base = OTHER; note = 2'-O-methyladenosine-3'-phosphate
  modified_base 6: mod_base = OTHER; note = 2'-deoxy-2'-fluorocytidine-3'-phosphate
  modified_base 7: mod_base = OTHER; note = 2'-O-methyluridine-3'-phosphate
  modified_base 8: mod_base = OTHER; note = 2'-deoxy-2'-fluoroadenosine-3'-phosphate
  modified_base 9: mod_base = OTHER; note = 2'-deoxy-2'-fluorocytidine-3'-phosphate
  modified_base 10: mod_base = OTHER; note = 2'-O-methyladenosine-3'-phosphate
  modified_base 11: mod_base = OTHER; note = 2'-O-methyluridine-3'-phosphate
  modified_base 12: mod_base = OTHER; note = 2'-O-methylcytidine-3'-phosphate
  modified_base 13: mod_base = OTHER; note = 2'-O-methyluridine-3'-phosphate
  modified_base 14: mod_base = OTHER; note = 2'-deoxy-2'-fluorouridine-3'-phosphate
  modified_base 15: mod_base = OTHER; note = 2'-O-methylcytidine-3'-phosphate
  modified_base 16: mod_base = OTHER; note = 2'-deoxy-2'-fluorouridine-3'-phosphate
  modified_base 17: mod_base = OTHER; note = 2'-O-methylguanosine-3'-phosphate
  modified_base 18: mod_base = OTHER; note = 2'-O-methyladenosine-3'-phosphate
  modified_base 19: mod_base = OTHER; note = 2'-O-methyladenosine-3'-phosphate
  modified_base 20: mod_base = OTHER; note = 2'-O-methyluridine-3'-phosphate
  modified_base 21: mod_base = OTHER; note = 2'-O-methyluridine-3'-phosphorothioate
  modified_base 22: mod_base = OTHER; note = 2'-O-methyluridine-3'-phosphorothioate
  modified_base 23: mod_base = OTHER; note = 2'-O-methylcytidine
aattactacatcttctgaatttc

SEQ ID NO: 465 - RNA, 23 nt, synthetic construct
  source 1..23: mol_type = other RNA
  modified_base 1: mod_base = OTHER; note = 2'-O-methyladenosine-3'-phosphorothioate
  modified_base 2: mod_base = OTHER; note = 2'-deoxy-2'-fluoroadenosine-3'-phosphorothioate
  modified_base 3: mod_base = OTHER; note = 2'-O-methylguanosine-3'-phosphate
  modified_base 4: mod_base = OTHER; note = 2'-O-methyladenosine-3'-phosphate
  modified_base 5: mod_base = OTHER; note = 2'-O-methyladenosine-3'-phosphate
  modified_base 6: mod_base = OTHER; note = 2'-deoxy-2'-fluoroguanosine-3'-phosphate
  modified_base 7: mod_base = OTHER; note = 2'-O-methyluridine-3'-phosphate
  modified_base 8: mod_base = OTHER; note = 2'-deoxy-2'-fluorouridine-3'-phosphate
  modified_base 9: mod_base = OTHER; note = 2'-deoxy-2'-fluoroguanosine-3'-phosphate
  modified_base 10: mod_base = OTHER; note = 2'-O-methyladenosine-3'-phosphate
  modified_base 11: mod_base = OTHER; note = 2'-O-methylguanosine-3'-phosphate
  modified_base 12: mod_base = OTHER; note = 2'-O-methyluridine-3'-phosphate
  modified_base 13: mod_base = OTHER; note = 2'-O-methyluridine-3'-phosphate
  modified_base 14: mod_base = OTHER; note = 2'-deoxy-2'-fluorocytidine-3'-phosphate
  modified_base 15: mod_base = OTHER; note = 2'-O-methylguanosine-3'-phosphate
  modified_base 16: mod_base = OTHER; note = 2'-deoxy-2'-fluoroadenosine-3'-phosphate
  modified_base 17: mod_base = OTHER; note = 2'-O-methyladenosine-3'-phosphate
  modified_base 18: mod_base = OTHER; note = 2'-O-methylguanosine-3'-phosphate
  modified_base 19: mod_base = OTHER; note = 2'-O-methyladenosine-3'-phosphate
  modified_base 20: mod_base = OTHER; note = 2'-O-methylcytidine-3'-phosphate
  modified_base 21: mod_base = OTHER; note = 2'-O-methyluridine-3'-phosphorothioate
  modified_base 22: mod_base = OTHER; note = 2'-O-methylguanosine-3'-phosphorothioate
  modified_base 23: mod_base = OTHER; note = 2'-O-methyladenosine
aagaagttgagttcgaagactga

SEQ ID NO: 466 - RNA, 23 nt, synthetic construct
  source 1..23: mol_type = other RNA
  modified_base 1: mod_base = OTHER; note = 2'-O-methyladenosine-3'-phosphorothioate
  modified_base 2: mod_base = OTHER; note = 2'-deoxy-2'-fluorocytidine-3'-phosphorothioate
  modified_base 3: mod_base = OTHER; note = 2'-O-methyladenosine-3'-phosphate
  modified_base 4: mod_base = OTHER; note = 2'-O-methyluridine-3'-phosphate
  modified_base 5: mod_base = OTHER; note = 2'-O-methylguanosine-3'-phosphate
  modified_base 6: mod_base = OTHER; note = 2'-deoxy-2'-fluoroadenosine-3'-phosphate
  modified_base 7: mod_base = OTHER; note = 2'-O-methyluridine-3'-phosphate
  modified_base 8: mod_base = OTHER; note = 2'-deoxy-2'-fluoroadenosine-3'-phosphate
  modified_base 9: mod_base = OTHER; note = 2'-deoxy-2'-fluoroadenosine-3'-phosphate
  modified_base 10: mod_base = OTHER; note = 2'-O-methyladenosine-3'-phosphate
  modified_base 11: mod_base = OTHER; note = 2'-O-methylguanosine-3'-phosphate
  modified_base 12: mod_base = OTHER; note = 2'-O-methyladenosine-3'-phosphate
  modified_base 13: mod_base = OTHER; note = 2'-O-methylcytidine-3'-phosphate
  modified_base 14: mod_base = OTHER; note = 2'-deoxy-2'-fluoroadenosine-3'-phosphate
  modified_base 15: mod_base = OTHER; note = 2'-O-methyluridine-3'-phosphate
  modified_base 16: mod_base = OTHER; note = 2'-deoxy-2'-fluoroguanosine-3'-phosphate
  modified_base 17: mod_base = OTHER; note = 2'-O-methyladenosine-3'-phosphate
  modified_base 18: mod_base = OTHER; note = 2'-O-methyladenosine-3'-phosphate
  modified_base 19: mod_base = OTHER; note = 2'-O-methylguanosine-3'-phosphate
  modified_base 20: mod_base = OTHER; note = 2'-O-methyluridine-3'-phosphate
  modified_base 21: mod_base = OTHER; note = 2'-O-methyladenosine-3'-phosphorothioate
  modified_base 22: mod_base = OTHER; note = 2'-O-methylcytidine-3'-phosphorothioate
  modified_base 23: mod_base = OTHER; note = 2'-O-methylcytidine
acatgataaagacatgaagtacc

SEQ ID NO: 467 - RNA, 23 nt, synthetic construct
  source 1..23: mol_type = other RNA
  modified_base 1: mod_base = OTHER; note = 2'-O-methyladenosine-3'-phosphorothioate
  modified_base 2: mod_base = OTHER; note = 2'-deoxy-2'-fluorouridine-3'-phosphorothioate
  modified_base 3: mod_base = OTHER; note = 2'-O-methylcytidine-3'-phosphate
  modified_base 4: mod_base = OTHER; note = 2'-O-methyluridine-3'-phosphate
  modified_base 5: mod_base = OTHER; note = 2'-O-methyluridine-3'-phosphate
  modified_base 6: mod_base = OTHER; note = 2'-deoxy-2'-fluoroguanosine-3'-phosphate
  modified_base 7: mod_base = OTHER; note = 2'-O-methyluridine-3'-phosphate
  modified_base 8: mod_base = OTHER; note = 2'-deoxy-2'-fluorouridine-3'-phosphate
  modified_base 9: mod_base = OTHER; note = 2'-deoxy-2'-fluorocytidine-3'-phosphate
  modified_base 10: mod_base = OTHER; note = 2'-O-methyladenosine-3'-phosphate
  modified_base 11: mod_base = OTHER; note = 2'-O-methylguanosine-3'-phosphate
  modified_base 12: mod_base = OTHER; note = 2'-O-methyladenosine-3'-phosphate
  modified_base 13: mod_base = OTHER; note = 2'-O-methyladenosine-3'-phosphate
  modified_base 14: mod_base = OTHER; note = 2'-deoxy-2'-fluorocytidine-3'-phosphate
  modified_base 15: mod_base = OTHER; note = 2'-O-methyluridine-3'-phosphate
  modified_base 16: mod_base = OTHER; note = 2'-deoxy-2'-fluoroguanosine-3'-phosphate
  modified_base 17: mod_base = OTHER; note = 2'-O-methylcytidine-3'-phosphate
  modified_base 18: mod_base = OTHER; note = 2'-O-methyladenosine-3'-phosphate
  modified_base 19: mod_base = OTHER; note = 2'-O-methyluridine-3'-phosphate
  modified_base 20: mod_base = OTHER; note = 2'-O-methyladenosine-3'-phosphate
  modified_base 21: mod_base = OTHER; note = 2'-O-methyladenosine-3'-phosphorothioate
  modified_base 22: mod_base = OTHER; note = 2'-O-methyladenosine-3'-phosphorothioate
  modified_base 23: mod_base = OTHER; note = 2'-O-methylguanosine
atcttgttcagaactgcataaag

SEQ ID NO: 468 - RNA, 23 nt, synthetic construct
  source 1..23: mol_type = other RNA
  modified_base 1: mod_base = OTHER; note = 2'-O-methyladenosine-3'-phosphorothioate
  modified_base 2: mod_base = OTHER; note = 2'-deoxy-2'-fluoroadenosine-3'-phosphorothioate
  modified_base 3: mod_base = OTHER; note = 2'-O-methyluridine-3'-phosphate
  modified_base 4: mod_base = OTHER; note = 2'-O-methyladenosine-3'-phosphate
  modified_base 5: mod_base = OTHER; note = 2'-O-methyladenosine-3'-phosphate
  modified_base 6: mod_base = OTHER; note = 2'-deoxy-2'-fluoroadenosine-3'-phosphate
  modified_base 7: mod_base = OTHER; note = 2'-O-methylcytidine-3'-phosphate
  modified_base 8: mod_base = OTHER; note = 2'-deoxy-2'-fluorouridine-3'-phosphate
  modified_base 9: mod_base = OTHER; note = 2'-deoxy-2'-fluorouridine-3'-phosphate
  modified_base 10: mod_base = OTHER; note = 2'-O-methyluridine-3'-phosphate
  modified_base 11: mod_base = OTHER; note = 2'-O-methylcytidine-3'-phosphate
  modified_base 12: mod_base = OTHER; note = 2'-O-methylcytidine-3'-phosphate
  modified_base 13: mod_base = OTHER; note = 2'-O-methyluridine-3'-phosphate
  modified_base 14: mod_base = OTHER; note = 2'-deoxy-2'-fluoroadenosine-3'-phosphate
  modified_base 15: mod_base = OTHER; note = 2'-O-methylcytidine-3'-phosphate
  modified_base 16: mod_base = OTHER; note = 2'-deoxy-2'-fluorouridine-3'-phosphate
  modified_base 17: mod_base = OTHER; note = 2'-O-methylguanosine-3'-phosphate
  modified_base 18: mod_base = OTHER; note = 2'-O-methyluridine-3'-phosphate
  modified_base 19: mod_base = OTHER; note = 2'-O-methyluridine-3'-phosphate
  modified_base 20: mod_base = OTHER; note = 2'-O-methyluridine-3'-phosphate
  modified_base 21: mod_base = OTHER; note = 2'-O-methylcytidine-3'-phosphorothioate
  modified_base 22: mod_base = OTHER; note = 2'-O-methyladenosine-3'-phosphorothioate
  modified_base 23: mod_base = OTHER; note = 2'-O-methyluridine
aataaactttcctactgtttcat

SEQ ID NO: 469 - RNA, 23 nt, synthetic construct
  source 1..23: mol_type = other RNA
  modified_base 1: mod_base = OTHER; note = 2'-O-methyladenosine-3'-phosphorothioate
  modified_base 2: mod_base = OTHER; note = 2'-deoxy-2'-fluorouridine-3'-phosphorothioate
  modified_base 3: mod_base = OTHER; note = 2'-O-methylcytidine-3'-phosphate
  modified_base 4: mod_base = OTHER; note = 2'-O-methyluridine-3'-phosphate
  modified_base 5: mod_base = OTHER; note = 2'-O-methyluridine-3'-phosphate
  modified_base 6: mod_base = OTHER; note = 2'-deoxy-2'-fluorocytidine-3'-phosphate
  modified_base 7: mod_base = OTHER; note = 2'-O-methyluridine-3'-phosphate
  modified_base 8: mod_base = OTHER; note = 2'-deoxy-2'-fluorouridine-3'-phosphate
  modified_base 9: mod_base = OTHER; note = 2'-deoxy-2'-fluorocytidine-3'-phosphate
  modified_base 10: mod_base = OTHER; note = 2'-O-methyladenosine-3'-phosphate
  modified_base 11: mod_base = OTHER; note = 2'-O-methyluridine-3'-phosphate
  modified_base 12: mod_base = OTHER; note = 2'-O-methylcytidine-3'-phosphate
  modified_base 13: mod_base = OTHER; note = 2'-O-methyladenosine-3'-phosphate
  modified_base 14: mod_base = OTHER; note = 2'-deoxy-2'-fluorocytidine-3'-phosphate
  modified_base 15: mod_base = OTHER; note = 2'-O-methyluridine-3'-phosphate
  modified_base 16: mod_base = OTHER; note = 2'-deoxy-2'-fluorouridine-3'-phosphate
  modified_base 17: mod_base = OTHER; note = 2'-O-methylcytidine-3'-phosphate
  modified_base 18: mod_base = OTHER; note = 2'-O-methyluridine-3'-phosphate
  modified_base 19: mod_base = OTHER; note = 2'-O-methylcytidine-3'-phosphate
  modified_base 20: mod_base = OTHER; note = 2'-O-methylcytidine-3'-phosphate
  modified_base 21: mod_base = OTHER; note = 2'-O-methyladenosine-3'-phosphorothioate
  modified_base 22: mod_base = OTHER; note = 2'-O-methyladenosine-3'-phosphorothioate
  modified_base 23: mod_base = OTHER; note = 2'-O-methylguanosine
atcttcttcatcacttctccaag

SEQ ID NO: 470 - RNA, 23 nt, synthetic construct
  source 1..23: mol_type = other RNA
  modified_base 1: mod_base = OTHER; note = 2'-O-methyladenosine-3'-phosphorothioate
  modified_base 2: mod_base = OTHER; note = 2'-deoxy-2'-fluorouridine-3'-phosphorothioate
  modified_base 3: mod_base = OTHER; note = 2'-O-methylcytidine-3'-phosphate
  modified_base 4: mod_base = OTHER; note = 2'-O-methyluridine-3'-phosphate
  modified_base 5: mod_base = OTHER; note = 2'-O-methylguanosine-3'-phosphate
  modified_base 6: mod_base = OTHER; note = 2'-deoxy-2'-fluorouridine-3'-phosphate
  modified_base 7: mod_base = OTHER; note = 2'-O-methyladenosine-3'-phosphate
  modified_base 8: mod_base = OTHER; note = 2'-deoxy-2'-fluoroadenosine-3'-phosphate
  modified_base 9: mod_base = OTHER; note = 2'-deoxy-2'-fluoroguanosine-3'-phosphate
  modified_base 10: mod_base = OTHER; note = 2'-O-methyladenosine-3'-phosphate
  modified_base 11: mod_base = OTHER; note = 2'-O-methyladenosine-3'-phosphate
  modified_base 12: mod_base = OTHER; note = 2'-O-methylguanosine-3'-phosphate
  modified_base 13: mod_base = OTHER; note = 2'-O-methylguanosine-3'-phosphate
  modified_base 14: mod_base = OTHER; note = 2'-deoxy-2'-fluorouridine-3'-phosphate
  modified_base 15: mod_base = OTHER; note = 2'-O-methylguanosine-3'-phosphate
  modified_base 16: mod_base = OTHER; note = 2'-deoxy-2'-fluoroadenosine-3'-phosphate
  modified_base 17: mod_base = OTHER; note = 2'-O-methyluridine-3'-phosphate
  modified_base 18: mod_base = OTHER; note = 2'-O-methyladenosine-3'-phosphate
  modified_base 19: mod_base = OTHER; note = 2'-O-methyladenosine-3'-phosphate
  modified_base 20: mod_base = OTHER; note = 2'-O-methyladenosine-3'-phosphate
  modified_base 21: mod_base = OTHER; note = 2'-O-methylcytidine-3'-phosphorothioate
  modified_base 22: mod_base = OTHER; note = 2'-O-methyluridine-3'-phosphorothioate
  modified_base 23: mod_base = OTHER; note = 2'-O-methylguanosine
atctgtaagaaggtgataaactg

SEQ ID NO: 471 - RNA, 23 nt, synthetic construct
  source 1..23: mol_type = other RNA
  modified_base 1: mod_base = OTHER; note = 2'-O-methyladenosine-3'-phosphorothioate
  modified_base 2: mod_base = OTHER; note = 2'-deoxy-2'-fluorouridine-3'-phosphorothioate
  modified_base 3: mod_base = OTHER; note = 2'-O-methyluridine-3'-phosphate
  modified_base 4: mod_base = OTHER; note = 2'-O-methyluridine-3'-phosphate
  modified_base 5: mod_base = OTHER; note = 2'-O-methyluridine-3'-phosphate
  modified_base 6: mod_base = OTHER; note = 2'-deoxy-2'-fluoroguanosine-3'-phosphate
  modified_base 7: mod_base = OTHER; note = 2'-O-methylcytidine-3'-phosphate
  modified_base 8: mod_base = OTHER; note = 2'-deoxy-2'-fluoroadenosine-3'-phosphate
  modified_base 9: mod_base = OTHER; note = 2'-deoxy-2'-fluoroguanosine-3'-phosphate
  modified_base 10: mod_base = OTHER; note = 2'-O-methyladenosine-3'-phosphate
  modified_base 11: mod_base = OTHER; note = 2'-O-methyluridine-3'-phosphate
  modified_base 12: mod_base = OTHER; note = 2'-O-methyladenosine-3'-phosphate
  modified_base 13: mod_base = OTHER; note = 2'-O-methylcytidine-3'-phosphate
  modified_base 14: mod_base = OTHER; note = 2'-deoxy-2'-fluorouridine-3'-phosphate
  modified_base 15: mod_base = OTHER; note = 2'-O-methylcytidine-3'-phosphate
  modified_base 16: mod_base = OTHER; note = 2'-deoxy-2'-fluoroadenosine-3'-phosphate
  modified_base 17: mod_base = OTHER; note = 2'-O-methylguanosine-3'-phosphate
  modified_base 18: mod_base = OTHER; note = 2'-O-methylguanosine-3'-phosphate
  modified_base 19: mod_base = OTHER; note = 2'-O-methyluridine-3'-phosphate
  modified_base 20: mod_base = OTHER; note = 2'-O-methyluridine-3'-phosphate
  modified_base 21: mod_base = OTHER; note = 2'-O-methylcytidine-3'-phosphorothioate
  modified_base 22: mod_base = OTHER; note = 2'-O-methyluridine-3'-phosphorothioate
  modified_base 23: mod_base = OTHER; note = 2'-O-methylguanosine
attttgcagatactcaggttctg

SEQ ID NO: 472 - RNA, 23 nt, synthetic construct
  source 1..23: mol_type = other RNA
  modified_base 1: mod_base = OTHER; note = 2'-O-methyladenosine-3'-phosphorothioate
  modified_base 2: mod_base = OTHER; note = 2'-deoxy-2'-fluorouridine-3'-phosphorothioate
  modified_base 3: mod_base = OTHER; note = 2'-O-methyluridine-3'-phosphate
  modified_base 4: mod_base = OTHER; note = 2'-O-methyladenosine-3'-phosphate
  modified_base 5: mod_base = OTHER; note = 2'-O-methyluridine-3'-phosphate
  modified_base 6: mod_base = OTHER; note = 2'-deoxy-2'-fluorouridine-3'-phosphate
  modified_base 7: mod_base = OTHER; note = 2'-O-methyladenosine-3'-phosphate
  modified_base 8: mod_base = OTHER; note = 2'-deoxy-2'-fluoroguanosine-3'-phosphate
  modified_base 9: mod_base = OTHER; note = 2'-deoxy-2'-fluoroguanosine-3'-phosphate
  modified_base 10: mod_base = OTHER; note = 2'-O-methyluridine-3'-phosphate
  modified_base 11: mod_base = OTHER; note = 2'-O-methyladenosine-3'-phosphate
  modified_base 12: mod_base = OTHER; note = 2'-O-methyluridine-3'-phosphate
  modified_base 13: mod_base = OTHER; note = 2'-O-methyluridine-3'-phosphate
  modified_base 14: mod_base = OTHER; note = 2'-deoxy-2'-fluorouridine-3'-phosphate
  modified_base 15: mod_base = OTHER; note = 2'-O-methylguanosine-3'-phosphate
  modified_base 16: mod_base = OTHER; note = 2'-deoxy-2'-fluorouridine-3'-phosphate
  modified_base 17: mod_base = OTHER; note = 2'-O-methylguanosine-3'-phosphate
  modified_base 18: mod_base = OTHER; note = 2'-O-methylcytidine-3'-phosphate
  modified_base 19: mod_base = OTHER; note = 2'-O-methyladenosine-3'-phosphate
  modified_base 20: mod_base = OTHER; note = 2'-O-methyladenosine-3'-phosphate
  modified_base 21: mod_base = OTHER; note = 2'-O-methylcytidine-3'-phosphorothioate
  modified_base 22: mod_base = OTHER; note = 2'-O-methyluridine-3'-phosphorothioate
  modified_base 23: mod_base = OTHER; note = 2'-O-methyluridine
attattaggtatttgtgcaactt

SEQ ID NO: 473 - RNA, 23 nt, synthetic construct
  source 1..23: mol_type = other RNA
  modified_base 1: mod_base = OTHER; note = 2'-O-methyladenosine-3'-phosphorothioate
  modified_base 2: mod_base = OTHER; note = 2'-deoxy-2'-fluoroadenosine-3'-phosphorothioate
  modified_base 3: mod_base = OTHER; note = 2'-O-methyluridine-3'-phosphate
  modified_base 4: mod_base = OTHER; note = 2'-O-methyluridine-3'-phosphate
  modified_base 5: mod_base = OTHER; note = 2'-O-methyluridine-3'-phosphate
  modified_base 6: mod_base = OTHER; note = 2'-deoxy-2'-fluorocytidine-3'-phosphate
  modified_base 7: mod_base = OTHER; note = 2'-O-methyluridine-3'-phosphate
  modified_base 8: mod_base = OTHER; note = 2'-deoxy-2'-fluorouridine-3'-phosphate
  modified_base 9: mod_base = OTHER; note = 2'-deoxy-2'-fluorouridine-3'-phosphate
  modified_base 10: mod_base = OTHER; note = 2'-O-methylcytidine-3'-phosphate
  modified_base 11: mod_base = OTHER; note = 2'-O-methyluridine-3'-phosphate
  modified_base 12: mod_base = OTHER; note = 2'-O-methylguanosine-3'-phosphate
  modified_base 13: mod_base = OTHER; note = 2'-O-methyluridine-3'-phosphate
  modified_base 14: mod_base = OTHER; note = 2'-deoxy-2'-fluorouridine-3'-phosphate
  modified_base 15: mod_base = OTHER; note = 2'-O-methylcytidine-3'-phosphate
  modified_base 16: mod_base = OTHER; note = 2'-deoxy-2'-fluorouridine-3'-phosphate
  modified_base 17: mod_base = OTHER; note = 2'-O-methylguanosine-3'-phosphate
  modified_base 18: mod_base = OTHER; note = 2'-O-methylguanosine-3'-phosphate
  modified_base 19: mod_base = OTHER; note = 2'-O-methyluridine-3'-phosphate
  modified_base 20: mod_base = OTHER; note = 2'-O-methyluridine-3'-phosphate
  modified_base 21: mod_base = OTHER; note = 2'-O-methyladenosine-3'-phosphorothioate
  modified_base 22: mod_base = OTHER; note = 2'-O-methyluridine-3'-phosphorothioate
  modified_base 23: mod_base = OTHER; note = 2'-O-methyluridine
aatttctttctgttctggttatt

SEQ ID NO: 474 - RNA, 23 nt, synthetic construct
  source 1..23: mol_type = other RNA
  modified_base 1: mod_base = OTHER; note = 2'-O-methyladenosine-3'-phosphorothioate
  modified_base 2: mod_base = OTHER; note = 2'-deoxy-2'-fluoroadenosine-3'-phosphorothioate
  modified_base 3: mod_base = OTHER; note = 2'-O-methyluridine-3'-phosphate
  modified_base 4: mod_base = OTHER; note = 2'-O-methyluridine-3'-phosphate
  modified_base 5: mod_base = OTHER; note = 2'-O-methylcytidine-3'-phosphate
  modified_base 6: mod_base = OTHER; note = 2'-deoxy-2'-fluorouridine-3'-phosphate
  modified_base 7: mod_base = OTHER; note = 2'-O-methyluridine-3'-phosphate
  modified_base 8: mod_base = OTHER; note = 2'-deoxy-2'-fluorocytidine-3'-phosphate
  modified_base 9: mod_base = OTHER; note = 2'-deoxy-2'-fluoroadenosine-3'-phosphate
  modified_base 10: mod_base = OTHER; note = 2'-O-methylcytidine-3'-phosphate
  modified_base 11: mod_base = OTHER; note = 2'-O-methyladenosine-3'-phosphate
  modified_base 12: mod_base = OTHER; note = 2'-O-methyladenosine-3'-phosphate
  modified_base 13: mod_base = OTHER; note = 2'-O-methylguanosine-3'-phosphate
  modified_base 14: mod_base = OTHER; note = 2'-deoxy-2'-fluoroadenosine-3'-phosphate
  modified_base 15: mod_base = OTHER; note = 2'-O-methylcytidine-3'-phosphate
  modified_base 16: mod_base = OTHER; note = 2'-deoxy-2'-fluoroadenosine-3'-phosphate
  modified_base 17: mod_base = OTHER; note = 2'-O-methyladenosine-3'-phosphate
  modified_base 18: mod_base = OTHER; note = 2'-O-methyluridine-3'-phosphate
  modified_base 19: mod_base = OTHER; note = 2'-O-methyladenosine-3'-phosphate
  modified_base 20: mod_base = OTHER; note = 2'-O-methyluridine-3'-phosphate
  modified_base 21: mod_base = OTHER; note = 2'-O-methylguanosine-3'-phosphorothioate
  modified_base 22: mod_base = OTHER; note = 2'-O-methyluridine-3'-phosphorothioate
  modified_base 23: mod_base = OTHER; note = 2'-O-methylguanosine
aattcttcacaagacaatatgtg

SEQ ID NO: 475 - RNA, 23 nt, synthetic construct
  source 1..23: mol_type = other RNA
  modified_base 1: mod_base = OTHER; note = 2'-O-methyladenosine-3'-phosphorothioate
  modified_base 2: mod_base = OTHER; note = 2'-deoxy-2'-fluorouridine-3'-phosphorothioate
  modified_base 3: mod_base = OTHER; note = 2'-O-methyluridine-3'-phosphate
  modified_base 4: mod_base = OTHER; note = 2'-O-methyladenosine-3'-phosphate
  modified_base 5: mod_base = OTHER; note = 2'-O-methyladenosine-3'-phosphate
  modified_base 6: mod_base = OTHER; note = 2'-deoxy-2'-fluoroadenosine-3'-phosphate
  modified_base 7: mod_base = OTHER; note = 2'-O-methylcytidine-3'-phosphate
  modified_base 8: mod_base = OTHER; note = 2'-deoxy-2'-fluoroadenosine-3'-phosphate
  modified_base 9: mod_base = OTHER; note = 2'-deoxy-2'-fluorouridine-3'-phosphate
  modified_base 10: mod_base = OTHER; note = 2'-O-methyluridine-3'-phosphate
  modified_base 11: mod_base = OTHER; note = 2'-O-methyluridine-3'-phosphate
  modified_base 12: mod_base = OTHER; note = 2'-O-methyluridine-3'-phosphate
  modified_base 13: mod_base = OTHER; note = 2'-O-methylcytidine-3'-phosphate
  modified_base 14: mod_base = OTHER; note = 2'-deoxy-2'-fluoroadenosine-3'-phosphate
  modified_base 15: mod_base = OTHER; note = 2'-O-methylcytidine-3'-phosphate
  modified_base 16: mod_base = OTHER; note = 2'-deoxy-2'-fluoroadenosine-3'-phosphate
  modified_base 17: mod_base = OTHER; note = 2'-O-methylguanosine-3'-phosphate
  modified_base 18: mod_base = OTHER; note = 2'-O-methylcytidine-3'-phosphate
  modified_base 19: mod_base = OTHER; note = 2'-O-methyladenosine-3'-phosphate
  modified_base 20: mod_base = OTHER; note = 2'-O-methyluridine-3'-phosphate
  modified_base 21: mod_base = OTHER; note = 2'-O-methyluridine-3'-phosphorothioate
  modified_base 22: mod_base = OTHER; note = 2'-O-methylcytidine-3'-phosphorothioate
  modified_base 23: mod_base = OTHER; note = 2'-O-methyluridine
attaaacattttcacagcattct

SEQ ID NO: 476 - RNA, 23 nt, synthetic construct
  source 1..23: mol_type = other RNA
  modified_base 1: mod_base = OTHER; note = 2'-O-methyladenosine-3'-phosphorothioate
  modified_base 2: mod_base = OTHER; note = 2'-deoxy-2'-fluoroadenosine-3'-phosphorothioate
  modified_base 3: mod_base = OTHER; note = 2'-O-methylguanosine-3'-phosphate
  modified_base 4: mod_base = OTHER; note = 2'-O-methyluridine-3'-phosphate
  modified_base 5: mod_base = OTHER; note = 2'-O-methyluridine-3'-phosphate
  modified_base 6: mod_base = OTHER; note = 2'-deoxy-2'-fluorocytidine-3'-phosphate
  modified_base 7: mod_base = OTHER; note = 2'-O-methyluridine-3'-phosphate
  modified_base 8: mod_base = OTHER; note = 2'-deoxy-2'-fluoroadenosine-3'-phosphate
  modified_base 9: mod_base = OTHER; note = 2'-deoxy-2'-fluoroadenosine-3'-phosphate
  modified_base 10: mod_base = OTHER; note = 2'-O-methyladenosine-3'-phosphate
  modified_base 11: mod_base = OTHER; note = 2'-O-methyladenosine-3'-phosphate
  modified_base 12: mod_base = OTHER; note = 2'-O-methylcytidine-3'-phosphate
  modified_base 13: mod_base = OTHER; note = 2'-O-methyladenosine-3'-phosphate
  modified_base 14: mod_base = OTHER; note = 2'-deoxy-2'-fluoroguanosine-3'-phosphate
  modified_base 15: mod_base = OTHER; note = 2'-O-methyladenosine-3'-phosphate
  modified_base 16: mod_base = OTHER; note = 2'-deoxy-2'-fluorocytidine-3'-phosphate
  modified_base 17: mod_base = OTHER; note = 2'-O-methyladenosine-3'-phosphate
  modified_base 18: mod_base = OTHER; note = 2'-O-methylcytidine-3'-phosphate
  modified_base 19: mod_base = OTHER; note = 2'-O-methyluridine-3'-phosphate
  modified_base 20: mod_base = OTHER; note = 2'-O-methylcytidine-3'-phosphate
  modified_base 21: mod_base = OTHER; note = 2'-O-methyluridine-3'-phosphorothioate
  modified_base 22: mod_base = OTHER; note = 2'-O-methylcytidine-3'-phosphorothioate
  modified_base 23: mod_base = OTHER; note = 2'-O-methyluridine
aagttctaaaacagacactctct

SEQ ID NO: 477 - RNA, 23 nt, synthetic construct
  source 1..23: mol_type = other RNA
  modified_base 1: mod_base = OTHER; note = 2'-O-methyladenosine-3'-phosphorothioate
  modified_base 2: mod_base = OTHER; note = 2'-deoxy-2'-fluoroadenosine-3'-phosphorothioate
  modified_base 3: mod_base = OTHER; note = 2'-O-methylcytidine-3'-phosphate
  modified_base 4: mod_base = OTHER; note = 2'-O-methylcytidine-3'-phosphate
  modified_base 5: mod_base = OTHER; note = 2'-O-methyladenosine-3'-phosphate
  modified_base 6: mod_base = OTHER; note = 2'-deoxy-2'-fluorocytidine-3'-phosphate
  modified_base 7: mod_base = OTHER; note = 2'-O-methyladenosine-3'-phosphate
  modified_base 8: mod_base = OTHER; note = 2'-deoxy-2'-fluoroadenosine-3'-phosphate
  modified_base 9: mod_base = OTHER; note = 2'-deoxy-2'-fluoroadenosine-3'-phosphate
  modified_base 10: mod_base = OTHER; note = 2'-O-methyladenosine-3'-phosphate
  modified_base 11: mod_base = OTHER; note = 2'-O-methylcytidine-3'-phosphate
  modified_base 12: mod_base = OTHER; note = 2'-O-methyluridine-3'-phosphate
  modified_base 13: mod_base = OTHER; note = 2'-O-methylcytidine-3'-phosphate
  modified_base 14: mod_base = OTHER; note = 2'-deoxy-2'-fluoroadenosine-3'-phosphate
  modified_base 15: mod_base = OTHER; note = 2'-O-methylguanosine-3'-phosphate
  modified_base 16: mod_base = OTHER; note = 2'-deoxy-2'-fluoroadenosine-3'-phosphate
  modified_base 17: mod_base = OTHER; note = 2'-O-methyladenosine-3'-phosphate
  modified_base 18: mod_base = OTHER; note = 2'-O-methyluridine-3'-phosphate
  modified_base 19: mod_base = OTHER; note = 2'-O-methyladenosine-3'-phosphate
  modified_base 20: mod_base = OTHER; note = 2'-O-methyluridine-3'-phosphate
  modified_base 21: mod_base = OTHER; note = 2'-O-methyladenosine-3'-phosphorothioate
  modified_base 22: mod_base = OTHER; note = 2'-O-methyluridine-3'-phosphorothioate
  modified_base 23: mod_base = OTHER; note = 2'-O-methyluridine
aaccacaaaactcagaatatatt

SEQ ID NO: 478 - RNA, 23 nt, synthetic construct
  source 1..23: mol_type = other RNA
  modified_base 1: mod_base = OTHER; note = 2'-O-methyladenosine-3'-phosphorothioate
  modified_base 2: mod_base = OTHER; note = 2'-deoxy-2'-fluorocytidine-3'-phosphorothioate
  modified_base 3: mod_base = OTHER; note = 2'-O-methyluridine-3'-phosphate
  modified_base 4: mod_base = OTHER; note = 2'-O-methyladenosine-3'-phosphate
  modified_base 5: mod_base = OTHER; note = 2'-O-methylcytidine-3'-phosphate
  modified_base 6: mod_base = OTHER; note = 2'-deoxy-2'-fluoroadenosine-3'-phosphate
  modified_base 7: mod_base = OTHER; note = 2'-O-methyladenosine-3'-phosphate
  modified_base 8: mod_base = OTHER; note = 2'-deoxy-2'-fluoroguanosine-3'-phosphate
  modified_base 9: mod_base = OTHER; note = 2'-deoxy-2'-fluoroguanosine-3'-phosphate
  modified_base 10: mod_base = OTHER; note = 2'-O-methyladenosine-3'-phosphate
  modified_base 11: mod_base = OTHER; note = 2'-O-methyladenosine-3'-phosphate
  modified_base 12: mod_base = OTHER; note = 2'-O-methylcytidine-3'-phosphate
  modified_base 13: mod_base = OTHER; note = 2'-O-methyluridine-3'-phosphate
  modified_base 14: mod_base = OTHER; note = 2'-deoxy-2'-fluorocytidine-3'-phosphate
  modified_base 15: mod_base = OTHER; note = 2'-O-methyladenosine-3'-phosphate
  modified_base 16: mod_base = OTHER; note = 2'-deoxy-2'-fluorouridine-3'-phosphate
  modified_base 17: mod_base = OTHER; note = 2'-O-methylcytidine-3'-phosphate
  modified_base 18: mod_base = OTHER; note = 2'-O-methyluridine-3'-phosphate
  modified_base 19: mod_base = OTHER; note = 2'-O-methylcytidine-3'-phosphate
  modified_base 20: mod_base = OTHER; note = 2'-O-methyladenosine-3'-phosphate
  modified_base 21: mod_base = OTHER; note = 2'-O-methyluridine-3'-phosphorothioate
  modified_base 22: mod_base = OTHER; note = 2'-O-methylguanosine-3'-phosphorothioate
  modified_base 23: mod_base = OTHER; note = 2'-O-methyladenosine
actacaaggaactcatctcatga

SEQ ID NO: 479 - RNA, 23 nt, synthetic construct
  source 1..23: mol_type = other RNA
  modified_base 1: mod_base = OTHER; note = 2'-O-methyladenosine-3'-phosphorothioate
  modified_base 2: mod_base = OTHER; note = 2'-deoxy-2'-fluorouridine-3'-phosphorothioate
  modified_base 3: mod_base = OTHER; note = 2'-O-methyluridine-3'-phosphate
  modified_base 4: mod_base = OTHER; note = 2'-O-methyladenosine-3'-phosphate
  modified_base 5: mod_base = OTHER; note = 2'-O-methyluridine-3'-phosphate
  modified_base 6: mod_base = OTHER; note = 2'-deoxy-2'-fluorouridine-3'-phosphate
  modified_base 7: mod_base = OTHER; note = 2'-O-methylguanosine-3'-phosphate
  modified_base 8: mod_base = OTHER; note = 2'-deoxy-2'-fluoroadenosine-3'-phosphate
  modified_base 9: mod_base = OTHER; note = 2'-deoxy-2'-fluoroguanosine-3'-phosphate
  modified_base 10: mod_base = OTHER; note = 2'-O-methyladenosine-3'-phosphate
  modified_base 11: mod_base = OTHER; note = 2'-O-methyluridine-3'-phosphate
  modified_base 12: mod_base = OTHER; note = 2'-O-methyluridine-3'-phosphate
  modified_base 13: mod_base = OTHER; note = 2'-O-methyluridine-3'-phosphate
  modified_base 14: mod_base = OTHER; note = 2'-deoxy-2'-fluorocytidine-3'-phosphate
  modified_base 15: mod_base = OTHER; note = 2'-O-methyladenosine-3'-phosphate
  modified_base 16: mod_base = OTHER; note = 2'-deoxy-2'-fluorouridine-3'-phosphate
  modified_base 17: mod_base = OTHER; note = 2'-O-methylcytidine-3'-phosphate
  modified_base 18: mod_base = OTHER; note = 2'-O-methyluridine-3'-phosphate
  modified_base 19: mod_base = OTHER; note = 2'-O-methyluridine-3'-phosphate
  modified_base 20: mod_base = OTHER; note = 2'-O-methylguanosine-3'-phosphate
  modified_base 21: mod_base = OTHER; note = 2'-O-methyluridine-3'-phosphorothioate
  modified_base 22: mod_base = OTHER; note = 2'-O-methyladenosine-3'-phosphorothioate
  modified_base 23: mod_base = OTHER; note = 2'-O-methylguanosine
attattgagatttcatcttgtag

SEQ ID NO: 480 - RNA, 23 nt, synthetic construct
  source 1..23: mol_type = other RNA
  modified_base 1: mod_base = OTHER; note = 2'-O-methyladenosine-3'-phosphorothioate
  modified_base 2: mod_base = OTHER; note = 2'-deoxy-2'-fluoroadenosine-3'-phosphorothioate
  modified_base 3: mod_base = OTHER; note = 2'-O-methyladenosine-3'-phosphate
  modified_base 4: mod_base = OTHER; note = 2'-O-methyluridine-3'-phosphate
  modified_base 5: mod_base = OTHER; note = 2'-O-methyluridine-3'-phosphate
  modified_base 6: mod_base = OTHER; note = 2'-deoxy-2'-fluoroadenosine-3'-phosphate
  modified_base 7: mod_base = OTHER; note = 2'-O-methylguanosine-3'-phosphate
  modified_base 8: mod_base = OTHER; note = 2'-deoxy-2'-fluorouridine-3'-phosphate
  modified_base 9: mod_base = OTHER; note = 2'-deoxy-2'-fluorocytidine-3'-phosphate
  modified_base 10: mod_base = OTHER; note = 2'-O-methylcytidine-3'-phosphate
  modified_base 11: mod_base = OTHER; note = 2'-O-methyluridine-3'-phosphate
  modified_base 12: mod_base = OTHER; note = 2'-O-methyluridine-3'-phosphate
  modified_base 13: mod_base = OTHER; note = 2'-O-methyladenosine-3'-phosphate
  modified_base 14: mod_base = OTHER; note = 2'-deoxy-2'-fluoroadenosine-3'-phosphate
  modified_base 15: mod_base = OTHER; note = 2'-O-methyladenosine-3'-phosphate
  modified_base 16: mod_base = OTHER; note = 2'-deoxy-2'-fluoroadenosine-3'-phosphate
  modified_base 17: mod_base = OTHER; note = 2'-O-methylguanosine-3'-phosphate
  modified_base 18: mod_base = OTHER; note = 2'-O-methyluridine-3'-phosphate
  modified_base 19: mod_base = OTHER; note = 2'-O-methyluridine-3'-phosphate
  modified_base 20: mod_base = OTHER; note = 2'-O-methylguanosine-3'-phosphate
  modified_base 21: mod_base = OTHER; note = 2'-O-methyluridine-3'-phosphorothioate
  modified_base 22: mod_base = OTHER; note = 2'-O-methyladenosine-3'-phosphorothioate
  modified_base 23: mod_base = OTHER; note = 2'-O-methylcytidine
aaattagtccttaaaagttgtac

SEQ ID NO: 481 - RNA, 23 nt, synthetic construct
  source 1..23: mol_type = other RNA
  modified_base 1: mod_base = OTHER; note = 2'-O-methyladenosine-3'-phosphorothioate
  modified_base 2: mod_base = OTHER; note = 2'-deoxy-2'-fluorouridine-3'-phosphorothioate
  modified_base 3: mod_base = OTHER; note = 2'-O-methyladenosine-3'-phosphate
  modified_base 4: mod_base = OTHER; note = 2'-O-methyladenosine-3'-phosphate
  modified_base 5: mod_base = OTHER; note = 2'-O-methylguanosine-3'-phosphate
  modified_base 6: mod_base = OTHER; note = 2'-deoxy-2'-fluorouridine-3'-phosphate
  modified_base 7: mod_base = OTHER; note = 2'-O-methyladenosine-3'-phosphate
  modified_base 8: mod_base = OTHER; note = 2'-deoxy-2'-fluorouridine-3'-phosphate
  modified_base 9: mod_base = OTHER; note = 2'-deoxy-2'-fluoroadenosine-3'-phosphate
  modified_base 10: mod_base = OTHER; note = 2'-O-methylcytidine-3'-phosphate
  modified_base 11: mod_base = OTHER; note = 2'-O-methylcytidine-3'-phosphate
  modified_base 12: mod_base = OTHER; note = 2'-O-methyladenosine-3'-phosphate
  modified_base 13: mod_base = OTHER; note = 2'-O-methyluridine-3'-phosphate
  modified_base 14: mod_base = OTHER; note = 2'-deoxy-2'-fluoroguanosine-3'-phosphate
  modified_base 15: mod_base = OTHER; note = 2'-O-methyluridine-3'-phosphate
  modified_base 16: mod_base = OTHER; note = 2'-deoxy-2'-fluoroadenosine-3'-phosphate
  modified_base 17: mod_base = OTHER; note = 2'-O-methyladenosine-3'-phosphate
  modified_base 18: mod_base = OTHER; note = 2'-O-methylguanosine-3'-phosphate
  modified_base 19: mod_base = OTHER; note = 2'-O-methyladenosine-3'-phosphate
  modified_base 20: mod_base = OTHER; note = 2'-O-methyluridine-3'-phosphate
  modified_base 21: mod_base = OTHER; note = 2'-O-methyluridine-3'-phosphorothioate
  modified_base 22: mod_base = OTHER; note = 2'-O-methylcytidine-3'-phosphorothioate
  modified_base 23: mod_base = OTHER; note = 2'-O-methyladenosine
ataagtataccatgtaagattca

SEQ ID NO: 482 - RNA, 23 nt, synthetic construct
  source 1..23: mol_type = other RNA
  modified_base 1: mod_base = OTHER; note = 2'-O-methyladenosine-3'-phosphorothioate
  modified_base 2: mod_base = OTHER; note = 2'-deoxy-2'-fluoroadenosine-3'-phosphorothioate
  modified_base 3: mod_base = OTHER; note = 2'-O-methyladenosine-3'-phosphate
  modified_base 4: mod_base = OTHER; note = 2'-O-methylcytidine-3'-phosphate
  modified_base 5: mod_base = OTHER; note = 2'-O-methylcytidine-3'-phosphate
  modified_base 6: mod_base = OTHER; note = 2'-deoxy-2'-fluoroadenosine-3'-phosphate
  modified_base 7: mod_base = OTHER; note = 2'-O-methylguanosine-3'-phosphate
  modified_base 8: mod_base = OTHER; note = 2'-deoxy-2'-fluoroadenosine-3'-phosphate
  modified_base 9: mod_base = OTHER; note = 2'-deoxy-2'-fluorouridine-3'-phosphate
  modified_base 10: mod_base = OTHER; note = 2'-O-methyladenosine-3'-phosphate
  modified_base 11: mod_base = OTHER; note = 2'-O-methyladenosine-3'-phosphate
  modified_base 12: mod_base = OTHER; note = 2'-O-methyluridine-3'-phosphate
  modified_base 13: mod_base = OTHER; note = 2'-O-methyladenosine-3'-phosphate
  modified_base 14: mod_base = OTHER; note = 2'-deoxy-2'-fluorouridine-3'-phosphate
  modified_base 15: mod_base = OTHER; note = 2'-O-methyladenosine-3'-phosphate
  modified_base 16: mod_base = OTHER; note = 2'-deoxy-2'-fluorocytidine-3'-phosphate
  modified_base 17: mod_base = OTHER; note = 2'-O-methylcytidine-3'-phosphate
  modified_base 18: mod_base = OTHER; note = 2'-O-methyladenosine-3'-phosphate
  modified_base 19: mod_base = OTHER; note = 2'-O-methyladenosine-3'-phosphate
  modified_base 20: mod_base = OTHER; note = 2'-O-methylcytidine-3'-phosphate
  modified_base 21: mod_base = OTHER; note = 2'-O-methyladenosine-3'-phosphorothioate
  modified_base 22: mod_base = OTHER; note = 2'-O-methyladenosine-3'-phosphorothioate
  modified_base 23: mod_base = OTHER; note = 2'-O-methyladenosine
aaaccagataatataccaacaaa

SEQ ID NO: 483 - RNA, 23 nt, synthetic construct
  source 1..23: mol_type = other RNA
  modified_base 1: mod_base = OTHER; note = 2'-O-methyladenosine-3'-phosphorothioate
  modified_base 2: mod_base = OTHER; note = 2'-deoxy-2'-fluoroadenosine-3'-phosphorothioate
  modified_base 3: mod_base = OTHER; note = 2'-O-methyladenosine-3'-phosphate
  modified_base 4: mod_base = OTHER; note = 2'-O-methylguanosine-3'-phosphate
  modified_base 5: mod_base = OTHER; note = 2'-O-methylguanosine-3'-phosphate
  modified_base 6: mod_base = OTHER; note = 2'-deoxy-2'-fluoroadenosine-3'-phosphate
  modified_base 7: mod_base = OTHER; note = 2'-O-methyladenosine-3'-phosphate
  modified_base 8: mod_base = OTHER; note = 2'-deoxy-2'-fluoroguanosine-3'-phosphate
  modified_base 9: mod_base = OTHER; note = 2'-deoxy-2'-fluorocytidine-3'-phosphate
  modified_base 10: mod_base = OTHER; note = 2'-O-methyladenosine-3'-phosphate
  modified_base 11: mod_base = OTHER; note = 2'-O-methyluridine-3'-phosphate
  modified_base 12: mod_base = OTHER; note = 2'-O-methyluridine-3'-phosphate
  modified_base 13: mod_base = OTHER; note = 2'-O-methyladenosine-3'-phosphate
  modified_base 14: mod_base = OTHER; note = 2'-deoxy-2'-fluoroadenosine-3'-phosphate
  modified_base 15: mod_base = OTHER; note = 2'-O-methylcytidine-3'-phosphate
  modified_base 16: mod_base = OTHER; note = 2'-deoxy-2'-fluorocytidine-3'-phosphate
  modified_base 17: mod_base = OTHER; note = 2'-O-methyladenosine-3'-phosphate
  modified_base 18: mod_base = OTHER; note = 2'-O-methylcytidine-3'-phosphate
  modified_base 19: mod_base = OTHER; note = 2'-O-methyluridine-3'-phosphate
  modified_base 20: mod_base = OTHER; note = 2'-O-methyladenosine-3'-phosphate
  modified_base 21: mod_base = OTHER; note = 2'-O-methyladenosine-3'-phosphorothioate
  modified_base 22: mod_base = OTHER; note = 2'-O-methylcytidine-3'-phosphorothioate
  modified_base 23: mod_base = OTHER; note = 2'-O-methylcytidine
aaaggaagcattaaccactaacc

SEQ ID NO: 484 - RNA, 23 nt, synthetic construct
  source 1..23: mol_type = other RNA
  modified_base 1: mod_base = OTHER; note = 2'-O-methyladenosine-3'-phosphorothioate
  modified_base 2: mod_base = OTHER; note = 2'-deoxy-2'-fluoroadenosine-3'-phosphorothioate
  modified_base 3: mod_base = OTHER; note = 2'-O-methyladenosine-3'-phosphate
  modified_base 4: mod_base = OTHER; note = 2'-O-methylguanosine-3'-phosphate
  modified_base 5: mod_base = OTHER; note = 2'-O-methyladenosine-3'-phosphate
  modified_base 6: mod_base = OTHER; note = 2'-deoxy-2'-fluoroguanosine-3'-phosphate
  modified_base 7: mod_base = OTHER; note = 2'-O-methyluridine-3'-phosphate
  modified_base 8: mod_base = OTHER; note = 2'-deoxy-2'-fluoroguanosine-3'-phosphate
  modified_base 9: mod_base = OTHER; note = 2'-deoxy-2'-fluoroadenosine-3'-phosphate
  modified_base 10: mod_base = OTHER; note = 2'-O-methyladenosine-3'-phosphate
  modified_base 11: mod_base = OTHER; note = 2'-O-methyluridine-3'-phosphate
  modified_base 12: mod_base = OTHER; note = 2'-O-methylguanosine-3'-phosphate
  modified_base 13: mod_base = OTHER; note = 2'-O-methylguanosine-3'-phosphate
  modified_base 14: mod_base = OTHER; note = 2'-deoxy-2'-fluoroadenosine-3'-phosphate
  modified_base 15: mod_base = OTHER; note = 2'-O-methyluridine-3'-phosphate
  modified_base 16: mod_base = OTHER; note = 2'-deoxy-2'-fluoroguanosine-3'-phosphate
  modified_base 17: mod_base = OTHER; note = 2'-O-methyladenosine-3'-phosphate
  modified_base 18: mod_base = OTHER; note = 2'-O-methylcytidine-3'-phosphate
  modified_base 19: mod_base = OTHER; note = 2'-O-methyluridine-3'-phosphate
  modified_base 20: mod_base = OTHER; note = 2'-O-methylcytidine-3'-phosphate
  modified_base 21: mod_base = OTHER; note = 2'-O-methyladenosine-3'-phosphorothioate
  modified_base 22: mod_base = OTHER; note = 2'-O-methyladenosine-3'-phosphorothioate
  modified_base 23: mod_base = OTHER; note = 2'-O-methyluridine
aaagagtgaatggatgactcaat

SEQ ID NO: 485 - RNA, 23 nt, synthetic construct
  source 1..23: mol_type = other RNA
  modified_base 1: mod_base = OTHER; note = 2'-O-methyladenosine-3'-phosphorothioate
  modified_base 2: mod_base = OTHER; note = 2'-deoxy-2'-fluoroadenosine-3'-phosphorothioate
  modified_base 3: mod_base = OTHER; note = 2'-O-methylcytidine-3'-phosphate
  modified_base 4: mod_base = OTHER; note = 2'-O-methyluridine-3'-phosphate
  modified_base 5: mod_base = OTHER; note = 2'-O-methyladenosine-3'-phosphate
  modified_base 6: mod_base = OTHER; note = 2'-deoxy-2'-fluorouridine-3'-phosphate
  modified_base 7: mod_base = OTHER; note = 2'-O-methyluridine-3'-phosphate
  modified_base 8: mod_base = OTHER; note = 2'-deoxy-2'-fluoroguanosine-3'-phosphate
  modified_base 9: mod_base = OTHER; note = 2'-deoxy-2'-fluoroadenosine-3'-phosphate
  modified_base 10: mod_base = OTHER; note = 2'-O-methylcytidine-3'-phosphate
  modified_base 11: mod_base = OTHER; note = 2'-O-methyladenosine-3'-phosphate
  modified_base 12: mod_base = OTHER; note = 2'-O-methylguanosine-3'-phosphate
  modified_base 13: mod_base = OTHER; note = 2'-O-methyladenosine-3'-phosphate
  modified_base 14: mod_base = OTHER; note = 2'-deoxy-2'-fluorouridine-3'-phosphate
  modified_base 15: mod_base = OTHER; note = 2'-O-methyladenosine-3'-phosphate
  modified_base 16: mod_base = OTHER; note = 2'-deoxy-2'-fluoroadenosine-3'-phosphate
  modified_base 17: mod_base = OTHER; note = 2'-O-methyladenosine-3'-phosphate
  modified_base 18: mod_base = OTHER; note = 2'-O-methyladenosine-3'-phosphate
  modified_base 19: mod_base = OTHER; note = 2'-O-methylcytidine-3'-phosphate
  modified_base 20: mod_base = OTHER; note = 2'-O-methyluridine-3'-phosphate
  modified_base 21: mod_base = OTHER; note = 2'-O-methylguanosine-3'-phosphorothioate
  modified_base 22: mod_base = OTHER; note = 2'-O-methyladenosine-3'-phosphorothioate
  modified_base 23: mod_base = OTHER; note = 2'-O-methyladenosine
aactattgacagataaaactgaa

SEQ ID NO: 486 - RNA, 23 nt, synthetic construct
  source 1..23: mol_type = other RNA
  modified_base 1: mod_base = OTHER; note = 2'-O-methyladenosine-3'-phosphorothioate
  modified_base 2: mod_base = OTHER; note = 2'-deoxy-2'-fluoroadenosine-3'-phosphorothioate
  modified_base 3: mod_base = OTHER; note = 2'-O-methyladenosine-3'-phosphate
  modified_base 4: mod_base = OTHER; note = 2'-O-methyluridine-3'-phosphate
  modified_base 5: mod_base = OTHER; note = 2'-O-methyluridine-3'-phosphate
  modified_base 6: mod_base = OTHER; note = 2'-deoxy-2'-fluorouridine-3'-phosphate
  modified_base 7: mod_base = OTHER; note = 2'-O-methyladenosine-3'-phosphate
  modified_base 8: mod_base = OTHER; note = 2'-deoxy-2'-fluorouridine-3'-phosphate
  modified_base 9: mod_base = OTHER; note = 2'-deoxy-2'-fluoroadenosine-3'-phosphate
  modified_base 10: mod_base = OTHER; note = 2'-O-methyladenosine-3'-phosphate
  modified_base 11: mod_base = OTHER; note = 2'-O-methyladenosine-3'-phosphate
  modified_base 12: mod_base = OTHER; note = 2'-O-methylguanosine-3'-phosphate
  modified_base 13: mod_base = OTHER; note = 2'-O-methylcytidine-3'-phosphate
  modified_base 14: mod_base = OTHER; note = 2'-deoxy-2'-fluoroadenosine-3'-phosphate
  modified_base 15: mod_base = OTHER; note = 2'-O-methylcytidine-3'-phosphate
  modified_base 16: mod_base = OTHER; note = 2'-deoxy-2'-fluorouridine-3'-phosphate
  modified_base 17: mod_base = OTHER; note = 2'-O-methyluridine-3'-phosphate
  modified_base 18: mod_base = OTHER; note = 2'-O-methyluridine-3'-phosphate
  modified_base 19: mod_base = OTHER; note = 2'-O-methylguanosine-3'-phosphate
  modified_base 20: mod_base = OTHER; note = 2'-O-methylguanosine-3'-phosphate
  modified_base 21: mod_base = OTHER; note = 2'-O-methylguanosine-3'-phosphorothioate
  modified_base 22: mod_base = OTHER; note = 2'-O-methyladenosine-3'-phosphorothioate
  modified_base 23: mod_base = OTHER; note = 2'-O-methyluridine
aaatttataaagcactttgggat

SEQ ID NO: 487 - RNA, 23 nt, synthetic construct
  source 1..23: mol_type = other RNA
  modified_base 1: mod_base = OTHER; note = 2'-O-methyladenosine-3'-phosphorothioate
  modified_base 2: mod_base = OTHER; note = 2'-deoxy-2'-fluoroadenosine-3'-phosphorothioate
  modified_base 3: mod_base = OTHER; note = 2'-O-methyladenosine-3'-phosphate
  modified_base 4: mod_base = OTHER; note = 2'-O-methyladenosine-3'-phosphate
  modified_base 5: mod_base = OTHER; note = 2'-O-methylcytidine-3'-phosphate
  modified_base 6: mod_base = OTHER; note = 2'-deoxy-2'-fluoroadenosine-3'-phosphate
  modified_base 7: mod_base = OTHER; note = 2'-O-methyluridine-3'-phosphate
  modified_base 8: mod_base = OTHER; note = 2'-deoxy-2'-fluorouridine-3'-phosphate
  modified_base 9: mod_base = OTHER; note = 2'-deoxy-2'-fluorouridine-3'-phosphate
  modified_base 10: mod_base = OTHER; note = 2'-O-methylcytidine-3'-phosphate
  modified_base 11: mod_base = OTHER; note = 2'-O-methyluridine-3'-phosphate
  modified_base 12: mod_base = OTHER; note = 2'-O-methyladenosine-3'-phosphate
  modified_base 13: mod_base = OTHER; note = 2'-O-methyladenosine-3'-phosphate
  modified_base 14: mod_base = OTHER; note = 2'-deoxy-2'-fluoroadenosine-3'-phosphate
  modified_base 15: mod_base = OTHER; note = 2'-O-methyluridine-3'-phosphate
  modified_base 16: mod_base = OTHER; note = 2'-deoxy-2'-fluorocytidine-3'-phosphate
  modified_base 17: mod_base = OTHER; note = 2'-O-methyluridine-3'-phosphate
  modified_base 18: mod_base = OTHER; note = 2'-O-methylguanosine-3'-phosphate
  modified_base 19: mod_base = OTHER; note = 2'-O-methyladenosine-3'-phosphate
  modified_base 20: mod_base = OTHER; note = 2'-O-methylcytidine-3'-phosphate
  modified_base 21: mod_base = OTHER; note = 2'-O-methyladenosine-3'-phosphorothioate
  modified_base 22: mod_base = OTHER; note = 2'-O-methylguanosine-3'-phosphorothioate
  modified_base 23: mod_base = OTHER; note = 2'-O-methylcytidine
aaaacatttctaaatctgacagc

SEQ ID NO: 488 - RNA, 23 nt, synthetic construct
  source 1..23: mol_type = other RNA
  modified_base 1: mod_base = OTHER; note = 2'-O-methyladenosine-3'-phosphorothioate
  modified_base 2: mod_base = OTHER; note = 2'-deoxy-2'-fluoroadenosine-3'-phosphorothioate
  modified_base 3: mod_base = OTHER; note = 2'-O-methyladenosine-3'-phosphate
  modified_base 4: mod_base = OTHER; note = 2'-O-methyluridine-3'-phosphate
  modified_base 5: mod_base = OTHER; note = 2'-O-methyladenosine-3'-phosphate
  modified_base 6: mod_base = OTHER; note = 2'-deoxy-2'-fluorouridine-3'-phosphate
  modified_base 7: mod_base = OTHER; note = 2'-O-methyluridine-3'-phosphate
  modified_base 8: mod_base = OTHER; note = 2'-deoxy-2'-fluoroguanosine-3'-phosphate
  modified_base 9: mod_base = OTHER; note = 2'-deoxy-2'-fluorouridine-3'-phosphate
  modified_base 10: mod_base = OTHER; note = 2'-O-methylcytidine-3'-phosphate
  modified_base 11: mod_base = OTHER; note = 2'-O-methyluridine-3'-phosphate
  modified_base 12: mod_base = OTHER; note = 2'-O-methylguanosine-3'-phosphate
  modified_base 13: mod_base = OTHER; note = 2'-O-methyluridine-3'-phosphate
  modified_base 14: mod_base = OTHER; note = 2'-deoxy-2'-fluorouridine-3'-phosphate
  modified_base 15: mod_base = OTHER; note = 2'-O-methyluridine-3'-phosphate
  modified_base 16: mod_base = OTHER; note = 2'-deoxy-2'-fluorouridine-3'-phosphate
  modified_base 17: mod_base = OTHER; note = 2'-O-methylcytidine-3'-phosphate
  modified_base 18: mod_base = OTHER; note = 2'-O-methyladenosine-3'-phosphate
  modified_base 19: mod_base = OTHER; note = 2'-O-methylcytidine-3'-phosphate
  modified_base 20: mod_base = OTHER; note = 2'-O-methyladenosine-3'-phosphate
  modified_base 21: mod_base = OTHER; note = 2'-O-methyluridine-3'-phosphorothioate
  modified_base 22: mod_base = OTHER; note = 2'-O-methyladenosine-3'-phosphorothioate
  modified_base 23: mod_base = OTHER; note = 2'-O-methylguanosine
aaatattgtctgttttcacatag

SEQ ID NO: 489 - RNA, 23 nt, synthetic construct
  source 1..23: mol_type = other RNA
  modified_base 1: mod_base = OTHER; note = 2'-O-methyladenosine-3'-phosphorothioate
  modified_base 2: mod_base = OTHER; note = 2'-deoxy-2'-fluorouridine-3'-phosphorothioate
  modified_base 3: mod_base = OTHER; note = 2'-O-methyluridine-3'-phosphate
  modified_base 4: mod_base = OTHER; note = 2'-O-methylguanosine-3'-phosphate
  modified_base 5: mod_base = OTHER; note = 2'-O-methyladenosine-3'-phosphate
  modified_base 6: mod_base = OTHER; note = 2'-deoxy-2'-fluorouridine-3'-phosphate
  modified_base 7: mod_base = OTHER; note = 2'-O-methyluridine-3'-phosphate
  modified_base 8: mod_base = OTHER; note = 2'-deoxy-2'-fluoroadenosine-3'-phosphate
  modified_base 9: mod_base = OTHER; note = 2'-deoxy-2'-fluorocytidine-3'-phosphate
  modified_base 10: mod_base = OTHER; note = 2'-O-methyladenosine-3'-phosphate
  modified_base 11: mod_base = OTHER; note = 2'-O-methyladenosine-3'-phosphate
  modified_base 12: mod_base = OTHER; note = 2'-O-methyluridine-3'-phosphate
  modified_base 13: mod_base = OTHER; note = 2'-O-methyladenosine-3'-phosphate
  modified_base 14: mod_base = OTHER; note = 2'-deoxy-2'-fluorouridine-3'-phosphate
  modified_base 15: mod_base = OTHER; note = 2'-O-methylcytidine-3'-phosphate
  modified_base 16: mod_base = OTHER; note = 2'-deoxy-2'-fluorouridine-3'-phosphate
  modified_base 17: mod_base = OTHER; note = 2'-O-methylcytidine-3'-phosphate
  modified_base 18: mod_base = OTHER; note = 2'-O-methyladenosine-3'-phosphate
  modified_base 19: mod_base = OTHER; note = 2'-O-methylguanosine-3'-phosphate
  modified_base 20: mod_base = OTHER; note = 2'-O-methyluridine-3'-phosphate
  modified_base 21: mod_base = OTHER; note = 2'-O-methyluridine-3'-phosphorothioate
  modified_base 22: mod_base = OTHER; note = 2'-O-methylcytidine-3'-phosphorothioate
  modified_base 23: mod_base = OTHER; note = 2'-O-methylcytidine
attgattacaatatctcagttcc

SEQ ID NO: 490 - RNA, 23 nt, synthetic construct
  source 1..23: mol_type = other RNA
  modified_base 1: mod_base = OTHER; note = 2'-O-methyladenosine-3'-phosphorothioate
  modified_base 2: mod_base = OTHER; note = 2'-deoxy-2'-fluoroadenosine-3'-phosphorothioate
  modified_base 3: mod_base = OTHER; note = 2'-O-methyladenosine-3'-phosphate
  modified_base 4: mod_base = OTHER; note = 2'-O-methyladenosine-3'-phosphate
  modified_base 5: mod_base = OTHER; note = 2'-O-methyluridine-3'-phosphate
  modified_base 6: mod_base = OTHER; note = 2'-deoxy-2'-fluorouridine-3'-phosphate
  modified_base 7: mod_base = OTHER; note = 2'-O-methyladenosine-3'-phosphate
  modified_base 8: mod_base = OTHER; note = 2'-deoxy-2'-fluoroadenosine-3'-phosphate
  modified_base 9: mod_base = OTHER; note = 2'-deoxy-2'-fluorocytidine-3'-phosphate
  modified_base 10: mod_base = OTHER; note = 2'-O-methyluridine-3'-phosphate
  modified_base 11: mod_base = OTHER; note = 2'-O-methyluridine-3'-phosphate
  modified_base 12: mod_base = OTHER; note = 2'-O-methylcytidine-3'-phosphate
  modified_base 13: mod_base = OTHER; note = 2'-O-methylcytidine-3'-phosphate
  modified_base 14: mod_base = OTHER; note = 2'-deoxy-2'-fluorouridine-3'-phosphate
  modified_base 15: mod_base = OTHER; note = 2'-O-methylguanosine-3'-phosphate
  modified_base 16: mod_base = OTHER; note = 2'-deoxy-2'-fluoroadenosine-3'-phosphate
  modified_base 17: mod_base = OTHER; note = 2'-O-methyluridine-3'-phosphate
  modified_base 18: mod_base = OTHER; note = 2'-O-methylguanosine-3'-phosphate
  modified_base 19: mod_base = OTHER; note = 2'-O-methyluridine-3'-phosphate
  modified_base 20: mod_base = OTHER; note = 2'-O-methyluridine-3'-phosphate
  modified_base 21: mod_base = OTHER; note = 2'-O-methyladenosine-3'-phosphorothioate
  modified_base 22: mod_base = OTHER; note = 2'-O-methyladenosine-3'-phosphorothioate
  modified_base 23: mod_base = OTHER; note = 2'-O-methylcytidine
aaaattaacttcctgatgttaac

SEQ ID NO: 491 - RNA, 23 nt, synthetic construct
  source 1..23: mol_type = other RNA
  modified_base 1: mod_base = OTHER; note = 2'-O-methyladenosine-3'-phosphorothioate
  modified_base 2: mod_base = OTHER; note = 2'-deoxy-2'-fluoroadenosine-3'-phosphorothioate
  modified_base 3: mod_base = OTHER; note = 2'-O-methyladenosine-3'-phosphate
  modified_base 4: mod_base = OTHER; note = 2'-O-methylguanosine-3'-phosphate
  modified_base 5: mod_base = OTHER; note = 2'-O-methyluridine-3'-phosphate
  modified_base 6: mod_base = OTHER; note = 2'-deoxy-2'-fluorouridine-3'-phosphate
  modified_base 7: mod_base = OTHER; note = 2'-O-methyluridine-3'-phosphate
  modified_base 8: mod_base = OTHER; note = 2'-deoxy-2'-fluorocytidine-3'-phosphate
  modified_base 9: mod_base = OTHER; note = 2'-deoxy-2'-fluorocytidine-3'-phosphate
  modified_base 10: mod_base = OTHER; note = 2'-O-methylcytidine-3'-phosphate
  modified_base 11: mod_base = OTHER; note = 2'-O-methyluridine-3'-phosphate
  modified_base 12: mod_base = OTHER; note = 2'-O-methyladenosine-3'-phosphate
  modified_base 13: mod_base = OTHER; note = 2'-O-methylguanosine-3'-phosphate
  modified_base 14: mod_base = OTHER; note = 2'-deoxy-2'-fluoroadenosine-3'-phosphate
  modified_base 15: mod_base = OTHER; note = 2'-O-methyladenosine-3'-phosphate
  modified_base 16: mod_base = OTHER; note = 2'-deoxy-2'-fluorouridine-3'-phosphate
  modified_base 17: mod_base = OTHER; note = 2'-O-methyluridine-3'-phosphate
  modified_base 18: mod_base = OTHER; note = 2'-O-methyluridine-3'-phosphate
  modified_base 19: mod_base = OTHER; note = 2'-O-methyluridine-3'-phosphate
  modified_base 20: mod_base = OTHER; note = 2'-O-methylguanosine-3'-phosphate
  modified_base 21: mod_base = OTHER; note = 2'-O-methylcytidine-3'-phosphorothioate
  modified_base 22: mod_base = OTHER; note = 2'-O-methylcytidine-3'-phosphorothioate
  modified_base 23: mod_base = OTHER; note = 2'-O-methyladenosine
aaagtttccctagaattttgcca

SEQ ID NO: 492 - RNA, 23 nt, synthetic construct
  source 1..23: mol_type = other RNA
  modified_base 1: mod_base = OTHER; note = 2'-O-methyladenosine-3'-phosphorothioate
  modified_base 2: mod_base = OTHER; note = 2'-deoxy-2'-fluorouridine-3'-phosphorothioate
  modified_base 3: mod_base = OTHER; note = 2'-O-methyluridine-3'-phosphate
  modified_base 4: mod_base = OTHER; note = 2'-O-methyluridine-3'-phosphate
  modified_base 5: mod_base = OTHER; note = 2'-O-methyladenosine-3'-phosphate
  modified_base 6: mod_base = OTHER; note = 2'-deoxy-2'-fluorouridine-3'-phosphate
  modified_base 7: mod_base = OTHER; note = 2'-O-methyladenosine-3'-phosphate
  modified_base 8: mod_base = OTHER; note = 2'-deoxy-2'-fluorouridine-3'-phosphate
  modified_base 9: mod_base = OTHER; note = 2'-deoxy-2'-fluoroguanosine-3'-phosphate
  modified_base 10: mod_base = OTHER; note = 2'-O-methyladenosine-3'-phosphate
  modified_base 11: mod_base = OTHER; note = 2'-O-methylguanosine-3'-phosphate
  modified_base 12: mod_base = OTHER; note = 2'-O-methylcytidine-3'-phosphate
  modified_base 13: mod_base = OTHER; note = 2'-O-methyladenosine-3'-phosphate
  modified_base 14: mod_base = OTHER; note = 2'-deoxy-2'-fluoroadenosine-3'-phosphate
  modified_base 15: mod_base = OTHER; note = 2'-O-methyladenosine-3'-phosphate
  modified_base 16: mod_base = OTHER; note = 2'-deoxy-2'-fluoroadenosine-3'-phosphate
  modified_base 17: mod_base = OTHER; note = 2'-O-methylguanosine-3'-phosphate
  modified_base 18: mod_base = OTHER; note = 2'-O-methylcytidine-3'-phosphate
  modified_base 19: mod_base = OTHER; note = 2'-O-methylcytidine-3'-phosphate
  modified_base 20: mod_base = OTHER; note = 2'-O-methyluridine-3'-phosphate
  modified_base 21: mod_base = OTHER; note = 2'-O-methyluridine-3'-phosphorothioate
  modified_base 22: mod_base = OTHER; note = 2'-O-methylcytidine-3'-phosphorothioate
  modified_base 23: mod_base = OTHER; note = 2'-O-methyladenosine
atttatatgagcaaaagccttca

SEQ ID NO: 493 - RNA, 23 nt, synthetic construct
  source 1..23: mol_type = other RNA
  modified_base 1: mod_base = OTHER; note = 2'-O-methyladenosine-3'-phosphorothioate
  modified_base 2: mod_base = OTHER; note = 2'-deoxy-2'-fluorouridine-3'-phosphorothioate
  modified_base 3: mod_base = OTHER; note = 2'-O-methylcytidine-3'-phosphate
  modified_base 4: mod_base = OTHER; note = 2'-O-methyladenosine-3'-phosphate
  modified_base 5: mod_base = OTHER; note = 2'-O-methyluridine-3'-phosphate
  modified_base 6: mod_base = OTHER; note = 2'-deoxy-2'-fluorouridine-3'-phosphate
  modified_base 7: mod_base = OTHER; note = 2'-O-methyluridine-3'-phosphate
  modified_base 8: mod_base = OTHER; note = 2'-deoxy-2'-fluoroguanosine-3'-phosphate
  modified_base 9: mod_base = OTHER; note = 2'-deoxy-2'-fluoroadenosine-3'-phosphate
  modified_base 10: mod_base = OTHER; note = 2'-O-methyladenosine-3'-phosphate
  modified_base 11: mod_base = OTHER; note = 2'-O-methyladenosine-3'-phosphate
  modified_base 12: mod_base = OTHER; note = 2'-O-methylcytidine-3'-phosphate
  modified_base 13: mod_base = OTHER; note = 2'-O-methyluridine-3'-phosphate
  modified_base 14: mod_base = OTHER; note = 2'-deoxy-2'-fluorocytidine-3'-phosphate
  modified_base 15: mod_base = OTHER; note = 2'-O-methyladenosine-3'-phosphate
  modified_base 16: mod_base = OTHER; note = 2'-deoxy-2'-fluoroadenosine-3'-phosphate
  modified_base 17: mod_base = OTHER; note = 2'-O-methyluridine-3'-phosphate
  modified_base 18: mod_base = OTHER; note = 2'-O-methylguanosine-3'-phosphate
  modified_base 19: mod_base = OTHER; note = 2'-O-methylguanosine-3'-phosphate
  modified_base 20: mod_base = OTHER; note = 2'-O-methylcytidine-3'-phosphate
  modified_base 21: mod_base = OTHER; note = 2'-O-methyladenosine-3'-phosphorothioate
  modified_base 22: mod_base = OTHER; note = 2'-O-methylcytidine-3'-phosphorothioate
  modified_base 23: mod_base = OTHER; note = 2'-O-methyluridine
atcatttgaaactcaatggcact

SEQ ID NO: 494 - RNA, 23 nt, synthetic construct
  source 1..23: mol_type = other RNA
  modified_base 1: mod_base = OTHER; note = 2'-O-methyladenosine-3'-phosphorothioate
  modified_base 2: mod_base = OTHER; note = 2'-deoxy-2'-fluorouridine-3'-phosphorothioate
  modified_base 3: mod_base = OTHER; note = 2'-O-methylcytidine-3'-phosphate
  modified_base 4: mod_base = OTHER; note = 2'-O-methyluridine-3'-phosphate
  modified_base 5: mod_base = OTHER; note = 2'-O-methyladenosine-3'-phosphate
  modified_base 6: mod_base = OTHER; note = 2'-deoxy-2'-fluoroadenosine-3'-phosphate
  modified_base 7: mod_base = OTHER; note = 2'-O-methyladenosine-3'-phosphate
  modified_base 8: mod_base = OTHER; note = 2'-deoxy-2'-fluorouridine-3'-phosphate
  modified_base 9: mod_base = OTHER; note = 2'-deoxy-2'-fluoroadenosine-3'-phosphate
  modified_base 10: mod_base = OTHER; note = 2'-O-methyluridine-3'-phosphate
  modified_base 11: mod_base = OTHER; note = 2'-O-methyladenosine-3'-phosphate
  modified_base 12: mod_base = OTHER; note = 2'-O-methyluridine-3'-phosphate
  modified_base 13: mod_base = OTHER; note = 2'-O-methyluridine-3'-phosphate
  modified_base 14: mod_base = OTHER; note = 2'-deoxy-2'-fluorouridine-3'-phosphate
  modified_base 15: mod_base = OTHER; note = 2'-O-methylguanosine-3'-phosphate
  modified_base 16: mod_base = OTHER; note = 2'-deoxy-2'-fluorocytidine-3'-phosphate
  modified_base 17: mod_base = OTHER; note = 2'-O-methyluridine-3'-phosphate
  modified_base 18: mod_base = OTHER; note = 2'-O-methylguanosine-3'-phosphate
  modified_base 19: mod_base = OTHER; note = 2'-O-methylguanosine-3'-phosphate
  modified_base 20: mod_base = OTHER; note = 2'-O-methyluridine-3'-phosphate
  modified_base 21: mod_base = OTHER; note = 2'-O-methylcytidine-3'-phosphorothioate
  modified_base 22: mod_base = OTHER; note = 2'-O-methyladenosine-3'-phosphorothioate
  modified_base 23: mod_base = OTHER; note = 2'-O-methyluridine
atctaaatatatttgctggtcat

SEQ ID NO: 495 - RNA, 23 nt, synthetic construct
  source 1..23: mol_type = other RNA
  modified_base 1: mod_base = OTHER; note = 2'-O-methyladenosine-3'-phosphorothioate
  modified_base 2: mod_base = OTHER; note = 2'-deoxy-2'-fluorouridine-3'-phosphorothioate
  modified_base 3: mod_base = OTHER; note = 2'-O-methyluridine-3'-phosphate
  modified_base 4: mod_base = OTHER; note = 2'-O-methylguanosine-3'-phosphate
  modified_base 5: mod_base = OTHER; note = 2'-O-methylguanosine-3'-phosphate
  modified_base 6: mod_base = OTHER; note = 2'-deoxy-2'-fluorouridine-3'-phosphate
  modified_base 7: mod_base = OTHER; note = 2'-O-methyluridine-3'-phosphate
  modified_base 8: mod_base = OTHER; note = 2'-deoxy-2'-fluoroguanosine-3'-phosphate
  modified_base 9: mod_base = OTHER; note = 2'-deoxy-2'-fluoroguanosine-3'-phosphate
  modified_base 10: mod_base = OTHER; note = 2'-O-methyladenosine-3'-phosphate
  modified_base 11: mod_base = OTHER; note = 2'-O-methylguanosine-3'-phosphate
  modified_base 12: mod_base = OTHER; note = 2'-O-methylguanosine-3'-phosphate
  modified_base 13: mod_base = OTHER; note = 2'-O-methyladenosine-3'-phosphate
  modified_base 14: mod_base = OTHER; note = 2'-deoxy-2'-fluorouridine-3'-phosphate
  modified_base 15: mod_base = OTHER; note = 2'-O-methyluridine-3'-phosphate
  modified_base 16: mod_base = OTHER; note = 2'-deoxy-2'-fluorouridine-3'-phosphate
  modified_base 17: mod_base = OTHER; note = 2'-O-methylcytidine-3'-phosphate
  modified_base 18: mod_base = OTHER; note = 2'-O-methylcytidine-3'-phosphate
  modified_base 19: mod_base = OTHER; note = 2'-O-methyladenosine-3'-phosphate
  modified_base 20: mod_base = OTHER; note = 2'-O-methyladenosine-3'-phosphate
  modified_base 21: mod_base = OTHER; note = 2'-O-methylguanosine-3'-phosphorothioate
  modified_base 22: mod_base = OTHER; note = 2'-O-methyladenosine-3'-phosphorothioate
  modified_base 23: mod_base = OTHER; note = 2'-O-methyladenosine
attggttggaggatttccaagaa

SEQ ID NO: 496 - RNA, 23 nt, synthetic construct
  source 1..23: mol_type = other RNA
  modified_base 1: mod_base = OTHER; note = 2'-O-methyladenosine-3'-phosphorothioate
  modified_base 2: mod_base = OTHER; note = 2'-deoxy-2'-fluoroadenosine-3'-phosphorothioate
  modified_base 3: mod_base = OTHER; note = 2'-O-methylguanosine-3'-phosphate
  modified_base 4: mod_base = OTHER; note = 2'-O-methyluridine-3'-phosphate
  modified_base 5: mod_base = OTHER; note = 2'-O-methyluridine-3'-phosphate
  modified_base 6: mod_base = OTHER; note = 2'-deoxy-2'-fluoroadenosine-3'-phosphate
  modified_base 7: mod_base = OTHER; note = 2'-O-methylguanosine-3'-phosphate
  modified_base 8: mod_base = OTHER; note = 2'-deoxy-2'-fluoroguanosine-3'-phosphate
  modified_base 9: mod_base = OTHER; note = 2'-deoxy-2'-fluoroadenosine-3'-phosphate
  modified_base 10: mod_base = OTHER; note = 2'-O-methyladenosine-3'-phosphate
  modified_base 11: mod_base = OTHER; note = 2'-O-methyladenosine-3'-phosphate
  modified_base 12: mod_base = OTHER; note = 2'-O-methyladenosine-3'-phosphate
  modified_base 13: mod_base = OTHER; note = 2'-O-methylcytidine-3'-phosphate
  modified_base 14: mod_base = OTHER; note = 2'-deoxy-2'-fluorouridine-3'-phosphate
  modified_base 15: mod_base = OTHER; note = 2'-O-methylguanosine-3'-phosphate
  modified_base 16: mod_base = OTHER; note = 2'-deoxy-2'-fluorocytidine-3'-phosphate
  modified_base 17: mod_base = OTHER; note = 2'-O-methyluridine-3'-phosphate
  modified_base 18: mod_base = OTHER; note = 2'-O-methyladenosine-3'-phosphate
  modified_base 19: mod_base = OTHER; note = 2'-O-methyluridine-3'-phosphate
  modified_base 20: mod_base = OTHER; note = 2'-O-methyluridine-3'-phosphate
  modified_base 21: mod_base = OTHER; note = 2'-O-methyluridine-3'-phosphorothioate
  modified_base 22: mod_base = OTHER; note = 2'-O-methylguanosine-3'-phosphorothioate
  modified_base 23: mod_base = OTHER; note = 2'-O-methylguanosine
aagttaggaaaactgctatttgg

SEQ ID NO: 497 - RNA, 23 nt, synthetic construct
  source 1..23: mol_type = other RNA
  modified_base 1: mod_base = OTHER; note = 2'-O-methyladenosine-3'-phosphorothioate
  modified_base 2: mod_base = OTHER; note = 2'-deoxy-2'-fluoroadenosine-3'-phosphorothioate
  modified_base 3: mod_base = OTHER; note = 2'-O-methyluridine-3'-phosphate
  modified_base 4: mod_base = OTHER; note = 2'-O-methyluridine-3'-phosphate
  modified_base 5: mod_base = OTHER; note = 2'-O-methylcytidine-3'-phosphate
  modified_base 6: mod_base = OTHER; note = 2'-deoxy-2'-fluorouridine-3'-phosphate
  modified_base 7: mod_base = OTHER; note = 2'-O-methyladenosine-3'-phosphate
  modified_base 8: mod_base = OTHER; note = 2'-deoxy-2'-fluoroadenosine-3'-phosphate
  modified_base 9: mod_base = OTHER; note = 2'-deoxy-2'-fluorocytidine-3'-phosphate
  modified_base 10: mod_base = OTHER; note = 2'-O-methyladenosine-3'-phosphate
  modified_base 11: mod_base = OTHER; note = 2'-O-methylguanosine-3'-phosphate
  modified_base 12: mod_base = OTHER; note = 2'-O-methyluridine-3'-phosphate
  modified_base 13: mod_base = OTHER; note = 2'-O-methylcytidine-3'-phosphate
  modified_base 14: mod_base = OTHER; note = 2'-deoxy-2'-fluorouridine-3'-phosphate
  modified_base 15: mod_base = OTHER; note = 2'-O-methylguanosine-3'-phosphate
  modified_base 16: mod_base = OTHER; note = 2'-deoxy-2'-fluorouridine-3'-phosphate
  modified_base 17: mod_base = OTHER; note = 2'-O-methylcytidine-3'-phosphate
  modified_base 18: mod_base = OTHER; note = 2'-O-methyladenosine-3'-phosphate
  modified_base 19: mod_base = OTHER; note = 2'-O-methylguanosine-3'-phosphate
  modified_base 20: mod_base = OTHER; note = 2'-O-methylcytidine-3'-phosphate
  modified_base 21: mod_base = OTHER; note = 2'-O-methyluridine-3'-phosphorothioate
  modified_base 22: mod_base = OTHER; note = 2'-O-methylcytidine-3'-phosphorothioate
  modified_base 23: mod_base = OTHER; note = 2'-O-methyladenosine
aattctaacagtctgtcagctca

SEQ ID NO: 498 - RNA, 23 nt, synthetic construct
  source 1..23: mol_type = other RNA
  modified_base 1: mod_base = OTHER; note = 2'-O-methyladenosine-3'-phosphorothioate
  modified_base 2: mod_base = OTHER; note = 2'-deoxy-2'-fluoroadenosine-3'-phosphorothioate
  modified_base 3: mod_base = OTHER; note = 2'-O-methyladenosine-3'-phosphate
  modified_base 4: mod_base = OTHER; note = 2'-O-methyladenosine-3'-phosphate
  modified_base 5: mod_base = OTHER; note = 2'-O-methyluridine-3'-phosphate
  modified_base 6: mod_base = OTHER; note = 2'-deoxy-2'-fluorocytidine-3'-phosphate
  modified_base 7: mod_base = OTHER; note = 2'-O-methylcytidine-3'-phosphate
  modified_base 8: mod_base = OTHER; note = 2'-deoxy-2'-fluoroadenosine-3'-phosphate
  modified_base 9: mod_base = OTHER; note = 2'-deoxy-2'-fluorouridine-3'-phosphate
  modified_base 10: mod_base = OTHER; note = 2'-O-methyladenosine-3'-phosphate
  modified_base 11: mod_base = OTHER; note = 2'-O-methyladenosine-3'-phosphate
  modified_base 12: mod_base = OTHER; note = 2'-O-methyladenosine-3'-phosphate
  modified_base 13: mod_base = OTHER; note = 2'-O-methyluridine-3'-phosphate
  modified_base 14: mod_base = OTHER; note = 2'-deoxy-2'-fluoroguanosine-3'-phosphate
  modified_base 15: mod_base = OTHER; note = 2'-O-methylcytidine-3'-phosphate
  modified_base 16: mod_base = OTHER; note = 2'-deoxy-2'-fluorocytidine-3'-phosphate
  modified_base 17: mod_base = OTHER; note = 2'-O-methyluridine-3'-phosphate
  modified_base 18: mod_base = OTHER; note = 2'-O-methylcytidine-3'-phosphate
  modified_base 19: mod_base = OTHER; note = 2'-O-methyluridine-3'-phosphate
  modified_base 20: mod_base = OTHER; note = 2'-O-methyladenosine-3'-phosphate
  modified_base 21: mod_base = OTHER; note = 2'-O-methyladenosine-3'-phosphorothioate
  modified_base 22: mod_base = OTHER; note = 2'-O-methylcytidine-3'-phosphorothioate
  modified_base 23: mod_base = OTHER; note = 2'-O-methylcytidine
aaaatccataaatgcctctaacc

SEQ ID NO: 499 - RNA, 23 nt, synthetic construct
  source 1..23: mol_type = other RNA
  modified_base 1: mod_base = OTHER; note = 2'-O-methyladenosine-3'-phosphorothioate
  modified_base 2: mod_base = OTHER; note = 2'-deoxy-2'-fluoroguanosine-3'-phosphorothioate
  modified_base 3: mod_base = OTHER; note = 2'-O-methyluridine-3'-phosphate
  modified_base 4: mod_base = OTHER; note = 2'-O-methyluridine-3'-phosphate
  modified_base 5: mod_base = OTHER; note = 2'-O-methyluridine-3'-phosphate
  modified_base 6: mod_base = OTHER; note = 2'-deoxy-2'-fluoroadenosine-3'-phosphate
  modified_base 7: mod_base = OTHER; note = 2'-O-methylguanosine-3'-phosphate
  modified_base 8: mod_base = OTHER; note = 2'-deoxy-2'-fluoroguanosine-3'-phosphate
  modified_base 9: mod_base = OTHER; note = 2'-deoxy-2'-fluorocytidine-3'-phosphate
  modified_base 10: mod_base = OTHER; note = 2'-O-methyladenosine-3'-phosphate
  modified_base 11: mod_base = OTHER; note = 2'-O-methyluridine-3'-phosphate
  modified_base 12: mod_base = OTHER; note = 2'-O-methyladenosine-3'-phosphate
  modified_base 13: mod_base = OTHER; note = 2'-O-methyluridine-3'-phosphate
  modified_base 14: mod_base = OTHER; note = 2'-deoxy-2'-fluoroadenosine-3'-phosphate
  modified_base 15: mod_base = OTHER; note = 2'-O-methyladenosine-3'-phosphate
  modified_base 16: mod_base = OTHER; note = 2'-deoxy-2'-fluorocytidine-3'-phosphate
  modified_base 17: mod_base = OTHER; note = 2'-O-methylcytidine-3'-phosphate
  modified_base 18: mod_base = OTHER; note = 2'-O-methylcytidine-3'-phosphate
  modified_base 19: mod_base = OTHER; note = 2'-O-methyladenosine-3'-phosphate
  modified_base 20: mod_base = OTHER; note = 2'-O-methyluridine-3'-phosphate
  modified_base 21: mod_base = OTHER; note = 2'-O-methyladenosine-3'-phosphorothioate
  modified_base 22: mod_base = OTHER; note = 2'-O-methyladenosine-3'-phosphorothioate
  modified_base 23: mod_base = OTHER; note = 2'-O-methyladenosine
agtttaggcatataacccataaa

SEQ ID NO: 500 - RNA, 23 nt, synthetic construct
  source 1..23: mol_type = other RNA
  modified_base 1: mod_base = OTHER; note = 2'-O-methyladenosine-3'-phosphorothioate
  modified_base 2: mod_base = OTHER; note = 2'-deoxy-2'-fluoroadenosine-3'-phosphorothioate
  modified_base 3: mod_base = OTHER; note = 2'-O-methyladenosine-3'-phosphate
  modified_base 4: mod_base = OTHER; note = 2'-O-methyluridine-3'-phosphate
  modified_base 5: mod_base = OTHER; note = 2'-O-methyluridine-3'-phosphate
  modified_base 6: mod_base = OTHER; note = 2'-deoxy-2'-fluoroadenosine-3'-phosphate
  modified_base 7: mod_base = OTHER; note = 2'-O-methyluridine-3'-phosphate
  modified_base 8: mod_base = OTHER; note = 2'-deoxy-2'-fluorouridine-3'-phosphate
  modified_base 9: mod_base = OTHER; note = 2'-deoxy-2'-fluorouridine-3'-phosphate
  modified_base 10: mod_base = OTHER; note = 2'-O-methyladenosine-3'-phosphate
  modified_base 11: mod_base = OTHER; note = 2'-O-methylcytidine-3'-phosphate
  modified_base 12: mod_base = OTHER; note = 2'-O-methylcytidine-3'-phosphate
  modified_base 13: mod_base = OTHER; note = 2'-O-methyladenosine-3'-phosphate
  modified_base 14: mod_base = OTHER; note = 2'-deoxy-2'-fluorocytidine-3'-phosphate
  modified_base 15: mod_base = OTHER; note = 2'-O-methyluridine-3'-phosphate
  modified_base 16: mod_base = OTHER; note = 2'-deoxy-2'-fluoroadenosine-3'-phosphate
  modified_base 17: mod_base = OTHER; note = 2'-O-methyluridine-3'-phosphate
  modified_base 18: mod_base = OTHER; note = 2'-O-methylguanosine-3'-phosphate
  modified_base 19: mod_base = OTHER; note = 2'-O-methyluridine-3'-phosphate
  modified_base 20: mod_base = OTHER; note = 2'-O-methylguanosine-3'-phosphate
  modified_base 21: mod_base = OTHER; note = 2'-O-methylguanosine-3'-phosphorothioate
  modified_base 22: mod_base = OTHER; note = 2'-O-methylcytidine-3'-phosphorothioate
  modified_base 23: mod_base = OTHER; note = 2'-O-methyladenosine
aaattatttaccactatgtggca

SEQ ID NO: 501 - RNA, 23 nt, synthetic construct
  source 1..23: mol_type = other RNA
  modified_base 1: mod_base = OTHER; note = 2'-O-methyladenosine-3'-phosphorothioate
  modified_base 2: mod_base = OTHER; note = 2'-deoxy-2'-fluorouridine-3'-phosphorothioate
  modified_base 3: mod_base = OTHER; note = 2'-O-methyladenosine-3'-phosphate
  modified_base 4: mod_base = OTHER; note = 2'-O-methylcytidine-3'-phosphate
  modified_base 5: mod_base = OTHER; note = 2'-O-methylcytidine-3'-phosphate
  modified_base 6: mod_base = OTHER; note = 2'-deoxy-2'-fluoroadenosine-3'-phosphate
  modified_base 7: mod_base = OTHER; note = 2'-O-methyladenosine-3'-phosphate
  modified_base 8: mod_base = OTHER; note = 2'-deoxy-2'-fluorouridine-3'-phosphate
  modified_base 9: mod_base = OTHER; note = 2'-deoxy-2'-fluorouridine-3'-phosphate
  modified_base 10: mod_base = OTHER; note = 2'-O-methyladenosine-3'-phosphate
  modified_base 11: mod_base = OTHER; note = 2'-O-methyluridine-3'-phosphate
  modified_base 12: mod_base = OTHER; note = 2'-O-methylguanosine-3'-phosphate
  modified_base 13: mod_base = OTHER; note = 2'-O-methyladenosine-3'-phosphate
  modified_base 14: mod_base = OTHER; note = 2'-deoxy-2'-fluoroadenosine-3'-phosphate
  modified_base 15: mod_base = OTHER; note = 2'-O-methylcytidine-3'-phosphate
  modified_base 16: mod_base = OTHER; note = 2'-deoxy-2'-fluoroadenosine-3'-phosphate
  modified_base 17: mod_base = OTHER; note = 2'-O-methylguanosine-3'-phosphate
  modified_base 18: mod_base = OTHER; note = 2'-O-methyladenosine-3'-phosphate
  modified_base 19: mod_base = OTHER; note = 2'-O-methylcytidine-3'-phosphate
  modified_base 20: mod_base = OTHER; note = 2'-O-methylcytidine-3'-phosphate
  modified_base 21: mod_base = OTHER; note = 2'-O-methyladenosine-3'-phosphorothioate
  modified_base 22: mod_base = OTHER; note = 2'-O-methyluridine-3'-phosphorothioate
  modified_base 23: mod_base = OTHER; note = 2'-O-methyluridine
ataccaattatgaacagaccatt

SEQ ID NO: 502 - RNA, 23 nt, synthetic construct
  source 1..23: mol_type = other RNA
  modified_base 1: mod_base = OTHER; note = 2'-O-methyladenosine-3'-phosphorothioate
  modified_base 2: mod_base = OTHER; note = 2'-deoxy-2'-fluoroadenosine-3'-phosphorothioate
  modified_base 3: mod_base = OTHER; note = 2'-O-methyluridine-3'-phosphate
  modified_base 4: mod_base = OTHER; note = 2'-O-methyladenosine-3'-phosphate
  modified_base 5: mod_base = OTHER; note = 2'-O-methyladenosine-3'-phosphate
  modified_base 6: mod_base = OTHER; note = 2'-deoxy-2'-fluoroadenosine-3'-phosphate
  modified_base 7: mod_base = OTHER; note = 2'-O-methylcytidine-3'-phosphate
  modified_base 8: mod_base = OTHER; note = 2'-deoxy-2'-fluorocytidine-3'-phosphate
  modified_base 9: mod_base = OTHER; note = 2'-deoxy-2'-fluoroadenosine-3'-phosphate
  modified_base 10: mod_base = OTHER; note = 2'-O-methyladenosine-3'-phosphate
  modified_base 11: mod_base = OTHER; note = 2'-O-methyluridine-3'-phosphate
  modified_base 12: mod_base = OTHER; note = 2'-O-methyladenosine-3'-phosphate
  modified_base 13: mod_base = OTHER; note = 2'-O-methyladenosine-3'-phosphate
  modified_base 14: mod_base = OTHER; note = 2'-deoxy-2'-fluorouridine-3'-phosphate
  modified_base 15: mod_base = OTHER; note = 2'-O-methyluridine-3'-phosphate
  modified_base 16: mod_base = OTHER; note = 2'-deoxy-2'-fluoroadenosine-3'-phosphate
  modified_base 17: mod_base = OTHER; note = 2'-O-methyluridine-3'-phosphate
  modified_base 18: mod_base = OTHER; note = 2'-O-methylguanosine-3'-phosphate
  modified_base 19: mod_base = OTHER; note = 2'-O-methylcytidine-3'-phosphate
  modified_base 20: mod_base = OTHER; note = 2'-O-methyluridine-3'-phosphate
  modified_base 21: mod_base = OTHER; note = 2'-O-methylcytidine-3'-phosphorothioate
  modified_base 22: mod_base = OTHER; note = 2'-O-methylcytidine-3'-phosphorothioate
  modified_base 23: mod_base = OTHER; note = 2'-O-methylcytidine
aataaaccaataattatgctccc

SEQ ID NO: 503 - RNA, 23 nt, synthetic construct
  source 1..23: mol_type = other RNA
  modified_base 1: mod_base = OTHER; note = 2'-O-methyladenosine-3'-phosphorothioate
  modified_base 2: mod_base = OTHER; note = 2'-deoxy-2'-fluoroadenosine-3'-phosphorothioate
  modified_base 3: mod_base = OTHER; note = 2'-O-methylcytidine-3'-phosphate
  modified_base 4: mod_base = OTHER; note = 2'-O-methylcytidine-3'-phosphate
  modified_base 5: mod_base = OTHER; note = 2'-O-methyladenosine-3'-phosphate
  modified_base 6: mod_base = OTHER; note = 2'-deoxy-2'-fluorouridine-3'-phosphate
  modified_base 7: mod_base = OTHER; note = 2'-O-methyladenosine-3'-phosphate
  modified_base 8: mod_base = OTHER; note = 2'-deoxy-2'-fluoroadenosine-3'-phosphate
  modified_base 9: mod_base = OTHER; note = 2'-deoxy-2'-fluorouridine-3'-phosphate
  modified_base 10: mod_base = OTHER; note = 2'-O-methyluridine-3'-phosphate
  modified_base 11: mod_base = OTHER; note = 2'-O-methyladenosine-3'-phosphate
  modified_base 12: mod_base = OTHER; note = 2'-O-methylcytidine-3'-phosphate
  modified_base 13: mod_base = OTHER; note = 2'-O-methylcytidine-3'-phosphate
  modified_base 14: mod_base = OTHER; note = 2'-deoxy-2'-fluoroadenosine-3'-phosphate
  modified_base 15: mod_base = OTHER; note = 2'-O-methyluridine-3'-phosphate
  modified_base 16: mod_base = OTHER; note = 2'-deoxy-2'-fluoroadenosine-3'-phosphate
  modified_base 17: mod_base = OTHER; note = 2'-O-methyladenosine-3'-phosphate
  modified_base 18: mod_base = OTHER; note = 2'-O-methyluridine-3'-phosphate
  modified_base 19: mod_base = OTHER; note = 2'-O-methyladenosine-3'-phosphate
  modified_base 20: mod_base = OTHER; note = 2'-O-methyladenosine-3'-phosphate
  modified_base 21: mod_base = OTHER; note = 2'-O-methyladenosine-3'-phosphorothioate
  modified_base 22: mod_base = OTHER; note = 2'-O-methylcytidine-3'-phosphorothioate
  modified_base 23: mod_base = OTHER; note = 2'-O-methylcytidine
aaccataattaccataataaacc

SEQ ID NO: 504 - RNA, 23 nt, synthetic construct
  source 1..23: mol_type = other RNA
  modified_base 1: mod_base = OTHER; note = 2'-O-methyladenosine-3'-phosphorothioate
  modified_base 2: mod_base = OTHER; note = 2'-deoxy-2'-fluoroadenosine-3'-phosphorothioate
  modified_base 3: mod_base = OTHER; note = 2'-O-methyladenosine-3'-phosphate
  modified_base 4: mod_base = OTHER; note = 2'-O-methylcytidine-3'-phosphate
  modified_base 5: mod_base = OTHER; note = 2'-O-methyluridine-3'-phosphate
  modified_base 6: mod_base = OTHER; note = 2'-deoxy-2'-fluoroguanosine-3'-phosphate
  modified_base 7: mod_base = OTHER; note = 2'-O-methyluridine-3'-phosphate
  modified_base 8: mod_base = OTHER; note = 2'-deoxy-2'-fluorouridine-3'-phosphate
  modified_base 9: mod_base = OTHER; note = 2'-deoxy-2'-fluoroadenosine-3'-phosphate
  modified_base 10: mod_base = OTHER; note = 2'-O-methylguanosine-3'-phosphate
  modified_base 11: mod_base = OTHER; note = 2'-O-methyladenosine-3'-phosphate
  modified_base 12: mod_base = OTHER; note = 2'-O-methyladenosine-3'-phosphate
  modified_base 13: mod_base = OTHER; note = 2'-O-methyladenosine-3'-phosphate
  modified_base 14: mod_base = OTHER; note = 2'-deoxy-2'-fluoroadenosine-3'-phosphate
  modified_base 15: mod_base = OTHER; note = 2'-O-methylcytidine-3'-phosphate
  modified_base 16: mod_base = OTHER; note = 2'-deoxy-2'-fluoroguanosine-3'-phosphate
  modified_base 17: mod_base = OTHER; note = 2'-O-methyluridine-3'-phosphate
  modified_base 18: mod_base = OTHER; note = 2'-O-methyluridine-3'-phosphate
  modified_base 19: mod_base = OTHER; note = 2'-O-methyluridine-3'-phosphate
  modified_base 20: mod_base = OTHER; note = 2'-O-methyluridine-3'-phosphate
  modified_base 21: mod_base = OTHER; note = 2'-O-methyladenosine-3'-phosphorothioate
  modified_base 22: mod_base = OTHER; note = 2'-O-methyladenosine-3'-phosphorothioate
  modified_base 23: mod_base = OTHER; note = 2'-O-methylcytidine
aaactgttagaaaacgttttaac

SEQ ID NO: 505 - RNA, 23 nt, synthetic construct
  source 1..23: mol_type = other RNA
  modified_base 1: mod_base = OTHER; note = 2'-O-methyladenosine-3'-phosphorothioate
  modified_base 2: mod_base = OTHER; note = 2'-deoxy-2'-fluoroadenosine-3'-phosphorothioate
  modified_base 3: mod_base = OTHER; note = 2'-O-methyladenosine-3'-phosphate
  modified_base 4: mod_base = OTHER; note = 2'-O-methyluridine-3'-phosphate
  modified_base 5: mod_base = OTHER; note = 2'-O-methyluridine-3'-phosphate
  modified_base 6: mod_base = OTHER; note = 2'-deoxy-2'-fluorocytidine-3'-phosphate
  modified_base 7: mod_base = OTHER; note = 2'-O-methylcytidine-3'-phosphate
  modified_base 8: mod_base = OTHER; note = 2'-deoxy-2'-fluoroadenosine-3'-phosphate
  modified_base 9: mod_base = OTHER; note = 2'-deoxy-2'-fluorouridine-3'-phosphate
  modified_base 10: mod_base = OTHER; note = 2'-O-methyladenosine-3'-phosphate
  modified_base 11: mod_base = OTHER; note = 2'-O-methyladenosine-3'-phosphate
  modified_base 12: mod_base = OTHER; note = 2'-O-methyluridine-3'-phosphate
  modified_base 13: mod_base = OTHER; note = 2'-O-methyladenosine-3'-phosphate
  modified_base 14: mod_base = OTHER; note = 2'-deoxy-2'-fluorouridine-3'-phosphate
  modified_base 15: mod_base = OTHER; note = 2'-O-methylcytidine-3'-phosphate
  modified_base 16: mod_base = OTHER; note = 2'-deoxy-2'-fluorouridine-3'-phosphate
  modified_base 17: mod_base = OTHER; note = 2'-O-methyluridine-3'-phosphate
  modified_base 18: mod_base = OTHER; note = 2'-O-methylguanosine-3'-phosphate
  modified_base 19: mod_base = OTHER; note = 2'-O-methylguanosine-3'-phosphate
  modified_base 20: mod_base = OTHER; note = 2'-O-methyladenosine-3'-phosphate
  modified_base 21: mod_base = OTHER; note = 2'-O-methylguanosine-3'-phosphorothioate
  modified_base 22: mod_base = OTHER; note = 2'-O-methyladenosine-3'-phosphorothioate
  modified_base 23: mod_base = OTHER; note = 2'-O-methyluridine
aaattccataatatcttggagat

SEQ ID NO: 506 - RNA, 23 nt, synthetic construct
  source 1..23: mol_type = other RNA
  modified_base 1: mod_base = OTHER; note = 2'-O-methyladenosine-3'-phosphorothioate
  modified_base 2: mod_base = OTHER; note = 2'-deoxy-2'-fluoroadenosine-3'-phosphorothioate
  modified_base 3: mod_base = OTHER; note = 2'-O-methyladenosine-3'-phosphate
  modified_base 4: mod_base = OTHER; note = 2'-O-methylguanosine-3'-phosphate
  modified_base 5: mod_base = OTHER; note = 2'-O-methyladenosine-3'-phosphate
  modified_base 6: mod_base = OTHER; note = 2'-deoxy-2'-fluoroadenosine-3'-phosphate
  modified_base 7: mod_base = OTHER; note = 2'-O-methyluridine-3'-phosphate
  modified_base 8: mod_base = OTHER; note = 2'-deoxy-2'-fluorocytidine-3'-phosphate
  modified_base 9: mod_base = OTHER; note = 2'-deoxy-2'-fluorouridine-3'-phosphate
  modified_base 10: mod_base = OTHER; note = 2'-O-methyladenosine-3'-phosphate
  modified_base 11: mod_base = OTHER; note = 2'-O-methyluridine-3'-phosphate
  modified_base 12: mod_base = OTHER; note = 2'-O-methylguanosine-3'-phosphate
  modified_base 13: mod_base = OTHER; note = 2'-O-methyluridine-3'-phosphate
  modified_base 14: mod_base = OTHER; note = 2'-deoxy-2'-fluoroadenosine-3'-phosphate
  modified_base 15: mod_base = OTHER; note = 2'-O-methyladenosine-3'-phosphate
  modified_base 16: mod_base = OTHER; note = 2'-deoxy-2'-fluorocytidine-3'-phosphate
  modified_base 17: mod_base = OTHER; note = 2'-O-methyladenosine-3'-phosphate
  modified_base 18: mod_base = OTHER; note = 2'-O-methylcytidine-3'-phosphate
  modified_base 19: mod_base = OTHER; note = 2'-O-methyluridine-3'-phosphate
  modified_base 20: mod_base = OTHER; note = 2'-O-methylcytidine-3'-phosphate
  modified_base 21: mod_base = OTHER; note = 2'-O-methyladenosine-3'-phosphorothioate
  modified_base 22: mod_base = OTHER; note = 2'-O-methyluridine-3'-phosphorothioate
  modified_base 23: mod_base = OTHER; note = 2'-O-methylcytidine
aaagaatctatgtaacactcatc

SEQ ID NO: 507 - RNA, 23 nt, synthetic construct
  source 1..23: mol_type = other RNA
  modified_base 1: mod_base = OTHER; note = 2'-O-methyladenosine-3'-phosphorothioate
  modified_base 2: mod_base = OTHER; note = 2'-deoxy-2'-fluorocytidine-3'-phosphorothioate
  modified_base 3: mod_base = OTHER; note = 2'-O-methyladenosine-3'-phosphate
  modified_base 4: mod_base = OTHER; note = 2'-O-methyladenosine-3'-phosphate
  modified_base 5: mod_base = OTHER; note = 2'-O-methyladenosine-3'-phosphate
  modified_base 6: mod_base = OTHER; note = 2'-deoxy-2'-fluorocytidine-3'-phosphate
  modified_base 7: mod_base = OTHER; note = 2'-O-methyluridine-3'-phosphate
  modified_base 8: mod_base = OTHER; note = 2'-deoxy-2'-fluorouridine-3'-phosphate
  modified_base 9: mod_base = OTHER; note = 2'-deoxy-2'-fluoroadenosine-3'-phosphate
  modified_base 10: mod_base = OTHER; note = 2'-O-methyladenosine-3'-phosphate
  modified_base 11: mod_base = OTHER; note = 2'-O-methyluridine-3'-phosphate
  modified_base 12: mod_base = OTHER; note = 2'-O-methyluridine-3'-phosphate
  modified_base 13: mod_base = OTHER; note = 2'-O-methylcytidine-3'-phosphate
  modified_base 14: mod_base = OTHER; note = 2'-deoxy-2'-fluorouridine-3'-phosphate
  modified_base 15: mod_base = OTHER; note = 2'-O-methylcytidine-3'-phosphate
  modified_base 16: mod_base = OTHER; note = 2'-deoxy-2'-fluoroadenosine-3'-phosphate
  modified_base 17: mod_base = OTHER; note = 2'-O-methylguanosine-3'-phosphate
  modified_base 18: mod_base = OTHER; note = 2'-O-methyluridine-3'-phosphate
  modified_base 19: mod_base = OTHER; note = 2'-O-methyladenosine-3'-phosphate
  modified_base 20: mod_base = OTHER; note = 2'-O-methylcytidine-3'-phosphate
  modified_base 21: mod_base = OTHER; note = 2'-O-methyluridine-3'-phosphorothioate
  modified_base 22: mod_base = OTHER; note = 2'-O-methyluridine-3'-phosphorothioate
  modified_base 23: mod_base = OTHER; note = 2'-O-methyluridine
acaaacttaattctcagtacttt

SEQ ID NO: 508 - RNA, 23 nt, synthetic construct
  source 1..23: mol_type = other RNA
  modified_base 1: mod_base = OTHER; note = 2'-O-methyladenosine-3'-phosphorothioate
  modified_base 2: mod_base = OTHER; note = 2'-deoxy-2'-fluoroadenosine-3'-phosphorothioate
  modified_base 3: mod_base = OTHER; note = 2'-O-methyluridine-3'-phosphate
  modified_base 4: mod_base = OTHER; note = 2'-O-methyladenosine-3'-phosphate
  modified_base 5: mod_base = OTHER; note = 2'-O-methylcytidine-3'-phosphate
  modified_base 6: mod_base = OTHER; note = 2'-deoxy-2'-fluorouridine-3'-phosphate
  modified_base 7: mod_base = OTHER; note = 2'-O-methyladenosine-3'-phosphate
  modified_base 8: mod_base = OTHER; note = 2'-deoxy-2'-fluorouridine-3'-phosphate
  modified_base 9: mod_base = OTHER; note = 2'-deoxy-2'-fluorocytidine-3'-phosphate
  modified_base 10: mod_base = OTHER; note = 2'-O-methyladenosine-3'-phosphate
  modified_base 11: mod_base = OTHER; note = 2'-O-methylguanosine-3'-phosphate
  modified_base 12: mod_base = OTHER; note = 2'-O-methyluridine-3'-phosphate
  modified_base 13: mod_base = OTHER; note = 2'-O-methylguanosine-3'-phosphate
  modified_base 14: mod_base = OTHER; note = 2'-deoxy-2'-fluorouridine-3'-phosphate
  modified_base 15: mod_base = OTHER; note = 2'-O-methyluridine-3'-phosphate
  modified_base 16: mod_base = OTHER; note = 2'-deoxy-2'-fluorouridine-3'-phosphate
  modified_base 17: mod_base = OTHER; note = 2'-O-methyladenosine-3'-phosphate
  modified_base 18: mod_base = OTHER; note = 2'-O-methyladenosine-3'-phosphate
  modified_base 19: mod_base = OTHER; note = 2'-O-methyladenosine-3'-phosphate
  modified_base 20: mod_base = OTHER; note = 2'-O-methyladenosine-3'-phosphate
  modified_base 21: mod_base = OTHER; note = 2'-O-methyluridine-3'-phosphorothioate
  modified_base 22: mod_base = OTHER; note = 2'-O-methylcytidine-3'-phosphorothioate
  modified_base 23: mod_base = OTHER; note = 2'-O-methylcytidine
aatactatcagtgtttaaaatcc

SEQ ID NO: 509 - RNA, 23 nt, synthetic construct
  source 1..23: mol_type = other RNA
  modified_base 1: mod_base = OTHER; note = 2'-O-methyladenosine-3'-phosphorothioate
  modified_base 2: mod_base = OTHER; note = 2'-deoxy-2'-fluoroadenosine-3'-phosphorothioate
  modified_base 3: mod_base = OTHER; note = 2'-O-methyladenosine-3'-phosphate
  modified_base 4: mod_base = OTHER; note = 2'-O-methyladenosine-3'-phosphate
  modified_base 5: mod_base = OTHER; note = 2'-O-methylcytidine-3'-phosphate
  modified_base 6: mod_base = OTHER; note = 2'-deoxy-2'-fluoroadenosine-3'-phosphate
  modified_base 7: mod_base = OTHER; note = 2'-O-methylcytidine-3'-phosphate
  modified_base 8: mod_base = OTHER; note = 2'-deoxy-2'-fluoroadenosine-3'-phosphate
  modified_base 9: mod_base = OTHER; note = 2'-deoxy-2'-fluorocytidine-3'-phosphate
  modified_base 10: mod_base = OTHER; note = 2'-O-methyladenosine-3'-phosphate
  modified_base 11: mod_base = OTHER; note = 2'-O-methyluridine-3'-phosphate
  modified_base 12: mod_base = OTHER; note = 2'-O-methyluridine-3'-phosphate
  modified_base 13: mod_base = OTHER; note = 2'-O-methyladenosine-3'-phosphate
  modified_base 14: mod_base = OTHER; note = 2'-deoxy-2'-fluorocytidine-3'-phosphate
  modified_base 15: mod_base = OTHER; note = 2'-O-methyluridine-3'-phosphate
  modified_base 16: mod_base = OTHER; note = 2'-deoxy-2'-fluorocytidine-3'-phosphate
  modified_base 17: mod_base = OTHER; note = 2'-O-methyladenosine-3'-phosphate
  modified_base 18: mod_base = OTHER; note = 2'-O-methyluridine-3'-phosphate
  modified_base 19: mod_base = OTHER; note = 2'-O-methylguanosine-3'-phosphate
  modified_base 20: mod_base = OTHER; note = 2'-O-methyladenosine-3'-phosphate
  modified_base 21: mod_base = OTHER; note = 2'-O-methylguanosine-3'-phosphorothioate
  modified_base 22: mod_base = OTHER; note = 2'-O-methyladenosine-3'-phosphorothioate
  modified_base 23: mod_base = OTHER; note = 2'-O-methyluridine
aaaacacacattactcatgagat

SEQ ID NO: 510 - RNA, 23 nt, synthetic construct
  source 1..23: mol_type = other RNA
  modified_base 1: mod_base = OTHER; note = 2'-O-methyladenosine-3'-phosphorothioate
  modified_base 2: mod_base = OTHER; note = 2'-deoxy-2'-fluorouridine-3'-phosphorothioate
  modified_base 3: mod_base = OTHER; note = 2'-O-methylguanosine-3'-phosphate
  modified_base 4: mod_base = OTHER; note = 2'-O-methyluridine-3'-phosphate
  modified_base 5: mod_base = OTHER; note = 2'-O-methylguanosine-3'-phosphate
  modified_base 6: mod_base = OTHER; note = 2'-deoxy-2'-fluoroadenosine-3'-phosphate
  modified_base 7: mod_base = OTHER; note = 2'-O-methyladenosine-3'-phosphate
  modified_base 8: mod_base = OTHER; note = 2'-deoxy-2'-fluoroadenosine-3'-phosphate
  modified_base 9: mod_base = OTHER; note = 2'-deoxy-2'-fluorouridine-3'-phosphate
  modified_base 10: mod_base = OTHER; note = 2'-O-methyladenosine-3'-phosphate
  modified_base 11: mod_base = OTHER; note = 2'-O-methyluridine-3'-phosphate
  modified_base 12: mod_base = OTHER; note = 2'-O-methylcytidine-3'-phosphate
  modified_base 13: mod_base = OTHER; note = 2'-O-methyladenosine-3'-phosphate
  modified_base 14: mod_base = OTHER; note = 2'-deoxy-2'-fluoroadenosine-3'-phosphate
  modified_base 15: mod_base = OTHER; note = 2'-O-methyluridine-3'-phosphate
  modified_base 16: mod_base = OTHER; note = 2'-deoxy-2'-fluorocytidine-3'-phosphate
  modified_base 17: mod_base = OTHER; note = 2'-O-methyladenosine-3'-phosphate
  modified_base 18: mod_base = OTHER; note = 2'-O-methylguanosine-3'-phosphate
  modified_base 19: mod_base = OTHER; note = 2'-O-methylcytidine-3'-phosphate
  modified_base 20: mod_base = OTHER; note = 2'-O-methyladenosine-3'-phosphate
  modified_base 21: mod_base = OTHER; note = 2'-O-methyluridine-3'-phosphorothioate
  modified_base 22: mod_base = OTHER; note = 2'-O-methylcytidine-3'-phosphorothioate
  modified_base 23: mod_base = OTHER; note = 2'-O-methylcytidine
atgtgaaatatcaatcagcatcc

SEQ ID NO: 511 - RNA, 23 nt, synthetic construct
  source 1..23: mol_type = other RNA
  modified_base 1: mod_base = OTHER; note = 2'-O-methyladenosine-3'-phosphorothioate
  modified_base 2: mod_base = OTHER; note = 2'-deoxy-2'-fluorouridine-3'-phosphorothioate
  modified_base 3: mod_base = OTHER; note = 2'-O-methyluridine-3'-phosphate
  modified_base 4: mod_base = OTHER; note = 2'-O-methylcytidine-3'-phosphate
  modified_base 5: mod_base = OTHER; note = 2'-O-methyladenosine-3'-phosphate
  modified_base 6: mod_base = OTHER; note = 2'-deoxy-2'-fluoroadenosine-3'-phosphate
  modified_base 7: mod_base = OTHER; note = 2'-O-methyladenosine-3'-phosphate
  modified_base 8: mod_base = OTHER; note = 2'-deoxy-2'-fluorocytidine-3'-phosphate
  modified_base 9: mod_base = OTHER; note = 2'-deoxy-2'-fluoroadenosine-3'-phosphate
  modified_base 10: mod_base = OTHER; note = 2'-O-methyluridine-3'-phosphate
  modified_base 11: mod_base = OTHER; note = 2'-O-methylguanosine-3'-phosphate
  modified_base 12: mod_base = OTHER; note = 2'-O-methylguanosine-3'-phosphate
  modified_base 13: mod_base = OTHER; note = 2'-O-methyluridine-3'-phosphate
  modified_base 14: mod_base = OTHER; note = 2'-deoxy-2'-fluoroadenosine-3'-phosphate
  modified_base 15: mod_base = OTHER; note = 2'-O-methyluridine-3'-phosphate
  modified_base 16: mod_base = OTHER; note = 2'-deoxy-2'-fluorouridine-3'-phosphate
  modified_base 17: mod_base = OTHER; note = 2'-O-methyluridine-3'-phosphate
  modified_base 18: mod_base = OTHER; note = 2'-O-methylcytidine-3'-phosphate
  modified_base 19: mod_base = OTHER; note = 2'-O-methyladenosine-3'-phosphate
  modified_base 20: mod_base = OTHER; note = 2'-O-methyluridine-3'-phosphate
  modified_base 21: mod_base = OTHER; note = 2'-O-methyladenosine-3'-phosphorothioate
  modified_base 22: mod_base = OTHER; note = 2'-O-methylcytidine-3'-phosphorothioate
  modified_base 23: mod_base = OTHER; note = 2'-O-methyladenosine
attcaaacatggtatttcataca

SEQ ID NO: 512 - RNA, 23 nt, synthetic construct
  source 1..23: mol_type = other RNA
  modified_base 1: mod_base = OTHER; note = 2'-O-methyladenosine-3'-phosphorothioate
  modified_base 2: mod_base = OTHER; note = 2'-deoxy-2'-fluoroadenosine-3'-phosphorothioate
  modified_base 3: mod_base = OTHER; note = 2'-O-methyluridine-3'-phosphate
  modified_base 4: mod_base = OTHER; note = 2'-O-methyluridine-3'-phosphate
  modified_base 5: mod_base = OTHER; note = 2'-O-methyladenosine-3'-phosphate
  modified_base 6: mod_base = OTHER; note = 2'-deoxy-2'-fluorouridine-3'-phosphate
  modified_base 7: mod_base = OTHER; note = 2'-O-methyluridine-3'-phosphate
  modified_base 8: mod_base = OTHER; note = 2'-deoxy-2'-fluoroguanosine-3'-phosphate
  modified_base 9: mod_base = OTHER; note = 2'-deoxy-2'-fluorocytidine-3'-phosphate
  modified_base 10: mod_base = OTHER; note = 2'-O-methyluridine-3'-phosphate
  modified_base 11: mod_base = OTHER; note = 2'-O-methyladenosine-3'-phosphate
  modified_base 12: mod_base = OTHER; note = 2'-O-methyluridine-3'-phosphate
  modified_base 13: mod_base = OTHER; note = 2'-O-methylguanosine-3'-phosphate
  modified_base 14: mod_base = OTHER; note = 2'-deoxy-2'-fluoroadenosine-3'-phosphate
  modified_base 15: mod_base = OTHER; note = 2'-O-methylguanosine-3'-phosphate
  modified_base 16: mod_base = OTHER; note = 2'-deoxy-2'-fluorouridine-3'-phosphate
  modified_base 17: mod_base = OTHER; note = 2'-O-methyluridine-3'-phosphate
  modified_base 18: mod_base = OTHER; note = 2'-O-methyluridine-3'-phosphate
  modified_base 19: mod_base = OTHER; note = 2'-O-methylcytidine-3'-phosphate
  modified_base 20: mod_base = OTHER; note = 2'-O-methyladenosine-3'-phosphate
  modified_base 21: mod_base = OTHER; note = 2'-O-methyladenosine-3'-phosphorothioate
  modified_base 22: mod_base = OTHER; note = 2'-O-methyladenosine-3'-phosphorothioate
  modified_base 23: mod_base = OTHER; note = 2'-O-methylcytidine
aattattgctatgagtttcaaac

SEQ ID NO: 513 - RNA, 23 nt, synthetic construct
  source 1..23: mol_type = other RNA
  modified_base 1: mod_base = OTHER; note = 2'-O-methyladenosine-3'-phosphorothioate
  modified_base 2: mod_base = OTHER; note = 2'-deoxy-2'-fluoroadenosine-3'-phosphorothioate
  modified_base 3: mod_base = OTHER; note = 2'-O-methyluridine-3'-phosphate
  modified_base 4: mod_base = OTHER; note = 2'-O-methylcytidine-3'-phosphate
  modified_base 5: mod_base = OTHER; note = 2'-O-methyladenosine-3'-phosphate
  modified_base 6: mod_base = OTHER; note = 2'-deoxy-2'-fluorocytidine-3'-phosphate
  modified_base 7: mod_base = OTHER; note = 2'-O-methyladenosine-3'-phosphate
  modified_base 8: mod_base = OTHER; note = 2'-deoxy-2'-fluoroadenosine-3'-phosphate
  modified_base 9: mod_base = OTHER; note = 2'-deoxy-2'-fluorocytidine-3'-phosphate
  modified_base 10: mod_base = OTHER; note = 2'-O-methyladenosine-3'-phosphate
  modified_base 11: mod_base = OTHER; note = 2'-O-methylguanosine-3'-phosphate
  modified_base 12: mod_base = OTHER; note = 2'-O-methylcytidine-3'-phosphate
  modified_base 13: mod_base = OTHER; note = 2'-O-methyladenosine-3'-phosphate
  modified_base 14: mod_base = OTHER; note = 2'-deoxy-2'-fluorouridine-3'-phosphate
  modified_base 15: mod_base = OTHER; note = 2'-O-methyladenosine-3'-phosphate
  modified_base 16: mod_base = OTHER; note = 2'-deoxy-2'-fluoroguanosine-3'-phosphate
  modified_base 17: mod_base = OTHER; note = 2'-O-methylcytidine-3'-phosphate
  modified_base 18: mod_base = OTHER; note = 2'-O-methyladenosine-3'-phosphate
  modified_base 19: mod_base = OTHER; note = 2'-O-methyluridine-3'-phosphate
  modified_base 20: mod_base = OTHER; note = 2'-O-methyluridine-3'-phosphate
  modified_base 21: mod_base = OTHER; note = 2'-O-methyladenosine-3'-phosphorothioate
  modified_base 22: mod_base = OTHER; note = 2'-O-methyluridine-3'-phosphorothioate
  modified_base 23: mod_base = OTHER; note = 2'-O-methyluridine
aatcacaacagcatagcattatt

SEQ ID NO: 514 - RNA, 23 nt, synthetic construct
  source 1..23: mol_type = other RNA
  modified_base 1: mod_base = OTHER; note = 2'-O-methyladenosine-3'-phosphorothioate
  modified_base 2: mod_base = OTHER; note = 2'-deoxy-2'-fluorouridine-3'-phosphorothioate
  modified_base 3: mod_base = OTHER; note = 2'-O-methyladenosine-3'-phosphate
  modified_base 4: mod_base = OTHER; note = 2'-O-methyluridine-3'-phosphate
  modified_base 5: mod_base = OTHER; note = 2'-O-methyluridine-3'-phosphate
  modified_base 6: mod_base = OTHER; note = 2'-deoxy-2'-fluorouridine-3'-phosphate
  modified_base 7: mod_base = OTHER; note = 2'-O-methyluridine-3'-phosphate
  modified_base 8: mod_base = OTHER; note = 2'-deoxy-2'-fluoroadenosine-3'-phosphate
  modified_base 9: mod_base = OTHER; note = 2'-deoxy-2'-fluoroadenosine-3'-phosphate
  modified_base 10: mod_base = OTHER; note = 2'-O-methyladenosine-3'-phosphate
  modified_base 11: mod_base = OTHER; note = 2'-O-methyluridine-3'-phosphate
  modified_base 12: mod_base = OTHER; note = 2'-O-methylguanosine-3'-phosphate
  modified_base 13: mod_base = OTHER; note = 2'-O-methylcytidine-3'-phosphate
  modified_base 14: mod_base = OTHER; note = 2'-deoxy-2'-fluoroadenosine-3'-phosphate
  modified_base 15: mod_base = OTHER; note = 2'-O-methylguanosine-3'-phosphate
  modified_base 16: mod_base = OTHER; note = 2'-deoxy-2'-fluoroadenosine-3'-phosphate
  modified_base 17: mod_base = OTHER; note = 2'-O-methyladenosine-3'-phosphate
  modified_base 18: mod_base = OTHER; note = 2'-O-methylcytidine-3'-phosphate
  modified_base 19: mod_base = OTHER; note = 2'-O-methyluridine-3'-phosphate
  modified_base 20: mod_base = OTHER; note = 2'-O-methyluridine-3'-phosphate
  modified_base 21: mod_base = OTHER; note = 2'-O-methylguanosine-3'-phosphorothioate
  modified_base 22: mod_base = OTHER; note = 2'-O-methyladenosine-3'-phosphorothioate
  modified_base 23: mod_base = OTHER; note = 2'-O-methylguanosine
atattttaaatgcagaacttgag

SEQ ID NO: 515 - RNA, 23 nt, synthetic construct
  source 1..23: mol_type = other RNA
  modified_base 1: mod_base = OTHER; note = 2'-O-methyladenosine-3'-phosphorothioate
  modified_base 2: mod_base = OTHER; note = 2'-deoxy-2'-fluoroadenosine-3'-phosphorothioate
  modified_base 3: mod_base = OTHER; note = 2'-O-methyluridine-3'-phosphate
  modified_base 4: mod_base = OTHER; note = 2'-O-methylguanosine-3'-phosphate
  modified_base 5: mod_base = OTHER; note = 2'-O-methyladenosine-3'-phosphate
  modified_base 6: mod_base = OTHER; note = 2'-deoxy-2'-fluorocytidine-3'-phosphate
  modified_base 7: mod_base = OTHER; note = 2'-O-methyluridine-3'-phosphate
  modified_base 8: mod_base = OTHER; note = 2'-deoxy-2'-fluorouridine-3'-phosphate
  modified_base 9: mod_base = OTHER; note = 2'-deoxy-2'-fluorocytidine-3'-phosphate
  modified_base 10: mod_base = OTHER; note = 2'-O-methyladenosine-3'-phosphate
  modified_base 11: mod_base = OTHER; note = 2'-O-methyluridine-3'-phosphate
  modified_base 12: mod_base = OTHER; note = 2'-O-methylguanosine-3'-phosphate
  modified_base 13: mod_base = OTHER; note = 2'-O-methylguanosine-3'-phosphate
  modified_base 14: mod_base = OTHER; note = 2'-deoxy-2'-fluorouridine-3'-phosphate
  modified_base 15: mod_base = OTHER; note = 2'-O-methyladenosine-3'-phosphate
  modified_base 16: mod_base = OTHER; note = 2'-deoxy-2'-fluorouridine-3'-phosphate
  modified_base 17: mod_base = OTHER; note = 2'-O-methyladenosine-3'-phosphate
  modified_base 18: mod_base = OTHER; note = 2'-O-methylcytidine-3'-phosphate
  modified_base 19: mod_base = OTHER; note = 2'-O-methyladenosine-3'-phosphate
  modified_base 20: mod_base = OTHER; note = 2'-O-methyluridine-3'-phosphate
  modified_base 21: mod_base = OTHER; note = 2'-O-methylcytidine-3'-phosphorothioate
  modified_base 22: mod_base = OTHER; note = 2'-O-methyladenosine-3'-phosphorothioate
  modified_base 23: mod_base = OTHER; note = 2'-O-methyladenosine
aatgacttcatggtatacatcaa

SEQ ID NO: 516 - RNA, 23 nt, synthetic construct
  source 1..23: mol_type = other RNA
  modified_base 1: mod_base = OTHER; note = 2'-O-methyladenosine-3'-phosphorothioate
  modified_base 2: mod_base = OTHER; note = 2'-deoxy-2'-fluoroadenosine-3'-phosphorothioate
  modified_base 3: mod_base = OTHER; note = 2'-O-methyladenosine-3'-phosphate
  modified_base 4: mod_base = OTHER; note = 2'-O-methylcytidine-3'-phosphate
  modified_base 5: mod_base = OTHER; note = 2'-O-methyladenosine-3'-phosphate
  modified_base 6: mod_base = OTHER; note = 2'-deoxy-2'-fluorouridine-3'-phosphate
  modified_base 7: mod_base = OTHER; note = 2'-O-methylcytidine-3'-phosphate
  modified_base 8: mod_base = OTHER; note = 2'-deoxy-2'-fluoroadenosine-3'-phosphate
  modified_base 9: mod_base = OTHER; note = 2'-deoxy-2'-fluoroguanosine-3'-phosphate
  modified_base 10: mod_base = OTHER; note = 2'-O-methyladenosine-3'-phosphate
  modified_base 11: mod_base = OTHER; note = 2'-O-methylguanosine-3'-phosphate
  modified_base 12: mod_base = OTHER; note = 2'-O-methylcytidine-3'-phosphate
  modified_base 13: mod_base = OTHER; note = 2'-O-methyluridine-3'-phosphate
  modified_base 14: mod_base = OTHER; note = 2'-deoxy-2'-fluoroadenosine-3'-phosphate
  modified_base 15: mod_base = OTHER; note = 2'-O-methylcytidine-3'-phosphate
  modified_base 16: mod_base = OTHER; note = 2'-deoxy-2'-fluorouridine-3'-phosphate
  modified_base 17: mod_base = OTHER; note = 2'-O-methyladenosine-3'-phosphate
  modified_base 18: mod_base = OTHER; note = 2'-O-methylcytidine-3'-phosphate
  modified_base 19: mod_base = OTHER; note = 2'-O-methyladenosine-3'-phosphate
  modified_base 20: mod_base = OTHER; note = 2'-O-methyladenosine-3'-phosphate
  modified_base 21: mod_base = OTHER; note = 2'-O-methylcytidine-3'-phosphorothioate
  modified_base 22: mod_base = OTHER; note = 2'-O-methyluridine-3'-phosphorothioate
  modified_base 23: mod_base = OTHER; note = 2'-O-methylguanosine
aaacatcagagctactacaactg

SEQ ID NO: 517 - RNA, 23 nt, synthetic construct
  source 1..23: mol_type = other RNA
  modified_base 1: mod_base = OTHER; note = 2'-O-methyladenosine-3'-phosphorothioate
  modified_base 2: mod_base = OTHER; note = 2'-deoxy-2'-fluoroadenosine-3'-phosphorothioate
  modified_base 3: mod_base = OTHER; note = 2'-O-methyladenosine-3'-phosphate
  modified_base 4: mod_base = OTHER; note = 2'-O-methyladenosine-3'-phosphate
  modified_base 5: mod_base = OTHER; note = 2'-O-methyladenosine-3'-phosphate
  modified_base 6: mod_base = OTHER; note = 2'-deoxy-2'-fluorocytidine-3'-phosphate
  modified_base 7: mod_base = OTHER; note = 2'-O-methyladenosine-3'-phosphate
  modified_base 8: mod_base = OTHER; note = 2'-deoxy-2'-fluorouridine-3'-phosphate
  modified_base 9: mod_base = OTHER; note = 2'-deoxy-2'-fluoroguanosine-3'-phosphate
  modified_base 10: mod_base = OTHER; note = 2'-O-methyladenosine-3'-phosphate
  modified_base 11: mod_base = OTHER; note = 2'-O-methyluridine-3'-phosphate
  modified_base 12: mod_base = OTHER; note = 2'-O-methyladenosine-3'-phosphate
  modified_base 13: mod_base = OTHER; note = 2'-O-methyluridine-3'-phosphate
  modified_base 14: mod_base = OTHER; note = 2'-deoxy-2'-fluorocytidine-3'-phosphate
  modified_base 15: mod_base = OTHER; note = 2'-O-methyluridine-3'-phosphate
  modified_base 16: mod_base = OTHER; note = 2'-deoxy-2'-fluorocytidine-3'-phosphate
  modified_base 17: mod_base = OTHER; note = 2'-O-methyladenosine-3'-phosphate
  modified_base 18: mod_base = OTHER; note = 2'-O-methyluridine-3'-phosphate
  modified_base 19: mod_base = OTHER; note = 2'-O-methyluridine-3'-phosphate
  modified_base 20: mod_base = OTHER; note = 2'-O-methylcytidine-3'-phosphate
  modified_base 21: mod_base = OTHER; note = 2'-O-methyladenosine-3'-phosphorothioate
  modified_base 22: mod_base = OTHER; note = 2'-O-methyladenosine-3'-phosphorothioate
  modified_base 23: mod_base = OTHER; note = 2'-O-methylcytidine
aaaaacatgatatctcattcaac

SEQ ID NO: 518 - RNA, 23 nt, synthetic construct
  source 1..23: mol_type = other RNA
  modified_base 1: mod_base = OTHER; note = 2'-O-methyladenosine-3'-phosphorothioate
  modified_base 2: mod_base = OTHER; note = 2'-deoxy-2'-fluoroadenosine-3'-phosphorothioate
  modified_base 3: mod_base = OTHER; note = 2'-O-methylguanosine-3'-phosphate
  modified_base 4: mod_base = OTHER; note = 2'-O-methyluridine-3'-phosphate
  modified_base 5: mod_base = OTHER; note = 2'-O-methyladenosine-3'-phosphate
  modified_base 6: mod_base = OTHER; note = 2'-deoxy-2'-fluoroadenosine-3'-phosphate
  modified_base 7: mod_base = OTHER; note = 2'-O-methyladenosine-3'-phosphate
  modified_base 8: mod_base = OTHER; note = 2'-deoxy-2'-fluoroadenosine-3'-phosphate
  modified_base 9: mod_base = OTHER; note = 2'-deoxy-2'-fluorouridine-3'-phosphate
  modified_base 10: mod_base = OTHER; note = 2'-O-methylguanosine-3'-phosphate
  modified_base 11: mod_base = OTHER; note = 2'-O-methylguanosine-3'-phosphate
  modified_base 12: mod_base = OTHER; note = 2'-O-methyladenosine-3'-phosphate
  modified_base 13: mod_base = OTHER; note = 2'-O-methyladenosine-3'-phosphate
  modified_base 14: mod_base = OTHER; note = 2'-deoxy-2'-fluorouridine-3'-phosphate
  modified_base 15: mod_base = OTHER; note = 2'-O-methylguanosine-3'-phosphate
  modified_base 16: mod_base = OTHER; note = 2'-deoxy-2'-fluorocytidine-3'-phosphate
  modified_base 17: mod_base = OTHER; note = 2'-O-methyluridine-3'-phosphate
  modified_base 18: mod_base = OTHER; note = 2'-O-methyladenosine-3'-phosphate
  modified_base 19: mod_base = OTHER; note = 2'-O-methyladenosine-3'-phosphate
  modified_base 20: mod_base = OTHER; note = 2'-O-methyladenosine-3'-phosphate
  modified_base 21: mod_base = OTHER; note = 2'-O-methyladenosine-3'-phosphorothioate
  modified_base 22: mod_base = OTHER; note = 2'-O-methylcytidine-3'-phosphorothioate
  modified_base 23: mod_base = OTHER; note = 2'-O-methyladenosine
aagtaaaatggaatgctaaaaca

SEQ ID NO: 519 - RNA, 23 nt, synthetic construct
  source 1..23: mol_type = other RNA
  modified_base 1: mod_base = OTHER; note = 2'-O-methyladenosine-3'-phosphorothioate
  modified_base 2: mod_base = OTHER; note = 2'-deoxy-2'-fluorocytidine-3'-phosphorothioate
  modified_base 3: mod_base = OTHER; note = 2'-O-methyluridine-3'-phosphate
  modified_base 4: mod_base = OTHER; note = 2'-O-methyluridine-3'-phosphate
  modified_base 5: mod_base = OTHER; note = 2'-O-methylguanosine-3'-phosphate
  modified_base 6: mod_base = OTHER; note = 2'-deoxy-2'-fluoroadenosine-3'-phosphate
  modified_base 7: mod_base = OTHER; note = 2'-O-methylguanosine-3'-phosphate
  modified_base 8: mod_base = OTHER; note = 2'-deoxy-2'-fluorouridine-3'-phosphate
  modified_base 9: mod_base = OTHER; note = 2'-deoxy-2'-fluoroadenosine-3'-phosphate
  modified_base 10: mod_base = OTHER; note = 2'-O-methyladenosine-3'-phosphate
  modified_base 11: mod_base = OTHER; note = 2'-O-methyluridine-3'-phosphate
  modified_base 12: mod_base = OTHER; note = 2'-O-methylcytidine-3'-phosphate
  modified_base 13: mod_base = OTHER; note = 2'-O-methylcytidine-3'-phosphate
  modified_base 14: mod_base = OTHER; note = 2'-deoxy-2'-fluorouridine-3'-phosphate
  modified_base 15: mod_base = OTHER; note = 2'-O-methyluridine-3'-phosphate
  modified_base 16: mod_base = OTHER; note = 2'-deoxy-2'-fluoroadenosine-3'-phosphate
  modified_base 17: mod_base = OTHER; note = 2'-O-methyladenosine-3'-phosphate
  modified_base 18: mod_base = OTHER; note = 2'-O-methyluridine-3'-phosphate
  modified_base 19: mod_base = OTHER; note = 2'-O-methyluridine-3'-phosphate
  modified_base 20: mod_base = OTHER; note = 2'-O-methyluridine-3'-phosphate
  modified_base 21: mod_base = OTHER; note = 2'-O-methyladenosine-3'-phosphorothioate
  modified_base 22: mod_base = OTHER; note = 2'-O-methylcytidine-3'-phosphorothioate
  modified_base 23: mod_base = OTHER; note = 2'-O-methyladenosine
acttgagtaatccttaatttaca

SEQ ID NO: 520 - RNA, 23 nt, synthetic construct
  source 1..23: mol_type = other RNA
  modified_base 1: mod_base = OTHER; note = 2'-O-methyladenosine-3'-phosphorothioate
  modified_base 2: mod_base = OTHER; note = 2'-deoxy-2'-fluoroadenosine-3'-phosphorothioate
  modified_base 3: mod_base = OTHER; note = 2'-O-methyladenosine-3'-phosphate
  modified_base 4: mod_base = OTHER; note = 2'-O-methyluridine-3'-phosphate
  modified_base 5: mod_base = OTHER; note = 2'-O-methylcytidine-3'-phosphate
  modified_base 6: mod_base = OTHER; note = 2'-deoxy-2'-fluorouridine-3'-phosphate
  modified_base 7: mod_base = OTHER; note = 2'-O-methyluridine-3'-phosphate
  modified_base 8: mod_base = OTHER; note = 2'-deoxy-2'-fluoroguanosine-3'-phosphate
  modified_base 9: mod_base = OTHER; note = 2'-deoxy-2'-fluoroadenosine-3'-phosphate
  modified_base 10: mod_base = OTHER; note = 2'-O-methyladenosine-3'-phosphate
  modified_base 11: mod_base = OTHER; note = 2'-O-methyluridine-3'-phosphate
  modified_base 12: mod_base = OTHER; note = 2'-O-methyladenosine-3'-phosphate
  modified_base 13: mod_base = OTHER; note = 2'-O-methyladenosine-3'-phosphate
  modified_base 14: mod_base = OTHER; note = 2'-deoxy-2'-fluorouridine-3'-phosphate
  modified_base 15: mod_base = OTHER; note = 2'-O-methylguanosine-3'-phosphate
  modified_base 16: mod_base = OTHER; note = 2'-deoxy-2'-fluoroguanosine-3'-phosphate
  modified_base 17: mod_base = OTHER; note = 2'-O-methyluridine-3'-phosphate
  modified_base 18: mod_base = OTHER; note = 2'-O-methylguanosine-3'-phosphate
  modified_base 19: mod_base = OTHER; note = 2'-O-methyladenosine-3'-phosphate
  modified_base 20: mod_base = OTHER; note = 2'-O-methylguanosine-3'-phosphate
  modified_base 21: mod_base = OTHER; note = 2'-O-methylcytidine-3'-phosphorothioate
  modified_base 22: mod_base = OTHER; note = 2'-O-methyluridine-3'-phosphorothioate
  modified_base 23: mod_base = OTHER; note = 2'-O-methyluridine
aaatcttgaataatggtgagctt

SEQ ID NO: 521 - RNA, 23 nt, synthetic construct
  source 1..23: mol_type = other RNA
  modified_base 1: mod_base = OTHER; note = 2'-O-methyladenosine-3'-phosphorothioate
  modified_base 2: mod_base = OTHER; note = 2'-deoxy-2'-fluoroadenosine-3'-phosphorothioate
  modified_base 3: mod_base = OTHER; note = 2'-O-methyladenosine-3'-phosphate
  modified_base 4: mod_base = OTHER; note = 2'-O-methyladenosine-3'-phosphate
  modified_base 5: mod_base = OTHER; note = 2'-O-methyladenosine-3'-phosphate
  modified_base 6: mod_base = OTHER; note = 2'-deoxy-2'-fluorouridine-3'-phosphate
  modified_base 7: mod_base = OTHER; note = 2'-O-methyladenosine-3'-phosphate
  modified_base 8: mod_base = OTHER; note = 2'-deoxy-2'-fluoroadenosine-3'-phosphate
  modified_base 9: mod_base = OTHER; note = 2'-deoxy-2'-fluorouridine-3'-phosphate
  modified_base 10: mod_base = OTHER; note = 2'-O-methylguanosine-3'-phosphate
  modified_base 11: mod_base = OTHER; note = 2'-O-methylcytidine-3'-phosphate
  modified_base 12: mod_base = OTHER; note = 2'-O-methyladenosine-3'-phosphate
  modified_base 13: mod_base = OTHER; note = 2'-O-methyladenosine-3'-phosphate
  modified_base 14: mod_base = OTHER; note = 2'-deoxy-2'-fluoroguanosine-3'-phosphate
  modified_base 15: mod_base = OTHER; note = 2'-O-methyladenosine-3'-phosphate
  modified_base 16: mod_base = OTHER; note = 2'-deoxy-2'-fluoroguanosine-3'-phosphate
  modified_base 17: mod_base = OTHER; note = 2'-O-methyladenosine-3'-phosphate
  modified_base 18: mod_base = OTHER; note = 2'-O-methyladenosine-3'-phosphate
  modified_base 19: mod_base = OTHER; note = 2'-O-methylguanosine-3'-phosphate
  modified_base 20: mod_base = OTHER; note = 2'-O-methylcytidine-3'-phosphate
  modified_base 21: mod_base = OTHER; note = 2'-O-methylcytidine-3'-phosphorothioate
  modified_base 22: mod_base = OTHER; note = 2'-O-methylguanosine-3'-phosphorothioate
  modified_base 23: mod_base = OTHER; note = 2'-O-methyluridine
aaaaataatgcaagagaagccgt

SEQ ID NO: 522 - RNA, 23 nt, synthetic construct
  source 1..23: mol_type = other RNA
  modified_base 1: mod_base = OTHER; note = 2'-O-methyladenosine-3'-phosphorothioate
  modified_base 2: mod_base = OTHER; note = 2'-deoxy-2'-fluorouridine-3'-phosphorothioate
  modified_base 3: mod_base = OTHER; note = 2'-O-methyladenosine-3'-phosphate
  modified_base 4: mod_base = OTHER; note = 2'-O-methylcytidine-3'-phosphate
  modified_base 5: mod_base = OTHER; note = 2'-O-methyluridine-3'-phosphate
  modified_base 6: mod_base = OTHER; note = 2'-deoxy-2'-fluorouridine-3'-phosphate
  modified_base 7: mod_base = OTHER; note = 2'-O-methylcytidine-3'-phosphate
  modified_base 8: mod_base = OTHER; note = 2'-deoxy-2'-fluorouridine-3'-phosphate
  modified_base 9: mod_base = OTHER; note = 2'-deoxy-2'-fluoroadenosine-3'-phosphate
  modified_base 10: mod_base = OTHER; note = 2'-O-methylguanosine-3'-phosphate
  modified_base 11: mod_base = OTHER; note = 2'-O-methyladenosine-3'-phosphate
  modified_base 12: mod_base = OTHER; note = 2'-O-methyladenosine-3'-phosphate
  modified_base 13: mod_base = OTHER; note = 2'-O-methyladenosine-3'-phosphate
  modified_base 14: mod_base = OTHER; note = 2'-deoxy-2'-fluoroadenosine-3'-phosphate
  modified_base 15: mod_base = OTHER; note = 2'-O-methylcytidine-3'-phosphate
  modified_base 16: mod_base = OTHER; note = 2'-deoxy-2'-fluoroadenosine-3'-phosphate
  modified_base 17: mod_base = OTHER; note = 2'-O-methyladenosine-3'-phosphate
  modified_base 18: mod_base = OTHER; note = 2'-O-methyladenosine-3'-phosphate
  modified_base 19: mod_base = OTHER; note = 2'-O-methylcytidine-3'-phosphate
  modified_base 20: mod_base = OTHER; note = 2'-O-methylcytidine-3'-phosphate
  modified_base 21: mod_base = OTHER; note = 2'-O-methyladenosine-3'-phosphorothioate
  modified_base 22: mod_base = OTHER; note = 2'-O-methyladenosine-3'-phosphorothioate
  modified_base 23: mod_base = OTHER; note = 2'-O-methylcytidine
atacttctagaaaacaaaccaac

SEQ ID NO: 523 - RNA, 23 nt, synthetic construct
  source 1..23: mol_type = other RNA
  modified_base 1: mod_base = OTHER; note = 2'-O-methyladenosine-3'-phosphorothioate
  modified_base 2: mod_base = OTHER; note = 2'-deoxy-2'-fluoroadenosine-3'-phosphorothioate
  modified_base 3: mod_base = OTHER; note = 2'-O-methyladenosine-3'-phosphate
  modified_base 4: mod_base = OTHER; note = 2'-O-methyladenosine-3'-phosphate
  modified_base 5: mod_base = OTHER; note = 2'-O-methylguanosine-3'-phosphate
  modified_base 6: mod_base = OTHER; note = 2'-deoxy-2'-fluoroadenosine-3'-phosphate
  modified_base 7: mod_base = OTHER; note = 2'-O-methyluridine-3'-phosphate
  modified_base 8: mod_base = OTHER; note = 2'-deoxy-2'-fluorouridine-3'-phosphate
  modified_base 9: mod_base = OTHER; note = 2'-deoxy-2'-fluorouridine-3'-phosphate
  modified_base 10: mod_base = OTHER; note = 2'-O-methyluridine-3'-phosphate
  modified_base 11: mod_base = OTHER; note = 2'-O-methylcytidine-3'-phosphate
  modified_base 12: mod_base = OTHER; note = 2'-O-methyladenosine-3'-phosphate
  modified_base 13: mod_base = OTHER; note = 2'-O-methyladenosine-3'-phosphate
  modified_base 14: mod_base = OTHER; note = 2'-deoxy-2'-fluoroadenosine-3'-phosphate
  modified_base 15: mod_base = OTHER; note = 2'-O-methylguanosine-3'-phosphate
  modified_base 16: mod_base = OTHER; note = 2'-deoxy-2'-fluorocytidine-3'-phosphate
  modified_base 17: mod_base = OTHER; note = 2'-O-methyladenosine-3'-phosphate
  modified_base 18: mod_base = OTHER; note = 2'-O-methylcytidine-3'-phosphate
  modified_base 19: mod_base = OTHER; note = 2'-O-methylcytidine-3'-phosphate
  modified_base 20: mod_base = OTHER; note = 2'-O-methyladenosine-3'-phosphate
  modified_base 21: mod_base = OTHER; note = 2'-O-methylguanosine-3'-phosphorothioate
  modified_base 22: mod_base = OTHER; note = 2'-O-methyluridine-3'-phosphorothioate
  modified_base 23: mod_base = OTHER; note = 2'-O-methyluridine
aaaagattttcaaagcaccagtt

SEQ ID NO: 524 - RNA, 23 nt, synthetic construct
  source 1..23: mol_type = other RNA
  modified_base 1: mod_base = OTHER; note = 2'-O-methyladenosine-3'-phosphorothioate
  modified_base 2: mod_base = OTHER; note = 2'-deoxy-2'-fluoroadenosine-3'-phosphorothioate
  modified_base 3: mod_base = OTHER; note = 2'-O-methyladenosine-3'-phosphate
  modified_base 4: mod_base = OTHER; note = 2'-O-methyladenosine-3'-phosphate
  modified_base 5: mod_base = OTHER; note = 2'-O-methyluridine-3'-phosphate
  modified_base 6: mod_base = OTHER; note = 2'-deoxy-2'-fluorouridine-3'-phosphate
  modified_base 7: mod_base = OTHER; note = 2'-O-methyladenosine-3'-phosphate
  modified_base 8: mod_base = OTHER; note = 2'-deoxy-2'-fluoroadenosine-3'-phosphate
  modified_base 9: mod_base = OTHER; note = 2'-deoxy-2'-fluorocytidine-3'-phosphate
  modified_base 10: mod_base = OTHER; note = 2'-O-methyluridine-3'-phosphate
  modified_base 11: mod_base = OTHER; note = 2'-O-methylcytidine-3'-phosphate
  modified_base 12: mod_base = OTHER; note = 2'-O-methyladenosine-3'-phosphate
  modified_base 13: mod_base = OTHER; note = 2'-O-methyladenosine-3'-phosphate
  modified_base 14: mod_base = OTHER; note = 2'-deoxy-2'-fluoroadenosine-3'-phosphate
  modified_base 15: mod_base = OTHER; note = 2'-O-methylguanosine-3'-phosphate
  modified_base 16: mod_base = OTHER; note = 2'-deoxy-2'-fluoroguanosine-3'-phosphate
  modified_base 17: mod_base = OTHER; note = 2'-O-methyluridine-3'-phosphate
  modified_base 18: mod_base = OTHER; note = 2'-O-methylcytidine-3'-phosphate
  modified_base 19: mod_base = OTHER; note = 2'-O-methyladenosine-3'-phosphate
  modified_base 20: mod_base = OTHER; note = 2'-O-methylguanosine-3'-phosphate
  modified_base 21: mod_base = OTHER; note = 2'-O-methylcytidine-3'-phosphorothioate
  modified_base 22: mod_base = OTHER; note = 2'-O-methyluridine-3'-phosphorothioate
  modified_base 23: mod_base = OTHER; note = 2'-O-methyluridine
aaaattaactcaaaggtcagctt

SEQ ID NO: 525 - RNA, 23 nt, synthetic construct
  source 1..23: mol_type = other RNA
  modified_base 1: mod_base = OTHER; note = 2'-O-methyladenosine-3'-phosphorothioate
  modified_base 2: mod_base = OTHER; note = 2'-deoxy-2'-fluoroadenosine-3'-phosphorothioate
  modified_base 3: mod_base = OTHER; note = 2'-O-methylcytidine-3'-phosphate
  modified_base 4: mod_base = OTHER; note = 2'-O-methyluridine-3'-phosphate
  modified_base 5: mod_base = OTHER; note = 2'-O-methylguanosine-3'-phosphate
  modified_base 6: mod_base = OTHER; note = 2'-deoxy-2'-fluoroadenosine-3'-phosphate
  modified_base 7: mod_base = OTHER; note = 2'-O-methyladenosine-3'-phosphate
  modified_base 8: mod_base = OTHER; note = 2'-deoxy-2'-fluoroguanosine-3'-phosphate
  modified_base 9: mod_base = OTHER; note = 2'-deoxy-2'-fluoroadenosine-3'-phosphate
  modified_base 10: mod_base = OTHER; note = 2'-O-methyladenosine-3'-phosphate
  modified_base 11: mod_base = OTHER; note = 2'-O-methyluridine-3'-phosphate
  modified_base 12: mod_base = OTHER; note = 2'-O-methylguanosine-3'-phosphate
  modified_base 13: mod_base = OTHER; note = 2'-O-methyladenosine-3'-phosphate
  modified_base 14: mod_base = OTHER; note = 2'-deoxy-2'-fluoroguanosine-3'-phosphate
  modified_base 15: mod_base = OTHER; note = 2'-O-methyluridine-3'-phosphate
  modified_base 16: mod_base = OTHER; note = 2'-deoxy-2'-fluorouridine-3'-phosphate
  modified_base 17: mod_base = OTHER; note = 2'-O-methylguanosine-3'-phosphate
  modified_base 18: mod_base = OTHER; note = 2'-O-methyluridine-3'-phosphate
  modified_base 19: mod_base = OTHER; note = 2'-O-methylguanosine-3'-phosphate
  modified_base 20: mod_base = OTHER; note = 2'-O-methylcytidine-3'-phosphate
  modified_base 21: mod_base = OTHER; note = 2'-O-methyluridine-3'-phosphorothioate
  modified_base 22: mod_base = OTHER; note = 2'-O-methylguanosine-3'-phosphorothioate
  modified_base 23: mod_base = OTHER; note = 2'-O-methyladenosine
aactgaagaatgagttgtgctga

SEQ ID NO: 526 - RNA, 23 nt, synthetic construct
  source 1..23: mol_type = other RNA
  modified_base 1: mod_base = OTHER; note = 2'-O-methyladenosine-3'-phosphorothioate
  modified_base 2: mod_base = OTHER; note = 2'-deoxy-2'-fluorouridine-3'-phosphorothioate
  modified_base 3: mod_base = OTHER; note = 2'-O-methyluridine-3'-phosphate
  modified_base 4: mod_base = OTHER; note = 2'-O-methylguanosine-3'-phosphate
  modified_base 5: mod_base = OTHER; note = 2'-O-methyluridine-3'-phosphate
  modified_base 6: mod_base = OTHER; note = 2'-deoxy-2'-fluorouridine-3'-phosphate
  modified_base 7: mod_base = OTHER; note = 2'-O-methyluridine-3'-phosphate
  modified_base 8: mod_base = OTHER; note = 2'-deoxy-2'-fluorouridine-3'-phosphate
  modified_base 9: mod_base = OTHER; note = 2'-deoxy-2'-fluorocytidine-3'-phosphate
  modified_base 10: mod_base = OTHER; note = 2'-O-methyladenosine-3'-phosphate
  modified_base 11: mod_base = OTHER; note = 2'-O-methylguanosine-3'-phosphate
  modified_base 12: mod_base = OTHER; note = 2'-O-methyluridine-3'-phosphate
  modified_base 13: mod_base = OTHER; note = 2'-O-methylcytidine-3'-phosphate
  modified_base 14: mod_base = OTHER; note = 2'-deoxy-2'-fluoroadenosine-3'-phosphate
  modified_base 15: mod_base = OTHER; note = 2'-O-methyluridine-3'-phosphate
  modified_base 16: mod_base = OTHER; note = 2'-deoxy-2'-fluoroguanosine-3'-phosphate
  modified_base 17: mod_base = OTHER; note = 2'-O-methyladenosine-3'-phosphate
  modified_base 18: mod_base = OTHER; note = 2'-O-methylguanosine-3'-phosphate
  modified_base 19: mod_base = OTHER; note = 2'-O-methylguanosine-3'-phosphate
  modified_base 20: mod_base = OTHER; note = 2'-O-methylcytidine-3'-phosphate
  modified_base 21: mod_base = OTHER; note = 2'-O-methyladenosine-3'-phosphorothioate
  modified_base 22: mod_base = OTHER; note = 2'-O-methylcytidine-3'-phosphorothioate
  modified_base 23: mod_base = OTHER; note = 2'-O-methyluridine
attgttttcagtcatgaggcact

SEQ ID NO: 527 - RNA, 23 nt, synthetic construct
  source 1..23: mol_type = other RNA
  modified_base 1: mod_base = OTHER; note = 2'-O-methyladenosine-3'-phosphorothioate
  modified_base 2: mod_base = OTHER; note = 2'-deoxy-2'-fluorouridine-3'-phosphorothioate
  modified_base 3: mod_base = OTHER; note = 2'-O-methylcytidine-3'-phosphate
  modified_base 4: mod_base = OTHER; note = 2'-O-methyladenosine-3'-phosphate
  modified_base 5: mod_base = OTHER; note = 2'-O-methyluridine-3'-phosphate
  modified_base 6: mod_base = OTHER; note = 2'-deoxy-2'-fluorouridine-3'-phosphate
  modified_base 7: mod_base = OTHER; note = 2'-O-methylguanosine-3'-phosphate
  modified_base 8: mod_base = OTHER; note = 2'-deoxy-2'-fluorouridine-3'-phosphate
  modified_base 9: mod_base = OTHER; note = 2'-deoxy-2'-fluoroguanosine-3'-phosphate
  modified_base 10: mod_base = OTHER; note = 2'-O-methyladenosine-3'-phosphate
  modified_base 11: mod_base = OTHER; note = 2'-O-methyladenosine-3'-phosphate
  modified_base 12: mod_base = OTHER; note = 2'-O-methylguanosine-3'-phosphate
  modified_base 13: mod_base = OTHER; note = 2'-O-methyladenosine-3'-phosphate
  modified_base 14: mod_base = OTHER; note = 2'-deoxy-2'-fluorouridine-3'-phosphate
  modified_base 15: mod_base = OTHER; note = 2'-O-methylguanosine-3'-phosphate
  modified_base 16: mod_base = OTHER; note = 2'-deoxy-2'-fluorocytidine-3'-phosphate
  modified_base 17: mod_base = OTHER; note = 2'-O-methyluridine-3'-phosphate
  modified_base 18: mod_base = OTHER; note = 2'-O-methyluridine-3'-phosphate
  modified_base 19: mod_base = OTHER; note = 2'-O-methyluridine-3'-phosphate
  modified_base 20: mod_base = OTHER; note = 2'-O-methylcytidine-3'-phosphate
  modified_base 21: mod_base = OTHER; note = 2'-O-methylguanosine-3'-phosphorothioate
  modified_base 22: mod_base = OTHER; note = 2'-O-methyluridine-3'-phosphorothioate
  modified_base 23: mod_base = OTHER; note = 2'-O-methyluridine
atcattgtgaagatgctttcgtt

SEQ ID NO: 528 - RNA, 23 nt, synthetic construct
  source 1..23: mol_type = other RNA
  modified_base 1: mod_base = OTHER; note = 2'-O-methyladenosine-3'-phosphorothioate
  modified_base 2: mod_base = OTHER; note = 2'-deoxy-2'-fluorouridine-3'-phosphorothioate
  modified_base 3: mod_base = OTHER; note = 2'-O-methyluridine-3'-phosphate
  modified_base 4: mod_base = OTHER; note = 2'-O-methyluridine-3'-phosphate
  modified_base 5: mod_base = OTHER; note = 2'-O-methyluridine-3'-phosphate
  modified_base 6: mod_base = OTHER; note = 2'-deoxy-2'-fluoroadenosine-3'-phosphate
  modified_base 7: mod_base = OTHER; note = 2'-O-methylguanosine-3'-phosphate
  modified_base 8: mod_base = OTHER; note = 2'-deoxy-2'-fluorocytidine-3'-phosphate
  modified_base 9: mod_base = OTHER; note = 2'-deoxy-2'-fluoroadenosine-3'-phosphate
  modified_base 10: mod_base = OTHER; note = 2'-O-methyladenosine-3'-phosphate
  modified_base 11: mod_base = OTHER; note = 2'-O-methyladenosine-3'-phosphate
  modified_base 12: mod_base = OTHER; note = 2'-O-methyladenosine-3'-phosphate
  modified_base 13: mod_base = OTHER; note = 2'-O-methylcytidine-3'-phosphate
  modified_base 14: mod_base = OTHER; note = 2'-deoxy-2'-fluoroguanosine-3'-phosphate
  modified_base 15: mod_base = OTHER; note = 2'-O-methylguanosine-3'-phosphate
  modified_base 16: mod_base = OTHER; note = 2'-deoxy-2'-fluorouridine-3'-phosphate
  modified_base 17: mod_base = OTHER; note = 2'-O-methylguanosine-3'-phosphate
  modified_base 18: mod_base = OTHER; note = 2'-O-methylcytidine-3'-phosphate
  modified_base 19: mod_base = OTHER; note = 2'-O-methyluridine-3'-phosphate
  modified_base 20: mod_base = OTHER; note = 2'-O-methyladenosine-3'-phosphate
  modified_base 21: mod_base = OTHER; note = 2'-O-methyluridine-3'-phosphorothioate
  modified_base 22: mod_base = OTHER; note = 2'-O-methylcytidine-3'-phosphorothioate
  modified_base 23: mod_base = OTHER; note = 2'-O-methyluridine
attttagcaaaacggtgctatct

SEQ ID NO: 529 - RNA, 23 nt, synthetic construct
  source 1..23: mol_type = other RNA
  modified_base 1: mod_base = OTHER; note = 2'-O-methyladenosine-3'-phosphorothioate
  modified_base 2: mod_base = OTHER; note = 2'-deoxy-2'-fluoroguanosine-3'-phosphorothioate
  modified_base 3: mod_base = OTHER; note = 2'-O-methyladenosine-3'-phosphate
  modified_base 4: mod_base = OTHER; note = 2'-O-methyladenosine-3'-phosphate
  modified_base 5: mod_base = OTHER; note = 2'-O-methyladenosine-3'-phosphate
  modified_base 6: mod_base = OTHER; note = 2'-deoxy-2'-fluoroadenosine-3'-phosphate
  modified_base 7: mod_base = OTHER; note = 2'-O-methylcytidine-3'-phosphate
  modified_base 8: mod_base = OTHER; note = 2'-deoxy-2'-fluoroadenosine-3'-phosphate
  modified_base 9: mod_base = OTHER; note = 2'-deoxy-2'-fluoroadenosine-3'-phosphate
  modified_base 10: mod_base = OTHER; note = 2'-O-methyluridine-3'-phosphate
  modified_base 11: mod_base = OTHER; note = 2'-O-methylguanosine-3'-phosphate
  modified_base 12: mod_base = OTHER; note = 2'-O-methyladenosine-3'-phosphate
  modified_base 13: mod_base = OTHER; note = 2'-O-methylguanosine-3'-phosphate
  modified_base 14: mod_base = OTHER; note = 2'-deoxy-2'-fluoroadenosine-3'-phosphate
  modified_base 15: mod_base = OTHER; note = 2'-O-methyladenosine-3'-phosphate
  modified_base 16: mod_base = OTHER; note = 2'-deoxy-2'-fluorouridine-3'-phosphate
  modified_base 17: mod_base = OTHER; note = 2'-O-methylguanosine-3'-phosphate
  modified_base 18: mod_base = OTHER; note = 2'-O-methyluridine-3'-phosphate
  modified_base 19: mod_base = OTHER; note = 2'-O-methyladenosine-3'-phosphate
  modified_base 20: mod_base = OTHER; note = 2'-O-methyluridine-3'-phosphate
  modified_base 21: mod_base = OTHER; note = 2'-O-methylcytidine-3'-phosphorothioate
  modified_base 22: mod_base = OTHER; note = 2'-O-methyluridine-3'-phosphorothioate
  modified_base 23: mod_base = OTHER; note = 2'-O-methyluridine
agaaaacaatgagaatgtatctt

SEQ ID NO: 530 - RNA, 23 nt, synthetic construct
  source 1..23: mol_type = other RNA
  modified_base 1: mod_base = OTHER; note = 2'-O-methyladenosine-3'-phosphorothioate
  modified_base 2: mod_base = OTHER; note = 2'-deoxy-2'-fluorouridine-3'-phosphorothioate
  modified_base 3: mod_base = OTHER; note = 2'-O-methyluridine-3'-phosphate
  modified_base 4: mod_base = OTHER; note = 2'-O-methyluridine-3'-phosphate
  modified_base 5: mod_base = OTHER; note = 2'-O-methylguanosine-3'-phosphate
  modified_base 6: mod_base = OTHER; note = 2'-deoxy-2'-fluorouridine-3'-phosphate
  modified_base 7: mod_base = OTHER; note = 2'-O-methyluridine-3'-phosphate
  modified_base 8: mod_base = OTHER; note = 2'-deoxy-2'-fluorouridine-3'-phosphate
  modified_base 9: mod_base = OTHER; note = 2'-deoxy-2'-fluoroadenosine-3'-phosphate
  modified_base 10: mod_base = OTHER; note = 2'-O-methyladenosine-3'-phosphate
  modified_base 11: mod_base = OTHER; note = 2'-O-methylcytidine-3'-phosphate
  modified_base 12: mod_base = OTHER; note = 2'-O-methylcytidine-3'-phosphate
  modified_base 13: mod_base = OTHER; note = 2'-O-methyluridine-3'-phosphate
  modified_base 14: mod_base = OTHER; note = 2'-deoxy-2'-fluorouridine-3'-phosphate
  modified_base 15: mod_base = OTHER; note = 2'-O-methyladenosine-3'-phosphate
  modified_base 16: mod_base = OTHER; note = 2'-deoxy-2'-fluorouridine-3'-phosphate
  modified_base 17: mod_base = OTHER; note = 2'-O-methylguanosine-3'-phosphate
  modified_base 18: mod_base = OTHER; note = 2'-O-methyluridine-3'-phosphate
  modified_base 19: mod_base = OTHER; note = 2'-O-methylguanosine-3'-phosphate
  modified_base 20: mod_base = OTHER; note = 2'-O-methylguanosine-3'-phosphate
  modified_base 21: mod_base = OTHER; note = 2'-O-methyladenosine-3'-phosphorothioate
  modified_base 22: mod_base = OTHER; note = 2'-O-methyladenosine-3'-phosphorothioate
  modified_base 23: mod_base = OTHER; note = 2'-O-methylguanosine
atttgtttaaccttatgtggaag

SEQ ID NO: 531 - RNA, 23 nt, synthetic construct
  source 1..23: mol_type = other RNA
  modified_base 1: mod_base = OTHER; note = 2'-O-methyladenosine-3'-phosphorothioate
  modified_base 2: mod_base = OTHER; note = 2'-deoxy-2'-fluorouridine-3'-phosphorothioate
  modified_base 3: mod_base = OTHER; note = 2'-O-methyladenosine-3'-phosphate
  modified_base 4: mod_base = OTHER; note = 2'-O-methyladenosine-3'-phosphate
  modified_base 5: mod_base = OTHER; note = 2'-O-methyladenosine-3'-phosphate
  modified_base 6: mod_base = OTHER; note = 2'-deoxy-2'-fluorouridine-3'-phosphate
  modified_base 7: mod_base = OTHER; note = 2'-O-methyluridine-3'-phosphate
  modified_base 8: mod_base = OTHER; note = 2'-deoxy-2'-fluoroadenosine-3'-phosphate
  modified_base 9: mod_base = OTHER; note = 2'-deoxy-2'-fluorouridine-3'-phosphate
  modified_base 10: mod_base = OTHER; note = 2'-O-methyluridine-3'-phosphate
  modified_base 11: mod_base = OTHER; note = 2'-O-methyluridine-3'-phosphate
  modified_base 12: mod_base = OTHER; note = 2'-O-methyladenosine-3'-phosphate
  modified_base 13: mod_base = OTHER; note = 2'-O-methylcytidine-3'-phosphate
  modified_base 14: mod_base = OTHER; note = 2'-deoxy-2'-fluoroadenosine-3'-phosphate
  modified_base 15: mod_base = OTHER; note = 2'-O-methyladenosine-3'-phosphate
  modified_base 16: mod_base = OTHER; note = 2'-deoxy-2'-fluoroguanosine-3'-phosphate
  modified_base 17: mod_base = OTHER; note = 2'-O-methylcytidine-3'-phosphate
  modified_base 18: mod_base = OTHER; note = 2'-O-methyladenosine-3'-phosphate
  modified_base 19: mod_base = OTHER; note = 2'-O-methylcytidine-3'-phosphate
  modified_base 20: mod_base = OTHER; note = 2'-O-methylcytidine-3'-phosphate
  modified_base 21: mod_base = OTHER; note = 2'-O-methyluridine-3'-phosphorothioate
  modified_base 22: mod_base = OTHER; note = 2'-O-methyladenosine-3'-phosphorothioate
  modified_base 23: mod_base = OTHER; note = 2'-O-methylguanosine
ataaattatttacaagcacctag

SEQ ID NO: 532 - RNA, 23 nt, synthetic construct
  source 1..23: mol_type = other RNA
  modified_base 1: mod_base = OTHER; note = 2'-O-methyladenosine-3'-phosphorothioate
  modified_base 2: mod_base = OTHER; note = 2'-deoxy-2'-fluoroguanosine-3'-phosphorothioate
  modified_base 3: mod_base = OTHER; note = 2'-O-methyluridine-3'-phosphate
  modified_base 4: mod_base = OTHER; note = 2'-O-methyluridine-3'-phosphate
  modified_base 5: mod_base = OTHER; note = 2'-O-methyladenosine-3'-phosphate
  modified_base 6: mod_base = OTHER; note = 2'-deoxy-2'-fluorocytidine-3'-phosphate
  modified_base 7: mod_base = OTHER; note = 2'-O-methyladenosine-3'-phosphate
  modified_base 8: mod_base = OTHER; note = 2'-deoxy-2'-fluoroguanosine-3'-phosphate
  modified_base 9: mod_base = OTHER; note = 2'-deoxy-2'-fluoroadenosine-3'-phosphate
  modified_base 10: mod_base = OTHER; note = 2'-O-methyladenosine-3'-phosphate
  modified_base 11: mod_base = OTHER; note = 2'-O-methyladenosine-3'-phosphate
  modified_base 12: mod_base = OTHER; note = 2'-O-methyluridine-3'-phosphate
  modified_base 13: mod_base = OTHER; note = 2'-O-methylguanosine-3'-phosphate
  modified_base 14: mod_base = OTHER; note = 2'-deoxy-2'-fluorocytidine-3'-phosphate
  modified_base 15: mod_base = OTHER; note = 2'-O-methylguanosine-3'-phosphate
  modified_base 16: mod_base = OTHER; note = 2'-deoxy-2'-fluoroadenosine-3'-phosphate
  modified_base 17: mod_base = OTHER; note = 2'-O-methyluridine-3'-phosphate
  modified_base 18: mod_base = OTHER; note = 2'-O-methyladenosine-3'-phosphate
  modified_base 19: mod_base = OTHER; note = 2'-O-methylguanosine-3'-phosphate
  modified_base 20: mod_base = OTHER; note = 2'-O-methyladenosine-3'-phosphate
  modified_base 21: mod_base = OTHER; note = 2'-O-methylguanosine-3'-phosphorothioate
  modified_base 22: mod_base = OTHER; note = 2'-O-methyluridine-3'-phosphorothioate
  modified_base 23: mod_base = OTHER; note = 2'-O-methyladenosine
agttacagaaatgcgatagagta

SEQ ID NO: 533 - RNA, 23 nt, synthetic construct
  source 1..23: mol_type = other RNA
  modified_base 1: mod_base = OTHER; note = 2'-O-methyladenosine-3'-phosphorothioate
  modified_base 2: mod_base = OTHER; note = 2'-deoxy-2'-fluoroadenosine-3'-phosphorothioate
  modified_base 3: mod_base = OTHER; note = 2'-O-methylcytidine-3'-phosphate
  modified_base 4: mod_base = OTHER; note = 2'-O-methyluridine-3'-phosphate
  modified_base 5: mod_base = OTHER; note = 2'-O-methyluridine-3'-phosphate
  modified_base 6: mod_base = OTHER; note = 2'-deoxy-2'-fluoroadenosine-3'-phosphate
  modified_base 7: mod_base = OTHER; note = 2'-O-methylguanosine-3'-phosphate
  modified_base 8: mod_base = OTHER; note = 2'-deoxy-2'-fluoroguanosine-3'-phosphate
  modified_base 9: mod_base = OTHER; note = 2'-deoxy-2'-fluoroadenosine-3'-phosphate
  modified_base 10: mod_base = OTHER; note = 2'-O-methylcytidine-3'-phosphate
  modified_base 11: mod_base = OTHER; note = 2'-O-methyladenosine-3'-phosphate
  modified_base 12: mod_base = OTHER; note = 2'-O-methyluridine-3'-phosphate
  modified_base 13: mod_base = OTHER; note = 2'-O-methyluridine-3'-phosphate
  modified_base 14: mod_base = OTHER; note = 2'-deoxy-2'-fluorocytidine-3'-phosphate
  modified_base 15: mod_base = OTHER; note = 2'-O-methyluridine-3'-phosphate
  modified_base 16: mod_base = OTHER; note = 2'-deoxy-2'-fluorocytidine-3'-phosphate
  modified_base 17: mod_base = OTHER; note = 2'-O-methyladenosine-3'-phosphate
  modified_base 18: mod_base = OTHER; note = 2'-O-methyluridine-3'-phosphate
  modified_base 19: mod_base = OTHER; note = 2'-O-methyluridine-3'-phosphate
  modified_base 20: mod_base = OTHER; note = 2'-O-methyluridine-3'-phosphate
  modified_base 21: mod_base = OTHER; note = 2'-O-methyluridine-3'-phosphorothioate
  modified_base 22: mod_base = OTHER; note = 2'-O-methylcytidine-3'-phosphorothioate
  modified_base 23: mod_base = OTHER; note = 2'-O-methyladenosine
aacttaggacattctcattttca

SEQ ID NO: 534 - RNA, 23 nt, synthetic construct
  source 1..23: mol_type = other RNA
  modified_base 1: mod_base = OTHER; note = 2'-O-methyladenosine-3'-phosphorothioate
  modified_base 2: mod_base = OTHER; note = 2'-deoxy-2'-fluorouridine-3'-phosphorothioate
  modified_base 3: mod_base = OTHER; note = 2'-O-methyluridine-3'-phosphate
  modified_base 4: mod_base = OTHER; note = 2'-O-methyluridine-3'-phosphate
  modified_base 5: mod_base = OTHER; note = 2'-O-methylcytidine-3'-phosphate
  modified_base 6: mod_base = OTHER; note = 2'-deoxy-2'-fluoroadenosine-3'-phosphate
  modified_base 7: mod_base = OTHER; note = 2'-O-methyluridine-3'-phosphate
  modified_base 8: mod_base = OTHER; note = 2'-deoxy-2'-fluoroguanosine-3'-phosphate
  modified_base 9: mod_base = OTHER; note = 2'-deoxy-2'-fluorocytidine-3'-phosphate
  modified_base 10: mod_base = OTHER; note = 2'-O-methyladenosine-3'-phosphate
  modified_base 11: mod_base = OTHER; note = 2'-O-methyluridine-3'-phosphate
  modified_base 12: mod_base = OTHER; note = 2'-O-methyluridine-3'-phosphate
  modified_base 13: mod_base = OTHER; note = 2'-O-methyluridine-3'-phosphate
  modified_base 14: mod_base = OTHER; note = 2'-deoxy-2'-fluorouridine-3'-phosphate
  modified_base 15: mod_base = OTHER; note = 2'-O-methylcytidine-3'-phosphate
  modified_base 16: mod_base = OTHER; note = 2'-deoxy-2'-fluoroadenosine-3'-phosphate
  modified_base 17: mod_base = OTHER; note = 2'-O-methylguanosine-3'-phosphate
  modified_base 18: mod_base = OTHER; note = 2'-O-methyladenosine-3'-phosphate
  modified_base 19: mod_base = OTHER; note = 2'-O-methylguanosine-3'-phosphate
  modified_base 20: mod_base = OTHER; note = 2'-O-methyluridine-3'-phosphate
  modified_base 21: mod_base = OTHER; note = 2'-O-methylguanosine-3'-phosphorothioate
  modified_base 22: mod_base = OTHER; note = 2'-O-methylcytidine-3'-phosphorothioate
  modified_base 23: mod_base = OTHER; note = 2'-O-methyladenosine
atttcatgcattttcagagtgca

SEQ ID NO: 535 - RNA, 23 nt, synthetic construct
  source 1..23: mol_type = other RNA
  modified_base 1: mod_base = OTHER; note = 2'-O-methyladenosine-3'-phosphorothioate
  modified_base 2: mod_base = OTHER; note = 2'-deoxy-2'-fluoroadenosine-3'-phosphorothioate
  modified_base 3: mod_base = OTHER; note = 2'-O-methylguanosine-3'-phosphate
  modified_base 4: mod_base = OTHER; note = 2'-O-methyluridine-3'-phosphate
  modified_base 5: mod_base = OTHER; note = 2'-O-methyluridine-3'-phosphate
  modified_base 6: mod_base = OTHER; note = 2'-deoxy-2'-fluoroadenosine-3'-phosphate
  modified_base 7: mod_base = OTHER; note = 2'-O-methyladenosine-3'-phosphate
  modified_base 8: mod_base = OTHER; note = 2'-deoxy-2'-fluorocytidine-3'-phosphate
  modified_base 9: mod_base = OTHER; note = 2'-deoxy-2'-fluoroadenosine-3'-phosphate
  modified_base 10: mod_base = OTHER; note = 2'-O-methylguanosine-3'-phosphate
  modified_base 11: mod_base = OTHER; note = 2'-O-methyluridine-3'-phosphate
  modified_base 12: mod_base = OTHER; note = 2'-O-methyluridine-3'-phosphate
  modified_base 13: mod_base = OTHER; note = 2'-O-methylcytidine-3'-phosphate
  modified_base 14: mod_base = OTHER; note = 2'-deoxy-2'-fluorouridine-3'-phosphate
  modified_base 15: mod_base = OTHER; note = 2'-O-methyladenosine-3'-phosphate
  modified_base 16: mod_base = OTHER; note = 2'-deoxy-2'-fluorocytidine-3'-phosphate
  modified_base 17: mod_base = OTHER; note = 2'-O-methyladenosine-3'-phosphate
  modified_base 18: mod_base = OTHER; note = 2'-O-methylcytidine-3'-phosphate
  modified_base 19: mod_base = OTHER; note = 2'-O-methyladenosine-3'-phosphate
  modified_base 20: mod_base = OTHER; note = 2'-O-methyluridine-3'-phosphate
  modified_base 21: mod_base = OTHER; note = 2'-O-methyluridine-3'-phosphorothioate
  modified_base 22: mod_base = OTHER; note = 2'-O-methyluridine-3'-phosphorothioate
  modified_base 23: mod_base = OTHER; note = 2'-O-methylcytidine
aagttaacagttctacacatttc

SEQ ID NO: 536 - RNA, 23 nt, synthetic construct
  source 1..23: mol_type = other RNA
  modified_base 1: mod_base = OTHER; note = 2'-O-methyladenosine-3'-phosphorothioate
  modified_base 2: mod_base = OTHER; note = 2'-deoxy-2'-fluoroadenosine-3'-phosphorothioate
  modified_base 3: mod_base = OTHER; note = 2'-O-methyladenosine-3'-phosphate
  modified_base 4: mod_base = OTHER; note = 2'-O-methyluridine-3'-phosphate
  modified_base 5: mod_base = OTHER; note = 2'-O-methyluridine-3'-phosphate
  modified_base 6: mod_base = OTHER; note = 2'-deoxy-2'-fluorouridine-3'-phosphate
  modified_base 7: mod_base = OTHER; note = 2'-O-methyladenosine-3'-phosphate
  modified_base 8: mod_base = OTHER; note = 2'-deoxy-2'-fluoroadenosine-3'-phosphate
  modified_base 9: mod_base = OTHER; note = 2'-deoxy-2'-fluorocytidine-3'-phosphate
  modified_base 10: mod_base = OTHER; note = 2'-O-methyladenosine-3'-phosphate
  modified_base 11: mod_base = OTHER; note = 2'-O-methylguanosine-3'-phosphate
  modified_base 12: mod_base = OTHER; note = 2'-O-methyladenosine-3'-phosphate
  modified_base 13: mod_base = OTHER; note = 2'-O-methyluridine-3'-phosphate
  modified_base 14: mod_base = OTHER; note = 2'-deoxy-2'-fluorouridine-3'-phosphate
  modified_base 15: mod_base = OTHER; note = 2'-O-methylcytidine-3'-phosphate
  modified_base 16: mod_base = OTHER; note = 2'-deoxy-2'-fluorocytidine-3'-phosphate
  modified_base 17: mod_base = OTHER; note = 2'-O-methyladenosine-3'-phosphate
  modified_base 18: mod_base = OTHER; note = 2'-O-methylguanosine-3'-phosphate
  modified_base 19: mod_base = OTHER; note = 2'-O-methyladenosine-3'-phosphate
  modified_base 20: mod_base = OTHER; note = 2'-O-methyladenosine-3'-phosphate
  modified_base 21: mod_base = OTHER; note = 2'-O-methylguanosine-3'-phosphorothioate
  modified_base 22: mod_base = OTHER; note = 2'-O-methylguanosine-3'-phosphorothioate
  modified_base 23: mod_base = OTHER; note = 2'-O-methyladenosine
aaatttaacagattccagaagga

SEQ ID NO: 537 - RNA, 23 nt, synthetic construct
  source 1..23: mol_type = other RNA
  modified_base 1: mod_base = OTHER; note = 2'-O-methyladenosine-3'-phosphorothioate
  modified_base 2: mod_base = OTHER; note = 2'-deoxy-2'-fluorouridine-3'-phosphorothioate
  modified_base 3: mod_base = OTHER; note = 2'-O-methyladenosine-3'-phosphate
  modified_base 4: mod_base = OTHER; note = 2'-O-methyluridine-3'-phosphate
  modified_base 5: mod_base = OTHER; note = 2'-O-methyluridine-3'-phosphate
  modified_base 6: mod_base = OTHER; note = 2'-deoxy-2'-fluorouridine-3'-phosphate
  modified_base 7: mod_base = OTHER; note = 2'-O-methyluridine-3'-phosphate
  modified_base 8: mod_base = OTHER; note = 2'-deoxy-2'-fluorocytidine-3'-phosphate
  modified_base 9: mod_base = OTHER; note = 2'-deoxy-2'-fluorouridine-3'-phosphate
  modified_base 10: mod_base = OTHER; note = 2'-O-methylcytidine-3'-phosphate
  modified_base 11: mod_base = OTHER; note = 2'-O-methylcytidine-3'-phosphate
  modified_base 12: mod_base = OTHER; note = 2'-O-methyladenosine-3'-phosphate
  modified_base 13: mod_base = OTHER; note = 2'-O-methyluridine-3'-phosphate
  modified_base 14: mod_base = OTHER; note = 2'-deoxy-2'-fluorouridine-3'-phosphate
  modified_base 15: mod_base = OTHER; note = 2'-O-methyluridine-3'-phosphate
  modified_base 16: mod_base = OTHER; note = 2'-deoxy-2'-fluoroadenosine-3'-phosphate
  modified_base 17: mod_base = OTHER; note = 2'-O-methylcytidine-3'-phosphate
  modified_base 18: mod_base = OTHER; note = 2'-O-methylcytidine-3'-phosphate
  modified_base 19: mod_base = OTHER; note = 2'-O-methylcytidine-3'-phosphate
  modified_base 20: mod_base = OTHER; note = 2'-O-methyluridine-3'-phosphate
  modified_base 21: mod_base = OTHER; note = 2'-O-methylcytidine-3'-phosphorothioate
  modified_base 22: mod_base = OTHER; note = 2'-O-methyladenosine-3'-phosphorothioate
  modified_base 23: mod_base = OTHER; note = 2'-O-methyluridine
atattttctccatttaccctcat

SEQ ID NO: 538 - RNA, 23 nt, synthetic construct
  source 1..23: mol_type = other RNA
  modified_base 1: mod_base = OTHER; note = 2'-O-methyladenosine-3'-phosphorothioate
  modified_base 2: mod_base = OTHER; note = 2'-deoxy-2'-fluorouridine-3'-phosphorothioate
  modified_base 3: mod_base = OTHER; note = 2'-O-methyluridine-3'-phosphate
  modified_base 4: mod_base = OTHER; note = 2'-O-methyladenosine-3'-phosphate
  modified_base 5: mod_base = OTHER; note = 2'-O-methylcytidine-3'-phosphate
  modified_base 6: mod_base = OTHER; note = 2'-deoxy-2'-fluoroadenosine-3'-phosphate
  modified_base 7: mod_base = OTHER; note = 2'-O-methyluridine-3'-phosphate
  modified_base 8: mod_base = OTHER; note = 2'-deoxy-2'-fluorouridine-3'-phosphate
  modified_base 9: mod_base = OTHER; note = 2'-deoxy-2'-fluorocytidine-3'-phosphate
  modified_base 10: mod_base = OTHER; note = 2'-O-methyladenosine-3'-phosphate
  modified_base 11: mod_base = OTHER; note = 2'-O-methyluridine-3'-phosphate
  modified_base 12: mod_base = OTHER; note = 2'-O-methyluridine-3'-phosphate
  modified_base 13: mod_base = OTHER; note = 2'-O-methylguanosine-3'-phosphate
  modified_base 14: mod_base = OTHER; note = 2'-deoxy-2'-fluorouridine-3'-phosphate
  modified_base 15: mod_base = OTHER; note = 2'-O-methyladenosine-3'-phosphate
  modified_base 16: mod_base = OTHER; note = 2'-deoxy-2'-fluoroadenosine-3'-phosphate
  modified_base 17: mod_base = OTHER; note = 2'-O-methyluridine-3'-phosphate
  modified_base 18: mod_base = OTHER; note = 2'-O-methylcytidine-3'-phosphate
  modified_base 19: mod_base = OTHER; note = 2'-O-methylcytidine-3'-phosphate
  modified_base 20: mod_base = OTHER; note = 2'-O-methylcytidine-3'-phosphate
  modified_base 21: mod_base = OTHER; note = 2'-O-methyladenosine-3'-phosphorothioate
  modified_base 22: mod_base = OTHER; note = 2'-O-methylguanosine-3'-phosphorothioate
  modified_base 23: mod_base = OTHER; note = 2'-O-methyladenosine
attacattcattgtaatcccaga

SEQ ID NO: 539 - RNA, 23 nt, synthetic construct
  source 1..23: mol_type = other RNA
  modified_base 1: mod_base = OTHER; note = 2'-O-methyladenosine-3'-phosphorothioate
  modified_base 2: mod_base = OTHER; note = 2'-deoxy-2'-fluoroadenosine-3'-phosphorothioate
  modified_base 3: mod_base = OTHER; note = 2'-O-methyladenosine-3'-phosphate
  modified_base 4: mod_base = OTHER; note = 2'-O-methyluridine-3'-phosphate
  modified_base 5: mod_base = OTHER; note = 2'-O-methyluridine-3'-phosphate
  modified_base 6: mod_base = OTHER; note = 2'-deoxy-2'-fluorocytidine-3'-phosphate
  modified_base 7: mod_base = OTHER; note = 2'-O-methylcytidine-3'-phosphate
  modified_base 8: mod_base = OTHER; note = 2'-deoxy-2'-fluoroadenosine-3'-phosphate
  modified_base 9: mod_base = OTHER; note = 2'-deoxy-2'-fluorocytidine-3'-phosphate
  modified_base 10: mod_base = OTHER; note = 2'-O-methyladenosine-3'-phosphate
  modified_base 11: mod_base = OTHER; note = 2'-O-methyladenosine-3'-phosphate
  modified_base 12: mod_base = OTHER; note = 2'-O-methyluridine-3'-phosphate
  modified_base 13: mod_base = OTHER; note = 2'-O-methyluridine-3'-phosphate
  modified_base 14: mod_base = OTHER; note = 2'-deoxy-2'-fluorouridine-3'-phosphate
  modified_base 15: mod_base = OTHER; note = 2'-O-methylguanosine-3'-phosphate
  modified_base 16: mod_base = OTHER; note = 2'-deoxy-2'-fluoroguanosine-3'-phosphate
  modified_base 17: mod_base = OTHER; note = 2'-O-methylguanosine-3'-phosphate
  modified_base 18: mod_base = OTHER; note = 2'-O-methylcytidine-3'-phosphate
  modified_base 19: mod_base = OTHER; note = 2'-O-methyluridine-3'-phosphate
  modified_base 20: mod_base = OTHER; note = 2'-O-methyluridine-3'-phosphate
  modified_base 21: mod_base = OTHER; note = 2'-O-methyladenosine-3'-phosphorothioate
  modified_base 22: mod_base = OTHER; note = 2'-O-methylcytidine-3'-phosphorothioate
  modified_base 23: mod_base = OTHER; note = 2'-O-methyladenosine
aaattccacaatttgggcttaca

SEQ ID NO: 540 - RNA, 23 nt, synthetic construct
  source 1..23: mol_type = other RNA
  modified_base 1: mod_base = OTHER; note = 2'-O-methyladenosine-3'-phosphorothioate
  modified_base 2: mod_base = OTHER; note = 2'-deoxy-2'-fluorouridine-3'-phosphorothioate
  modified_base 3: mod_base = OTHER; note = 2'-O-methyluridine-3'-phosphate
  modified_base 4: mod_base = OTHER; note = 2'-O-methyluridine-3'-phosphate
  modified_base 5: mod_base = OTHER; note = 2'-O-methylcytidine-3'-phosphate
  modified_base 6: mod_base = OTHER; note = 2'-deoxy-2'-fluorouridine-3'-phosphate
  modified_base 7: mod_base = OTHER; note = 2'-O-methyladenosine-3'-phosphate
  modified_base 8: mod_base = OTHER; note = 2'-deoxy-2'-fluorouridine-3'-phosphate
  modified_base 9: mod_base = OTHER; note = 2'-deoxy-2'-fluoroadenosine-3'-phosphate
  modified_base 10: mod_base = OTHER; note = 2'-O-methyladenosine-3'-phosphate
  modified_base 11: mod_base = OTHER; note = 2'-O-methyladenosine-3'-phosphate
  modified_base 12: mod_base = OTHER; note = 2'-O-methyladenosine-3'-phosphate
  modified_base 13: mod_base = OTHER; note = 2'-O-methylcytidine-3'-phosphate
  modified_base 14: mod_base = OTHER; note = 2'-deoxy-2'-fluoroadenosine-3'-phosphate
  modified_base 15: mod_base = OTHER; note = 2'-O-methylcytidine-3'-phosphate
  modified_base 16: mod_base = OTHER; note = 2'-deoxy-2'-fluorouridine-3'-phosphate
  modified_base 17: mod_base = OTHER; note = 2'-O-methylguanosine-3'-phosphate
  modified_base 18: mod_base = OTHER; note = 2'-O-methyladenosine-3'-phosphate
  modified_base 19: mod_base = OTHER; note = 2'-O-methyluridine-3'-phosphate
  modified_base 20: mod_base = OTHER; note = 2'-O-methylguanosine-3'-phosphate
  modified_base 21: mod_base = OTHER; note = 2'-O-methyladenosine-3'-phosphorothioate
  modified_base 22: mod_base = OTHER; note = 2'-O-methyladenosine-3'-phosphorothioate
  modified_base 23: mod_base = OTHER; note = 2'-O-methylcytidine
atttctataaaacactgatgaac

SEQ ID NO: 541 - RNA, 23 nt, synthetic construct
  source 1..23: mol_type = other RNA
  modified_base 1: mod_base = OTHER; note = 2'-O-methyladenosine-3'-phosphorothioate
  modified_base 2: mod_base = OTHER; note = 2'-deoxy-2'-fluoroguanosine-3'-phosphorothioate
  modified_base 3: mod_base = OTHER; note = 2'-O-methyluridine-3'-phosphate
  modified_base 4: mod_base = OTHER; note = 2'-O-methylcytidine-3'-phosphate
  modified_base 5: mod_base = OTHER; note = 2'-O-methyladenosine-3'-phosphate
  modified_base 6: mod_base = OTHER; note = 2'-deoxy-2'-fluoroadenosine-3'-phosphate
  modified_base 7: mod_base = OTHER; note = 2'-O-methyladenosine-3'-phosphate
  modified_base 8: mod_base = OTHER; note = 2'-deoxy-2'-fluoroadenosine-3'-phosphate
  modified_base 9: mod_base = OTHER; note = 2'-deoxy-2'-fluorouridine-3'-phosphate
  modified_base 10: mod_base = OTHER; note = 2'-O-methyladenosine-3'-phosphate
  modified_base 11: mod_base = OTHER; note = 2'-O-methylguanosine-3'-phosphate
  modified_base 12: mod_base = OTHER; note = 2'-O-methyluridine-3'-phosphate
  modified_base 13: mod_base = OTHER; note = 2'-O-methyluridine-3'-phosphate
  modified_base 14: mod_base = OTHER; note = 2'-deoxy-2'-fluorouridine-3'-phosphate
  modified_base 15: mod_base = OTHER; note = 2'-O-methylguanosine-3'-phosphate
  modified_base 16: mod_base = OTHER; note = 2'-deoxy-2'-fluoroguanosine-3'-phosphate
  modified_base 17: mod_base = OTHER; note = 2'-O-methylguanosine-3'-phosphate
  modified_base 18: mod_base = OTHER; note = 2'-O-methylcytidine-3'-phosphate
  modified_base 19: mod_base = OTHER; note = 2'-O-methyladenosine-3'-phosphate
  modified_base 20: mod_base = OTHER; note = 2'-O-methyladenosine-3'-phosphate
  modified_base 21: mod_base = OTHER; note = 2'-O-methyluridine-3'-phosphorothioate
  modified_base 22: mod_base = OTHER; note = 2'-O-methylguanosine-3'-phosphorothioate
  modified_base 23: mod_base = OTHER; note = 2'-O-methylcytidine
agtcaaaatagtttgggcaatgc

SEQ ID NO: 542 - RNA, 23 nt, synthetic construct
  source 1..23: mol_type = other RNA
  modified_base 1: mod_base = OTHER; note = 2'-O-methyladenosine-3'-phosphorothioate
  modified_base 2: mod_base = OTHER; note = 2'-deoxy-2'-fluorouridine-3'-phosphorothioate
  modified_base 3: mod_base = OTHER; note = 2'-O-methyluridine-3'-phosphate
  modified_base 4: mod_base = OTHER; note = 2'-O-methyladenosine-3'-phosphate
  modified_base 5: mod_base = OTHER; note = 2'-O-methylguanosine-3'-phosphate
  modified_base 6: mod_base = OTHER; note = 2'-deoxy-2'-fluorouridine-3'-phosphate
  modified_base 7: mod_base = OTHER; note = 2'-O-methylguanosine-3'-phosphate
  modified_base 8: mod_base = OTHER; note = 2'-deoxy-2'-fluoroadenosine-3'-phosphate
  modified_base 9: mod_base = OTHER; note = 2'-deoxy-2'-fluoroguanosine-3'-phosphate
  modified_base 10: mod_base = OTHER; note = 2'-O-methyladenosine-3'-phosphate
  modified_base 11: mod_base = OTHER; note = 2'-O-methylguanosine-3'-phosphate
  modified_base 12: mod_base = OTHER; note = 2'-O-methylguanosine-3'-phosphate
  modified_base 13: mod_base = OTHER; note = 2'-O-methyluridine-3'-phosphate
  modified_base 14: mod_base = OTHER; note = 2'-deoxy-2'-fluorouridine-3'-phosphate
  modified_base 15: mod_base = OTHER; note = 2'-O-methylcytidine-3'-phosphate
  modified_base 16: mod_base = OTHER; note = 2'-deoxy-2'-fluoroadenosine-3'-phosphate
  modified_base 17: mod_base = OTHER; note = 2'-O-methyluridine-3'-phosphate
  modified_base 18: mod_base = OTHER; note = 2'-O-methyladenosine-3'-phosphate
  modified_base 19: mod_base = OTHER; note = 2'-O-methyladenosine-3'-phosphate
  modified_base 20: mod_base = OTHER; note = 2'-O-methylguanosine-3'-phosphate
  modified_base 21: mod_base = OTHER; note = 2'-O-methyluridine-3'-phosphorothioate
  modified_base 22: mod_base = OTHER; note = 2'-O-methyladenosine-3'-phosphorothioate
  modified_base 23: mod_base = OTHER; note = 2'-O-methyluridine
attagtgagaggttcataagtat

SEQ ID NO: 543 - RNA, 23 nt, synthetic construct
  source 1..23: mol_type = other RNA
  modified_base 1: mod_base = OTHER; note = 2'-O-methyladenosine-3'-phosphorothioate
  modified_base 2: mod_base = OTHER; note = 2'-deoxy-2'-fluorouridine-3'-phosphorothioate
  modified_base 3: mod_base = OTHER; note = 2'-O-methylcytidine-3'-phosphate
  modified_base 4: mod_base = OTHER; note = 2'-O-methyluridine-3'-phosphate
  modified_base 5: mod_base = OTHER; note = 2'-O-methyladenosine-3'-phosphate
  modified_base 6: mod_base = OTHER; note = 2'-deoxy-2'-fluoroadenosine-3'-phosphate
  modified_base 7: mod_base = OTHER; note = 2'-O-methylcytidine-3'-phosphate
  modified_base 8: mod_base = OTHER; note = 2'-deoxy-2'-fluoroadenosine-3'-phosphate
  modified_base 9: mod_base = OTHER; note = 2'-deoxy-2'-fluorouridine-3'-phosphate
  modified_base 10: mod_base = OTHER; note = 2'-O-methyladenosine-3'-phosphate
  modified_base 11: mod_base = OTHER; note = 2'-O-methylguanosine-3'-phosphate
  modified_base 12: mod_base = OTHER; note = 2'-O-methyluridine-3'-phosphate
  modified_base 13: mod_base = OTHER; note = 2'-O-methylguanosine-3'-phosphate
  modified_base 14: mod_base = OTHER; note = 2'-deoxy-2'-fluorouridine-3'-phosphate
  modified_base 15: mod_base = OTHER; note = 2'-O-methyluridine-3'-phosphate
  modified_base 16: mod_base = OTHER; note = 2'-deoxy-2'-fluorouridine-3'-phosphate
  modified_base 17: mod_base = OTHER; note = 2'-O-methylcytidine-3'-phosphate
  modified_base 18: mod_base = OTHER; note = 2'-O-methylcytidine-3'-phosphate
  modified_base 19: mod_base = OTHER; note = 2'-O-methylcytidine-3'-phosphate
  modified_base 20: mod_base = OTHER; note = 2'-O-methyladenosine-3'-phosphate
  modified_base 21: mod_base = OTHER; note = 2'-O-methyladenosine-3'-phosphorothioate
  modified_base 22: mod_base = OTHER; note = 2'-O-methyladenosine-3'-phosphorothioate
  modified_base 23: mod_base = OTHER; note = 2'-O-methyladenosine
atctaacatagtgtttcccaaaa

SEQ ID NO: 544 - RNA, 23 nt, synthetic construct
  source 1..23: mol_type = other RNA
  modified_base 1: mod_base = OTHER; note = 2'-O-methyladenosine-3'-phosphorothioate
  modified_base 2: mod_base = OTHER; note = 2'-deoxy-2'-fluorouridine-3'-phosphorothioate
  modified_base 3: mod_base = OTHER; note = 2'-O-methyluridine-3'-phosphate
  modified_base 4: mod_base = OTHER; note = 2'-O-methyluridine-3'-phosphate
  modified_base 5: mod_base = OTHER; note = 2'-O-methyluridine-3'-phosphate
  modified_base 6: mod_base = OTHER; note = 2'-deoxy-2'-fluoroguanosine-3'-phosphate
  modified_base 7: mod_base = OTHER; note = 2'-O-methyluridine-3'-phosphate
  modified_base 8: mod_base = OTHER; note = 2'-deoxy-2'-fluorocytidine-3'-phosphate
  modified_base 9: mod_base = OTHER; note = 2'-deoxy-2'-fluorouridine-3'-phosphate
  modified_base 10: mod_base = OTHER; note = 2'-O-methylcytidine-3'-phosphate
  modified_base 11: mod_base = OTHER; note = 2'-O-methylcytidine-3'-phosphate
  modified_base 12: mod_base = OTHER; note = 2'-O-methyluridine-3'-phosphate
  modified_base 13: mod_base = OTHER; note = 2'-O-methyluridine-3'-phosphate
  modified_base 14: mod_base = OTHER; note = 2'-deoxy-2'-fluoroadenosine-3'-phosphate
  modified_base 15: mod_base = OTHER; note = 2'-O-methyladenosine-3'-phosphate
  modified_base 16: mod_base = OTHER; note = 2'-deoxy-2'-fluoroadenosine-3'-phosphate
  modified_base 17: mod_base = OTHER; note = 2'-O-methylguanosine-3'-phosphate
  modified_base 18: mod_base = OTHER; note = 2'-O-methyladenosine-3'-phosphate
  modified_base 19: mod_base = OTHER; note = 2'-O-methyladenosine-3'-phosphate
  modified_base 20: mod_base = OTHER; note = 2'-O-methylcytidine-3'-phosphate
  modified_base 21: mod_base = OTHER; note = 2'-O-methyluridine-3'-phosphorothioate
  modified_base 22: mod_base = OTHER; note = 2'-O-methyladenosine-3'-phosphorothioate
  modified_base 23: mod_base = OTHER; note = 2'-O-methyluridine
attttgtctccttaaagaactat

SEQ ID NO: 545 - RNA, 23 nt, synthetic construct
  source 1..23: mol_type = other RNA
  modified_base 1: mod_base = OTHER; note = 2'-O-methyladenosine-3'-phosphorothioate
  modified_base 2: mod_base = OTHER; note = 2'-deoxy-2'-fluoroguanosine-3'-phosphorothioate
  modified_base 3: mod_base = OTHER; note = 2'-O-methyluridine-3'-phosphate
  modified_base 4: mod_base = OTHER; note = 2'-O-methyluridine-3'-phosphate
  modified_base 5: mod_base = OTHER; note = 2'-O-methyladenosine-3'-phosphate
  modified_base 6: mod_base = OTHER; note = 2'-deoxy-2'-fluorocytidine-3'-phosphate
  modified_base 7: mod_base = OTHER; note = 2'-O-methyladenosine-3'-phosphate
  modified_base 8: mod_base = OTHER; note = 2'-deoxy-2'-fluoroadenosine-3'-phosphate
  modified_base 9: mod_base = OTHER; note = 2'-deoxy-2'-fluoroadenosine-3'-phosphate
  modified_base 10: mod_base = OTHER; note = 2'-O-methyladenosine-3'-phosphate
  modified_base 11: mod_base = OTHER; note = 2'-O-methyluridine-3'-phosphate
  modified_base 12: mod_base = OTHER; note = 2'-O-methylguanosine-3'-phosphate
  modified_base 13: mod_base = OTHER; note = 2'-O-methylcytidine-3'-phosphate
  modified_base 14: mod_base = OTHER; note = 2'-deoxy-2'-fluoroadenosine-3'-phosphate
  modified_base 15: mod_base = OTHER; note = 2'-O-methyluridine-3'-phosphate
  modified_base 16: mod_base = OTHER; note = 2'-deoxy-2'-fluoroguanosine-3'-phosphate
  modified_base 17: mod_base = OTHER; note = 2'-O-methylcytidine-3'-phosphate
  modified_base 18: mod_base = OTHER; note = 2'-O-methyladenosine-3'-phosphate
  modified_base 19: mod_base = OTHER; note = 2'-O-methyluridine-3'-phosphate
  modified_base 20: mod_base = OTHER; note = 2'-O-methyladenosine-3'-phosphate
  modified_base 21: mod_base = OTHER; note = 2'-O-methyluridine-3'-phosphorothioate
  modified_base 22: mod_base = OTHER; note = 2'-O-methyluridine-3'-phosphorothioate
  modified_base 23: mod_base = OTHER; note = 2'-O-methylcytidine
agttacaaaatgcatgcatattc

SEQ ID NO: 546 - RNA, 23 nt, synthetic construct
  source 1..23: mol_type = other RNA
  modified_base 1: mod_base = OTHER; note = 2'-O-methyladenosine-3'-phosphorothioate
  modified_base 2: mod_base = OTHER; note = 2'-deoxy-2'-fluoroadenosine-3'-phosphorothioate
  modified_base 3: mod_base = OTHER; note = 2'-O-methyladenosine-3'-phosphate
  modified_base 4: mod_base = OTHER; note = 2'-O-methyladenosine-3'-phosphate
  modified_base 5: mod_base = OTHER; note = 2'-O-methyluridine-3'-phosphate
  modified_base 6: mod_base = OTHER; note = 2'-deoxy-2'-fluoroadenosine-3'-phosphate
  modified_base 7: mod_base = OTHER; note = 2'-O-methylcytidine-3'-phosphate
  modified_base 8: mod_base = OTHER; note = 2'-deoxy-2'-fluoroadenosine-3'-phosphate
  modified_base 9: mod_base = OTHER; note = 2'-deoxy-2'-fluorocytidine-3'-phosphate
  modified_base 10: mod_base = OTHER; note = 2'-O-methyladenosine-3'-phosphate
  modified_base 11: mod_base = OTHER; note = 2'-O-methyluridine-3'-phosphate
  modified_base 12: mod_base = OTHER; note = 2'-O-methylcytidine-3'-phosphate
  modified_base 13: mod_base = OTHER; note = 2'-O-methyluridine-3'-phosphate
  modified_base 14: mod_base = OTHER; note = 2'-deoxy-2'-fluoroadenosine-3'-phosphate
  modified_base 15: mod_base = OTHER; note = 2'-O-methyluridine-3'-phosphate
  modified_base 16: mod_base = OTHER; note = 2'-deoxy-2'-fluorouridine-3'-phosphate
  modified_base 17: mod_base = OTHER; note = 2'-O-methylcytidine-3'-phosphate
  modified_base 18: mod_base = OTHER; note = 2'-O-methyladenosine-3'-phosphate
  modified_base 19: mod_base = OTHER; note = 2'-O-methyladenosine-3'-phosphate
  modified_base 20: mod_base = OTHER; note = 2'-O-methylcytidine-3'-phosphate
  modified_base 21: mod_base = OTHER; note = 2'-O-methylguanosine-3'-phosphorothioate
  modified_base 22: mod_base = OTHER; note = 2'-O-methylcytidine-3'-phosphorothioate
  modified_base 23: mod_base = OTHER; note = 2'-O-methylcytidine
aaaatacacatctattcaacgcc

SEQ ID NO: 547 - RNA, 23 nt, synthetic construct
  source 1..23: mol_type = other RNA
  modified_base 1: mod_base = OTHER; note = 2'-O-methyladenosine-3'-phosphorothioate
  modified_base 2: mod_base = OTHER; note = 2'-deoxy-2'-fluoroadenosine-3'-phosphorothioate
  modified_base 3: mod_base = OTHER; note = 2'-O-methyladenosine-3'-phosphate
  modified_base 4: mod_base = OTHER; note = 2'-O-methyluridine-3'-phosphate
  modified_base 5: mod_base = OTHER; note = 2'-O-methyluridine-3'-phosphate
  modified_base 6: mod_base = OTHER; note = 2'-deoxy-2'-fluorouridine-3'-phosphate
  modified_base 7: mod_base = OTHER; note = 2'-O-methyluridine-3'-phosphate
  modified_base 8: mod_base = OTHER; note = 2'-deoxy-2'-fluorocytidine-3'-phosphate
  modified_base 9: mod_base = OTHER; note = 2'-deoxy-2'-fluorouridine-3'-phosphate
  modified_base 10: mod_base = OTHER; note = 2'-O-methylguanosine-3'-phosphate
  modified_base 11: mod_base = OTHER; note = 2'-O-methyluridine-3'-phosphate
  modified_base 12: mod_base = OTHER; note = 2'-O-methylguanosine-3'-phosphate
  modified_base 13: mod_base = OTHER; note = 2'-O-methylcytidine-3'-phosphate
  modified_base 14: mod_base = OTHER; note = 2'-deoxy-2'-fluorouridine-3'-phosphate
  modified_base 15: mod_base = OTHER; note = 2'-O-methyluridine-3'-phosphate
  modified_base 16: mod_base = OTHER; note = 2'-deoxy-2'-fluoroadenosine-3'-phosphate
  modified_base 17: mod_base = OTHER; note = 2'-O-methyluridine-3'-phosphate
  modified_base 18: mod_base = OTHER; note = 2'-O-methyluridine-3'-phosphate
  modified_base 19: mod_base = OTHER; note = 2'-O-methyluridine-3'-phosphate
  modified_base 20: mod_base = OTHER; note = 2'-O-methyluridine-3'-phosphate
  modified_base 21: mod_base = OTHER; note = 2'-O-methylcytidine-3'-phosphorothioate
  modified_base 22: mod_base = OTHER; note = 2'-O-methyluridine-3'-phosphorothioate
  modified_base 23: mod_base = OTHER; note = 2'-O-methylguanosine
aaattttctgtgcttattttctg

SEQ ID NO: 548 - RNA, 23 nt, synthetic construct
  source 1..23: mol_type = other RNA
  modified_base 1: mod_base = OTHER; note = 2'-O-methyladenosine-3'-phosphorothioate
  modified_base 2: mod_base = OTHER; note = 2'-deoxy-2'-fluoroadenosine-3'-phosphorothioate
  modified_base 3: mod_base = OTHER; note = 2'-O-methyluridine-3'-phosphate
  modified_base 4: mod_base = OTHER; note = 2'-O-methyluridine-3'-phosphate
  modified_base 5: mod_base = OTHER; note = 2'-O-methylcytidine-3'-phosphate
  modified_base 6: mod_base = OTHER; note = 2'-deoxy-2'-fluorouridine-3'-phosphate
  modified_base 7: mod_base = OTHER; note = 2'-O-methylguanosine-3'-phosphate
  modified_base 8: mod_base = OTHER; note = 2'-deoxy-2'-fluoroadenosine-3'-phosphate
  modified_base 9: mod_base = OTHER; note = 2'-deoxy-2'-fluorouridine-3'-phosphate
  modified_base 10: mod_base = OTHER; note = 2'-O-methyladenosine-3'-phosphate
  modified_base 11: mod_base = OTHER; note = 2'-O-methylcytidine-3'-phosphate
  modified_base 12: mod_base = OTHER; note = 2'-O-methylguanosine-3'-phosphate
  modified_base 13: mod_base = OTHER; note = 2'-O-methyluridine-3'-phosphate
  modified_base 14: mod_base = OTHER; note = 2'-deoxy-2'-fluorouridine-3'-phosphate
  modified_base 15: mod_base = OTHER; note = 2'-O-methylcytidine-3'-phosphate
  modified_base 16: mod_base = OTHER; note = 2'-deoxy-2'-fluoroadenosine-3'-phosphate
  modified_base 17: mod_base = OTHER; note = 2'-O-methylguanosine-3'-phosphate
  modified_base 18: mod_base = OTHER; note = 2'-O-methyluridine-3'-phosphate
  modified_base 19: mod_base = OTHER; note = 2'-O-methylguanosine-3'-phosphate
  modified_base 20: mod_base = OTHER; note = 2'-O-methyladenosine-3'-phosphate
  modified_base 21: mod_base = OTHER; note = 2'-O-methyladenosine-3'-phosphorothioate
  modified_base 22: mod_base = OTHER; note = 2'-O-methyladenosine-3'-phosphorothioate
  modified_base 23: mod_base = OTHER; note = 2'-O-methyladenosine
aattctgatacgttcagtgaaaa

SEQ ID NO: 549 - RNA, 23 nt, synthetic construct
  source 1..23: mol_type = other RNA
  modified_base 1: mod_base = OTHER; note = 2'-O-methyladenosine-3'-phosphorothioate
  modified_base 2: mod_base = OTHER; note = 2'-deoxy-2'-fluorocytidine-3'-phosphorothioate
  modified_base 3: mod_base = OTHER; note = 2'-O-methyluridine-3'-phosphate
  modified_base 4: mod_base = OTHER; note = 2'-O-methylguanosine-3'-phosphate
  modified_base 5: mod_base = OTHER; note = 2'-O-methyladenosine-3'-phosphate
  modified_base 6: mod_base = OTHER; note = 2'-deoxy-2'-fluoroadenosine-3'-phosphate
  modified_base 7: mod_base = OTHER; note = 2'-O-methyluridine-3'-phosphate
  modified_base 8: mod_base = OTHER; note = 2'-deoxy-2'-fluorouridine-3'-phosphate
  modified_base 9: mod_base = OTHER; note = 2'-deoxy-2'-fluoroadenosine-3'-phosphate
  modified_base 10: mod_base = OTHER; note = 2'-O-methyladenosine-3'-phosphate
  modified_base 11: mod_base = OTHER; note = 2'-O-methyladenosine-3'-phosphate
  modified_base 12: mod_base = OTHER; note = 2'-O-methyladenosine-3'-phosphate
  modified_base 13: mod_base = OTHER; note = 2'-O-methylcytidine-3'-phosphate
  modified_base 14: mod_base = OTHER; note = 2'-deoxy-2'-fluorocytidine-3'-phosphate
  modified_base 15: mod_base = OTHER; note = 2'-O-methyluridine-3'-phosphate
  modified_base 16: mod_base = OTHER; note = 2'-deoxy-2'-fluorouridine-3'-phosphate
  modified_base 17: mod_base = OTHER; note = 2'-O-methyladenosine-3'-phosphate
  modified_base 18: mod_base = OTHER; note = 2'-O-methyluridine-3'-phosphate
  modified_base 19: mod_base = OTHER; note = 2'-O-methyluridine-3'-phosphate
  modified_base 20: mod_base = OTHER; note = 2'-O-methyluridine-3'-phosphate
  modified_base 21: mod_base = OTHER; note = 2'-O-methyladenosine-3'-phosphorothioate
  modified_base 22: mod_base = OTHER; note = 2'-O-methylcytidine-3'-phosphorothioate
  modified_base 23: mod_base = OTHER; note = 2'-O-methylcytidine
actgaattaaaaccttatttacc

SEQ ID NO: 550 - RNA, 23 nt, synthetic construct
  source 1..23: mol_type = other RNA
  modified_base 1: mod_base = OTHER; note = 2'-O-methyladenosine-3'-phosphorothioate
  modified_base 2: mod_base = OTHER; note = 2'-deoxy-2'-fluoroadenosine-3'-phosphorothioate
  modified_base 3: mod_base = OTHER; note = 2'-O-methyladenosine-3'-phosphate
  modified_base 4: mod_base = OTHER; note = 2'-O-methyluridine-3'-phosphate
  modified_base 5: mod_base = OTHER; note = 2'-O-methyladenosine-3'-phosphate
  modified_base 6: mod_base = OTHER; note = 2'-deoxy-2'-fluorocytidine-3'-phosphate
  modified_base 7: mod_base = OTHER; note = 2'-O-methyluridine-3'-phosphate
  modified_base 8: mod_base = OTHER; note = 2'-deoxy-2'-fluorouridine-3'-phosphate
  modified_base 9: mod_base = OTHER; note = 2'-deoxy-2'-fluorouridine-3'-phosphate
  modified_base 10: mod_base = OTHER; note = 2'-O-methylcytidine-3'-phosphate
  modified_base 11: mod_base = OTHER; note = 2'-O-methyluridine-3'-phosphate
  modified_base 12: mod_base = OTHER; note = 2'-O-methyluridine-3'-phosphate
  modified_base 13: mod_base = OTHER; note = 2'-O-methylcytidine-3'-phosphate
  modified_base 14: mod_base = OTHER; note = 2'-deoxy-2'-fluorouridine-3'-phosphate
  modified_base 15: mod_base = OTHER; note = 2'-O-methyladenosine-3'-phosphate
  modified_base 16: mod_base = OTHER; note = 2'-deoxy-2'-fluoroguanosine-3'-phosphate
  modified_base 17: mod_base = OTHER; note = 2'-O-methyladenosine-3'-phosphate
  modified_base 18: mod_base = OTHER; note = 2'-O-methyluridine-3'-phosphate
  modified_base 19: mod_base = OTHER; note = 2'-O-methylcytidine-3'-phosphate
  modified_base 20: mod_base = OTHER; note = 2'-O-methyluridine-3'-phosphate
  modified_base 21: mod_base = OTHER; note = 2'-O-methylguanosine-3'-phosphorothioate
  modified_base 22: mod_base = OTHER; note = 2'-O-methyladenosine-3'-phosphorothioate
  modified_base 23: mod_base = OTHER; note = 2'-O-methyladenosine
aaatactttcttctagatctgaa

SEQ ID NO: 551 - RNA, 23 nt, synthetic construct
  source 1..23: mol_type = other RNA
  modified_base 1: mod_base = OTHER; note = 2'-O-methyladenosine-3'-phosphorothioate
  modified_base 2: mod_base = OTHER; note = 2'-deoxy-2'-fluorouridine-3'-phosphorothioate
  modified_base 3: mod_base = OTHER; note = 2'-O-methyladenosine-3'-phosphate
  modified_base 4: mod_base = OTHER; note = 2'-O-methyladenosine-3'-phosphate
  modified_base 5: mod_base = OTHER; note = 2'-O-methyladenosine-3'-phosphate
  modified_base 6: mod_base = OTHER; note = 2'-deoxy-2'-fluorocytidine-3'-phosphate
  modified_base 7: mod_base = OTHER; note = 2'-O-methyladenosine-3'-phosphate
  modified_base 8: mod_base = OTHER; note = 2'-deoxy-2'-fluorocytidine-3'-phosphate
  modified_base 9: mod_base = OTHER; note = 2'-deoxy-2'-fluorouridine-3'-phosphate
  modified_base 10: mod_base = OTHER; note = 2'-O-methyladenosine-3'-phosphate
  modified_base 11: mod_base = OTHER; note = 2'-O-methylcytidine-3'-phosphate
  modified_base 12: mod_base = OTHER; note = 2'-O-methyladenosine-3'-phosphate
  modified_base 13: mod_base = OTHER; note = 2'-O-methyladenosine-3'-phosphate
  modified_base 14: mod_base = OTHER; note = 2'-deoxy-2'-fluorocytidine-3'-phosphate
  modified_base 15: mod_base = OTHER; note = 2'-O-methyluridine-3'-phosphate
  modified_base 16: mod_base = OTHER; note = 2'-deoxy-2'-fluoroadenosine-3'-phosphate
  modified_base 17: mod_base = OTHER; note = 2'-O-methyluridine-3'-phosphate
  modified_base 18: mod_base = OTHER; note = 2'-O-methylcytidine-3'-phosphate
  modified_base 19: mod_base = OTHER; note = 2'-O-methyluridine-3'-phosphate
  modified_base 20: mod_base = OTHER; note = 2'-O-methylguanosine-3'-phosphate
  modified_base 21: mod_base = OTHER; note = 2'-O-methyluridine-3'-phosphorothioate
  modified_base 22: mod_base = OTHER; note = 2'-O-methylguanosine-3'-phosphorothioate
  modified_base 23: mod_base = OTHER; note = 2'-O-methylguanosine
ataaacactacaactatctgtgg

SEQ ID NO: 552 - RNA, 23 nt, synthetic construct
  source 1..23: mol_type = other RNA
  modified_base 1: mod_base = OTHER; note = 2'-O-methyladenosine-3'-phosphorothioate
  modified_base 2: mod_base = OTHER; note = 2'-deoxy-2'-fluorouridine-3'-phosphorothioate
  modified_base 3: mod_base = OTHER; note = 2'-O-methyladenosine-3'-phosphate
  modified_base 4: mod_base = OTHER; note = 2'-O-methyladenosine-3'-phosphate
  modified_base 5: mod_base = OTHER; note = 2'-O-methylguanosine-3'-phosphate
  modified_base 6: mod_base = OTHER; note = 2'-deoxy-2'-fluorouridine-3'-phosphate
  modified_base 7: mod_base = OTHER; note = 2'-O-methylcytidine-3'-phosphate
  modified_base 8: mod_base = OTHER; note = 2'-deoxy-2'-fluorouridine-3'-phosphate
  modified_base 9: mod_base = OTHER; note = 2'-deoxy-2'-fluorouridine-3'-phosphate
  modified_base 10: mod_base = OTHER; note = 2'-O-methyladenosine-3'-phosphate
  modified_base 11: mod_base = OTHER; note = 2'-O-methylguanosine-3'-phosphate
  modified_base 12: mod_base = OTHER; note = 2'-O-methyladenosine-3'-phosphate
  modified_base 13: mod_base = OTHER; note = 2'-O-methyladenosine-3'-phosphate
  modified_base 14: mod_base = OTHER; note = 2'-deoxy-2'-fluoroadenosine-3'-phosphate
  modified_base 15: mod_base = OTHER; note = 2'-O-methylcytidine-3'-phosphate
  modified_base 16: mod_base = OTHER; note = 2'-deoxy-2'-fluorocytidine-3'-phosphate
  modified_base 17: mod_base = OTHER; note = 2'-O-methyluridine-3'-phosphate
  modified_base 18: mod_base = OTHER; note = 2'-O-methylcytidine-3'-phosphate
  modified_base 19: mod_base = OTHER; note = 2'-O-methyladenosine-3'-phosphate
  modified_base 20: mod_base = OTHER; note = 2'-O-methyladenosine-3'-phosphate
  modified_base 21: mod_base = OTHER; note = 2'-O-methylcytidine-3'-phosphorothioate
  modified_base 22: mod_base = OTHER; note = 2'-O-methylguanosine-3'-phosphorothioate
  modified_base 23: mod_base = OTHER; note = 2'-O-methyladenosine
ataagtcttagaaacctcaacga

SEQ ID NO: 553 - RNA, 23 nt, synthetic construct
  source 1..23: mol_type = other RNA
  modified_base 1: mod_base = OTHER; note = 2'-O-methyladenosine-3'-phosphorothioate
  modified_base 2: mod_base = OTHER; note = 2'-deoxy-2'-fluoroadenosine-3'-phosphorothioate
  modified_base 3: mod_base = OTHER; note = 2'-O-methyladenosine-3'-phosphate
  modified_base 4: mod_base = OTHER; note = 2'-O-methylguanosine-3'-phosphate
  modified_base 5: mod_base = OTHER; note = 2'-O-methyluridine-3'-phosphate
  modified_base 6: mod_base = OTHER; note = 2'-deoxy-2'-fluorocytidine-3'-phosphate
  modified_base 7: mod_base = OTHER; note = 2'-O-methyluridine-3'-phosphate
  modified_base 8: mod_base = OTHER; note = 2'-deoxy-2'-fluorocytidine-3'-phosphate
  modified_base 9: mod_base = OTHER; note = 2'-deoxy-2'-fluoroadenosine-3'-phosphate
  modified_base 10: mod_base = OTHER; note = 2'-O-methylguanosine-3'-phosphate
  modified_base 11: mod_base = OTHER; note = 2'-O-methylguanosine-3'-phosphate
  modified_base 12: mod_base = OTHER; note = 2'-O-methyluridine-3'-phosphate
  modified_base 13: mod_base = OTHER; note = 2'-O-methyluridine-3'-phosphate
  modified_base 14: mod_base = OTHER; note = 2'-deoxy-2'-fluorouridine-3'-phosphate
  modified_base 15: mod_base = OTHER; note = 2'-O-methylcytidine-3'-phosphate
  modified_base 16: mod_base = OTHER; note = 2'-deoxy-2'-fluorouridine-3'-phosphate
  modified_base 17: mod_base = OTHER; note = 2'-O-methyladenosine-3'-phosphate
  modified_base 18: mod_base = OTHER; note = 2'-O-methyladenosine-3'-phosphate
  modified_base 19: mod_base = OTHER; note = 2'-O-methyladenosine-3'-phosphate
  modified_base 20: mod_base = OTHER; note = 2'-O-methyladenosine-3'-phosphate
  modified_base 21: mod_base = OTHER; note = 2'-O-methyluridine-3'-phosphorothioate
  modified_base 22: mod_base = OTHER; note = 2'-O-methyladenosine-3'-phosphorothioate
  modified_base 23: mod_base = OTHER; note = 2'-O-methylguanosine
aaagtctcaggtttctaaaatag

SEQ ID NO: 554 - RNA, 23 nt, synthetic construct
  source 1..23: mol_type = other RNA
  modified_base 1: mod_base = OTHER; note = 2'-O-methyladenosine-3'-phosphorothioate
  modified_base 2: mod_base = OTHER; note = 2'-deoxy-2'-fluorouridine-3'-phosphorothioate
  modified_base 3: mod_base = OTHER; note = 2'-O-methyladenosine-3'-phosphate
  modified_base 4: mod_base = OTHER; note = 2'-O-methyluridine-3'-phosphate
  modified_base 5: mod_base = OTHER; note = 2'-O-methyluridine-3'-phosphate
  modified_base 6: mod_base = OTHER; note = 2'-deoxy-2'-fluoroadenosine-3'-phosphate
  modified_base 7: mod_base = OTHER; note = 2'-O-methyladenosine-3'-phosphate
  modified_base 8: mod_base = OTHER; note = 2'-deoxy-2'-fluoroadenosine-3'-phosphate
  modified_base 9: mod_base = OTHER; note = 2'-deoxy-2'-fluorocytidine-3'-phosphate
  modified_base 10: mod_base = OTHER; note = 2'-O-methyluridine-3'-phosphate
  modified_base 11: mod_base = OTHER; note = 2'-O-methyladenosine-3'-phosphate
  modified_base 12: mod_base = OTHER; note = 2'-O-methyladenosine-3'-phosphate
  modified_base 13: mod_base = OTHER; note = 2'-O-methyladenosine-3'-phosphate
  modified_base 14: mod_base = OTHER; note = 2'-deoxy-2'-fluoroadenosine-3'-phosphate
  modified_base 15: mod_base = OTHER; note = 2'-O-methyluridine-3'-phosphate
  modified_base 16: mod_base = OTHER; note = 2'-deoxy-2'-fluoroguanosine-3'-phosphate
  modified_base 17: mod_base = OTHER; note = 2'-O-methylcytidine-3'-phosphate
  modified_base 18: mod_base = OTHER; note = 2'-O-methylcytidine-3'-phosphate
  modified_base 19: mod_base = OTHER; note = 2'-O-methyladenosine-3'-phosphate
  modified_base 20: mod_base = OTHER; note = 2'-O-methylguanosine-3'-phosphate
  modified_base 21: mod_base = OTHER; note = 2'-O-methyladenosine-3'-phosphorothioate
  modified_base 22: mod_base = OTHER; note = 2'-O-methylcytidine-3'-phosphorothioate
  modified_base 23: mod_base = OTHER; note = 2'-O-methylguanosine
atattaaactaaaatgccagacg

SEQ ID NO: 555 - RNA, 23 nt, synthetic construct
  source 1..23: mol_type = other RNA
  modified_base 1: mod_base = OTHER; note = 2'-O-methyladenosine-3'-phosphorothioate
  modified_base 2: mod_base = OTHER; note = 2'-deoxy-2'-fluorouridine-3'-phosphorothioate
  modified_base 3: mod_base = OTHER; note = 2'-O-methyluridine-3'-phosphate
  modified_base 4: mod_base = OTHER; note = 2'-O-methylcytidine-3'-phosphate
  modified_base 5: mod_base = OTHER; note = 2'-O-methyladenosine-3'-phosphate
  modified_base 6: mod_base = OTHER; note = 2'-deoxy-2'-fluoroadenosine-3'-phosphate
  modified_base 7: mod_base = OTHER; note = 2'-O-methyladenosine-3'-phosphate
  modified_base 8: mod_base = OTHER; note = 2'-deoxy-2'-fluorouridine-3'-phosphate
  modified_base 9: mod_base = OTHER; note = 2'-deoxy-2'-fluoroguanosine-3'-phosphate
  modified_base 10: mod_base = OTHER; note = 2'-O-methylcytidine-3'-phosphate
  modified_base 11: mod_base = OTHER; note = 2'-O-methyladenosine-3'-phosphate
  modified_base 12: mod_base = OTHER; note = 2'-O-methyladenosine-3'-phosphate
  modified_base 13: mod_base = OTHER; note = 2'-O-methyluridine-3'-phosphate
  modified_base 14: mod_base = OTHER; note = 2'-deoxy-2'-fluorocytidine-3'-phosphate
  modified_base 15: mod_base = OTHER; note = 2'-O-methyladenosine-3'-phosphate
  modified_base 16: mod_base = OTHER; note = 2'-deoxy-2'-fluorouridine-3'-phosphate
  modified_base 17: mod_base = OTHER; note = 2'-O-methyluridine-3'-phosphate
  modified_base 18: mod_base = OTHER; note = 2'-O-methyladenosine-3'-phosphate
  modified_base 19: mod_base = OTHER; note = 2'-O-methylguanosine-3'-phosphate
  modified_base 20: mod_base = OTHER; note = 2'-O-methyluridine-3'-phosphate
  modified_base 21: mod_base = OTHER; note = 2'-O-methyluridine-3'-phosphorothioate
  modified_base 22: mod_base = OTHER; note = 2'-O-methyluridine-3'-phosphorothioate
  modified_base 23: mod_base = OTHER; note = 2'-O-methylguanosine
attcaaatgcaatcattagtttg

SEQ ID NO: 556 - RNA, 23 nt, synthetic construct
  source 1..23: mol_type = other RNA
  modified_base 1: mod_base = OTHER; note = 2'-O-methyladenosine-3'-phosphorothioate
  modified_base 2: mod_base = OTHER; note = 2'-deoxy-2'-fluoroadenosine-3'-phosphorothioate
  modified_base 3: mod_base = OTHER; note = 2'-O-methyluridine-3'-phosphate
  modified_base 4: mod_base = OTHER; note = 2'-O-methyladenosine-3'-phosphate
  modified_base 5: mod_base = OTHER; note = 2'-O-methyladenosine-3'-phosphate
  modified_base 6: mod_base = OTHER; note = 2'-deoxy-2'-fluoroguanosine-3'-phosphate
  modified_base 7: mod_base = OTHER; note = 2'-O-methylguanosine-3'-phosphate
  modified_base 8: mod_base = OTHER; note = 2'-deoxy-2'-fluorouridine-3'-phosphate
  modified_base 9: mod_base = OTHER; note = 2'-deoxy-2'-fluorocytidine-3'-phosphate
  modified_base 10: mod_base = OTHER; note = 2'-O-methyladenosine-3'-phosphate
  modified_base 11: mod_base = OTHER; note = 2'-O-methyladenosine-3'-phosphate
  modified_base 12: mod_base = OTHER; note = 2'-O-methylguanosine-3'-phosphate
  modified_base 13: mod_base = OTHER; note = 2'-O-methyladenosine-3'-phosphate
  modified_base 14: mod_base = OTHER; note = 2'-deoxy-2'-fluoroadenosine-3'-phosphate
  modified_base 15: mod_base = OTHER; note = 2'-O-methyluridine-3'-phosphate
  modified_base 16: mod_base = OTHER; note = 2'-deoxy-2'-fluorocytidine-3'-phosphate
  modified_base 17: mod_base = OTHER; note = 2'-O-methyluridine-3'-phosphate
  modified_base 18: mod_base = OTHER; note = 2'-O-methylcytidine-3'-phosphate
  modified_base 19: mod_base = OTHER; note = 2'-O-methyluridine-3'-phosphate
  modified_base 20: mod_base = OTHER; note = 2'-O-methyluridine-3'-phosphate
  modified_base 21: mod_base = OTHER; note = 2'-O-methyluridine-3'-phosphorothioate
  modified_base 22: mod_base = OTHER; note = 2'-O-methylcytidine-3'-phosphorothioate
  modified_base 23: mod_base = OTHER; note = 2'-O-methyladenosine
aataaggtcaagaatctctttca

SEQ ID NO: 557 - RNA, 23 nt, synthetic construct
  source 1..23: mol_type = other RNA
  modified_base 1: mod_base = OTHER; note = 2'-O-methyladenosine-3'-phosphorothioate
  modified_base 2: mod_base = OTHER; note = 2'-deoxy-2'-fluoroadenosine-3'-phosphorothioate
  modified_base 3: mod_base = OTHER; note = 2'-O-methyluridine-3'-phosphate
  modified_base 4: mod_base = OTHER; note = 2'-O-methylcytidine-3'-phosphate
  modified_base 5: mod_base = OTHER; note = 2'-O-methyladenosine-3'-phosphate
  modified_base 6: mod_base = OTHER; note = 2'-deoxy-2'-fluoroadenosine-3'-phosphate
  modified_base 7: mod_base = OTHER; note = 2'-O-methylguanosine-3'-phosphate
  modified_base 8: mod_base = OTHER; note = 2'-deoxy-2'-fluoroadenosine-3'-phosphate
  modified_base 9: mod_base = OTHER; note = 2'-deoxy-2'-fluorocytidine-3'-phosphate
  modified_base 10: mod_base = OTHER; note = 2'-O-methyladenosine-3'-phosphate
  modified_base 11: mod_base = OTHER; note = 2'-O-methyluridine-3'-phosphate
  modified_base 12: mod_base = OTHER; note = 2'-O-methyluridine-3'-phosphate
  modified_base 13: mod_base = OTHER; note = 2'-O-methyluridine-3'-phosphate
  modified_base 14: mod_base = OTHER; note = 2'-deoxy-2'-fluorocytidine-3'-phosphate
  modified_base 15: mod_base = OTHER; note = 2'-O-methyladenosine-3'-phosphate
  modified_base 16: mod_base = OTHER; note = 2'-deoxy-2'-fluoroguanosine-3'-phosphate
  modified_base 17: mod_base = OTHER; note = 2'-O-methyladenosine-3'-phosphate
  modified_base 18: mod_base = OTHER; note = 2'-O-methylguanosine-3'-phosphate
  modified_base 19: mod_base = OTHER; note = 2'-O-methylcytidine-3'-phosphate
  modified_base 20: mod_base = OTHER; note = 2'-O-methyluridine-3'-phosphate
  modified_base 21: mod_base = OTHER; note = 2'-O-methylcytidine-3'-phosphorothioate
  modified_base 22: mod_base = OTHER; note = 2'-O-methyluridine-3'-phosphorothioate
  modified_base 23: mod_base = OTHER; note = 2'-O-methyladenosine
aatcaagacatttcagagctcta

SEQ ID NO: 558 - RNA, 23 nt, synthetic construct
  source 1..23: mol_type = other RNA
  modified_base 1: mod_base = OTHER; note = 2'-O-methyladenosine-3'-phosphorothioate
  modified_base 2: mod_base = OTHER; note = 2'-deoxy-2'-fluoroadenosine-3'-phosphorothioate
  modified_base 3: mod_base = OTHER; note = 2'-O-methyladenosine-3'-phosphate
  modified_base 4: mod_base = OTHER; note = 2'-O-methyladenosine-3'-phosphate
  modified_base 5: mod_base = OTHER; note = 2'-O-methyluridine-3'-phosphate
  modified_base 6: mod_base = OTHER; note = 2'-deoxy-2'-fluoroadenosine-3'-phosphate
  modified_base 7: mod_base = OTHER; note = 2'-O-methylguanosine-3'-phosphate
  modified_base 8: mod_base = OTHER; note = 2'-deoxy-2'-fluorouridine-3'-phosphate
  modified_base 9: mod_base = OTHER; note = 2'-deoxy-2'-fluorouridine-3'-phosphate
  modified_base 10: mod_base = OTHER; note = 2'-O-methyluridine-3'-phosphate
  modified_base 11: mod_base = OTHER; note = 2'-O-methyladenosine-3'-phosphate
  modified_base 12: mod_base = OTHER; note = 2'-O-methyladenosine-3'-phosphate
  modified_base 13: mod_base = OTHER; note = 2'-O-methyluridine-3'-phosphate
  modified_base 14: mod_base = OTHER; note = 2'-deoxy-2'-fluoroadenosine-3'-phosphate
  modified_base 15: mod_base = OTHER; note = 2'-O-methylcytidine-3'-phosphate
  modified_base 16: mod_base = OTHER; note = 2'-deoxy-2'-fluorocytidine-3'-phosphate
  modified_base 17: mod_base = OTHER; note = 2'-O-methyluridine-3'-phosphate
  modified_base 18: mod_base = OTHER; note = 2'-O-methyluridine-3'-phosphate
  modified_base 19: mod_base = OTHER; note = 2'-O-methylcytidine-3'-phosphate
  modified_base 20: mod_base = OTHER; note = 2'-O-methylcytidine-3'-phosphate
  modified_base 21: mod_base = OTHER; note = 2'-O-methyladenosine-3'-phosphorothioate
  modified_base 22: mod_base = OTHER; note = 2'-O-methyluridine-3'-phosphorothioate
  modified_base 23: mod_base = OTHER; note = 2'-O-methylcytidine
aaaatagtttaataccttccatc

SEQ ID NO: 559 - RNA, 23 nt, synthetic construct
  source 1..23: mol_type = other RNA
  modified_base 1: mod_base = OTHER; note = 2'-O-methyladenosine-3'-phosphorothioate
  modified_base 2: mod_base = OTHER; note = 2'-deoxy-2'-fluoroadenosine-3'-phosphorothioate
  modified_base 3: mod_base = OTHER; note = 2'-O-methyluridine-3'-phosphate
  modified_base 4: mod_base = OTHER; note = 2'-O-methyluridine-3'-phosphate
  modified_base 5: mod_base = OTHER; note = 2'-O-methyluridine-3'-phosphate
  modified_base 6: mod_base = OTHER; note = 2'-deoxy-2'-fluorocytidine-3'-phosphate
  modified_base 7: mod_base = OTHER; note = 2'-O-methyluridine-3'-phosphate
  modified_base 8: mod_base = OTHER; note = 2'-deoxy-2'-fluorouridine-3'-phosphate
  modified_base 9: mod_base = OTHER; note = 2'-deoxy-2'-fluorouridine-3'-phosphate
  modified_base 10: mod_base = OTHER; note = 2'-O-methylguanosine-3'-phosphate
  modified_base 11: mod_base = OTHER; note = 2'-O-methyluridine-3'-phosphate
  modified_base 12: mod_base = OTHER; note = 2'-O-methyladenosine-3'-phosphate
  modified_base 13: mod_base = OTHER; note = 2'-O-methylcytidine-3'-phosphate
  modified_base 14: mod_base = OTHER; note = 2'-deoxy-2'-fluoroadenosine-3'-phosphate
  modified_base 15: mod_base = OTHER; note = 2'-O-methyladenosine-3'-phosphate
  modified_base 16: mod_base = OTHER; note = 2'-deoxy-2'-fluorocytidine-3'-phosphate
  modified_base 17: mod_base = OTHER; note = 2'-O-methyladenosine-3'-phosphate
  modified_base 18: mod_base = OTHER; note = 2'-O-methylguanosine-3'-phosphate
  modified_base 19: mod_base = OTHER; note = 2'-O-methylguanosine-3'-phosphate
  modified_base 20: mod_base = OTHER; note = 2'-O-methylcytidine-3'-phosphate
  modified_base 21: mod_base = OTHER; note = 2'-O-methyladenosine-3'-phosphorothioate
  modified_base 22: mod_base = OTHER; note = 2'-O-methyladenosine-3'-phosphorothioate
  modified_base 23: mod_base = OTHER; note = 2'-O-methyladenosine
aatttctttgtacaacaggcaaa

SEQ ID NO: 560 - RNA, 23 nt, synthetic construct
  source 1..23: mol_type = other RNA
  modified_base 1: mod_base = OTHER; note = 2'-O-methyladenosine-3'-phosphorothioate
  modified_base 2: mod_base = OTHER; note = 2'-deoxy-2'-fluorouridine-3'-phosphorothioate
  modified_base 3: mod_base = OTHER; note = 2'-O-methyladenosine-3'-phosphate
  modified_base 4: mod_base = OTHER; note = 2'-O-methylguanosine-3'-phosphate
  modified_base 5: mod_base = OTHER; note = 2'-O-methyluridine-3'-phosphate
  modified_base 6: mod_base = OTHER; note = 2'-deoxy-2'-fluoroadenosine-3'-phosphate
  modified_base 7: mod_base = OTHER; note = 2'-O-methyladenosine-3'-phosphate
  modified_base 8: mod_base = OTHER; note = 2'-deoxy-2'-fluorouridine-3'-phosphate
  modified_base 9: mod_base = OTHER; note = 2'-deoxy-2'-fluorouridine-3'-phosphate
  modified_base 10: mod_base = OTHER; note = 2'-O-methylcytidine-3'-phosphate
  modified_base 11: mod_base = OTHER; note = 2'-O-methyluridine-3'-phosphate
  modified_base 12: mod_base = OTHER; note = 2'-O-methyluridine-3'-phosphate
  modified_base 13: mod_base = OTHER; note = 2'-O-methyluridine-3'-phosphate
  modified_base 14: mod_base = OTHER; note = 2'-deoxy-2'-fluorouridine-3'-phosphate
  modified_base 15: mod_base = OTHER; note = 2'-O-methylcytidine-3'-phosphate
  modified_base 16: mod_base = OTHER; note = 2'-deoxy-2'-fluoroadenosine-3'-phosphate
  modified_base 17: mod_base = OTHER; note = 2'-O-methylcytidine-3'-phosphate
  modified_base 18: mod_base = OTHER; note = 2'-O-methylguanosine-3'-phosphate
  modified_base 19: mod_base = OTHER; note = 2'-O-methyladenosine-3'-phosphate
  modified_base 20: mod_base = OTHER; note = 2'-O-methylguanosine-3'-phosphate
  modified_base 21: mod_base = OTHER; note = 2'-O-methyluridine-3'-phosphorothioate
  modified_base 22: mod_base = OTHER; note = 2'-O-methylcytidine-3'-phosphorothioate
  modified_base 23: mod_base = OTHER; note = 2'-O-methyluridine
atagtaattcttttcacgagtct

SEQ ID NO: 561 - RNA, 23 nt, synthetic construct
  source 1..23: mol_type = other RNA
  modified_base 1: mod_base = OTHER; note = 2'-O-methyladenosine-3'-phosphorothioate
  modified_base 2: mod_base = OTHER; note = 2'-deoxy-2'-fluoroadenosine-3'-phosphorothioate
  modified_base 3: mod_base = OTHER; note = 2'-O-methylcytidine-3'-phosphate
  modified_base 4: mod_base = OTHER; note = 2'-O-methyladenosine-3'-phosphate
  modified_base 5: mod_base = OTHER; note = 2'-O-methyladenosine-3'-phosphate
  modified_base 6: mod_base = OTHER; note = 2'-deoxy-2'-fluoroadenosine-3'-phosphate
  modified_base 7: mod_base = OTHER; note = 2'-O-methyladenosine-3'-phosphate
  modified_base 8: mod_base = OTHER; note = 2'-deoxy-2'-fluorouridine-3'-phosphate
  modified_base 9: mod_base = OTHER; note = 2'-deoxy-2'-fluorocytidine-3'-phosphate
  modified_base 10: mod_base = OTHER; note = 2'-O-methylguanosine-3'-phosphate
  modified_base 11: mod_base = OTHER; note = 2'-O-methylcytidine-3'-phosphate
  modified_base 12: mod_base = OTHER; note = 2'-O-methyladenosine-3'-phosphate
  modified_base 13: mod_base = OTHER; note = 2'-O-methylguanosine-3'-phosphate
  modified_base 14: mod_base = OTHER; note = 2'-deoxy-2'-fluorouridine-3'-phosphate
  modified_base 15: mod_base = OTHER; note = 2'-O-methyluridine-3'-phosphate
  modified_base 16: mod_base = OTHER; note = 2'-deoxy-2'-fluoroadenosine-3'-phosphate
  modified_base 17: mod_base = OTHER; note = 2'-O-methyluridine-3'-phosphate
  modified_base 18: mod_base = OTHER; note = 2'-O-methyluridine-3'-phosphate
  modified_base 19: mod_base = OTHER; note = 2'-O-methyluridine-3'-phosphate
  modified_base 20: mod_base = OTHER; note = 2'-O-methylcytidine-3'-phosphate
  modified_base 21: mod_base = OTHER; note = 2'-O-methyladenosine-3'-phosphorothioate
  modified_base 22: mod_base = OTHER; note = 2'-O-methylcytidine-3'-phosphorothioate
  modified_base 23: mod_base = OTHER; note = 2'-O-methyladenosine
aacaaaatcgcagttatttcaca

SEQ ID NO: 562 - RNA, 23 nt, synthetic construct
  source 1..23: mol_type = other RNA
  modified_base 1: mod_base = OTHER; note = 2'-O-methyladenosine-3'-phosphorothioate
  modified_base 2: mod_base = OTHER; note = 2'-deoxy-2'-fluoroadenosine-3'-phosphorothioate
  modified_base 3: mod_base = OTHER; note = 2'-O-methyladenosine-3'-phosphate
  modified_base 4: mod_base = OTHER; note = 2'-O-methyladenosine-3'-phosphate
  modified_base 5: mod_base = OTHER; note = 2'-O-methyluridine-3'-phosphate
  modified_base 6: mod_base = OTHER; note = 2'-deoxy-2'-fluorocytidine-3'-phosphate
  modified_base 7: mod_base = OTHER; note = 2'-O-methyladenosine-3'-phosphate
  modified_base 8: mod_base = OTHER; note = 2'-deoxy-2'-fluoroadenosine-3'-phosphate
  modified_base 9: mod_base = OTHER; note = 2'-deoxy-2'-fluorouridine-3'-phosphate
  modified_base 10: mod_base = OTHER; note = 2'-O-methylcytidine-3'-phosphate
  modified_base 11: mod_base = OTHER; note = 2'-O-methyladenosine-3'-phosphate
  modified_base 12: mod_base = OTHER; note = 2'-O-methylguanosine-3'-phosphate
  modified_base 13: mod_base = OTHER; note = 2'-O-methylcytidine-3'-phosphate
  modified_base 14: mod_base = OTHER; note = 2'-deoxy-2'-fluoroadenosine-3'-phosphate
  modified_base 15: mod_base = OTHER; note = 2'-O-methyluridine-3'-phosphate
  modified_base 16: mod_base = OTHER; note = 2'-deoxy-2'-fluorouridine-3'-phosphate
  modified_base 17: mod_base = OTHER; note = 2'-O-methyluridine-3'-phosphate
  modified_base 18: mod_base = OTHER; note = 2'-O-methylcytidine-3'-phosphate
  modified_base 19: mod_base = OTHER; note = 2'-O-methylcytidine-3'-phosphate
  modified_base 20: mod_base = OTHER; note = 2'-O-methyladenosine-3'-phosphate
  modified_base 21: mod_base = OTHER; note = 2'-O-methyladenosine-3'-phosphorothioate
  modified_base 22: mod_base = OTHER; note = 2'-O-methylguanosine-3'-phosphorothioate
  modified_base 23: mod_base = OTHER; note = 2'-O-methyluridine
aaaatcaatcagcatttccaagt

SEQ ID NO: 563 - RNA, 23 nt, synthetic construct
  source 1..23: mol_type = other RNA
  modified_base 1: mod_base = OTHER; note = 2'-O-methyladenosine-3'-phosphorothioate
  modified_base 2: mod_base = OTHER; note = 2'-deoxy-2'-fluorouridine-3'-phosphorothioate
  modified_base 3: mod_base = OTHER; note = 2'-O-methylguanosine-3'-phosphate
  modified_base 4: mod_base = OTHER; note = 2'-O-methyluridine-3'-phosphate
  modified_base 5: mod_base = OTHER; note = 2'-O-methyluridine-3'-phosphate
  modified_base 6: mod_base = OTHER; note = 2'-deoxy-2'-fluorouridine-3'-phosphate
  modified_base 7: mod_base = OTHER; note = 2'-O-methylcytidine-3'-phosphate
  modified_base 8: mod_base = OTHER; note = 2'-deoxy-2'-fluorouridine-3'-phosphate
  modified_base 9: mod_base = OTHER; note = 2'-deoxy-2'-fluorouridine-3'-phosphate
  modified_base 10: mod_base = OTHER; note = 2'-O-methylguanosine-3'-phosphate
  modified_base 11: mod_base = OTHER; note = 2'-O-methylcytidine-3'-phosphate
  modified_base 12: mod_base = OTHER; note = 2'-O-methyladenosine-3'-phosphate
  modified_base 13: mod_base = OTHER; note = 2'-O-methyladenosine-3'-phosphate
  modified_base 14: mod_base = OTHER; note = 2'-deoxy-2'-fluorouridine-3'-phosphate
  modified_base 15: mod_base = OTHER; note = 2'-O-methyladenosine-3'-phosphate
  modified_base 16: mod_base = OTHER; note = 2'-deoxy-2'-fluorocytidine-3'-phosphate
  modified_base 17: mod_base = OTHER; note = 2'-O-methyladenosine-3'-phosphate
  modified_base 18: mod_base = OTHER; note = 2'-O-methylcytidine-3'-phosphate
  modified_base 19: mod_base = OTHER; note = 2'-O-methyluridine-3'-phosphate
  modified_base 20: mod_base = OTHER; note = 2'-O-methyladenosine-3'-phosphate
  modified_base 21: mod_base = OTHER; note = 2'-O-methyladenosine-3'-phosphorothioate
  modified_base 22: mod_base = OTHER; note = 2'-O-methylcytidine-3'-phosphorothioate
  modified_base 23: mod_base = OTHER; note = 2'-O-methyladenosine
atgtttcttgcaatacactaaca

SEQ ID NO: 564 - RNA, 23 nt, synthetic construct
  source 1..23: mol_type = other RNA
  modified_base 1: mod_base = OTHER; note = 2'-O-methyladenosine-3'-phosphorothioate
  modified_base 2: mod_base = OTHER; note = 2'-deoxy-2'-fluoroadenosine-3'-phosphorothioate
  modified_base 3: mod_base = OTHER; note = 2'-O-methyladenosine-3'-phosphate
  modified_base 4: mod_base = OTHER; note = 2'-O-methyladenosine-3'-phosphate
  modified_base 5: mod_base = OTHER; note = 2'-O-methylcytidine-3'-phosphate
  modified_base 6: mod_base = OTHER; note = 2'-deoxy-2'-fluoroadenosine-3'-phosphate
  modified_base 7: mod_base = OTHER; note = 2'-O-methyladenosine-3'-phosphate
  modified_base 8: mod_base = OTHER; note = 2'-deoxy-2'-fluoroadenosine-3'-phosphate
  modified_base 9: mod_base = OTHER; note = 2'-deoxy-2'-fluoroadenosine-3'-phosphate
  modified_base 10: mod_base = OTHER; note = 2'-O-methylcytidine-3'-phosphate
  modified_base 11: mod_base = OTHER; note = 2'-O-methyluridine-3'-phosphate
  modified_base 12: mod_base = OTHER; note = 2'-O-methyladenosine-3'-phosphate
  modified_base 13: mod_base = OTHER; note = 2'-O-methylcytidine-3'-phosphate
  modified_base 14: mod_base = OTHER; note = 2'-deoxy-2'-fluoroadenosine-3'-phosphate
  modified_base 15: mod_base = OTHER; note = 2'-O-methyluridine-3'-phosphate
  modified_base 16: mod_base = OTHER; note = 2'-deoxy-2'-fluorouridine-3'-phosphate
  modified_base 17: mod_base = OTHER; note = 2'-O-methyluridine-3'-phosphate
  modified_base 18: mod_base = OTHER; note = 2'-O-methyluridine-3'-phosphate
  modified_base 19: mod_base = OTHER; note = 2'-O-methylcytidine-3'-phosphate
  modified_base 20: mod_base = OTHER; note = 2'-O-methyluridine-3'-phosphate
  modified_base 21: mod_base = OTHER; note = 2'-O-methylguanosine-3'-phosphorothioate
  modified_base 22: mod_base = OTHER; note = 2'-O-methyluridine-3'-phosphorothioate
  modified_base 23: mod_base = OTHER; note = 2'-O-methylguanosine
aaaacaaaactacattttctgtg

SEQ ID NO: 565 - RNA, 23 nt, synthetic construct
  source 1..23: mol_type = other RNA
  modified_base 4: mod_base = OTHER; note = 5'-methyluridine-3'-phosphate
  modified_base 7: mod_base = OTHER; note = 5'-methyluridine-3'-phosphate
  modified_base 12: mod_base = OTHER; note = 5'-methyluridine-3'-phosphate
  modified_base 13: mod_base = OTHER; note = 5'-methyluridine-3'-phosphate
  modified_base 14: mod_base = OTHER; note = 5'-methyluridine-3'-phosphate
  modified_base 15: mod_base = OTHER; note = 5'-methyluridine-3'-phosphate
  modified_base 17: mod_base = OTHER; note = 5'-methyluridine-3'-phosphate
  modified_base 19: mod_base = OTHER; note = 5'-methyluridine-3'-phosphate
  modified_base 20: mod_base = OTHER; note = 5'-methyluridine-3'-phosphate
  modified_base 22: mod_base = OTHER; note = 5'-methyluridine-3'-phosphate
gagtcctgaagttttatgttatg

SEQ ID NO: 566 - RNA, 23 nt, synthetic construct
  source 1..23: mol_type = other RNA
  modified_base 2: mod_base = OTHER; note = 5'-methyluridine-3'-phosphate
  modified_base 4: mod_base = OTHER; note = 5'-methyluridine-3'-phosphate
  modified_base 5: mod_base = OTHER; note = 5'-methyluridine-3'-phosphate
  modified_base 7: mod_base = OTHER; note = 5'-methyluridine-3'-phosphate
  modified_base 21: mod_base = OTHER; note = 5'-methyluridine-3'-phosphate
  modified_base 22: mod_base = OTHER; note = 5'-methyluridine-3'-phosphate
  modified_base 23: mod_base = OTHER; note = 5'-methyluridine
atgttatgaaacagaagaacttt

SEQ ID NO: 567 - RNA, 23 nt, synthetic construct
  source 1..23: mol_type = other RNA
  modified_base 3: mod_base = OTHER; note = 5'-methyluridine-3'-phosphate
  modified_base 6: mod_base = OTHER; note = 5'-methyluridine-3'-phosphate
  modified_base 7: mod_base = OTHER; note = 5'-methyluridine-3'-phosphate
  modified_base 8: mod_base = OTHER; note = 5'-methyluridine-3'-phosphate
  modified_base 14: mod_base = OTHER; note = 5'-methyluridine-3'-phosphate
  modified_base 15: mod_base = OTHER; note = 5'-methyluridine-3'-phosphate
  modified_base 20: mod_base = OTHER; note = 5'-methyluridine-3'-phosphate
  modified_base 21: mod_base = OTHER; note = 5'-methyluridine-3'-phosphate
  modified_base 22: mod_base = OTHER; note = 5'-methyluridine-3'-phosphate
catgatttgggaattacactttg

SEQ ID NO: 568 - RNA, 23 nt, synthetic construct
  source 1..23: mol_type = other RNA
  modified_base 1: mod_base = OTHER; note = 5'-methyluridine-3'-phosphate
  modified_base 4: mod_base = OTHER; note = 5'-methyluridine-3'-phosphate
  modified_base 9: mod_base = OTHER; note = 5'-methyluridine-3'-phosphate
  modified_base 13: mod_base = OTHER; note = 5'-methyluridine-3'-phosphate
  modified_base 15: mod_base = OTHER; note = 5'-methyluridine-3'-phosphate
  modified_base 16: mod_base = OTHER; note = 5'-methyluridine-3'-phosphate
  modified_base 17: mod_base = OTHER; note = 5'-methyluridine-3'-phosphate
  modified_base 19: mod_base = OTHER; note = 5'-methyluridine-3'-phosphate
  modified_base 20: mod_base = OTHER; note = 5'-methyluridine-3'-phosphate
  modified_base 22: mod_base = OTHER; note = 5'-methyluridine-3'-phosphate
tggtacaatagatgtttcttatc

SEQ ID NO: 569 - RNA, 23 nt, synthetic construct
  source 1..23: mol_type = other RNA
  modified_base 4: mod_base = OTHER; note = 5'-methyluridine-3'-phosphate
  modified_base 5: mod_base = OTHER; note = 5'-methyluridine-3'-phosphate
  modified_base 8: mod_base = OTHER; note = 5'-methyluridine-3'-phosphate
  modified_base 14: mod_base = OTHER; note = 5'-methyluridine-3'-phosphate
  modified_base 19: mod_base = OTHER; note = 5'-methyluridine-3'-phosphate
  modified_base 21: mod_base = OTHER; note = 5'-methyluridine-3'-phosphate
  modified_base 22: mod_base = OTHER; note = 5'-methyluridine-3'-phosphate
acattcatcagaatacagtgttg

SEQ ID NO: 570 - RNA, 23 nt, synthetic construct
  source 1..23: mol_type = other RNA
  modified_base 1: mod_base = OTHER; note = 5'-methyluridine-3'-phosphate
  modified_base 2: mod_base = OTHER; note = 5'-methyluridine-3'-phosphate
  modified_base 7: mod_base = OTHER; note = 5'-methyluridine-3'-phosphate
  modified_base 9: mod_base = OTHER; note = 5'-methyluridine-3'-phosphate
  modified_base 15: mod_base = OTHER; note = 5'-methyluridine-3'-phosphate
  modified_base 16: mod_base = OTHER; note = 5'-methyluridine-3'-phosphate
  modified_base 17: mod_base = OTHER; note = 5'-methyluridine-3'-phosphate
  modified_base 22: mod_base = OTHER; note = 5'-methyluridine-3'-phosphate
ttcagatctgcaactttaaaatg

SEQ ID NO: 571 - RNA, 23 nt, synthetic construct
  source 1..23: mol_type = other RNA
  modified_base 1: mod_base = OTHER; note = 5'-methyluridine-3'-phosphate
  modified_base 6: mod_base = OTHER; note = 5'-methyluridine-3'-phosphate
  modified_base 19: mod_base = OTHER; note = 5'-methyluridine-3'-phosphate
  modified_base 22: mod_base = OTHER; note = 5'-methyluridine-3'-phosphate
taaaatggaaagaaagcctaatg

SEQ ID NO: 572 - RNA, 23 nt, synthetic construct
  source 1..23: mol_type = other RNA
  modified_base 2: mod_base = OTHER; note = 5'-methyluridine-3'-phosphate
  modified_base 3: mod_base = OTHER; note = 5'-methyluridine-3'-phosphate
  modified_base 4: mod_base = OTHER; note = 5'-methyluridine-3'-phosphate
  modified_base 6: mod_base = OTHER; note = 5'-methyluridine-3'-phosphate
  modified_base 7: mod_base = OTHER; note = 5'-methyluridine-3'-phosphate
  modified_base 14: mod_base = OTHER; note = 5'-methyluridine-3'-phosphate
  modified_base 16: mod_base = OTHER; note = 5'-methyluridine-3'-phosphate
  modified_base 17: mod_base = OTHER; note = 5'-methyluridine-3'-phosphate
  modified_base 19: mod_base = OTHER; note = 5'-methyluridine-3'-phosphate
  modified_base 20: mod_base = OTHER; note = 5'-methyluridine-3'-phosphate
  modified_base 23: mod_base = OTHER; note = 5'-methyluridine
atttgttggaagatgttgttact

SEQ ID NO: 573 - RNA, 23 nt, synthetic construct
  source 1..23: mol_type = other RNA
  modified_base 1: mod_base = OTHER; note = 5'-methyluridine-3'-phosphate
  modified_base 2: mod_base = OTHER; note = 5'-methyluridine-3'-phosphate
  modified_base 9: mod_base = OTHER; note = 5'-methyluridine-3'-phosphate
  modified_base 11: mod_base = OTHER; note = 5'-methyluridine-3'-phosphate
  modified_base 12: mod_base = OTHER; note = 5'-methyluridine-3'-phosphate
  modified_base 14: mod_base = OTHER; note = 5'-methyluridine-3'-phosphate
  modified_base 15: mod_base = OTHER; note = 5'-methyluridine-3'-phosphate
  modified_base 16: mod_base = OTHER; note = 5'-methyluridine-3'-phosphate
  modified_base 18: mod_base = OTHER; note = 5'-methyluridine-3'-phosphate
  modified_base 20: mod_base = OTHER; note = 5'-methyluridine-3'-phosphate
ttgcggaatgttatttatatcaa

SEQ ID NO: 574 - RNA, 23 nt, synthetic construct
  source 1..23: mol_type = other RNA
  modified_base 1: mod_base = OTHER; note = 5'-methyluridine-3'-phosphate
  modified_base 3: mod_base = OTHER; note = 5'-methyluridine-3'-phosphate
  modified_base 5: mod_base = OTHER; note = 5'-methyluridine-3'-phosphate
  modified_base 9: mod_base = OTHER; note = 5'-methyluridine-3'-phosphate
  modified_base 15: mod_base = OTHER; note = 5'-methyluridine-3'-phosphate
tatatcaatgaaactcacacaag

SEQ ID NO: 575 - RNA, 23 nt, synthetic construct
  source 1..23: mol_type = other RNA
  modified_base 9: mod_base = OTHER; note = 5'-methyluridine-3'-phosphate
  modified_base 10: mod_base = OTHER; note = 5'-methyluridine-3'-phosphate
  modified_base 11: mod_base = OTHER; note = 5'-methyluridine-3'-phosphate
  modified_base 13: mod_base = OTHER; note = 5'-methyluridine-3'-phosphate
  modified_base 14: mod_base = OTHER; note = 5'-methyluridine-3'-phosphate
  modified_base 18: mod_base = OTHER; note = 5'-methyluridine-3'-phosphate
  modified_base 19: mod_base = OTHER; note = 5'-methyluridine-3'-phosphate
  modified_base 21: mod_base = OTHER; note = 5'-methyluridine-3'-phosphate
  modified_base 22: mod_base = OTHER; note = 5'-methyluridine-3'-phosphate
  modified_base 23: mod_base = OTHER; note = 5'-methyluridine
aagacgcctttcttacgttcttt

SEQ ID NO: 576 - RNA, 23 nt, synthetic construct
  source 1..23: mol_type = other RNA
  modified_base 8: mod_base = OTHER; note = 5'-methyluridine-3'-phosphate
  modified_base 10: mod_base = OTHER; note = 5'-methyluridine-3'-phosphate
  modified_base 14: mod_base = OTHER; note = 5'-methyluridine-3'-phosphate
  modified_base 20: mod_base = OTHER; note = 5'-methyluridine-3'-phosphate
  modified_base 22: mod_base = OTHER; note = 5'-methyluridine-3'-phosphate
ccaccaatgtgactgaaaatgtg

SEQ ID NO: 577 - RNA, 23 nt, synthetic construct
  source 1..23: mol_type = other RNA
  modified_base 9: mod_base = OTHER; note = 5'-methyluridine-3'-phosphate
  modified_base 10: mod_base = OTHER; note = 5'-methyluridine-3'-phosphate
  modified_base 18: mod_base = OTHER; note = 5'-methyluridine-3'-phosphate
aaaagccgttaacaaagtgaaaa

SEQ ID NO: 578 - RNA, 23 nt, synthetic construct
  source 1..23: mol_type = other RNA
  modified_base 2: mod_base = OTHER; note = 5'-methyluridine-3'-phosphate
  modified_base 10: mod_base = OTHER; note = 5'-methyluridine-3'-phosphate
  modified_base 11: mod_base = OTHER; note = 5'-methyluridine-3'-phosphate
  modified_base 13: mod_base = OTHER; note = 5'-methyluridine-3'-phosphate
  modified_base 14: mod_base = OTHER; note = 5'-methyluridine-3'-phosphate
  modified_base 22: mod_base = OTHER; note = 5'-methyluridine-3'-phosphate
ctaaaaggattcttcaagaaatg

SEQ ID NO: 579 - RNA, 23 nt, synthetic construct
  source 1..23: mol_type = other RNA
  modified_base 2: mod_base = OTHER; note = 5'-methyluridine-3'-phosphate
  modified_base 3: mod_base = OTHER; note = 5'-methyluridine-3'-phosphate
  modified_base 5: mod_base = OTHER; note = 5'-methyluridine-3'-phosphate
  modified_base 6: mod_base = OTHER; note = 5'-methyluridine-3'-phosphate
  modified_base 7: mod_base = OTHER; note = 5'-methyluridine-3'-phosphate
  modified_base 8: mod_base = OTHER; note = 5'-methyluridine-3'-phosphate
  modified_base 15: mod_base = OTHER; note = 5'-methyluridine-3'-phosphate
  modified_base 16: mod_base = OTHER; note = 5'-methyluridine-3'-phosphate
  modified_base 21: mod_base = OTHER; note = 5'-methyluridine-3'-phosphate
  modified_base 22: mod_base = OTHER; note = 5'-methyluridine-3'-phosphate
cttcttttggaacattcaaattc

SEQ ID NO: 580 - RNA, 23 nt, synthetic construct
  source 1..23: mol_type = other RNA
  modified_base 1: mod_base = OTHER; note = 5'-methyluridine-3'-phosphate
  modified_base 6: mod_base = OTHER; note = 5'-methyluridine-3'-phosphate
  modified_base 7: mod_base = OTHER; note = 5'-methyluridine-3'-phosphate
  modified_base 16: mod_base = OTHER; note = 5'-methyluridine-3'-phosphate
  modified_base 21: mod_base = OTHER; note = 5'-methyluridine-3'-phosphate
  modified_base 22: mod_base = OTHER; note = 5'-methyluridine-3'-phosphate
tcaaattcacaaaggtcaacttg

SEQ ID NO: 581 - RNA, 23 nt, synthetic construct
  source 1..23: mol_type = other RNA
  modified_base 1: mod_base = OTHER; note = 5'-methyluridine-3'-phosphate
  modified_base 3: mod_base = OTHER; note = 5'-methyluridine-3'-phosphate
  modified_base 4: mod_base = OTHER; note = 5'-methyluridine-3'-phosphate
  modified_base 5: mod_base = OTHER; note = 5'-methyluridine-3'-phosphate
  modified_base 7: mod_base = OTHER; note = 5'-methyluridine-3'-phosphate
  modified_base 13: mod_base = OTHER; note = 5'-methyluridine-3'-phosphate
  modified_base 14: mod_base = OTHER; note = 5'-methyluridine-3'-phosphate
  modified_base 17: mod_base = OTHER; note = 5'-methyluridine-3'-phosphate
  modified_base 21: mod_base = OTHER; note = 5'-methyluridine-3'-phosphate
tgtttctaccagttcatagatcc

SEQ ID NO: 582 - RNA, 23 nt, synthetic construct
  source 1..23: mol_type = other RNA
  modified_base 2: mod_base = OTHER; note = 5'-methyluridine-3'-phosphate
  modified_base 6: mod_base = OTHER; note = 5'-methyluridine-3'-phosphate
  modified_base 11: mod_base = OTHER; note = 5'-methyluridine-3'-phosphate
  modified_base 13: mod_base = OTHER; note = 5'-methyluridine-3'-phosphate
  modified_base 14: mod_base = OTHER; note = 5'-methyluridine-3'-phosphate
  modified_base 18: mod_base = OTHER; note = 5'-methyluridine-3'-phosphate
  modified_base 20: mod_base = OTHER; note = 5'-methyluridine-3'-phosphate
  modified_base 22: mod_base = OTHER; note = 5'-methyluridine-3'-phosphate
atagatcccatattgactatctg

SEQ ID NO: 583 - RNA, 23 nt, synthetic construct
  source 1..23: mol_type = other RNA
  modified_base 2: mod_base = OTHER; note = 5'-methyluridine-3'-phosphate
  modified_base 5: mod_base = OTHER; note = 5'-methyluridine-3'-phosphate
  modified_base 9: mod_base = OTHER; note = 5'-methyluridine-3'-phosphate
  modified_base 10: mod_base = OTHER; note = 5'-methyluridine-3'-phosphate
  modified_base 11: mod_base = OTHER; note = 5'-methyluridine-3'-phosphate
  modified_base 14: mod_base = OTHER; note = 5'-methyluridine-3'-phosphate
  modified_base 15: mod_base = OTHER; note = 5'-methyluridine-3'-phosphate
  modified_base 17: mod_base = OTHER; note = 5'-methyluridine-3'-phosphate
  modified_base 19: mod_base = OTHER; note = 5'-methyluridine-3'-phosphate
  modified_base 20: mod_base = OTHER; note = 5'-methyluridine-3'-phosphate
  modified_base 22: mod_base = OTHER; note = 5'-methyluridine-3'-phosphate
ctgctcactttcattctcttctg

SEQ ID NO: 584 - RNA, 23 nt, synthetic construct
  source 1..23: mol_type = other RNA
  modified_base 2: mod_base = OTHER; note = 5'-methyluridine-3'-phosphate
  modified_base 3: mod_base = OTHER; note = 5'-methyluridine-3'-phosphate
  modified_base 11: mod_base = OTHER; note = 5'-methyluridine-3'-phosphate
  modified_base 14: mod_base = OTHER; note = 5'-methyluridine-3'-phosphate
  modified_base 16: mod_base = OTHER; note = 5'-methyluridine-3'-phosphate
  modified_base 22: mod_base = OTHER; note = 5'-methyluridine-3'-phosphate
cttcaggcaataatctcaacatc

SEQ ID NO: 585 - RNA, 23 nt, synthetic construct
  source 1..23: mol_type = other RNA
  modified_base 2: mod_base = OTHER; note = 5'-methyluridine-3'-phosphate
  modified_base 4: mod_base = OTHER; note = 5'-methyluridine-3'-phosphate
  modified_base 5: mod_base = OTHER; note = 5'-methyluridine-3'-phosphate
  modified_base 9: mod_base = OTHER; note = 5'-methyluridine-3'-phosphate
  modified_base 13: mod_base = OTHER; note = 5'-methyluridine-3'-phosphate
  modified_base 14: mod_base = OTHER; note = 5'-methyluridine-3'-phosphate
  modified_base 17: mod_base = OTHER; note = 5'-methyluridine-3'-phosphate
  modified_base 21: mod_base = OTHER; note = 5'-methyluridine-3'-phosphate
atcttcagtaccttgatccataa

SEQ ID NO: 586 - RNA, 23 nt, synthetic construct
  source 1..23: mol_type = other RNA
  modified_base 5: mod_base = OTHER; note = 5'-methyluridine-3'-phosphate
  modified_base 7: mod_base = OTHER; note = 5'-methyluridine-3'-phosphate
  modified_base 8: mod_base = OTHER; note = 5'-methyluridine-3'-phosphate
  modified_base 10: mod_base = OTHER; note = 5'-methyluridine-3'-phosphate
  modified_base 12: mod_base = OTHER; note = 5'-methyluridine-3'-phosphate
  modified_base 14: mod_base = OTHER; note = 5'-methyluridine-3'-phosphate
  modified_base 20: mod_base = OTHER; note = 5'-methyluridine-3'-phosphate
  modified_base 21: mod_base = OTHER; note = 5'-methyluridine-3'-phosphate
  modified_base 22: mod_base = OTHER; note = 5'-methyluridine-3'-phosphate
aagatgttctctatagagctttg

SEQ ID NO: 587 - RNA, 23 nt, synthetic construct
  source 1..23: mol_type = other RNA
  modified_base 1: mod_base = OTHER; note = 5'-methyluridine-3'-phosphate
  modified_base 7: mod_base = OTHER; note = 5'-methyluridine-3'-phosphate
  modified_base 9: mod_base = OTHER; note = 5'-methyluridine-3'-phosphate
  modified_base 12: mod_base = OTHER; note = 5'-methyluridine-3'-phosphate
  modified_base 13: mod_base = OTHER; note = 5'-methyluridine-3'-phosphate
  modified_base 17: mod_base = OTHER; note = 5'-methyluridine-3'-phosphate
  modified_base 18: mod_base = OTHER; note = 5'-methyluridine-3'-phosphate
  modified_base 21: mod_base = OTHER; note = 5'-methyluridine-3'-phosphate
  modified_base 22: mod_base = OTHER; note = 5'-methyluridine-3'-phosphate
tgggcatatagttgaattacttc

SEQ ID NO: 588 - RNA, 23 nt, synthetic construct
  source 1..23: mol_type = other RNA
  modified_base 3: mod_base = OTHER; note = 5'-methyluridine-3'-phosphate
  modified_base 7: mod_base = OTHER; note = 5'-methyluridine-3'-phosphate
  modified_base 10: mod_base = OTHER; note = 5'-methyluridine-3'-phosphate
  modified_base 12: mod_base = OTHER; note = 5'-methyluridine-3'-phosphate
  modified_base 14: mod_base = OTHER; note = 5'-methyluridine-3'-phosphate
  modified_base 16: mod_base = OTHER; note = 5'-methyluridine-3'-phosphate
  modified_base 22: mod_base = OTHER; note = 5'-methyluridine-3'-phosphate
ggtagatactctgtctaccaatg

SEQ ID NO: 589 - RNA, 23 nt, synthetic construct
  source 1..23: mol_type = other RNA
  modified_base 2: mod_base = OTHER; note = 5'-methyluridine-3'-phosphate
  modified_base 11: mod_base = OTHER; note = 5'-methyluridine-3'-phosphate
  modified_base 13: mod_base = OTHER; note = 5'-methyluridine-3'-phosphate
  modified_base 14: mod_base = OTHER; note = 5'-methyluridine-3'-phosphate
  modified_base 17: mod_base = OTHER; note = 5'-methyluridine-3'-phosphate
  modified_base 20: mod_base = OTHER; note = 5'-methyluridine-3'-phosphate
atcccagacatcttgataatacc

SEQ ID NO: 590 - RNA, 23 nt, synthetic construct
  source 1..23: mol_type = other RNA
  modified_base 4: mod_base = OTHER; note = 5'-methyluridine-3'-phosphate
  modified_base 6: mod_base = OTHER; note = 5'-methyluridine-3'-phosphate
  modified_base 7: mod_base = OTHER; note = 5'-methyluridine-3'-phosphate
  modified_base 12: mod_base = OTHER; note = 5'-methyluridine-3'-phosphate
  modified_base 14: mod_base = OTHER; note = 5'-methyluridine-3'-phosphate
  modified_base 17: mod_base = OTHER; note = 5'-methyluridine-3'-phosphate
  modified_base 19: mod_base = OTHER; note = 5'-methyluridine-3'-phosphate
  modified_base 22: mod_base = OTHER; note = 5'-methyluridine-3'-phosphate
acctgttggaatctcctatgatc

SEQ ID NO: 591 - RNA, 23 nt, synthetic construct
  source 1..23: mol_type = other RNA
  modified_base 4: mod_base = OTHER; note = 5'-methyluridine-3'-phosphate
  modified_base 14: mod_base = OTHER; note = 5'-methyluridine-3'-phosphate
  modified_base 23: mod_base = OTHER; note = 5'-methyluridine
aactgggcaaacctaagaagaat

SEQ ID NO: 592 - RNA, 23 nt, synthetic construct
  source 1..23: mol_type = other RNA
  modified_base 2: mod_base = OTHER; note = 5'-methyluridine-3'-phosphate
  modified_base 4: mod_base = OTHER; note = 5'-methyluridine-3'-phosphate
  modified_base 5: mod_base = OTHER; note = 5'-methyluridine-3'-phosphate
  modified_base 7: mod_base = OTHER; note = 5'-methyluridine-3'-phosphate
  modified_base 8: mod_base = OTHER; note = 5'-methyluridine-3'-phosphate
  modified_base 13: mod_base = OTHER; note = 5'-methyluridine-3'-phosphate
  modified_base 15: mod_base = OTHER; note = 5'-methyluridine-3'-phosphate
  modified_base 16: mod_base = OTHER; note = 5'-methyluridine-3'-phosphate
gtgttattagaatgttacgaaaa

SEQ ID NO: 593 - RNA, 23 nt, synthetic construct
  source 1..23: mol_type = other RNA
  modified_base 8: mod_base = OTHER; note = 5'-methyluridine-3'-phosphate
  modified_base 9: mod_base = OTHER; note = 5'-methyluridine-3'-phosphate
  modified_base 10: mod_base = OTHER; note = 5'-methyluridine-3'-phosphate
  modified_base 11: mod_base = OTHER; note = 5'-methyluridine-3'-phosphate
  modified_base 14: mod_base = OTHER; note = 5'-methyluridine-3'-phosphate
  modified_base 15: mod_base = OTHER; note = 5'-methyluridine-3'-phosphate
  modified_base 23: mod_base = OTHER; note = 5'-methyluridine
acagccattttccttaaaggaat

SEQ ID NO: 594 - RNA, 23 nt, synthetic construct
  source 1..23: mol_type = other RNA
  modified_base 5: mod_base = OTHER; note = 5'-methyluridine-3'-phosphate
  modified_base 7: mod_base = OTHER; note = 5'-methyluridine-3'-phosphate
  modified_base 8: mod_base = OTHER; note = 5'-methyluridine-3'-phosphate
  modified_base 9: mod_base = OTHER; note = 5'-methyluridine-3'-phosphate
  modified_base 22: mod_base = OTHER; note = 5'-methyluridine-3'-phosphate
ggaatatttagaaagccaaagtc

SEQ ID NO: 595 - RNA, 23 nt, synthetic construct
  source 1..23: mol_type = other RNA
  modified_base 1: mod_base = OTHER; note = 5'-methyluridine-3'-phosphate
  modified_base 2: mod_base = OTHER; note = 5'-methyluridine-3'-phosphate
  modified_base 9: mod_base = OTHER; note = 5'-methyluridine-3'-phosphate
  modified_base 11: mod_base = OTHER; note = 5'-methyluridine-3'-phosphate
  modified_base 14: mod_base = OTHER; note = 5'-methyluridine-3'-phosphate
  modified_base 15: mod_base = OTHER; note = 5'-methyluridine-3'-phosphate
  modified_base 18: mod_base = OTHER; note = 5'-methyluridine-3'-phosphate
  modified_base 19: mod_base = OTHER; note = 5'-methyluridine-3'-phosphate
ttaccagctatacttccttcaag

SEQ ID NO: 596 - RNA, 23 nt, synthetic construct
  source 1..23: mol_type = other RNA
  modified_base 2: mod_base = OTHER; note = 5'-methyluridine-3'-phosphate
  modified_base 3: mod_base = OTHER; note = 5'-methyluridine-3'-phosphate
  modified_base 6: mod_base = OTHER; note = 5'-methyluridine-3'-phosphate
  modified_base 10: mod_base = OTHER; note = 5'-methyluridine-3'-phosphate
  modified_base 18: mod_base = OTHER; note = 5'-methyluridine-3'-phosphate
attaatgagtccagaaatgcaac

SEQ ID NO: 597 - RNA, 23 nt, synthetic construct
  source 1..23: mol_type = other RNA
  modified_base 9: mod_base = OTHER; note = 5'-methyluridine-3'-phosphate
  modified_base 10: mod_base = OTHER; note = 5'-methyluridine-3'-phosphate
  modified_base 13: mod_base = OTHER; note = 5'-methyluridine-3'-phosphate
  modified_base 14: mod_base = OTHER; note = 5'-methyluridine-3'-phosphate
  modified_base 20: mod_base = OTHER; note = 5'-methyluridine-3'-phosphate
  modified_base 22: mod_base = OTHER; note = 5'-methyluridine-3'-phosphate
gaaggaggttgattgcaaatctg

SEQ ID NO: 598 - RNA, 23 nt, synthetic construct
  source 1..23: mol_type = other RNA
  modified_base 1: mod_base = OTHER; note = 5'-methyluridine-3'-phosphate
  modified_base 9: mod_base = OTHER; note = 5'-methyluridine-3'-phosphate
  modified_base 10: mod_base = OTHER; note = 5'-methyluridine-3'-phosphate
  modified_base 12: mod_base = OTHER; note = 5'-methyluridine-3'-phosphate
  modified_base 13: mod_base = OTHER; note = 5'-methyluridine-3'-phosphate
  modified_base 14: mod_base = OTHER; note = 5'-methyluridine-3'-phosphate
  modified_base 16: mod_base = OTHER; note = 5'-methyluridine-3'-phosphate
  modified_base 19: mod_base = OTHER; note = 5'-methyluridine-3'-phosphate
tcgaagacttctttgtgatgaaa

SEQ ID NO: 599 - RNA, 23 nt, synthetic construct
  source 1..23: mol_type = other RNA
  modified_base 5: mod_base = OTHER; note = 5'-methyluridine-3'-phosphate
  modified_base 6: mod_base = OTHER; note = 5'-methyluridine-3'-phosphate
  modified_base 14: mod_base = OTHER; note = 5'-methyluridine-3'-phosphate
  modified_base 16: mod_base = OTHER; note = 5'-methyluridine-3'-phosphate
  modified_base 19: mod_base = OTHER; note = 5'-methyluridine-3'-phosphate
  modified_base 22: mod_base = OTHER; note = 5'-methyluridine-3'-phosphate
gaaattcagaagatgtagtaatg

SEQ ID NO: 600 - RNA, 23 nt, synthetic construct
  source 1..23: mol_type = other RNA
  modified_base 1: mod_base = OTHER; note = 5'-methyluridine-3'-phosphate
  modified_base 5: mod_base = OTHER; note = 5'-methyluridine-3'-phosphate
  modified_base 7: mod_base = OTHER; note = 5'-methyluridine-3'-phosphate
  modified_base 8: mod_base = OTHER; note = 5'-methyluridine-3'-phosphate
  modified_base 14: mod_base = OTHER; note = 5'-methyluridine-3'-phosphate
  modified_base 19: mod_base = OTHER; note = 5'-methyluridine-3'-phosphate
  modified_base 20: mod_base = OTHER; note = 5'-methyluridine-3'-phosphate
  modified_base 22: mod_base = OTHER; note = 5'-methyluridine-3'-phosphate
tcagtcttcgaactcaacttcta

SEQ ID NO: 601 - RNA, 23 nt, synthetic construct
  source 1..23: mol_type = other RNA
  modified_base 3: mod_base = OTHER; note = 5'-methyluridine-3'-phosphate
  modified_base 6: mod_base = OTHER; note = 5'-methyluridine-3'-phosphate
  modified_base 7: mod_base = OTHER; note = 5'-methyluridine-3'-phosphate
  modified_base 10: mod_base = OTHER; note = 5'-methyluridine-3'-phosphate
  modified_base 12: mod_base = OTHER; note = 5'-methyluridine-3'-phosphate
  modified_base 14: mod_base = OTHER; note = 5'-methyluridine-3'-phosphate
  modified_base 15: mod_base = OTHER; note = 5'-methyluridine-3'-phosphate
  modified_base 16: mod_base = OTHER; note = 5'-methyluridine-3'-phosphate
  modified_base 18: mod_base = OTHER; note = 5'-methyluridine-3'-phosphate
  modified_base 21: mod_base = OTHER; note = 5'-methyluridine-3'-phosphate
ggtacttcatgtctttatcatgg

SEQ ID NO: 602 - RNA, 23 nt, synthetic construct
  source 1..23: mol_type = other RNA
  modified_base 2: mod_base = OTHER; note = 5'-methyluridine-3'-phosphate
  modified_base 3: mod_base = OTHER; note = 5'-methyluridine-3'-phosphate
  modified_base 4: mod_base = OTHER; note = 5'-methyluridine-3'-phosphate
  modified_base 6: mod_base = OTHER; note = 5'-methyluridine-3'-phosphate
  modified_base 11: mod_base = OTHER; note = 5'-methyluridine-3'-phosphate
  modified_base 12: mod_base = OTHER; note = 5'-methyluridine-3'-phosphate
  modified_base 14: mod_base = OTHER; note = 5'-methyluridine-3'-phosphate
ctttatgcagttctgaacaagag

SEQ ID NO: 603 - RNA, 23 nt, synthetic construct
  source 1..23: mol_type = other RNA
  modified_base 2: mod_base = OTHER; note = 5'-methyluridine-3'-phosphate
  modified_base 10: mod_base = OTHER; note = 5'-methyluridine-3'-phosphate
  modified_base 18: mod_base = OTHER; note = 5'-methyluridine-3'-phosphate
  modified_base 19: mod_base = OTHER; note = 5'-methyluridine-3'-phosphate
  modified_base 20: mod_base = OTHER; note = 5'-methyluridine-3'-phosphate
  modified_base 22: mod_base = OTHER; note = 5'-methyluridine-3'-phosphate
atgaaacagtaggaaagtttatc

SEQ ID NO: 604 - RNA, 23 nt, synthetic construct
  source 1..23: mol_type = other RNA
  modified_base 2: mod_base = OTHER; note = 5'-methyluridine-3'-phosphate
  modified_base 3: mod_base = OTHER; note = 5'-methyluridine-3'-phosphate
  modified_base 11: mod_base = OTHER; note = 5'-methyluridine-3'-phosphate
  modified_base 14: mod_base = OTHER; note = 5'-methyluridine-3'-phosphate
  modified_base 23: mod_base = OTHER; note = 5'-methyluridine
cttggagaagtgatgaagaagat

SEQ ID NO: 605 - RNA, 23 nt, synthetic construct
  source 1..23: mol_type = other RNA
  modified_base 4: mod_base = OTHER; note = 5'-methyluridine-3'-phosphate
  modified_base 5: mod_base = OTHER; note = 5'-methyluridine-3'-phosphate
  modified_base 6: mod_base = OTHER; note = 5'-methyluridine-3'-phosphate
  modified_base 8: mod_base = OTHER; note = 5'-methyluridine-3'-phosphate
  modified_base 13: mod_base = OTHER; note = 5'-methyluridine-3'-phosphate
  modified_base 14: mod_base = OTHER; note = 5'-methyluridine-3'-phosphate
  modified_base 16: mod_base = OTHER; note = 5'-methyluridine-3'-phosphate
  modified_base 17: mod_base = OTHER; note = 5'-methyluridine-3'-phosphate
cagtttatcaccttcttacagag

SEQ ID NO: 606 - RNA, 23 nt, synthetic construct
  source 1..23: mol_type = other RNA
  modified_base 8: mod_base = OTHER; note = 5'-methyluridine-3'-phosphate
  modified_base 12: mod_base = OTHER; note = 5'-methyluridine-3'-phosphate
  modified_base 14: mod_base = OTHER; note = 5'-methyluridine-3'-phosphate
  modified_base 16: mod_base = OTHER; note = 5'-methyluridine-3'-phosphate
cagaacctgagtatctgcaaaag

SEQ ID NO: 607 - RNA, 23 nt, synthetic construct
  source 1..23: mol_type = other RNA
  modified_base 4: mod_base = OTHER; note = 5'-methyluridine-3'-phosphate
  modified_base 5: mod_base = OTHER; note = 5'-methyluridine-3'-phosphate
  modified_base 13: mod_base = OTHER; note = 5'-methyluridine-3'-phosphate
  modified_base 17: mod_base = OTHER; note = 5'-methyluridine-3'-phosphate
  modified_base 20: mod_base = OTHER; note = 5'-methyluridine-3'-phosphate
aagttgcacaaatacctaataac

SEQ ID NO: 608 - RNA, 23 nt, synthetic construct
  source 1..23: mol_type = other RNA
  modified_base 3: mod_base = OTHER; note = 5'-methyluridine-3'-phosphate
  modified_base 22: mod_base = OTHER; note = 5'-methyluridine-3'-phosphate
aataaccagaacagaaagaaatg

SEQ ID NO: 609 - RNA, 23 nt, synthetic construct
  source 1..23: mol_type = other RNA
  modified_base 5: mod_base = OTHER; note = 5'-methyluridine-3'-phosphate
  modified_base 7: mod_base = OTHER; note = 5'-methyluridine-3'-phosphate
  modified_base 8: mod_base = OTHER; note = 5'-methyluridine-3'-phosphate
  modified_base 10: mod_base = OTHER; note = 5'-methyluridine-3'-phosphate
  modified_base 12: mod_base = OTHER; note = 5'-methyluridine-3'-phosphate
  modified_base 13: mod_base = OTHER; note = 5'-methyluridine-3'-phosphate
  modified_base 15: mod_base = OTHER; note = 5'-methyluridine-3'-phosphate
  modified_base 22: mod_base = OTHER; note = 5'-methyluridine-3'-phosphate
cacatattgtcttgtgaagaatg

SEQ ID NO: 610 - RNA, 23 nt, synthetic construct
  source 1..23: mol_type = other RNA
  modified_base 5: mod_base = OTHER; note = 5'-methyluridine-3'-phosphate
  modified_base 8: mod_base = OTHER; note = 5'-methyluridine-3'-phosphate
  modified_base 10: mod_base = OTHER; note = 5'-methyluridine-3'-phosphate
  modified_base 16: mod_base = OTHER; note = 5'-methyluridine-3'-phosphate
  modified_base 18: mod_base = OTHER; note = 5'-methyluridine-3'-phosphate
  modified_base 19: mod_base = OTHER; note = 5'-methyluridine-3'-phosphate
  modified_base 20: mod_base = OTHER; note = 5'-methyluridine-3'-phosphate
agaatgctgtgaaaatgtttaag

SEQ ID NO: 611 - RNA, 23 nt, synthetic construct
  source 1..23: mol_type = other RNA
  modified_base 7: mod_base = OTHER; note = 5'-methyluridine-3'-phosphate
  modified_base 9: mod_base = OTHER; note = 5'-methyluridine-3'-phosphate
  modified_base 11: mod_base = OTHER; note = 5'-methyluridine-3'-phosphate
  modified_base 13: mod_base = OTHER; note = 5'-methyluridine-3'-phosphate
  modified_base 14: mod_base = OTHER; note = 5'-methyluridine-3'-phosphate
  modified_base 15: mod_base = OTHER; note = 5'-methyluridine-3'-phosphate
  modified_base 16: mod_base = OTHER; note = 5'-methyluridine-3'-phosphate
  modified_base 22: mod_base = OTHER; note = 5'-methyluridine-3'-phosphate
agagagtgtctgttttagaactg

SEQ ID NO: 612 - RNA, 23 nt, synthetic construct
  source 1..23: mol_type = other RNA
  modified_base 3: mod_base = OTHER; note = 5'-methyluridine-3'-phosphate
  modified_base 5: mod_base = OTHER; note = 5'-methyluridine-3'-phosphate
  modified_base 7: mod_base = OTHER; note = 5'-methyluridine-3'-phosphate
  modified_base 8: mod_base = OTHER; note = 5'-methyluridine-3'-phosphate
  modified_base 10: mod_base = OTHER; note = 5'-methyluridine-3'-phosphate
  modified_base 14: mod_base = OTHER; note = 5'-methyluridine-3'-phosphate
  modified_base 15: mod_base = OTHER; note = 5'-methyluridine-3'-phosphate
  modified_base 16: mod_base = OTHER; note = 5'-methyluridine-3'-phosphate
  modified_base 17: mod_base = OTHER; note = 5'-methyluridine-3'-phosphate
  modified_base 19: mod_base = OTHER; note = 5'-methyluridine-3'-phosphate
  modified_base 22: mod_base = OTHER; note = 5'-methyluridine-3'-phosphate
aatatattctgagttttgtggtg

SEQ ID NO: 613 - RNA, 23 nt, synthetic construct
  source 1..23: mol_type = other RNA
  modified_base 1: mod_base = OTHER; note = 5'-methyluridine-3'-phosphate
  modified_base 4: mod_base = OTHER; note = 5'-methyluridine-3'-phosphate
  modified_base 9: mod_base = OTHER; note = 5'-methyluridine-3'-phosphate
  modified_base 13: mod_base = OTHER; note = 5'-methyluridine-3'-phosphate
  modified_base 14: mod_base = OTHER; note = 5'-methyluridine-3'-phosphate
  modified_base 17: mod_base = OTHER; note = 5'-methyluridine-3'-phosphate
  modified_base 18: mod_base = OTHER; note = 5'-methyluridine-3'-phosphate
  modified_base 20: mod_base = OTHER; note = 5'-methyluridine-3'-phosphate
tcatgagatgagttccttgtagg

SEQ ID NO: 614 - RNA, 23 nt, synthetic construct
  source 1..23: mol_type = other RNA
  modified_base 2: mod_base = OTHER; note = 5'-methyluridine-3'-phosphate
  modified_base 9: mod_base = OTHER; note = 5'-methyluridine-3'-phosphate
  modified_base 14: mod_base = OTHER; note = 5'-methyluridine-3'-phosphate
  modified_base 16: mod_base = OTHER; note = 5'-methyluridine-3'-phosphate
  modified_base 20: mod_base = OTHER; note = 5'-methyluridine-3'-phosphate
ctacaagatgaaatctcaataaa

SEQ ID NO: 615 - RNA, 23 nt, synthetic construct
  source 1..23: mol_type = other RNA
  modified_base 2: mod_base = OTHER; note = 5'-methyluridine-3'-phosphate
  modified_base 8: mod_base = OTHER; note = 5'-methyluridine-3'-phosphate
  modified_base 9: mod_base = OTHER; note = 5'-methyluridine-3'-phosphate
  modified_base 10: mod_base = OTHER; note = 5'-methyluridine-3'-phosphate
  modified_base 11: mod_base = OTHER; note = 5'-methyluridine-3'-phosphate
  modified_base 18: mod_base = OTHER; note = 5'-methyluridine-3'-phosphate
  modified_base 21: mod_base = OTHER; note = 5'-methyluridine-3'-phosphate
  modified_base 22: mod_base = OTHER; note = 5'-methyluridine-3'-phosphate
gtacaacttttaaggactaatta

SEQ ID NO: 616 - RNA, 23 nt, synthetic construct
  source 1..23: mol_type = other RNA
  modified_base 1: mod_base = OTHER; note = 5'-methyluridine-3'-phosphate
  modified_base 5: mod_base = OTHER; note = 5'-methyluridine-3'-phosphate
  modified_base 7: mod_base = OTHER; note = 5'-methyluridine-3'-phosphate
  modified_base 8: mod_base = OTHER; note = 5'-methyluridine-3'-phosphate
  modified_base 12: mod_base = OTHER; note = 5'-methyluridine-3'-phosphate
  modified_base 15: mod_base = OTHER; note = 5'-methyluridine-3'-phosphate
  modified_base 17: mod_base = OTHER; note = 5'-methyluridine-3'-phosphate
  modified_base 20: mod_base = OTHER; note = 5'-methyluridine-3'-phosphate
  modified_base 21: mod_base = OTHER; note = 5'-methyluridine-3'-phosphate
tgaatcttacatggtatacttag

SEQ ID NO: 617 - RNA, 23 nt, synthetic construct
  source 1..23: mol_type = other RNA
  modified_base 1: mod_base = OTHER; note = 5'-methyluridine-3'-phosphate
  modified_base 2: mod_base = OTHER; note = 5'-methyluridine-3'-phosphate
  modified_base 3: mod_base = OTHER; note = 5'-methyluridine-3'-phosphate
  modified_base 5: mod_base = OTHER; note = 5'-methyluridine-3'-phosphate
  modified_base 6: mod_base = OTHER; note = 5'-methyluridine-3'-phosphate
  modified_base 9: mod_base = OTHER; note = 5'-methyluridine-3'-phosphate
  modified_base 11: mod_base = OTHER; note = 5'-methyluridine-3'-phosphate
  modified_base 13: mod_base = OTHER; note = 5'-methyluridine-3'-phosphate
  modified_base 14: mod_base = OTHER; note = 5'-methyluridine-3'-phosphate
  modified_base 16: mod_base = OTHER; note = 5'-methyluridine-3'-phosphate
  modified_base 18: mod_base = OTHER; note = 5'-methyluridine-3'-phosphate
  modified_base 21: mod_base = OTHER; note = 5'-methyluridine-3'-phosphate
  modified_base 22: mod_base = OTHER; note = 5'-methyluridine-3'-phosphate
tttgttggtatattatctggtta

SEQ ID NO: 618 - RNA, 23 nt, synthetic construct
  source 1..23: mol_type = other RNA
  modified_base 3: mod_base = OTHER; note = 5'-methyluridine-3'-phosphate
  modified_base 4: mod_base = OTHER; note = 5'-methyluridine-3'-phosphate
  modified_base 7: mod_base = OTHER; note = 5'-methyluridine-3'-phosphate
  modified_base 10: mod_base = OTHER; note = 5'-methyluridine-3'-phosphate
  modified_base 11: mod_base = OTHER; note = 5'-methyluridine-3'-phosphate
  modified_base 14: mod_base = OTHER; note = 5'-methyluridine-3'-phosphate
  modified_base 17: mod_base = OTHER; note = 5'-methyluridine-3'-phosphate
  modified_base 18: mod_base = OTHER; note = 5'-methyluridine-3'-phosphate
  modified_base 21: mod_base = OTHER; note = 5'-methyluridine-3'-phosphate
  modified_base 22: mod_base = OTHER; note = 5'-methyluridine-3'-phosphate
  modified_base 23: mod_base = OTHER; note = 5'-methyluridine
ggttagtggttaatgcttccttt

SEQ ID NO: 619 - RNA, 23 nt, synthetic construct
  source 1..23: mol_type = other RNA
  modified_base 2: mod_base = OTHER; note = 5'-methyluridine-3'-phosphate
  modified_base 3: mod_base = OTHER; note = 5'-methyluridine-3'-phosphate
  modified_base 7: mod_base = OTHER; note = 5'-methyluridine-3'-phosphate
  modified_base 10: mod_base = OTHER; note = 5'-methyluridine-3'-phosphate
  modified_base 14: mod_base = OTHER; note = 5'-methyluridine-3'-phosphate
  modified_base 15: mod_base = OTHER; note = 5'-methyluridine-3'-phosphate
  modified_base 19: mod_base = OTHER; note = 5'-methyluridine-3'-phosphate
  modified_base 21: mod_base = OTHER; note = 5'-methyluridine-3'-phosphate
  modified_base 22: mod_base = OTHER; note = 5'-methyluridine-3'-phosphate
  modified_base 23: mod_base = OTHER; note = 5'-methyluridine
attgagtcatccattcactcttt

SEQ ID NO: 620 - RNA, 23 nt, synthetic construct
  source 1..23: mol_type = other RNA
  modified_base 1: mod_base = OTHER; note = 5'-methyluridine-3'-phosphate
  modified_base 2: mod_base = OTHER; note = 5'-methyluridine-3'-phosphate
  modified_base 6: mod_base = OTHER; note = 5'-methyluridine-3'-phosphate
  modified_base 7: mod_base = OTHER; note = 5'-methyluridine-3'-phosphate
  modified_base 8: mod_base = OTHER; note = 5'-methyluridine-3'-phosphate
  modified_base 9: mod_base = OTHER; note = 5'-methyluridine-3'-phosphate
  modified_base 11: mod_base = OTHER; note = 5'-methyluridine-3'-phosphate
  modified_base 13: mod_base = OTHER; note = 5'-methyluridine-3'-phosphate
  modified_base 15: mod_base = OTHER; note = 5'-methyluridine-3'-phosphate
  modified_base 19: mod_base = OTHER; note = 5'-methyluridine-3'-phosphate
  modified_base 22: mod_base = OTHER; note = 5'-methyluridine-3'-phosphate
ttcagttttatctgtcaatagta

SEQ ID NO: 621 - RNA, 23 nt, synthetic construct
  source 1..23: mol_type = other RNA
  modified_base 2: mod_base = OTHER; note = 5'-methyluridine-3'-phosphate
  modified_base 10: mod_base = OTHER; note = 5'-methyluridine-3'-phosphate
  modified_base 13: mod_base = OTHER; note = 5'-methyluridine-3'-phosphate
  modified_base 14: mod_base = OTHER; note = 5'-methyluridine-3'-phosphate
  modified_base 15: mod_base = OTHER; note = 5'-methyluridine-3'-phosphate
  modified_base 17: mod_base = OTHER; note = 5'-methyluridine-3'-phosphate
  modified_base 21: mod_base = OTHER; note = 5'-methyluridine-3'-phosphate
  modified_base 22: mod_base = OTHER; note = 5'-methyluridine-3'-phosphate
atcccaaagtgctttataaattg

SEQ ID NO: 622 - RNA, 23 nt, synthetic construct
  source 1..23: mol_type = other RNA
  modified_base 3: mod_base = OTHER; note = 5'-methyluridine-3'-phosphate
  modified_base 5: mod_base = OTHER; note = 5'-methyluridine-3'-phosphate
  modified_base 10: mod_base = OTHER; note = 5'-methyluridine-3'-phosphate
  modified_base 11: mod_base = OTHER; note = 5'-methyluridine-3'-phosphate
  modified_base 12: mod_base = OTHER; note = 5'-methyluridine-3'-phosphate
  modified_base 18: mod_base = OTHER; note = 5'-methyluridine-3'-phosphate
  modified_base 20: mod_base = OTHER; note = 5'-methyluridine-3'-phosphate
  modified_base 21: mod_base = OTHER; note = 5'-methyluridine-3'-phosphate
  modified_base 22: mod_base = OTHER; note = 5'-methyluridine-3'-phosphate
  modified_base 23: mod_base = OTHER; note = 5'-methyluridine
gctgtcagatttagaaatgtttt

SEQ ID NO: 623 - RNA, 23 nt, synthetic construct
  source 1..23: mol_type = other RNA
  modified_base 2: mod_base = OTHER; note = 5'-methyluridine-3'-phosphate
  modified_base 4: mod_base = OTHER; note = 5'-methyluridine-3'-phosphate
  modified_base 6: mod_base = OTHER; note = 5'-methyluridine-3'-phosphate
  modified_base 19: mod_base = OTHER; note = 5'-methyluridine-3'-phosphate
  modified_base 21: mod_base = OTHER; note = 5'-methyluridine-3'-phosphate
  modified_base 22: mod_base = OTHER; note = 5'-methyluridine-3'-phosphate
ctatgtgaaaacagacaatatta

SEQ ID NO: 624 - RNA, 23 nt, synthetic construct
  source 1..23: mol_type = other RNA
  modified_base 6: mod_base = OTHER; note = 5'-methyluridine-3'-phosphate
  modified_base 11: mod_base = OTHER; note = 5'-methyluridine-3'-phosphate
  modified_base 13: mod_base = OTHER; note = 5'-methyluridine-3'-phosphate
  modified_base 14: mod_base = OTHER; note = 5'-methyluridine-3'-phosphate
  modified_base 16: mod_base = OTHER; note = 5'-methyluridine-3'-phosphate
  modified_base 19: mod_base = OTHER; note = 5'-methyluridine-3'-phosphate
ggaactgagatattgtaatcaaa

SEQ ID NO: 625 - RNA, 23 nt, synthetic construct
  source 1..23: mol_type = other RNA
  modified_base 2: mod_base = OTHER; note = 5'-methyluridine-3'-phosphate
  modified_base 3: mod_base = OTHER; note = 5'-methyluridine-3'-phosphate
  modified_base 8: mod_base = OTHER; note = 5'-methyluridine-3'-phosphate
  modified_base 16: mod_base = OTHER; note = 5'-methyluridine-3'-phosphate
  modified_base 17: mod_base = OTHER; note = 5'-methyluridine-3'-phosphate
  modified_base 20: mod_base = OTHER; note = 5'-methyluridine-3'-phosphate
  modified_base 21: mod_base = OTHER; note = 5'-methyluridine-3'-phosphate
  modified_base 22: mod_base = OTHER; note = 5'-methyluridine-3'-phosphate
gttaacatcaggaagttaatttg

SEQ ID NO: 626 - RNA, 23 nt, synthetic construct
  source 1..23: mol_type = other RNA
  modified_base 1: mod_base = OTHER; note = 5'-methyluridine-3'-phosphate
  modified_base 9: mod_base = OTHER; note = 5'-methyluridine-3'-phosphate
  modified_base 10: mod_base = OTHER; note = 5'-methyluridine-3'-phosphate
  modified_base 12: mod_base = OTHER; note = 5'-methyluridine-3'-phosphate
  modified_base 21: mod_base = OTHER; note = 5'-methyluridine-3'-phosphate
  modified_base 22: mod_base = OTHER; note = 5'-methyluridine-3'-phosphate
tggcaaaattctagggaaacttg

SEQ ID NO: 627 - RNA, 23 nt, synthetic construct
  source 1..23: mol_type = other RNA
  modified_base 1: mod_base = OTHER; note = 5'-methyluridine-3'-phosphate
  modified_base 8: mod_base = OTHER; note = 5'-methyluridine-3'-phosphate
  modified_base 9: mod_base = OTHER; note = 5'-methyluridine-3'-phosphate
  modified_base 10: mod_base = OTHER; note = 5'-methyluridine-3'-phosphate
  modified_base 11: mod_base = OTHER; note = 5'-methyluridine-3'-phosphate
  modified_base 14: mod_base = OTHER; note = 5'-methyluridine-3'-phosphate
  modified_base 17: mod_base = OTHER; note = 5'-methyluridine-3'-phosphate
  modified_base 19: mod_base = OTHER; note = 5'-methyluridine-3'-phosphate
tgaaggcttttgctcatataaac

SEQ ID NO: 628 - RNA, 23 nt, synthetic construct
  source 1..23: mol_type = other RNA
  modified_base 3: mod_base = OTHER; note = 5'-methyluridine-3'-phosphate
  modified_base 8: mod_base = OTHER; note = 5'-methyluridine-3'-phosphate
  modified_base 9: mod_base = OTHER; note = 5'-methyluridine-3'-phosphate
  modified_base 13: mod_base = OTHER; note = 5'-methyluridine-3'-phosphate
  modified_base 14: mod_base = OTHER; note = 5'-methyluridine-3'-phosphate
  modified_base 15: mod_base = OTHER; note = 5'-methyluridine-3'-phosphate
  modified_base 20: mod_base = OTHER; note = 5'-methyluridine-3'-phosphate
agtgccattgagtttcaaatgac

SEQ ID NO: 629 - RNA, 23 nt, synthetic construct
  source 1..23: mol_type = other RNA
  modified_base 2: mod_base = OTHER; note = 5'-methyluridine-3'-phosphate
  modified_base 13: mod_base = OTHER; note = 5'-methyluridine-3'-phosphate
  modified_base 15: mod_base = OTHER; note = 5'-methyluridine-3'-phosphate
  modified_base 17: mod_base = OTHER; note = 5'-methyluridine-3'-phosphate
  modified_base 18: mod_base = OTHER; note = 5'-methyluridine-3'-phosphate
  modified_base 19: mod_base = OTHER; note = 5'-methyluridine-3'-phosphate
atgaccagcaaatatatttagaa

SEQ ID NO: 630 - RNA, 23 nt, synthetic construct
  source 1..23: mol_type = other RNA
  modified_base 1: mod_base = OTHER; note = 5'-methyluridine-3'-phosphate
  modified_base 2: mod_base = OTHER; note = 5'-methyluridine-3'-phosphate
  modified_base 4: mod_base = OTHER; note = 5'-methyluridine-3'-phosphate
  modified_base 5: mod_base = OTHER; note = 5'-methyluridine-3'-phosphate
  modified_base 11: mod_base = OTHER; note = 5'-methyluridine-3'-phosphate
  modified_base 14: mod_base = OTHER; note = 5'-methyluridine-3'-phosphate
ttcttggaaatcctccaaccaaa

SEQ ID NO: 631 - RNA, 23 nt, synthetic construct
  source 1..23: mol_type = other RNA
  modified_base 6: mod_base = OTHER; note = 5'-methyluridine-3'-phosphate
  modified_base 12: mod_base = OTHER; note = 5'-methyluridine-3'-phosphate
  modified_base 13: mod_base = OTHER; note = 5'-methyluridine-3'-phosphate
  modified_base 14: mod_base = OTHER; note = 5'-methyluridine-3'-phosphate
  modified_base 15: mod_base = OTHER; note = 5'-methyluridine-3'-phosphate
  modified_base 18: mod_base = OTHER; note = 5'-methyluridine-3'-phosphate
  modified_base 22: mod_base = OTHER; note = 5'-methyluridine-3'-phosphate
  modified_base 23: mod_base = OTHER; note = 5'-methyluridine
ccaaatagcagttttcctaactt

SEQ ID NO: 632 - RNA, 23 nt, synthetic construct
  source 1..23: mol_type = other RNA
  modified_base 1: mod_base = OTHER; note = 5'-methyluridine-3'-phosphate
  modified_base 6: mod_base = OTHER; note = 5'-methyluridine-3'-phosphate
  modified_base 14: mod_base = OTHER; note = 5'-methyluridine-3'-phosphate
  modified_base 16: mod_base = OTHER; note = 5'-methyluridine-3'-phosphate
  modified_base 17: mod_base = OTHER; note = 5'-methyluridine-3'-phosphate
  modified_base 22: mod_base = OTHER; note = 5'-methyluridine-3'-phosphate
tgagctgacagactgttagaata

SEQ ID NO: 633 - RNA, 23 nt, synthetic construct
  source 1..23: mol_type = other RNA
  modified_base 3: mod_base = OTHER; note = 5'-methyluridine-3'-phosphate
  modified_base 4: mod_base = OTHER; note = 5'-methyluridine-3'-phosphate
  modified_base 12: mod_base = OTHER; note = 5'-methyluridine-3'-phosphate
  modified_base 13: mod_base = OTHER; note = 5'-methyluridine-3'-phosphate
  modified_base 14: mod_base = OTHER; note = 5'-methyluridine-3'-phosphate
  modified_base 16: mod_base = OTHER; note = 5'-methyluridine-3'-phosphate
  modified_base 20: mod_base = OTHER; note = 5'-methyluridine-3'-phosphate
  modified_base 21: mod_base = OTHER; note = 5'-methyluridine-3'-phosphate
  modified_base 22: mod_base = OTHER; note = 5'-methyluridine-3'-phosphate
  modified_base 23: mod_base = OTHER; note = 5'-methyluridine
ggttagaggcatttatggatttt

SEQ ID NO: 634 - RNA, 23 nt, synthetic construct
  source 1..23: mol_type = other RNA
  modified_base 1: mod_base = OTHER; note = 5'-methyluridine-3'-phosphate
  modified_base 2: mod_base = OTHER; note = 5'-methyluridine-3'-phosphate
  modified_base 3: mod_base = OTHER; note = 5'-methyluridine-3'-phosphate
  modified_base 5: mod_base = OTHER; note = 5'-methyluridine-3'-phosphate
  modified_base 9: mod_base = OTHER; note = 5'-methyluridine-3'-phosphate
  modified_base 10: mod_base = OTHER; note = 5'-methyluridine-3'-phosphate
  modified_base 12: mod_base = OTHER; note = 5'-methyluridine-3'-phosphate
  modified_base 14: mod_base = OTHER; note = 5'-methyluridine-3'-phosphate
  modified_base 18: mod_base = OTHER; note = 5'-methyluridine-3'-phosphate
tttatgggttatatgcctaaacc

SEQ ID NO: 635 - RNA, 23 nt, synthetic construct
  source 1..23: mol_type = other RNA
  modified_base 1: mod_base = OTHER; note = 5'-methyluridine-3'-phosphate
  modified_base 8: mod_base = OTHER; note = 5'-methyluridine-3'-phosphate
  modified_base 11: mod_base = OTHER; note = 5'-methyluridine-3'-phosphate
  modified_base 14: mod_base = OTHER; note = 5'-methyluridine-3'-phosphate
  modified_base 18: mod_base = OTHER; note = 5'-methyluridine-3'-phosphate
  modified_base 21: mod_base = OTHER; note = 5'-methyluridine-3'-phosphate
  modified_base 22: mod_base = OTHER; note = 5'-methyluridine-3'-phosphate
tgccacatagtggtaaataatta

SEQ ID NO: 636 - RNA, 23 nt, synthetic construct
  source 1..23: mol_type = other RNA
  modified_base 3: mod_base = OTHER; note = 5'-methyluridine-3'-phosphate
  modified_base 6: mod_base = OTHER; note = 5'-methyluridine-3'-phosphate
  modified_base 8: mod_base = OTHER; note = 5'-methyluridine-3'-phosphate
  modified_base 10: mod_base = OTHER; note = 5'-methyluridine-3'-phosphate
  modified_base 11: mod_base = OTHER; note = 5'-methyluridine-3'-phosphate
  modified_base 14: mod_base = OTHER; note = 5'-methyluridine-3'-phosphate
  modified_base 17: mod_base = OTHER; note = 5'-methyluridine-3'-phosphate
  modified_base 18: mod_base = OTHER; note = 5'-methyluridine-3'-phosphate
  modified_base 21: mod_base = OTHER; note = 5'-methyluridine-3'-phosphate
aatggtctgttcataattggtag

SEQ ID NO: 637 - RNA, 23 nt, synthetic construct
  source 1..23: mol_type = other RNA
  modified_base 8: mod_base = OTHER; note = 5'-methyluridine-3'-phosphate
  modified_base 11: mod_base = OTHER; note = 5'-methyluridine-3'-phosphate
  modified_base 12: mod_base = OTHER; note = 5'-methyluridine-3'-phosphate
  modified_base 14: mod_base = OTHER; note = 5'-methyluridine-3'-phosphate
  modified_base 15: mod_base = OTHER; note = 5'-methyluridine-3'-phosphate
  modified_base 18: mod_base = OTHER; note = 5'-methyluridine-3'-phosphate
  modified_base 19: mod_base = OTHER; note = 5'-methyluridine-3'-phosphate
  modified_base 20: mod_base = OTHER; note = 5'-methyluridine-3'-phosphate
  modified_base 22: mod_base = OTHER; note = 5'-methyluridine-3'-phosphate
  modified_base 23: mod_base = OTHER; note = 5'-methyluridine
gggagcataattattggtttatt

SEQ ID NO: 638 - RNA, 23 nt, synthetic construct
  source 1..23: mol_type = other RNA
  modified_base 3: mod_base = OTHER; note = 5'-methyluridine-3'-phosphate
  modified_base 4: mod_base = OTHER; note = 5'-methyluridine-3'-phosphate
  modified_base 5: mod_base = OTHER; note = 5'-methyluridine-3'-phosphate
  modified_base 7: mod_base = OTHER; note = 5'-methyluridine-3'-phosphate
  modified_base 8: mod_base = OTHER; note = 5'-methyluridine-3'-phosphate
  modified_base 10: mod_base = OTHER; note = 5'-methyluridine-3'-phosphate
  modified_base 13: mod_base = OTHER; note = 5'-methyluridine-3'-phosphate
  modified_base 16: mod_base = OTHER; note = 5'-methyluridine-3'-phosphate
  modified_base 17: mod_base = OTHER; note = 5'-methyluridine-3'-phosphate
  modified_base 19: mod_base = OTHER; note = 5'-methyluridine-3'-phosphate
  modified_base 22: mod_base = OTHER; note = 5'-methyluridine-3'-phosphate
ggtttattatggtaattatggtg

SEQ ID NO: 639 - RNA, 23 nt, synthetic construct
  source 1..23: mol_type = other RNA
  modified_base 2: mod_base = OTHER; note = 5'-methyluridine-3'-phosphate
  modified_base 3: mod_base = OTHER; note = 5'-methyluridine-3'-phosphate
  modified_base 10: mod_base = OTHER; note = 5'-methyluridine-3'-phosphate
  modified_base 11: mod_base = OTHER; note = 5'-methyluridine-3'-phosphate
  modified_base 12: mod_base = OTHER; note = 5'-methyluridine-3'-phosphate
  modified_base 13: mod_base = OTHER; note = 5'-methyluridine-3'-phosphate
  modified_base 15: mod_base = OTHER; note = 5'-methyluridine-3'-phosphate
  modified_base 21: mod_base = OTHER; note = 5'-methyluridine-3'-phosphate
  modified_base 22: mod_base = OTHER; note = 5'-methyluridine-3'-phosphate
  modified_base 23: mod_base = OTHER; note = 5'-methyluridine
gttaaaacgttttctaacagttt

SEQ ID NO: 640 - RNA, 23 nt, synthetic construct
  source 1..23: mol_type = other RNA
  modified_base 2: mod_base = OTHER; note = 5'-methyluridine-3'-phosphate
  modified_base 4: mod_base = OTHER; note = 5'-methyluridine-3'-phosphate
  modified_base 11: mod_base = OTHER; note = 5'-methyluridine-3'-phosphate
  modified_base 13: mod_base = OTHER; note = 5'-methyluridine-3'-phosphate
  modified_base 14: mod_base = OTHER; note = 5'-methyluridine-3'-phosphate
  modified_base 16: mod_base = OTHER; note = 5'-methyluridine-3'-phosphate
  modified_base 21: mod_base = OTHER; note = 5'-methyluridine-3'-phosphate
  modified_base 22: mod_base = OTHER; note = 5'-methyluridine-3'-phosphate
atctccaagatattatggaatta

SEQ ID NO: 641 - RNA, 23 nt, synthetic construct
  source 1..23: mol_type = other RNA
  modified_base 3: mod_base = OTHER; note = 5'-methyluridine-3'-phosphate
  modified_base 7: mod_base = OTHER; note = 5'-methyluridine-3'-phosphate
  modified_base 9: mod_base = OTHER; note = 5'-methyluridine-3'-phosphate
  modified_base 10: mod_base = OTHER; note = 5'-methyluridine-3'-phosphate
  modified_base 14: mod_base = OTHER; note = 5'-methyluridine-3'-phosphate
  modified_base 18: mod_base = OTHER; note = 5'-methyluridine-3'-phosphate
  modified_base 19: mod_base = OTHER; note = 5'-methyluridine-3'-phosphate
  modified_base 21: mod_base = OTHER; note = 5'-methyluridine-3'-phosphate
  modified_base 22: mod_base = OTHER; note = 5'-methyluridine-3'-phosphate
  modified_base 23: mod_base = OTHER; note = 5'-methyluridine
gatgagtgttacatagattcttt

SEQ ID NO: 642 - RNA, 23 nt, synthetic construct
  source 1..23: mol_type = other RNA
  modified_base 5: mod_base = OTHER; note = 5'-methyluridine-3'-phosphate
  modified_base 8: mod_base = OTHER; note = 5'-methyluridine-3'-phosphate
  modified_base 14: mod_base = OTHER; note = 5'-methyluridine-3'-phosphate
  modified_base 15: mod_base = OTHER; note = 5'-methyluridine-3'-phosphate
  modified_base 19: mod_base = OTHER; note = 5'-methyluridine-3'-phosphate
  modified_base 20: mod_base = OTHER; note = 5'-methyluridine-3'-phosphate
  modified_base 21: mod_base = OTHER; note = 5'-methyluridine-3'-phosphate
  modified_base 23: mod_base = OTHER; note = 5'-methyluridine
aaagtactgagaattaagtttgt

SEQ ID NO: 643 - RNA, 23 nt, synthetic construct
  source 1..23: mol_type = other RNA
  modified_base 4: mod_base = OTHER; note = 5'-methyluridine-3'-phosphate
  modified_base 5: mod_base = OTHER; note = 5'-methyluridine-3'-phosphate
  modified_base 6: mod_base = OTHER; note = 5'-methyluridine-3'-phosphate
  modified_base 7: mod_base = OTHER; note = 5'-methyluridine-3'-phosphate
  modified_base 14: mod_base = OTHER; note = 5'-methyluridine-3'-phosphate
  modified_base 17: mod_base = OTHER; note = 5'-methyluridine-3'-phosphate
  modified_base 20: mod_base = OTHER; note = 5'-methyluridine-3'-phosphate
  modified_base 22: mod_base = OTHER; note = 5'-methyluridine-3'-phosphate
ggattttaaacactgatagtatc

SEQ ID NO: 644 - RNA, 23 nt, synthetic construct
  source 1..23: mol_type = other RNA
  modified_base 2: mod_base = OTHER; note = 5'-methyluridine-3'-phosphate
  modified_base 4: mod_base = OTHER; note = 5'-methyluridine-3'-phosphate
  modified_base 7: mod_base = OTHER; note = 5'-methyluridine-3'-phosphate
  modified_base 11: mod_base = OTHER; note = 5'-methyluridine-3'-phosphate
  modified_base 14: mod_base = OTHER; note = 5'-methyluridine-3'-phosphate
  modified_base 16: mod_base = OTHER; note = 5'-methyluridine-3'-phosphate
  modified_base 18: mod_base = OTHER; note = 5'-methyluridine-3'-phosphate
  modified_base 20: mod_base = OTHER; note = 5'-methyluridine-3'-phosphate
  modified_base 21: mod_base = OTHER; note = 5'-methyluridine-3'-phosphate
  modified_base 22: mod_base = OTHER; note = 5'-methyluridine-3'-phosphate
  modified_base 23: mod_base = OTHER; note = 5'-methyluridine
atctcatgagtaatgtgtgtttt

SEQ ID NO: 645 - RNA, 23 nt, synthetic construct
  source 1..23: mol_type = other RNA
  modified_base 4: mod_base = OTHER; note = 5'-methyluridine-3'-phosphate
  modified_base 7: mod_base = OTHER; note = 5'-methyluridine-3'-phosphate
  modified_base 10: mod_base = OTHER; note = 5'-methyluridine-3'-phosphate
  modified_base 11: mod_base = OTHER; note = 5'-methyluridine-3'-phosphate
  modified_base 14: mod_base = OTHER; note = 5'-methyluridine-3'-phosphate
  modified_base 16: mod_base = OTHER; note = 5'-methyluridine-3'-phosphate
  modified_base 17: mod_base = OTHER; note = 5'-methyluridine-3'-phosphate
  modified_base 18: mod_base = OTHER; note = 5'-methyluridine-3'-phosphate
  modified_base 23: mod_base = OTHER; note = 5'-methyluridine
ggatgctgattgatatttcacat

SEQ ID NO: 646 - RNA, 23 nt, synthetic construct
  source 1..23: mol_type = other RNA
  modified_base 1: mod_base = OTHER; note = 5'-methyluridine-3'-phosphate
  modified_base 3: mod_base = OTHER; note = 5'-methyluridine-3'-phosphate
  modified_base 5: mod_base = OTHER; note = 5'-methyluridine-3'-phosphate
  modified_base 10: mod_base = OTHER; note = 5'-methyluridine-3'-phosphate
  modified_base 15: mod_base = OTHER; note = 5'-methyluridine-3'-phosphate
  modified_base 17: mod_base = OTHER; note = 5'-methyluridine-3'-phosphate
  modified_base 18: mod_base = OTHER; note = 5'-methyluridine-3'-phosphate
  modified_base 19: mod_base = OTHER; note = 5'-methyluridine-3'-phosphate
tgtatgaaataccatgtttgaaa

SEQ ID NO: 647 - RNA, 23 nt, synthetic construct
  source 1..23: mol_type = other RNA
  modified_base 2: mod_base = OTHER; note = 5'-methyluridine-3'-phosphate
  modified_base 3: mod_base = OTHER; note = 5'-methyluridine-3'-phosphate
  modified_base 4: mod_base = OTHER; note = 5'-methyluridine-3'-phosphate
  modified_base 10: mod_base = OTHER; note = 5'-methyluridine-3'-phosphate
  modified_base 13: mod_base = OTHER; note = 5'-methyluridine-3'-phosphate
  modified_base 19: mod_base = OTHER; note = 5'-methyluridine-3'-phosphate
  modified_base 22: mod_base = OTHER; note = 5'-methyluridine-3'-phosphate
gtttgaaactcatagcaataatg

SEQ ID NO: 648 - RNA, 23 nt, synthetic construct
  source 1..23: mol_type = other RNA
  modified_base 3: mod_base = OTHER; note = 5'-methyluridine-3'-phosphate
  modified_base 6: mod_base = OTHER; note = 5'-methyluridine-3'-phosphate
  modified_base 9: mod_base = OTHER; note = 5'-methyluridine-3'-phosphate
  modified_base 11: mod_base = OTHER; note = 5'-methyluridine-3'-phosphate
  modified_base 14: mod_base = OTHER; note = 5'-methyluridine-3'-phosphate
  modified_base 16: mod_base = OTHER; note = 5'-methyluridine-3'-phosphate
  modified_base 17: mod_base = OTHER; note = 5'-methyluridine-3'-phosphate
  modified_base 19: mod_base = OTHER; note = 5'-methyluridine-3'-phosphate
  modified_base 22: mod_base = OTHER; note = 5'-methyluridine-3'-phosphate
aataatgctatgctgttgtgatc

SEQ ID NO: 649 - RNA, 23 nt, synthetic construct
  source 1..23: mol_type = other RNA
  modified_base 2: mod_base = OTHER; note = 5'-methyluridine-3'-phosphate
  modified_base 7: mod_base = OTHER; note = 5'-methyluridine-3'-phosphate
  modified_base 8: mod_base = OTHER; note = 5'-methyluridine-3'-phosphate
  modified_base 10: mod_base = OTHER; note = 5'-methyluridine-3'-phosphate
  modified_base 14: mod_base = OTHER; note = 5'-methyluridine-3'-phosphate
  modified_base 15: mod_base = OTHER; note = 5'-methyluridine-3'-phosphate
  modified_base 16: mod_base = OTHER; note = 5'-methyluridine-3'-phosphate
  modified_base 21: mod_base = OTHER; note = 5'-methyluridine-3'-phosphate
  modified_base 23: mod_base = OTHER; note = 5'-methyluridine
ctcaagttctgcatttaaaatat

SEQ ID NO: 650 - RNA, 23 nt, synthetic construct
  source 1..23: mol_type = other RNA
  modified_base 1: mod_base = OTHER; note = 5'-methyluridine-3'-phosphate
  modified_base 2: mod_base = OTHER; note = 5'-methyluridine-3'-phosphate
  modified_base 5: mod_base = OTHER; note = 5'-methyluridine-3'-phosphate
  modified_base 7: mod_base = OTHER; note = 5'-methyluridine-3'-phosphate
  modified_base 9: mod_base = OTHER; note = 5'-methyluridine-3'-phosphate
  modified_base 14: mod_base = OTHER; note = 5'-methyluridine-3'-phosphate
  modified_base 19: mod_base = OTHER; note = 5'-methyluridine-3'-phosphate
  modified_base 22: mod_base = OTHER; note = 5'-methyluridine-3'-phosphate
  modified_base 23: mod_base = OTHER; note = 5'-methyluridine
ttgatgtataccatgaagtcatt

SEQ ID NO: 651 - RNA, 23 nt, synthetic construct
  source 1..23: mol_type = other RNA
  modified_base 4: mod_base = OTHER; note = 5'-methyluridine-3'-phosphate
  modified_base 5: mod_base = OTHER; note = 5'-methyluridine-3'-phosphate
  modified_base 7: mod_base = OTHER; note = 5'-methyluridine-3'-phosphate
  modified_base 10: mod_base = OTHER; note = 5'-methyluridine-3'-phosphate
  modified_base 14: mod_base = OTHER; note = 5'-methyluridine-3'-phosphate
  modified_base 16: mod_base = OTHER; note = 5'-methyluridine-3'-phosphate
  modified_base 19: mod_base = OTHER; note = 5'-methyluridine-3'-phosphate
  modified_base 21: mod_base = OTHER; note = 5'-methyluridine-3'-phosphate
  modified_base 22: mod_base = OTHER; note = 5'-methyluridine-3'-phosphate
cagttgtagtagctctgatgttg

SEQ ID NO: 652 - RNA, 23 nt, synthetic construct
  source 1..23: mol_type = other RNA
  modified_base 2: mod_base = OTHER; note = 5'-methyluridine-3'-phosphate
  modified_base 3: mod_base = OTHER; note = 5'-methyluridine-3'-phosphate
  modified_base 7: mod_base = OTHER; note = 5'-methyluridine-3'-phosphate
  modified_base 12: mod_base = OTHER; note = 5'-methyluridine-3'-phosphate
  modified_base 14: mod_base = OTHER; note = 5'-methyluridine-3'-phosphate
  modified_base 17: mod_base = OTHER; note = 5'-methyluridine-3'-phosphate
  modified_base 19: mod_base = OTHER; note = 5'-methyluridine-3'-phosphate
  modified_base 20: mod_base = OTHER; note = 5'-methyluridine-3'-phosphate
  modified_base 21: mod_base = OTHER; note = 5'-methyluridine-3'-phosphate
  modified_base 22: mod_base = OTHER; note = 5'-methyluridine-3'-phosphate
gttgaatgagatatcatgtttta

SEQ ID NO: 653 - RNA, 23 nt, synthetic construct
  source 1..23: mol_type = other RNA
  modified_base 1: mod_base = OTHER; note = 5'-methyluridine-3'-phosphate
  modified_base 3: mod_base = OTHER; note = 5'-methyluridine-3'-phosphate
  modified_base 4: mod_base = OTHER; note = 5'-methyluridine-3'-phosphate
  modified_base 5: mod_base = OTHER; note = 5'-methyluridine-3'-phosphate
  modified_base 6: mod_base = OTHER; note = 5'-methyluridine-3'-phosphate
  modified_base 11: mod_base = OTHER; note = 5'-methyluridine-3'-phosphate
  modified_base 12: mod_base = OTHER; note = 5'-methyluridine-3'-phosphate
  modified_base 16: mod_base = OTHER; note = 5'-methyluridine-3'-phosphate
  modified_base 17: mod_base = OTHER; note = 5'-methyluridine-3'-phosphate
  modified_base 18: mod_base = OTHER; note = 5'-methyluridine-3'-phosphate
  modified_base 19: mod_base = OTHER; note = 5'-methyluridine-3'-phosphate
  modified_base 22: mod_base = OTHER; note = 5'-methyluridine-3'-phosphate
tgttttagcattccattttactg

SEQ ID NO: 654 - RNA, 23 nt, synthetic construct
  source 1..23: mol_type = other RNA
  modified_base 1: mod_base = OTHER; note = 5'-methyluridine-3'-phosphate
  modified_base 3: mod_base = OTHER; note = 5'-methyluridine-3'-phosphate
  modified_base 7: mod_base = OTHER; note = 5'-methyluridine-3'-phosphate
  modified_base 8: mod_base = OTHER; note = 5'-methyluridine-3'-phosphate
  modified_base 14: mod_base = OTHER; note = 5'-methyluridine-3'-phosphate
  modified_base 15: mod_base = OTHER; note = 5'-methyluridine-3'-phosphate
  modified_base 18: mod_base = OTHER; note = 5'-methyluridine-3'-phosphate
tgtaaattaaggattactcaagc

SEQ ID NO: 655 - RNA, 23 nt, synthetic construct
  source 1..23: mol_type = other RNA
  modified_base 5: mod_base = OTHER; note = 5'-methyluridine-3'-phosphate
  modified_base 11: mod_base = OTHER; note = 5'-methyluridine-3'-phosphate
  modified_base 12: mod_base = OTHER; note = 5'-methyluridine-3'-phosphate
  modified_base 14: mod_base = OTHER; note = 5'-methyluridine-3'-phosphate
  modified_base 15: mod_base = OTHER; note = 5'-methyluridine-3'-phosphate
  modified_base 21: mod_base = OTHER; note = 5'-methyluridine-3'-phosphate
  modified_base 22: mod_base = OTHER; note = 5'-methyluridine-3'-phosphate
aagctcaccattattcaagattg

SEQ ID NO: 656 - RNA, 23 nt, synthetic construct
  source 1..23: mol_type = other RNA
  modified_base 6: mod_base = OTHER; note = 5'-methyluridine-3'-phosphate
  modified_base 7: mod_base = OTHER; note = 5'-methyluridine-3'-phosphate
  modified_base 9: mod_base = OTHER; note = 5'-methyluridine-3'-phosphate
  modified_base 11: mod_base = OTHER; note = 5'-methyluridine-3'-phosphate
  modified_base 12: mod_base = OTHER; note = 5'-methyluridine-3'-phosphate
  modified_base 16: mod_base = OTHER; note = 5'-methyluridine-3'-phosphate
  modified_base 17: mod_base = OTHER; note = 5'-methyluridine-3'-phosphate
  modified_base 19: mod_base = OTHER; note = 5'-methyluridine-3'-phosphate
  modified_base 20: mod_base = OTHER; note = 5'-methyluridine-3'-phosphate
  modified_base 21: mod_base = OTHER; note = 5'-methyluridine-3'-phosphate
  modified_base 22: mod_base = OTHER; note = 5'-methyluridine-3'-phosphate
acggcttctcttgcattattttc

SEQ ID NO: 657 - RNA, 23 nt, synthetic construct
  source 1..23: mol_type = other RNA
  modified_base 2: mod_base = OTHER; note = 5'-methyluridine-3'-phosphate
  modified_base 3: mod_base = OTHER; note = 5'-methyluridine-3'-phosphate
  modified_base 6: mod_base = OTHER; note = 5'-methyluridine-3'-phosphate
  modified_base 7: mod_base = OTHER; note = 5'-methyluridine-3'-phosphate
  modified_base 8: mod_base = OTHER; note = 5'-methyluridine-3'-phosphate
  modified_base 10: mod_base = OTHER; note = 5'-methyluridine-3'-phosphate
  modified_base 11: mod_base = OTHER; note = 5'-methyluridine-3'-phosphate
  modified_base 12: mod_base = OTHER; note = 5'-methyluridine-3'-phosphate
  modified_base 13: mod_base = OTHER; note = 5'-methyluridine-3'-phosphate
  modified_base 15: mod_base = OTHER; note = 5'-methyluridine-3'-phosphate
  modified_base 21: mod_base = OTHER; note = 5'-methyluridine-3'-phosphate
gttggtttgttttctagaagtac

SEQ ID NO: 658 - RNA, 23 nt, synthetic construct
  source 1..23: mol_type = other RNA
  modified_base 4: mod_base = OTHER; note = 5'-methyluridine-3'-phosphate
  modified_base 7: mod_base = OTHER; note = 5'-methyluridine-3'-phosphate
  modified_base 10: mod_base = OTHER; note = 5'-methyluridine-3'-phosphate
  modified_base 11: mod_base = OTHER; note = 5'-methyluridine-3'-phosphate
  modified_base 12: mod_base = OTHER; note = 5'-methyluridine-3'-phosphate
  modified_base 18: mod_base = OTHER; note = 5'-methyluridine-3'-phosphate
  modified_base 20: mod_base = OTHER; note = 5'-methyluridine-3'-phosphate
  modified_base 21: mod_base = OTHER; note = 5'-methyluridine-3'-phosphate
  modified_base 22: mod_base = OTHER; note = 5'-methyluridine-3'-phosphate
  modified_base 23: mod_base = OTHER; note = 5'-methyluridine
aactggtgctttgaaaatctttt

SEQ ID NO: 659 - RNA, 23 nt, synthetic construct
  source 1..23: mol_type = other RNA
  modified_base 5: mod_base = OTHER; note = 5'-methyluridine-3'-phosphate
  modified_base 10: mod_base = OTHER; note = 5'-methyluridine-3'-phosphate
  modified_base 11: mod_base = OTHER; note = 5'-methyluridine-3'-phosphate
  modified_base 12: mod_base = OTHER; note = 5'-methyluridine-3'-phosphate
  modified_base 16: mod_base = OTHER; note = 5'-methyluridine-3'-phosphate
  modified_base 17: mod_base = OTHER; note = 5'-methyluridine-3'-phosphate
  modified_base 20: mod_base = OTHER; note = 5'-methyluridine-3'-phosphate
  modified_base 21: mod_base = OTHER; note = 5'-methyluridine-3'-phosphate
  modified_base 22: mod_base = OTHER; note = 5'-methyluridine-3'-phosphate
aagctgacctttgagttaatttc

SEQ ID NO: 660 - RNA, 23 nt, synthetic construct
  source 1..23: mol_type = other RNA
  modified_base 1: mod_base = OTHER; note = 5'-methyluridine-3'-phosphate
  modified_base 11: mod_base = OTHER; note = 5'-methyluridine-3'-phosphate
  modified_base 14: mod_base = OTHER; note = 5'-methyluridine-3'-phosphate
  modified_base 15: mod_base = OTHER; note = 5'-methyluridine-3'-phosphate
  modified_base 17: mod_base = OTHER; note = 5'-methyluridine-3'-phosphate
  modified_base 18: mod_base = OTHER; note = 5'-methyluridine-3'-phosphate
  modified_base 22: mod_base = OTHER; note = 5'-methyluridine-3'-phosphate
tcagcacaactcattcttcagtg

SEQ ID NO: 661 - RNA, 23 nt, synthetic construct
  source 1..23: mol_type = other RNA
  modified_base 3: mod_base = OTHER; note = 5'-methyluridine-3'-phosphate
  modified_base 7: mod_base = OTHER; note = 5'-methyluridine-3'-phosphate
  modified_base 10: mod_base = OTHER; note = 5'-methyluridine-3'-phosphate
  modified_base 14: mod_base = OTHER; note = 5'-methyluridine-3'-phosphate
agtgcctcatgactgaaaacaaa

SEQ ID NO: 662 - RNA, 23 nt, synthetic construct
  source 1..23: mol_type = other RNA
  modified_base 11: mod_base = OTHER; note = 5'-methyluridine-3'-phosphate
  modified_base 13: mod_base = OTHER; note = 5'-methyluridine-3'-phosphate
  modified_base 14: mod_base = OTHER; note = 5'-methyluridine-3'-phosphate
  modified_base 20: mod_base = OTHER; note = 5'-methyluridine-3'-phosphate
aacgaaagcatcttcacaatgaa

SEQ ID NO: 663 - RNA, 23 nt, synthetic construct
  source 1..23: mol_type = other RNA
  modified_base 4: mod_base = OTHER; note = 5'-methyluridine-3'-phosphate
  modified_base 12: mod_base = OTHER; note = 5'-methyluridine-3'-phosphate
  modified_base 13: mod_base = OTHER; note = 5'-methyluridine-3'-phosphate
  modified_base 14: mod_base = OTHER; note = 5'-methyluridine-3'-phosphate
  modified_base 15: mod_base = OTHER; note = 5'-methyluridine-3'-phosphate
  modified_base 18: mod_base = OTHER; note = 5'-methyluridine-3'-phosphate
agatagcaccgttttgctaaaag

SEQ ID NO: 664 - RNA, 23 nt, synthetic construct
  source 1..23: mol_type = other RNA
  modified_base 5: mod_base = OTHER; note = 5'-methyluridine-3'-phosphate
  modified_base 9: mod_base = OTHER; note = 5'-methyluridine-3'-phosphate
  modified_base 10: mod_base = OTHER; note = 5'-methyluridine-3'-phosphate
  modified_base 12: mod_base = OTHER; note = 5'-methyluridine-3'-phosphate
  modified_base 15: mod_base = OTHER; note = 5'-methyluridine-3'-phosphate
  modified_base 16: mod_base = OTHER; note = 5'-methyluridine-3'-phosphate
  modified_base 18: mod_base = OTHER; note = 5'-methyluridine-3'-phosphate
  modified_base 19: mod_base = OTHER; note = 5'-methyluridine-3'-phosphate
  modified_base 20: mod_base = OTHER; note = 5'-methyluridine-3'-phosphate
  modified_base 21: mod_base = OTHER; note = 5'-methyluridine-3'-phosphate
aagatacattctcattgttttcc

SEQ ID NO: 665 - RNA, 23 nt, synthetic construct
  source 1..23: mol_type = other RNA
  modified_base 2: mod_base = OTHER; note = 5'-methyluridine-3'-phosphate
  modified_base 3: mod_base = OTHER; note = 5'-methyluridine-3'-phosphate
  modified_base 9: mod_base = OTHER; note = 5'-methyluridine-3'-phosphate
  modified_base 14: mod_base = OTHER; note = 5'-methyluridine-3'-phosphate
  modified_base 15: mod_base = OTHER; note = 5'-methyluridine-3'-phosphate
cttccacataaggttaaacaaac

SEQ ID NO: 666 - RNA, 23 nt, synthetic construct
  source 1..23: mol_type = other RNA
  modified_base 2: mod_base = OTHER; note = 5'-methyluridine-3'-phosphate
  modified_base 6: mod_base = OTHER; note = 5'-methyluridine-3'-phosphate
  modified_base 9: mod_base = OTHER; note = 5'-methyluridine-3'-phosphate
  modified_base 10: mod_base = OTHER; note = 5'-methyluridine-3'-phosphate
  modified_base 12: mod_base = OTHER; note = 5'-methyluridine-3'-phosphate
  modified_base 16: mod_base = OTHER; note = 5'-methyluridine-3'-phosphate
  modified_base 19: mod_base = OTHER; note = 5'-methyluridine-3'-phosphate
  modified_base 20: mod_base = OTHER; note = 5'-methyluridine-3'-phosphate
  modified_base 21: mod_base = OTHER; note = 5'-methyluridine-3'-phosphate
  modified_base 23: mod_base = OTHER; note = 5'-methyluridine
ctaggtgcttgtaaataatttat

SEQ ID NO: 667 - RNA, 23 nt, synthetic construct
  source 1..23: mol_type = other RNA
  modified_base 1: mod_base = OTHER; note = 5'-methyluridine-3'-phosphate
  modified_base 4: mod_base = OTHER; note = 5'-methyluridine-3'-phosphate
  modified_base 6: mod_base = OTHER; note = 5'-methyluridine-3'-phosphate
  modified_base 8: mod_base = OTHER; note = 5'-methyluridine-3'-phosphate
  modified_base 13: mod_base = OTHER; note = 5'-methyluridine-3'-phosphate
  modified_base 14: mod_base = OTHER; note = 5'-methyluridine-3'-phosphate
  modified_base 15: mod_base = OTHER; note = 5'-methyluridine-3'-phosphate
  modified_base 17: mod_base = OTHER; note = 5'-methyluridine-3'-phosphate
  modified_base 19: mod_base = OTHER; note = 5'-methyluridine-3'-phosphate
tactctatcgcatttctgtaaca

SEQ ID NO: 668 - RNA, 23 nt, synthetic construct
  source 1..23: mol_type = other RNA
  modified_base 1: mod_base = OTHER; note = 5'-methyluridine-3'-phosphate
  modified_base 7: mod_base = OTHER; note = 5'-methyluridine-3'-phosphate
  modified_base 13: mod_base = OTHER; note = 5'-methyluridine-3'-phosphate
  modified_base 15: mod_base = OTHER; note = 5'-methyluridine-3'-phosphate
  modified_base 18: mod_base = OTHER; note = 5'-methyluridine-3'-phosphate
  modified_base 22: mod_base = OTHER; note = 5'-methyluridine-3'-phosphate
tgaaaatgagaatgtcctaagtg

SEQ ID NO: 669 - RNA, 23 nt, synthetic construct
  source 1..23: mol_type = other RNA
  modified_base 1: mod_base = OTHER; note = 5'-methyluridine-3'-phosphate
  modified_base 6: mod_base = OTHER; note = 5'-methyluridine-3'-phosphate
  modified_base 8: mod_base = OTHER; note = 5'-methyluridine-3'-phosphate
  modified_base 14: mod_base = OTHER; note = 5'-methyluridine-3'-phosphate
  modified_base 18: mod_base = OTHER; note = 5'-methyluridine-3'-phosphate
tgcactctgaaaatgcatgaaaa

SEQ ID NO: 670 - RNA, 23 nt, synthetic construct
  source 1..23: mol_type = other RNA
  modified_base 5: mod_base = OTHER; note = 5'-methyluridine-3'-phosphate
  modified_base 7: mod_base = OTHER; note = 5'-methyluridine-3'-phosphate
  modified_base 9: mod_base = OTHER; note = 5'-methyluridine-3'-phosphate
  modified_base 15: mod_base = OTHER; note = 5'-methyluridine-3'-phosphate
  modified_base 17: mod_base = OTHER; note = 5'-methyluridine-3'-phosphate
  modified_base 18: mod_base = OTHER; note = 5'-methyluridine-3'-phosphate
  modified_base 22: mod_base = OTHER; note = 5'-methyluridine-3'-phosphate
gaaatgtgtagaactgttaactg

SEQ ID NO: 671 - RNA, 23 nt, synthetic construct
  source 1..23: mol_type = other RNA
  modified_base 1: mod_base = OTHER; note = 5'-methyluridine-3'-phosphate
  modified_base 4: mod_base = OTHER; note = 5'-methyluridine-3'-phosphate
  modified_base 5: mod_base = OTHER; note = 5'-methyluridine-3'-phosphate
  modified_base 7: mod_base = OTHER; note = 5'-methyluridine-3'-phosphate
  modified_base 12: mod_base = OTHER; note = 5'-methyluridine-3'-phosphate
  modified_base 14: mod_base = OTHER; note = 5'-methyluridine-3'-phosphate
  modified_base 16: mod_base = OTHER; note = 5'-methyluridine-3'-phosphate
  modified_base 17: mod_base = OTHER; note = 5'-methyluridine-3'-phosphate
  modified_base 21: mod_base = OTHER; note = 5'-methyluridine-3'-phosphate
  modified_base 22: mod_base = OTHER; note = 5'-methyluridine-3'-phosphate
  modified_base 23: mod_base = OTHER; note = 5'-methyluridine
tccttctggaatctgttaaattt

SEQ ID NO: 672 - RNA, 23 nt, synthetic construct
  source 1..23: mol_type = other RNA
  modified_base 2: mod_base = OTHER; note = 5'-methyluridine-3'-phosphate
  modified_base 8: mod_base = OTHER; note = 5'-methyluridine-3'-phosphate
  modified_base 12: mod_base = OTHER; note = 5'-methyluridine-3'-phosphate
  modified_base 21: mod_base = OTHER; note = 5'-methyluridine-3'-phosphate
  modified_base 23: mod_base = OTHER; note = 5'-methyluridine
atgagggtaaatggagaaaatat

SEQ ID NO: 673 - RNA, 23 nt, synthetic construct
  source 1..23: mol_type = other RNA
  modified_base 1: mod_base = OTHER; note = 5'-methyluridine-3'-phosphate
  modified_base 3: mod_base = OTHER; note = 5'-methyluridine-3'-phosphate
  modified_base 8: mod_base = OTHER; note = 5'-methyluridine-3'-phosphate
  modified_base 9: mod_base = OTHER; note = 5'-methyluridine-3'-phosphate
  modified_base 14: mod_base = OTHER; note = 5'-methyluridine-3'-phosphate
  modified_base 18: mod_base = OTHER; note = 5'-methyluridine-3'-phosphate
  modified_base 20: mod_base = OTHER; note = 5'-methyluridine-3'-phosphate
tctgggattacaatgaatgtaag

SEQ ID NO: 674 - RNA, 23 nt, synthetic construct
  source 1..23: mol_type = other RNA
  modified_base 1: mod_base = OTHER; note = 5'-methyluridine-3'-phosphate
  modified_base 3: mod_base = OTHER; note = 5'-methyluridine-3'-phosphate
  modified_base 13: mod_base = OTHER; note = 5'-methyluridine-3'-phosphate
  modified_base 14: mod_base = OTHER; note = 5'-methyluridine-3'-phosphate
  modified_base 16: mod_base = OTHER; note = 5'-methyluridine-3'-phosphate
  modified_base 21: mod_base = OTHER; note = 5'-methyluridine-3'-phosphate
  modified_base 22: mod_base = OTHER; note = 5'-methyluridine-3'-phosphate
tgtaagcccaaattgtggaattg

SEQ ID NO: 675 - RNA, 23 nt, synthetic construct
  source 1..23: mol_type = other RNA
  modified_base 2: mod_base = OTHER; note = 5'-methyluridine-3'-phosphate
  modified_base 3: mod_base = OTHER; note = 5'-methyluridine-3'-phosphate
  modified_base 6: mod_base = OTHER; note = 5'-methyluridine-3'-phosphate
  modified_base 10: mod_base = OTHER; note = 5'-methyluridine-3'-phosphate
  modified_base 12: mod_base = OTHER; note = 5'-methyluridine-3'-phosphate
  modified_base 13: mod_base = OTHER; note = 5'-methyluridine-3'-phosphate
  modified_base 14: mod_base = OTHER; note = 5'-methyluridine-3'-phosphate
  modified_base 15: mod_base = OTHER; note = 5'-methyluridine-3'-phosphate
  modified_base 17: mod_base = OTHER; note = 5'-methyluridine-3'-phosphate
  modified_base 23: mod_base = OTHER; note = 5'-methyluridine
gttcatcagtgttttatagaaat

SEQ ID NO: 676 - RNA, 23 nt, synthetic construct
  source 1..23: mol_type = other RNA
  modified_base 4: mod_base = OTHER; note = 5'-methyluridine-3'-phosphate
  modified_base 5: mod_base = OTHER; note = 5'-methyluridine-3'-phosphate
  modified_base 14: mod_base = OTHER; note = 5'-methyluridine-3'-phosphate
  modified_base 16: mod_base = OTHER; note = 5'-methyluridine-3'-phosphate
  modified_base 17: mod_base = OTHER; note = 5'-methyluridine-3'-phosphate
  modified_base 18: mod_base = OTHER; note = 5'-methyluridine-3'-phosphate
  modified_base 19: mod_base = OTHER; note = 5'-methyluridine-3'-phosphate
gcattgcccaaactattttgaca

SEQ ID NO: 677 - RNA, 23 nt, synthetic construct
  source 1..23: mol_type = other RNA
  modified_base 2: mod_base = OTHER; note = 5'-methyluridine-3'-phosphate
  modified_base 5: mod_base = OTHER; note = 5'-methyluridine-3'-phosphate
  modified_base 6: mod_base = OTHER; note = 5'-methyluridine-3'-phosphate
  modified_base 8: mod_base = OTHER; note = 5'-methyluridine-3'-phosphate
  modified_base 14: mod_base = OTHER; note = 5'-methyluridine-3'-phosphate
  modified_base 16: mod_base = OTHER; note = 5'-methyluridine-3'-phosphate
  modified_base 20: mod_base = OTHER; note = 5'-methyluridine-3'-phosphate
  modified_base 23: mod_base = OTHER; note = 5'-methyluridine
atacttatgaacctctcactaat

SEQ ID NO: 678 - RNA, 23 nt, synthetic construct
  source 1..23: mol_type = other RNA
  modified_base 1: mod_base = OTHER; note = 5'-methyluridine-3'-phosphate
  modified_base 2: mod_base = OTHER; note = 5'-methyluridine-3'-phosphate
  modified_base 3: mod_base = OTHER; note = 5'-methyluridine-3'-phosphate
  modified_base 4: mod_base = OTHER; note = 5'-methyluridine-3'-phosphate
  modified_base 14: mod_base = OTHER; note = 5'-methyluridine-3'-phosphate
  modified_base 16: mod_base = OTHER; note = 5'-methyluridine-3'-phosphate
  modified_base 18: mod_base = OTHER; note = 5'-methyluridine-3'-phosphate
  modified_base 19: mod_base = OTHER; note = 5'-methyluridine-3'-phosphate
  modified_base 23: mod_base = OTHER; note = 5'-methyluridine
ttttgggaaacactatgttagat

SEQ ID NO: 679 - RNA, 23 nt, synthetic construct
  source 1..23: mol_type = other RNA
  modified_base 2: mod_base = OTHER; note = 5'-methyluridine-3'-phosphate
  modified_base 5: mod_base = OTHER; note = 5'-methyluridine-3'-phosphate
  modified_base 6: mod_base = OTHER; note = 5'-methyluridine-3'-phosphate
  modified_base 8: mod_base = OTHER; note = 5'-methyluridine-3'-phosphate
  modified_base 9: mod_base = OTHER; note = 5'-methyluridine-3'-phosphate
  modified_base 10: mod_base = OTHER; note = 5'-methyluridine-3'-phosphate
atagttctttaaggagacaaaac

SEQ ID NO: 680 - RNA, 23 nt, synthetic construct
  source 1..23: mol_type = other RNA
  modified_base 4: mod_base = OTHER; note = 5'-methyluridine-3'-phosphate
  modified_base 6: mod_base = OTHER; note = 5'-methyluridine-3'-phosphate
  modified_base 10: mod_base = OTHER; note = 5'-methyluridine-3'-phosphate
  modified_base 14: mod_base = OTHER; note = 5'-methyluridine-3'-phosphate
  modified_base 15: mod_base = OTHER; note = 5'-methyluridine-3'-phosphate
  modified_base 16: mod_base = OTHER; note = 5'-methyluridine-3'-phosphate
  modified_base 17: mod_base = OTHER; note = 5'-methyluridine-3'-phosphate
  modified_base 19: mod_base = OTHER; note = 5'-methyluridine-3'-phosphate
gaatatgcatgcattttgtaacg

SEQ ID NO: 681 - RNA, 23 nt, synthetic construct
  source 1..23: mol_type = other RNA
  modified_base 5: mod_base = OTHER; note = 5'-methyluridine-3'-phosphate
  modified_base 6: mod_base = OTHER; note = 5'-methyluridine-3'-phosphate
  modified_base 10: mod_base = OTHER; note = 5'-methyluridine-3'-phosphate
  modified_base 14: mod_base = OTHER; note = 5'-methyluridine-3'-phosphate
  modified_base 16: mod_base = OTHER; note = 5'-methyluridine-3'-phosphate
  modified_base 18: mod_base = OTHER; note = 5'-methyluridine-3'-phosphate
  modified_base 20: mod_base = OTHER; note = 5'-methyluridine-3'-phosphate
  modified_base 21: mod_base = OTHER; note = 5'-methyluridine-3'-phosphate
  modified_base 22: mod_base = OTHER; note = 5'-methyluridine-3'-phosphate
ggcgttgaatagatgtgtatttc

SEQ ID NO: 682 - RNA, 23 nt, synthetic construct
  source 1..23: mol_type = other RNA
  modified_base 8: mod_base = OTHER; note = 5'-methyluridine-3'-phosphate
  modified_base 21: mod_base = OTHER; note = 5'-methyluridine-3'-phosphate
  modified_base 22: mod_base = OTHER; note = 5'-methyluridine-3'-phosphate
cagaaaataagcacagaaaatta

SEQ ID NO: 683 - RNA, 23 nt, synthetic construct
  source 1..23: mol_type = other RNA
  modified_base 1: mod_base = OTHER; note = 5'-methyluridine-3'-phosphate
  modified_base 2: mod_base = OTHER; note = 5'-methyluridine-3'-phosphate
  modified_base 3: mod_base = OTHER; note = 5'-methyluridine-3'-phosphate
  modified_base 4: mod_base = OTHER; note = 5'-methyluridine-3'-phosphate
  modified_base 8: mod_base = OTHER; note = 5'-methyluridine-3'-phosphate
  modified_base 14: mod_base = OTHER; note = 5'-methyluridine-3'-phosphate
  modified_base 16: mod_base = OTHER; note = 5'-methyluridine-3'-phosphate
  modified_base 22: mod_base = OTHER; note = 5'-methyluridine-3'-phosphate
ttttcactgaacgtatcagaata

SEQ ID NO: 684 - RNA, 23 nt, synthetic construct
  source 1..23: mol_type = other RNA
  modified_base 3: mod_base = OTHER; note = 5'-methyluridine-3'-phosphate
  modified_base 7: mod_base = OTHER; note = 5'-methyluridine-3'-phosphate
  modified_base 12: mod_base = OTHER; note = 5'-methyluridine-3'-phosphate
  modified_base 13: mod_base = OTHER; note = 5'-methyluridine-3'-phosphate
  modified_base 14: mod_base = OTHER; note = 5'-methyluridine-3'-phosphate
  modified_base 15: mod_base = OTHER; note = 5'-methyluridine-3'-phosphate
  modified_base 18: mod_base = OTHER; note = 5'-methyluridine-3'-phosphate
  modified_base 19: mod_base = OTHER; note = 5'-methyluridine-3'-phosphate
ggtaaataaggttttaattcaga

SEQ ID NO: 685 - RNA, 23 nt, synthetic construct
  source 1..23: mol_type = other RNA
  modified_base 1: mod_base = OTHER; note = 5'-methyluridine-3'-phosphate
  modified_base 2: mod_base = OTHER; note = 5'-methyluridine-3'-phosphate
  modified_base 7: mod_base = OTHER; note = 5'-methyluridine-3'-phosphate
  modified_base 9: mod_base = OTHER; note = 5'-methyluridine-3'-phosphate
  modified_base 19: mod_base = OTHER; note = 5'-methyluridine-3'-phosphate
  modified_base 21: mod_base = OTHER; note = 5'-methyluridine-3'-phosphate
  modified_base 22: mod_base = OTHER; note = 5'-methyluridine-3'-phosphate
ttcagatctagaagaaagtattg

SEQ ID NO: 686 - RNA, 23 nt, synthetic construct
  source 1..23: mol_type = other RNA
  modified_base 8: mod_base = OTHER; note = 5'-methyluridine-3'-phosphate
  modified_base 11: mod_base = OTHER; note = 5'-methyluridine-3'-phosphate
  modified_base 12: mod_base = OTHER; note = 5'-methyluridine-3'-phosphate
  modified_base 14: mod_base = OTHER; note = 5'-methyluridine-3'-phosphate
  modified_base 17: mod_base = OTHER; note = 5'-methyluridine-3'-phosphate
  modified_base 19: mod_base = OTHER; note = 5'-methyluridine-3'-phosphate
  modified_base 20: mod_base = OTHER; note = 5'-methyluridine-3'-phosphate
  modified_base 21: mod_base = OTHER; note = 5'-methyluridine-3'-phosphate
ccacagatagttgtagtgtttag

SEQ ID NO: 687 - RNA, 23 nt, synthetic construct
  source 1..23: mol_type = other RNA
  modified_base 1: mod_base = OTHER; note = 5'-methyluridine-3'-phosphate
  modified_base 4: mod_base = OTHER; note = 5'-methyluridine-3'-phosphate
  modified_base 5: mod_base = OTHER; note = 5'-methyluridine-3'-phosphate
  modified_base 10: mod_base = OTHER; note = 5'-methyluridine-3'-phosphate
  modified_base 11: mod_base = OTHER; note = 5'-methyluridine-3'-phosphate
  modified_base 12: mod_base = OTHER; note = 5'-methyluridine-3'-phosphate
  modified_base 14: mod_base = OTHER; note = 5'-methyluridine-3'-phosphate
  modified_base 20: mod_base = OTHER; note = 5'-methyluridine-3'-phosphate
  modified_base 21: mod_base = OTHER; note = 5'-methyluridine-3'-phosphate
tcgttgaggtttctaagacttac

SEQ ID NO: 688 - RNA, 23 nt, synthetic construct
  source 1..23: mol_type = other RNA
  modified_base 2: mod_base = OTHER; note = 5'-methyluridine-3'-phosphate
  modified_base 4: mod_base = OTHER; note = 5'-methyluridine-3'-phosphate
  modified_base 5: mod_base = OTHER; note = 5'-methyluridine-3'-phosphate
  modified_base 6: mod_base = OTHER; note = 5'-methyluridine-3'-phosphate
  modified_base 7: mod_base = OTHER; note = 5'-methyluridine-3'-phosphate
  modified_base 15: mod_base = OTHER; note = 5'-methyluridine-3'-phosphate
  modified_base 21: mod_base = OTHER; note = 5'-methyluridine-3'-phosphate
  modified_base 22: mod_base = OTHER; note = 5'-methyluridine-3'-phosphate
ctattttagaaacctgagacttg

SEQ ID NO: 689 - RNA, 23 nt, synthetic construct
  source 1..23: mol_type = other RNA
  modified_base 3: mod_base = OTHER; note = 5'-methyluridine-3'-phosphate
  modified_base 5: mod_base = OTHER; note = 5'-methyluridine-3'-phosphate
  modified_base 10: mod_base = OTHER; note = 5'-methyluridine-3'-phosphate
  modified_base 11: mod_base = OTHER; note = 5'-methyluridine-3'-phosphate
  modified_base 12: mod_base = OTHER; note = 5'-methyluridine-3'-phosphate
  modified_base 13: mod_base = OTHER; note = 5'-methyluridine-3'-phosphate
  modified_base 16: mod_base = OTHER; note = 5'-methyluridine-3'-phosphate
  modified_base 17: mod_base = OTHER; note = 5'-methyluridine-3'-phosphate
  modified_base 18: mod_base = OTHER; note = 5'-methyluridine-3'-phosphate
  modified_base 21: mod_base = OTHER; note = 5'-methyluridine-3'-phosphate
cgtctggcattttagtttaatac

SEQ ID NO: 690 - RNA, 23 nt, synthetic construct
  source 1..23: mol_type = other RNA
  modified_base 6: mod_base = OTHER; note = 5'-methyluridine-3'-phosphate
  modified_base 9: mod_base = OTHER; note = 5'-methyluridine-3'-phosphate
  modified_base 12: mod_base = OTHER; note = 5'-methyluridine-3'-phosphate
  modified_base 13: mod_base = OTHER; note = 5'-methyluridine-3'-phosphate
  modified_base 17: mod_base = OTHER; note = 5'-methyluridine-3'-phosphate
  modified_base 18: mod_base = OTHER; note = 5'-methyluridine-3'-phosphate
  modified_base 19: mod_base = OTHER; note = 5'-methyluridine-3'-phosphate
caaactaatgattgcatttgaaa

SEQ ID NO: 691 - RNA, 23 nt, synthetic construct
  source 1..23: mol_type = other RNA
  modified_base 1: mod_base = OTHER; note = 5'-methyluridine-3'-phosphate
  modified_base 10: mod_base = OTHER; note = 5'-methyluridine-3'-phosphate
  modified_base 11: mod_base = OTHER; note = 5'-methyluridine-3'-phosphate
  modified_base 13: mod_base = OTHER; note = 5'-methyluridine-3'-phosphate
  modified_base 14: mod_base = OTHER; note = 5'-methyluridine-3'-phosphate
  modified_base 19: mod_base = OTHER; note = 5'-methyluridine-3'-phosphate
  modified_base 20: mod_base = OTHER; note = 5'-methyluridine-3'-phosphate
  modified_base 22: mod_base = OTHER; note = 5'-methyluridine-3'-phosphate
  modified_base 23: mod_base = OTHER; note = 5'-methyluridine
tgaaagagattcttgaccttatt

SEQ ID NO: 692 - RNA, 23 nt, synthetic construct
  source 1..23: mol_type = other RNA
  modified_base 1: mod_base = OTHER; note = 5'-methyluridine-3'-phosphate
  modified_base 7: mod_base = OTHER; note = 5'-methyluridine-3'-phosphate
  modified_base 9: mod_base = OTHER; note = 5'-methyluridine-3'-phosphate
  modified_base 14: mod_base = OTHER; note = 5'-methyluridine-3'-phosphate
  modified_base 16: mod_base = OTHER; note = 5'-methyluridine-3'-phosphate
  modified_base 18: mod_base = OTHER; note = 5'-methyluridine-3'-phosphate
  modified_base 19: mod_base = OTHER; note = 5'-methyluridine-3'-phosphate
  modified_base 22: mod_base = OTHER; note = 5'-methyluridine-3'-phosphate
tagagctctgaaatgtcttgatg

SEQ ID NO: 693 - RNA, 23 nt, synthetic construct
  source 1..23: mol_type = other RNA
  modified_base 3: mod_base = OTHER; note = 5'-methyluridine-3'-phosphate
  modified_base 10: mod_base = OTHER; note = 5'-methyluridine-3'-phosphate
  modified_base 12: mod_base = OTHER; note = 5'-methyluridine-3'-phosphate
  modified_base 13: mod_base = OTHER; note = 5'-methyluridine-3'-phosphate
  modified_base 18: mod_base = OTHER; note = 5'-methyluridine-3'-phosphate
  modified_base 20: mod_base = OTHER; note = 5'-methyluridine-3'-phosphate
  modified_base 21: mod_base = OTHER; note = 5'-methyluridine-3'-phosphate
  modified_base 22: mod_base = OTHER; note = 5'-methyluridine-3'-phosphate
gatggaaggtattaaactatttg

SEQ ID NO: 694 - RNA, 23 nt, synthetic construct
  source 1..23: mol_type = other RNA
  modified_base 1: mod_base = OTHER; note = 5'-methyluridine-3'-phosphate
  modified_base 2: mod_base = OTHER; note = 5'-methyluridine-3'-phosphate
  modified_base 3: mod_base = OTHER; note = 5'-methyluridine-3'-phosphate
  modified_base 7: mod_base = OTHER; note = 5'-methyluridine-3'-phosphate
  modified_base 9: mod_base = OTHER; note = 5'-methyluridine-3'-phosphate
  modified_base 10: mod_base = OTHER; note = 5'-methyluridine-3'-phosphate
  modified_base 12: mod_base = OTHER; note = 5'-methyluridine-3'-phosphate
  modified_base 22: mod_base = OTHER; note = 5'-methyluridine-3'-phosphate
tttgcctgttgtacaaagaaatg

SEQ ID NO: 695 - RNA, 23 nt, synthetic construct
  source 1..23: mol_type = other RNA
  modified_base 5: mod_base = OTHER; note = 5'-methyluridine-3'-phosphate
  modified_base 8: mod_base = OTHER; note = 5'-methyluridine-3'-phosphate
  modified_base 17: mod_base = OTHER; note = 5'-methyluridine-3'-phosphate
  modified_base 18: mod_base = OTHER; note = 5'-methyluridine-3'-phosphate
  modified_base 21: mod_base = OTHER; note = 5'-methyluridine-3'-phosphate
  modified_base 23: mod_base = OTHER; note = 5'-methyluridine
agactcgtgaaaagaattactat

SEQ ID NO: 696 - RNA, 23 nt, synthetic construct
  source 1..23: mol_type = other RNA
  modified_base 1: mod_base = OTHER; note = 5'-methyluridine-3'-phosphate
  modified_base 3: mod_base = OTHER; note = 5'-methyluridine-3'-phosphate
  modified_base 8: mod_base = OTHER; note = 5'-methyluridine-3'-phosphate
  modified_base 12: mod_base = OTHER; note = 5'-methyluridine-3'-phosphate
  modified_base 17: mod_base = OTHER; note = 5'-methyluridine-3'-phosphate
  modified_base 18: mod_base = OTHER; note = 5'-methyluridine-3'-phosphate
  modified_base 19: mod_base = OTHER; note = 5'-methyluridine-3'-phosphate
  modified_base 20: mod_base = OTHER; note = 5'-methyluridine-3'-phosphate
  modified_base 22: mod_base = OTHER; note = 5'-methyluridine-3'-phosphate
tgtgaaataactgcgattttgtg

SEQ ID NO: 697 - RNA, 23 nt, synthetic construct
  source 1..23: mol_type = other RNA
  modified_base 3: mod_base = OTHER; note = 5'-methyluridine-3'-phosphate
  modified_base 4: mod_base = OTHER; note = 5'-methyluridine-3'-phosphate
  modified_base 10: mod_base = OTHER; note = 5'-methyluridine-3'-phosphate
  modified_base 13: mod_base = OTHER; note = 5'-methyluridine-3'-phosphate
  modified_base 16: mod_base = OTHER; note = 5'-methyluridine-3'-phosphate
  modified_base 17: mod_base = OTHER; note = 5'-methyluridine-3'-phosphate
  modified_base 20: mod_base = OTHER; note = 5'-methyluridine-3'-phosphate
  modified_base 21: mod_base = OTHER; note = 5'-methyluridine-3'-phosphate
  modified_base 22: mod_base = OTHER; note = 5'-methyluridine-3'-phosphate
  modified_base 23: mod_base = OTHER; note = 5'-methyluridine
acttggaaatgctgattgatttt

SEQ ID NO: 698 - RNA, 23 nt, synthetic construct
  source 1..23: mol_type = other RNA
  modified_base 1: mod_base = OTHER; note = 5'-methyluridine-3'-phosphate
  modified_base 3: mod_base = OTHER; note = 5'-methyluridine-3'-phosphate
  modified_base 4: mod_base = OTHER; note = 5'-methyluridine-3'-phosphate
  modified_base 7: mod_base = OTHER; note = 5'-methyluridine-3'-phosphate
  modified_base 9: mod_base = OTHER; note = 5'-methyluridine-3'-phosphate
  modified_base 11: mod_base = OTHER; note = 5'-methyluridine-3'-phosphate
  modified_base 12: mod_base = OTHER; note = 5'-methyluridine-3'-phosphate
tgttagtgtattgcaagaaacac

SEQ ID NO: 699 - RNA, 23 nt, synthetic construct
  source 1..23: mol_type = other RNA
  modified_base 10: mod_base = OTHER; note = 5'-methyluridine-3'-phosphate
  modified_base 12: mod_base = OTHER; note = 5'-methyluridine-3'-phosphate
  modified_base 15: mod_base = OTHER; note = 5'-methyluridine-3'-phosphate
  modified_base 16: mod_base = OTHER; note = 5'-methyluridine-3'-phosphate
  modified_base 17: mod_base = OTHER; note = 5'-methyluridine-3'-phosphate
  modified_base 18: mod_base = OTHER; note = 5'-methyluridine-3'-phosphate
  modified_base 20: mod_base = OTHER; note = 5'-methyluridine-3'-phosphate
  modified_base 21: mod_base = OTHER; note = 5'-methyluridine-3'-phosphate
  modified_base 22: mod_base = OTHER; note = 5'-methyluridine-3'-phosphate
  modified_base 23: mod_base = OTHER; note = 5'-methyluridine
cacagaaaatgtagttttgtttt

SEQ ID NO: 700 - RNA, 21 nt, synthetic construct
  source 1..21: mol_type = other RNA
acaatagacgtttcttatcta

SEQ ID NO: 701 - RNA, 21 nt, synthetic construct
  source 1..21: mol_type = other RNA
tgcggaatgttatttatatca

SEQ ID NO: 702 - RNA, 21 nt, synthetic construct
  source 1..21: mol_type = other RNA
gtcttacatcctttttgttca

SEQ ID NO: 703 - RNA, 21 nt, synthetic construct
  source 1..21: mol_type = other RNA
ctcttcaacagcttcttctga

SEQ ID NO: 704 - RNA, 21 nt, synthetic construct
  source 1..21: mol_type = other RNA
cttcaacagcttcttctggaa

SEQ ID NO: 705 - RNA, 21 nt, synthetic construct
  source 1..21: mol_type = other RNA
cgtcttcagtaccttgattca

SEQ ID NO: 706 - RNA, 21 nt, synthetic construct
  source 1..21: mol_type = other RNA
tcttcagtaccttgattcaca

SEQ ID NO: 707 - RNA, 21 nt, synthetic construct
  source 1..21: mol_type = other RNA
cagtctttgaactcaacttca

SEQ ID NO: 708 - RNA, 21 nt, synthetic construct
  source 1..21: mol_type = other RNA
cagcaattcatcacctttcta

SEQ ID NO: 709 - RNA, 21 nt, synthetic construct
  source 1..21: mol_type = other RNA
taggtgaaatctcagtaagta

SEQ ID NO: 710 - RNA, 21 nt, synthetic construct
  source 1..21: mol_type = other RNA
tgaaatctcagtaagttatta

SEQ ID NO: 711 - RNA, 23 nt, synthetic construct
  source 1..23: mol_type = other RNA
tagataagaaacgtctattgtgc

SEQ ID NO: 712 - RNA, 23 nt, synthetic construct
  source 1..23: mol_type = other RNA
tgatataaataacattccgcaaa

SEQ ID NO: 713 - RNA, 23 nt, synthetic construct
  source 1..23: mol_type = other RNA
tgaacaaaaaggatgtaagacag

SEQ ID NO: 714 - RNA, 23 nt, synthetic construct
  source 1..23: mol_type = other RNA
tcagaagaagctgttgaagagct

SEQ ID NO: 715 - RNA, 23 nt, synthetic construct
  source 1..23: mol_type = other RNA
ttccagaagaagctgttgaagag

SEQ ID NO: 716 - RNA, 23 nt, synthetic construct
  source 1..23: mol_type = other RNA
tgaatcaaggtactgaagacggg

SEQ ID NO: 717 - RNA, 23 nt, synthetic construct
  source 1..23: mol_type = other RNA
tgtgaatcaaggtactgaagacg

SEQ ID NO: 718 - RNA, 23 nt, synthetic construct
  source 1..23: mol_type = other RNA
tgaagttgagttcaaagactgac

SEQ ID NO: 719 - RNA, 23 nt, synthetic construct
  source 1..23: mol_type = other RNA
tagaaaggtgatgaattgctggt

SEQ ID NO: 720 - RNA, 23 nt, synthetic construct
  source 1..23: mol_type = other RNA
tacttactgagatttcacctata

SEQ ID NO: 721 - RNA, 23 nt, synthetic construct
  source 1..23: mol_type = other RNA
taataacttactgagatttcacc

SEQ ID NO: 722 - RNA, 21 nt, synthetic construct
  source 1..21: mol_type = other RNA
  modified_base 1: mod_base = OTHER; note = 2'-O-methyladenosine-3'-phosphorothioate
  modified_base 2: mod_base = OTHER; note = 2'-O-methylcytidine-3'-phosphorothioate
  modified_base 3: mod_base = OTHER; note = 2'-O-methyladenosine-3'-phosphate
  modified_base 4: mod_base = OTHER; note = 2'-O-methyladenosine-3'-phosphate
  modified_base 5: mod_base = OTHER; note = 2'-O-methyluridine-3'-phosphate
  modified_base 6: mod_base = OTHER; note = 2'-O-methyladenosine-3'-phosphate
  modified_base 7: mod_base = OTHER; note = 2'-deoxy-2'-fluoroguanosine-3'-phosphate
  modified_base 8: mod_base = OTHER; note = 2'-O-methyladenosine-3'-phosphate
  modified_base 9: mod_base = OTHER; note = 2'-deoxy-2'-fluorocytidine-3'-phosphate
  modified_base 10: mod_base = OTHER; note = 2'-deoxy-2'-fluoroguanosine-3'-phosphate
  modified_base 11: mod_base = OTHER; note = 2'-deoxy-2'-fluorouridine-3'-phosphate
  modified_base 12: mod_base = OTHER; note = 2'-O-methyluridine-3'-phosphate
  modified_base 13: mod_base = OTHER; note = 2'-O-methyluridine-3'-phosphate
  modified_base 14: mod_base = OTHER; note = 2'-O-methylcytidine-3'-phosphate
  modified_base 15: mod_base = OTHER; note = 2'-O-methyluridine-3'-phosphate
  modified_base 16: mod_base = OTHER; note = 2'-O-methyluridine-3'-phosphate
  modified_base 17: mod_base = OTHER; note = 2'-O-methyladenosine-3'-phosphate
  modified_base 18: mod_base = OTHER; note = 2'-O-methyluridine-3'-phosphate
  modified_base 19: mod_base = OTHER; note = 2'-O-methylcytidine-3'-phosphate
  modified_base 20: mod_base = OTHER; note = 2'-O-methyluridine-3'-phosphate
  modified_base 21: mod_base = OTHER; note = 2'-O-methyladenosine-3'-phosphate ((2S,4R)-1-[29-[[2-(acetylamino)-2-deoxy-beta-D-galactopyranosyl]oxy]-14,14-bis[[3-[[3-[[5-[[2-(acetylamino)-2-deoxy-beta-D-galactopyranosyl]oxy]-1-oxopentyl]amino]propyl]amino]-3-oxopropoxy]methyl]-1,12,19,25-tetraoxo-16-oxa-13,20,24-triazanonacos-1-yl]-4-hydroxy-2-pyrrolidinyl)methyl ester
acaatagacgtttcttatcta

SEQ ID NO: 723 - RNA, 21 nt, synthetic construct
  source 1..21: mol_type = other RNA
  modified_base 1: mod_base = OTHER; note = 2'-O-methyluridine-3'-phosphorothioate
  modified_base 2: mod_base = OTHER; note = 2'-O-methylguanosine-3'-phosphorothioate
  modified_base 3: mod_base = OTHER; note = 2'-O-methylcytidine-3'-phosphate
  modified_base 4: mod_base = OTHER; note = 2'-O-methylguanosine-3'-phosphate
  modified_base 5: mod_base = OTHER; note = 2'-O-methylguanosine-3'-phosphate
  modified_base 6: mod_base = OTHER; note = 2'-O-methyladenosine-3'-phosphate
  modified_base 7: mod_base = OTHER; note = 2'-deoxy-2'-fluoroadenosine-3'-phosphate
  modified_base 8: mod_base = OTHER; note = 2'-O-methyluridine-3'-phosphate
  modified_base 9: mod_base = OTHER; note = 2'-deoxy-2'-fluoroguanosine-3'-phosphate
  modified_base 10: mod_base = OTHER; note = 2'-deoxy-2'-fluorouridine-3'-phosphate
  modified_base 11: mod_base = OTHER; note = 2'-deoxy-2'-fluorouridine-3'-phosphate
  modified_base 12: mod_base = OTHER; note = 2'-O-methyladenosine-3'-phosphate
  modified_base 13: mod_base = OTHER; note = 2'-O-methyluridine-3'-phosphate
  modified_base 14: mod_base = OTHER; note = 2'-O-methyluridine-3'-phosphate
  modified_base 15: mod_base = OTHER; note = 2'-O-methyluridine-3'-phosphate
  modified_base 16: mod_base = OTHER; note = 2'-O-methyladenosine-3'-phosphate
  modified_base 17: mod_base = OTHER; note = 2'-O-methyluridine-3'-phosphate
  modified_base 18: mod_base = OTHER; note = 2'-O-methyladenosine-3'-phosphate
  modified_base 19: mod_base = OTHER; note = 2'-O-methyluridine-3'-phosphate
  modified_base 20: mod_base = OTHER; note = 2'-O-methylcytidine-3'-phosphate
  modified_base 21: mod_base = OTHER; note = 2'-O-methyladenosine-3'-phosphate ((2S,4R)-1-[29-[[2-(acetylamino)-2-deoxy-beta-D-galactopyranosyl]oxy]-14,14-bis[[3-[[3-[[5-[[2-(acetylamino)-2-deoxy-beta-D-galactopyranosyl]oxy]-1-oxopentyl]amino]propyl]amino]-3-oxopropoxy]methyl]-1,12,19,25-tetraoxo-16-oxa-13,20,24-triazanonacos-1-yl]-4-hydroxy-2-pyrrolidinyl)methyl ester
tgcggaatgttatttatatca

SEQ ID NO: 724 - RNA, 21 nt, synthetic construct
  source 1..21: mol_type = other RNA
  modified_base 1: mod_base = OTHER; note = 2'-O-methylguanosine-3'-phosphorothioate
  modified_base 2: mod_base = OTHER; note = 2'-O-methyluridine-3'-phosphorothioate
  modified_base 3: mod_base = OTHER; note = 2'-O-methylcytidine-3'-phosphate
  modified_base 4: mod_base = OTHER; note = 2'-O-methyluridine-3'-phosphate
  modified_base 5: mod_base = OTHER; note = 2'-O-methyluridine-3'-phosphate
  modified_base 6: mod_base = OTHER; note = 2'-O-methyladenosine-3'-phosphate
  modified_base 7: mod_base = OTHER; note = 2'-deoxy-2'-fluorocytidine-3'-phosphate
  modified_base 8: mod_base = OTHER; note = 2'-O-methyladenosine-3'-phosphate
  modified_base 9: mod_base = OTHER; note = 2'-deoxy-2'-fluorouridine-3'-phosphate
  modified_base 10: mod_base = OTHER; note = 2'-deoxy-2'-fluorocytidine-3'-phosphate
  modified_base 11: mod_base = OTHER; note = 2'-deoxy-2'-fluorocytidine-3'-phosphate
  modified_base 12: mod_base = OTHER; note = 2'-O-methyluridine-3'-phosphate
  modified_base 13: mod_base = OTHER; note = 2'-O-methyluridine-3'-phosphate
  modified_base 14: mod_base = OTHER; note = 2'-O-methyluridine-3'-phosphate
  modified_base 15: mod_base = OTHER; note = 2'-O-methyluridine-3'-phosphate
  modified_base 16: mod_base = OTHER; note = 2'-O-methyluridine-3'-phosphate
  modified_base 17: mod_base = OTHER; note = 2'-O-methylguanosine-3'-phosphate
  modified_base 18: mod_base = OTHER; note = 2'-O-methyluridine-3'-phosphate
  modified_base 19: mod_base = OTHER; note = 2'-O-methyluridine-3'-phosphate
  modified_base 20: mod_base = OTHER; note = 2'-O-methylcytidine-3'-phosphate
  modified_base 21: mod_base = OTHER; note = 2'-O-methyladenosine-3'-phosphate ((2S,4R)-1-[29-[[2-(acetylamino)-2-deoxy-beta-D-galactopyranosyl]oxy]-14,14-bis[[3-[[3-[[5-[[2-(acetylamino)-2-deoxy-beta-D-galactopyranosyl]oxy]-1-oxopentyl]amino]propyl]amino]-3-oxopropoxy]methyl]-1,12,19,25-tetraoxo-16-oxa-13,20,24-triazanonacos-1-yl]-4-hydroxy-2-pyrrolidinyl)methyl ester
gtcttacatcctttttgttca

SEQ ID NO: 725 - RNA, 21 nt, synthetic construct
  source 1..21: mol_type = other RNA
  modified_base 1: mod_base = OTHER; note = 2'-O-methylcytidine-3'-phosphorothioate
  modified_base 2: mod_base = OTHER; note = 2'-O-methyluridine-3'-phosphorothioate
  modified_base 3: mod_base = OTHER; note = 2'-O-methylcytidine-3'-phosphate
  modified_base 4: mod_base = OTHER; note = 2'-O-methyluridine-3'-phosphate
  modified_base 5: mod_base = OTHER; note = 2'-O-methyluridine-3'-phosphate
  modified_base 6: mod_base = OTHER; note = 2'-O-methylcytidine-3'-phosphate
  modified_base 7: mod_base = OTHER; note = 2'-deoxy-2'-fluoroadenosine-3'-phosphate
  modified_base 8: mod_base = OTHER; note = 2'-O-methyladenosine-3'-phosphate
  modified_base 9: mod_base = OTHER; note = 2'-deoxy-2'-fluorocytidine-3'-phosphate
  modified_base 10: mod_base = OTHER; note = 2'-deoxy-2'-fluoroadenosine-3'-phosphate
  modified_base 11: mod_base = OTHER; note = 2'-deoxy-2'-fluoroguanosine-3'-phosphate
  modified_base 12: mod_base = OTHER; note = 2'-O-methylcytidine-3'-phosphate
  modified_base 13: mod_base = OTHER; note = 2'-O-methyluridine-3'-phosphate
  modified_base 14: mod_base = OTHER; note = 2'-O-methyluridine-3'-phosphate
  modified_base 15: mod_base = OTHER; note = 2'-O-methylcytidine-3'-phosphate
  modified_base 16: mod_base = OTHER; note = 2'-O-methyluridine-3'-phosphate
  modified_base 17: mod_base = OTHER; note = 2'-O-methyluridine-3'-phosphate
  modified_base 18: mod_base = OTHER; note = 2'-O-methylcytidine-3'-phosphate
  modified_base 19: mod_base = OTHER; note = 2'-O-methyluridine-3'-phosphate
  modified_base 20: mod_base = OTHER; note = 2'-O-methylguanosine-3'-phosphate
  modified_base 21: mod_base = OTHER; note = 2'-O-methyladenosine-3'-phosphate ((2S,4R)-1-[29-[[2-(acetylamino)-2-deoxy-beta-D-galactopyranosyl]oxy]-14,14-bis[[3-[[3-[[5-[[2-(acetylamino)-2-deoxy-beta-D-galactopyranosyl]oxy]-1-oxopentyl]amino]propyl]amino]-3-oxopropoxy]methyl]-1,12,19,25-tetraoxo-16-oxa-13,20,24-triazanonacos-1-yl]-4-hydroxy-2-pyrrolidinyl)methyl ester
ctcttcaacagcttcttctga

SEQ ID NO: 726 - RNA, 21 nt, synthetic construct
  source 1..21: mol_type = other RNA
  modified_base 1: mod_base = OTHER; note = 2'-O-methylcytidine-3'-phosphorothioate
  modified_base 2: mod_base = OTHER; note = 2'-O-methyluridine-3'-phosphorothioate
  modified_base 3: mod_base = OTHER; note = 2'-O-methyluridine-3'-phosphate
  modified_base 4: mod_base = OTHER; note = 2'-O-methylcytidine-3'-phosphate
  modified_base 5: mod_base = OTHER; note = 2'-O-methyladenosine-3'-phosphate
  modified_base 6: mod_base = OTHER; note = 2'-O-methyladenosine-3'-phosphate
  modified_base 7: mod_base = OTHER; note = 2'-deoxy-2'-fluorocytidine-3'-phosphate
  modified_base 8: mod_base = OTHER; note = 2'-O-methyladenosine-3'-phosphate
  modified_base 9: mod_base = OTHER; note = 2'-deoxy-2'-fluoroguanosine-3'-phosphate
  modified_base 10: mod_base = OTHER; note = 2'-deoxy-2'-fluorocytidine-3'-phosphate
  modified_base 11: mod_base = OTHER; note = 2'-deoxy-2'-fluorouridine-3'-phosphate
  modified_base 12: mod_base = OTHER; note = 2'-O-methyluridine-3'-phosphate
  modified_base 13: mod_base = OTHER; note = 2'-O-methylcytidine-3'-phosphate
  modified_base 14: mod_base = OTHER; note = 2'-O-methyluridine-3'-phosphate
  modified_base 15: mod_base = OTHER; note = 2'-O-methyluridine-3'-phosphate
  modified_base 16: mod_base = OTHER; note = 2'-O-methylcytidine-3'-phosphate
  modified_base 17: mod_base = OTHER; note = 2'-O-methyluridine-3'-phosphate
  modified_base 18: mod_base = OTHER; note = 2'-O-methylguanosine-3'-phosphate
  modified_base 19: mod_base = OTHER; note = 2'-O-methylguanosine-3'-phosphate
  modified_base 20: mod_base = OTHER; note = 2'-O-methyladenosine-3'-phosphate
  modified_base 21: mod_base = OTHER; note = 2'-O-methyladenosine-3'-phosphate ((2S,4R)-1-[29-[[2-(acetylamino)-2-deoxy-beta-D-galactopyranosyl]oxy]-14,14-bis[[3-[[3-[[5-[[2-(acetylamino)-2-deoxy-beta-D-galactopyranosyl]oxy]-1-oxopentyl]amino]propyl]amino]-3-oxopropoxy]methyl]-1,12,19,25-tetraoxo-16-oxa-13,20,24-triazanonacos-1-yl]-4-hydroxy-2-pyrrolidinyl)methyl ester
cttcaacagcttcttctggaa

SEQ ID NO: 727 - RNA, 21 nt, synthetic construct
  source 1..21: mol_type = other RNA
  modified_base 1: mod_base = OTHER; note = 2'-O-methylcytidine-3'-phosphorothioate
  modified_base 2: mod_base = OTHER; note = 2'-O-methylguanosine-3'-phosphorothioate
  modified_base 3: mod_base = OTHER; note = 2'-O-methyluridine-3'-phosphate
  modified_base 4: mod_base = OTHER; note = 2'-O-methylcytidine-3'-phosphate
  modified_base 5: mod_base = OTHER; note = 2'-O-methyluridine-3'-phosphate
  modified_base 6: mod_base = OTHER; note = 2'-O-methyluridine-3'-phosphate
  modified_base 7: mod_base = OTHER; note = 2'-deoxy-2'-fluorocytidine-3'-phosphate
  modified_base 8: mod_base = OTHER; note = 2'-O-methyladenosine-3'-phosphate
  modified_base 9: mod_base = OTHER; note = 2'-deoxy-2'-fluoroguanosine-3'-phosphate
  modified_base 10: mod_base = OTHER; note = 2'-deoxy-2'-fluorouridine-3'-phosphate
  modified_base 11: mod_base = OTHER; note = 2'-deoxy-2'-fluoroadenosine-3'-phosphate
  modified_base 12: mod_base = OTHER; note = 2'-O-methylcytidine-3'-phosphate
  modified_base 13: mod_base = OTHER; note = 2'-O-methylcytidine-3'-phosphate
  modified_base 14: mod_base = OTHER; note = 2'-O-methyluridine-3'-phosphate
  modified_base 15: mod_base = OTHER; note = 2'-O-methyluridine-3'-phosphate
  modified_base 16: mod_base = OTHER; note = 2'-O-methylguanosine-3'-phosphate
  modified_base 17: mod_base = OTHER; note = 2'-O-methyladenosine-3'-phosphate
  modified_base 18: mod_base = OTHER; note = 2'-O-methyluridine-3'-phosphate
  modified_base 19: mod_base = OTHER; note = 2'-O-methyluridine-3'-phosphate
  modified_base 20: mod_base = OTHER; note = 2'-O-methylcytidine-3'-phosphate
  modified_base 21: mod_base = OTHER; note = 2'-O-methyladenosine-3'-phosphate ((2S,4R)-1-[29-[[2-(acetylamino)-2-deoxy-beta-D-galactopyranosyl]oxy]-14,14-bis[[3-[[3-[[5-[[2-(acetylamino)-2-deoxy-beta-D-galactopyranosyl]oxy]-1-oxopentyl]amino]propyl]amino]-3-oxopropoxy]methyl]-1,12,19,25-tetraoxo-16-oxa-13,20,24-triazanonacos-1-yl]-4-hydroxy-2-pyrrolidinyl)methyl ester
cgtcttcagtaccttgattca

SEQ ID NO: 728 - RNA, 21 nt, synthetic construct
  source 1..21: mol_type = other RNA
  modified_base 1: mod_base = OTHER; note = 2'-O-methyluridine-3'-phosphorothioate
  modified_base 2: mod_base = OTHER; note = 2'-O-methylcytidine-3'-phosphorothioate
  modified_base 3: mod_base = OTHER; note = 2'-O-methyluridine-3'-phosphate
  modified_base 4: mod_base = OTHER; note = 2'-O-methyluridine-3'-phosphate
  modified_base 5: mod_base = OTHER; note = 2'-O-methylcytidine-3'-phosphate
  modified_base 6: mod_base = OTHER; note = 2'-O-methyladenosine-3'-phosphate
  modified_base 7: mod_base = OTHER; note = 2'-deoxy-2'-fluoroguanosine-3'-phosphate
  modified_base 8: mod_base = OTHER; note = 2'-O-methyluridine-3'-phosphate
  modified_base 9: mod_base = OTHER; note = 2'-deoxy-2'-fluoroadenosine-3'-phosphate
  modified_base 10: mod_base = OTHER; note = 2'-deoxy-2'-fluorocytidine-3'-phosphate
  modified_base 11: mod_base = OTHER; note = 2'-deoxy-2'-fluorocytidine-3'-phosphate
  modified_base 12: mod_base = OTHER; note = 2'-O-methyluridine-3'-phosphate
  modified_base 13: mod_base = OTHER; note = 2'-O-methyluridine-3'-phosphate
  modified_base 14: mod_base = OTHER; note = 2'-O-methylguanosine-3'-phosphate
  modified_base 15: mod_base = OTHER; note = 2'-O-methyladenosine-3'-phosphate
  modified_base 16: mod_base = OTHER; note = 2'-O-methyluridine-3'-phosphate
  modified_base 17: mod_base = OTHER; note = 2'-O-methyluridine-3'-phosphate
  modified_base 18: mod_base = OTHER; note = 2'-O-methylcytidine-3'-phosphate
  modified_base 19: mod_base = OTHER; note = 2'-O-methyladenosine-3'-phosphate
  modified_base 20: mod_base = OTHER; note = 2'-O-methylcytidine-3'-phosphate
  modified_base 21: mod_base = OTHER; note = 2'-O-methyladenosine-3'-phosphate ((2S,4R)-1-[29-[[2-(acetylamino)-2-deoxy-beta-D-galactopyranosyl]oxy]-14,14-bis[[3-[[3-[[5-[[2-(acetylamino)-2-deoxy-beta-D-galactopyranosyl]oxy]-1-oxopentyl]amino]propyl]amino]-3-oxopropoxy]methyl]-1,12,19,25-tetraoxo-16-oxa-13,20,24-triazanonacos-1-yl]-4-hydroxy-2-pyrrolidinyl)methyl ester
tcttcagtaccttgattcaca

SEQ ID NO: 729 - RNA, 21 nt, synthetic construct
  source 1..21: mol_type = other RNA
  modified_base 1: mod_base = OTHER; note = 2'-O-methylcytidine-3'-phosphorothioate
  modified_base 2: mod_base = OTHER; note = 2'-O-methyladenosine-3'-phosphorothioate
  modified_base 3: mod_base = OTHER; note = 2'-O-methylguanosine-3'-phosphate
  modified_base 4: mod_base = OTHER; note = 2'-O-methyluridine-3'-phosphate
  modified_base 5: mod_base = OTHER; note = 2'-O-methylcytidine-3'-phosphate
  modified_base 6: mod_base = OTHER; note = 2'-O-methyluridine-3'-phosphate
  modified_base 7: mod_base = OTHER; note = 2'-deoxy-2'-fluorouridine-3'-phosphate
  modified_base 8: mod_base = OTHER; note = 2'-O-methyluridine-3'-phosphate
  modified_base 9: mod_base = OTHER; note = 2'-deoxy-2'-fluoroguanosine-3'-phosphate
  modified_base 10: mod_base = OTHER; note = 2'-deoxy-2'-fluoroadenosine-3'-phosphate
  modified_base 11: mod_base = OTHER; note = 2'-deoxy-2'-fluoroadenosine-3'-phosphate
  modified_base 12: mod_base = OTHER; note = 2'-O-methylcytidine-3'-phosphate
  modified_base 13: mod_base = OTHER; note = 2'-O-methyluridine-3'-phosphate
  modified_base 14: mod_base = OTHER; note = 2'-O-methylcytidine-3'-phosphate
  modified_base 15: mod_base = OTHER; note = 2'-O-methyladenosine-3'-phosphate
  modified_base 16: mod_base = OTHER; note = 2'-O-methyladenosine-3'-phosphate
  modified_base 17: mod_base = OTHER; note = 2'-O-methylcytidine-3'-phosphate
  modified_base 18: mod_base = OTHER; note = 2'-O-methyluridine-3'-phosphate
  modified_base 19: mod_base = OTHER; note = 2'-O-methyluridine-3'-phosphate
  modified_base 20: mod_base = OTHER; note = 2'-O-methylcytidine-3'-phosphate
  modified_base 21: mod_base = OTHER; note = 2'-O-methyladenosine-3'-phosphate ((2S,4R)-1-[29-[[2-(acetylamino)-2-deoxy-beta-D-galactopyranosyl]oxy]-14,14-bis[[3-[[3-[[5-[[2-(acetylamino)-2-deoxy-beta-D-galactopyranosyl]oxy]-1-oxopentyl]amino]propyl]amino]-3-oxopropoxy]methyl]-1,12,19,25-tetraoxo-16-oxa-13,20,24-triazanonacos-1-yl]-4-hydroxy-2-pyrrolidinyl)methyl ester
cagtctttgaactcaacttca

SEQ ID NO: 730 - RNA, 21 nt, synthetic construct
  source 1..21: mol_type = other RNA
  modified_base 1: mod_base = OTHER; note = 2'-O-methylcytidine-3'-phosphorothioate
  modified_base 2: mod_base = OTHER; note = 2'-O-methyladenosine-3'-phosphorothioate
  modified_base 3: mod_base = OTHER; note = 2'-O-methylguanosine-3'-phosphate
  modified_base 4: mod_base = OTHER; note = 2'-O-methylcytidine-3'-phosphate
  modified_base 5: mod_base = OTHER; note = 2'-O-methyladenosine-3'-phosphate
  modified_base 6: mod_base = OTHER; note = 2'-O-methyladenosine-3'-phosphate
  modified_base 7: mod_base = OTHER; note = 2'-deoxy-2'-fluorouridine-3'-phosphate
  modified_base 8: mod_base = OTHER; note = 2'-O-methyluridine-3'-phosphate
  modified_base 9: mod_base = OTHER; note = 2'-deoxy-2'-fluorocytidine-3'-phosphate
  modified_base 10: mod_base = OTHER; note = 2'-deoxy-2'-fluoroadenosine-3'-phosphate
  modified_base 11: mod_base = OTHER; note = 2'-deoxy-2'-fluorouridine-3'-phosphate
  modified_base 12: mod_base = OTHER; note = 2'-O-methylcytidine-3'-phosphate
  modified_base 13: mod_base = OTHER; note = 2'-O-methyladenosine-3'-phosphate
  modified_base 14: mod_base = OTHER; note = 2'-O-methylcytidine-3'-phosphate
  modified_base 15: mod_base = OTHER; note = 2'-O-methylcytidine-3'-phosphate
  modified_base 16: mod_base = OTHER; note = 2'-O-methyluridine-3'-phosphate
  modified_base 17: mod_base = OTHER; note = 2'-O-methyluridine-3'-phosphate
  modified_base 18: mod_base = OTHER; note = 2'-O-methyluridine-3'-phosphate
  modified_base 19: mod_base = OTHER; note = 2'-O-methylcytidine-3'-phosphate
  modified_base 20: mod_base = OTHER; note = 2'-O-methyluridine-3'-phosphate
  modified_base 21: mod_base = OTHER; note = 2'-O-methyladenosine-3'-phosphate ((2S,4R)-1-[29-[[2-(acetylamino)-2-deoxy-beta-D-galactopyranosyl]oxy]-14,14-bis[[3-[[3-[[5-[[2-(acetylamino)-2-deoxy-beta-D-galactopyranosyl]oxy]-1-oxopentyl]amino]propyl]amino]-3-oxopropoxy]methyl]-1,12,19,25-tetraoxo-16-oxa-13,20,24-triazanonacos-1-yl]-4-hydroxy-2-pyrrolidinyl)methyl ester
cagcaattcatcacctttcta

SEQ ID NO: 731 - RNA, 21 nt, synthetic construct
  source 1..21: mol_type = other RNA
  modified_base 1: mod_base = OTHER; note = 2'-O-methyluridine-3'-phosphorothioate
  modified_base 2: mod_base = OTHER; note = 2'-O-methyladenosine-3'-phosphorothioate
  modified_base 3: mod_base = OTHER; note = 2'-O-methylguanosine-3'-phosphate
  modified_base 4: mod_base = OTHER; note = 2'-O-methylguanosine-3'-phosphate
  modified_base 5: mod_base = OTHER; note = 2'-O-methyluridine-3'-phosphate
  modified_base 6: mod_base = OTHER; note = 2'-O-methylguanosine-3'-phosphate
  modified_base 7: mod_base = OTHER; note = 2'-deoxy-2'-fluoroadenosine-3'-phosphate
  modified_base 8: mod_base = OTHER; note = 2'-O-methyladenosine-3'-phosphate
  modified_base 9: mod_base = OTHER; note = 2'-deoxy-2'-fluoroadenosine-3'-phosphate
  modified_base 10: mod_base = OTHER; note = 2'-deoxy-2'-fluorouridine-3'-phosphate
  modified_base 11: mod_base = OTHER; note = 2'-deoxy-2'-fluorocytidine-3'-phosphate
  modified_base 12: mod_base = OTHER; note = 2'-O-methyluridine-3'-phosphate
  modified_base 13: mod_base = OTHER; note = 2'-O-methylcytidine-3'-phosphate
  modified_base 14: mod_base = OTHER; note = 2'-O-methyladenosine-3'-phosphate
  modified_base 15: mod_base = OTHER; note = 2'-O-methylguanosine-3'-phosphate
  modified_base 16: mod_base = OTHER; note = 2'-O-methyluridine-3'-phosphate
  modified_base 17: mod_base = OTHER; note = 2'-O-methyladenosine-3'-phosphate
  modified_base 18: mod_base = OTHER; note = 2'-O-methyladenosine-3'-phosphate
  modified_base 19: mod_base = OTHER; note = 2'-O-methylguanosine-3'-phosphate
  modified_base 20: mod_base = OTHER; note = 2'-O-methyluridine-3'-phosphate
  modified_base 21: mod_base = OTHER; note = 2'-O-methyladenosine-3'-phosphate ((2S,4R)-1-[29-[[2-(acetylamino)-2-deoxy-beta-D-galactopyranosyl]oxy]-14,14-bis[[3-[[3-[[5-[[2-(acetylamino)-2-deoxy-beta-D-galactopyranosyl]oxy]-1-oxopentyl]amino]propyl]amino]-3-oxopropoxy]methyl]-1,12,19,25-tetraoxo-16-oxa-13,20,24-triazanonacos-1-yl]-4-hydroxy-2-pyrrolidinyl)methyl ester
taggtgaaatctcagtaagta

SEQ ID NO: 732 - RNA, 21 nt, synthetic construct
  source 1..21: mol_type = other RNA
  modified_base 1: mod_base = OTHER; note = 2'-O-methyluridine-3'-phosphorothioate
  modified_base 2: mod_base = OTHER; note = 2'-O-methylguanosine-3'-phosphorothioate
  modified_base 3: mod_base = OTHER; note = 2'-O-methyladenosine-3'-phosphate
  modified_base 4: mod_base = OTHER; note = 2'-O-methyladenosine-3'-phosphate
  modified_base 5: mod_base = OTHER; note = 2'-O-methyladenosine-3'-phosphate
  modified_base 6: mod_base = OTHER; note = 2'-O-methyluridine-3'-phosphate
  modified_base 7: mod_base = OTHER; note = 2'-deoxy-2'-fluorocytidine-3'-phosphate
  modified_base 8: mod_base = OTHER; note = 2'-O-methyluridine-3'-phosphate
  modified_base 9: mod_base = OTHER; note = 2'-deoxy-2'-fluorocytidine-3'-phosphate
  modified_base 10: mod_base = OTHER; note = 2'-deoxy-2'-fluoroadenosine-3'-phosphate
  modified_base 11: mod_base = OTHER; note = 2'-deoxy-2'-fluoroguanosine-3'-phosphate
  modified_base 12: mod_base = OTHER; note = 2'-O-methyluridine-3'-phosphate
  modified_base 13: mod_base = OTHER; note = 2'-O-methyladenosine-3'-phosphate
  modified_base 14: mod_base = OTHER; note = 2'-O-methyladenosine-3'-phosphate
  modified_base 15: mod_base = OTHER; note = 2'-O-methylguanosine-3'-phosphate
  modified_base 16: mod_base = OTHER; note = 2'-O-methyluridine-3'-phosphate
  modified_base 17: mod_base = OTHER; note = 2'-O-methyluridine-3'-phosphate
  modified_base 18: mod_base = OTHER; note = 2'-O-methyladenosine-3'-phosphate
  modified_base 19: mod_base = OTHER; note = 2'-O-methyluridine-3'-phosphate
  modified_base 20: mod_base = OTHER; note = 2'-O-methyluridine-3'-phosphate
  modified_base 21: mod_base = OTHER; note = 2'-O-methyladenosine-3'-phosphate ((2S,4R)-1-[29-[[2-(acetylamino)-2-deoxy-beta-D-galactopyranosyl]oxy]-14,14-bis[[3-[[3-[[5-[[2-(acetylamino)-2-deoxy-beta-D-galactopyranosyl]oxy]-1-oxopentyl]amino]propyl]amino]-3-oxopropoxy]methyl]-1,12,19,25-tetraoxo-16-oxa-13,20,24-triazanonacos-1-yl]-4-hydroxy-2-pyrrolidinyl)methyl ester
tgaaatctcagtaagttatta

SEQ ID NO: 733 - RNA, 23 nt, synthetic construct
  source 1..23: mol_type = other RNA
  modified_base 1: mod_base = OTHER; note = 2'-O-methyluridine-3'-phosphorothioate 5'-(E)-Vinylphosphonate
  modified_base 2: mod_base = OTHER; note = 2'-deoxy-2'-fluoroadenosine-3'-phosphorothioate
  modified_base 3: mod_base = OTHER; note = 2'-O-methylguanosine-3'-phosphate
  modified_base 4: mod_base = OTHER; note = 2'-O-methyladenosine-3'-phosphate
  modified_base 5: mod_base = OTHER; note = 2'-O-methyluridine-3'-phosphate
  modified_base 6: mod_base = OTHER; note = 2'-deoxy-2'-fluoroadenosine-3'-phosphate
  modified_base 7: mod_base = OTHER; note = 2'-O-methyladenosine-3'-phosphate
  modified_base 8: mod_base = OTHER; note = 2'-deoxy-2'-fluoroguanosine-3'-phosphate
  modified_base 9: mod_base = OTHER; note = 2'-deoxy-2'-fluoroadenosine-3'-phosphate
  modified_base 10: mod_base = OTHER; note = 2'-O-methyladenosine-3'-phosphate
  modified_base 11: mod_base = OTHER; note = 2'-O-methyladenosine-3'-phosphate
  modified_base 12: mod_base = OTHER; note = 2'-O-methylcytidine-3'-phosphate
  modified_base 13: mod_base = OTHER; note = 2'-O-methylguanosine-3'-phosphate
  modified_base 14: mod_base = OTHER; note = 2'-deoxy-2'-fluorouridine-3'-phosphate
  modified_base 15: mod_base = OTHER; note = 2'-O-methylcytidine-3'-phosphate
  modified_base 16: mod_base = OTHER; note = 2'-deoxy-2'-fluorouridine-3'-phosphate
  modified_base 17: mod_base = OTHER; note = 2'-O-methyladenosine-3'-phosphate
  modified_base 18: mod_base = OTHER; note = 2'-O-methyluridine-3'-phosphate
  modified_base 19: mod_base = OTHER; note = 2'-O-methyluridine-3'-phosphate
  modified_base 20: mod_base = OTHER; note = 2'-O-methylguanosine-3'-phosphate
  modified_base 21: mod_base = OTHER; note = 2'-O-methyluridine-3'-phosphorothioate
  modified_base 22: mod_base = OTHER; note = 2'-O-methylguanosine-3'-phosphorothioate
  modified_base 23: mod_base = OTHER; note = 2'-O-methylcytidine
tagataagaaacgtctattgtgc

SEQ ID NO: 734 - RNA, 23 nt, synthetic construct
  source 1..23: mol_type = other RNA
  modified_base 1: mod_base = OTHER; note = 2'-O-methyluridine-3'-phosphorothioate 5'-(E)-Vinylphosphonate
  modified_base 2: mod_base = OTHER; note = 2'-deoxy-2'-fluoroguanosine-3'-phosphorothioate
  modified_base 3: mod_base = OTHER; note = 2'-O-methyladenosine-3'-phosphate
  modified_base 4: mod_base = OTHER; note = 2'-O-methyluridine-3'-phosphate
  modified_base 5: mod_base = OTHER; note = 2'-O-methyladenosine-3'-phosphate
  modified_base 6: mod_base = OTHER; note = 2'-deoxy-2'-fluorouridine-3'-phosphate
  modified_base 7: mod_base = OTHER; note = 2'-O-methyladenosine-3'-phosphate
  modified_base 8: mod_base = OTHER; note = 2'-deoxy-2'-fluoroadenosine-3'-phosphate
  modified_base 9: mod_base = OTHER; note = 2'-deoxy-2'-fluoroadenosine-3'-phosphate
  modified_base 10: mod_base = OTHER; note = 2'-O-methyluridine-3'-phosphate
  modified_base 11: mod_base = OTHER; note = 2'-O-methyladenosine-3'-phosphate
  modified_base 12: mod_base = OTHER; note = 2'-O-methyladenosine-3'-phosphate
  modified_base 13: mod_base = OTHER; note = 2'-O-methylcytidine-3'-phosphate
  modified_base 14: mod_base = OTHER; note = 2'-deoxy-2'-fluoroadenosine-3'-phosphate
  modified_base 15: mod_base = OTHER; note = 2'-O-methyluridine-3'-phosphate
  modified_base 16: mod_base = OTHER; note = 2'-deoxy-2'-fluorouridine-3'-phosphate
  modified_base 17: mod_base = OTHER; note = 2'-O-methylcytidine-3'-phosphate
  modified_base 18: mod_base = OTHER; note = 2'-O-methylcytidine-3'-phosphate
  modified_base 19: mod_base = OTHER; note = 2'-O-methylguanosine-3'-phosphate
  modified_base 20: mod_base = OTHER; note = 2'-O-methylcytidine-3'-phosphate
  modified_base 21: mod_base = OTHER; note = 2'-O-methyladenosine-3'-phosphorothioate
  modified_base 22: mod_base = OTHER; note = 2'-O-methyladenosine-3'-phosphorothioate
  modified_base 23: mod_base = OTHER; note = 2'-O-methyladenosine
tgatataaataacattccgcaaa

SEQ ID NO: 735 - RNA, 23 nt, synthetic construct
  source 1..23: mol_type = other RNA
  modified_base 1: mod_base = OTHER; note = 2'-O-methyluridine-3'-phosphorothioate 5'-(E)-Vinylphosphonate
  modified_base 2: mod_base = OTHER; note = 2'-deoxy-2'-fluoroguanosine-3'-phosphorothioate
  modified_base 3: mod_base = OTHER; note = 2'-O-methyladenosine-3'-phosphate
  modified_base 4: mod_base = OTHER; note = 2'-O-methyladenosine-3'-phosphate
  modified_base 5: mod_base = OTHER; note = 2'-O-methylcytidine-3'-phosphate
  modified_base 6: mod_base = OTHER; note = 2'-deoxy-2'-fluoroadenosine-3'-phosphate
  modified_base 7: mod_base = OTHER; note = 2'-O-methyladenosine-3'-phosphate
  modified_base 8: mod_base = OTHER; note = 2'-deoxy-2'-fluoroadenosine-3'-phosphate
  modified_base 9: mod_base = OTHER; note = 2'-deoxy-2'-fluoroadenosine-3'-phosphate
  modified_base 10: mod_base = OTHER; note = 2'-O-methyladenosine-3'-phosphate
  modified_base 11: mod_base = OTHER; note = 2'-O-methylguanosine-3'-phosphate
  modified_base 12: mod_base = OTHER; note = 2'-O-methylguanosine-3'-phosphate
  modified_base 13: mod_base = OTHER; note = 2'-O-methyladenosine-3'-phosphate
  modified_base 14: mod_base = OTHER; note = 2'-deoxy-2'-fluorouridine-3'-phosphate
  modified_base 15: mod_base = OTHER; note = 2'-O-methylguanosine-3'-phosphate
  modified_base 16: mod_base = OTHER; note = 2'-deoxy-2'-fluorouridine-3'-phosphate
  modified_base 17: mod_base = OTHER; note = 2'-O-methyladenosine-3'-phosphate
  modified_base 18: mod_base = OTHER; note = 2'-O-methyladenosine-3'-phosphate
  modified_base 19: mod_base = OTHER; note = 2'-O-methylguanosine-3'-phosphate
  modified_base 20: mod_base = OTHER; note = 2'-O-methyladenosine-3'-phosphate
  modified_base 21: mod_base = OTHER; note = 2'-O-methylcytidine-3'-phosphorothioate
  modified_base 22: mod_base = OTHER; note = 2'-O-methyladenosine-3'-phosphorothioate
  modified_base 23: mod_base = OTHER; note = 2'-O-methylguanosine
tgaacaaaaaggatgtaagacag

SEQ ID NO: 736 - RNA, 23 nt, synthetic construct
  source 1..23: mol_type = other RNA
  modified_base 1: mod_base = OTHER; note = 2'-O-methyluridine-3'-phosphorothioate 5'-(E)-Vinylphosphonate
  modified_base 2: mod_base = OTHER; note = 2'-deoxy-2'-fluorocytidine-3'-phosphorothioate
  modified_base 3: mod_base = OTHER; note = 2'-O-methyladenosine-3'-phosphate
  modified_base 4: mod_base = OTHER; note = 2'-O-methylguanosine-3'-phosphate
  modified_base 5: mod_base = OTHER; note = 2'-O-methyladenosine-3'-phosphate
  modified_base 6: mod_base = OTHER; note = 2'-deoxy-2'-fluoroadenosine-3'-phosphate
  modified_base 7: mod_base = OTHER; note = 2'-O-methylguanosine-3'-phosphate
  modified_base 8: mod_base = OTHER; note = 2'-deoxy-2'-fluoroadenosine-3'-phosphate
  modified_base 9: mod_base = OTHER; note = 2'-deoxy-2'-fluoroadenosine-3'-phosphate
  modified_base 10: mod_base = OTHER; note = 2'-O-methylguanosine-3'-phosphate
  modified_base 11: mod_base = OTHER; note = 2'-O-methylcytidine-3'-phosphate
  modified_base 12: mod_base = OTHER; note = 2'-O-methyluridine-3'-phosphate
  modified_base 13: mod_base = OTHER; note = 2'-O-methylguanosine-3'-phosphate
  modified_base 14: mod_base = OTHER; note = 2'-deoxy-2'-fluorouridine-3'-phosphate
  modified_base 15: mod_base = OTHER; note = 2'-O-methyluridine-3'-phosphate
  modified_base 16: mod_base = OTHER; note = 2'-deoxy-2'-fluoroguanosine-3'-phosphate
  modified_base 17: mod_base = OTHER; note = 2'-O-methyladenosine-3'-phosphate
  modified_base 18: mod_base = OTHER; note = 2'-O-methyladenosine-3'-phosphate
  modified_base 19: mod_base = OTHER; note = 2'-O-methylguanosine-3'-phosphate
  modified_base 20: mod_base = OTHER; note = 2'-O-methyladenosine-3'-phosphate
  modified_base 21: mod_base = OTHER; note = 2'-O-methylguanosine-3'-phosphorothioate
  modified_base 22: mod_base = OTHER; note = 2'-O-methylcytidine-3'-phosphorothioate
  modified_base 23: mod_base = OTHER; note = 2'-O-methyluridine
tcagaagaagctgttgaagagct

SEQ ID NO: 737 - RNA, 23 nt, synthetic construct
  source 1..23: mol_type = other RNA
  modified_base 1: mod_base = OTHER; note = 2'-O-methyluridine-3'-phosphorothioate 5'-(E)-Vinylphosphonate
  modified_base 2: mod_base = OTHER; note = 2'-deoxy-2'-fluorouridine-3'-phosphorothioate
  modified_base 3: mod_base = OTHER; note = 2'-O-methylcytidine-3'-phosphate
  modified_base 4: mod_base = OTHER; note = 2'-O-methylcytidine-3'-phosphate
  modified_base 5: mod_base = OTHER; note = 2'-O-methyladenosine-3'-phosphate
  modified_base 6: mod_base = OTHER; note = 2'-deoxy-2'-fluoroguanosine-3'-phosphate
  modified_base 7: mod_base = OTHER; note = 2'-O-methyladenosine-3'-phosphate
  modified_base 8: mod_base = OTHER; note = 2'-deoxy-2'-fluoroadenosine-3'-phosphate
  modified_base 9: mod_base = OTHER; note = 2'-deoxy-2'-fluoroguanosine-3'-phosphate
  modified_base 10: mod_base = OTHER; note = 2'-O-methyladenosine-3'-phosphate
  modified_base 11: mod_base = OTHER; note = 2'-O-methyladenosine-3'-phosphate
  modified_base 12: mod_base = OTHER; note = 2'-O-methylguanosine-3'-phosphate
  modified_base 13: mod_base = OTHER; note = 2'-O-methylcytidine-3'-phosphate
  modified_base 14: mod_base = OTHER; note = 2'-deoxy-2'-fluorouridine-3'-phosphate
  modified_base 15: mod_base = OTHER; note = 2'-O-methylguanosine-3'-phosphate
  modified_base 16: mod_base = OTHER; note = 2'-deoxy-2'-fluorouridine-3'-phosphate
  modified_base 17: mod_base = OTHER; note = 2'-O-methyluridine-3'-phosphate
  modified_base 18: mod_base = OTHER; note = 2'-O-methylguanosine-3'-phosphate
  modified_base 19: mod_base = OTHER; note = 2'-O-methyladenosine-3'-phosphate
  modified_base 20: mod_base = OTHER; note = 2'-O-methyladenosine-3'-phosphate
  modified_base 21: mod_base = OTHER; note = 2'-O-methylguanosine-3'-phosphorothioate
  modified_base 22: mod_base = OTHER; note = 2'-O-methyladenosine-3'-phosphorothioate
  modified_base 23: mod_base = OTHER; note = 2'-O-methylguanosine
ttccagaagaagctgttgaagag

SEQ ID NO: 738 - RNA, 23 nt, synthetic construct
  source 1..23: mol_type = other RNA
  modified_base 1: mod_base = OTHER; note = 2'-O-methyluridine-3'-phosphorothioate 5'-(E)-Vinylphosphonate
  modified_base 2: mod_base = OTHER; note = 2'-deoxy-2'-fluoroguanosine-3'-phosphorothioate
  modified_base 3: mod_base = OTHER; note = 2'-O-methyladenosine-3'-phosphate
  modified_base 4: mod_base = OTHER; note = 2'-O-methyladenosine-3'-phosphate
  modified_base 5: mod_base = OTHER; note = 2'-O-methyluridine-3'-phosphate
  modified_base 6: mod_base = OTHER; note = 2'-deoxy-2'-fluorocytidine-3'-phosphate
  modified_base 7: mod_base = OTHER; note = 2'-O-methyladenosine-3'-phosphate
  modified_base 8: mod_base = OTHER; note = 2'-deoxy-2'-fluoroadenosine-3'-phosphate
  modified_base 9: mod_base = OTHER; note = 2'-deoxy-2'-fluoroguanosine-3'-phosphate
  modified_base 10: mod_base = OTHER; note = 2'-O-methylguanosine-3'-phosphate
  modified_base 11: mod_base = OTHER; note = 2'-O-methyluridine-3'-phosphate
  modified_base 12: mod_base = OTHER; note = 2'-O-methyladenosine-3'-phosphate
  modified_base 13: mod_base = OTHER; note = 2'-O-methylcytidine-3'-phosphate
  modified_base 14: mod_base = OTHER; note = 2'-deoxy-2'-fluorouridine-3'-phosphate
  modified_base 15: mod_base = OTHER; note = 2'-O-methylguanosine-3'-phosphate
  modified_base 16: mod_base = OTHER; note = 2'-deoxy-2'-fluoroadenosine-3'-phosphate
  modified_base 17: mod_base = OTHER; note = 2'-O-methyladenosine-3'-phosphate
  modified_base 18: mod_base = OTHER; note = 2'-O-methylguanosine-3'-phosphate
  modified_base 19: mod_base = OTHER; note = 2'-O-methyladenosine-3'-phosphate
  modified_base 20: mod_base = OTHER; note = 2'-O-methylcytidine-3'-phosphate
  modified_base 21: mod_base = OTHER; note = 2'-O-methylguanosine-3'-phosphorothioate
  modified_base 22: mod_base = OTHER; note = 2'-O-methylguanosine-3'-phosphorothioate
  modified_base 23: mod_base = OTHER; note = 2'-O-methylguanosine
tgaatcaaggtactgaagacggg

SEQ ID NO: 739 - RNA, 23 nt, synthetic construct
  source 1..23: mol_type = other RNA
  modified_base 1: mod_base = OTHER; note = 2'-O-methyluridine-3'-phosphorothioate 5'-(E)-Vinylphosphonate
  modified_base 2: mod_base = OTHER; note = 2'-deoxy-2'-fluoroguanosine-3'-phosphorothioate
  modified_base 3: mod_base = OTHER; note = 2'-O-methyluridine-3'-phosphate
  modified_base 4: mod_base = OTHER; note = 2'-O-methylguanosine-3'-phosphate
  modified_base 5: mod_base = OTHER; note = 2'-O-methyladenosine-3'-phosphate
  modified_base 6: mod_base = OTHER; note = 2'-deoxy-2'-fluoroadenosine-3'-phosphate
  modified_base 7: mod_base = OTHER; note = 2'-O-methyluridine-3'-phosphate
  modified_base 8: mod_base = OTHER; note = 2'-deoxy-2'-fluorocytidine-3'-phosphate
  modified_base 9: mod_base = OTHER; note = 2'-deoxy-2'-fluoroadenosine-3'-phosphate
  modified_base 10: mod_base = OTHER; note = 2'-O-methyladenosine-3'-phosphate
  modified_base 11: mod_base = OTHER; note = 2'-O-methylguanosine-3'-phosphate
  modified_base 12: mod_base = OTHER; note = 2'-O-methylguanosine-3'-phosphate
  modified_base 13: mod_base = OTHER; note = 2'-O-methyluridine-3'-phosphate
  modified_base 14: mod_base = OTHER; note = 2'-deoxy-2'-fluoroadenosine-3'-phosphate
  modified_base 15: mod_base = OTHER; note = 2'-O-methylcytidine-3'-phosphate
  modified_base 16: mod_base = OTHER; note = 2'-deoxy-2'-fluorouridine-3'-phosphate
  modified_base 17: mod_base = OTHER; note = 2'-O-methylguanosine-3'-phosphate
  modified_base 18: mod_base = OTHER; note = 2'-O-methyladenosine-3'-phosphate
  modified_base 19: mod_base = OTHER; note = 2'-O-methyladenosine-3'-phosphate
  modified_base 20: mod_base = OTHER; note = 2'-O-methylguanosine-3'-phosphate
  modified_base 21: mod_base = OTHER; note = 2'-O-methyladenosine-3'-phosphorothioate
  modified_base 22: mod_base = OTHER; note = 2'-O-methylcytidine-3'-phosphorothioate
  modified_base 23: mod_base = OTHER; note = 2'-O-methylguanosine
tgtgaatcaaggtactgaagacg

SEQ ID NO: 740 - RNA, 23 nt, synthetic construct
  source 1..23: mol_type = other RNA
  modified_base 1: mod_base = OTHER; note = 2'-O-methyluridine-3'-phosphorothioate 5'-(E)-Vinylphosphonate
  modified_base 2: mod_base = OTHER; note = 2'-deoxy-2'-fluoroguanosine-3'-phosphorothioate
  modified_base 3: mod_base = OTHER; note = 2'-O-methyladenosine-3'-phosphate
  modified_base 4: mod_base = OTHER; note = 2'-O-methyladenosine-3'-phosphate
  modified_base 5: mod_base = OTHER; note = 2'-O-methylguanosine-3'-phosphate
  modified_base 6: mod_base = OTHER; note = 2'-deoxy-2'-fluorouridine-3'-phosphate
  modified_base 7: mod_base = OTHER; note = 2'-O-methyluridine-3'-phosphate
  modified_base 8: mod_base = OTHER; note = 2'-deoxy-2'-fluoroguanosine-3'-phosphate
  modified_base 9: mod_base = OTHER; note = 2'-deoxy-2'-fluoroadenosine-3'-phosphate
  modified_base 10: mod_base = OTHER; note = 2'-O-methylguanosine-3'-phosphate
  modified_base 11: mod_base = OTHER; note = 2'-O-methyluridine-3'-phosphate
  modified_base 12: mod_base = OTHER; note = 2'-O-methyluridine-3'-phosphate
  modified_base 13: mod_base = OTHER; note = 2'-O-methylcytidine-3'-phosphate
  modified_base 14: mod_base = OTHER; note = 2'-deoxy-2'-fluoroadenosine-3'-phosphate
  modified_base 15: mod_base = OTHER; note = 2'-O-methyladenosine-3'-phosphate
  modified_base 16: mod_base = OTHER; note = 2'-deoxy-2'-fluoroadenosine-3'-phosphate
  modified_base 17: mod_base = OTHER; note = 2'-O-methylguanosine-3'-phosphate
  modified_base 18: mod_base = OTHER; note = 2'-O-methyladenosine-3'-phosphate
  modified_base 19: mod_base = OTHER; note = 2'-O-methylcytidine-3'-phosphate
  modified_base 20: mod_base = OTHER; note = 2'-O-methyluridine-3'-phosphate
  modified_base 21: mod_base = OTHER; note = 2'-O-methylguanosine-3'-phosphorothioate
  modified_base 22: mod_base = OTHER; note = 2'-O-methyladenosine-3'-phosphorothioate
  modified_base 23: mod_base = OTHER; note = 2'-O-methylcytidine
tgaagttgagttcaaagactgac

SEQ ID NO: 741 - RNA, 23 nt, synthetic construct
  source 1..23: mol_type = other RNA
  modified_base 1: mod_base = OTHER; note = 2'-O-methyluridine-3'-phosphorothioate 5'-(E)-Vinylphosphonate
  modified_base 2: mod_base = OTHER; note = 2'-deoxy-2'-fluoroadenosine-3'-phosphorothioate
  modified_base 3: mod_base = OTHER; note = 2'-O-methylguanosine-3'-phosphate
  modified_base 4: mod_base = OTHER; note = 2'-O-methyladenosine-3'-phosphate
  modified_base 5: mod_base = OTHER; note = 2'-O-methyladenosine-3'-phosphate
  modified_base 6: mod_base = OTHER; note = 2'-deoxy-2'-fluoroadenosine-3'-phosphate
  modified_base 7: mod_base = OTHER; note = 2'-O-methylguanosine-3'-phosphate
  modified_base 8: mod_base = OTHER; note = 2'-deoxy-2'-fluoroguanosine-3'-phosphate
  modified_base 9: mod_base = OTHER; note = 2'-deoxy-2'-fluorouridine-3'-phosphate
  modified_base 10: mod_base = OTHER; note = 2'-O-methylguanosine-3'-phosphate
  modified_base 11: mod_base = OTHER; note = 2'-O-methyladenosine-3'-phosphate
  modified_base 12: mod_base = OTHER; note = 2'-O-methyluridine-3'-phosphate
  modified_base 13: mod_base = OTHER; note = 2'-O-methylguanosine-3'-phosphate
  modified_base 14: mod_base = OTHER; note = 2'-deoxy-2'-fluoroadenosine-3'-phosphate
  modified_base 15: mod_base = OTHER; note = 2'-O-methyladenosine-3'-phosphate
  modified_base 16: mod_base = OTHER; note = 2'-deoxy-2'-fluorouridine-3'-phosphate
  modified_base 17: mod_base = OTHER; note = 2'-O-methyluridine-3'-phosphate
  modified_base 18: mod_base = OTHER; note = 2'-O-methylguanosine-3'-phosphate
  modified_base 19: mod_base = OTHER; note = 2'-O-methylcytidine-3'-phosphate
  modified_base 20: mod_base = OTHER; note = 2'-O-methyluridine-3'-phosphate
  modified_base 21: mod_base = OTHER; note = 2'-O-methylguanosine-3'-phosphorothioate
  modified_base 22: mod_base = OTHER; note = 2'-O-methylguanosine-3'-phosphorothioate
  modified_base 23: mod_base = OTHER; note = 2'-O-methyluridine
tagaaaggtgatgaattgctggt

SEQ ID NO: 742 - RNA, 23 nt, synthetic construct
  source 1..23: mol_type = other RNA
  modified_base 1: mod_base = OTHER; note = 2'-O-methyluridine-3'-phosphorothioate 5'-(E)-Vinylphosphonate
  modified_base 2: mod_base = OTHER; note = 2'-deoxy-2'-fluoroadenosine-3'-phosphorothioate
  modified_base 3: mod_base = OTHER; note = 2'-O-methylcytidine-3'-phosphate
  modified_base 4: mod_base = OTHER; note = 2'-O-methyluridine-3'-phosphate
  modified_base 5: mod_base = OTHER; note = 2'-O-methyluridine-3'-phosphate
  modified_base 6: mod_base = OTHER; note = 2'-deoxy-2'-fluoroadenosine-3'-phosphate
  modified_base 7: mod_base = OTHER; note = 2'-O-methylcytidine-3'-phosphate
  modified_base 8: mod_base = OTHER; note = 2'-deoxy-2'-fluorouridine-3'-phosphate
  modified_base 9: mod_base = OTHER; note = 2'-deoxy-2'-fluoroguanosine-3'-phosphate
  modified_base 10: mod_base = OTHER; note = 2'-O-methyladenosine-3'-phosphate
  modified_base 11: mod_base = OTHER; note = 2'-O-methylguanosine-3'-phosphate
  modified_base 12: mod_base = OTHER; note = 2'-O-methyladenosine-3'-phosphate
  modified_base 13: mod_base = OTHER; note = 2'-O-methyluridine-3'-phosphate
  modified_base 14: mod_base = OTHER; note = 2'-deoxy-2'-fluorouridine-3'-phosphate
  modified_base 15: mod_base = OTHER; note = 2'-O-methyluridine-3'-phosphate
  modified_base 16: mod_base = OTHER; note = 2'-deoxy-2'-fluorocytidine-3'-phosphate
  modified_base 17: mod_base = OTHER; note = 2'-O-methyladenosine-3'-phosphate
  modified_base 18: mod_base = OTHER; note = 2'-O-methylcytidine-3'-phosphate
  modified_base 19: mod_base = OTHER; note = 2'-O-methylcytidine-3'-phosphate
  modified_base 20: mod_base = OTHER; note = 2'-O-methyluridine-3'-phosphate
  modified_base 21: mod_base = OTHER; note = 2'-O-methyladenosine-3'-phosphorothioate
  modified_base 22: mod_base = OTHER; note = 2'-O-methyluridine-3'-phosphorothioate
  modified_base 23: mod_base = OTHER; note = 2'-O-methyladenosine
tacttactgagatttcacctata

SEQ ID NO: 743 - RNA, 23 nt, synthetic construct
  source 1..23: mol_type = other RNA
  modified_base 1: mod_base = OTHER; note = 2'-O-methyluridine-3'-phosphorothioate 5'-(E)-Vinylphosphonate
  modified_base 2: mod_base = OTHER; note = 2'-deoxy-2'-fluoroadenosine-3'-phosphorothioate
  modified_base 3: mod_base = OTHER; note = 2'-O-methyladenosine-3'-phosphate
  modified_base 4: mod_base = OTHER; note = 2'-O-methyluridine-3'-phosphate
  modified_base 5: mod_base = OTHER; note = 2'-O-methyladenosine-3'-phosphate
  modified_base 6: mod_base = OTHER; note = 2'-deoxy-2'-fluoroadenosine-3'-phosphate
  modified_base 7: mod_base = OTHER; note = 2'-O-methylcytidine-3'-phosphate
  modified_base 8: mod_base = OTHER; note = 2'-deoxy-2'-fluorouridine-3'-phosphate
  modified_base 9: mod_base = OTHER; note = 2'-deoxy-2'-fluorouridine-3'-phosphate
  modified_base 10: mod_base = OTHER; note = 2'-O-methyladenosine-3'-phosphate
  modified_base 11: mod_base = OTHER; note = 2'-O-methylcytidine-3'-phosphate
  modified_base 12: mod_base = OTHER; note = 2'-O-methyluridine-3'-phosphate
  modified_base 13: mod_base = OTHER; note = 2'-O-methylguanosine-3'-phosphate
  modified_base 14: mod_base = OTHER; note = 2'-deoxy-2'-fluoroadenosine-3'-phosphate
  modified_base 15: mod_base = OTHER; note = 2'-O-methylguanosine-3'-phosphate
  modified_base 16: mod_base = OTHER; note = 2'-deoxy-2'-fluoroadenosine-3'-phosphate
  modified_base 17: mod_base = OTHER; note = 2'-O-methyluridine-3'-phosphate
  modified_base 18: mod_base = OTHER; note = 2'-O-methyluridine-3'-phosphate
  modified_base 19: mod_base = OTHER; note = 2'-O-methyluridine-3'-phosphate
  modified_base 20: mod_base = OTHER; note = 2'-O-methylcytidine-3'-phosphate
  modified_base 21: mod_base = OTHER; note = 2'-O-methyladenosine-3'-phosphorothioate
  modified_base 22: mod_base = OTHER; note = 2'-O-methylcytidine-3'-phosphorothioate
  modified_base 23: mod_base = OTHER; note = 2'-O-methylcytidine
taataacttactgagatttcacc

SEQ ID NO: 744 - RNA, 23 nt, synthetic construct
  source 1..23: mol_type = other RNA
tagataagaaacgtctattgtgc

SEQ ID NO: 745 - RNA, 23 nt, synthetic construct
  source 1..23: mol_type = other RNA
tgatataaataacattccgcaaa

SEQ ID NO: 746 - RNA, 23 nt, synthetic construct
  source 1..23: mol_type = other RNA
tgaacaaaaaggatgtaagacag

SEQ ID NO: 747 - RNA, 23 nt, synthetic construct
  source 1..23: mol_type = other RNA
tcagaagaagctgttgaagagct

SEQ ID NO: 748 - RNA, 23 nt, synthetic construct
  source 1..23: mol_type = other RNA
ttccagaagaagctgttgaagag

SEQ ID NO: 749 - RNA, 23 nt, synthetic construct
  source 1..23: mol_type = other RNA
tgaatcaaggtactgaagacggg

SEQ ID NO: 750 - RNA, 23 nt, synthetic construct
  source 1..23: mol_type = other RNA
tgtgaatcaaggtactgaagacg

SEQ ID NO: 751 - RNA, 23 nt, synthetic construct
  source 1..23: mol_type = other RNA
tgaagttgagttcaaagactgac

SEQ ID NO: 752 - RNA, 23 nt, synthetic construct
  source 1..23: mol_type = other RNA
tagaaaggtgatgaattgctggt

SEQ ID NO: 753 - RNA, 23 nt, synthetic construct
  source 1..23: mol_type = other RNA
tacttactgagatttcacctata

SEQ ID NO: 754 - RNA, 23 nt, synthetic construct
  source 1..23: mol_type = other RNA
taataacttactgagatttcacc